European Patent Application EP 4 417 688 A1, published August 21, 2024. Title: BACTERIOPHAGE COMPOSITION AGAINST FIRE BLIGHT. Applicant: De Ceuster Meststoffen N.V. The sequence listing filed with the application follows.

SEQUENCE LISTING (4 sequences)

SEQ ID NO: 1 - DNA, 262788 bp, unidentified
  source 1..262788: mol_type = genomic DNA
atgttttcgcttggcctggaagttcgggccattcgaactattacgaacccaaagattaaggaaggattcaggacggctatgatgggtcgtcttggtcctgcccactttagttcggaagtaactcgcaagtcattccgccgtattacaaagctggtggagtcacgtagcgaaataattgattgggaagacttgctggaagaccctaacttgacggaagagttcagggacagtctgcgtgaagcagaagaaaagccagcgaagaccatgaaaggctttgacaagatattcgatagtctggagaagtatcgccagcgtcgtgatatcatgaacctcggtaagcagattgctaaggactttagtgacgctgacccagaggagttcgacgaacaaacgtacatgcaagagctggctgataagctgggtcaagcgcagcgtggcactcgtaagactgagaaggtttggtcattcgggggcaagaagtcgaacgccatgaagttagcgaagcaggtaatcaccaacccgaaagaggtgatgtacaagactggcttcaagacgtatgacaataagaacggcggttggcctacgactggtgttgtgttgttagctggttcaacgtctgggggtaagtctgttatctcaatgaacctagctgatgcaatggcgaaagtgaacggcattcactgtctcaaggtcacactcgaaatgaccgccgagcaggaaatgaagcgtatgctttcgatgatcagcggcatcgacttctggaagattaagcagggcaagttgtcgaaacgcgagcagacgcaattgctgagagccgcgaaagactacgacaagatcatgaagaagtcgaagggacgtaactcattcacgtctcctgagcgcggtatgtcgattgatgatgttttgtgtatgtcgattccatatggcgttcacgtaaccttcatcgactatgttggtctgttggaaggtatcgacaacgacaaccagtggcgcgaactgtctacgattgttcgtaaagcgaaagtacacgcgaacgcaacaggtcagcttgttgttatcctgtgtcagcttgatgaccagactgggcgtattcgttactctggtggtatgcgtgagcacgccgacgttgtgtgggcatggaactactctgaccctgagattcgtgaaggcaaggtgattcctgttcaggtaatgaaagcgcgtgatggtgagttgttcgaaatggcgttggaagatgcgttcgaaacaatgaccgtgcgtgatgctggcgccgatgctgaaataccgaagtcaggaaaggttatcgcaactgacgatatggaaggtaagggagattccaagaagaaattcgggaaaggtaatttcaagaagaaagataaaattgagattaagaagtctcgtcgtggtgctgctgcatttctcgatgcgggtaacagtgatgacgatgacggcgacctgccgaagaaaaagaaaaagcgtaagtcttatgacgtagcttaggagtctctatggacgaaatccagtggctagtcttcgatgacgaggccaacctaaacatagacaaggattatgtctatcacgttcgcaccaaggagggtgcagagcattctggtatgtaccctaacggagctggctttcattgtcagaacccaggacagcctggtcgtgtagcaatgtccgacgtaacgcattatgctgtgcagatgacattcgatgaccatgcagataagttcgtattcggccgtgagtaacttcgaagggccgtacggactcgtcgagtctgaccagatgatcccacgctggtcgtaccctgttaagcatggacaggtacgtagagtcgaagcgtgggaactcgatactttgccaaataccacgcagcaagtacgcatggtaaatgacattcatgcaattcatagcacacctgtagaggattatgatgacgctctcgacctcgacgaagaagccgcaacgatctcaaaaactgagtcccgacttcttatcaagcctcgactcgatgaagtccgttcccgtaaaaacaaagaccacactggtccagagaacgtcttctccgtcaccgacgaagtgattgacggtgcgcttgatagcatcgactcttactctgaaactttccgggactacctgatgcaccatgtgtttagcccgatacttgggtttgacattgcagcaggtgaagttgaagcaatcgccaaagactgtctcaagacggacctagagattgacagcgagcttgtgccgtatatcgagcgcgtaggtcttgctaacatcatcggcgtaatgctgtctaagtctaactctgtaccggaacaagtacgtgctgacgtgctgaaagactggctgattaaagcattcgatgatgtacgtgcagagcataagtcgaaaggcaattctctgcgtgatcagattcgtcgtctgatgcacggcaatactgacctcgttgctaaaggagctggtatcggcacgacgcgaggattctctgaatacaggaaacagatgaccgagaatggccaagcctaagaagggcccagctttcaccttacgtcccaaacgcattgcagcctttgatgcgctgctgggcgatgacgtaaaggtggaggcttctgctgacatggacttcttgtcagacaatagttcaagtgcgattaacttcttggagaagggtgaggtaaacatcgttgacttggttgagggtgcgttagagcaacgtaccatcgtgccacgcgatttgaagtttgatgatagttcaatgcccaaggcgaaaaacttccttgagtggtgtacgagtccagacttcttaaaagccgagccgtatcttgaacaggccttgattggtctacgcttgtttggagagatttgcgttcgctgttctccagacctgcaatggcagcacactgaaaaccacgagccgcaagaaactacagccgcaatcgaggatcacttacacctgttacataatggtgtgtgccctcattgcggcgctcgtcgttctgacatgattcgcaagaaggagatgaacttctacaacgagctggctgtgaatgccggacagcgttgtgtgattgcttcgactcctgtagtaacttctcgcggcatcatgccaatcggtcatatgatgatcggacatgacacacctggcttccacaaaccgagacgcaacttcaatgcgcacaacgggcgtgagattaagaaggtcaatcaggtgtacgtgtctgacgaaagcccgaccaaagtcgtgtctctggctaatggcatgtggcttgaagcaactcatgagcaccctgtacgcactgagcaaggcttcaagaaagtgtctaagctcaaagagggcgaccgcgttgagatcaaactcggcactaacgcgtggggcaagattcaacgaccagtatctatctatgatgcaggactttcagtccgtgaagaagcactgcgttatgttgttgatcgctctctcgcaatcggcgacaagatgcagtatgtgacagaagatgcagacgcgctacagatggtgtggtcgattcttatcaatgctggatacatgcctcaagtgttgcatgacacgcgaagctggagcgttgtatacgatcataccgcagagcctgactgtcgctctgttcacattgaagtaaccgcagtcgatgaaggtacagcgcaggtcacgtatgacttgcagatggaaggactgcctcagtttgtggcttccggccttgtgcatcataacagcggtaagtctgtggtagtagcgatgatctcgacctacctgacgcatagactgcttatgtcgcagtcgcctactggcatcttgagtatcgacaacactaccgttctgcacggcacgttcgttgcgctcacccagaaacaagcgtcagatacgctatggactccttacttcaactacatcatgggcagtccttggttccaagcataccatgacctgattcgtaaacacgaacggcgctatggtatcgaggtgatgaagattcgtgatacgttcgttctgtacggacacaggaacttcgttatctatccagcagggcctgatggtcgtattcttcgtggtcgaacccgcgtattggcggtgatcgatgaagtggcgtattttgacaacgacgcccaatcgaagaaaatcaaagtcagcgcaaacgcagtatatggcgcacttgaccgttcacttgcgactgtgcgagcgaaagaacgaaggcaggtggaggcaggctacgacgaggcattcacgggttacttctgcaacatcagtagcccggtacacgctcgtgataagatcaacgagttgttgcgtatgtcagtcggcagtgagaagctgttaggcattcatgctcctacgtggaagatgaaccctgacatgccacgcgattcagagttcctgcttgaggcgttcaagcgtgaccctgttggcgcagcgcgagattacggagcagaagcacctctgtctgcaaacccgttcatcacgcagcccacgttcatcgcagacgctatccgtgagaaaggccgttcgatgtgtacctatacgcatcacatcattcgacacaaagacggtgaacgccagcgttatggttctcttgtgaaagctgcttcgacaaccagagcctcaatccttgcgatagatgcaggcttctcgaacaacagttttgcacttgtgacaggctcacgtggtgatgacggtattatcagtgttgactgtctggtggagatcgttcctaagccaggcatacctctgaactataccttaatctttgacgaactgcttatccctttatgtaaagcgcgtaacgttcgtgtaatgcttgctgaccagtggcagtcattgaagctgctgcaggatgctaaactgaaagtggactcgattgaagaatcagatcagtacagcctgaaatatcaggacatgtggactgtgaagacgatgttcgaatctactccaagtcgcatcagtctgccccgcatgacacacgctaagacgatcatggacacgctgaaatacgacggcgacgaatatccacagtgcttcgagaacaaaccaacagagcacttgatgatgcaactccagacggtgcaggatactggccgcagcgttatcaagaacacaggggcaaccgatgacctgtggcgagcaatggcactcatggtgtatggcttcgagtgtggtgagtacgacgagtatctgataaaagcgcaagaagtaacagtgaaccgtgacccaaatcgtttaggccgcgtagcacatagacttaactccggctcggctagttcgactggcagacctgcacttagtggtgggcgcgttcttggttcagctcgtactcggatgattggccgtaaataagctaatttcaatgagacagttcatacaaggaatacgatcatgaccaagcattacaacccactactgtcctcgaacactgtaaagtcagagtcgagcgacacgcatcagagcacctcggcagcgttcgtagttgagagcgctaacgtgtgccctaagtgtggctctgcaaatgtgccgacacaactactctcaggcgagggtgttatgttctgcacaggctgccgcgtaagtctcgcaatccctttgaagtgaggtatatatgggcgtccaggttggtcgtcgtcaattaggcggcgcaccctcggagcctgcaaagaagaaagaaacttctctcggcgcagcctccttaccgcgcgagataggcaaagcaatccgcagtgagagttcacgtcgtcactccgacttcgtgtctcaatctgcgggtggcgcaggaatggctgctggtaatatgcagattggttccgtccctcttgatatcgacttagagccgatgatggaaggtatggactatgatgctgacgaccgacagctattcaatgtctaccgcgatatgtatcacttcgacccaatctgcggctcctatgtggacttgttctcaacgctaccattctccgatgtgagtttcagtggcgcgaaggacagtgtgcttgagccgtactacgaagtgaatgaacgtctgtcactgaccaccagcatgccgaacatcacaaccgatattcaggttactggcgcgtttgttggctcgatgatctacaacaaagaccgtaagaagtttatcgacttgatgacgcaccgttacgacaacatcgacgtaacgccactgccgtttatcagtcaggaccctatgttcgaactgcgcatccctcagtacgtgaagtctgctttcgctaaagaaggtaaacgtattgacgcgctgaaaaaagaactcgggcctgggtttgtcgataagctcatgaacgacaccacgatggagcttgaccccatcggtacgatctacatcccgcgtaaaacgttcagctttggcgaaggtatctcggtgttacgccgtgtgctgcctatctggctgattgagaagaatctctatcgcggtacgttgattgaatctggtcgtcgtcaacgtggtatcttacatgcccagttgggtgatggagatcagtgggaaccgtcgcaagaagaaatggactttatgacagaccttcttctgtctgcggatagtgacccgattggatctatcatcacaactcgtctgggcgtgaacatcagtgagttccgtcagggcggtgacttctggaagattacggatatctgggaccagactgctcaattcaaaatgcgagcgatgggtatcagtgaagcgttcctgagtggtgaagcaaactacgactctggtgctgctggcttgactatcttcgttgaagcgatgcgagcattccgtgatcacctgacgcgtaaagtttactacgagaaagtcttcccacttatcagcatgatgaatggcctggctgttcagcgtaacggtaagatcatcaaaaagaacaacatgatggaaggcggcatggccgaagtaatgtacaagatgaatgatggctccaagctattcattccgaacgtgcattggtccaagcaactccgtcctgatgttgatcaggcgatgatggaaaacttacgtgcgatgactgaactgggtgttccagttccgttacgtgctatcgctgctgctggcgggtacaacttcgaccagattcttatggaccaggatgaagacctcgcaatgcgtcgtaagctgatggcctatcgccgacgtcagacagagatcgatcaagagttcgctcctcctgaggccggtgctggtgatggtgacagctttagctccgttagctctatgtctgctgatttgcagcgccgtcgtcgtcatgtggctggtatcggtctgtcttctgccgtgctgggaggggagcaacgtaagctgcttaaccgtgacttcggtgagcgttctgaaatcttcgaactgtccaagacaggtaagaagaaacacgtctaccgccagtctgtcgctaactcaaaagcgaacgaccagatctggaaagctgctaagaactatgaagccaacaagacgatgcctctggatgacggtaaagtgtcgttcaagccaacgccgggtgagcttcgtgctatgtcgagacttcgttaatgtacaacgtttctacgtgtccaattgacggtactgattcggtggttgtgtatcgccaccctgtctttactgacttcggtcttgggttgaagatcaatcgtagtggtgagatgcctgttgttgagtgcaacatcgtgacaggcacaatcgacggtcagtctacgcttgagaccatcagcgatcatactgcaccgctcgaagttcaagtgtggtgctttaccgggatgctaactctgcgggaatctgtaaatatgcagagcttatcattagatgccttgttcccaaataacggaggcatcgtatactaccgaccaaatcaggagagtacatcgtgagtggattgttcccgcatcgcgttatcacgcagaaagaaggtttcgtgtttatcgtccagcctgccgacgatactgatcaggatgccgtagaagcctctcaagagattgaagcgcttctggtggaagcgtggccgactgcgccgtctgagctgtctgtgaatgacgtgcgcgacccagaagaagccgagctggtattcgctgatatcatgcaactgctggaagaagcagagcgcgaagaagcacatcagatcgtaatcagtggtatcgttgttgtcggcgaactggccgtcgtaacctgtatgctgaccggcgaagatctggaaagcgacgatgaagaagacgaagacgatgattccgttgaagttgacgaagaagaattcgattaacgtctgccatgaggaccttcgggtcctcatgaatctcactgattcgaatccagcgtatgcagccaagttcctgacgaacaaaacagaggatgaagcacgtactctgctggctgcactcaataacgatgaagtaacatcactgtacgacttaatggtgacgtgatggataataccgtggacgaaagtcctaatagcgcaaggcatcgcattttcttcaagcagccgaaacgagtacctcccttcgatacagctttcattcgttcatctaatcgtgaaggtctgaaagtcctcctatcggctgcccctgaacactgtcagatcattttgtttacggacggtcccggcatcgcttatgccatgaaacgcctctttaagcgcaacttcaaactctgttcgcaagctctacaactggatttaaaaactctgtccttaactggtcaggtcgtgtatcaattcactcgtggtggagccgtgtatgacccattggctcgctacttctgtgctggtgatagctatttgcatgagctggcgcagacaacgaagttaggaagctccgagacagatacgattgacttgttctgttgcggtctggcgttccatcgcgttttacttgagcgtggccgaggtcgttctctcgtattcgcggaggaacaatgagtagatcgtttgcgtcaataggcaagacgcctgttgctggcgctataccgaagatgaagattaagtacggcgaccagcctatgctgcatgttgttgacgcatcgaactggatgtgccgtgcttacttcgcaacccaaaagagcgcaacgtatgccaaagacggaactccgacttacggcctgcgtcaattcatgtacatggtcaaagacctgatcgatattgcagcgaaagaccctaacggtcagttcattgcattctgtttcgacgttagctctgagtctacatggcgttatcgtgctatgcagcaatgggcagcggagcataagaagaagtatatccgtcaggtgtttaaaaagagtagcgactacaagggcaaccgcgatcgttctcttaccaaagagctgggtgtgcagatggcgctggcgcgtgacatactacagttggctggctactatgtagggattaaagccccttacgagtgcgatgacattgttggtacgttgagcgaccgcttcaaatatgattacctgatcaagctgtactcgcgggataaggactacgtgcaacttgttgaccacaagaacgttgagcttatcatgcaggctcagtctaatgcagccgagcgtcgcttcacgcttaaaactgccaaaggattcttcggtgttcctgccaaccgtgttattgatatgctcgcgctatctggcgatagcgtcgataacgtacctgggattcctggcattggcgataagactgctgctgagttcatcaatcgttttggtggtgctatcgaactccgagacgcactgctatctggtgagatgaagtccaatgctggttgggcgaaagcgctgacaatgcaagcgccttcaatggatattgagctgcaaatggagcttgtaactatcgaccgtaacgttccgggcttacctcgtaagatcgaagcgtttattccaggccgtccagatataaaagcgttgaaagcagttaagaaacgcctggcactgcctcaactattacacgtctaagagggtagtatgacggacaagattacgcagttggcgaagtggtatgacgctgctaaaaccgcgtttaagatgggacagcataatcctaatggtaatgctgctctgctgttgagtatattagctcgcctgaacaagaacgtggaagtggctgcacctggctccgaccacgacgctgctgaacaggaacgtgccgagtttctcgacgatcttgcggctgaggtcaagatgtacgaactcattcgcaagcgattcaacaacgacctgtacccaggcattaccgtgagcgaagacgtgaaggtgtatgttgcgctcatggctgatcgccctggtagcgctgtaatggcgatgaccttcctgcaccttgctcgttgctacacgctcaaggatatgatcattaactttctcccgaatggctttcctggtgaagacgcacttggtctcacctggagcatacagaagacggacgctggcaacttggtggatgatattgattctgtaaatagcctctatactaagatgtataactctggagataagtaatggatttatctgcattaggttacgcgccgaagccgtatcgagtgattcctgtcgaaaaagagaacctcgttactgactttattcaaggtaagttccgcgttattggtgttgagtgcaacgcccgcggtgtttacggcaacccaatccaaaagagtattgctcgtcgtttcccggaagtcatgaatcgcgtcaacgccgttgattacgaacatgaattaactatcggcaagacgcatctgattcgcgttcgtactcaagcccgtcgtgatttgtttgttgctaacatgcacatcgctcgcggctttggtctgggcctgaacggctcggttgagggctatcataagcctgtcaatcgtttcagtgaaaaattcctgacgcgggcgttcgaacatctgctggagcaatgcgataaagagaacatcgcaccagaccgacagattgctattcaacgcttctacggcggactcggcggagtttcttgggaagaggtttgtgttgtgcttgatgctatctgcgagaagcatcagttcaacatgtatgcctatctaccaaagaactacaatactaactacgtgcggggctccgcacaataactctggggtgtattgatgaacacaatacgcggatttgattggctcttttacggagatggaaccgatagtggccaacactcaattgtaagtatcgttgtcgaacaggcatcgaaatcaatacaggtagaagtaacgccgggatgcgccgtgcctgtaattcaagcgattcaggaaaatgatgtcctgtacgcccagaccgaagctggtctatatcgtctacgctacagttgctcgttccgaacgttggatgctaacgtcttcccgccaaacaaaacagagttccgtttgaagctcattgcgtgtgacttcttggctggtgttactactcacgataaacttctggactaagcactatgatcacagcaaagaacgttgaaagccttttggcaaaaataaactatactcggcccgacccgtcacgggaagagctggaggaacttgtaagtcacggcagaactcgtattctaaagacctcaggcattgacggcttctgcccactgtctcgaaaatactttgagttctgcttgaagcaagttggttctttctgcgcgacttcgtacaatgcagttgaaatagcaatgtgtgtaggcattcagcctatctatgttgctgctgcgctccatctttacggcagcgactggtcatatcgtttgctcaaactgaaacgctttggtcacctcgatcgtggcattcatagtgtgtgggaatccggcggtgcatggttctcgcttggtgaatgccgcagtcgcattgtaggttcgcagattgtatctcatggtcagggtaacctgaagactgcaattcgtcttggtgacatggaacagattcggcaaattgttgcgctgtacccgcaccgaaccatgagcgtactcgcacctcgcatcggacttctctacactgaccagcgtcgtgaaaagagtaagcgtgaccttgaagccaagaagaaagctcttgaggcagaaggtaagaagatggccgaacagggatcgtataacgacctcagccctgtcttcaacggctcgatatctaaacctaactacggtagggtataattgtggataaaaagataatcagttttctcgtggatagcttgagtagcgacgcacgggagcctgccgaaaagtatgcaggtaagactgctggtcagattgtcaaagaagaaacaggcattgtgtttatctgcaacaacgcattcgtcatggatcgtcttctctggttgcctgacatggagcatgagtggttcacaccagtcgaagctctggttcatctgtctagcggtcttattggtcatgtaggagatgtgcctgtctatagcgattggtactacggcagcccgtccgatcgccagcgtccttgcgaccaaatccctcaagtcggtgtggtcaacgtggcaaccaatgaaatttctttgattactgttgaacaatttgctcgctaacggtaatttcgacaggtcaaaacaaataacggaacactatcatgagcaacgttgatcaaacaatgccacaaggccgctgggaatttaacgaaccagttgctgctgtcttcgataacatgttgcaaaactccattccttcgtatgaccgtatgcgtgacctgacctaccgtctgggccgtcagttcgtaactcctggcagcgctatcgttgacttaggcgcatcgctcggtcgtgcagtcgaaccgttctgtgctgagttcggcgagtacatgtaccaccacgcggcagaccgtcctgagcctgattcagaaacaggcaacatgtactgctgttacgaagtcgctccggcaatgcttgagcgtctgcgtcagaacgaagtgctgaaagcggctaaggctaaaatcagtagtgagtcgctgattgaagtggacacctttagattcgacgagcaggttgaatgctctttgattctgagtgtgctcactctccagttcactcctatcgaacatcgccagcatatcttggagaaggtgtatgactctctccagactggaggcgctttcattctggttgagaaggtgttgggtgatgacaacttcctcgaccgtctgctggtagatacttactaccacatgaaaggcagcaacggctattcgcaagagagcattgcaactaaacgcaaatcgctcgaaggtgtactggtccctgtgaaagccgcatggaacgaagaactgttacgcaaagcaggcttcaaccgtgttgagtgtttctatcgcgatctgaacttcgctggatggattgcaattaagtaacaagtgtgggtggcttcggctgccccttgttacacaggagattagcaatggccaacaaacgccaagaacgttgtgcgtcaatgattcgtgagtcgttgattgcagagatcaaaaaagcacgttctaaacaaccatacgtcttccttagtggtggtgtagattctaactgcattctgtttgctgcgcttgaggcaggatgccgtccaattactctttccttccacatggaagggattaatagtcgtgacttccgggcggctcaggcgatagcaaaagagtttgaccttgagctgattgaggtcgtgctgccaaactcatacgagaagctcaaaagcgatgtgctgcttatggccgaacgctacaagtgtgtgcagaagaatgagttcgaatgttcatggcctatgctgtatagcttcttccgcgtccgcaatcatgcgcgtgaaaacgacatcaagaatcctgtgaccttcacgggtcaaggcgctgacttgatgtacctgtcctctaagaaggccagcatccactataaagatcgtccagatgtgtggcgcaaggaaggacgtgctaatcctcaccgcactcaggggcgcattctccctaagatggcacaagatgcaggcattcgtaatatcaagccgtgggatagcgaagaaatccttcaggcgtttctcggtacgtcatgggaagacgttaacaagccacgtcagaaagaaccttctcgtatggcttttgaagattacttcaagcgcgtccgagtattcaaccatcagaacttccagcttggcgatactggtattgcagagcacttcgagaagctgttggaggattctgaaatgaatccagacctcaaatataaaagtgttgtcggcgtctacggagagctggctcgcgcataccaggacaaatcctgatgacaatgattcacatcatagacggctctgttggtggaagttacgtttattcaaagctggtggatgcaggcttcaatgctcgcatccacgcaccgccaaatccgagagttcgtgccgcatacgctacgcacccatcactttctatgggtcactcggagcaagaaattgagcgccatatcagtcaggtcttaggcacgtttcgtggtctattcctgatcagtagttacgttggttctctggttgcgaacaacatgattgacatgtgcggacagtcagacaacgtgattacctgtgacgacctgaactgcggttccattccagtcgttgcttcctcaatttctgtaaacgtatatctgaaacaacgcaagctggctcgcattcatcatcgtctaaagcactatgacctcgatcacgagttcgccatagcggacaaggctgttcgattcgcggcgggtgatgattacgcaaagcaggacgcaaagcaggaactgaacaatcacgcgaagttcctgtccagcccgtctttgattgtggccgcacacaaactcggtgtgaaaggcagcatgtaccataactatgcaggtctggtgaaagagtttatcgaaaatcgccagaagcagtaacgtgagggcacgatgattaatcgcttccaaatgaaaaaagttcctacgctcgaagcgtgtcagtggaacggggagaacgttgaggagatgaatgagttcctcaacggtcatggttatgtcaaaggacgttacgttgaaatcggcgtgttggataagtatcagaaaccaactatcgctaacgtgtctgtaggcaactatgcagttaagcacgaagacggttccttcgacgcaatgactgcgagtgaattgatggacaaatacgttctggctgattgagggcacaatgaatctgttttctattttaaagcagcaggtgaagaaagcgctgtccaccgaagctgcccacgagccagaagttcgtgcgatgtttgactggcgctattcagttgacgttaagggtcagatgtacatcgtaggcaagactggagcaaacacttgcttctacgttgagccaggtactgatgaacctatcgcgtgttatccagatgcgctgctggcgaagattgacgagtggggcgcaagcaagtatgtgtcttacgcaatctattttaagcgtttcgaatctcctgttttcgaaaacatcaagactctggaaaaagcgctgagaggtaagccgaagacattcaagaagggttacttcttgtgtggcctgacgccgaaaggcaagcgtgtcaaactgttccgattgcaaaaaggcttgtctggtatgcagtgggtggcagtcgaacctaaacctaaatcttaatctcacggcactgtccgtgttaggagcaagtatgattgacgacattatcgtaggtcacatttatcagtcatctaatggccatccgtacaaagtggaaggtcgtgctgaacacgggcaagacccagaagacaagtgggtgcaactccataacttgaccgatactcccttgtacgccaagggatataagtttagtgtgcgagagcctgtgttcaaggaagttttctctgtgtatacagaaggggaataccatgaacacaacgttaaggcatcatctgaaatgccgccacttcaatcctgcattctaccattgctgggttagcgaaacgcaaatgaccgtgccgttgttctcgtttgatagagcaatgcgcgggctacaggtctacacaccagacgcaccgaagcacgataagaaccctaaagcctgtcgctacttcacacgggcgttcggtggcaagcagttggtgtggggatcggaaattaaacctgaacgggtcgaccgtgttcttaactgagtcagtattcaaggcatgtgctctgcatcgtcttggactcaatgcttggtccgttcttggttcaaacgtgagcgagtacctgtaccaccagcttcgtctattgggtctgcgtttcgtctgtcttggcgataacgatagagctggtcaggagtttagtcagacgtttggactaggcgctgtcagtaatgaccttgacgagatgcctgatgaacagctactcgatctaactttaccattcctgaggaagtagaaatgtcacgagaagttattgtccgtatcttaggacctgttggtgttggcaagtcggctgtgtacgcgactttggttaatgctctgtctcaaatcggtgttagcgttaaacacgcagacgagaaagtgtggaagtctttggagaacgctggtgaagttgcgatctctactgagactcttaacgaactcactcctgttgtgacgttcgaagaagttggtattcgtaccgacgctgctgcttctccaaatcagatcatgcagtatttcgcatacgctcacctgccgccacatctgcaagcggtaagcaagccgttcgcgttgctggcccaggagatggaccagaacctgccaaacggtcctgaaaagtctactggtctgcgcaagttgcttgaagcgaaagactgcatggtacgtcaactcgtagctaagtaatggaggctatcatgagcgattggttctacggcggttaatgtgcagtaactcaaagggtggccattaggctgcccttttctgatcttagacaactaaaataagcccaaaaggaccatgcagaaccgtgcgtaaacagtatagaaccatgtgtaggcagcgtagaaacaccaccttttttctaagcagcatcaagcgcttgaaatctgtaaataaacatcagataccaataatgccccttgagaaggataaaaatgagacctgataccatagctcgcacatatagggttccaagcaagacgcttgaactggcccacaacatctgcggacgccaaggcatcaagctgtctgacattgttcgtcggtacgcccagcacgttgtgagaactcgtggggagtttctgcgtactgctgtgcggcacgaaacgtcccagcttaacgtgcgtatgccctttgacgtagcgcactcgtttggcactgtgtgtcgtaatgcgggttcgggttcaagtaacgccatgtgtgatctcctgaatgagatcatccaacttgatcgtatcccagaggaacttctgcaagagacagaggaagatgtgcgggaatatatccgtactgaacgtgagcgccttgctacgttagaggctcaactcggaaaaatctaatgacggtaataagcccaatccgatatcagggtaataagcgtagcctaatccctattattcttgaaaatacaccacccgtaaaagactgtcctcgtatggtcgatatgtttggcggaagcgctactgtctgcgcgaacatgcctcagaagtttcgcgtttacaacgagcttagtcctcaggtgtatgagatcgtcaagatgctggtcgagcaggacccgaagaaaactttgggacaagtcaagcgactggtacgccattggtgtctgacgaacagcaacgaagaaaactacgatgcgttccgtacagtagttcagaagaagcgcactgcaatcctgcactacgttgcacaccgacacgcacactcgaatatgttgcgcttcaaccaacagggcgtgtataacgtgggctttggtgatcgtggtctgattggtaagttcgatgaactcgaacacgaactcacatctttccatcagcacatgcagggcgtccacctgacgaacatgaagtacggcaagctgctaagtaagctcggcaatcaactggactgcaatacgttctgttacttcgacccgccatatctggcgagtggtgcaatgcagtacggtaagtggaccgaagccaacgagcgcaatctgctggcgacgcttgagcaactcaatcgcttgggcgtaccgtggatgttgagcaacgttatcgagcatcgagagttctcgaacgatctgctaaagcgttggttaaagaaacacgcgacgaccgtgctctacccaaacaaaagctatgcgatgaacaacggccagagtggttcgcatagtacaattgaaattctggcgatgaactattgaggtaatcatggaaccaccagtcggaacgaatatgaagttgtggcgcattcttggttgcgtcgttcgtgaactcgaaagcattaattctcaagcgtggtatttgtcccaggacccgaaagatacctgcggctcaattggctacgctatccctgactacacggatgggactctgatcaaagagattgagatgcgtgttggccagattgaagaacgcaagcgttacatcgcaggtctgcatggaggtgagcaaggtcatcgtcgtgcctgtgacttccgtgctgatgaactctatcagaaatactgcggtaagcgcggatgaatctcgtctgctacctgttcgacaaaatcccagagtacgagaaagcgatctatgcgatggtcgctaagtaccattctgatatgggtgaatggggacagttagctccagttgctagaatggaaactgttcgccgtatcttcatcgcacgtactcggggtgcatattgtatgctgcgtcgttgcacaaacctcgagacagcgtatcgtgaaatcaaaaccctgttggccaaccctgttgctcaagagattgagttaatgtcggatgcagttatcaaccagaggtataaataaagtggaacaagaacaagatatgagtcagaaccctaagcacatcattaacggtttctctttccgtgaaggctctgcgcaactgatggcgtttgctctggacgtcgtgcgtctcggtggtaagattgaagaatctttctggaccgaccacatcgtcgagaacctcaaagagcttgacctgatggacaatctgcacatcactggaccgatcatcgatcgtggccagttcgacattttcgaatcactggagcagtgccgtaagaacgcacacgtcctgctggacgccctgatgtacagcttcgacctgatgatggaagaactgcgcaccagcttctgctccgaagagcgtgtgtctcagttcattgcgcataacaaacagaacatgttcagtcgtgacttgcgtggctacctgacgcggcctgtgcaagagtctgacctgcacctcgttcatgcttatcgtcgtcgggctatcgcactgaatgatgccgagcctgtgctgttgcacatcggtggaacggacagccaccaatgggtctggaacggtgaatggcgagcgctgctgggtgcgtccgaagaaacacgtatgcgtcagttccagacgtggtactacaatcacgctttcaccgagcatcgcctgaaagcactcgtcaatcattacctgcactacaaattccctgagcacttcaaccgaggttaatcatgaccggtattaatgaattgcgtagtcgtctggtggccgcacttgacctagaagtgaagacggcaccgaacgccgacatagaatactatgttgactcggatggtctacctatgggcttagttaaagactggaggcctgatgtgcctgagaaaatcgttcaggtcatcgagcagtacggtctgcgtgtcgagcgtgttgttaagccaggtatccctaagccaatcgacgctgataacgttcagtgggtgtaccacgtctggtcacgtcaccctgtatatcgctcgctgtctgtcgataactttgcccgacgcgaaggccctcgtgtcgcaggtgaaacactaacgctcgccgtactgacttgggcagtcctccgtgcagagcgcatcaaagaactacgggcatgtcctgtgcagtccaagtcctacaacttcgaacgcttacaggagcgtgtgtatgtatcatccgttgggggataaagcaaccgactccgaagtacgtgcgtactaccagaagcaacatgatcgggcagaagccactatgcgagaaatctgggcgctgcgcggttggacgattcgctgggaatggcacaatggagtatgtgacgactgcgagttcctatttgatgaaacaggcaagcagatgtgcccgtaccatgacgcgattccgcagacacattcgattggccgttatattgagaagcatcgcctcaatgtgacattcacgaagaaatctgtaaaattgactaacaagcaagatcccaatccagttgaaggtaaagctgatacgctacgtcaggcatatctcaattggttacttgctcttgaaaagcagaaagctgaggagaaaacgtgcgctgcgacctgaaagaattaccactggctttagaccaagctgaacacatcatggcgagcgtgttcactctggcggcttcctccaagtctaagcgtcgtgcgacggctgcaatgttggtgcatttccataacggcttcccgatgattctaagtagtggcgtcaacgggacaatgcctggcgagagcaatgtcatggaaacccctgacttgactctttcactggacactgtaattcacgcagaagtgaattgcttggatcgtctcgaagactactcgctgtggacggacttccgtgacgtgttattctgcactgactctccgtgcccaaactgtcttgccgagcttgaagttgctggcgttaagaccgttgtgtacgcgcgtgagtatcgcctgactgatcatctggacgcatctgatatcaagatgttctgtctggacatgaagtcggttgaacatcgtatgcttcgcggcatcgaacgcatgaacgaagtgatcgcaacaacacccggcgtctaattaaggccaataactgagagactctcaacatgaaattcaagattcaaccacatcaagatatgtccatacctaccgatgcgcaagtgcagcaggttgctgatcacgaagatcgtatcttccttgattcgttgtgtgaatttgaaaacatgcaacgtcgcaacatggagcgttttgcagaaatggttgaatctaatccaaagttgaggttccaaatggggcaggctcgacgccacggccatgagcagaagtttggaagtttggacttctccaaactcgaagacagggttatggctaatgctgtccttggccgcatgtcttcgcagcataataacatcgaagaacgtgtttctgatacgtttgaacattcatcaggtgtcgttcgaggcatagttcaatgctatccacgtatgtccgacaatctgcctcgtgacggccgcattaaagttgacgaaataccggggaaacgtatgctgcaaactgatattcatctaggcgatgtgaagacagaagacctgtcgcttgctatggctgccgttgcattcggtcttagtggtgagcagcttggcgttatccctgctcccggtgacagtcagttcgttgagccggaaacgcagttgagttacatcgacgaagctccatttattccaaatcatctgcctcagcactacctgcaatctgataaaggccccacgcaggcactgggccgtgctttgcgtatagctccgaaagattcatggtcccccgaacgtcgtgatcgtgctgcgacgtctgcacctgctcgtaagaaacttcgtgcccgtacacgcgcccagaagaaagcgcgccgtaaacaacgctaaggaacaatcgtggaacctttcctgaaagaaatcaaagataacttcgcccgtgctctaggtatcgaccctaaagttctcgacgtgccagtagacgaagaagctacggcacgttggaccgaaatgctgcgtgaagatcgtcgcaagatcactgtcggccttgcgctgtgtcatctgcaaatcccagatgatattcgctacagcctggtgcatgatcatctggacacgactgatcgcttgctgcgagaggcgttcgaaaacctcgctgcccagcttgttgctgttaatagcactggcggtggcgatgaaaaacaagcggcgtctggtgcgtttcgtctagctatgctgatgaacatcctgggcttcgacaacgaaacactgaaaggtgtgcttaccgacccaagccttactcgtcaggctggtcttatcgctatgactggcctgaacgatatgggtcagaaaattcaacaactgtacgacgagagagcaaaatgagccaaccagaaaaccaactcgccaaattctttgacgaagaagcattcatcccaggtttagacgaagcgcaagatcgcgtagagactatgcgtgacggtggaggtgagatcgttgaagcatccgacgagtgcgaaggcggcggctgtaagatctaactgtctaactcatggggcctcgtgccccattcttgtttcggagctgaaatgcaaacggcatatcgctgtatcagttgtaagtacgtccacgttgggaaagtcagtagttgtgactgcaacaataccaaatttgaatacacgttggtgcaaatcatcgacgtgcctgagaacgaagaacaagtacctaagttcaaagatctcaggcactcacgcgcccagcgttatgtgaacgtcaaagatggtgtatacggtaacggcgtttacgaggtccgtaagattcgggataatggctccgtgatctggacacatctaggcaatatgcagagcggctatgacagtaccgacatgagctataagttcatcgaagacaatcgcaaagcaaactgtgtactggccgccgctggtcctgagatgctcgaagcactctatatgtgctatcagtatttcaatctgaaacgtgaagtgcagggcagttcagtcaagaatgatagccgcatttccgtgatcgcagaagcaatcgtacatgctactgatatcagtgtgttcgacaagcagagggaactaccaaatgattaaacgtctgaaagataaactggctgcattcggcctggctgtacacaatcgtcgtcaggagaatcgtaaacgtcttgccgcgctacgtgcaattcaggacaatgcaattcacggaggccaagtatggaagtcgaacgagaacaacgctgagtatcaagtgctgttcctgactaacctgtatactgacggttcgattcaggtagtatactctcggcactgggcatacatatcctctatgcctctggaagacttctttgacaagttcacgcatgttaaagagattgataactcattgcccccagcgtctgacgatctcatggctatggcaaccaacatgtttggacgtagcacagtgcgaaagcctcaagaaggtgaatactggtcgcgtgttgatcgtctacccagtggctttgatgaacaacgcgaacctgtattcatggacaagaaagccacgattcaggttcgctctatcgtccaccaaactccgtctcagccgtttgtgctgtacaaagagaacggagaagacctagtgctgaacatgcaccaattcttaaatcgctacagtccggagcctgaataaaatgttgattgattttctgaaagcatttccagcaataatcttgtgttacatcatctggcgctggttgctgacaaagcgggacaggcgtcgtcatctggaacaagcgcagtcacactacaactgtggtcgccttgatagtggtaacgtctggattcatttgaagacagggcgttcttataccgtgctgtatctgactaacacgggtgtgaataaatccaactggcgcaatgactgggagatcaatgttgtatacaccaacgatttcgagcaagtctggaacaggccgtttagtgagttctgccataagttcgcgcacgtcagtcgcggaggcaatgaagaagacttctctacggttctgatgggtatgcagatggaggcaaacacgcgcattcttattccgcacgaaggtgagatgtggttcgaaggcactgtccatgctactcctcctgaactggttgctcgtggacatgcacctcaggttgtgtctcagcgccgtgctcgaatcgacatggtgctgggtgtaggagaagcgcaccctgttgtcgtatatactgtaaatgatacgcagacagcaatgctgctttcgcagttcatcttcatcttccgaaaagaggtttctttcgatgggacagtcagctcttgtatttaagtatgtgatgttcgtccgtacgcgtaacaaagaacgtgacgacggcgtccacatgccagtcatctttcctactcatatcatgcactccgatatgggcgaagcgatgataggttacgcaatccagaacggtataatcgaaaacaaatactatcagcgcatggacccggttagtgctggctttatcgatctgtctgacctgcgctgtttcggcgagtccgaatctctggagctcaaatcccgtgaacaggacagcgagatcattcgtgagtacatgaagactcagggcaagggggcagagacaccgccaggagacgacaagtgaaagacttactgctgtctatctggaactcaccgttctggaacgaacctgttagcgcgttcgttgtgccagtgtgcgtcatctcgtacttcttgatcgaacattatctggagaaacgtgcgctgcgtctgtctcgtgctgtgtttgcgtctggctggaatcctgttaagggtaccgagtatcgtcatcgctttctgccttggcgcacatgccgtatgtgctacacgtcaaacagcccgaatgataagttcatgccgtctgtcgtgattaatgttgagcgtggtggtatcgtagagctgccagcacacgtcttccgttttcgctatagagagattgaaaatgccaactccagtgattctactcaaacagcagactcgtgatctgctgttgaagatgttcggtcagaacaagccgttcatcgtcgtgcgtcgtgatgccattgttgaagaaggaaaatcattcggagatcgtgtgtacttctccaacggtaccaacactgttactgtgccaaacattcagggccttgacctgggtgataagctctacgtcgcagaagacggtgacgtgtatgagtggcatcctcatttcgagcgtccgtacgaagctgtgtcaaacaatcagaccgaagcgctcgcgtttggtcttcatcccattatcttccatactgacagtcggaatatctaatgtcacaacctcttgatttacgcaatcccaatcactacgaactgtactccctgcactgtgttgacgagcagtacgtcaacctgtgtgacgcgattctcgcaactggtacgcaggagtcagacccaggtcgctctgacgatacgtggacaactctgattggtgttggcttccagttgcagaacacgcacatcgccttccccgcactactcagcgcacgtaagaactggtcggcggccgtcgatgaatcatgctggatgatgcgcggcgaaacgaacatcgaatcccttaactccaaaatctgggacgagtgggcagacgaatcgggcgagtgcggtccaatctacggtgagcagtggcgtcgttggcctgatatcaaagcgttccatgacttcactaagccgtctggtgtttgtccttctgccgatgctattcgtgcgcgtgacgaaatcttgcgtatgcgtgaagacggttacatcgaaacgcaaatggctgatgggcgcattctgtttgaaggtgaaatcgaccagttcgctaacgcactgcgtcaggttcaggcgcgctctcgctctcgtcgtattcgtgtgcaggggttcaatccaggctacgtgaacatgcaaggtctgcctccgtgtcataccgagtttgagttcaacgtaacgaagtccactcgttacgaacaggctcaggccgaagcacgtggtgtagctgtgtcagaagacagcctgcacatcactgtgacaatgcgcagtaacgactgcctgctcgggcgtcccttcaatatcatcggctacagtgccatgcaccagatgatcgcgaagtgggcaggtctgaatgttggtggattcacgctgaacactaccaacacgcatctgtacgatcatcaccgcgacgcgtatcagacgcaacgcgctcagtggatgctgttgcgtgagcgtatgcagaagactggtgagcctgttaaataccctgtactggaaatcagcgacgacattctcggcctgacgccagaacagttactcgataacgcaaacgtagactggttcgagctggtggactacagcccgcagcctgcggtcaaaggacgtgtaaccaaatgaaaaacttcatgctgattgagcgtgtcagctcttatctgtatctgggctttgcagaaaacatcccagacattcctcgccgcggtgttgagaagttcgaagtgctgattcctgacggccgtgatggcgagaacgatcctattctccaaatgactgcgcgttgtatctatcatctgccgcataactgcttcctgatcagcattgcagaaggtaccgaaggacacgagtaccctacgctgatgaagtctcactgcaagtacaacatggaactgttcctgcgttctggccatggacgtgagaagatcgcagttaagcagattctggatgaattgcatgatgcagaagtgcagcatcctcaatggccagaagaggcgattcatgctgcgtcaatcgtcacggaagaggcaggtgagctgctgcgtgactgtgctaccttcgaagaaaacggtgaccagcgtctgattgtcaacatgctcggtgaagccacgcaggtcggcgcaatggcagttcgctttatgaagaacttgcctacttcccaacgtcgtactatccctaacaatgcgctacgctcaatcctggactctgacatgaccccagagcaacaactgattgaagtgcgtcgcctgatgaatgacggagtccagtaatgcgtttactctcatacggagcttgtggcggtacaccatttcgtcgtctggtagttaaagacgacggtcagttcgaagtcggcgttcatcctaaaattgaagcgttcggctgtgtgttcactaacgttaacgtcggacgtattgctgacgatgccgttgagttcgatctacctgacgcgggcgactggtccatcaacatggcagattacttcctgtcgcctgagtacaagcagtgggttggtgggcatacgccacgtatcgaaactatgctggacgcccacgtcatcaaaggcaagctgcccacgctggtgcaggacttcgatgcgttctatgctgatctacagcagaagatcaatgcactcaatctgactgacattgtgtttgaacacaacacgattaagcagacgaacctcaatcagaagttcgatgtgtggatgctgtacaagtacaacttgatgcttgacggcaagatctctgttactcgttcgaacgtcggcgagctggtctttcaggaagacttcatctccgcgaaaggcacaacgtggtggctgcgtgagcataacaaaactctgatggaactggcccgcaggcacgacatgttggctgcgttcattacgttcggtacgtcccaccgaaatgagcgtgagttcttctactcgtttgtcacacaggaaggtgatacgtcacatcgtcctgttgacccggcagagttcctccatctgtccgtgcatggtcagttcccagagctggatatcaaggatgaaggcgaagggtatcgtctgactgtcaactacggtcaatacttcccgcaagcgtatcacgatctccaaaaagctgtgaacatcactatcggtagtaactacgcactgaacctcttgcgctttatctgacggccagagtctctcagtaatttatgtttcaacaagggagactcgccatgcaatacgataagacgaaagactatcaaccgttccgctatctaggaacaccaaaactgcctagcgtaggattcatcgccagcactgtcacactcgtcgaaaatgaagtattgatcggcaacgacgagtgtgagttcgtgtttactgtggagcagatgaatactatggacaggggtaccatgacgtttcgtgctaaagacatgggcggtggtatcacgataaagaaatgctcagtctctggattgaaaatggtaattaagctggaacgacgcgttgtgcagttcggcaaagtacaggtcgagtggcatagcaccagccgtaaatatctttattaatctgtaaagacagagaaagagcaaccacaagagatactactaatggcaaaaattgctaaaacaaaggaagggaaaaagagcagcgcgatgaagattgacttgacgaaattcaagacagcttcgcaactgaaaggtgctgactacaacccacgtttcattacagacagtcgcctgaaagcgctcgaaagttctttgggtagctttggtgacttgtctggtatcgtgtttaacaatagcgttaaaagcggtgtgctggtctctggccaccagcgtttgaaatccattgacggatggaagacacgcatcgaagtacagaagacgactgataagtacggcactatcggtctgggttacatccacgcaacgcatccgaagaagcctgaaaaggttatcagcattccgcttcgtatcgttaactggactgacaagaaaaccgagtacgctgcgaacatcgcggcgaatgctcatggcggtgagttcgacaacaagaaactcgccaagctggttgagaagctggacttgacaacaatcaagcctcagttactcggccttgacccgttagaaattcgtgggctgcaacaaaagctgaaaggtcaagctgccgttgtcactcaagaacgtgcaggtaaaactaccggccagatgaacggcagtagtggtgcgttcaaagagtacggcactgacgaagttggtgagagcctgaactgcacctgcccgcgttgtggatttaagttcgagggataatatgatcatcaagccgcctacgatgaaagaaatcaacaagctggataaaccctggcgtggtatgagtttcttcgcaggttgcggtgggtcttctaccggtcacaaaatggccggtatcaacattctgttgagtaacgagttcgtggactctgcccgcgaatcgtatgaagcgaatcacccaacaaccaaagtgctgccccatgatattcgtcgccttgacccaagcaagctcatgcgctactgtggcttggctaaaggcgaactggatctgcttgacggtagtcctccgtgctttaccgaagacactctcattcatacagcggacggcatgaagttcatctcggatatgaatgtgggtgaccaagcaatgacctcagtcggtcgttacttccctgtgtacgacacgatggttcgtccgtacgttggcacaatgcacaagattgaaactctaatcagtgcaaacaacgcaacgcctgagcatccgttcttcatcagacgcaacactgctccgggagaatacagcgaaccgttctggtgtgatgcgaaagacgtgcaggaaggcgacttgctcggcacgccgcgaacgacacctgacatgggactcgacgtatatcagtctcaactcgaccagctgcctaagcagattgcagagtgggttgtgtttcctgagttctggtggatggttggtcactggtgtgatcgtggtacgattgagtacgttagcggtgttgaagtcgttagctttgaatcgcattcaagcctcgaaaacgctatgatcgaacaggcgtttgacgcactgaaaatcagcagcctgaatcgtatcgacacgatgacctcacagcgcaaaacgttccgtattgttatggacgcagagctgttgcagttcttacgtcgatttgtcagtcagggtaatgaccgcttctcgcgccgtctacccgcgattgtcttccatctgacacctgagttgaagcaacaattcatcttaggctgtgctggctacgactacgttaccggcatgggaacaggcctgtctatcacgtctgaaagtcgccgcttcctgattgagatgaactacctgtgctgctctgcgttcaacaggcctttgtttgatggtctgacttggggcgacgtttacttcggtagcccgatgactcctcgtgaccgcaacagctctaagccacttattggctatctgttcctgcaggacgagcacaacttcttccacgagttctctgatgccgacccgcatctttgggtcgaagtgattgagaacctagcgtaccaaactacgtgtgacgtgtacaacttctccgttgagacggacgagacatacgttgcaaacagcgtggtcgttcacaactgcaaaggcttctctactgcgggtgtgaaagaagaaggctggggcaaggaagttaaatacagcgataacaagtatcagcaggttgatgacctgttcgatcagtattgccgtatgctcgaaggcatgatgcctaaagtgttcactgcggaaaacgttagtggtatggttaaaggtgccgctaaaggttacttcatcgaagtcatgaaagagttcgaccgtcttggctattacgttcgagcacctatgttaaatgcagcgtggctcggtgttccccagtctcgtgagcgtatcatcttcatgggtgtgcgtaaagacgttgcacacgcactcggatataaatcagcgaagactgctgtgcctgatgttgtgccttgtgagagtatggcgttccttgcagatgctctgcctcacatacagcgctacaagtcaacgaagaaagatatcatcacttatcttcctgcgatgaacggtccgatgcctacgattactgctgccgatgcgattgcgtatgagactgcgcgtttctcgtctgctggctttgtcgaagataacaaaggtcatcgccgcaagttgactatagacgaactcaaagtgatctctggcatgccgtcagactacaaactgaaaggcaagttcgaggagcagtgggaacgtcttggtcgtatctgtgttcctgctatgacacacgctgcgtctaaggctcttattgaacacatcctgattccttatgcgaagaagcgtaagaagaagccaggcgatatcttcaagtaggtgaatcatgttctggacagggcttgtattaggtatcgtgataggcgtagtggctacacttggcttcgcatggtaccacctcagaggcttttcagtatttaagccttagcgacaatctgtgtgatactctccgaagcggtcgcgatttaaaggccagaatgtttctggctaggagatatcactatgaaaaacgaaaactggtatgaagcagacgacgagcaattgaccgtagagcaaatcgaagctattcaacgaaaagcgaacgaagacgctatacggtcaggcaagcctctgcccgacgcagatgacccgtgttgggttcgtctgttctaacctagcttaacaaacaggacaaggacgtccaggagatttaaaatgtcatactgtttgattaagaatatcatggtggcgtatgtacgcaacggccaactggtatgtgcgaaagtcaaagtgaaattgagcggcgatgattctgtcgtgctctacaacacgatgcaccgtattcatcatgatacgtgcggtcgcattctgcttgagcaagaatctgatcgtgacttcctgccgacgattctctatcgtgaacgtgcggcagtgattgaaggtcatggtggtgcgttgaaacgcatcgagcagttcgccaagagcgtcggcctagactgccgtgttgttgacctgttcaaagattctgtgttgagcatcggcttcctgttctacctgaaccagcctaacgctgtggtctgtcagatcattgagacagacaaggaagaactcgcgggtaagacgctgttcattggcgcagaccctgacgtggattacgttggtgcgaatgttgttcctatgcttgtcgatgaaaacttcgacgttgacgacaagctgttgggcaacaaaatctactccctgaacgatgaccagaacaagatgttggtctcggtaggcaaataagatgatacgctacctgatcgttttcttcgctacatggattctggtagcgtactctctatcgacactggacgttccctctgagtggtgtgataggcttgcgttagttagtgccgcattcatcacgcacttcgaaatgaaatggcaacgcttcatcaaggagcaacaatgagcaagcgtcagaaggcaattgctgtactgaaagagttctactttgaccaccagcgtggcttcattcgcttctcccgcgagaacaactacctgtcttcgttccagttccatctggacgagattcgtgaagtgaacattcatcgtgggtcgggcatcaataaagcggacggcagcatcgttacagttgctcgggtgaacatcgatctaattggtggtggtagtgctcattcatgtccgatgcaccctgaaaaagatttatcagatttgaagagccttacgtccgcattcttgctgctacgtgatgctgcgtgtggtctgccttacgctgaatacgaagcgcgtattgttgacactgagttctacatcaataagcctgtagttacctggcctgttgaaacccccgccgaataatcggcattcggtgtgcagcacaaacgtgattgcaccctctacctaaaaggtatgtactatgactaagcaacacacttcctacagctctgcgtttgctatcggtgaaatggcagtgctgtctctcgataactttgggcagaacaaagtaccttacggcgttgttagcggctgtatggcttatggcgaacaacgtatgtatcgtgtctcgctgtttgtgaacgatggtcctgctgataaccctactgcgttcttgcatcagggccgtccagtcgatggcttcattgcgtctgacctgaaagaaatcaaagagcagtacgttgatcacatcggtcatgtaggccgtttcgaatcaccacaccataagctcggcgactctgtgtttatgtttggccagctggtggaagttgatatcgacctcgaactcgacggtgagtatgacaagttcaacatccctgtgatgatctccggcgttacttacgtcgaaggtaaagtgctgtatgaagtaagcatccaacgagcctactataatgacggtcgtgttaacggcggtcgtctggtgcgcgacacgttgagtaacatcgacagcatctacattaagcctatcggtggttggcctgagacagtccttgaagcaaaaggagaggcgactctgactgtcaagagcgatggtgctatcactattgactctgaggctgacgtgataatcacagccagcagtatcgcactcgaacctgtagtatcaggcagaacgtcgggactcgtagagaaccaaagcaacgttcctcgctctaagtaacaacttgtgggtggcttcggctgcccctttttgtatctgaatactgtaaatatctgacaggaggacagtatggaaaagaaagtagaagaattgaaacagtatgtactaaggcgtgtcaacgagaacgcaagccccgaacttaatattagccctgacgctatacagagtcatgcgcgtgatgttgttcaaggcataatgaagtcactggctgagagcgataatgggattcgtgttgtctgtgatgaatcgaataacccgcagtacaacctcgacaataacatcttgtcgttggatctgattatcaccaaaccgtcagtagttaaaatggtctttgagaaaggaaacgataatgctaaaacgtctgttggctttattcagcaagaaaccatcgtcccaaaagacgtttgaagaaaagttggagcgcttgaaaggagaatcacttgccgatgaaattcgccgcgatgatgaatcattacgtcgggcgctacaccctgggcatactccaagtgctaaaccacagctaccgcctgatagttctttcgaccgtactgctgtacttgatgctcatggcaatctgcgttacgccaaagatgcagcaagacagaagcctgttaagcaatatgcaccaccagccaaacgtcatatgcagaaaactcgtcgcggcatgacagtcaatcaggcttcatctagtagggctcagacggatgatatgatgttggctatgatgatgcaacaaacaatcattaacacgccaagcgctctggatgatacttgccgcattacgccaagtcacggcggatacgatacaagccctagcgacggtggcagttcaaacgatggcggtggtggaggttcatgtgattaaacgtctgtgtaactggataggcttgatgcttatctctgacaagaacaagcgcaagctccgtcaacacgaagcgatgatgcgcgcctgcactgacgtatacgactggtgcggtgccgacttccctcaagcggccgaagctgttgagtatgttcgtacaatggcactcggctatgaaggacgcctgaactataacaaccacatcatgagtcctcgtgagtgtcatgtaggtatcagcgattggcgagaagcaatgcgtcgtaagtatctgcgcaccgaactggactttgatggtaagacattcaaggcaccagcggcagagaaggactggacgactaagagcgtttctgtaaactaagaacacaatcaacatataccgagaataaactatggaacgtaattcggacgatacagttgtggtgctggacgttgaagtcttcaacacgcttgtacaatacgcacattgcggtgaacgtgattgcggggaaggtttatacgggaagtccgtgaaagatattgagaaacatgcacggcattttaatcctcacttacgcgcggcctatgcgcaggagctgactaacgaacgtctgggtaaagccgaacgccgtcgtctgattaagaaagcacgtcgtcttagctctcagcgtgagcctgttcgtttccttgttgaccaccagcataaggttatctatccgattatcattacgggtgtagcgtcagacaaccaactgcgtttgaaatatcacgcactgtctgacggctgggactctgctgcaatggtagatcgcatcttcgaaacaccagaagaactgcctcagtcatatcgtctgttcaaggaaggggagaagacagaatgaaggcactgtctatacgccaaccgtgggcatggctgattgttaagggctacaagaagattgagaatcgcacatgggacacgaagaagcgcggtcgttttctcgttcacgccagctctaagcgtccgtctgatcacgacatgcaggtagcgaaagaaatctgtgatggcctgaacatcaagctaccggagaagcaggagttcgtgctgggctccatagttggttacgctactgtgtgcggtacagtcacgcagtcagacgatccattcttcttcgggcccgtaggcattcagttaaaagactgccgtgctgtcgagcctatccgattcaagggcgctctcagtttcttcaacacaccgttctgtgtcgttggcggtaaggtagttcagtcaccgagatgttaagacccatactcgtacctcagttaggcaagctcgtcttagcacaccttgtcaatgaagaccgctcggatgtttacttcgtgcgtcacattactgtcagaggtgtggctatgtgtcatgttgggcttgctcctgtcaaaagcgtaacgttcctgtacggctacacacctacacccgacgattacgaaattgtaaagcagatgcgtaaataacaacagggtggccttcgggtcgccctttctcgtttaaggattaacatgctaccgttagctccaaagaccagagtagttagtatgcgtaacggcaataaggactatgatgttcgtattgaccgagaaaccaagtggggtaacaagttctacatgacccacgaatgtgtcgcagaacgcaatagagtgtgcgacgaacacgaagttgatttgtgggagaagatcgagaacggcgagatactgctgcgtcatttacttgaactctacggaaagcgacttggttgttggtgcagccctaagcgttgtcatggtgatgcgttggtcagagccgctgaatgggcatatcagctaaactgtaaatatgagcgtatcaaagctacttacaggaaacgcagacgtgctaataaaaccagagcaaacaatatcaagaagaaagtttctcggccgtagtccttcaatgaaagccattagctgggaagtgttccagtctcaacgtggcgatggtgtgtacggtcagttccgcctagcatggggtgctgactgtattaccattcatgctctcgaccagacacgcaaagactatgagtacgagtatctggagaagctggataagatcatcgaagcactcaaaggctatgcaccagtacttggtacaaagaaccacgcatcatatcgtgaatggcttaaccctatcgagacaggcgctacaggcagtctggcatatcactatgatgtagtgtcgcctgagaacctcatattctttgaactggcctcatgtgacggtaaggtcagaatctatccccatcattttgggcgccaaccactgcgtaagatgcagagctgtttggatgccattcgtgtggagctagtcaaccacaggacgtcatttgtgctgttaatgaaagccatagaatctgtaaagaatagctatacagaacaaaacaaggtggtttgactatggctatgacccatgtgcaatacgcactgaataagctggcagaagaattgacagaggccgcccaagagtgtgccaagattgctcagtttggatttgactcctacaatcctacggacgaatcgaagaccaccaaccttgttcgtctgcttaacgaactgcatgatgttgaaggcgctaaggcattcctgaccgaagtatctcggggtgagttcgagtttgtgcctaacacgattcgcgctctgaataagacggataagatcaaacgccatctcgcaatttccatcagcatgggtcacgttgaatcgttcggagacgaagaagaagaagaggacgaataatgtcatacacgatgatcgttcagcacaacatcaagctgaaatctgatacacctaagcgcgtactaaacaagatacgtgagtggcacaaagcgccgtgggctttcgattaccttgaccgacacttcaaaatcaacgtggccaaagcgcttggccctggctgcggtggtgtgtactgtaacttggagtgcaagcgcatcttcaataccggtagcggtgttgtcccgcacatccgcacaactgcgatgtttaatcgtggtaacgaaggcgcagaagtcctgcaacaattcttcgactgccttgccgattacgtcgctaacactgacgaagtgattgcggttattcgcggcgaggataatctttatgaccgtaacgaagggcgctccaacatgtttgaagcgatacctccttcatacggttactatgaagtgcgcatcgtaaacaaccacgcgaagataaaatgggttgtcaacgatctctatgaacaattaccttgggtaacctatgcttactaacattgctcgacttgtcgctacacaagcacacgaaggtcagttccgtaaattcaacggcgaaccctacatcaatcaccctgaacgtgtatcagcatggctggcgcagttcaatgttggtgagttgatcgaagctggtgctctctgccacgatgttctggaagactgcgatgtgtcgcacaacacgctgtctctgctggtggatatgcctgtcgcagatctggtgcaggaggtgactaaccgcacttaccctgaaggtacgccccgcatcaagaagttctggggcaatatcgttaagctgattacagccagtcatcaggcgcagactctcaagtgtggtgacgcttacgataactgcaaagacgtatacgagaaagaccctgtatacggtgcgcagtacattgcagaaaagttcttcctcgtctgcctgttcacccgagcacaagctgatgttaagcaagcgctgttggatctgcttaatgatatttaccataaccgcatgactgacgagcatcgcacttatgcgtgggaatatcttggacgtttagacgccgagtgtcctatcgagtaccgccagctctacgaagaaacaagtcgtgaagctcgcagtctgtctcgcgcagggcttgtctttggagatcacaatggaattgcgcctgcctccgtttaaaactcgtagcgtgttagtagagcacatggaagtcaaacacaaacacgctaccgcagtagtcgatgtgaccgaaacaagctggtggggttatcgtaaacgccggttgcgtgttgcaatgaagtgcgacaaggttaatcgtaaagagcctaagtggtctgcacttgtgcgctgggacgacggctacatcgttgctccaatctgtgaggacagtgaagtcctgacgatagcaactaatacactacgcgatatgcgcaatatgaacatgacacactttgatcagttgctcgcacatcgcctttcaatccatttgaggaagcatcatggccgctctctccctgaacctgtttgaaaagattgacgacgaaaaggctttcaccgaacgccgcttccataaaagcattatgttcatgcacggcgtatcgtccaatagtccttacgccaaagacagtttgcctgtaacgttcgctgtgtatgaagtgggtgatactcgcacgtatgccgcaactgttgggcacaagctgtcggagcagttgcagtacgcaatgaatctcgaacctgtgcgtgtttggcagttggttcgtcgcggtagcaacgtttactttgttggcgagagttccgaagcgattgttgctgataacgtagtaccaatggagattcgtgtcgaaggagggcaagatgcagagcgatgctgggctacatcttgaactaacggcgaaagacgttgaagcctactggaagggacgggtctttattgaagcggcccgcatggcgcacgacgcgcacgaagataagcgagctaacactccgacttatcctgcgattgaaccgtatctcgaacaaggccgcgctgtcattgaccctattcgtgaacagcatgaaggtgagttgcctgacgccgtgtttgaagagggtgaaacactcgaacctcgtttcgtcgttatgctggcgttgatgcttgaaagcgaaaatcagcatattggcggcaagacgattaagtctatggcgtatctgtcatctgctgcccgtgataaaaagatcgtgttagtgctcaacaaacacaacacggcgctgtctcggcatctggctattgagtctggctttgaggtgcgtgagtctggacttatcgaagtggcagaagccattcgagataagatgactggcttcttcgaactggacactccccggcctgttaaagagcctgatattaatctccacgctgtcaggcagaagcacaatcgtgtcggccgcaattcaggtaatcagcgtttcaatgcgaagccgcagcgccagaacttcaaaggccgtggccgatgattcacgaaatgtatgcgattgggtacgtgaataatgttcctactagcgtccacgtatttcggccagagaaagacacacagcaatctgattatcgtgctctcgtcagcatgggcgctttcgataagcgtatgggtcaggcatgtgctcgcgatcttacagcgaaacgcttctggttgaaacgcaagttcgaatgggaacaactggtggagagcgacaggcgtatgatgcgcctacgccattctcctatttgggttaatcttccaaagcagatacacgatgacctgtggtcgttctatcgtgcggtcggctgggactacaagagcaagcgattcatttgacaaccaaaccatctctgccgtgtgaagtaacgagcatactcacggtatcaacgcgcagcgggaagtatctcgaagtgctgaataataacatcataccagctgggcaaagtatcagtcatgttgtcgatgccgcccttgctcaggagactgaacatggatctgaaagactggctgataacaacggagacagtcatacataagatggttgtcgatacaaaagacgggaccgccgttggtcttgtcgagactgtctactatcgtcctaagcgtttgggtggtaagcgtcttcacggcaccacactgtcctgcatctgtcatgatatctaccgtcgtcatctgacgtggacggacgttaatggcatggacgagttgatgcccaaagataatcgtgcgaagtcactttgtcgtcggctacgcacagaacttaataaactcgtagctgagggtaaaatcaatggcgagtccattatcggaaatgcaaataggcagtcctttgcctaatcacaaagacctgatatcgaagcaacttattgaaggtcagattgagttcctgtcaggtattgctgacctgcacgaacacagtgccgtacaaatgcgtaacccgcgcagtctcggcctagacgtattgaacggtacgtgggtgtatacgccacgatacatgtatgaaaatcgtcacccactctcgtatacgtttggccacatgcaacatggcggtgatgaagaaggctatgttacgctgcttaaaacgctggcgcagaaagcagagcaagagttctactacggcccgctattggctgtacgcaagttccttattcggcacgacaagattagtggtaagactgacctgctgatgcctgattcgtggtctgttgtgattgacgatgatctgaaaatgtccgacttcatgggcgtcatcgaaggctacgtgcagtccgatcagcgtcaggcgatttgcagcgcggtgtatgagcaatactatgccacgttgcgtagtcacagtgacctgtcagtaagactgatgtttagtcagaataaactgattctggtcgatgctggtgctgcgttggttggagcgggtagcctgttcgacttaacgcctatcatgcgcttcatttcgaaccctaaaggtcacggtctgacgcaagagattttccgtgcttatcgcaagctcgtaaatctgtaaatactgattgctaaagttatctgtctaatctaactatcaactatgtaaggaaaataacatggcttctgctaatggtggtgctcgcggtgcaggctctcgttcgggtgctgtagataacagcgctaagtctgctaaagttactcgttccgatcgtcctatcgcggccgcatctgctgctcctgcttactctcaggtgaatacgcctatcgctgctggtagcgttgcggtctctctgtctgctcgtgctgccaatgtgggtgtagcgcaggaagacctggcggcggtattaggtcgtctcggtctgtacgaaccaactccggcaacccgagaagattttgcgtgtactgaaaacgttctcgaagtgttgacttctcaggtgaatgtcggtctacgcagtctgcaacgtatgctggaaagctccattaacggctctgattgcggagataaagacggcgaagaagatcaggaagaagcgaccggtaacatcgctcaaacgtcatacggacgtagcttctactacgcggccgatactgcaagcgctcaattgcgtgatgttcgtaacaagctggagcgtctgcgtacttctctgctgggtgaacgtcctactgccgatctgaaaactgcggcgcatgacagcacaggcagtctgtatgcggcggtctctgtcctgtgtgataacatggacaacactgttaatcagattaacgaactgatcgctgaaatccgtaacacgctgctcggcgagtaatcgctgtgcccacacttaatcctgttggagaaatagtcgtgattgattttgaaaacactgttattcgtttcgacgaagaacgccgcccgtactacactgctcgtggcgctaaaggtaagttcgagcgcgtgtatctgaatgacgccgaacagcaagcgcacaaagagcacgaagtggaaaaacgtgatcgtctgaacagcgctgcggtggctcctgcttgcagcttccttaaaagtggtcccacaggtcctgtaggtccgggcccatgtcctgtcggcgcaattggtgcagaaggcgttaccggcctcaacgtacctttgtctctggaagaaagcgttgcggaaactctgcctgttgctgattgcctggcatcacgcactgtaagcctgattaactctatgagcaatctgtcgggcgctctgtacgcgttcggtgtgctggacaataatcacgtaggcaacctgatgcacctggtgctgacctacgacgagcgcaacgaacacgaagcggaagatgaaaacaacggtctggtatctgcccgcgcgttcactaatcgcattgcgtaccatatgtgggatgcgtaccgcgatgatcgttcggctagcccgatgtttgttgtcgcacagcaagtaactcctgttgtgacgcttatgcaatacctgatgggtagcgcgttcccagacagtgacatggctgtacgtgcgcaacaacaaagtctgatgttccgtaagtcagatgacctacgcagtctggttgaagacttccacacagtctacaacaacattcaggctgacctgggctatatgggcgaaacgttcatcggtatcgtaccagaagagattggtggtgacactaatctaccggaagatctgtctaaaatcggtctggttcgcgctgtagacgaaatggtttcgtacttgattcgtcgtactgataacctggtcgatctgctgaatgcagaaatgtaattcgctgtagaaatgaaaaagggcgactctcttgattgagggccgccctttttgcgttatagtgctaaacctataccgatggctgctgcgatacgtgtcatccacagctggaagtttgctgccttttgatcttcaatgcgagccttacgctccgccaccaaatcctcagacaaaccgttagccctaacttcttctgcttgggccaaacgcagtagcttgttgcgttcatcgatcgtgaggttgagaacatcaatcagcttattgcgctcttcggtgcggtcttctcccgccttatataggttgatcaaatcaaccatacccttgttatcgagtacagccaccttcctgtcatcaatcactttgatcttaacagtcggctttgctggtaccttctcgggtgtccactcaactttgtttatctgttggatgtcctgcatggttgttttgtgttgctcgtcaatgcctgacaaagaactgcaaccagaaacgagcaacaacaggagtaacgtgattattctcatagcttattgtacctgtctaccagctcttccatgctgtcatcttcggacggtggcttaacagtctcaggcttccgctcgttcaggtccttcaccgcatcgttaacagtcttgctgtcatcgacttggttcttgattgcctgttcacgcgtattctcagcggctttctgctcacctgtcgtagtctcggacttagcgctagggcgacgaaacaacaacgccgaaacgataagcaccgcaacagatgcgaaaaccttccagtatttcttaaacaattcaatagccttagacataatcagcactcccgcttattctgcgtcttctttctttgctgccttagaagtctgcgtgttaatcaggttctcaacggtgaatgcaagagagaagtaggtcagatggtcagtctgtcctgcggtcagcataccgatgaacatgcccgtagacacaaacactgcggcgatagacgagattggatttgacgtccaatactctttccagttaaggccttcccgcttggtcttgaccacatagttcatcaagaccccgccgacatatgaaagcaagaaggctacgatttgaatcggcgcaagattcgttactacatcacccattttcaatactccgtatcgacaaaagaaagggagagccgaagccctccctatggttaaagttgatcagaggtaatctgaccatctttatacagttcgcgcttacgttctttccatgttgaagtaagctcagagaagaactctttcatgcggtcatcgtccagctcgaaaggttgattcacttcgtacttaccacacagggcgttgaacgtattcgcatattcctgctgtaggaatgatttgtccgcgcttacgctaagatactgctgcgctgacagggctaccgatacttgcatgatattatcctctatgtttgacttgcttaaattactaagcgaatttcaaaacgaggtcgttaacgataacagcttttgactggtctgtaggcgtagtgctgtttgcgtatactttacccccaaccagcttcaagtctgcatttgagttttcatcaccaacagagcacacagcaacgaaagcagcaggcacatcagtaacaccagactgaacgttgatcgtagccgctgcaccaccaagaacgatacaccaagtaggcgtagcgtcttttgtgaagtagcttgcacgatagtcagaataggacgcattgatacgcatgttaaacgcagacgctaacagcacaggtacgttgttggccgcgagagtcatagccgctttgttccctacaacaccaccaacgtagtcggcgattcgtgctgaggtcaaaagaccaggacgctgatagattgcgtttccgccagtgagctgcgtaccttctccaatcagtgcctgtagctctgctttggttggcatcgttcctgtgtagaacaggatagcgcaagcaaccgtagtgaagtttgaaggtaccccagagtttacaaacgaactataggcattacgttgcatcgcatttgcagtggctggaagcattttcattacacgccctccaagaagttatccgcaatacgaatagtgagatctgggacagccatttggtcgtactgaccgatgtttgtcgtaccgatagtcacgtctgtgcctacatccagcacaagaccgtaatagtcctcttgcgtctgagacagataggcctgagtactggatgggttggctaatgtcagcggcaccagcacaacatgcgtcaaggcggcagaaacaaagtcgctgcctttctctgcgtatggtgtgaagtacatgtcatttgttgttgacgtgccgttcatgctcagcctaagtttacgcgcaactatatcaagaccgtcattcatgccagccacaacagtaatgcgcgtccagacgagagtggttggatcttgatattcgaagcgaacgttacctgcattaatgcccgagacagatggaatgaagaagctacggaagcgcagagttcgaccgtagtcatactcaacagcgtcggcagcactccagccgctacccacatcgttagcgatatcagaacaagcaccaaccatagccataatttgctgaggacttttgttgatgttagcggtcaacgtgaagcgactgtactcaggatagactgcataggtttggatattcgtcttcgtcgcagggtcgaagtaggtgcgcccctggccatagccgccgattggcatcatactacgtccacgagagaacacgcgacagaacgtgctattcgcatcggttgtttgttgctggaacttgtactcgacggcgcagcggcttgtcgccaccaaatcaaggaatgacttgggtacgctactgctacttccgttgcgaaagaacgccatgaacccatgagtgttcgcagtcgttcccacagtctggagtagctgatacaacgctgatttttcagagactaacattaggtgtctccttagtatttgatacgcatgtctgcaagacgcagaggctggccagcggtaacagtaccgccaacgattttcagatcagcattagagttctcgtcgcctacagtgcctgtaatgacaacataggcactacttccagcagcgaatcctgcaaatgtatctgccgcagaagcggccgcagtcaaacgcatcatgaaccacgtaggtgtacctgacgcagcaatggttgctaagttagcttgggcgctgaatggaagctgcatgacgttgttatccagatccatggtgacagtcataataccacacgtaacatcgcctacgaagttaagggcggaagcaaaactattaatggccgccgctgaccatgggattgtctggccagacgtggtaatcatagcatttaactgagcatctgtaggaggctcccctgagaacaaagcgatatgcacagcgttgactgccgtattgctgttaggtggcaatcgtggattaagtgctgtcattgccataaacgagttgtacgctttagatacgcgcatattagtatacctccagtgtaataggcggataggacactgtgaatgagttgaccgcctgttcctgtgctggatacgctgtggcgtcagttatcaacagatcgaagttcgcggcctgcttgatatcgtcagtgatagtgagtccgtaatgcgggaagaatcgtccgtagttattgacgttcattgccgcagacatagcgggcaggccataggcagtaccgaagccatgcggaaacatcactacgtgctgaactttacccagcgtacgtggggaggaacctgctacatagtcaccgtagaagtgcagagcaaacgtaccaataccgatgaagaatgggttggttgctgccgcagacttagacacaattcggaagcgacgcccttgaaccgaggccggaagctgataatatttctcaacgttacccgctgtctggaacaggttagttactaggttagttacatcaacccacgaactaccttgctgtacctgcaagaataccaagttagcaggtacgttagcgaacaggttgttattcgctgtagtctgagtaatactggtcagagcgttaataaccacatctgcgccgaagtcatactcggctaaagtccaggatccgtcagagttcttgttcttaacagttggaacagatgcccctgatgttggtgacgtacatggcatctgagttgcagaagttgttgaagcgcaacggtgccacagaatggtagcgaacaacatatccagttgcaactgagcacttgcaatcccagtatcaacaaggtcttgatacacttgactgtaggacgcgaacgttactttaggcagaacgcgttttccacggaagccctgtgcagttgtccacgcaggagcaggagaagactgcaagctggtggtgtttggaaccagagtatgttgggcattaccaatctgggtctgtaagaaggcgcgaccactgagcatgttgttcagcacagtctgcatgtcatagttcactgggttaggaagattcccttccatgaaagccccgtacatcacggtaggtgtattttgataaatcggtagaattttcatatcatgcccttggtttaaagacagttcaaattaatgaggtgacgccactacaaggacgccacccacttattacagttggaaagtcatatcaaggaagcgatatgcttggcctgtcttaatcgtacctccgatgaactggagctccgcatcagagccttgatctcctacggttcccatccacgcaggacctgcgagcaacgtaccaggagaagacgacagtacgaagttagcccatgaggctatacccgcgccaccagaagcaacgatacgagccacatagtaggtaggagtaccgtcagcaacaccagtcaatgtcgcagcattaccaccaaacggaagtgtcagtgtgcgagcacttgggttgacgataggtgtcatggcagcaaatgcaattgagcctaagaagttcgcctgtgtcaaccccaacgcggtaactgctttgacattccagccggcaccatgggccagcgtgaagatctgattgaagtcaggcttagagcctttgaacagagcgatgtgcagcgtgttcgcaggaatcgcagtcgcaggaaatccggcgttgattgctgccagtgatgccgctttgttgctgatcatactcccctcccgataacagacgcgagttgcacacggaacgctgggacaggcacaggaccaagtgctgtgttgtacgtcgtgtccagcatattgatatcaaagttcgcagcctgtttaacatcatccgtaatagtgagatgcaccatagagcagtaacgactctgcactgtagttgttgcagctggccagttaaacgcccacgtggtgcctgcattataggaagcaagcgcttgtaaatgcagcacggtcatgtgcttgaactttccgagtgtgcgaggcttctgtcctgtgtatgttgcatagaactggatgccgaatggatagtgacctgatgtagaccaaggccacgtaacagccttgttcaccagtcggaacttctgcgctttgactttcgtaggcagttcgtatgttacagctacgttatttcctgtggtccgcaggctatcgtaggtatgaataacgtccgtccagataccattaacctgagcttgcagatacgtctgttgggtacctagtaccatctgagcggatacagttgcccctgaggaatagcctgctagagcacccagttcaatctctgcaccgaagtcatattcggcacacagataccaaccttccgtagtcaagttgtactgaggactcaagttgtttgtgatgctcgccagagggtaatctccagacaacactattcgatgcgaaagcaggcaggcggccacagcttctaagtacgtgtttactgtactggcaaaacgagcatccagcgcaggtaactttatcttaggaatgattcgtgtcttcgtggagaaagcactaccgtatccgttagctactccgtttgattcgatccacgcaggcaagaaacgaagggtatcaaacgccgatacggatacgggctgatactgccaacgggcagaaggtaaggcaaccgacgttctctggaacaggcgtaatgcaatcgcatcgttgatcgcactatgcagagatttctcgccattttcaggagcatcagtatcgtacaaaagacctaagcaaatgttcgatgcagcgttcatgctctggaaaggatatagttccatgttagctccatacgatgttgttgagactgatagtaccgttgagcgtaaacgtaccatctccattgtctgtcagaggagcacccataccaagcaggtcttgcgcagtaagctcgatcacagaccctatagacgcagtacccgcagcgattacagtcaggttggtcccgagcataatgtacatgcggttgaatggcttagcatagctaaaacgtccaagttggttgaacaaatcgagcatacgcttaccctgacctaagttcacgatacgcacagttccgtttgagattggcgcagcatccatgacacatccaggaagatttgcagccagatatgtacgcagtgaggtcaggctgaacagagcaagcgattggttattccacaccgtgtctgtgatcgtatcaccggtagaaaacacaatagctgccgtgcgttctgcgctgattgtactgccgccaccttgtatcgtacctgcgttggctgctacagcgacgttagatgaccaaggtgcatcaatcgttgaggcaacgttagatcccaaagagtcaccacgcatattgagcatagcttttgaaatatacatcagttgctcctttgggtgaaacgcagtttaggacagtacatgacagtcttctgcgtagggataatatcgccgatgattttgtacggaccttgagcacctacagcacctgcggcatacatgatatcgtcagagtagtcaatgtcaccgtgagtgaacgtgttgcagtgtgcaagcgccgtccaagtagggacagtttgcgcagaggctggtggagtatcgacggtagacagcagtacgcgctgcgctgtggtggttgtaggcttagcgtatttgtagcgataacgttttgacgcaacaggagtagacagtgcgagacaaagggcatcgcccgcgattgctgtagccgtgcctagggaagtctcggtctgaccatcatcagacaaggcgacgagaacgaacgcatcccctgtgcttcccgtgaacttaacatgagtgacggtagttggagtgtcgaactcaaattcaacgtcactgacgaaacgcgaggccggaaccatcgtcgaacctgagcctaaaatcaacccgatgctacgatcagtaaaacctgaacgagtgatacgatgaggcataagctgataagccacagtattagcgctgccaatggtcccatagtacgatacccctttaggaatatactgagactgtaaggcaagcgttagaacgttcccggactccacaccgctaatcgggttgcggatcataccgatagacgcgttgtacaaatcagcaagtgacttgttattgaaggcagcatcgaagccttcttttgacgtaggcattttaccactaaacgcaaagatattccaacccgcaccgacattgggatcgtttatcagtgctgcattgtttgcgttcgtgcccatcattgcctgcgccatgatacggttattgataatcttcattagctcaccaccggcgcagcagatttgttgttcgctttagtgtcagacaggtcaagcgcaccaacagttacacggaagacgatgttatcaaacagagggtcaatcgtctggtcagtagcgaactgtccgcttacaagagggaagtcgatacgaggtgtagccaaattcgaagtgaacgtcttcggagtaaacttactcaccacttggccaatcgcattagctacgaacagcacttgatcgattgcagagacttgtctgcgctgaatccaagatgccttgcttgctgtatacgccacttgagcaacgtcagcagtctggtgattgggtacagcggtgattgattccactgcccgcttctggggctgcgagtcagaactaacttcaatctgagacataacgaacacgaagtccgcgaacatgtccgggtcatacgttacgactggtacgaacatggttaggctccttgacggatcgcgtagttattgatgataggagtgtatgcagcattggcgcccgccgcatagccaccagtcacttgcatacctacagcaacaggcttgagcacggcatacgtgaacgtatctaccactgtaccatcaatagagattttgtgtgtagacgttgccgcatcgtattcatatttgatatgaacaacactgcctccccacatagctgagtatggagatatcgggcgaactactttaggcgtaccaccaccgccacccacgttattccacacgcatagacctttctcatttgagcggtcgaatgagatagtatagcggtcagtcagagaagcgctggaacggaacagcgtccattctgcgtaatcagcattgcctgactggtggtagtcgcactcaatcgtgaaggacttgcttgggtcaaacgtagaggacgcagccattgtcacggcgcctgtagtacctaagtcaacacccgagccgtcagcagcaaacttcaagttaccgctggtggtgcaggcattgcctgtcaggtcagtgaatgcgccggtattaaacgtacctacattgaacgcagcacgttcagtgccagtaagccacgtagcgttagcattctccacccacatttgcgtcaggctaatagtaaacgcattgattgtaacctgggtcttatatccgttcggatcatagcgaacaacaaggtcaggatagagcagcgtaacatcaggacctacctgcaagcacacaggcaagataccaccgagaatgagatgtgttggaacaccttcggcagcagcggtcaactgacagtcagagatagacagcttgttgcggtcaatagtacgaacgcagttagtgcctttcgccaacacggtacagataccactcgaagcagcaagagcagcatcgaagatatagcctgcaccagtctgagcctggaagtttaagcagcgattcagatcagcttccacgaacccactattcagcttaacgagatagcaggacttatcgtctgccgtagcctgagcgaataaacgcgtcaattggggaacggcagagtttgcgaataacttataattcatgttatacctcggtggacagacgaagctgggcgacagatgcgaactcaccaggaccgagtgcagtagacattaactcgattggcttaccgctaccgatcgcaccaacttcacaggcgaagtaagtaggcacatagttaccgttggccaaagcaccgtagttagtgtcctgaataactaccagcgcactacgcattgttttgtatgaagcagttcgaccaacatccgaagcagtcacaggaagaacacggcgtgtacccgacgtttgaatgaagcggaagcgcttagaagaagttgttggcgtagctagtacgttaccttcttggttagcagcaatcgcccacgcacgagcagttccaacattgccggcgccgtcgataggagcaacagtacctgcagcggcagaagtcatatcaccagcgtctgacagaaccgcgtcgatagtcacttcgtaatcgaacgtcaggtcagtggtggacagatgaatgcctggcgtcaggctatcatgcggaacgcctgcgtaatcccatgcgcgatatcctgcaggaccgataccccacagcgctttattgcctgcgtcattgcttgttgtgtaggcagtgttgatctgaacagacgcagcaccattgtagcctactggtcgcgctttcgatggataatgaatggtagcaccgttcttgatctcgtacacatgaccagaacgtgctttccatccctcctgcagatcggccagaggaacaagaccttctgtgtttgggcgcagaacgatgcgcgttgcagcaacagcgttatctgtaagattacgcagatcttgcaggtgttgagagaaatcaccctggtcagcgagtgctgtatcaaagaagaagcagttagcgacgataccgttagcagcattcgaccaccagccgctcccaagattcagtacgctgaacggaagcaagttgtgtcctaagatgcgcattagaactccttagagtctttaactacggttgctaagaatttaccgttgcgcagattggctgaggtcagaatcaagtctgcaccagaacccgcagcaccgatagtcagaataaggaagccaccgtatggagtgcttgcaatatctttgttgaagacaatcacgttgtacgtgctcaacagagttgccaagtcacctgcgaatgttccttgcagtgtagccgacagacggaacttatatttgttatcttgaccatgaatccagcgcactgggttagtactggcgctagtcaagtcgagcacagcagtcgcaccaatagcagtctgaacagtagtaccatcggcaacaacgatgttggccgggtcaggtacgtgtgcgagacaaatggtcttctgcatgtttgacaggccgtacttcaatggcggatcagacgcgggacgtttgcctgcatctgggatcgtaatgccattgacgaccaaagggaacgaaactatttccattgtgttatctccaattgactcgcagtaaattactgagaactcatagcgagtaggaagtggttgctataaagagaaacgttttggcaacacgacgggctcatacgcagtgaacgtgccactcaatatctccgtaggaagaacaggtccgtgtacgaggactttctatcgggagcagcaacatccgatgaaaacagaaacatgcgctttcgtgctgtctctatgtccttctccagtaactgagcaccgttcgaaacaaataacataccggctcctatagttcaatagtgtccgtgttatatatgacgggcatttctggcatagatagggagagggtcgcacccacatttgcactacgtggggcgaagtcatcggcgttgtacacaacagctcgtatccctagaccctcatagataaaaattgcaaacttatcaatgctaatcgaagactctgcctgttcacttgaaccaaactgattagagcatggtgtaaacaggttggcgtccagcgcgtttcgtctggtgattgggcctgctctccagtaaccaccaccgtataccatctccacataagcactcattgagaaagccatacagccaggtgcatccaacgcccagcttgacatgtttgtgcctgtgaagttatacgaccagctatgaggagttgtcagcgcttcgctgtaacctgtcgcagtgtagattcttcgtctgtgcctatacgaatctcctgtctgcctacttgcaccactcacctgaactgtggtgtcagggaacgagacttggtatgaggtaggcacagtgacattacctactttggtaggcactaagcagaacggtgatggtacccaggaaccgttgttgccgttgaaaggcgtattccctgcgaaggtatcagtcaaagacatttgagaacctttacgaccactaccgcctttaattcctgttactaaaagagtccttataaagttttcgtcagatgtaaagttaggaggctctgacataatcgttagcttagagtaatacacacgagatcccgtaccgtaggcagcaatgcccataatagggtgcgtgactataacgttttcattctgagattggacagacgcccggctgtttcgtattagatctcgtagttcactcactgaactgaaatctatggcttgcccggagtcgaaaaagaatccgtacttacgcacatcatcctgtctaggaagtacgagttgcataaactttccttattacatctgggtgagagacttatctggaaatagttgtgtgctcgtcagagacaaagtggctatagacgctgttggaatagcgcccgcctgtgtgagatcttttccctgaccaatttcaccgcgcacaagatatttcaggccattcacttggaaggctgacatgcacgaagtcaagacaacatcatctgtgtttgccttgcctgtgatagcaactcgcatcggataggcttggttctcaggccgagtatatccagatacgccgttaccagactgtggggtgtacgtcgcacttgactgattcaggccgttagcagaatacctcatacccattgtgcgcacgaacactagatggtccaaagcggcgtatgtgttatgtagcgttgcctgttggtttggtgtacctgtggtctggatataagaatagccaacagggctagtctccataagcatatccagacccaagccaccgttgttgaaacctgcatcgtagccgctgtacgttccccagaaagggtctgtgttacggctgtattgactacctgccttggagctgtatgtttgcagatgaacgtttgtgttacgcatacctgcagggaagataagcatacagttcgatggccagtagagagattccgacgtatcactcgaaggtcctgactgacctgtaaacactggagcgcccgcagcccatagactatagttagacgtgtccgatacagtaaagtatcgcgtgagtgcggcttccggtgtttgttgtgcagtgtatgacgcatagccactactactgactggagaattgcctaataggcaggcgcttcttgcaggatagaaaaagttgtctttgatgccgctcattggactcaaggtgactacgctttctgtacctaatacagagttaccccaagccctggcgcctttaacctttgagatatacttcgcagcacttacatgagcgtctgacaggtcagtctggctgtcaaagtacagagcacggtgcgtggccaacagagcgatcttgttggcctttatggggtgtggcgttgcaaagagcattatgctcctcctacagtaggtatttagacttagcattggcgtaagacataacttcgtcagagaagtttaggtcagcaatctctgctatgctgttgcctgtctgcctaacatcatttgtgcttgcatcaccgattgaaagaactatcaaacctttttcaagaggatattcgtatgcgatagcaccgaaagataaaacgcaaggaggactatctgccgttacatcctttagaggtacatacaggggttctgcaataccgcaatttgggaagtcagatagagttggcgagtaggagaaactggtatagcctccacctataggccagctttgagtctcttcctgagtcgatataaacatgacgcagggtgcagatgcagaatacatagcaggagctactacaggaagagtgttgccttgaccgtattgcttagtcgtgtctgtagtcgtgaggtttgtttgcgtctgcaacgtattagtcataggcaaatatgcaccacttgaccaatagagcgtgtactgaaagtttcgcccaagccacgagttagattcgtatttagtgatcgatagggtttgacctttgaaactcaagttggctcgaataccacctgtagcagaaacacgcatcgaggtaacaagcgtctcaggaacaaagtacatcctattgctgaacatactcgatgttgggtcataggctctacttttaccaacgccaaagaaattagacttcaaatcactcatggcaccttttgtctgtgccgtagttacggtaacatatcggtatgcttgagcatcggctgtctggttgtctgtggagcttccgtagtagtaccaatccttgttgttgctattctggttgaaccccattaagtcggcagtgtgtgctatatagtgtttgttgttcttcacgccagatagggcagttgtcttcgccgtattgtcagagagtccccatgcagtaccacgacaatacggaatattcttgagcagattaactcttgactgtcggacggcagccacatctacggttgaatcaaatagaaacaatgcagacagtgcatccttgcgcatcttgccaaccttgacagcaccgactgaatgaaactgcatatacgccccttttcgactcaaaatcccagatacaaggtaaaacggcccgtaccattacgatacaggccatctaggttacaccagcaaacgtcctgcaacagtgatcgcaacaccattcagtgttgtgtccgcagtatcaggtgcgatgacacgcatctggtcaccagcaacaagaatgatctcttggtcctgatatgcaaccaaaggtgcaaacacaccaactttagaccctgcggcgaaagacacagtgccaagctgaataacagcagaggtggctgagtcatacgcgcttatcttgaagacagacgcagcggtggcagcaacatcggctacagccatagagccgccgaagtttttgatgattgcagttgtacgcacagacaggtagcgagcaatctcctgtccaccagcataacgcttgagtacagacagacccacgtcatatgggtttacagactgcaactgattaacccacttgttacgcacttggctgaacacgtacaagcctggttggttctgacctgaaacagcagtcagattccacacacgaccattagctggagatgatggaaaggttgggccagaggagttcgggtcacccggagcacgaacgatttgagcctgttcacccgcgagctgtagaccataagttaacattgtttatctccttaggcgattcgcacttcgcccgtaacagcgtacgggaaagttactttgactgtattaacatccacaaagataacgtccagaggcagtacctgatggagtttaccatctggctgcatcgtacacgtagtcactgcgaccatacgtccgaagttgtgcgtaatcacccattcagcagaaggcgtttcctgtttgtaggagcgccccatcgaatagttgagcataagttcctcacaattcatatgtgtattttggcacgactgcattagacagcattgccgtaccgtttccattcaccacaggacttacttgcataaggtcggactcagcaagcagagctatatgcagcgttttcttttcatcaacgattgcagccataccccatgtaggaacagagacacctggtgtgccattcgtgatagcgtgataaagatttggtactccccaccacaacgagaagtagttgccgcctgagttgttgaagttcacgtttctgaccactacggcgtatgacatagcgttcgcctgtatggcattccctacgacgacgcgatagccattcgagttccatgaataaccatccccgcccacagaaagagcagcatcaagagatactggatagttatacatcaacatggaagtgccatacatactgctaccgacttgatcgttcaacaacttgtctgacattataggctgcgtcttgtcaacaccttgagctgcaagcgaggttggacccgacgcctcactctgcattaatgtcatacccaaagagtctgacaggtcgagagcgaactgacgttccatgtggcggtacgaaggaactgttggcgcattcacaggagctaaagaacctgttgatacgcccctgttgctcgtatacgtatggtggacagaacgtgtgtgcagccatcgccttgtaccatcagcactgataccggcagcaggattaagaggtatagttccgttgaccgcaaagtcttttgagctggtcacagacttctcggcacacaacttaacgaagttattccaagtaagagaactcatgtcaggcttagacgtagaggcctcgaataagaacagacttcgctctatcatatgcttttgtacactgcgatagttttgagcgaaaagcatatgagcgcctcttaatacagaatgacggtgcctgactcaggattatcgaaggtgatagtgagcagacttgtgctgtcatgcacgatagacttcggctggacttctttcgtgccttgcatgatacgcactgctggattgtagcccagattgtgcgtaacagtccacacagcttcgtcagtgaatgacgcagtgaatgcaacggtaggagtaggcagaccgctttcaataccagacagcagcacagccgtaccagcaacaggctcggggaacaacacgatggtagtgtttgcgtcctgagagtgaatggatgagggcataacaacgtcaccgttaccgtcgtagcactgaacgataggtgtgcccgtgttcatgttgtgtgcgatttcccaacggcttgatgcagatgcctgcgagtagcggaacatcgtcatctgttgcgtcaacggtacccagataggtaggtcagcgatctcaacacagaacatcagacgcttgtccatgaagattgccatgcccggctgaggattggttggccagtcagtcacttcatcaaatttgaagttcttgatcgagccgaactctaagtctaaagtcccaacgactttcataaatcatctcctgaaaggtaaaaagggcaggcagaagcccaccctttattatgttacggctgtcgttgtcgattacgcttctggttcaacgtaagtgttggttccagttacgaatgcgattgcaactttcttagcggtggtcagttcgacacgcaggctgtttgcgtcgatgaacacaacttcgtcggggatgatctggtagccagtgtcatcaacaacggtaacaacaccgaacttgtggcctgcgttgtgcgtgaaggtgtgcgcagtagctgcaacatcaccgcttgcagtcttatcatactgatagaccttagcagcagaaccaccagaacccgcagcgattgcatcgtccacatacttcttggtagggacgctggtatcggtcagcggatcggtaccagtcagagtcagtgcttcaacagaaccaccgtcagcgtcgatgaagccgccagcagtcttaacagcagcaacgtcaacgatgattttgctgttatcaacgtcctgttttaggcctgtgcccagagcagcagcagcaatctgaccgtagccaacaccaccgtctgcaatagcgataccatcaacagagcgggccaaagtagcaccgtccagtttaacgcgagtgctgcctgcgttgtcttccaggccgccgttagcgtcaagtttggcagtcacggcattgctggagatctgaatacccgcgccgactttaacattgacaacgttaccagctttttccagaccgtcaccagcgttgaactcagaagcgccgccgaaggtagtccactcagtaccatcgaaacgacgatactctttgatatctttaacccaggtaaccgcaccaccagcttcgctgtcagttgggtcgaacacgataacgaacgcagtgccgttatagcgaacgatcatgttgtcagccagaccagtgatagaaccgaagttcgggttgatggtatcagcagacaggatgatgtactgcttaccattttccagaacagggtccagagtgccgtcagcctgaataccgtcagagtctttcagccagtcgatgccagcgatagcgttgtcgatatcgatcttacgagcagcatcgttcgggttagcaggagcggccaggttagcaacggtattaccgttagcgtcgaggtcgccagtcagttgaccgttagccgcattcagcttaccgtccagcgcagtttcgtttgcgttagctttgttgctgacagcagtgatctgagactggatgttagagcttgcgccagacaggtagcccagctcggaggcagtaatggtagagctttgcagttctgaatcagcaccagcaataacaactgcgttctcggtcaggccgctgatcttgtcttgcttggtagcaacaactgtctcaacgtgtttcttagaaacagccgcgttatcgccagaagcagactggtcaggaccagacagttcgaggtcagcagtcattgccactgaaccgtcagccagaaccacaccttctacagaaccaccgctaccgcccagctctttgatgacagtgccgttgaagtatttgtacttatcttcggtgctgttgtaccagatacgtgctgtctgggatgcaaccagatcgcctactacagggtcggcggtaagaacttcaggacggaagttcttaatctgggcgccgagcattaaatcaagattaccagtacgcattgtaaatctcctgttgcgtgggattagaagaaagtaccttcacaatcatctaggctacaacgtagcttttgataggctgcgattcgttcttccgtcagattgatatacttatcatcaatattgtacttcactctgattggtacatcgtacccatcgagcaggccgtgtcgcttataagcattcaggcgtagcacaggtgaactgacctgacagaactccataattgtcaggtcaatcttgtcggcgtatatgaatggtcgctctctcttacataagatgtaatcaatctcatgcaaattaaagagtgtgaaattcatatagccaattatgaactccgcaatcagcctgaatgagtcaaacatgtcaggcctaaattgttgtgtgagaatctggtcaacgtaaggtctgatctcggtacgcatctcgtaccaactctcacagaacaatgcagggaagtcttcagggtgatgggccataaggcccaacacgtctttttctgtatctgcgaaagagcttagaatgtcggcagcatcatcggatgcctcgacgcctctcccagttgaaataaaacgacgttcaatgtctctcaaccaagactctgatgcagacaggtattgaagcagtgtttctctcgcggcagccgaaaactcatgcctgtttgagtcaagaacctcaccaagcataaaggctttcgctttgtagaaatcactatagcgttcggcagtgaatcgtcgaaaccctatgttattcctcaaatagcccatcatcgcaatgccctcagatcattcaactccgtgttgccttgcgcattaggagttgtatatagagagcttgagatactctgcaatcgcaggccgagcttctcaagctcctgctggttgccacccaacttctcaaggacctctcgcattagctcgacagaaccttgatggtcacgggattgctgagagatgattcgttcgaaacgctgcatcgcgcgaagaacagagttcaatccctctttcatatccaaattatcgaccggcgcagagtcagagattgattgaatcattcgcatcatctgcgccaagtcggcttgtagctcgtcgttgtctggattgccgctcataccgctttccagttctgcattacgcgccttaactttctccagttcttcaagctgaggcagtagtttccaccaaacgtaggcaccaccgagaatcagtagaacaacagaaccgacagtcgcgtagttggacgcaagcaacttgtctaaaatttccgcccacattatattcaacccttacaggtgttatcgttcagatcaacaatgacccgttcggcacctggttcgtttacgtcagtggttttgtacgtgtgcgccatcctaggcttgaactctaagcagctttgtccgtaacgtccatcgacaacacagatggcggacaggcagctaacatcttccttgagtattaaattttcaggagcttggttggtactcctaactgccgtgagtacaaagcccaccacagcgatagcaatgacaaccagaatggcaatccgaagtcgcttggcttgcatttttggttctacctcatggtcctttcatctgactgaaattagcgaaccacacgcctagcagaagatttattcctccaatacgccactaatctccgcaaacatattcttgtacactaaactcccatcgagcttgtctagcctgctaacaagcacatagagttttggagtcgtgcgcatgttagcccacgtcttttcgtttgtgtcgagtccgccaacgttcgggacaatgaccatgctaagattgttgttagcacgaacgaaaccaatatccatatgcgtcctgtttatagttctgataagcctattgattgcgtccaaaccaacaggcttgttgaattccgtatcattcacagtgttgactaagctaataagaattcccttatctctgctgttaatctcaaacaaagttgacttgagatctcctacagtcgtagcagagtagtaggacacgtcatgccctaagtccttcaggcaggaacctaacgcacgagccgactcgatgtgtgctatgttatcatcccgaagaatgtacatcggagcatcaggctggtacgtgcgcttggtaaccatgtcaataagatcacaagaggggcgaccaacagtggccagccccctatttgcgatatagaacttatctttatatggcccgtagatattgggcggcatatatttcaagtaatcatcgtccagactaagtatcatgcgaggcttagttatctgaatgacgagttgcatggtgcgaagcgaggccttgtactctgtatcggagagcactcggcttataggcaaatactgcacgacaacgaagcgttcatcaatcgaatcaactacagaacgaatcaacgtacttcccagcgtagggccagcagagaactgggtaacaatcatcacaccgccttgaacaagacttcttgcaccagcgatagtagcaccgttacctagttgctgcgtagacgcttcccacgttaaggctggtcggtcgtctccgatatcggcatgtacataagctgcgctacaccagagacaggctccaagaaggtaagcagcaatacgttttccggatcggcctcggctggattgacagtctcgggccatagcacttctcctcttgcgtcagtgacgtaaggaatgccggcgcctttacccaatccatgacgtaaggcccatactgtatcggcattctcctgcacgaacactaaccctttgacttgcgcttcgtctgtagcagtctccagcacctcaacacgcttcccaagaagctcggcattggattgcagcacacgaatagcagccaggttagagttaacgcgctggttcatgttgttgaacatggtgaagaacgagttgttcatcgccgtgcgaacgccgtccgtataggacttgggaatcagttcatcgttatcgtaggttgttacgcccgaacgcacaagaactttaccggtaagacgtccaccacttgcgcttatgatctgaggagcaggcaaatctgcttcgtcccagacctgaacagtggtcatcaccgtattgtagtcggtctcttcctgccacgtattcttatacggtgcagtggctgctttggacttacgtcgcatgacttttttatagcctgcgttcgaaccatcagcaatgacccagagaccgttcagtggaaatacgtgagtaatcggttcggcaaacgaaagaatgattgtaacgtccgcccctaccttgtacgcaatatcgttcgacgcagaaagcccttgctgttgtgcaagagcaatcaacgtgtccacgtagttagtcaactggctcatccgaaactcctaacgattgtaaaattgaagaacttgtatcggagaaggccttagcaatatgagaggcagcagccttatcgacaacgagagtgctgattcgcccttttgtattacacacaatagtctgaggtgagtacggtgcaagcgcaagagcgaatagcagatggttgcctagatcgccagagatagatacttctacgtccagttcaggaacgtaaatgttctggttgatttcagcaacaaactgcgccagcgccactgggtcgaattctgggagcgctgtatcgtaatcttcaacgagatcaatctgtcccgtctcagggtaataacggaaagctgctgggtcagagaggattctgccgaacagctcgtcactgacttcaatgcagtctgtgtccgtcttttcccgcacacgaccaacgatgctgttgttcgtggggttgatacgaatgataggcatcgttaatctcctactgctgtataccagaagtcccaaccgacagtgttagtgccgctggacttaatggtaaagccacccaacagggcgttctcgttcatcgcactggtaccatccaggttatacaacgtatacgtcttagcttggttggtagcggcgttaacgaacgtgatctgcaagctgatgcagcggttaatgaacggactgttgaagataacgtgcagggtatcagttgttgatttgttcacgacacgggccatgttgtgagtaaagcccgtgttcatgtttcgattactaccaacccaagcattaggtactaccgcacccgttactgggtcaagcgcttgcgacacgcgatattcatcaatcgcagcatcgcgtccaggactgcctgtaggtcctgttgcaccagtgggtcctactgcaccagtgttacctgttgcgcctacaggacccgtattaccagtaggaccgttgcgccctctagggccgcgaggacctgggcagccgtcatcaccatcacgaccatcacgaccgttggtgccggacagaccgcgcaagccttctttgccctgcttaccttcacggccagacttgagctggtcagcagtaggcaaaccgataacgtttgtctgactgccgtctggccagatgatagaaagcgtaccggtagtagtatcgaactgagcaccctgtgagcctggaatcttcgatgcttctgcagggtcgataaatgcaaccgctgtcgaagtcttcttacccagcactttaccaacggggtcagtaccgccgtcaataagtgatgggttaattcgtgttaaagacatgggtgagctcctaaccagtcagtgttgtccaatcaggttgacccgattgtccggcttctggatttttgactttcgtgttgttgactgtcatacgaatccaacgaacagttccgtctgtatcttgccaccggaccttcgtgccaccgtatgctaaattagctacccatctgtctctgcttgggtctttgaatgctaaacgtgcatatgcgggcataaattctccttactcgatttcactcggttcccagcaaaggataggtctgcgccacacttggaacacaccgatagggtcagctcggccgccatcaatgaaacagtccatggtgcgaccgccggagttgccactccgcattaacgtctgcaagttagcaatccaagaagcacgacctccagaatcagcttcgaacaatccttcccacaccatatcgaacgcaccgttccacgcattgaagtgatgcgatgaatacgcaccgtcgccaacactacaaagaaccatgtactgatagtctttcacgcatgggatgttgtagttgttaccacgaggaacagtcgcactgttattgttgaatatacattcccaaccagtacgatccgccgaacctgttgttaagaacagaggacgacgaatgatcatcatgataccattctgcccaccgttatcgctagacctttcgcagtacgcattgcagcgtaaggcacgatcaacggtaaaggtagttgagttggagaagtcgcggcagtagtagttcgaaccccacttcggcagatactctgctggtggtacgaagaaatgacgttcagcaagttcaacttcaccgtagcggtcatacgcgaatacgatgtactcgaagcctgcttcaatctggatgttgtgcccctgagtgccgacaccattccatttccagacaacttgccaatcgttcgtatcacggtcaggcagttcagtgataagctgataaggacgctcatacacatgccacactttcccttcttctgtcgtgttgatatacagagaactaggatcgttgatgttaccgttagacgtaccgcaataaactttatgcgatgcaccagcagagttatagatagtgcctgagccgattgaactaaacatgtcccagttcatcatcaggtgagaggtacacatttcgttctggccatcgccatccgaagtcgtaagcagatattcgttcaagtctttgaacgcatagcgaacgtagttcgaaccagcacggttaacacgatgtacccagtcatgcgattgaaccttcggcacagggaagcatgggttagtgacagacacgacgaagtttttagtttcgtacataggcagtttcttgaagcggttatcacgaatcgttaccgtgtgcttcatgccataggtttgtccaccatccattccacccaacactttgtagtacgactcatgcgcactcttggtgttttcgaacaaaccagtaatgcccaacgcaagtgtaccatcacgatctgtaccggtgcaataaggaacgttgcccgaatcgaagtcaaagcctaccgagtagtagctatcaggtgagcttgatttggggccccagtacagttctgtgtgcgccgaaccttcacctataccaggctcgccgaacacacaataggcagcacggtacacatactgactgccttggaacacacggcgcgaggcaccaatgcgatacatagcagcaggaagaccgccctgtacacggttaacgtcggctgtatcatacgacacaacgaagacataacagtctgtgccgattgagttgaggaacgcagcacaggcagcagcattagcaacgccagggttagtgccctccgcagatgcgtgaatgtcaaacgagcggcgttcaagcagcgcaagatctgatttacgaatcttatagacgttcaagccgcgcgtatcgttatactgggtaccgttgtaaacagtgtagccgtaatcacctgtatcgagatgacgctgatatcctactacatgcgagaacagtcggctgcgtgcctgcaacgcttgaccattctgattcgaccacgtgacagatacatctccagcagcaagacgagctgcccaatcatcaggcttgtatgggtaggtagtaacatcgaagttaacaccgtacgccgagccaggctccacacagcatgggtcacgatagataatagctgggtcgagaatcacatcatctggaatatcaacctgcccacaatacagttgtttccacgctccaggctgaccgccgagtgaagaaggtcctgctggaggagttgtattaaactgatagattgcagacgtgcgatagttaatctgattatgaagctgcggaacattcgtccaagcaacatggttgcctaatgcgttgatgctcttatcgtgcgcagcctttgtggagacgacgtatgcctgtccgttactgcgaatgcctagtgggttgaagatagcattgaagttcacgttaccttcatatgcgttcttctgcaatacgattaaactaacgccgttgcgatgcgcctcacggagcgcggtgagcattgctgtgggcatactttgattggtggcagacagaagaagcattacacagctaaactgtttgaaatacttatacgagccgtcatagccgtatgcaccagcgttgatttcctgccagctgtgtgcaagcatatccaaaggcatacgctgcatgtaaccaacaagctgaccccaggactccatggatgtatcatcattgacaggagctaagtccgagatgacaagcatggaagtgccgttagtgatatttgaattgtaaccacgttgtgtcagaaagtgacgcaacgcgcccatgttgttgatggtcttgtttctgtagttgccaagccacccgtatgaggcatccaccagcgggctaccatctcgcacgaagcgaccattcataaacacagaaccaaagccgcacacataagctaaagcgtgtccgtctacaacgaatgacgtaaaacgtgaggcatcgacacccatagcatctaccgcagcctctgtgccattgccaggactgccgctgaatactggagttatgcctctagcatacaagcaactttgttgtagcatgttatgtccttaagatcggcaagaggggccgaagccccttcttttacccaaatactatttcagtgattgcaagataggtcaagtcgttcgagtcgcctctatctcctccgccatgataatacagccacacctcttcacctacagggatgttcgtatcaaacgtaaagcgttggagaacgttagacctactcgatacatcttgttcagcacctgcgccagcgtaacgttcataaatacttatgttatgccagccaccatttcggccatcatacacccagtcaaatgtgatacgcttgattggtcgagtaaagaagttattccacttgaaccaaccactggtacctccccataagttcttgtagtcaccatcccacgaagtgaggttacttacgtcactgctaataccacgtccacctgtttgtgcgaacgtataacagtaccaagggaatgtatcagactcaggaggtaacgcgctgcctccagctatagtcacgcaacgataaggtacagtgaagtcactcacgttgatgtgcggaggctgaatagggcagtacacatagtacgaccaatcacatccgataggtgcagtcacgcgcacagtgatgttagcgcgaagcacatgctcagggtatttccaaaattcgagtgtaccagttttcccagctacaacgattgacgtatcaagcaggttcatgttctggtcaaacacttcaaacttcgtatcaaacgaattggctacacaaacaacaagctcggcgcgtatatccgtttgagttcctaacgcaaaattatcttctgtagttggatgaccggcagagtacacgctatagctctggcatgggtgcatgaactcacgagcaccgcgttcgcctgggcagtacaagctgtagaagcaactggccagtgaggcagcattaccgaagtctttgctgaccacacgcaccatgatatcacaagcaacgttctgagggtcgaagtagaagtatagataaccttctcctgtcttagcgtcaagcgtagttgcgatacgacgaccagattgatagacctcaatgaagtcgaacgtttcccatgatgtgtaatcgagatacatccagcccgctacccaaccgatgaagtgataatactcaaatgcgttagcattctgaatacgatctgcgattggccaaacagttgcatggcaaggcgcagggaagattgggctgccgatatagtcagggtggataacgtcagggaagttgataacgtcatacgcagcctgactatcgagcgctaacccaccacggtcagaaggtgcagcaagtctaggaggatagacttcgagactccaaccgaacccctgagtagtacgaacacgcaccatgatacgcatgtcagcagcgtcagggtcgaactggaatttgatacgagaacgtcccgtaactttaccacacgtcgaagcaacacgcacacccatatggtacacgtcaacactcgcacctgcaggagcatacgaggcaatcatcagctcaacgtaaccttcaacagcaggcatggcgtagattgtttctgtgattgtagcgccacgaccatgaacagacgcataaggtacgttagggttagcgtatgtacctaagccggaacgagaagcaacaccaacagggtcgtaagtctcgatggctttgatacctggtctattaatcgatcgaccagtcggaggagcaaaggaattaacgagaccgaagccagtacggccagcatccggcaagtcgaagcctgctggatagcctttgagtacgtcatacttctcacggcctcctgagccaataccgttgcctgagcctttggttgtagatgtaggaccgccgccacaagcacccgtctcgacattcgaacacgggtcatcatatgtagggtcaaacgagtcatcaataagatgccagcgcttgccccactgattacggacgctgaacttctctggggtcagaggagtccagtcgccgtcttgtgtgcgtatgaacatgggcgtgtccacacaatcatgccaaccgttattcgcagcattacgaacgcgaaaacgtgccacatgatctccttatgggcgaacccaaatagcgccggcttccacctcattgtcgatagcagggtccgtatcctgtacgaacaccattaccttaccgggattgccgggagaaccagtaggacctgtcgggcccgtaggaccagctggaccacggttgcctacatagccttgcttaccttgcagaccatctgaacctctaggcccagggcaaccgtcagtaccacgacgaccatcaccgcccataagaccgtcaagaccatcacgacctgaaggacctacgtcaccagatgggccgtagccgatgctgtgaatagtaggcagccctgcgatctgtatcttaccaatcgtagggatgttcagtgcgagtacaccggtgagttggtcaaatgaaccgctgagtgtactatagtcttcttcggtgtctactgtcacaccgccttgagtggctttcacaggaccagaagcattggtcttgagaagcgcaatatcaactttttctaccatgattactccttacggccaggtagtgccttgatctttagtagggtcgacccagatggtgcctgcggcaactgctcctggctgggtagcactaacgatgatagacagacgacccgcaggacccgcagcaccggtaggaccagtagggcctgtagaaccagtattgcctgtaggtccagtacctcctcgagggccggtaggtccggtaggtcccatagggccagtacgtccatcaggtccggtaggtcctacagggcccggtagaccatcacgcccgtctggaccaggaatgccttgctctccgtcgggacctatattaccatcacacccctgttcgcccggactaccatcacgtccatcacgtccatctttaccatcagcgccagtctcacctctaccgccttgacgcccttcaggtatatcagaagcagtagggaagccttgcactttgacagtctgaccattagcgaacttgagagtcaagattccgctagtcgcatcaaacgacgagtcacctgttagttctgacggcacctctgagtcatcaggactgaccgttagtgtgcccttagaggcacgaacggcagtaggcgtagaagacgcaccagcttgaatgaggccggtacttactttaatcagacccattacgttttctccgctttcgcaacaatatccgtattatgcacaagcacatcaccaacgaagtaacagtcgaatgggtcaacgtcgatatcgactgtctgcacttgttcgtctacacgacgcatctcatatacagagataggtcctttgcgaccaagaacagtttgacccgcttgcacatcacgcgcaggaacatagcgccatacgatatcatcgtaaatcaaaacaggatgttcgtgcgtgaacttctgtccattaatcacgtagtaatgatcttcttggccgcgcacgagagctttaacagtcgcgtatacggttgtgccttttatgctaggcgaagaccatctgcgaaactcttttggctgattcgaatagccaagtaacgcatcaccaacacgtaagtcttcaactgctttcggaccaacgatagtgttaacgacagagccgtacacgatacagccggatgttgcagtattagtagggttacgagccacaacagtaagcgcagacctaacagtaacagtcggacgcgatgtttgacccatatcagttaccagacagctaatggtgcctttgattgtacgatcagcacctaagccaagtctcaggtagaagttaacaatgcaagtgcttgtctcaatggcatcaagagtcacaccctctgtagttgtgatagtccatttatacttatacggaccgacaccaccacgcgcattgacaggtagatatgccagcgacgtaaacacatcagaaccctgcactgtacgttgaccaaccatgtacaggctagagactgacgcagcaagaggcgttattgtaggcaggggaggagcaggagtaacgttcgtcgtagggtacaaccacacgaatactttgctatcgagaggctgcgtagacgaaagaactgctgtagttataggagcgggtccggtagcgccagtagcgccagctatacagctagggccatcatttcctttaggccctattggccctgtaggaccggtagccccgtctggccctgtaggaccgtctggacccatgcgaccagtatctccatcagggccgtcttcaccgtcacgtcccggttctccaactggccccgtcttccctctattacctacaccacccggacaaccctgtctgcctgtctctccgtctcgaccatcacggccaggacgaccgggagagccaggagcgcctcgacgccccggcttcccttcaccaaatactgatacagtaggcagaccggggacgttaactacatccccgttctttttgatgaagactaacacaccggtcttgctgttaaatcttacgctggcgatttgtgttagtgttgccacatcggagttttcaaattgaacacctccgtcaacgccgactaaggatttaccttcgtcattctgcgttgtttcgacttgcgaaagttttaactgtgttgtcatttcggttcaaccttaatgcacaagttaccagtcagcttcgagccgtagctagtgatctgcgaatcggtgatacgcaccttagccacgatatcaatgaagccctgaggttggttctcaataagcacggtgaacatctgcgtcaggctaacgttagcatacgcaatcacttccgtaagattggcgtcagacgtgacaacgttgaatccagcgctgcctgtgccctttaaaccacgaccgtattcagcttctgctgtgcctgggattttgaacgacagaacatattcaatgtgctctttaccgctggtggccgcaaagcctgggcccagttgacactggaagtcagcgatacaggtaagcatcacacctttcgagaagtcgatacgctgagtgatagtcagctcctctgaatcctctactgtctggtggatgttgaacatgttcttcggatcagcttcttcggctaatgcctgagtgttgctgatagtaatctctggccacgtacccttaatcagtataccttcaccctgaatgatggctggtgcagcgataggcacatcaatcggagggagaccctgacgcttgaacatgtaaccggttggcgtagggatagcgtcaatgataacaccatcaacagaactatcttttgagcctaccgccatgacgttctcgaagatagtgacctcaacgagtgtgtcagcaggaacaggtgacgttgttttaatcacgttaccagcgacggtgaagtccataggatgtactgtcagaccacccatggccataacgcagtgcgctttgtttagtggtgtagtcggcagagtaaatgtatcagaatcataagggaagcgatactgaccaatacgaatgcgagtagaccagttggcgcgttcttcatagcgagccacatagaatgagtagcgttgtcctgacgggattgcttctgtcagcgttaccttgttacctgcgttgagcttgtagacagttgtaggctgccacgtactaccaacgacgcagaagatcatgtccacgctatcaatcggcttgctgcccaaagagaacgtagtggtttgaccgtcaccagtaccttcatacgtttcaaacagaacaacgtgaccttgagaaggttcgatgcggaactgtctcaagtcaagagacatgcgctgctcagggaaagatgaaagaagaagctggtcatccacaacgctatacgcggtacgcggttgcaagatacctgatgttccgacaaacaaatcagtcgagctatcgaggttctcggtcagcgtgtatcgcatcttatcaggcgtagcagtagtcaccacagaactgaacaacatcttaccgggaggtacaaacaatgttgctgtggtctgacgcgtagagccaccaacaggtgcccaataaggcttgttgtctttaccgcgcattaacgcccatgtgtcaggcacatcgttattgtcaggccaaggcagaccggctgatggtgttgttgggttagtgattcgacgccatactgcgatagtagtctgagcactgataaacggaatagggtcgtcttggttaactagctgaccaccaacgtacttgaagtgacgacatgcaccagcaccagtgcctgcgattgtctgaatgatcacaacttcattcgctttcagagttgcagcaaggctggcaatcttaaacgtgttggcgttgatgaacccagcagtcgttatctggccgctgaataaacgatcatgctcgctgaatccccagtagtaggagcctgcgccgtagcgataagcaacacccggagacttagagccgtcagagttaacatgtaagtcaagtaccgatacggcattgaacacgttatcttttaagctcggcagattttgcagcgtagccacactaggaatagaagtgtagtccgccattttaacagcaagaatcttttgaatgtcctgctggatatgtacgagcaagctaacacggctgatagagttcggtacagcgatgataggctcttccagaacaacgtgcccgaatgggcggttatccgagagcatgatcaacagctcacctacacgcttcatctgctcgccagcaacgtagttgattttaatatcgaagacaaatcgggcactgttctcggtaagtacctgaacataggacagggcgcccgacgcaagctcgttgccaagtaactgctctggaaccactgacgggtttgagcctacaaagtcacctgctttaaacgacactggctgaattgctagtccaccagagttagcgttcgcaacggcctgttctccctgaggcgttagacgcagagcgtcaacgtagatagattcagtggccatcaaagaactccttgggttttaactattctaaattagcaagaaacaaaaagggagccaggaacaagcgctccagactccctttattttactgatagcgcactgtgattacggcggtaccgaacgcacgagcattggtgcgatagatcaagacgttttctgtcaagttatcgtacacgattttgcccacgattggtcccttcttaccgttatcgccggtgacaggccactgagcaccatcgaacccaagccatgacttattcacaacaccagcactatccgccgctgccgcaaatacagcttgaccgtatgactgcctaacaacaaagtaaccatactcgtcagtcttggtcgatagcacaaactgaccaccgacgttcgaacgtaagcgcgtaggcaactgagccaatgcaatactgacaccagtaataccaaatggtgcgatgccgaatctaggataagaagacatagccttcatgaagtgcgtttgctgtaggcgttgctggccttcgatatacagagctttcacaccaaagtcagtatcgttcaacagcaggccaatggtcaggcgcccagtagaagcgttgattgaaatgccttgcacatcaaccacatcgcctttgctgttcgttatctgccacaagcacttagcactaacatcatccttcacgaacgtgccggtacgtcctagcattgcgttcatctgcatcgagctatcatcacggacgttggtgtacccaccgactgtcaagtcttgtgggaagcctacgccaggacaagtaatctcttgcaccaaactgatttcagtacgctgctcggtgatgatacattcaactttaactgtctgtgggtctttcgaagcagggaagcggaaggtaccgtcctgcgacaaactgaaaccactaacagattgaatgacgttccactggaacttaaccgagttggcgtcaggtagagcggacgatccaccagcgcctgaacgacgttgatagtacgcaataaagcgatagtccacattagggttgatgttacctgcaggattctcaatgtagccattaagaatcgtattctgcgtctgcaactgaatggtacgagtaccaataatcgtttcatcggcaagtgactgagggttctgcttggtgaacacagcacgaagcccgatcacaccatcagagagttgagactgcccgataaacagatgcccattgaggttatcaatagacacaccatccacgtttgtctcgtcaccaatcgaccacagtgcatcagtcgaaaggaactcgtcatcagggtcgatgataacacgcagagagtaaggcacgtaccagcgtccgttctcatacccaatagtcgggttacggtcagacacatcccacacaacgtcaggacccacgataccgatttgtctcagatacgtgttggcctgaacaaggaataccagtaatgtcttctcgatctgatactggtcgcaggtgaaacgcgcacgaataagcacagcaccattaacgttctgtctcggtgtcagagaaccttcagcatcaatctctgcaacaatatctgtcgtaggcatgagcacctgcgtattgttgggaccttcctgcgtgtagtagttctgcactaccgaccattcagaatccacttcgagatcaaacgtcttagggttttcttcaacatacgaaccatcgagcgttcgcattacaccgccagtcttgtacgtgttaaccagagtgtatgactcggaaagcacgtcagcactgatttgcgttgcaccttcgatgcgactgttgacgatgttgttcacgctctgcttaggtgtaggcgatacgaccaaatcgatcttattgcttacgcggaagaatgaagcaatgacctgagtgtacacatcgtagtcatacaggattttacctgtctgtaggatagcaccatcgtaatacgctttatccagatcagcgagactgccgatcgcattgaacataggcaacttgcttacgtccatagagcggaagtctttatagcttgttggtgtgcgtccttcgatgatctctacgacggatgtgcctgagtaacgcgcaggactaaactgcaagaattgatattcatcagtgtccttgtctggccagttacctacccactctgcggcagtcacatactcttgagaaccgtcaacataagttgcaagcagacgaacaaacgtgcgcgacttctcatacatagtatcggggcactcaatcatgatactatccaccagcgaacgcgcaggtataagttgcaggtcgcggtagttagtgagcgtgtgtccttcaaactcgtaggtcatgttgatacgcgcagagccgtgcaggtcaccctgaaaataaagcacatgctctttcacgctacgctgcataacagggtcatacacatcaatcgttgagaagctaacgttcaacgtaacccaacgtgcatagtcaggatgatcggggtcaaactgacttgggtcctgtccctgctcaactgcttgctgctgtaggcgaatggttcgtgcccttgcctcctctttcgcactatccgatggcagatactcgacagtaacggcagcggccgcagcatatgagagtccgttgttccacagacacaacacgggtagcatcaacgacgaaccactactgatagttggagagctacgtaggtccacagacttaggaatcatgatcgtatcgttaatcatgatcgtgcggttgaatgtgattgcagtgctgccgtcaatatacgagaagttgagaacataaggcacagcgtcgccatcgacaagcggggcttcgaactcacctgtctgttggtcaacacggggcagagcatgtgtgcctgtggcagtatcttggctgctaaaccagatgccaaacacttctgcataagctacgacaatcgcagggtcacgcgaagcaatctgctcaggagtagcagatgccagcacatacaaagccatagccttgggtcgaataatatcacgctcaaccacagtctcaggaacaactaggtcaatcgtcgccagattaatctctggtgctttcagagtaacctgcttcaccgcctcaatgggaacacctgaaccaaacgaagcgtagatagacgttagatagtcttggcgtaataccttagacttcaaaacgttctcaacaatctctgtatattcgctggtggtgcgagcctgcgctataccgagtttggacgtaccatcgttatacgtgatggcgtagcgtaggtcgaactcctcaccttgaggaatctcgtcatcaacgatgatgcgcagctcagtaggaacaagctcaatcacacttcggttaacatcgaactcttccgtctgggacatatcaaactgaccctgatactttacgttaatgtcaatcgttgtgtctgcgtcaacactaggaagtattaacgttgtaccattgaacgtaccaagcgtggagctcaaagcaatcatgccgctgtctgtcagttctttggtagagcctgtagcgagatacttaccatatactctgactttagcgcttgcgttaccgaatagcgtagggcattcgatcagcaattcatctgggtcaggctcgacacccataggatagatgcgagactcaagtgggaagctggtggtattgtaggtaagagtcaggttgataaccgatatagctagaggctcattaaagcgcactgcgttaccatcacgctctgctatccaatccgagtcttctacccagacctcgactgtttcttccgtgttatcactgtagctgaccacagcaccaaacgtagtccactcgccaccacgaatgaactcaggctggatgaatgcgatggatgactgtagaggtcgcccaacgttgaaacgacgaactgattcgacaacgacgtgagcgccgaggtataacttcgcgccgagattgaccgtcgcatagacaccctccaatacttcttcgattggtgcccactgatagaacaggtctgcgatgcgtcgctggaacatagcactacgcgccgtaaattgttcaatatcgttattcacaggttcaaagccgatgtggttgttgaaccaatcctccgcttcctgctgtgtcatgccaacttcttgcagtgcgttaacaacgtctttctctgcatctttcgtgatcgtcaggtcaataccaccgtcgatcagatgtgcgtcaacttcgagattgaccttgttcgtcttgtaccattgaccaccatcttgaatcaaaacaccaagaggtgtaggcacaaacgtttgatagtctgctgtgtacatgcgagtagtgtcgaactgaccaccaagcaacatgcctacaaacttaggccattgagttgtaccagatacttgctgccagtcaggcaggcagtcgatgacacgtttcaacgaaggcaaacgatactgcatcagatcacgcgtgatgttgatgccgagctggcgaatggcggcttcggccagctcgtcgtttgtgtctgccgtgatgcgacgaaggtccaacaactgttggatgactgccaggttatgttcgtcgttgtgtgcatcgagcatctcgaacaactctgcccacgctggattgctttcgagaaagtcaatgttgaaggctagagtgtttgatttcactggttcatcttcctttcgctatacgtgatattgatgcgaaggttacgcagcgcaacgtattcgaggaccgtgttcggaatgatatcctgaacagggctttcaatgttgcagtagtcaacttctggtctacgtgctggctggtctacgtcggtccaatcatacaggacgcgatctgtgatatcagatagagccaagcgtttacccagcataccaggacgacgcttgaacagttcgagcacggacgcttcaagtaccgcctgatttgattcgcgggtaccaggtgcatcagcatacagagccacattcaacgtacaatcaatctggagcttatctggattccatgattgcacatcgagaggactatggaattgcgccaaccagttcaggaacttagtccactgtgcggatactgggttaggattgatgcctccccaagtgcttgtgtttctaggcaatacgcacacacgcacaactccttgccactcgcggtcattaggtgcaatctctgcttgaccctgaacgacaacatctgcaacatctgggtagagagcaatagcagctttccattcatcacggcgaatcagttttttacggctgcgccctacgataggactatagttgcggtagtagtcaacaggcgtttcatcagagccacccaaacaggcgctcacagtcttaccctgcaactgcgagttagacaggcactgtactttcagtccgatactgtctgtgttgccgctggcaccaagcgctttgatgcctcgcactttcaacgtatacccaacaggaggctgtgctccccactgctcaccaccaaattgaatctcaacgtcgccttcatcggttgttacatcgaggaatatttgttgatcagcatacgcctcaaacaagcacttatcgaagcgctgatattcaatgcgcgtaccagtcgggtgttcgaaccaaactcgtaggtcatccgtaagctggaagttctctgtgcccaatttgattgacatgtaatcggttgcactaggaacaatctggctgaacgtgaatgtttcagcgatgatgaagtcaacattcttaacctcacctggctcccattgagttacttctgcaagcaacgcattgaaactaccgatagtgaacggcgtatacttgtcgtaagattgctttacactactcaggttagcaaccgaagcagtaacagtagatactgacttacggccaatatcgacacccagatagcgagcattcgcaagtattgaagtgttacgtctggccagacgactgaatgcctcacgggcagcaatcaagttggcatatgagttcgtaacacccaagtcaccaagtgcgtctgcaagcagggacgtaagtgaactgacctgtgcgtctgtccagtagctggacttattgatacgattcaggaagtcctgcgcgaactcctcatgcgaggtgtatgtattaagcatggacatgttactgtgccctcatagcaaacgtaacggattctttcgattcgagcttaggacaacgccatgtgataacacatacataggtctgctcgtattgatcgctcatggtacacgcggtctggacattcgtcacatcgtttgtcaggccgttagctctgtcttcgagagcaaggcgcatgtacgttgcaatccagtcggcagtagtctggtcgaaaggctcaaatagatactgatacacatcagcaccgaaggactcacgccatttacgtgttctctttctggtacctattaccatcagaatcttctggacaatgctgtccatgttctgcacgttatcgcgaggttcgagttgaatccacgcattgatatcacaatagattcgttcgctaataggaacgtctattagtctgactccgattccagccattagccaaatctcacattaggactaccgttagatgcagtgtcgccacaactgttgccgtcacccgcacgttgggcaggcttaccgttaacacgcacactcgaactggaagtagctttacctgtatgaggagggctgtctttcttccagtgtggcatgtacgagtcgccctgtctaacgcttccttttccgttaataagcacgttagcagacgcctgcgcagcgactacagggaagtagccgttatgtccagtggacttgtctgtgcctagtcgaatagctttctgtcccatgaatattctcctctgttagacacaaattagcttgttaagcagtagaaacaaaaacgggcagcctaatggccacccagtttctgtacgcttggatttgtgtcgcttaactccctcacacccgaagcgagtgctcggtagccgaagctactaagccggagttaatggccgagagtgaagccgcacggcgcggcaacagcatgtgactctcgggaccagatagcaagtgaccaagcatcgcaattgctatcaacgacactaagaacaaaagcatgtttcgctccttgtgtcatactttaagagactacgtttgatcaactggtactttgctctgcccgtcgtccaacatcacttgggtatcagaacgtttctctgtttttaccgcctacgttgcggcaagccgcgcacgacactcacatatcaaggacactcggcggaaaggggaagttccgaatgccctaacaacatgagtgaagcgaaggaggtcccgtatcggtgatctgcaggggttcatgcacgtttaacattcgcttctttgtgcgttaaaccctcgaggacccgaatgccctgctaatcattccacgaggatattgcacaccttagtgaacaaggtttcaagctatggcagcacgtcaacaacagcggacacactccattgcaatctgttaagggcagagtgcaacaggctgtgaacagcttggtcggaataggtttcgctcgtcgcccaactccacttgagtatctcgacctaaacttttactctccacgcgaactacaaggaagtgccgcgcttctgtggcctgcggatgtttatcactctcagactcttagctcctgactggaaatcaacacgttgagtcgtccgctggatgacgtgttgattctcctcacctcgtagtgcgaaggccagaacaggtgccgatggaattgtcatgaaggaatccctgggggtcatcgcttcccaatgcacacagggtgaaagtctatgcacatcaggcagcgtctgctgcgatactgctattccctattagagtggccatagcgttgagttttcgcttcgccagtctacatgcctgaaggtatatgccgtgccaagtatgtatcagcatggttcctgctgggccttttgggcgtcagcgacagagcacatattcatcacgtgggtgccggggttgtcctcacgattacagagcgaactcaaaccggctggaggcttgtatgctcaagatgcacatacaagtttgcgcaggaggacgatggccgctatgacacatcgttcccttgagacatattgatattactatctgcaatttttatttacagatttcagaatgcttttcgttccacattcgaataataagtttcgtatgggtcagagtacaactcaggaccacgttgagcacgtacagtcacgtaaccagtgtgacggttgaacgcgatgatttcgacggtaggctgcttaggcttaatggtcgcataaatcggtgcgttcattgtcggctcgtccttctgtagcatatttacagatttcagagcttcaccagtaagcgtaggcagattgaatctgatctccgcacgtttctggccgaaagcaatcttgattgcaccagcaggcatatcgacgccgttctgcttcatgtacgcgccaatgcgacgagcgatacccgtcaactggtcacgagtacgcgggtcgaaagtaccttcaaagctgatagcttccgtaggctggcgcacagacaaatgcaagcctgtgttaaaatagccctcagccagcagacgcacaacctcctgcacgatttctttcgtgttagatttgattgcagcgatacgcaaatcaggcacatcagccttaatagggtcacgcagttcggtctggttatccatgtagccgagggatacgtgcttcgctttggtgtacgtgtgttgcaacacaccagtagcgcgaatcaagacggaaccagacttagcctgatcgtacagttcatcgctggtggttgtgctaaacagatagtagtctgtaggcaccgccatacgattgacagcttcgacagctttggtctggacttctttcactgtcttaccgaatacgacacggctgcggtttggctgcgatgcggacacagggaagaacgcaccgtagacaacctgcacgttcttttgaataggtttctctgactggactttaatgccacccttcagaggaggcagcttcatgcccaccagcttaccactaacgattgctttgttagcgactacaggcttgaggccggacagaagtttctgcaactcagaaccgtcaagaatcttctccagcggaacagctaagttttgtgccaggtaatgcttcttacggaacgagtagataaccgtgtctttcttgatctgcaacggcgtagccatattgcgaccaatctgacctacaggctggaaggtgtttttcttatcgtctgccacagagccgaatgctttcgtgaactccgtctggccgatgatgttagcaacgcgctgatgaccacgaacaatgaagatgatcttcgggtcgtctttcatgcgcagttcataacgatctcggttgagatacgtcatgctgtacttatcgcctttctccaactcaagatcgtattcatcgttggcgtcatcgacaacaactttcttaccttgataggttgcgtactgacgagcaggtgcggaggtcgaagcgatctccatagccttacctgtgttagacagcgcaacagcgaagtcagtcacagcaggcatcaggtcaacagcagaagcaacggcgtagctattacgatgctcaccgagatgcagatgtacggcacttgaagcggacatgaatacagtgttacctgtgtcttcatgtttacccgcaaagttcataccgctaatgcgttcgatgatgtttgcgcttaacgcagggaacgagatatcgctaccagcagtgaagtcgaagatttcaccctgacgccatgcgtaggcaacgttgttggagctaagtccgataaacgcatcgccgatctgtttgacagtcatcggcatgatactcaagtcacgaatgaccgagttttgcttttgaataagattcatataaatccctaatacgaaacaaggcggaaggcgttctgcttgagcagattgagattgcccagcattaggctatacgccaatgtgccgtgctgttcaagcaaactgtcaggaacaatagacccgaagtaaatcgagttgtctggccgaacattaatctcctcaccactagacttcattgcgtcagggacaacgaagcaccacggttcagcgatgtatttacccttcacatactgaatcctatagccaacagccatgtgctgacctttggttgggcggcacgaaaacacatccgtgttctggttacgcgacttgcgtaccgtgaacagcgccatagtcaaaaagcgttgttcgaactgcgggatgaatgcgttatcttcgcaaatctttttcagtaccgcctcttgtcgagctttaggcatcgacgagaatagatttagattcatgacagccgagcgagaatctgacgaacaacatcagagacagaattaacctctgtgtcaatgaccaaatcaaagccgccaggcacttcaaggtagcgttgattatattgttcgtacacttctttggtctgacgcttttcgatgcggtcttcaccgccaatacgaatcttacggcgctcaatagacgtttcatagctacacgtcagaagcacggtcaggcggttctcaggagcaagtgcttcccaagtgtgctgatagatgtgcgcgttaacatcagacgcaccagcctgatagacgtaagtagaaggataaccacgatcggcgataatgatcgtatctggttcattttccagaatgcgctcataagcattcatcgttgaggaacgtgcagcaaggaagagcagcagttcggtacgcgagtccatatcctcgttgagagggttggtgttggacagcagaacatcacgaatatgttcagcaagtggcgtaccgccaggctcacgcagacgtagagtttttgcaccacgttgcgtcagtatctcagacagcgcattgcacacagtggatttgccaccaccttcgccgccttcgattaaaatataggttgatttcatattgattccttaggcaaatcgcccaccacgccatgcggccttaatgagcaacttcgccacgatttcgttcttcattgtctttcgcttggcgttgcttctgacaaatgcagagccgaacttattcacgacgattaggccgcagcctaactctttaatgcgaccaatgatcttgtcgccgtgagattcaaacagtcgttcatcaatgatgaagtacatacgcatacagaaaggcaaatacttgtgccacttcttatcggtgttgaagtcagcccaacaactcttaacctcggtgataatcatatcacacttggtattcaggcagaatacatcagcccgtaagttgccatgcttaatcagaccaagttcaacgtggcatgaatagcgtttgtcaatccagtagcgttgtgcagcttccgtgagaaaggccgtcttatcaggacggctcattgatttgaacacagcttgaaggggttcagctttgcgccgcttataagccatacgagtcgataatgtccagggcttgcgatactatcggtcgaagtttcttatcgactttagtaagcgccttatccgctttaaaccatttgcgttcgcgtgtcatggcttcgtcgtattcagtcaacatggtcttgaccttcatgacgaaccattcaacgtgttgctcacggccggtcttgcctttgacgtagcgcatgatatctacgaagtctttaggcttaccgagaacaccagcttcttccattgcttctttaagcgcactgtcgagcgcagtcattcccttctccacgccgccttttgggagaccccagttgccagcgtgtgtggtgcgaatgagcaagatctcaatcgtaccgtcctttttctttctatatgggatgacgccagactgcttacgaggcttcttctcgaatggcagtttggctgacaatgacacgcgaatcttcataagtaatcaagtcctctcggaaggtcaacatcccacgagccagcgttgtctttccacagaccctgatgttgcaactccttatacgcatcataaagagaaacacgagcctgcacagagagttcgttgatacccgcggtgcctaagctgtatgcgtacatacagcctgggaagtattgtgtacgattggcttcatgtgtgtcaaacacaatctggccctcactgttagaaataacagcgtgggctgccataccaccttgaccgagaatgacgatatcatagtcggggtgctgtttgtagcagcgttgaacatactcggcgcagtctgcaaatggtcgagctacagcagcagcgcggttgcagttgaactgggcagcagactcagacagagaacgtgcgccagtcagattcatagccgaggcaaagataagagttgcgagcgattcaggctcaacggcagtggggaaaaactttgtgccccacgcttgtgatagcgaaagcatggacgtctccttatacgatagtctcaactaaattagtgtgcttagtcttctgggcagataagcacctgacgaccctgttgataatagctgtcgggtgctcgccctacaacgatagcgcgtttgcacataaatgcaggcttacgcagagcgacattgcagcctccgtgagataacacggcaagcgcttctgctttacaaggaccagtcagacacagcatatgcgaatagaaaggcttctgcgccttcttcatcgtgcgtgatattaaggcacgaatacgctccgcttgttgtgcggtaggtgcatgatcgcagtacacagcgatgttcataatcagtccttaacagtcagaagacctgcgtaaacaccgaagcgatcagtgagtgtagcgagagcgccatgcacgtcaccgtcagaataactaaggcacacagcattagcattcgacacagatacgttgttcgcaccttcctcgtacaggaagatggtagccccgtcatgcttacgtcggtcagtgtagaacagaccgtacgaagtccacgaattagtgccgctttccataacatatacagatgcctcaaagaacagggattcgaaatcgagagcattggcatcaatgaagttacggtcttcactgtcagacactaccacgtcgagagtgatgaggtcaattgcttctggcttggagcgtaaccagatcttcatgcaactgtctaagtagtcggcgatagcacaacaaatacagctacggttgttcgggtcacgttccgcacgaggtatagcagtcagaacacggtcgcttattttccatgagatgtggtctgtctcaaggcgcccgttatgatactcataatcctcgtctttgatcacaaacaggttggtacgctgcattgcaatgttagacagtacgtgcttggcgcggttaatcaagtcaggtgggaattgaatcataacacgcgcggaaacgacacgaggaacgcctttttcgatgtaggcgaagttcatcgtgcgatgtaaaagagaacgcataatgcttccttagttcaggttgatagtctgtccatttacagttacatcctgaccagcctcaatctgaatgccacctttcacatcaagcacgtcatctcccttgacagtgatcttacgactaccaccaatctctacagtctggttgcctgtgattttagtgtattgattacctgcatcgttcttggcaacacccttaaacttgatgcgcttcttcgggtcaggcttcaaggacttaggcgtcatcacagggtcattcagaatgtagtcagggatatcgttcttactgcctgtgacaatcagttgctgattgcctacgatagtctggttaacatcgcccatgattgtcatgttgaagtcgccggaggtcacgagaaagtgctcgtttgtcagacggtcgatgataagctgggtgccagtagacagacgtacaccgatacgatgtgggtagttgacaaggaactccggtaacatgtctgcgtctgtcatacgcacgttggtattgtacataccttcatgcaactgacctgtaggaaacttaacactgactttagccccacgagtagggatgaatgacgcgccgaatgtcacaccctgattaccgcctttaagtccttcgagatgcccgacagcaggacgaatccacggaatcatttcatccgcaatatcatcagtcagacccataatacgagcacgaatctgacctatcttgcgggggtcattgttgtcgataacgatagcctcataatccatttgagggtcaatgcctttcttggcgttcacactgttaagaggaatcatttgttcacccgtggcatatacatttcaagacgctcaccgtcaggcgtaccgttcttgcttgaaccgtctaccgtaccatctccaagagagcacaggaagttacgcaggttctcttcctgctggcgaataagctgactcaggtttgtactcggacctaagagcttgctaatagacaaagcatcgagacacttatccggtaaggcatctgacaccatacggttcatatcatccagcttgttactgacacaacgctgattgatttgaggaccgtctaggtattcagcggggatatcaccgttagcaatcaagccgttcacatcattcgtgaaaccacccagcatgttctccatgctatccagacgcgatgcgagtccgtcgagtatgccacccttgtagttgattgcaaggttgacactcaacttctccagagagttcaggacgttacagataccagtcaggtactttgccatgttgaactcttgcatcaaagcatttaggtagtcaacgccttctccgtacttagccgcaagctcagggaatttgaacgcctctgattctgtctggaactgatcaagcatcacatcgagttgtaggctatgttgctgcgatagccagtcaatagggttcgaaccgtcgagtgcttgtttgatgttcgcattaatctggaacggacgcaggacgttagcgacagttgacagcggagtctggatgatgttctggccaccaccaatgttcgacgtaccctcaacaggagtgaagttacgactcaacaagaatgcttcgctatacatgcctccggagaacacgcgagtacgacctataacaagccatttacctgacactttgatatcagtttcaacttcacgttgaccgttgattacaccagcagatacttcgacaatatcaaagatatctacctcaggacatccgcctaagataagagcgcgagctgtctcggtgtacgccatagactgacgcttgttgttgtaatacgcttccatgtacttgtcatggatgttgatatcgttcgtaggtcttgcgtatgctttacgtgcaccagcaatatcaccacgcgtgtcgctgttaatgtttaacgggtcacggcccttcacggtcacggtagatagttcgttcgtcttacctttcgagtcagaccacagcagcttctcaccatagttagacataccgttgaagataccgctcatggatttcggtctaaactcatgaacgttatagatagggctatcgcctgtgggcttgtggttaaataaccagtacgcctttggttcttcatcaaacagcttgttgatatcacgcacgaccatgcgcttatcggccgtgataaacatcttaggcagggcttcttcacttacccacatgtgctgttcgatttcgtgcgcaaacttcttaggcgagcacgttgcagatacccagctcatgatatctttcgtttgcagatcgccgaagtctggagtcaagccgcccatagaggccacttgttttaatgcgtcaagggaggttccacgaatagcgaagctacgtgtgtcgaataggaaagtaggcgcatcgagagcacacaacacggtgagcattggactgcccccgtcaccagattcgcgtacagcaaacacagagaacgtgaacgtagacgctgattcagaatcaggtcctagtaccaatgttattttcgtgccgtccacaatcgcgtgggaggatcgtaatacgttcgtctgatcagagaatacaatcagagcgcagggcacagcgaatgtgttttcgaacacttgaacggaacgaatgagattcggcatagacggcggtgctttgccgtctaacaaaagaccaagaaagccttggtcctttacgccgccagatgtagcttggtcagccatgattaaccctcagcatcaagctcaatcgcaatggctttaagtttcgcagcaagcaacttgagttcagaagacttcgcctgcatgttaaagccaccgcgaccaggtttgatttcagaatcgtttttggtgttgtaccacttacgcacctcaacaacgcgattaccggcatcatcgttagcgagatcaacggacagaaagccatgaggacctatttgaacgcgaaacagctcaggagcagaagtctctacgcaagttttcttctttttctttgctggcgcttcttcgacaatctctttcttgaagtcttcccatccctcacggatagtattcttcttggatttcttttctttaggacgcttgagttccgtgtctttctcagacagaacctttggcgtcttcttgagagtgtctttgatcttcttcgctttcgcgccaacaattttgccgttaaccatagccattagatttgcgtcctcttaacttttttgattgcagcgctaggccgcttttgcggaagaacgacgagcatccccgctttaagttcagagggatgtatcagtgcgttcgccaccagtatgaaattccagtagacgttcgagccgtagttatctactgataatagttgtgggttgccctcaatcgaggcatcaatacgcttggacgttcctgtctgcgctgcatcaacatcctcgaatagcttcatgctaagagggtcaattccccacttgtcaattacgccgattgtttcagccatttacgtaggtcctcacgagtaacagcgaagtaactactcacctgaaggatgaagtccacgctgattgggttccctgtaccatcttcccacacgttgtcgaagttagcactaacgctatcgactacacagggactcatggagaagaaattaccaatatcaacgaagaacgcctcactgtcctcaagtataccaccaattgcagcattagcagcgtccgcactacctccgccagcagcaatggtcatagactccatactgactgacttcaatggacttggtcctggaggtaagagtaagccgccctgctcagaaggagcacacagcgaaagcagattgatagttgtatctactacttcgcttttcgtgtcagagtaggcatcgacaaagataggcaggtcgattgataagaagctcggccctccccacactcgcgcactcgccagtttgtgcatagaactcgcaccagcgaacttgagagctttgtccattgaacccgcagtgttaccaatgaacccaccaacagcacccagcttaccaccagcaccagacagagcgttaccggcagcgccagcaacatcagcaagtgaagtgttcatgaatggcgcttcccaagaagacgccaagctgaatgtgaagtcaggtggaatgaaacccgtaaacttaatcgtaccactcttgttatagattttgactcgatacatgttatcgacagagataatgtcatcacgagatcgagccgtacctatagcagtggcttgcccaccatcagtaggcattagatagttagccacacagactccttattacatgtagcccatagtgatcatattcagcatcgggtcatccatgaagataggaatcgcgtcaagcgtatgaccagcagcaggactaccgctactgttacctgaagaggacggcttagatgcagcgcccgctttcggttgattagcaacaggctgaggtgcaacagaaggctgtggagtagcaggaggttctgatcgagcgatatccccaggagtaactagaggttgacgctctacagcagcttccggctgtaccgtaggttcgatgcggttaacatcaggagcagccaatgcaacacgttctttgagttgccgttcgtattcttctgaacttgaacgaggtgcttctggcccttttgctgtaaggtcaggaagattctttagattcctatcgacagtagtgtctgcggtatctaaggcacctgaggtacctgagcctttaggcagatccgggaatttctccgcaatacgagcatccaatgcagcatccgcatctggagtatttacagctttcttcttgcgctccgcctctgccaccttgagcaatacgtccttctcgttctgcgctcgcgtcgccactgattgttgcgtttgcgccgaacttgatttgaagtaacgatcagtcgtcgctgccttgtaatcctgaatggtcttaatcagatcatcgtcggacatggcgttaacgtctttgccttgcagcgcattggatataacgcttgtgcctgcaccgtactgtactgccgtgctgtacatcaattctttcacaccagcaccgcgcttcgtcaggtcaacacccacttcgttctgcatcttcgcagcaagtggtgcatagtgagtacgcgtgatatagtcagattgtgctttatcaaactcggcgctgttattgctcgctacgtctttgtagacagagttgaactgtgaggtacctggagcaagacctccgaaacgctgcaagaacggtttaccttcagggctgttcaggaagttcatcatgctgccgttgtttgtagcaagctggtgcttcccataagacacaccaccagcatctccctgtccagtagagactgtaccgacaccacgaccgcccgactcaaactgttctgatactgaaccaagaccaccctctgcaattgcgcgttgagcgatatcggttacttgcttgctgtccatacgacgcgcaggttgtgctcgcatcggacctgcatatgtacctgcaccggagcccggcatgccacccataccacccataccaccaaagccaaaaggcatgatgacaggctgagggaatttcgctttgttctgattctctgcggtagtgtcgttgtattcgtccatcttctctttgcggtctttctcaccgtcagcgagcatcttgtccgattcatcagtaatcttttcagcgacatattcgcccacagagctaccgaagtagtcacccagtatgttaccaagcagaccacccaacgcagcaccggcagcagtaccaactacgggtacaactgaacccagtgccccacctatccatgcaccagcaatagcaccagtcgtaccaccggcagcacctcctatagcagagccaccagctttcttcttctctttagccttctcagcatcggtcagagtttcatctgcgtctatatgctgcgcttcattcgcataagacagaccgttacccagcgcaggtccgatgatagggatcttcttcgaggcaccagcaagcagcatactcgtgccagctaccgctaggtcttgcgtttcagaaggcggcttaggcaagtcacctttagcagcatcttctgcacgttttacctcaggggcgctaggcattggagtaggcttagcatctgaatcgggcgcagcgtcggtcttctgatagtccggtgtaccggcacctccattctctgcgttctgttcttcaaactccttctgagacctgtgcttcaaccacagaccaccgcctacagcagcgcctaacgcaagagcaagacccagcttacctttgatcttaccgaagcgactacgacgaggcagtctacgacctggacctctacgttcgcctcgattgcgaccatagcgtttaccgcgacgacgtgaacgacgttcatctgggccgaagtctccgcctccatcattgttgtcaggacccgggtcatcattagcagaatcaggtcctcctgctctgcccgcaccaggctgattaccatgtgggtctgacttagcgcggttcttctctttgaatgcctcgcgcttctcccactccaaccaatcttcgagagctttctgcgtcttggtcgaaacagcattgccgtcacgaatagccttaacgatatcttcgccagacttctcccctgcaatgaacaggtcctcaagagcagcttcgacttcacgaggattgggcggggatgctactgcccgcggtgctgacggagcttcttcactcgctgttggtgcatagcgcacacgagtgttggccatcttctcacgagcagctttggccgccctgttcttagcgcgtgaaccgggaccgacgtagacaacttcttcgtcatacatctccggatcataatcttcaacgtcatttgcagcacgacgtttacgctttgctttaggcatgccagctactgaggaacttacattgtccgcatgttcgatcattagttcgagtgcggtcagttctttctcttggggcttagccattatccacctctacgacctcgctgcgccgcaagtgcaagcgctcgctgttcttcggctttgttcttatcgtgaacgtaagcactatgccagtacagcaatttgttgatcgttatattgtcgggtacgtagatgttcttggcactagcaaggtccagtgtcatgttcatcattgacgtatcagagaacacacggaagtagcctaagatatcaattggacttttatacttatacgtacggaagcatttgttgcacttgtgcgttgtctccaactcacagctaacgtatacatggttgcctgcgtccatcaattcaatggggtcggcatagtcgagcgtttgctccagaggcaagtcgctatccatgtacattgcgttcataacctgagtacggtcacgttcttccgagagtgtttcagcatcaatccagcgctgaacggtaggatggcgcaagccttgaggaaggtcgcgccatttgttggacactacgttctgtcgcatgacttcttcggtattgagcaggttgcattctacttctacgaatttgcaaccacgtggcctgtcatagtaccgctctcctcgcatatcaacgaagaacgtttgggtgcatcgccattcgtatagacggtgcgacttcggccaactattagcgtcgaacattgccagcatgtatctaaagtcttcgaggtacatatctcggactttaacattggtgaatcgctgcaacgtatcaacaaagagatcaggcagtctatacttctgggcgttgaacaggctggacatggcgtcagcagtaatctgttcgatacgcacatcggacctgcctgagggcagataaatctctaacattagcgcacgaacatcgctgggttcatgtcccaagcacgaacgcttttgcgtttacatgcagggcaagtgagttcgatatccgtaagcacaccgtggcgtgatgcagttacccactcagacagttgaagccagagtgttaggtcttcctgttcttccagcagagccacgttacgatcaaactcgcgtcccatgtgagctacgtgccagccaaacatatcctcagaagcacgttcgaagtgacgcatacgaggcaggtcgaagcgctcatgttcagcagccagcatcgcaactgtcattgacgtttcatcaacaacaccgatgttgtttgcagcacacggaaacgtgttgatagctccgccctcaggacgcagttcattcacgataccgtcggaatattcaaacagcggtttattgcatcgccagtgagtcatcagaggcataacagagttcatccacatacgctgctggaagacgagcgcatacgcatcaggcactgtcagttcttcgagaggaatagacaggcatggagctaaagcgtcgagcaggatgtacttcatgtccttcgcatcaatcgcctttgcaatcgcacggttctctttaccaccaaagcggcgcatcgtaaacaactcaggaagctgcgctttatagccacgcgaaggtaaactcgctgtttgaatttccatttgttcttatctcacatcaaaggacgggaaacatcaagagccatttgcacagaccacataccacgaccaccggtgccgttaagcgtaatgctttgaccgccgataggccagcagttgcggagctgttgttcgccaaccatttgcccttggttgtcgtatagctcaatgataatgtttttcttatacactgagggtaatctaaatccaccagtgtatgggttctgaatcaaactctgccacgcattcatatacttcatgactgcgagtttctgatcgagtccgaacagcagactgaatccatccacactcgaaccatgtggccagttgatttgtacagtggccacttctttagatttcgattgatagacagagaacggcaggtcgacttcttcacacgcgaacgggcttaacgatatattaccaataacaggaaattctcgcacacgccacttgtcctgcatgaaaggatcgtcaaggccaggagcagaggagtcattcagatcgtcaagtgtcggcagcggcatgattaatcctctactatgacaagcacaggtcgaacatcattatcgagcttgaggaacgtcgcaccaaccagatagccacctttctcaatctgcttcactacagctttctcgtagtccgtctcccattgctcacgctgcgaggacttgtagccttcgaacgtttcagaagcatcgtagtagttatacgtacctccagtaggcatagggatacgtgcaaggaactgaatacggccagcgttcttaaacttggctttatgcagttcttgagtcagcttcgtgttctcagctttagagccaggaacagccttgaaagatttcttcggttgtggttctttaggcgcagcagggagtttctcacgcgcaggagtattcttgtctgtagccttcttaacgcgaatgccactgaccgttcctgtgaatggacgactgcgacttaacagcgaacgcgcaacaggcgcatcaacggtgaagactacagacgggtcatccttgtgcagcacatagaacttattacgcttcgcagcaacgataccgtacacatctttttcttcgatgtcggcttcgtgctctttgttctcgatactgaccttgcgcttaccttcgaagcgataccagtcgcagtcttgaatagacacgtcaggcttacgtgcgctttcgctcagtaaaataagcatagagtctccaaaacgaaaaagggccagaacgaatcttggcccttatgtttcttacacgcgctctgcgtagtcgaaggaccattcgattgaaaccggaacagcctgcgcagcaccagagaagttcaagtctggtacctgtttcggccacacgccgtagatgttgtactcagcaacaactgaaccgtccatgtcgaatacacggaacagagctttcgttgcgtagtcagctttacgtgcgcccagctgggtttgcgtagcacgaacgaactcatgccagtcttccagttgcttgtacacggccatctcagagttttcgttgtactcagtagagagcgcatgagagaagatcttacgaccagcgtagttgagctggtggccgaacgcttctttcaatacttcttccagagtagaacctggcttgataccggtcttacagaacaagcgcagagtacgcgcataatccgacccaccgacaggagggttaggaatcaggaactcgaagttgtcatcgagtaacggatctttcgtagacgaaaattcgtcaagagttacctttggcatctaaaagctccttagagtgcaccagagttgatcagttgcagcgcgtactggatatcgcctacaggaggcacgatagcagttacgtggatgcgtttggtgtaacgagtcgggtcaaggaacacgtcgatgatcagatcgccacgcgcttcgtcttctgcggtgttgtttttgtagtcacactcgactgcataccaacgcagaccacggccgagtttaatcggttcgaggattgcttccatcgcagacttctggcgctgtttcagaatgtcgtcgttcggttcgaacacggcagtcaggttgttagcacgggcagaagcatgaagcattgccagcagacgacgcacaccgatatcctgaagaggagacttcgtagtgtaagtggtgtcagcaccccacatgaagataccttcgccttcgaagatagcaatcgggttaatctggttatcaaccagaatgtcgcggtcgttctgcttgaagcgataacgaacatcagttgcgaagtccagcttaccgcgctgcataccaccaggagcaagccaagaagcaacttggtcagcagtcaacatgcagtacgccatacataccgacgcaggaacatagaagtcacgagcgttggtattgtcacgcgctttaacgtcagagttcgacagcgcagaccaagaaccgatgatggagaactcggcttctttgtagggcttgttaccacgacgatacgcaacagaagcatcacgtgcctgcatagttacaggaacaccgtgtgttgcgatacagtccatgcggctttcggccaattcatcgatcttattcgcaataacaggatgctcaaggccaccagcgcacaggatgccagcctgaatgtcttcccagtcgcggtagttatcccacgcggtcagcacagcagacagactgcggttagagatgatcgggtctgaatgatcgatatcaatcaggtcgccatcgctaccaccagtgaactgaccgttaggtgcagttggattggttgggtcagcaggaccaccgccgatggagttgatgaccacgaagttcgggtcttccagcagcttgtagtggttctcattcagcttaacgcgaatgtacttcgagttaacgttgataacgtcttcaaggaagaactgattgcctgcttcgtctttgtagtaacgagtagtcaccacgtgagtttcaagcggtgtcaggtaaccaaccatgtacactttgatgatggacttaatgcccagcgcatcggtcacgtcaggttcgaacgtgatatacatgttgttcgcgtcagcgtactgagacatggaatagatcaggcagatatcgcgatcagagaaagcaatctgctctgggtcaaccagtccagcatcgcccagaggacggcaggtagcgaagttgttgtacgttgtgagatacacacctgcgtacttcacagagagagcgacacgagtaatgttcagtctggtcgctttcgtcatcagaatttttgcactctgaacgttgttagcgtatttaccagtggctggaccgaagatagcgtcgatctcgtctttagaggtaacagttgtgttcacacccacaggacctcgcgggaacggcagaaccagagtacacatgccgtactggacaagtgacgcctgattcgagcgatcgttctcctgcgagtatacccccggagaggggtgattaggttgtagcatcgtgaatctccatgagaatgggcatcgtgaaacgactgtatgaaattagcgtgttatcagtagcaaatcacattaacgcgctggtctacgtcacttaccaataccgattgatccattttgcctgtgagcgtaaactgaccttcgatagtcatctgcccaccagcatactggaggatgataggctctgcggtatcaatgtacagcagccctttgatctcaggcagttgatagccttttggtccaacgataactgattgttgcacgaacaggccgtcttcaggaataccaacagcggtcttctgcgttttcatgatagcattctgttggcctgatactgatcgcacacggctatcgacgactagtgtacggtcgagcttacggtacttctcgcgggtatacattagtcatgctcctcttcgtcttgaacccgagcagcctctgcgcgtgggcccaaatcaatatcaatctcaacgttctcggtaacttcaccgtagttgttgatcttagcctgctcaaggttgaatccaatcttagagtgaatcgtgattggaatctccagctcgaagctacccggcgtactaccttcatcgaggtcatcaatgttgggcatagggatagagtcgtcgagtttaacgcgcacagtccacttggacgtaggcatctcaatggagaagctcattaagtccgtcaggcctgcaataagcaactgttgaacgtatagcagtgcttgattgacgtccatgaacttgaggaacagcgtaccagtgagggtcacagggaagtaatagttagttacaaccacagcgtttgagccatccccgtcggcacctagcgcccaaccactaccatgtcgtgcaatgttcttcacgttcacagactcgtcgcggttgaatgccatagtaggcagcttaaaccaaccatatggataatcagtgctttgattgttcgttgcacgaataccctgcttagggttattatgcacagaccaaacaaaacgctttaggttgaagccttgacggaactggcgttgaaagccaaagatggttgctcgcagcgatgtgctgttcttgagcataccggataggtttgcactcatttgtggtgctccagatacgaaaaagggcggccgaagccacccttttggttacccgcaatcgggtgctagtcgtcgaatcgtaaacgaatcagagaagaagtagcggcagagtcggactcaacagtaatgtcgtcttcgtcttccagatcttcttcatcatccatgtcttcatcttcttcctcttcggaatcggagttcagactgatgatttcgtcatcgccatacagcgacgcgacttgttcttcctcggcattaagcgctaaagcagcagataacgcagcgacggattcattcatgcccgatgcggaactaacggagttaacgaggcatgatgcttcgaagttgtccgagagttcacaacagagaaagtcctcagtgtctggcgccacagcagcttgagcaagcaagcgggaagcatccatccactgtccgtcacgcgctgcgacgattgccagtgcagctaaggaaccagataatgtcttcatgcttggtcctcagttaagagggcaacattacgctgccctcaattgcacagtcaattagccacgtactgctttcgctacagaacgcacgttcgccagagtgaaggagaaggtgctagacagcaaccaaccgcggtcggtgttgccctggtttgcgccgctggtaggggtagactgggtgccgccacgagtggtgtacactgcgtggtagtcctggtctgccagaacgtacagctcaccgtcatgcagaacgcggtgttctggagcgcggaagccgtcagttaccagttccatacccagcagggtacccagacgaccggtggtgatcaggtcatacttagacactgggtccagagcagagctgaactgatcgttaccaacgatatcgttccagtagtcctgcgccatcacagcggtgctaacaggcagcggccatgaagacacagaatttttcagagtagacagcagacgcggagtcaggtcaccatgcacgaaggtgattgggttagcaacgccaacagcctgatcacaagcacgtttccacagacggtcttctgcaaccatgatagaagacaggccgtcttgctgcgcacggtccagcaggtcaccgttgatctggtccagatccattttgctgacgcgaatgttggatttcagttcgaactcagcaggcgtgtaaacacggccgcggaattggtagtaacccatgtcagaaggaccggtcgcgatgattgcttccgcctggtgaattttcagttcgatacgagcgatatcgccctgacgaacggtagcgcctttacacactttgcgcagcaggccagcacgttcagcacggtcttcgatagatgcaacgatagaagcacccagagaagcccacttctcaccagagctgtcagccacagcttcctggaacagttcgattttctcttgctcagtcaggccgcctgcgttagcagaggtagagtgaaccagttcgccgttctggaatgcgcccatcagcttagtgatttggcccagcaggtctttttggctcgatgcgttgatctcaccagtggaagaggaaagcgccagctcacctttaccaccaaaacgcaggtcttcgattggcgcgccgttacgcagggttactttagcgccgcgcattaaagagttgttcattagttgctcctgagattaatctcgtaagttttcagatactaaacagtcacggtgcgcgacgattaagcgccgtaagaggaagtggtttcgatgatcaggtagccgcgctcagtagttggcgcttgcttgatgatcagacctttcagctcggtaccgttaccaccgatggtcagcagaccgttcgggcccagagttgggtgcagtacgttgtcagcagaccagtcagcggttgggtcaaacatagaggtagcaacgttacccagtttgatgtacgcgatacgaccttcaacgttagaaggcaggccgccgataggagcatcagcagtgtacgaacgcgcttcggtcacggtcagttcgtaagcatactggatgcgaactttcttaccaatgtcgtcggcgtggaagtacaggtcagcaccctgaacaccgactttaccttcagcagtaggagcagcgttagcttcctgatctgctttagtaccgtcgattttaaccagcagtgcgccagcgttaggaacgcgggatgcagtgaattttttggtggcgtcgataacgaactcttcaacgcggttcatgttcgctggtggcatagagcgagccagagcgaaaccggcgaatacttcgtcagcagcaccagtagacagacgcaggaaggagtgaccgccttcgcgagtccaaaccagtgcaacgccttcttcgtggattacttcacccggcagcagatcagcttcctgggtctgtacgattgcggtagcattttgaaacaacataatcagtttctccaatgagagattgtgcgattaactgtcgtacggcttcaattagaagcgcatacgtgccagcttgtcgtcgaaggatgagccagtggaagctgaactctgggattgaacagactctttgtcctgattcaggagttccgcagcggaaggctgtttgaccggagcggtcgtaacctgctgctgaacaaccggcgcacgttcggcactaacagtaccagcagccgcgtcgatagattcagagatttcgttctgcgcgacttctgatttgctcataagctcattggctttggatagagcagttgtcaggaagtctttaccgtgggcgatgaacgcacgttcaatcagagcgcgtggctctttgataccagcagcggagagtgaacccaccaggctatcaacgattgggttacgtgtatcaccccagtagtttttcgtaacgcccagctgggcagaagacagagcagcgacgaagcgctcaccgtgatttgcaacggcgtcttcgatggttgaagtaacgttcgcagtagcttcgctaatacgtgcgtcggcgtcagccaccagcattttgtcaacaggcagttcgaactgatgcggcataaagccgaacgattcacaagtacctgcaacgcccgtgttgttcaacgagtgcgatacggcacggatgaaattatcagtatcgaaagatttcaccgcattttcttcgcctactgcattagatacagaagcgagagttgcgcgggccagaggttcgccgtcgtagaacatgtgaacggtgttcactttaccacttacgcggctcaggctaaccagagacgggtcgagcgtaccgtgttgtgcggtagcagaagacaggctgtcgaaggtgcgactgacgacattgctttcagaatcgaagtcgtcatcaaggtcgaggtcgtcttcttccaggtcttcgtcgtccagatcatcttcgtcgccgtcagagctagactcggaatcgaagtcgtcttcatccagatcgtcttcgtcgaggtcgtcttcttccaggtcttcgtcgaggtcgtcttcatccagatcgtcttcatccagatcgtcttcatccagatcgtcgtcgtcagagctggattcagaatcgaagtcgtcttcttccaggtcttcgtcatccagatcgtcttcatccagatcgtcgtcgtcgaggtcgtcttcgtagtcgatatcatcttcatcatcgttggatgattcagaatcaaaatcgtcttcgtcgtcgatatcgtcttcatcatcgagatcgtcttcttcaacgatatcaatgtcgctgtcgtcaccgctgttggattcgataggttcatcgaccagcgcagcagaacaatgcgcacagaacacaggctcttcatcggagcttacagtgaatggctgttcgcatttagcagagcagctatacatgtgcgcttcaacttcatcgccagcagaagacagagccgttacagcttctggagcttcttgcggctcacaggaagtaacttcctggccggtgtacgggtcgaagtttgcggcagtagcagcgttaaagctaccagtaccagacagcgcggtaaacgtgtgtgcgttgctcagggccagcgcgaagttgcgttgtgcagcttcggcactttcgccagtagcaaccagaccagcgtgttcaatttgctcgtcagcagaagcggattcagccagagcttgagtaacacgttcgtctgtgatttcggacaggtcagcagagcacgatgggcaggagccctgaaccagtgcagaactgtcggaaataacgtggcagccacaaccatcaaggcagatggtgtaatgagctttcacgtcacccgcagaggactgcgactggacttcggctttctcaaccaaatcaggatgctctaccagcagttcttcaccgccgttaggattgtaaaggtctgcgccgctctgcgaagcaaagcctacaccggcagagttcccgaaaatcatcaggttctgaccaagtgcagtacggcgaaagttctctactgcctgattatggttttgaccgacacacaggatacccgcgagttgggtaatctttggcatggttaaaaccctcatagaatttttagtcgttgaatcgacaggttaaaattaacgattgcagaaaaaattcaggtatttttaaacttttctgctatcaatgtcagcttgcggaatatagcgattttcgaagtatttattgaccacttctactccgtttaacgagtaaacgttacgcatactatcaccccaaaccattagctctgcaagggttgcgaaatgctccgttggtacggatttcattgtcctagcgtcgagcgaatccgggtggattttcttaccacgaatggcctgttcaaacttcatacggtcaacgtttcgtatcatcgtatggtccacaaagtgagccaattcgtgggtcattgcatggccgaatgatcgactattatagccaccaaacaaatcaaccaactgccggggactcattgaaattacaccatacaggaatcctgacacggtataagtcattatatgagaaccaccaacgtcattgccctgtttaacgatacctacgtataaacgcttgaatggcagaggcacgttcagacctatgccgggcatgacgttctcctgaatgtctttcagtacataatcaggagggctgacgccttctaagtgaatacgtctaccgccaataagcaagtcatcagcacctaatacttcaagatgcacattgccacacttaggtatcttttggacagcgtagttatttggagtaccgcccggataagtagcgttagcatacaccagagctttcttatcgccaaacataggcatgtcttgcaggcgacgcgctcttgctctcagggactcaggagtatcgctaccatctggtgtcggcataccggcatcttccggttctgctggtggtgcgggctgttcctgctcaggtttcgctttgactggcacgggctttggcttaggcgcagtagctattttcttcttctcctcataaggagtgaagtcaaagtccggcttgaagagggcgtcaggcttagcagtgaatgggcgactctgtgcaactaccttgtcaccgtcatctccactgatttcataagccatgtcgtatttaggatgggctatgtagtacaggtcgttgcttaccttgagcaaacccacgacctcacgggtatgcagatgcaccccgtttgagatcgctacgtctggtcccagataacgatagtacggatagtccgatatgactagacttcccaccattacgccatccgcataaggtgttctttgtacgtggcagcacaggcgaatgccggatcatcgaccgagctacattcgaagccagtcaacatcttgcagtcacgatataccagacggcctgtgcgaccatcaaggtacgttggtttgttgaacgcggtgtgcgaacagaagttacgatgacgaggagtaaccaactgaccacagatgctgcacttataggctttgtacgttgtgcctttagagtacgtgttaagctcgccgctaaggatgcgatcacaacgttcttcgcagcgtgtacggtcaaacgccaacagcagagtcagacgagcatgattaccgcggaagttctggagctttgacaggttgctgtcgaagatcatacccattgcttggcgataatctttgttgttatgctcgatgaacgtaggcttaccgatgaacgtttgataagcaagacgtccttggtcggggttaaacgtcagccactcttccagactgaatgcgtcaccatttgtgttaggcagctccgtgatgtttacaggcacaggcacaataacataatcacgaatgttgcgtgacgtgttatactgctcggctgctttcgacagccacacgtttacgtccagattgaatgagcctgtttgaaggccaaaacgcgaagggtcaacacgaatagacttagctgtttggctaacatcttctttgtgcatatcaatcgcgcctagtccaacgaggcccatgtccgaggtatcaaatgactcggagcgaatggacttgtccatcgtgttctccctattggaaattgttgatgttatctggcccagcgtttgctagacgcacacaaccctcttcaacttggaaggcgttgagtccgtccatagtgcttagccagtaacgtaagcgtccatctgaaattactgcgttctcaacatatgcaggaacttctttgcctgaatctttcatacaggcaatgacttcgacgcccggatagaacacgtcaaaggactttgtactgaatatcggtttaacgatatcagactcggacacagggtgcatggcgtagcgactttgaatcatatagatcgcttcgttagcaccaatcagaatcgagttgatagtgccgcgcaatgtacaacgagcactaccgtcgagagtacgtccgtggtagaacgtaacaatatccgcgatgttatacgcgaaagagaattgagccatattaacctcgcagcgcaccacgagcccatgacttagcgagcgccaaagtcatacggcttgggttttgcaatttgacttcaccattatgcacagcagtgaaaggttcatgcgcattctctccgcgaccagaacgatacgctgcttcattgaagccgtcgaataacgttacgacccagcctgtggatttgtcagaacattcaccacaggctttgtcccagctaatcttaccgcacacacgaccaccagcgttaaccgcatagcttacttgctcagtacctttatacaggtcttgagatttcagcgttttgaacgttacacgcgcagcagactcagaccgcggcgtcatcttctctttcagcgcttcaatatcaagtgaagaccagaaggactcaaacaacgccgcaaatttctgctcaataggcaggtcgatagcgttgatttgtgcgatggtgctggaactgtcattaagcacacggttgatgaagtaaccgccgaggattactggcatctgtgtaccctgatctccagtggtcaagcccgcccgcttcgcatacatctcacacataccgatagcaagacgtgccaaagtctggaaagtctgcttctctgtactgttggcaatctcagtatagatgcggctggcgattgcaggaaccaccgtacgcttcgctacactcagaatgtcttctggtgtaattgattggccgagcttcttcttggcagcaagttcgaaagcattaatcagacttgctttgttcgctggtgtcagagactcgctcaacttgatagttgtctgctccgagctgttcaccagattcggctgctgtggctccctcagtctgcgaactcccgtcgttttcaatcgagctactgtcatttgtttcttcctgattaggagcctgtagatattgcaacaggccagagttcataatctcctcgttaacatcaagaccgcgaagcgtagccaagttagcgaggtaattgagagcaggttctaccatacccagattgcgacagccccaataggctaagtcgtagcacaggtctaaattaataggagtctggtcgaacaggaaactttttggattctgctttgacgcttcgataccctgaatagcttgaccaatcgcattgatgttgtcaccatgacgatagaagatatcagcgagcatcgcatagcactcaatacggtctgggcggaatgcaatagcacgatagcaggcgcacaccgactcttgagtgaagccctgcttgaatgtagctttcgccagttcgatgttagccaaagcaacatagtctggccacttagctatgccagccaatcggtcaacttcacgccgtgcatcttccagaagatctgggcgctcataataactgacagagtagcagagttcacgcgcataatagaaactgcaacgatcatcatgtggatagtcaccaacatccagaccaagctccagcagataattacgtgctttgtcgtggtctggatagtggtcagttgcgaacggcgcttctactgatttgagtggttgtcctggcttgcgcgaggccaggacttcatgcgcacggtacttccagaaataagagcgacgacgatatgctttcatctgctggtagtgactgtcgccgttacgcatcagaatccaaacagcttctgctttcttaatgccttgcgtattgcgtagcgcctcaacccaattagggtcatcgaagcgctcgtcaatatcaagccacactacaaggtcgtcttccgagaaaggcgtagcggccatctcacgactcgcgcctagattgcgttcttctgacacatcgaacacatgatacaggttagggtgcgtgaacgccgaaatgatgttcgtggtttggtcttcgctgcctgtgtccacgatactaattgcatcggcacctgcaacgtgcttcaaccactcaccgatattcttttcttcattacggcagatagccgctacacagattctcatgtttgcctcattgggttatatcaaaacgttaccgctatcccaccactgcttaccgtagatatcagacacacggtactcaaggatgagaggctggtccaggtcgacttgcaaaatgtatcggcctaatgatggactccacactgttttctcctcagtgtaaagccgaatctcaagctcaatgtcgccttgtgagttcttcggtacgaacggatgtgaataatcaccatcgaaacccgcaccaagagagtcgtcgaagtatgtgtaggctcgaacttcttcaccagtattgatgatggtcggcgcatatacctgacggttatagtacgaggtgtagtcggcaacagttgtctgccagacgacacgacgcttatagatacgagtcacgcctttgctgtctgtctctgcacgatactggttgtagtaccagcttatctgtgcgaattttacaggcttcaatggcgcttgccctgatgcgtatttcaggaacggcttcgcagtgaaacggtggtatgtcttctgcgtgttcaatctatacaacaggacttgatatgtgtaccattgataaacatcaagggtaatcgtacctgagtctgattgctgcgtaccgttggtcaggatgtaagagaaacagtctgcaccaacgtaaccgctgcgtgggctatagaggaacgcatcgttgaaatagttcagacgcaccgtaccaaccatagggtcattgaccttaatagcagaaaggcgccaacccctttgagctggaaccttatcgagtacaccctctgtagggctgtgcaacgtcacttcatcacgagcgccttgtaagatcttttcgagtgttatctcggtttcacccgagttacgcactcgcaccgtaaggttcggagctagtggcttatagttccgccagtagtcgaacgtacaaggcaaagagagcatagttactccagtttgtacttgctcttaaactctgcgagtcccataacagggatgcctttgtccatcgctttttggagtttcgcagaaccagagccagggtcttttgcgatcagtatcgtcgtatcggacttcatgctatcagaagcagtcccgccgagttcaacgatacgcttcatcaagtcacggtcacgaataccagtgaatgctacgttcacgcctttcagtttggcgctaactactttcaccttcttcggagcaacgagagtcacacccatattcgcagccatgtcgtaagacttcacggcagcttctgctatagcgggtccgagtttgtcgatgccgtgcatagcgccaatcttcaacgtcaggtcagcggtatatccacgcttgagataatattcaaggttaggaattgcatcgacaactttgtcaaacgtagtgttagcaccgcgcataaagaatgacgctgtagccttcaaccacgtattcattggcacgccagctttcagcgccttaaggtctttcgccaactgacgaccacgagagtcgccaacaatctcacgcagcgcacccatcgaggcatcgaacaactgctcaggtgttttaatgccagacgcaatcagcatcttgcatgtaccaggacctgtgttagcaacgtccagccctttcaagaacgagcctagcatacgggcatcagcagcagacgacttcgtttttacgacgaactctacaccactaatcttgtaaggcacgtcaggtagctgaggcttcttggctggcttgagaatctccatgatgtatgggattactttgccacttcgaatcaatttaaccttagcaccagggccgaggggccgtttaggacccatcactgcgcctttcttcttcggcttgagatagccgtgctcaacatagaaaccgttgtgcgcagaagcacgttcgacagtcacgccgccaggcatgatagtcggagggaagatagcgacaggagccattacgccatacttggactcttgatagataatctctttgaccgtaacgatgaccgtatcagactcaacgttcatcttgaacttgaatgcgtgtcgtgggttagatgcggtagcttttggggtcgctacgtcgcgtgtcatcacgatgccatcaagttcatacttcgctttagcgattcgcctatccaaccaaggaattagttcttcctggttgtcaaaacgcataggaccaaagtgacgaaccacttcgaagccccaacgctccagtcggacgaactgcttagactgccggtcagttgcgcctttacctgcaagaataccgaagcataccatatggacgtacttgaactctttgggagttttaaagttacgcacaaggccggacgcagcactacgtgcagccttatatttaccaccagcagactcgtgcatcttcgccatgaaggtcttatatggaatcagagcttcgaagcgcatgataaccgtacccttttcagaaatcttctgagggatacgcatggcgggtatatggtgagaaacatctttaccgtgcgtagcatcaccgcgagtgaacgcccgtactggtacgcctttctcataaacgagttcaatgctcagaccatccaatttgtccgtaagaatccagtcaacatcttcggccagagccttagacagttgcttaccgccgagcgtatactgatcgagactcgccataggaacaggcagcttaacatcagagtcatcacgcgcaccaaccttacgagccaactttgacttaggccagcgtgtgtcgatgtagccacgaatgtggtcatagaccgcatctgatatcaagccttccgaatcagtgtggaacgcatcatcaagatgcgccacaagtttcgttgtctgcgtcagattgagcgtgtccagaaccttatcggggttcctttcgagccgcttcaatgagatttgcatgttgttttctccgatcgtcatcaacactggtatttacagcattagctggcgatggggtctttgttgacagggaaatcttccaccatatcgtacacgcgattgaatagcttaggtgccatatctttcacatgctcggcatagtcaaagaggttctgtttacgcgcacgattcacacgcacctgacgcacttcgtctgggctattggtaatatcgtacagcgtatagataacgatgttgtcggaggagttatgcgtactcacacgaacaaccagccagtcgcgtttgagtttagcatctgccttgaactgcaacacatcaccttcttctgcctcttctgcgcgagcgcttggagtagattggttggctgctgcaatcttcttagcagtttctttcgcttcatcttcggcggccgcaacgtcagagtcctgatcttcctctgcgccagcttcgtctaccgcgtccgtagcatctgcgtctgcgtctgcgtcatcgtcggactgttcgtcatcttcaccttctgaatcagctccttcgtcgtcagcatcggcatcatccacggattcgtcgtcgcttccatcggattcatcagccccatcttctgaatcatcagtgtccggatcgctatcgtcaggatcttcttctgcatcgggatcttcctcatcatcagtgccagaagtatcttcttcctcttcctcctctggcggagcttcgacaggcttcttgcctttgaccttagcgcgtactttggacggcgctacatcttcttcgtcgtcttctggttcgtctatatcggacaggtcaagcgcaggctcttcgtggtcttgtgaatcatctccaccaaacaaggacccgatagaatcttcgatgttgaacatgtcacctgcgaatgggctgcgtgatagaacgtcttcgagtttctgctcgtcgaagtccaaatcaacttccacttcctcaatcgcatcatccagttcttcatgctcgatgattttcacacgcttgccacgtttgtctataccatcctcatagacagtacggacttctgctttaggcgcttcaatctcaccgctcttaaccttgttgcgtaggtcacgcatctcggctgcacgttctgcggcagtcttacgcgcttgtttctggagttctttgcgctgctgtttctgctccagaaccttagcgttgttggagaggcgtactgcttcttcctcctccaactgagaacgcttgcggtgacgacgtacctgtttgcgatacgctttgactgtatcaacgtcaatctcacccttaggccaatcattgaatggcaggatgttcgtgtcgtgtacaatcaggtcaaactgactgtcatccactttgacgtacaggccttctgtattgatgactacgccacctttaccttgacgcaagaaacgcacaccaatcatgtcgttcttgtagagcttgatcatacccttagaagttttcacagggtattccatgctaggcaccatacgccactggtagttatcaaagttgataccatacacagcctcagccttcacagacttaggagcgaaacgtgcggcatcgaactgaacacgattgatctggcgctgcatagtacgagcaccagcagtcttcgtgcgagaatcacgctggacaacatcaggcactttacgcagcttggtactacgctccataaggaatagaccagtagtcttgtccagaggaaagtccacatgcggcatgtctgcaaagataagagtgtagcgtccgccattacgcagcgggagaatgccaaaagtatctccttcacgaatcatacgcttatgagttcgttgagatacttcctttccgcgtgaacctttgtacttcatccacgcgtacttcgttactgcatcttcgtgagatgcggacacggaaagtatcatgttattgtctctatgttgtactgtcactcgttgaaattagcttactcaaggtaaagcggggattaacccccgcttaaatatcctcttgcagcgcacgacatagagccacaagattcttcgcacacggtgatttgtgcccacgtccagtaaccgttaggctgctggatagcgtacacaacagatgggtcaaagccccagacctgcgtagcgttttggagcgccagcaattctgtttcgaaatatccttcttcgagtggcttatctatcgaaccgtgatttggttcgactgaccacacctcaactacaggtgcaacgacagcgtaagtcttattgctatctgctttacgcgacttcctgatctctactgcgataggtgcgcgtgtagctggagcccctggagtacgtgcaacaggtatgattctcggcgccttaataagatcaggctcaagaacatccgtgttgatctgaggagcaccctgaatgagcttaccctgaatcagatgcagatacacctcaggcgtcttagcaccaagaggactatgaggcacaacaggtgcagcaatcaggcgcagttgttcgaactcaccaggagcaggactcacaggatatttaacaagatgctccatacgcatcggcgtagatggtgcacagtgataaatctgcgaaggctgcaaccaacgtgtgaacggtatctcaggcataaacagcacagcagggtggtagtcaggatcgacatacttcgccaccagcgtgtctgctttatacgtgacactaacagggcgccagataggacgtgcccaacctacataatagacagcagacggttcaacatacttaccgcttgccatctcctgtgggtacagaccgctgtcagttgcatgacgcgggtcagtcattccctgctgatacagaccaccagcatctaccttcttaccttcaatagcgttagcaggatagttacctttagtgtcagcaaacttaggcagtatctggtcggacaccgcttttatggtagtgcgatatacagggtctcgaagatcgaaatactgaggcgcatcatccatgtgctccacaaagttgttgatgaaggtatcgttgaccacagccacatcagtgaagaatgttggccagaacgagtcagagacaatactgtcaccagcaatagcttcgaacaacgggaactctgaggcagtatctacctgaccctgaataagctcgaacatagggaacgtatcggttgctgcaccttcattcgtaccaataaatgcaggcagcggcgtagcagtaataacgtccttctggccccctgtcaattcaaacagagggaaatcgtcagatgctattgcaggagcgtctgtcagttcgaacagagggaagcggtcatagatgatatctgacttagcaatcagatcagccatgcggaagttatccacaaagtctttatgacctgtatcgaagtcattcccttttgtcatctgcatgacgtgcgtggcagcgtcttcgaagtcaagccactgtagctgaacatccagctcagggtcatacacaggagtgagcacaacgttctgatcagacgcagccacataagtcttagcgtcaaacacagacacggcatcggtagtagcatcaagataagacaagccgaacaactgcacagagtcagtgccgtacgcggtatacgtagggtcaaccgtcatatcgtagagccagcctgctttcgcgttaccgaactgcaacgtgtgcggttggtcatgagaaggtaagccgtagatcttgagcatcgtgtctgcgcattcgaacggaccaactacgaggccctgctctttgtacacaccacgactatcaagttcttgctcaacacgcacaccatcaatgtccagcaacataccagcaggaatcgtgaagtacgtccagaagttatctgggatattgtcgataaagaacgtaccgctatcacccatgacataacgttcagcacgtttagtctgaggcaatgttcctagccactgattatctgcccacacataccactcataggaatactgctccgagcggaacttaatcgcgtactgctcattctctgtaggagtgaacttaatgctggtggtcgcgccaacagcaagtgtgatcgtctgcgtaccgttggagaatacagcatcggtatcagtgatagtcagcaccagagggatggtgcctgtgttcttcaacacatctgactgcacttgcttacctacagggacgtaggcccaatggcgaccaacatccaactgcgcttcgacaatagtaaataggctaaagtgggaggtactttgacctacgtctacgtcaatacgggaagtatcgttctcatgcagaatttcaaagccgagtttctgattgttgcgaatgagcacaggcattgctgtctctacaccatcaacaaaaatcttcacacggtcgtaatcttctacaccatccaccagcacactaacaggtacagcaacgttgataccactaatcgtaacgtcttcggtacggttccaagtatcgttttcgatacccagaatgttctgccacgagaatgcgtttggcgtatcgtctgctttcatctcaaactgatagacagtatgaccgatagcaacagggaacgacgagccggtaatgtacgcatggctaagtgtgatggtaacttcctgaccgtcatacactttggtgactggctccgcagtcacagtcgtaacctctttgccgtctacgatatcgatcgtggtaacatcaatcgtcgcagacacagtaacacccgcaggtgcagtgataggcagagggatatctgggtcaccagcatcgacaagcactttgaacttaacactcgggcctagttcgatattcgtcaaatcaggccacacgatatcgtagttacgaatcgccaaatgcttcaagcctgtagtaggtcgagctgcatagtagaacagtcgatcatacgtatcggcctgagcgtacggtggtgttagtagttcgacatacggccaaccagcgcgtgtctgagtaggcgtttcagcagaagcgaagttgaacagagcgttggagccattcgtgtccatacctgcgacgagcttaccgcccttatccgtccacgccgcagtcgtgttaaacacaacgaggtcattagcgacaagagggcgtgccgctacgttctgaacgttgtcacgaatgttgaactgatagatgtttgtaccgtcatgaccgagcaccaacagtgaactcggaacgaactggtaccagaagacagatgcaggtgcagcggctgtattgccacccaccagcttaccgtccagagttgacaacacatcatagctgtcagagccgttaacgtagaactgatcggacttaaccgaagtctccacgaaactggcattgagatagtgcgcacggccatctttgtcgaaagcaacatagctgtcaacggtgtttgtaccaacgccagcgcgacgacagataacgcggttgacttcatatcctaattgcttaggctcaccgaactgagtcatcgcttcgtcaagcacatcaacctgaccagacgtgtggaagactacagcactgcgtttattgttcgtgtcataactgactttatagccagcgatatcaacattgtccatgctaccgaacacttttgtattcgaagcatcaccatcagtgtgcaaataataaagacggcgtccttggcggtcatggacgattgaaataggcttggtcaaatcgaagaacgtgctatcgaagtccgagaacttcgctacactactttgctgcatgtcctgagtcgtgggtatgcgtacacccccaccaagaacaagaccaccataggtaggattaagtgcagcgcctagaggcattgcatccataccttttgtgacaagacggtagtccagctctttcgtctgtggacgaatgaagatgcgagacagtgaatgcacaagcacccaaaggtcaccgtcgagataatacagcagaacaggttgcgtagcggcggctgagaccgtaactgtagccagaagactcacagaatagtcagagccagaactcggcgtgatatctttctctgtagaagcatccgcaaacgtaccgccaacaacacggaatttgagaacgtcagtatggccagcagcagttacgctacctgaccaagactgcgcacccgttgccgatacaacaggaatcatttcagccattgttcacctcacgatgtagaaacgaaaaagggcggccgaagccaccctgtgaggaataggcttagccgcctgttacttctgattctttgtaaccctgcaggaagaagacgcgcataccagtgttgttcggactgttagcagtcagagctttgtatgtacgcttcttcggagtgctaccgtcatcttctttctcgttgtacacctgcacgtcgatcagggtaccgttagagataacgtcagaagacgcatagcccacgatatccatttcatacgggtagctgtagcgctgagtgttgaagcccgcaggcagacggaagtcgaagtggttgtcttctgagaacggaaccatctggtacgggttgataaccgcgtagctgtctgcgctgtgtacgtgtgcaggtacaggcagagttggtgcgttcacgtctgcttcacgaacggtgtagcgcataatctggaacgagcctgggctattagtagcaggacgtacttccagatcgttattcattgagccaccgccgttcacactgaacatgcagaacagaggagctttaccatcaacaactactgtaccatcagagttgatagcacgttgaactaccatccacgcaccacggcaaccgtcagagtcgcggccttcaactgcgatgtgcagcgcgaagccgtgttcagtcagagagatgtgataagtaaacggagacgcttctgggtcagcccaaatcaggctatcagggttctgctgaccagaactctggttagttgagttggtagggtacgccatggtgccgccgtagtagacgctgccattgcctgggccaacgatgccgcgatgccagaagcacacgtcgtaatcgccagtagtaccgccggtgttcccgttaaagcgagcaccaatctgacctgcatattcagggaaagaagtgctgcctacagtaacagtacccgttttagcgatggtgcctgtgtcagagatctgctctggagcagcaacgtacagattggtacgcttatcagtgactttacaggccacacgccagcgttgtttaccaacaccagtacctgccagtggatcgacagtcgcagttgcttcaacaacgaacgcagtcaggtccgtggatggaatagccgaggcaatagtgccgttgacactcaccagctggaagccgttatccaccaggtcctgcaggatagatttccacatcttgatgttgctggtgaatccggattttacaatcagtttgttcatgagtcgttatcccttaagattaagccgcatcaccagtgccgacaggaagcatcagacgcataccacggttgtctttaccgttagcgttcatgcccagatacttggttttgttggttgctttcagtgggttcaactgaacttccgaaccggcagaaagaacgtcggcagaagtatatcccagcatatccagtgtagcgaagtacacatagcgctgagtgttgatcatctgagggaacaggacgatagcacgattaccctctgcgatcataacctgctggagcgggttaatgattggggctgagtcaggagttggctgaacagcagacagaggaacagtcgcggagtagataccggcttcgataacagtgaagcgctgaattgcttcaggcttgattgtatctgggtcgccagccagaccgccgccacatgagaaaatgcagaacagtgggctgtgatcacctggattagtgtcacctgtctgtacgccacgctgcgcaacaaaccaactgaacgcggtgccggtattgtcgaagccttctgcgttgatatgcagagcgatgccgtggtcggtggtgatgaagtcataggtcagcgggaatgcagccagatcagcagttgcatccatcttccagtcagcaaccagatcgatgaagctgttggccatcaggccggacttagacagacgaccgatttccacagttgcagagcgcttagccgcagagaagtcagtgtcattcacctgaaggtcaggcagaatgttgacggacagagttttggcggtgttatcggctttgaggatgataccccattgctgagtttcgaacagcgggtcaaccgattcagatgccagcaagtagaatgctttaccgtctggtttaacctcagtgccagcgacaccatcaactgctacgagttcaaaacccccagcaatcattttcgccaccagatcacgggtcagagcttccagaccaatgagcttagtggcagttacacgttgaatagccatatgttaatcactccattaccagataggttacagtgagtttcggtttcgacggtgatgtaccgatattcttcatacgccacgaaattgtaggcgagttgtctttgttggacaagaagctatatcggcgcagcttgcgaataactggattaccttcgctatccacatctgagaacacgccatcatcttcgaggaaattagcagtggagcgaaataaatacgggtttctgtcatctcgctgtgccgtagggaacgcagagagttccacatcaaacgcattgagtttaacagaaagcaacatcaccgtacggttcatttgcaggtcaaagtcaacctgttgtcccggagtaatgtatgcaggagattcgtactccaccgttttacgcacaccagcactttcattgccgttcaggtcggcccagaacatcgtaccgttagcgccagatacgagggtcatacccgcatactcaggctcaggtacttgtttgcttgggtcgaggcctacgacagtgagtcctgtttcatccacagcagtgacgaacggagattcaaacttgtagttggcacctccgaacttcgcttcttcccacgttacgttgtctgtaccaagttgatacatcttcttggtctcggtgacgtaacataacatcccaggctttttattacctacggacattatgtcacgatcagccagagtaggcagacagcgcatacctcctcgaagatatttatcctcaaggaggtatgggagtgctgcggatgcaggcaacaggaacgaagtcatgtttaccggcatcttattctccttacgcgatacctgaaccagggttcgatgaaccgtaggtcagtttaaacgtatacgccagactatcgaacgggaagtcgttacgataaataacgtaatcgacaccattgataacaacttctgctgggcctgcaaagttaaagtcatcgaactccaacgcaccatcccatgaaccagcaaagccctgaacggattcgacaaagtaaccatagccgagagacttaggccacgcaacgtagaagaacacgttgttcgaacttgtactggtatttcccggacagttcaggagctgctgaccggtcagagtcaatgcagtttgcagaccagcaacgaacgctgcgtcatagccagaggtagatttaatcttggaatgcgaaccgaagcgagcacccagatcagaaacctgctcaggcttgagcgtaacgtctttagttgccgtgacagtcttgccgttcttaacgtaagtcacggtgattgtcactacagcatcagcagtaactttgtcagacttcaacgaaccacccacaacactcaggccggttgccgtaccagacttcacagataccgcccacgttgtaccactatcagcagtcacgtcaggagtggtaccatcagacagagttgccgttgcagtatatgcagtagttacgccgccgatgattgaagcaggcccagtgatagtcacagagtcaggagtcgcaggagctggagtgttcgtcacagtcaacgttgccgtttggactacgctgttgaacgaagcagtaccagtaatcacagcggtctgcacagtgctaaccgtattacctgtaatcgtgttgttgccgttgaacgtgaagcccgtagtagagccggagctacgtgtaacaacaggcgtcaggtcaaccgtagtgttatcagagaacgtcaggcgaagaatgtaggtaccagtctcacctttgttcacagcagtaggacctaccagctcgcgcttagtgatcgttgctgtctgattgatgatctgaatagtcttctcaggcgcgtaagtcttaccatcgacggtgacattagcagcacggagcgtgacagtctggttctgcgtgattgagttaggtgcagaggtcagcttcgcacgagtcgaagtagtaccaacacccagcgtcacataggcagcaccctgaggcagtgaccaagtaggcagagaagcatactcgttcgttgcgccagacagacgagtgatacgcaccagataatcacctgacacagtaccttcgttcatcgaatcagcaccgatgatttccacagtgttcacgtcatcggtaggacctgtgaccgtgaactgtacgctaccagttttagacacagcacctacagtcgctacgacgttaagctggaaggtcagagtcccgaagaaaccgctgagagttttcttggtacgaatacgccagcccgttgtaccaccagcaacgatctcaaagtattcttgagccgcggtggataacgtgtagctgagttcgccgcttgtaccctcacgggtagatgaatcagagaacgtcagggtactatgcaggtcgcgtgttacagcagccgcagtaccgaagtcaaacacaggtgctggcgccagaggctgtacgctcaacaacgagatgacgatgatgttcttaaccaacacagatttctgcgcgttacgtccgtcgaacgttgcacgaatcagaacggttgtgtcctgagtcacttcaccagcagacagcataccagtctgcgcgatgcttgcgactgcgctaccctgaataacagaccacgtaggtgaggtcacctgacgctctgaaccatcagaaagaatctcccatgcagtaaactgcgatgtagtgttttcattcatttggtcagcaccacgaacttccagagaagtcacaaccggcgggttaccgacgatggttacgttctgcgtggcagtcttagtgataccgttttcagtgtacgacgcatagatcgttacgctggtgtttgcgatgttcaccgcacccgcgatcagattcgagtcagagaacgttgcatagattgaagcctgttgcagacggaactcgttaggactaatagtagccgtgtgtccgtcagagtaagttgccagcaccgtgtatggtgtagtggtcttctcttgaacagacgacggaccgacgatcttaatgctcgacaggtctactacaggcacaacgttaacgataagaatatcgagagtcgcagtcttagtgatgccgttctccgtgtacgttgcagacagcttcacaggaatgtcagaagacaccttacctgcgttaacagtcttgttcacgatagtaacaacatccagacggtccgcagtgaacgtcgttgggtcaatcagcttggtgctgttatccgagtaagttgcgaggaacgtatagttcgcgctttcttcgctgcggattgtattcgcaccctgaatggccagagaagtcagcacaacggcctcggtctctttcagaatcgtgacgttcttcttacctgtgacagtctgatcagcagtgatgtacgttgcagtcaacacgatatcacggttcgaggttgtttctttacgcgctgtaaccacgttaccactaatagtggtgtacgttgtaggtgcagcgacgaaagagttctgcgttaccatctcggtatcgccattcgaccacgtaatacggaacgtgtaggttgcgctttgctgggacgtgatggtggaagcaccaagcacttcaagcagcgtaatcaactgcgctttaaccgtgacgttcttattcgcagtgaatgtaacgccgttatacacatacgtggcagtcagcttgacgactgtatcagtcgagactttcttaccagtaccctgcaggccaacgaggtccagagcgtttacgttatcaaccacgaagttcgtaggcatgatagtcgcaacgttaccagacttgtagcgagcagtaacggtgtaggtttctttctgcttatagaacagcgtaccagtaccaacgatagcgatggacaccagctcgtcatcaatgatgaacgtgttcttgatcagcagattgtaggtagctgttacccagttgccgtacacagggtcgcgcttacgggcagtcactttcagaacaacgtcagcagctaaatcaggagcagtgactgtaccgtcctgcgtgatagtcacaccgattacgttttcttcgatagaccactcgacgccagcaggctggtgctcgatacggtctgaccactcagcgtcaacgttcagtttgacactactgttatccgacatgtaacttgcgttgcccggcaggctaatacgcaggttcatcaagtgaggtgattcccactcgacgttatcagcagtaggcttaacccacttaccgatatacttgttagggttaacagggtcctgatcgacgatagccagcacgtagccttcttgcggttcgttagagcttgcgacttcaacgaatgcggtagcgttcaggcgaatcatggtgcgagcgtaatcaggatggtcgtggttagtcggataacgtgcattactcatgcgcgtatcagagctggacacagcaactgtttcagcagtcgattctggttcatctttagtgacgacattccccagacggctggtggtcgcatgtgggatttccagatcgccaacttcaatccccagatcacctgcgttctcaacaacgaagcggaagaactgtttctgattgaacagtgcagcgtagtcgttcacagttacccatgaaccacggtgattaccgtcagacacggctgaggtacgacgcagcacatacatatactgcgggctgcctgtgttggcatcaatccaaatcaggttgtacggcttttcagaaaacgacggctcggtcatagacacgataacctgatgcacttccgtttgatcgttcgcgttaggacggaacaggaaagtgattgggttacgtggcgtcagaccgcgagtgcgagccaggccgatatactgtttagcaaagccgtcgatcgtggttacgctcattcattattctccagaatgtcggtcgcaatcagatggccgtaagatgctttcacgttagtgtcagcgatgaacgtagcaccgttatcacctacatcggcgtccatgttcactttatcctgcacggtcttcacttcaaccagcggcttctctgggtgcatttcatcatgcggcagaggagtacgcttgtcagtgttacgcgggtcagtcaccgacacaaatgtaggacgaccaacagaagcaggctcagcggtcagacgagcgatcccgtattcgtcaacagacgcgttaggaatatcttccgtaccgctaatatcagacgggtcgtaatactgcggcgcccagaacgagttgaagttcttcacttcttcccatgtgttctgaaagccaccagcaggcgtcttagacttacgcgcaaggaacttacgatagaacacactatcgcgtaccatacacaaccagacgacgttcattggcaacacgatcccaacaggttcttcctgtgcgatgatgtgcgtacaactgatgttgagtgttgggttaatctgacgaacaacctgctccttagcagtgttatccatgaagcccgtaacattcaacagagcagcggcgatatcattcagtgtagtcataaccgctccttagtcagtcggctggccgagttcagattcacgcaccttacgccactggagcgtactatcttcaagcaccattacttggttcacttgaggaaccagctggtctttgattggcacatgttcttcaccgtaactaccattgatgctgatcatggtagcgggcttctcaggatgggtgtggtcgagtgggtcacgattgttggtaagtgtttcatcaccttcaatcaggacacgcgactcggcttctggatatgacagatagccaacaccacgagtgacgctagtagccagaggaggcagcgtacggttgatgatttgcagatcgttcgggtcatacgtctgttcagtcatcgcgtcatcgtagaaatacaacgcagtccaaacatctttgtatgggtccgagttatctttcgcagtacgcttgaaagctgtaccgaaagtagacgactcagggttgtagtcaatccaaatcgcattgattggaaggaccacgaaacgcggaactgcatacgagcagtagaacaacagacctaactgagagccttccagtggaagacgaaacatgatcgggtttttgttctgctggtggatattcgtaagcaactcaacgttactgatgaactgttcaagtttcagttccattgtgttctccgtttaccagaagcggtagttaaaattatacagggtcaccggacttcggactggtggaaccgtatttaatgcggaacacgtagtcaagactatcgaacgggaagtcattgcgatagacgacataatcaaagccgcccaacgagacctcagccgcaccctcgaagttgaagtcgttaaactccattgcaccgtcccacgagccagagaatccttgtgcagtttcttggaaatatccatagagcaagcgctttggccacgcgacatagaagaagcggttgttgtctgatgtagactggttaggaggacatgtaatttcttgcggactcgactcacctagaactgtaggaagtgagcggaaaaaggtatcgttatagtcaagcaacgacaacactttatcatgaataccaaagcgtgggccatactcaccactgaacggcacagacacccgcacctgattcgacgttgagttcagaacagtgctgacgttatatgctttggctacgatatcatgctcgcctgtatcaaaaggcagagtgaagtcgaagtaggcagtcgtacctgacgtaggcatatcaagtttcttgagcaccgtacccgcagcgttctcaatctggagagtaccgcgcaacggcggattatccatcgagaccaagaagcgcagctccttgttacgcagcgagaagcagtattccaagttaccttgaatggtcaaagtaaacatagaacctcacaatacgaaaaaaggaggaccgaagccctccctttgtgattacagactcagacttgtggaggtactgcctgacgggttgatgttgaaacgatagatcagacgcttagtggtgcgtgtcgggtctaacacgatatccagaatcaagtcgccgttagcgatagtctggttggtgttgttgacttcgttacaaacaacctgatagccctgcgagccagaagaaccgccacgaagaccacgaccgagtttaatctcttcgaggaacttctcaacgataccctgcaggtagccacgaaggatagcatcgttcggatcgaacaagccaaccttacaggtgcggtgacatacttcaagcacgtaaccgaccatacgctgaatctgaatctgctggaatgcagagttcatgttgtactgcgtactggcttcccacaccgcgtaaccaccaccagcaatgtcaggcagcttacggatgtagttgacctgctcacgggtcatagcatcacggtcatcctgatcgtacttctgagcaatagccaagaagtcaagaggggcagatgcagtaatacccgcaggtgcgaaccacgtaccacgattgttgtcagtgtacgcaaacacagcacagatctgtccgacacatgctgtccacagatagcgaccagtatcttcatcgaagactttaatgtcaggcgtgtacagtgccatgttcgtgtcgttcacgttcaacgtctggcggcgatagcgaattgccttagacacagactgctcggcggatggaataccgcagataacgaagcagttgatgtgcgcagcagcagccgctttcatgccacgatggatgatgtaatcctgagtaggactaatcagcaacgttacacgaacttcttctgggtcaccgaagtaatcctgatacgcttgcgccagctgatcagaaccaaccgtgtcaccgtccgagccaccctggaagaagatgaagtcagtggtgaagaagtcgatatcagtggtgaagtacggattacggatgaagcggaagtttgagctttcgttctccatcgcatagtcgatacgatactgacgttcaaattcgtcggcgtaatcgaacaggctgcattggtagctgtttaccggagcgcttcctgcctgatagttttcgtactcgtcgatatagaacagtttcgtattgtacttcgtgcggtcatcgaatgggtcgaggccacgaggcgtagcagggcgaatctgcatagccattgcgttgttccagtcgcccgggttttcaagaatgacgtagccgatgatattctcattcagcgggccatctggcaggaagcccagttggtctggagagtccacaccgacaatgttaccttcgtcgtcagtgtaaggactgatacgcagcacaggttgaacagccgacgggtcatctacagtcacgacaccgaccgcgtatttcgcgttcttagtcacgcggacgtatttgagttggttggtctgttttgccacaggcagcgctagatacaagccgaggccatacttgggatcttttgcaccgaagatgtttttcaaatcatctttattacgcacatcaacacgctgattgacaggacctcgacgggcctgaccaacgatgcctacgacggacgtagataaagacgttgcaccaacggagagatcccgtacgccagtgtagacaccagcagaggaatgcgttgagttaacgggcatgtttcgtctccttatatgactgtctgaaattatcgtataagcagttagaaacgcaaaaggggcagccgaagccacccctttgttttagcaatcacaacctacggaatcgaagtcaagtttcaggccaggatagagttggttaaactcctccagtggcatattaaagcctgcggcattaacgtgaccattaccaccacgagaacgtgcgataaaacgagcactacctacgtgaccttcaggtaaaccacgagaacgacagctaacgtaaaccttgcttgggtcacgatggccttggcgcacaagcatcactgtttggaaatggtcatagttctcatagacatacgttcctgtctcggacgcaatgcctttatcacaaggcacgactgcgtgtttgacaccaatcaaatggttaggttccgagaagaagctattggtagcaatcagaccacgaatcttttcattacgcgcttcgatattaacgaagccccgagcgatgatttcttcgatatcgccagacaaaatgatcttatacgcagcacggacggtaggaggcatttcagcgtagacgtgaccacacttctctacctctttgaagacgtccttaacgtaaccttcatagaaggcaaaggcacgttcattggtacgaatccacaggtcacggtcagacaccagctgcgcactgcgaatgatgttatcagtgcaggcatattgatgctgctggaactctgacacatgagccatgtatgtgagcagcgtaccactgccgccagctttgaaagtaagacccagcggagatacgtcaagcgcagcacactctttggcgtacagctcttggctgcggcaatcatggtgatcaagcaccttgaagttaccaccatagcgtttagtcatgacagccatctggcgctcggtcagagagaagtcaacaacgacaacgcgcgtatactcggaaggttcaccgattaacttaccgtcggcgtctttctgcaaatcgctgagtttgataccttcgagacccttcatgtcttcgaacttagtaccatcggcagaaacgatatctccctggtcgttggcgtacacggcaggatagaaatgaagagtatcgttagggtatgcaagtgctgtaatggcagcagcgaaactaccatcagcacatccttgatgatagacaacaagtgtagtcatgactaaacccagtggttattatgattcgttccagattggacgctgcgcatatgctcaagcatttgacgcaggcccgccaacgtccgctccagtgatacgcggtactgatcagaagccacactctctccgtggcgcagcgaaagaatataaagcgaccattcttccgattgacgcaggcgctccattttcttggagagaatctgacggcgttcacgagcacgtagcagacgctgcattaaattaagaggttcatgagattttttcagcaattcaatgtgaatcgcatccagtcgctcataatccaaacgcaacagggcctctttggcctcaaggaaaagtttggaacgacgcagtgcttcatccacaggaagattacgacacttatctgggtgagtgatacgtgcgataaccttgtagatagccttacatttcttacgcagatgcgtcttcgaccattgttcgtgctcggccatcatatctgcatctgcttcgttgtcctgagtttcatgctcagtgtcctcaacgaatgcttcttccatgatctttttgatatcatccgcgttggcttgatcttccaagtcatcggagttagccatttgcacgaccatcgcctgaatctcattgttcaagatttcaatctcggcgatgattggtcgatgttctttgttcaggccgtccaccagctttgtaacgcgttcgcaatcagcgccatagcgcagttcaagcgctgcgacttcttcgaggatttcgtcaagcgtttcgcctgtgtcttcctcaaactgctctaccgcatctaccagttcagtgggtgcggtgtgcggcacagggagttgagggataaccatcaactgagtatttgtcatgggcgcacaagctccgaaattggtttagctaccagctctgcaatgcgcggcggacactgagggttgcgtttcaaattcttatgcaaccactgcaagttattacctgacgaagatacctcagcacggaagctggggagtttgagttcgtcacgatgtttggccagcagcacattcagttcattcagcaacattgtttttccttaaagagatgaagtcatgagttcaagtaaatttgaaactacatgcgcaggtcctatggagatccctgtttgcgcctgtagatgaatacgtttcgtaaatagctcaagagggtcaggactgccgcctgtaactacaatgcgaggtatctttgggaacatctcaaggatatcacgcagtcgttcgatcttatagctggtgctatctagtgttacgttggtcagcactaacagtgagggacgcttgcttttgagttgttcatagtcgaagcgatcaccatacagcgttacccatcgtggcttgagtgcggttgtctctgagtcttcaacggcagcattgaagatagacagcgcggccatctttgcacggtagtcattcgggaaactactgattaccgtgatacgtgggtcagccttgaaagggtcctgaatcatacgtgcaagatgcgtaagctgtttcgctttaccaaccaccttgcccttgaagtaaggagaaatagtcttgtagtcctgtgcggcttctgccacatcaaactgctcttgcttaccgaataatagttgtgggtcaacgcccagcgtctgcatctgctttgctacagcaggttcaaagtcaaatgttagcacaataccctccgttgttcatgttaggtatttacagattctgtggcgcgctgccatactacgaacttgacgttcagggcatgttcttcaagctctgcctcacgtctaggatcatacttcggggagtgccagcgtgtatgatcaggacgttctacaggtttggtcacaaactgctgtattggatttggtacttgaaaatattcatggctctcgataacaactaagttatcaatgcggagaacaccaggaacatcaaacactttcggcaaggtgctcggtgtgagtgcagaccccataactgtttcatggtagtcaacaagtgctttaactaaagcacgaccagcacacgtagacagtgtaagattgtactcggtacgatattccatggtgctctccttagtattacatcagagccagttcagggtcgatatacgtgtattgccacacaatattccaacctgaggcggcgtctttgtttgggtgaatgcgatagccgtagatcatcagcttgcccttagtgtcaggttcaagcgtaggttcatactccagccatgctgcttcgagcttcaacttatcggcgatatctttcgcccaaccatcgaagtcgtaatcttctggtacttcccaagacagagaatgcttgcgccagtgttcagcctgcatgtcagtgtctttggagatccagtccagatgtgctacgcccagatggtaagcaatggcgtgtgcatatccatgctcattcatgtgacgctgtaactgatcaagacgcattaggttgctccttaaagcgtgggaatacggtaacgctaatgcgcgtagaacctttctcatactcacgctcactatgagacacaagtaggacgtctgtgacctccaaagtatctctaatgagagtgagcaactgcccaacaacggacagtggatggatatagttggagacaatcatattgatctctgttacctgatcaggattgcctacagcaccatttccatcccattcttctacgctcatacacgctcgggctccttcactctttagcaggtccatctccagagtgaagggtaaacgctctttcatcataaactccttatagcctgttgaaaagagacagactataaattagagagcgatgcctttaaggaacgttcgagcgaatttaataaagatcttctgctttgcctcaggcagcttgcgacagcgctggataatgtcttccagtgaatcttcatcagtggtgagatgaacgccctcgattgtaccgacttcacctttctgccagttagctttggtcactgtcaataggaaggtaccacgatactcctccatgctacgaccaccagcaccaccaacaggattgcgtactttagtgtagtcgatatcagcaatgcgctggacggcaaaaccatcagggaattgcgtaaacacagaagacagatcaatatctgctttattgtcaggtgcaggggatttagcaacgaactgcacacggaacgattcaccgccttcaacatcgtactggccatcgaagatgatgttgtcgtgcgcacgtagcgtatcggtaatgagtttgaaaatcggatcgttgaacatgttacttcctcagatagtcggccagcatttcaacatgattacgaatcatcttcctctggtcgagagtgagcttgctgaaaggaggcaggtctgggtaaataccctgcatcgccagatatgttgtctgtatattgcgcttcggttcgggcgcttcgccaaccgcaaagatacagtctttgaataaatatgatggcgggcagccgaatggggtgtccataacctcaatgtggccgcatccgagtaacatcagacagttacctaaagtcttacgcacatcactcatacccaagacggacagcttttcgtaggtagcatcaacaatgctggtggctgcaccttcgatagaaattttgactgtcacgtccagagtcgccgtggacgcacctaatacggacttgggcacaagagtaatgccctcctccgcgagggcacgccgcaacaaagtttcaaggtctctgtgtggctcggattgcatttcattaagatccattagagtcgcctcatacctaagttagatggctggcctttcacacgcgcttctggttcaaagaagtcaggcagttctccatcgagcgcttcttctctcgacacaactcccatccagtcacgcagtttcttcggtgtacgtttcgctttcgcgtagccaaatttccagcacatcttcaacacagagcgagcacactgcatcgagcgatccatcttctgatcgatgaacatgcgtatgactggagtgcgcttaccttccattggcgtcagaatacgacacgactcctgtttccagttcggctcgttattcattggcatgatgtagtacagcgtatcccacttcggaacgtttaggccgcgctgcatcaacttacgcataccaacaacgcagcgaatcttaccttcacgcgctgcatcaatgattggcttacgacgcttcgcttctttcgctcccccaaggaacactgccgcaacttcttccatgtaatgctcattgatacgctgcacaaggcgccgcgcctgatcagtgaacataatcggtatcgcaatgcttcgtcctgcatcgagatctttgataacccactcaaagattttgtcgttacgatcaggatggttggcaaggaacttacagaaacgaacccagccagctttcccgttatactgcgcacgggtctgcactttcttcgaggtcttatgcagcgtcactttcgggacaagctcttccacgaaggcttctgcaatcacaggcccgaagattgattcgatcaggtagtgacgtccatctttacgtttaggagtcgcagtcagaccgaaacgatacttcatcttgagagaggccagtgtgcgactgtagcagctcgcattaccggcgtgacattcatcgacgaacaaagtaccgtagttttcgttcagaagtttcaggcgcttcttcgagttcttactgtccgagataagtgactggtaagtaacgaggatgatctgaaagttcttgtagtcgtcgagagtctttgggaagccgtacagcttcttaccatgcttctcttccaactcaggcaggttcgtcatctgctcgatagtctcaagaaacccatcgagaaagtctttctggtcagccataatgacggtacggaatccagagtgacacgcaccagcagtaccgataactgtcttaccagaacgcggaggtgctttgaacacaccacacagttcgccgaacatcttctcgaacggctcttcctgatagtcacgcagcttaccagtaaacttcactttgtagtcatatggcacacggcttgtaccattgacgaacttcacttctttcaggcttaaccctgctgtacgttcgaagcggtgcatctcgccgtaaggaatcgaaacgtaacgcttacccttgatatcagagtatttagccagcacggttatatcaaccagaccacccttcgaacattgacggcattcttcggacggacgtatagaacgaaactcacagttcttacaagcggcgttgtcgaactcatagtgagtcatcttcttaatgatgttgtcagcgtctacatgcgtaacaggaatatgcagacggctatcgaccagtaccttggctgtcacatctatttcctttgattcggcagaccgtactcacgctgattaatcaagttcatcgtatcgaccagcgcacggtaggcaaacccgcacttgtcgatatccttgatataaaggtctaactcttccttgagcaaatcaagctgatcagcgtaacggtaatactccgccataatgtttctgacacaacgctcacgctctttggcggcgccgacggctttcagatctcgtgcataggttaccgaggcataatcctgaaaacgttccagcatatcatttaacagcttcgaggctgcgtggacatgcgtcatgatttcagtcatacggcttcgataagactgatcttgaattatcgactccgctaccttgttaagagcattagggtcaccagtcacattcagcgttctgaccttgcgcatcttaaacagcttacgcgcttcgtcctgatactctgccagaggcatctgaaacaggtcattggtcttgtagatatcgcgcaacttcttatagcgcttatcttccttgaccttgagtcgtatacgctttaggtcatccatcaatcgcctctatcggttacaagcagtggactgtcaggagtcttatgaggcatggcaaagaaacttccatgctcgtcacgataaatcaacagaccaccagacggcccttcaatcgggcaggtgaagttaaagagtttttcgagtggtggcatatagcccacagacacatcgttaaacgtacaccacttcgcagatatctccagcatagagccaacaacagtgtcagccaaacgcaggtatgattgtttgaagtggtagctgtgttcgataggagcaacgctatcaatcgttaactcagtaccatacaccgctttataaattaggcagaaacgtctgcgtccccgaggggcattcggtatttcatacaacacatcatgtatgagagatgaaacgtccccagagaggacgtttttcttgacaactagtgccgtcatgctgggaggtaaccgaagtacagcagagtgtgcgtgtcgaacttatagttcaggctgaacgcattcaacgagttgatgctgctaccgtgaaagcccatgttgtgtcgttcttcacgcccaatgttacgcagcaactcacggatgatacgcatgtcgagagaggtggtgaactccttctcaatcggcttcgccagtttcaggctgtcctgtacgctaccgctatcattaccaaacttgagtcggaactcttgtttcttaacatgcagcttcgcgttcgtgttgcctttcttctcaatcagcgtcgagatgttagcaaacggtgcagacaggtcacctttgattacgcaacccagaataggtttacctagctgtgcaatcatgttgtccatatagcgatagtcttcatcgcttgcctgaatcgggggcagagtcagaacgaacgattcggcttcggcagcaaacgatgtgctgtcaacatggaacgttaccttttcttcgccgcagaagcgatagacaaggtcgaacatctcacctgtcatgctgaaacggaacgcaggcactttcttcttcaactcgaaacgataacgcgatgaagtccagtgaccaggactgactaagctaaggctcttaccgtcgcagataacacgacacataacagtctgtcctgtgatggtatctttcagacgagtcagcttgacgccctgagtcatcgcgtcgattacttcacgcgtcatctcatggccaccttcgatgtggtgatgcagaccctgttcaaccatcggaatttgttcggcagatactggacgcagtttcacttctgctttgtatttgcctttctgctcgcggatgttcaagactttaccatcgaactcaacgctcagttccttacgcttgttaatcagaccagtcaactgaatcgggtcgatgttcatgattgtatcagcgtcagcagttgcaccaggaacaaggtacgctacgaacgtgtcaggcgtacggcccagcacgaacacgtcagacttatacgttaccagcagatggatatgcgtcaacttatcgtccgactcagagaagcgcgtcacaaggtcaacacgtttcagaatatccgacaggaacgtaccgttcaatgtcaggttgcacttcttagcgggattcttcggcagtcggcaagtcttcatctctatcctctaaaacaaattgtagtgtgccctgtatatttacagcttcaaggcgcttacctgttggcataagcagaccgtttaacaggccaacgaagtcagcgctgtagcagtctggagcgatctggtggacgtagatatcgtcaggaacatcctgaggattaagctgccaagcagtacgcaaggcagctcccatgaaagcaggacgctcgaccagatgcctgttcagaaacgaacaaatatcttcggcgcttaacgtcatttcttgctgatccccttaattgcgttcttgagaagggacttgctgattttgattttcttcggagcactttcaccagcagaggctgcggctttcttagcttcctcttctgctttatatttctcgaaggtcttggtgttcttaggaagctcggcaagccattctttgacgttcttcttatccttgttggtaagaggattgactttgtccatcgaccgaatcttaatgtcgttagcccaaagctgtttcttcatccaatcggacataaggtgatactggtcctgcaggatgctgtcaacagtcttgtcaacatcaaggtccttctcaccaagctcgtcacgtttaatgatcaagccgtctttgataagtttgtggagctgaacataagagaagttccagccctgcacatctttctcggacgcaccaatctcaaagtcaatctcaggaacggacgtgaactcaaacccttcatgacgcttctgcacaacttcgaccactgcgctggtcatcgcacgttcgatcatatcgagtgcaaggaagatccatttgtaatcgcagtctacggtcaaggagtcgtgtacagatacgttcatgtcgaagtcaggatagtcgccattagctctccagtattcaaacttcatgcggtccagaatacgaatcgcggacatcatcaagtcagagccgaagccctgcactggactgtttaccgcacgacggtcacaagcggcatgaaccatgttcgcttctttgtgtgactcaggcagcatcaggccccatagatgacgacgacgaccaactggagattcaacatagaagttctcgtgtgcaaacttcttgattttgtcgaaccattttaagccaacagggaaacgtgttaagaacttgcctttgatttctgcaatctctttcacgtcacggccagtagacttagcaagacctttatcgccctgctgatagatcagtccgaagataactgtcttaaccgcgttacgtacggacttggttacatccattacgtttggaataccgaagaagtatgcggcgttgattttgtggacgtcaccctctgcttcgacgcggtgttcaatccacggatctggcacagtacggtaacgatgacgcagcgttcgaccctgttcgaatacgtctgctacgccttggtcgccagagatgatcgaccagccccttacttcgtgggctgagtagtcgaccttgatcagtaagcgatttcgacgtgcaatcaagatacgcttgatcagtttacccatctcactacggctcggtacctgctgcaagttggggtcagacgctgaggtacgacccgttacaaccccaagataaccatacgtcggtcggattgatctatcgtgtttgaagtcttccgattcgccccagagtttaagcaggctgttaacgtaggcgttcttgagcttgtacgcctttccgagtttcgagtagagagcaacaagcggtatatctgcatacgccgcctggaagtccttgtccagcttgcctgtcttcttaccgttctcacgtaactgttccccttctttcagaggcttgagtttcatcacgtcgaagaacaggatttgtttatgctccgacttcgacatatcaaacttcgttacctcaacgcgtcccataagacccatcttaggaacgttatcgtcttggcatatcagtttgttcgcagccttgacctcagggctgttcatgaactcacgctccacgtttcgaatctcctcgttaatcggggagttcggtaagttgagcttaaacaggtagtcgatatcagcaccagcgcctgttgtctccagaatcgagaacgcatgaatctggtcggagatttgttcactgaccatagactcatacttggcgtacttgatatcgttcgcacgaagcatctgcttctctgctatacggaaaggtacgataacgtcgagacccgcgtattcttgaacactctcgtccaagtcaacatcggcaatcgttgctcgcatctccttaccgaacgatacttcatgatacacctgacagccatactgcattgtcaggttcgctaagttgtagtaaccagcgccagtaacgttaagcaatgacttcgcgttttcatcgttcgcaaattcacctgcctgaatatcccagacgttcgctgcataactacgaatgccgaagttggagcgcattacgttcaggtcgaacttcgcgttggtatagatctgatacttgttggagttatcctcgaagtagtctttcaacatcgagctgactttacgcaactctttaggagtaaacgggctgtcgcggtgatagattggaatgacatacgccttcttgccgtcacaggaaagctgtaccgtcagaatcttattcttgatacgattcaggttctctgtttcggtatcgactgcaaccttcttggcgcgcttcatacgcttcaagattttctcaagttgcttgaccttagttacatacacaaggtcccagttacgcttcttaccacacgtaacctcgtcgatcttataacgcattcccttgttcaaccaaggcaacatccaacgtgccatgtagcctaacgtgtacgatgaccctttgatgtgcattgggttcaatacggtatgatagctcacgttcggcagatggatgaagctatgcttcttaccatcactcttaaccttggttggaatctcgacaccgtaccaatgctcgtagtggtctttcgagaattgaatcttctcgttgttcagcgccttgaacggtgccttaccgaacgtcaaaacatagtcaggcttatagctgacgatgatctcacgaatacgttcggcgaatgctgcgtcagcgtcttccttaaactgctcacccttatcataggttttgaacatgttatacgagataacaaggaagctccagtcgtcgagagtggtcttgaccggaaacgtatcttcaagatactgcatctggttcagaaacaactcaccttcggttgaagtaaagatcttaccgctgcgcaagtcttctgtaggcatatgatcgaggacgagtagtgctttaccgcctttagcgcttttacttacgcttttcagaagtcgaacaccgtcataggtctgcgtgtctgcaaactgctctggcgggtcgaagtcaagagctataaacttgggtttgttcaccatctagtcctatcaaagtgtgtatcacaatatgatggcagttatttacagatttagaaatgaaaaagggcaccctaaggcaccctttttgtctagttatgctcggcgttgccgacgctggatatcggatcgttcctcagaacgagcatcagcagcgccgcgtttggctacgtcagtatgatcggcaatgaaagatgcgatgcctttcttatcagtgatagcaaacgattgaattttaggatttggatggaacttaccgctacttgcgatacgccagctatctccgatagattcaatgcggaaggttacgaaattaccacgattgagcacgaagtagtcagcagactcattcgaaattttgaagccagtgcgcttaatccctgtgtctgcaaagaataagtcagacattttgccctgacgttttcctttagacgtccgtgcttcttttttagtggcggacttaccgataacgtccttgacagccttagcgagagcagcagccgtaggagacttcagttcgttgcctacgtagataccacctctgttatctaccgcagacactgcccatttaattgagcgcatctgagagtggaacgcataaggcgggtcaatagacacgctcttgtatcctgctttaggattagttgcttcgaagacccacggactagactgaccgttagtctcctggtagatgggcaggaatttcaggcctgtagctttcgacaactgatcggcaatggcgtcagtttgtgcctgggtgactgtcttcatgaacgcaggagtaatgcgcgccagatcgactttaggcagttctgcgttttgattgacgcgggtcgccacaactctagcagacttgatacctacatcaccttttgtcttagcgacaggtgcaggcttaacgtctactttagccgcagcatttggtgcagtcactttgattttgattgcacgtaggccgttgatggtagctaccagagtcttcgccttgaacaagtttttaatcgcagtgactgcgttcttgcctgctgctttcttggcgaaggccgtcgtcgcttctgtgtctttcagaatgtctagaacggcttcgagcttagacgtgtccagctctttgatcttcgtcagctcgtcgatacgcttgatcaacactttggcgttcttaccaaagagaatctctgcgttagtggcctgagctttagtcacagcggatagtgataccactgaaccgttgttcatcgtcatgttgtacattgctgttccttatcgcttcttggtccagttggagttctgtttgccctgctgctgctgctgctgctgcgtgttctgcgcgggctgttctgtgttttccatttcttcttctgtctcaacgtcatcttcttcctcgtcgatgactggcttcgcttctggctctggtgcctgcgtctgcgtgttgagcgatgttgccgctagaggtgctgcctgcaacgtatttacagtagctacaggctcctgcacggcaaccttgcgcgcctgagcaacttcacctactgcgtgttcgtgcaccagatcgacagtcacgagctgacctttctctttcaagatttcatcagctcgtgcttggtcccattgatcccaaagaatgtccagacctttgtgcaggtagttcatacccttcggcagcttaccgcgaccgttgaatggcaggccgttcgaaggagtagctggctcaaactcgtccatcatctcccacttacgtttcgcttcaatacacttcggtccccatacgccgtcacacaaaccatcatagagtcccatcatggtcatgatcagctggagcttttggtagaacttgtttagcattgtcgttctcctaagagaaaggggccgaagcccctcagtctaattacactgccttgtttttggtagtggtgagtttcagacggtcaagcgccgtcgtcactttcttgatgttcgtgatattgtaaccagctttcacgatcttgttgatacgtgctttagcgccagcgacattcttcacgaaaccaatccacatgccaggtgaggagtcgaaagtaccaaacttacgagtgtttggaatcttcgtaccgatgaagcgtttcatctgcgggttcgtgttcaggtcgaacatgatgcgcagacgatcttccatcaccatcgggtatgccttgacgtgtttcttatcagaggctgccttgtgacgaatcaggaagaactgcttcaactgctcttgagctttcaacgccagtttgatgttgaagcccatacgcggcgtagactcgtcgaagaagtccagcacgaactccaagcgcttctcagaaggcttgtcgaacaccagtttcttcttaacctctatgaagtcgagcatcttctcgaagtctgcatagtaggcacagtcgtaatacacgtagtcaccaaactccacgaagtcgaatgctttgagggctttcgcatcagggtcggtggcgttcgcgtacagagccacgaagccgttgtatacggtaggagtcaattcgagctccatgtccgcaccagttgcgtcttcaacagcggcagcaacaggtttcttacgacgggttgtgttgtccagcgcaggcagatcagcaggcttacgacgacgaacacgaccagcagcctcagcaacaccttcgttgattggcttaccttctgccttgttctcggtacgtttcttggcacgagcggtcttacgcgctactgccacaaccttcttctctgtctcaaccgtatcggcagtctcagtctcgtcctgaatggtgtcttcaacttcaacacgattcgcttcggctgtagcacgtttgcgatctttctcattcgcccacggcttacgagtctcgaagaacttcttgagatcagacttatcaactttcgttgcgatgtgaaccttagacgcagggaagctgacggtctcgcctgtaccagccagacgcacacgcacggtactgattggactgtctgcacggagtttaccgtcaacagtacgcacagtcacagacactacaacaccattgccgtactcagtcacgacaggcgcacggaccagagagtctttcaggccttcgccgcttgtgaagttacggttacgcgcccagtcaagcagacgctcaaggccccagccgtagcggtcaggaatcttctggttagcaacaaacggagtctgttccataacacggaagtcgttcagagcaggcgtggacggcagtgcttgcattgctgcaatcgtcgtcttacgcatctcttggaactcctgagactcgatatcgttcagctcacgtttcgcaatgaagtaatctgcgaagtccgccattgtgttgttatcaatcaggagcttggcgctcattttgattgggtccaacttgaactgatcgagtgcttcgtaacgctggttgcccttctcgtcgaagcgcgttttctccagtgtcttccacatcagacgagcgaccttaccaacttcaagggtcttgttcgtcatcacccagtcgataaacacaacttcacgggccatgtcacctggcttaccgttctcgtcgagttttgcagcagcaacatcaggacggaagatacgcgcagtagactggtcgtaagtacctggtgaccacggcgtatcgcagcggatgatacggctacccatctgcatgttgtggccttcggagattgcctgttcgttcgcaatcagaatctggacgttgttgtccgttttgaatgcgtcgaggttagcgtctttgttttgccccagcttaccaacttcaccgtgatagactacagcgactttcttgtagttctcaggcagagcgttgtagatagcgtttgcggaacggacatagcgcgtgaagacaatcagtttaccttgcacctctggtttccagtagtctggatcatccggtggaggcgtcattgaaggtggcagcgcttgacgcttgaactcttcggactgcttacgtgccagatacttctgaccgttgtagacagcaatgtccagttcacgaggagtaacgcctggcttccagtcgaagatctgctgttcaccaaccatctggtcacgctcaggctgcacttcgaagtgcttcttgatgcggtcgatgattgtcatgactttagcagaagtgaagctggtaacgcctgcggcttcaaacgtcatacgtgcaacgtcatcacccatcgggtcagtcaacatcatttccatacgctggaagtacatgttcaggtcagcgttgcctgcgagcagcgcacccaggtcatcgccttcttcgatatcgtcttcgtcaatgtcggaagcggcatcgttatcaccaccagcatcttcgtcgtcgtcatcgttggaggcagaggctttgcgcttcgcagcgttagcagcttcctgcaatttctccagcacctgctcatacatcgcgctgtacacttcaaggtgtaggcccgagtttggaacagatgggtcatcgatctcaacctgaataaaggtatcaatcgggttaggcagcatgaacgcccagtgcttacgcttgaacgagatgaacgcagtgtggttcgccatacgggagtgagcacgacgaatcatttcgatatcgtccttcgcaccgtcgtaagccacatcaaggttatcaccaaacatagctggtgtcatcaacgcagcctgacctacgatatcacgcacacggtctgttaccagagtaccggtagcgatacgagcatagcgaacggacggagcggtgaacactgctttggtgttgaagtgcacctgagaaccagcctgaccaccagagaagttcttcaccttgtgcgattcatcaagcagcacatagctgaaacggaagcggttgacgaactctacagcaccacgaatacgaacgcgcacaccgccaatgtcaacgttgaacgtaccagtctgcaagaagctcaagcccacgatgtagatcgtgttgcgaggagcctgctggataacgtcatacatgcggtcttcgccccacgtgttaacagtgtcagcagtaataggcactgcgttccagccgtcaacgattttgtggaggtcatcacaccagttcgccacgaggttagatgggcagatgatcagaggacgaattgtttcttcacccaggtcatccagctctttaatcagagcagcaacgtcagacagaccgatgatagtcttaccaccgccaggcgcgataaagatagtcgcaaagcgaggacggcgacgcagagttttatgcgcttcaacctgatgtggaagtaacgcagcaccatcacgtaaacctgggatacggatatcgtcaatcgtgataccgctgtccggtttcagtttctcaatctccacctcagcctgttcgaagtattcgagagacttaggaatcacttcgctgtacagcgcggcgaacggcagaatgatctgctgcaaacggtcggagccaggagccgtgtcgctttcaatcagagagctaaacagcttcttacgatcagacttagtgatcgcattggacatttcacggtagactgcaccaccaaagtagttgttcagtcgggccatgtcagccagcttcgacgtttcacccatcacgaagtagtgagtgtgtgacggcagcgattctgttgcagcctgaatgcttcccatctcggtgagagaggtagagatcaggtttgaaccacgcagaccagcagcatcgttcagtacgcgaatcatgatacgcatcatggtcagtgctggacgctcttccgcaatctcagggatcgagaagtcgttctcaatcaggttctgatacaggttctggtccattggactttctgccaatgaagcgttctccgcatccataccgattgcaacacgcgcgttctgaatcagcgtcttcatgtcaggaacttgtttgttcttgagcatgaactcatacgtctgacaagtagacgcaatgatctgaatcagttcgtgaaggtttgaaccttcggtgctgttgtacttgatagtgctatcagaaacagcctctaccaaacgacctgcaccagactcagctttcgccgcttcaatcatcatgtcgttagacgtgcgataagcaggcatcatgccagaggactggttcttatggatgttaccgatcacgttcgacacagagcgatagttcggtgcttcaccaggctctgcaaagtcataacccaatgagtcagcaacgtccagagatgtaggagatttcataccaacggtacgagtctctttaacatcaaggccgccaccattcgaagtgttaacgatcagcgcgaagtctgggtcgataccaatacacacgttgctgaaacgattcagggttttagctttagcctgaatatcgcggtcgaagtccagattgccgttctgaatagcgaatatgctggtgcgcagtgtatcgtggtcagtagacagtggcacacctttctcaaacaggctctccagcacatcgttcagcgtagtctcgtagttacggaccatctcaacgtcaatatcttcgcggcgaggcaacacagcgagagtaccgttcggcatgatcgtcagaccgttgtcatcagcaacaacgtcattaactacataaccaaacttctcacggagtttcttcaactcaggcagagtggtggccgaggtgacgtaccgtgggatacgcgcagcacgagtgatacctgtacgggtcgaaccagcaacacggaagtaatagctcgcccagccttggaaccaacgatacagacacatggtctgcgtgtcagcgccctgagagatatactccaccagctctttttcgaagttaacgatcaacccagcttcaacacgaacgtcgatagcgagagcaacatcgttaaagtcaacaggcgtgtcgtgactgatcttcatcgcctggagcttgcgctcaatcattgccttgcccggcacaggacgaataccgatagtcatgaagtcgcccagcgcttctgaggcagacttatccagattacggaacaagtcaatgtcgatgccgttcatcgcagggtgaatagagcgtagtgctgcgttataaacagaccagtctttatcgagagagatacggaccatcttcgtatcaaagacattgccgttggagcgctctacgccgaagatatctttgtacagagtcttcgccacacgaatcgcagactgagcgatctcggagctgtatgtacgcagattggcgctttcgaagctcgcatcgttatcaacgcgaggacggtcgctaccctgattgttcaggacgttgaagttaccgtgcgcggccagttggctggtaggaacaggcgtaccggccatgacgatatctttaccgccaggatagcgcgtactgttttcaacgatagcgccagacgaggcagacagatgctcggcgagtgaggtcttaatctcacggctcagcttatctccgttcagcgtcatgttaatgcgcatggtcgccagatcgatgttcgccttgatacgcttggtaaactcctcaggagcaacttccagcatatcttcgaactctgcaccgttgacgacgatgtagctgatcaggtcaaaggctgcgtataagcgagcgacggtcgacgcggtgaatactgcaagggtttcgtagttacgacgagacttccctgtagcatacatcttcgacattttaccatcgaacgcgggcggcaacgcacggatagcaagcgcctggttaaaggtgtcggcgatctgctgggttgcggttgctgaggtactgatcatttgattcatcattcacccagtttactatagttgtcgattacagacgtccacaccgcaggtacaggcaggcgtcggtccgcagcaatatcagaaagcacgatggccagcgcataagcacgaagtggtttcaatccctcaaacttatcgcgggtgaacaccgaagtcagttgctcattggtcaacgtctgatactgcgctctgtattcagtcaggtaggtgcgatacttaccgtcgtcaacaggcgtggtgtcaggagtgttttgcacatagagcagcgctttccccaacgcatccataatcagcagcaggtctgcttgatcgtacggcgtgatatcaggaacgttagaagtgccgagcagttcaatgactgactcaggcaattggataggctcttgggcctcagatatggactcaataatcccctgcgcagcacccgcatagctctttccgcttaacgagatacttgacagtaaggaatggagccgcgtatttacgtcgtgcgtcacggttcttctcctagataaaaatgctcttgaccagagagttgagtttcttttccacagcatgtttcttatgcgtggtcaggaagctgcacaggcgacgggactgtagatgcagagcaatagcattgcccttgacgcgcatacaatcaacacccagatcaatattccacggatgccaagcacggggtgcaagcatcgcctgttggatatttggataagtgtccaccacaacgggtatcgcagacttcgccagtttcttggtcaaattatcagttttgaacaaagccttaggctgtttgttcgaaaaccagtaaggaatctgcttgtgaagcaactcacccactttcggaataccactacgagtagtctgaggtacatagaccaaatagatatcgatcgtggtattgatgcagttcgcaacacggttataatcgctggtggtccgtgaatgaacttcggcgagtttgaacttattggtgaactcaatgcgttgtaaccactgacgcaagtcctgttgttgcagacggagcagagcgcgggccgtctcaagagaatgcttagtcacagaaggaataggacggagcagatacttagtgctcgtcttcgccagcgaggacatgaaaccttcaacaacacgctgcatgcccaaaggctgaggcagcgaatggaataaatcgactgcggtctgtgttgttatgaacgcaccccacgcttcgatgtactctgggctaacgcaatcagggaacgcacgtaggttcagtcctacttcggagccatagcgtttcaaacgactcactttctacctccgtgcagcagtctggaacctctgcggttcgcagtgcctatctgattattatcgcacacatagcatagcagttcaagattgtgcttcatgttagagccgccattagcgtgtgcaattttatggttgagtataagctctcgcgtaggcttaccacaacgttcgcagtaatagccacgctcgtcgatgatactcattttgagcgtggtccattctgctcgatccatacggacgtgagtgcctgcgcgagcgcgttcaaatccagttactccagcaagacgctgagaggtagacagactccgcccacgtcctccttgtgctcttgctgcaataccacctctaggtctgtatgccatgtgcctattctcctaaatacaatgatatttacagacttacgcagaggcggagaagatctgtaccgtcttatccagtccagcttgatacgattgctccacgtcttttgcagcacgtcgaatgatgttctgcgtagagttctgggcagcagagataagctcaacaggcaggttctttttgttccaggcattaatctggtggaacacgccaacaagaatcgtaccagcagattcggcgaacgggccaagtacctctgcgttaagaatctcacccaactggccaacgtcacgcagcgcacgtaggtctgcaatgatctcacgcatctggttatacagttgcataagcgcgtagatatcacggctctgtttcttgtctcggtaggcaccttcgcatagacgcgccatgttctgacattgtttgaacatggtcatgtactctgcaatctggtcgttctcctgtttgatgacgtcagggatttcatccatgacttccatcaactgcccttcgagaacagccacatcggtaatgcctttcttaatcttatccttcttggacttcttcttgattgtatcggcagcgttttctttcttctttttcttcttcggcttttcgtcgatagaagatattgccttttgggtactggcgatatctgcgtaaagttcttctgggttaagaacacctggcatgatatctttcgaagggtctttcttctttttctttttgactttcacgcctttgctaactgtcttagctttaacagcggtagtcttagctttcactttcgctttgcctttctttgtaggctgtgcgtaagagccaatgtcatccaagcttatggccgccatgtgaaaatcctctgtagaaacgaaaaagggaaccccgcgaggctccctttagggtttgattagaaactgtgacctttgatgataccagcaatcttgctgtagtagtccgggctgtagcggaacacttgagcatagtagctcaacagcttaggtacgtcaacgccagcagcggcagacacgctatcaacggcagggaactggttcgggtccagttcgtcgccagacagaacagcaaccatagacatggagctaatctgttcttcgttgccttcctgatcaaccaccagcatggtgttgtcatcggtaacgttagcagcaacgaaaccaatcttcaacgcgcctgagttagacacgaagctgaccatatcgccgcctacagcagccgccagaaccgcttcattgcgcaggatagcctgagccaattcaggacgctgagccgagaagttaacagtcgatgcaccgctgacagaacgaatcatgtcaatcagttcagcgttgtcattggcggagctgtcacgcaccagaacgtcttcaccggattcagatttacgcacatgccacatgcgctcgctctggtccatgtacatgttcttagacagtgcctggaactgatcgcccatctgagacacagggatgatatcctgcatacggctcatgatagtacgcacgaagctggtggtcttaccgccttcgatcagagtggatgcaccgtcgactggaagatattcgcggttgcaggatgcacttacgattgcgccgaagttatcagcgatgttctcaccctgtgcgtgggttaactgtacgatggcaacgctctgagtgtcgttgacctgatcgatctgtttaatgaaagccttcattgtcatctcctgaatatttcgacaatatgaaattagtatacttagggttagccagtgacgcgataacgtgcattgacccagatactgcggttaccaacagtagcccatttggtggttgggctgtttgtgatgccgagcttgccgagtgaacgtgcaccgtcaatcgcattggcaccctgagaaccatcaccgtcgtttattccagctttagacagtttgttcttcaagttcgtaacaggaccttgaatctccgtttcgagtttgcctaaagcagactcgatagacggcgtacggtccatgtttaagttaaccacctgaccggtgaagtcaaatgccaactgaccttctgcttgcagttgagccgcaagcgcgtagtacgaagcgcagataacccaaccattaaggatggtgccttgcatattcgtgccgttgaaacccgtcacacgaggaccaatcgtgttgaacagcgcaagcccacgatagagatagttgatgatctctgcctgagtatattccaactcagggataacgttcatcgcacgggctttgttgatgtggtcttctaccatagatgctgcgatcagaatctgcggtgtaacaacccagagcttgtacgtgaacatcttcgtggtcttacgagtgttcgatgtgtgctgtgcgattaagctgataggctccagtcgtctgactgctacccacacaggaatctgaaacacacaagtcttggcgcggttcacaaccatcttcacaccagaatcaccgccgtcgatatccgaagcaatgatttggttgttgagtgcaagttggaatctcagcttatcgccacgcgtgtcgaagtgaaacggcaacgtcatctcaaacgtttcgtcatcaccgaacaggcacacgatatctgtcacgcggttctctgtcataggctcaacaatgagttcctgacgagactgcatgattccttcttccgactcatagcgccatgagagcagcaaacgtttatcgtccaccagccccatgttaggcacagcaacatcagcagtccatgcgcccgggatttccccaggcgtagcgactacctgtgccagaatcgatctatcatcagggtcaatgaggcttacgacaggccccatgtcatctgatagcgggtacagtggttcgtctaggtcgttatagaaactttcctcgactaccagtacgttaccttctgttgtgcgcatatcagtctgccttagtgagtcccagatactcaatcagattgcgtagctggtcgttatacccaccttcgattagcgctctcgccattgatacgtggttggagttcgctgtacgcactaccttagcctgatagtcaggaacgttttgcatgttctgattcaggttgtagaagtagctacgcacgaagttcgttcgctccacgttactcgcttccatgtcgctggtgtcctgtgtaggtgtcagcaacaggtagagggcggcaagcagttcaggagactgatcgaccatcggagaggcaagcgaagcagcgagcttcatcagacccttcgatacgaagtcaacaacagtcttctcaatatacgccgtgcccgctttgcctacgttaggcagatacaggccaggcaggatgtagatgcagaagtacagcgggaagtctttacgcatcacgtcagagataagcatctctgagtagtccttccagatgttcacgttgaagtgccattcgtcgtaaggcacagtgcgcattaagttagacacggacaggtctttcacttggttcgcctgcgatgcaagatcgcgagcgctctgcgaaggagtcagtgacgaactagataccagctggacgtagttgcgagtgactgcgcctacagtgttgtagactacgttcaacatttcaacgccgttaccgttcaggccgaagataacagaacgaggaagaccgatggtgatgtactcgttgttattgtccacgccccacaagcgccagtaacgcccgcgtccaagttgagtcataggctgcgggagaatacggttagcgcgaggtttcaggcagaacgtgaaacagataccgctgtcaatcatgatcactgaatcatcagggcgattcgaataacccatcgacatatcgttgtcggtactgtacacgttcaccagagtgaagttcagagccttagtgaaaggcatctgcgcttcaatcaaatagccgaggacttgtcgaaggatagtatcgagcacatatggagtagcagaacgcatttgctgcggacgatattgcccgctgtatgtgttctctttaaatgtgcgatctaccttgaagtgcgtcaacgccattacttaaccgattgcttgagcaaacgtttctgcgcagggttcaggcccatcacgtctgcgatttcatcaatcttacgcagagtcagaacgcccttagcagtaccacctgaacctgtcaggctgatcttaaccagctcgcgcccgctacgaccacgaacgatctgatggataacgctgttcttacctccacgccccgcacgaagtacggtagatgccatgcccaggatttcagtgatagcttctttcttctcggtggggctaaggccaggcaccagacgaacgtacaggctatcgttctgcacacgcacgttgtcgaagatctctttcttacgaccacgaatatcgtgttgagcattacccagttgcgtagtgtcgcgcaggttctgagtagagcggttgattggcttgcgttcgctatagttcaggaagccgtcaacagccatgagctggttgatagtacgcttcatttctggagcagtagcaatcagacggcccatagggaaactacccggaaccttctcgtcaacgagtgacgtaaggaagttttcgctaatgccgcttgccaccgcgatcgtggtagacagcaccattgcgtagttcggatagtgcaggccttctgagttcacgaagttatcaatgaacacataggtctggaagcagatagggtccgtgccagacgcgatgaaggtacgtgtacgaatcttcgaatagtcttctttattcagaatcttcgacaggtagttggcgatggttgcagccagcttggtatgttctttaggagcgccgttcttaacgtcgatgctcataagtttaaccagacgttgctgctgggtcttcgcctgttcgatgacacttaacagagacttcgcggctgcgttctgatctttgaatgcgctgaaagttttgctgctaagaatctggtaggctactgccagttcaccaattgcttggctcagttggctcacctgattgttatactgcgctttactgcggacgtcagtgatatcaatcttagacaggtcgataacctgattcaggtcaatcgctttggcctgtttgcctttgattgagccttcgagatcagccagctcaacagctttagggctggcgctgaccgacagaagtttctttggaatagtgactgaggtggctttagcgataactttgtcgagtacgttacggaactctttcgctgtacgcgcaccgcgtaacgcagtcatattcccagagctatagtcaacagatgcgctgatgctgctaacttcattgtttttggcagtcttagccatgatcatcctctactgggtctagtattcatgtcgggtaaaaattagcgactaaggccggttttacccgacatgactactttacaatttattgttgagtgaactgcttcataagagaattaaggaacgattcacgcacggtaacgtactcggtaccaagcactcttgacgcagagaggaatgaaatagcaccagagccttcggtgaggaacatcatctcagctacaggcacgcctgcttccttggctgcttctttgatatagaattcgagaatgctggtattgtttaccgcaccttcaaatcgacgcaacgctgctctatgttctttcttgcccaaggacataacgttatctttcaactgccctcggatctcagtatacaggttgatgtttaacggcgtgaagcctgacataacctttgacgcaggttcgaagtaaggagactgcgtgatgtaccggcgcatgagcgtgttgttagcgacaggagggacagggtctgggcgctcacgttcgaagtacagagaggttaccgctgtacccatctccatgtccttcatatcgaagtcagcacggaagaaattcataggcgttgtgaatgtacgactgacgctctgggcaatttcccagaatgcagcctcacgtttatcggcctctacctgctgcacgttagcccagatctctgtaagcgcattagggtaagcgcccatcagttgttcagacctgttgtacatactcaccattctaatcttctggcgcatatctgtatcagggtctgcaatcaacgcgaggccaagcgcaatcggtgcacagttctctgcggtacgttgcagatcacgcgcctccgttctgccccagttcttcttaacgaaagccaagaagcgattagcgagggccagttgcttactcggcacaggcacgccagtgatagcgtcaatcacacgttgagggaatgcagggtacgcccaacgctctttcagtagatcagcaacgacgtcgaaatggtcgatcgtcaaatctgccagggtcttgatgagagagttacgaggtgcagtaatccgaagcatttgctgcaccagctctttgggatcagtacgagccatctgtgaatagcggagttcattatacaccgtatcgttctgttcagcagtaggcttagaggcatcgtgctggaaatcacctcgctgcacatcatcgtacaggccttcatgaccaatcagagtcaacgtggtcgcaccgttagacaacgctgggttgatgttagcgtcaaaccaatcctgcacacgcataacgaacgtggcattcttatctggatacgcacggtctgccagatataccacagggctgcctttcttaccgacacgaggcttagcgtcgttaacgtcgaagtaaggtttcaacagacagcgagacacaggacgattgaggttcttatcttgcgcgtcaatcaggtatgcgataagcgttccgttcttcacgtccgctttaacgtgctggcgctctgcaccatgagtcagttccatgcagctaacccaaccacgatcagtggacatgcctgcgatatcatatgggtgcattgatacacagaccatgcgacctactttggactcctgcgcaacgatcttacgattaggatcagaatcgaacatctttttgagttcagcttctttcgcaagcactttacccagacgcacagtacgtccgtgtgagtcacgaccaacaccagcaaagtaatcgagtacagtgattttctttgaagcgaggaagtcattgataggctgcggtgcagatgaagtagggtcagctttcttgataacgttatggcccacatcgaaatagatgcgcattgccttgcgtcccttcttgccgctaatcttttcaaacacttttaacagtgctttattcggcacccaacttttcaggaagggtctgtactgggaaggctttagcgcagatagacttacgttaagttccatggtgtctctcattgttcaggagtgatgcgaaaaattagcgacaagaatacaaaaaggggcagccgaagccacccctttttgtttgtgtatcgtagtaccgaccaggtcgattaaacgatcactttaccttttttcttggtcttagcagctttcttaccagctactttctgagccgcggtgccggtgtgcttaacggctttagcagtagtctgcttaccgcctttcaggcgcggcagtggtttcagcttaggcttaaccagagttactgctttcggctgtacttttggagttaccagcttgccgtctttaacggtaggcttacgcgctttacgtgcggccatacgcgctttctgttttgcgatcaggtttttgtagccagctttctgtttggctgccaggttgctctgagcaactttctgacgggccagcagcagcttgcgaactttgtcctgagaaactttggtagctttcaggccagcctgatacttacccagacgctctttcagacgctgctcgatagacttcgctttacctttcttagcctgcttacgcaggtgattagcacgttcgttgtcgaacttcttctcggaagaagtacgcgcagccttcttcgctttggctggcttggcggcagcaggagctttagcagcttttgctttcttcgcttttgcaggtttagcagcggctggcttggcagcttttgcttttttagctttaggcgctttcgcagccgcaggctttttggtcatctttggatctttggtgcttttcagtttgcgttttacggccatgattatatcctcaagttacaattgaactttcgtccttcgggacattaaagtttttgaaatcagcatgtaaaaattagtataatctctccaggattcctgaggaaatttcctaaacatttttacatagcagtataccctatttcagataacaccgcgttaagttctttgcgagcacttatccgcaaagactttttaattccagacgccttaaggtaatccttgaggccatcacgtgggtcaatatccgcaagcgccagctcactaacatcaactgtatctatattatcgagatcgacacgtttattcgtggaattaatttgggaaatatttggaacgcgagtacggatatctgctgggatcgacacggtatcttttacgatgacacgataacggatcgctgggtttacttcaaggcgtgaccaatccttttgattttcaatcataactgtttctaatctaaacccaggcttactgtcaacgaacttccgctgaaccaccagctcgcctttcttatacttggcccgaatgtggatgaatcctttcggcaacgcttcaccaaacgttttctggtagggcgagccgcaatactcgaagcgtttcttctccagcacttgagccagatggatgtgaccactgattgtatagtcacgtgggtcaaccttgatatcgtgcttcgctttaagagggcgtccgttatcccccaacgcacccacagcttctacgtgacagaagttgaggcagggcttcttgtgtttaatgctctccttcgcagggtgtgctaagaagttcacaactataccatcaatctctacttgctcagggcgtagatagatatgcaacgatttgaggaagtcccactcacagaatgttttgataaggtccatgctggtattagacatatcagcccaatcatggttgccgccacagtaccatgtgtcgataacaccttcgtacttgaggaagaactggagcagcttgcgctttgtctcgtcgtccatcttgaacttgtcagtaatatccccaggaacaaagatgtgacgtatgccttgctcaacagcgtattgatagatgcggtcgatcgtttccagttgacggtcaacgtggtcgacagggaaatgattcgctagtccttcgaagtgccagtcagcagtcactaaggcttcaaggaaggccgctactttgttctttttcattagtgtaatccgcaggtttcaatgtctgctatttacagaaaaatgggcagcccggaggccacccatgtggtttatttctttctttctttctgcaaccatgggctgtattgcgagtctttcgactccagcaggctttcgagttcttcaacgttgatgttgtgtttcttggcagcagttgcgctcaggtagtgagtcttgtcagtggtctggtcaaagaaagtcataccgcctttcttgtccataggaccatacgccatagtcttcaaacgagatggtttgaagtcgtcgcccatgaacgctttcaggcctttcatgttcttggcgttctctttcttccgtgccgctttcagcacagcaatcatttcatcagcactaggtttcaccttagtgaaacggttcgcacgttgtgattcaagctctttggctttagcaggagtcttcgcaccagtcactgcacctttacgtttggcagcaatttttgcttcaactttctttacgccacgcttgacagcctctgcgtgacttggcttcttaccgctactggcaagaattttggcaacgtcaccgaacttaggcttaaaggtgcctttcttgcctttgatacgaacctggtcaacttgcgcagcgttaactgtgcgcagcgaacggcccggaccagtagtcagagtgatcgcagacgcaggaagcgcaagtgctagagaagacaatcctgctttacgcagagaagcggcagcagtacgcagcaactcttttgccgctttggcctcagcgcttgctttggctttcagagtcttgtacttggtgaccagctttgtcttagcagcaccctctgcacgggaagcctgactatgggctgtagtagaatcaattttcgctttaagcgcaccagcagcaagtttcttcgctttcttagccgaagacagagcagcagccacggtagctttgtgagacttgtcgatgacaagcgtagtagcaccgctgacctgagcaaaaatatgcgcaggtgttttagcggccgattcagaaacgatattgctaccgtcgagttttaaacgaatgagtgccatggtatgcctctaatgaatgagtatgctgtgactaaaaaattagcaactaccttcttttgatgtggtcttgatacgcattaaatcgtagccaatcattccacaaataagtcacaggtttagagtttctcagtgcgtagtcgatacagttctgtgtaccagacggtgcaccgcagcagagtgcaactagacggtcagtgttatctaccatgaagtgattgcgcttgttcaacgcaaacccagcttgaccgtccatgtgaacccaatcttctttcgaagtaacaatatggacttcgtggctcttgttcaacagaccgtcaagttcaaatacactcgatatcttccacagtttgttaaagccaggaaaaggaagacaggacacgactctgtgtccttgctcaatagcagcggtggcgatagccatgtcaaaccctagagcgcagcccacccatatttcggtgtctgtctcaaggcgcagcaatcgtctatgagcaaaagtatagaggcgacgttttgcctcagggctaaagccacctagatactgtgggcgatgaccggtaaaggatagtttctccatgcagtatatttacagatactacaggttagtgatgaagcctgcgttgaaggcgaaacttggtttagttccaggtactagaggactattagattgacctgaaactagaatctcattggcaacaaacttgatcaacataccatccataggacttgtgatcgcatcagtcacagtaggagtttcatccacacctgtctgagcaatatagcagttaacttctgcatcacgttgtacccactggccaccataaccagtaccagtatgtccaccaggtacacctgtgatatatgtatcgacaccgttcagggatatgtcggcagttggtctagtatagataaaagaaccctcagatccagtaaggttcgaatacacggacaagacttgagccgcagttccgcgcacaatagtcatattagaaaaactattgccattgctattgtatgcgactttcataccgaactcagggaatgttactggtatagtgccactacctacctgcaatgcttttggtacaatcgaacaaaagcctggagtatagggagttgcagtcggactatttgcgccagaacatagattagccgcgccagtagttggagcatcaatcttcgatgcaaatgtagagccgcctctgtatttaaagttggtgcagtaatatctgttgttcttacggccggaaactccattaacgataccttttcctacaagacccctagcttgtgtagctacagctttcagtgttgtcctatctacaatgctgtcaatatcaacaccatcagctctatcgaacagaaagatttcagggaagatatccgtcacagcaagatgatttgcagttgagataaattgcataagatattccttattagtcaggtcagggcctgcgtgaaacgcaagctcactgaactttggtgggagcacatccatgtgctatgtaagtattatgctactacttcgagatcgtgatcacctgagttccaaatgagttcacgaatgttgcgtggcataatgatgcagccactcgatgcagtgccaggagctttgatgctatcgccatgaatctggaaagacgagcgactgaacatcacgttgtctttgttcggatcgagaggcatagcatacggacctgtcttagcacttgtacgaggcgaagtgataacgtacttacctacaggtagaggacctacgccaacaagattctgatcagcgtgtttattcttgtgctcacctttaccagcatagccagtagctacgagcttacctgtcttgtcatacatacgacctgttgattgttcatatttccacatgagtattgcctctgcgttggataaaaacaaaagggcctacacctctcgatgcaagcccctttcttataaaatgattgtcacgaactcgttgcgattcttcttagggttaaaccatacttcatctatgatctttcccataccgaagttgatcatgcacacagtgcgcctactgactaactgccaatgctttttgtgatcaaacatcactggtccttaatcattttgactcgggtatgatcgaaaatgccgaatgtaggcacgtcatggttttgaccttcattgcctttgattgagtcgtaaccagcaaggttcagtatcttactgatctcggtgtactcgtcccaccacatgtagacgcgtttgtgcttactggcgggaatgagtttgttcaacctatctaggcgtgatactaaggtcagtgcttcgtcgcggccaacacgcttatcctgaaacgcttccatgataagtttcttaacccgactatagatctcagcgaacttgacctctgtccagagagaacgaaagttcaggctggcatagcgtccagggtccgcgtgaaatttgtagaggcgcccgtcctcagcatacaattcagcatacgcacgatcaggagttacccacgtcatgtgttgcttcttcgcatgatcgtcggaccagtcttctgctagtccgcgatagtagattgagggcgacgacagactaacgaatatctgcattagcgcgcacgaatagcatcgtcacgttcacgctcggccattttcattttctgcttagccgtctcaagacgcttaccagtagcaccatcacgaatgatgttatcgtacttggttacctgcttgtccagtcgggtgatagctcgctcacgcgctgccggagtcatttcgctatagtcaacgccatcaagggcagcggcacgttttgctttcagctctttagctttggctggagtgcgagccccggtaactgcacctttacgtttagtcgcagcaacaggcttcggcttatcgctcggcttagcgcctggcgtagattttttagcagcagcggaggcaccgatcttatcgaacttatcacctgttgcgaaacgaggtttgagtaacgatggactgcgattagcgccgctcgctttcacccaaaagctatcagccttagctttaccaatcttagacagtgtatagtcaggctgcgtcgaagtgatgtaagacggacggataggtgtggacaaaactttcaagccagctttagcaagagaggcaacagcagatgcagccagcttcttagcggcagtaacatcttttttgatcttggcattgttggccttgatcttagcactgataggagctttcttttctgagtctcgcgttgacttcaacttgagtttcaacttcgcagtagtctgaccaagtttagccgcagccacacctaacgtcttcgcctgcttcaaggaagcagcagccttagcgacaacaggcttgtacttagagttgattacgatcatcggaccgttaggggattgaacgatatgatacgacgatttctttgtagcagactctgaggacaatgtctgagccacattaagtttgattttcattttagtccttacaccagcgctcggcctgggatatcgaagtttttaccagcggaataatcacccaatgcgcgatacagtgaatcacgtaacatttgctcgatgatatcggagttatgcgcagatgcgtctttgaaggcaacctcaatcgaatcagttctcggattcactactgcgtatcgcagaggacagatcgtttgtgcttcacaccaggcgtcgattcgcggctgcaagtcaggcgtaatgggaatgcggaaatcagcgagagcaaagatcacgctttgaattggtggtggtgaggactgcgacatgtacttgccgttaggactcaggcgttccatagcagtcgaggcttcaaagatcgattggtaaccttcaccgattgtggtaatgttactgagcttgaagctatgcgtcgtcagtcctttgcgaatgagtttggcgactttcagatcgtagtcacctgaatcatcttgcgcaaaacagacgaaagcgtagaaggaaaatccagagtcttcgcgcagcagacgatggtccagcacacggaaccccacgacactttgcagcgcctgtgaggtgatctgaattcccttagatagagagacaaagatttgcattaacgcatcgctttaagtgctttcttagcgtcggccagagtagagtaaaactcttggtcatcgttaatctcaggctcaatctggaagccgacttcgagaatagcgaagcctgcgtcttcgtcttcgtctgcaacaacaacaccgaaacgtgcagtgctgttcatgatgttgatgaaacggaagtcaagaatatcgttcgcgctaccgatatcagacggcataccgtcagcagtaagcagggcgaacaggcctttcttgtcgatgcttttgaagaaagtagtagcagccgcagacgaggtagacttaacggtttcttccagattcagtttgataagactcatggttagtttactccaacttgtttggtgatggtgataacacgctggtaccagccgtaaatgttatcttcctgggtttcgtctgccttagcaatgttcttcaacttcgcaatacggcatccattgtaggcgtaagccagaactttgatatcgcgcactttgcagtaagctgtcagtgctgcaatagtcttcggaccaatattcgcagcaggtgcaaagtctggatagagtttaccgcgctggttcaggatgttcaactggtcttgcagttctgcaattgcagctggtggtcctgagttaactgcatagtcaaatacccacagagccagctcttggctgaacttcgcaagttcatcacacttgcagaaatcccaaaagttagcgctatagatagcatatgcaatttcatacggaagattctgcatatcgcctttatatccatacgcacgagcattcttctcggtgacgccccaacgagttgggccaccacgatctgccgcacgattcgtgtacttctcgccaccttcacggtcaatgacctcagcgatggctttctttctgaatgtcagagcgtccataatgattcctcttggtcgacgtatcaaaattagcgtcagacagacaactttgaagatttgaaccgcattctagggcgtgtaccaggcactgcatcaaacggagtaaaatcagtgctgtcaaacttaacaaagcctctgaactcattcagataacaaaacgctctatccagatgtactgtttcatccaatcccgtttgcgtttgataaagaagaccatcgcctgtagtctgcgtcaatgtaggcgtgccgctggagctacctgttacacttgttgatatagcgacttgcagcaactggaagggcaaaccaactgaggagtatgagggtttaacttctacgaaacggcaggcagggactcctgtgtactgtgttgctattccatttagttgaatgcctccctcatgaacatatcttatacctatctgaggagatccagattgaccataaggacagtttgagtcggacagacgcacaggaggaaacacaagagtaccttgtccttcttgggtaagggagatcgaaccttcacctatatgcagagttgtcgccgaatcaagaccaagagcataggactgctcctcggcaatggaactaattccagacagagttccgtaccctgtctgcttaactatctcagtagttttctcaatcagagaagatcgtggttgggtgtacttcaaattgggaagatagtatttgttgtcctttctacctcgtacaggattgagaaagccattgaaggccaacaccgctctagccttacgtgcgacagcattagcagtagtaaagtctgtcaggtcgatggtctgattctcggagctatcatacagaaacacgttcgggttctgggcggacgacccagccaacccgaaaaaagaatgaatatattgcatggactgtgcctcgtcaatgaagggaatgttctacgcgcttgcctaaaaattagctccaagatcgacaaaaggggccgaagccccttagaatatccaacgcgttgaccaagcgatcaatcctgatataataccgatgtgcgacagatacccatactgcaacacatagcctcttacatagtgcttcatgccgccctcatacgcaccatcatacaaggcagagatcatcgtgaacgacatgacgtatgtgaatacatgccacgttgtcatttccatcacttcgttacaaaacactatcaggaatagtgcgatgctcatgatgtacaatgtgcgtttagtctcggttagattaataccaagcacaacagggcgcatcacgaaggacgcgaatatcgaaaccagcattagcgtttcatagtcggctgacatgctgcgtccacctgatcaggagtgatatgtgctttattgcgcaggtcgagtgccagttgagccttacgccctatgcgggcatacgactcaagatcatcatcggagtaaccactcatgctttcgcgtacatgagacagctcggccatttggcgtggactcagttcgttcgaacgcgcataggcagtcgcatgatcaatgttacctacattaaggcctgcacaacgattccagataggctcggcactagggtccgtctgcaccatcaacgtaccgtgacgatcaacgtcatgaatgttacgactcatatcaaactccctggttagaaacgtaggtgtcggtgatgttagcagtcttctccacgttaccgcgaatataaccaatctcaaacacctgtacgttatgcttgaccacagcctcacctactgtctcacatgcaccgctatgcagatcaaggaatgcctgacacaaacgttctgctacaggcttcgcaagaatcttcatcagcgtatgtctctggacggcagacagcttgatgggcatcgcatcgatctcacgctcaatcgactttcgtccaccattgaatatccacttacagatagtggcagtcagtggcttctggtgcgtcttagatggcagcgtatagatgtatgtcattaagctgtagaacaaacttccgtcgatagcacgacgcttgaggtcatcaaggtattgacctacaggctgcaacttaccacgctgcggaaccatgtcatccagtttaaaatcaacatcaagaccgaaacgcttcaacgattcagagtggccgaatacatagacgatgtgctgcggcatatctcggattgctacagcattacgcgaatactctttcgcaccaacaacgaacaggtgcttacggtatttctttgaagggtcaatcgtaccaccaagcggaacaaacgtcacacgatcggcttgacctttcttcttcaaccaacccatgacttgctctgggctttggcgtgtcaccgcgattacaggcatcattactccacagtgttgagtgctttagccgtgtactcacgcagagtacgttcgatatcttccgcaacatcaggatgacagatcaactgatatcccctgataaatacgcgttgggaagggcgcatcactttgcgatgggaaggccagataccaaagaacttgtgcataggagttttgtagtacgtctccttatgctcgtccatgcaattgtggttggagactacatcatacttggcataaatgtctacgctctttttgatgtagttgaccgatacaggcatgctgtgcttttcatgatcgcgattgagctgaccaaagatcatcatatcaccttacgagacaggctggacgttccaccttgtttggtcactgtccattgattattagagaagtgctctacgtcattcggagttatccaatagatgttcgggataatctgtttgagtataggcaggaagttttcaatgatgtgctcactcactgcggggctgcaactgttatcaggctcgtcgaggatgataaagttcgtgcgtcgattagcaggaatgaacggcatgatcgcaacagcaaacagcaagcggaagcagttagtctctgcaccactcatgataccaatgtccgtagtcttcttagaagtcatacgggtcaccaacgcaactacaccttgcttgctggtggatagagtgaagtgcataggctctgggaacacgaggctgctgtattcgttcagcttattttcgatctgcttcaatcggctttcaacggctttcagtttgagagcgttgttgctgtacgctttatagagaacttcgaataccttgcgcttatcgatcaggggctggagcttggagagtttgctgcgaagttcccgcagtgtttcctcatagtgctcatgctcctgaatacgcatctggatgccttgagccttgcgttctttcttgtcgatatcgttacgaagttgttctgacttagcctcaatctttttgtaacgaccatcgagaatataaaacgggtcttctggttcacctacggccttcattgcagaagtcaggtctttcagaatctcaagatccttgatgcgattcttgattgtcttacgagccttcttcggctgcttaatcgctttaggtttcttgagcgctgctttacgtgcttgcagcttctccaacttcttcgcctgttcgaattgttcttcgatagcgtcaagctgtttgcccagcttcttgatttgtttctcaagggcttcacggtcgtgcttaggcttcttcaccttgtcgtcttgcaacgcagtgagttcagcgttcagcttatgatagtcgatagcctcaatacactcgtcaatgatcgcctgtgctttggttgcagcgcgtgacatagctttcaggtcaacatcctgaccgcatgtcgggcaagagttaccgtcgtggtcgtgttcttcaaacgcacgatacgcctgaactattgctttggattctgcgcgggcatcctgtgcctcttcctgagttcgtttaggacttttgagcttagacagtcgcttggtgagctttgcgcaggcttctcgccagtcgtcgtactcttcctgttgttcatctaccttctccagtagttcctgtgcagcctcttcctctttaaccagcttgccatgcttcttgcgcagctttttgttatctaggtctgcaacgtcaccaagtgctttgatacgcttcttaacgtcagcgagttcctgctcgtactcatccagcgcttcaacgtagtcatcatacttgtcgtgatcaatcaattgaccacgcaggtcattcagttcgcctttgagatcggttgtctcaatgccgagagtgtccagctggtgtttcagcttctcgtacttacgcgcattgctacgtgcggaactaagctccagcagttcttcgttcaggcgattacgccgtgctttcatcttatccagatgttcgatgatagcttttagcgtattcttttcttcggcgtgaatggacagcgcgttctgcttacgctgtgtcacgtcgagcatgtcggccagacctttcgattctgtctcggcatcttttgccaagtccagtttcttcttcaacgccatacgaatgttatcaaagatatcgaggttgaacagacgtgtcaggtataccagacgctccgacggagttgcacgttggaacggatgttgaatctgcgattggatgtagcaatagctgtagaactcttcctttgacagaggccagtgcttctgtacccaaccacgcgcaacgtcctgacgaccaaccttctggtcttcgccgttgtagtatacttggtacttcgtggctgtctgcacgatacgcacaacaccaccaagaggtgagttccacgacaggtcaatcgaactacctttgccgagcatgttccccttgtctttcttcttcattgcaagggggtcagcttcatacagcaaggtaggtattgcagcgaacagcatacttttacctacgccgttcgtgttgtccttaacgtttggactatcgaggttctttccgcagatagttgcgaagccctctttgtctaggccttcaatatcgagttccttgtacacgccaacgtcgcgcaagtgaatctctttcaggccgataccatgttgctgtactttctttttggccattagaaatactcgacggtttcttcctgcacaagacctttaccgtgagtctgctcaaacacttcgatctcgtcttgcgagtattcggtggaggactccgcgataacatcatacgaaacggattcgtcgcgcgtatcagacacgacaggtttgatgatacgccacagaggcagtgcgattgggtcacgcttaatcatagacattagtggaataccgccgttggttcgacccagagttcagggttgttgtacttcgcacggagttcctccatctgatcatcagtcagaggacggtcggagatgtgaatgcactgaggaactttttcctcttggcctgtaacaggatgaatgtcacggtcattgcgcataactgcccagcgtttggttacgttgatgtggatggtgcgttccatagtgaagacctatgtatagtgtatgaatgatactcgctatttacagtttttaaggctatagacaaaaagaagggccaccgttaggcagcccctgcgaacactttacgcaccccattatccagatagtggtctgcgtagaaaggtccgttttcattttcaataccaatacgacggcagagctgacgacgcaagcgcttaggccacaccatctcgtcatccagcagatgaataaccgcaggtagcgcttcgagttgagtcattgtcagatcacgaatcttatcgtcaatcttacagagttccgcgtagtcttgttcaggtgtgggcacaggacgtttgggcttagataggtctacggtgagttccatcaatacctccgaggcttcttgattttcttaatcgtggacttaggacgtttgattgccctcagtgctttacgtgcttcgacaatcttcttggacaactcagagcgttgagccttaacagcatcagtgtcctgctcggtgcctttaagtttctcaaggcgattccactctttgaccaaacgatcaacgacgttagcacgagacacacgttgctggttaacgcgcacaatgtcttgttgcttcttcacggagtcacgagtgttattcacttcgtcccgcgcagacttcacacctttagtatcaccttcggactgtttgtcgttcagcttctttcgtgcaacttgcgaacgtcgctgggcacccttaagatcatctttcgagttctcaaggctaaccttcgtatcttcaagtgggctggtacgcgcactcaaactgataagtattttcatactgacctcaaatagaaaagggtgaccctaaggccaccctgtgtagaatggcgcgctatgcacccgactggttaggtctactacgattatttaacctcgcagtagtgagcgaggagatagggatcacctcctcatgcggattgaagttgaatgatttcttcgtcttcgatatccgcgccagaccacgaacgaatcacggatgcgttaccacgattgcctgtcagcatcgacttaactgctggacgtgcttcgcgttctgcatagtggtcgacaagagctttgtcgttgacgaaccacataatggagtgaccacccttagggcagatcaggaattgggctggacgttgtggtacgttcaacgtcatatagaagtcgccagcgccttcgggactcatcattggcatcggcttcatgatctgttggaagtcttttgcatctttaagacgcgtatcacccaacaaccaaatagcaccttcttcaccttcacgcacggcagacaatgtacctttacgcgtagtgatagatccgaatacatcttgatcgaatcgagccagcccaaagataagtgatgcgagtttcttcaaatcaggagtggtgcatggactgtcaattttagccatgccctcagacccgattgtaatcttcgataacgaaacaaagattttcatattgtcttccagagctgtatgattaattgtgttataaaattagtgtttgatcagacaattctgaaacaaaaatgggcggcacaaaggccacccgtttttcacttatttacttcttcttctttttctttttcgctggcttgtcgtcttcgtcgtcttcgcccatcttgactgacagcttaccttcgtagatatccgccatgagagtaagcactttggattccagcataatgtctgctggtacggacgttgagttgaaggctacttcggcatcagcgagtgcagattgcagatagaccatgctgaccagattaactttgatattgtctttcttggtcatgttcatgaacatcttgaggccagcagactgccacttattcgtttcggcgtaatgacctaacacgccgtgaataatccaacgagctttcgcaacgattgcacgtgggttgttcgcttcacgcaggaactggattacggcaatcaggtccatagacagatacgcaccaatcatctggacagctttcgcttccatgtcgatttctggatctgctgctgcgagttcggcaacgaggttcttatcgaactcctcaccacctttgaccgacgcatagatgttctgcaacatcgtgattgcaccacgcatctggccaccagcatactcagctacctgatgaagtgccgacgtagccttatcgagagctttgtctttcttcggcagtatggagagttgctcgctaatctcgaccaaacgcttatgaataacatcggtcgggataggtctgataggcagttgcgtcatgcgactgatcatcgtgttcttcatcttctcagggttcgttgttacgaagatgaatacaacgtgagctggtggttgctcggtgattttcaacagcttggattctgctgcgctggacattaagtgggattcatcgaagatgaacacacggcgtttgaacataggactcagaggtgcgctgtccacaatcttctggctgccgtccactttacctgcatcgccacccatgtcgaactcttgctcgtcagggtgtgcaccacggtcgtgcatctcacacgaacgacacttaccgcaggcgctgaatgtttcgcagttgatatacttcgccaccagacgagcgaacgttgtcttaccagaaccgagatgacctgtgatgatcatcgttgatggaactgtcttcgacttctgccagcctttcatgatcttaacgatgtggtcttgtcccacatagtcttcgatacgcttcggtctaaactgatcagcaaagttaatcgtggtcagttcaacagactcggaagaatcgcctttctttttcttcgacggcttaccatcgtcaaagctacgcgacttcttctttttcttttcttctttagccattttcaattcgcccttagttctaatgcgttacaccagttatttacagtatttagacaaaaagaaaggaccacatccaaaacggagggtcctcttacgtgtagcaataaagtttggaatgataacgcatcggcagtgggcgctgacgattaggcaaagctcaactcccaacgtggaaccacgcggaagaattgcttaaagtgggacggtgggttattcttgattgattcaagtttcttttccactacgtcataatcttttatgccactctcgactgtgtgagtggtgaacgtaccgtcagcctgaatcaagtcggcgacaacacggtagcttggttttctcagcatctattctcctgaaaacgaaattcttattgctctgaattatgtttacagattactggagtagtcataaaagaataaagtaagacaaatcttaaactccaatagggactcgttagaaatcctattggagttcaccctcagttgcgatgacggtcgcccgaaggtgttctccccgtgtcttttaaatgcaccgacacggtagcgcttgcggtcttacgctcttgtgtgtgcagcgcgtcggcagcaggtagcatttacgcgcagcaaagagcagccgctttcggccattagcgataacgcggtgttacgcttaacggcctgtatgactctggccgagtctgtacaaaaaaagagttcggcctatccccaattcggcaaaaagaacaggccgaactaaacagtcaacacacactccatgtgcgctgttttgtacagttacaaattagaaacatgttgaaataatcagacaattcttagttgagcatcggaagaagattttctaagaaatgttggcgatcaaatgaactaattcggtgaggatgtttgatgtgcaggttccacgccttgtcaaacagcaacacgttctttggcaggactacgttaacgccaacacgagtgaaggaatcacgaacggccgtaactggattgtcgtcaacaagaatccaagtaccttcaccgtaagtcgcattcagaaaagcaaccttgtcaggatactcaacgctgtttaagcagtgaacatgatcgaacaatgacaggtgcttctccagagacttgcgcgtgtagcgttcacctttttcatggtaaccgcgatgcgtacagatgcccgcactgaatccatcacgcaccaacattgcaactgtctggatgaagtacggacgcatgttcgcattcaacatgaacgtaccgtcggcaagcatgtcaatgaaaggctgcttaccgttctcaggcgtgatgaaggtgtcagtgcctgggtagattccgtaattcataagatgacacagcatgaagttatgcgtatcaaatgccgtgtcgtccatgtcgaagaaaatatgtttgatcattaatgcctcgtgctcttaactaccagaggaatatcgttaatgaatgccagagtcagcaactcgctgttaaagcgcaggcgcatttcatcggcattcgtaacaagaataatatcagacagaggatcaaccttgaagattggaacctcaataagtacggcggtgtcctcggcttcgtcaccatcaacaatgaagtaaccaccgtacatcaaaacagtatcaccagaatcgacgagatgaccaacgattgcgtcctctccgtccatgatcatgtgcagaggctgatcgatgtagtagccgctatcatcgtctgccccgaactcaaagtggaaatcatcatcgctcatggttaggccctcaaatcaaccaatatcgaagcactcaggtctcggagcatatctctcccaagagaagtgtacatcgtctgcgctataactattcgttcaaggaaaagacgagaactattaacgtcatgtcctgtcttctgctgaacgaagtcgatgattgatgacgcaggctgaatgaggaatgtgagtatctcggcgtcgtgaagcacgttgcccatagccgtcacaggacgcatctctgtttcctgatcgagaatgtatgagatgactcggtcttcattgcctatgttagggaatatcttaaagaacttgcgtaccgacttgactgtcgccatgaagtcatagtttgggttggtgggcatacgcaagaagagggaggcgagcaacaagtttatttctaactgtggaccttgttcaatgttcaacattgcatgtgaagtcagcacaacattcaacgagaagtcacgagtgtagagcgggtgagaggtcgctgtctggtcaaaatagtcaagggcggaacgcaacccctgacgtattaacaggtgctctgctttaatgcgagtcaggcgatgcactactcagcaccgcgaatctctttcaggctattcttgatcgctttgcgtagcgtcttacctacgtcgatgccgtcgatgtgacgagcaaacacgttggcgaatagcgtggtcgggtttttcataatcgccttgtcgagatcagggcgaccctctgcaatctgcaactcgcccggccagagttctgcaactgccgcgctgtcattagcagcaatcagttcaagctcacggacggagatagagttctgtcgggcaatcgtacggaagattatgtcaacgaacggcagcatgtcctcgctaacaacgttcttcacgtccttagcatcaccagcacgttggaaatcttccagcaggctttcgagatgtgactgcgtgatcttctggacgttacgcagtttcttgaacagcatcatccagcggaccttgcgcttggaactcagcaggtgagtccacacagattcaccgagcgcaatcatcagacgattgtacacgtcaacgctcaggctatcacgatcaacaaagacagtcatctcgtcatgccattcgtccttacggaacttagaacggaacgcatgagtcttcgaccctgactgctggacgaagttgatttgtttgcatcggcgaacagcttccgcaagatgatatttctcaatcaccttaggaagtttcttaacgcccatacgacacgcttttgctacttcggcctcacgaccgaaaagagacagacggggcaagccaccgtagacaggcattgaagcatacggtctgactgtcacaccgcatacggacatacctggctcagggtcaggacctaatacgcagagaacatcacccgccttaggactgaacttgattgtctcagggtctggcgtactaagcgtgttggccaatataccaacagtgttcccagtagccagtaccaaatggtttttgttaccctgccttacaacaaggtaatccttttcactgtgtttcataacgacctttattgaagttgatcagcgatatcgaacgtatggacttcggctgtgtaaccttgacggaacatacgaccttccgaacggccagtagcttgctcaaacgaaggaggagaccacgaagttgaggcttcgattgagataagaacttgctcgtcccacatatcaccgtcttcaagatagtcggcaatcatgttaagagcagcaggacgatcgaggcccagatgcgcaagctcggcgataatgagtcgcggtgcggtgcggtctttcatttcgtcgagttcatattgcagttcagcaagcgttgtgactttgtgagagtccgcacctgtcatgccagcatagtcatctggtccgaaataagcaatatcaaagtcagggatatcggtttgactaataaagaaatgaggtgcgtccaccaaaattgaaggtgaggcgcacatctggagaaaacccatataaggatgtttaatctcatgggcttctaccgaacaggacttcccagcaaggtcttgcttaatgctgtgtgcgagattattcatggtaacctcatttctcaggagtaggggtaaaggggctgtgaacaaacaggtttgtcttattgacatacaggaacccgaatgcgttttgtttgtaactttgacgcgcggccgattgcttacgtttagcttcggctcgttgtgcgtcctgctcgtcaaagatacctcgacgatggaacttaaaatcagggtgtactgaaatatctttgacgatagcagtcatacgttattccttatacaggcttaaggtttaggtgatgccacggaaaatctgctttctccaccagctcattggcggtacccatctccgagaacttgtcgaatacatgaccgtacatcgcggcgaactcagcgttctccaactctgcctgccagtcttcgtcttcggtaacatgtttcctccacacttcgtcgtgcaacttcataaatgtatcggaacgtttcgggtaaagcaaagagaataggtcacgcgcaaaacaaacgcgatatgtacctttatctttaagggcctgcaaagaagtcagtggatgcgctgcgtcaaaagccgcaagcacttctccatactgtttgaatagacgcttattctttacagcaatcaattctaatgggcagtctttgattagtcgcatcacaattttacgtgaacgcaactctggccactcagttggaggcaacacggcactttgagataacttgaactcaagccgaaacagaatttcaataggactcattctgcatcctctaaaaatgtaaggtgatcggagaattgcttcttaaggaataatgcaccgtcagaatgaaccgaatcaccgaccgtttccattaaagcaccatcatgctccagagaataaacgtgtttcacctgtgtgtcatctacgataagacggaacaggcactcagactctatgccgctgaaaatgtgattgagcacctttcgtctgcgacgttctgatattcttgctttcttgagatcgtacttgacgcccgatttgcacgttaaagttttttcgccatgcttcgtctcacggaccgagccaatataaatgtcggtcaactctcttagggccacgctcaaaggtatcgcgttgttattccatttgcgcacaaaatcaaatactttcaggaacggcatatgatgcgttagttcttggaagactcgacttttatacgacggaaccaattggcccatagaaaagagtgtggcataaaaacaaatcttcgtcgcagctttcggtagatcatttcttttcgctatatcgtcaacggaggtcacatcgtccataaacgaacaatgaatcccgtgtgcttcgagttcacgcaacagaatgtttagctggctgctggacatatcccagttggtgcctatagcactgcactcctgtttgagctccgcagggaatgactggaagccaccccccttctcaaataaacgaccaccaatcttagccaagcggtatacaggcatatagcgaatagtcagtggatgctcacgcacaatctgcacaggcccgctcaggatagattgaagactggacaaaacatgatggtattgaccctgtgagcgttgtgacttcatatacgacttatgctcaaggtacgccagaattggatcgattaaaatctcattcggggccagcttattaagcacggacgtatagagtttcttcgcttcacgatccctgttagaacatagagcggtgagatcgtgcctaggccatttgaacggcttcttcacggcttcatcgagcatgtccttaattgtctgaccgtactgctcattaaccagacgcaaggggctatataaacgagttaccgacaacaagtctttgcttgtctgagggttctcagggtacatgcaacccagaaccccaggactaatacggaagcggcggcatatacccgacttacctttcttgaacaaatgatttttgtattcgagaacattttcgagcaaccaatcaagggctctgctaaaatgttggtctgttttcttaaagttaggcgacacaggaccgcccctttgagattttaccccgaacaccataggcaacactttacgtccgaacgttgaagggaaaggcgtccaaacctccccgaacttagcgttacgctgtttgctctttgttggcgtatagattgacaattgcagaatatgccagaagaacagatttatctggcgtctatactctggttcgagttttcgcggcccgtcgtacggacaggcataaactacgtgggtttgtacccactgtatcggaaacatctcttgatacgtgggattcttgactaaatacggagaagccattgcatactccagaaaaagtgcttcttgctcttgttttttacagttttaggtgctttcgaccattttcttttgctttaggtacaaaacagagtcacataacgacacaatcacctccctcaccatctagattcctgccacccaggagccacgccaagcaacccgcttaccgcgacagcttactaatagcttcgctggacacaagctagctgggatagctggaatggctggaaggacgggctacaatcgctagggacaatagggctttaatgggtatccgagataagaaatactcacctacgtagatcgctgtatgaagctctctgcgtgtagggaatacgtcgtaggatagccaaacgctaaaagtcttaggctcaatttgcgtcagaaataccatgtaacttttttcgaaaaactagcactcaactgtagaatcgagatgaattttatgaaaagcagaggaaaatccgagaaaaatcaaggactttccccgctatcatcactttttctgcgaaacgcgcttcccgagcttaactccgatttgagtcaggatgcgtttcactgtatcgccgtcgtgttcttccatagcggcacccaaacgctcgccctgctcacgcgatagctcaggcataatcattttgagcatctgcgaacgctgttttgctgctttagacttgccttttgagacagacacgccttcattagcagataacgcactgctaatagccttttgcacacgacggtcgccgaagatatcgccgaagatatcgccgaacaggtccttgaacgacattcctccgctcatgatatcatccttagtgaagcgaacaggctgccccagcgcattcgtcttcgtgctgtgcgtcgattcaacttcattcgttgtacgcccgccagcacggaagttctcgtcaggacgtgacgctttgccctctgcgcccggctttgtgttgccgttacgcaaatctgggtcaccctcaacagccttgtccgggtcgaacatgtcgtccgccgtttcgctctggtttggatcgaaaggaatcttacctgttatcttattcgggtccggccagctatctggaatatcagacgccggttgaggcttgttcgtcatatcgttcacatcgccgctcaggctgatcttaatgcgagtcatggttgctcctatcgaattttattgcctttgaaaatgttgtacgcaatctctttgcgctgaacaggacgcgtggtgcatacccattcccattgttcgttctttgcggtacgcttcttaggtgcttccataactttcagcacataattcttgaacggcaggacgagaatatcctccggctcaatagcaccgctacgcgcaggaaggactactgtaatgttaccaacagtcagttcctgatcgtagttcaacacgtttgcttcttcgctgatgttgcctttaacggcagacacacccaaatcgaagataatcgtagcgtgggtgaatgctgcaacgtccttgatgcggacaatcacatgcttgcctcgccacggttccagattggctgctgtcagctcttgctcgacgccattgaccaccagcacaggacgagggaatgcaggcagcatctgatcgtttagacgtaccgaataagtcgcctgcgtaaagtattttggaataagctgatcgaaatcaacgtgtccgtctttacgcacctgcctgaaagttgcagggctggtggactgatcgagcgtgtatgctgtcagcacttttgcgtgatggtgagtcataacgttgtatacgaagcctgtgctgataaagccgggcacaacgccttgacggaagcagataccgcagttcacaacgttacctgcatcccatccgtttgaaacttcttcgtcaccgttacccataaggtcggcagcgtccattactgcattcatgccatcgtcgatatcatcaagggatactgtctggcgcccaccgccgaacataccttttgacaccgtgcctagtttaactccagcgtccattgcagacgattcgcggccgagcgacttcatgccgcccacctgctcgtcgaatatatcgttgtccactttgttgcagctacaggtcagacccatcttcgctttcttgaagatgattacatcggtggcatcaacctgcaacgcctgttcaactttcgactgcacaaccttctgaactgagtcgaggcgttgctggacacggtccgtttcgtaggtcttatggcggtcatatgaatttcgagggcgtcctcgttcaatccagctcataatcgttctcctctgtgtgctttaaattagtgtacaaaatttaggaccttcaccctagtaaatacttatttagagtacgttaaaacacggagccttttatgcgtattctttcaggcgacccgggcaaagtgaacttcgcgttggctgttcaggagtttaaagacagacgcatcactgtgcttgggacgaggatgtttaagaaacccatccaaaatcttcatctggacatgcggcagcccaccaaagagttcctcgctgaactcgaagaaatgtggaagctatatggaccgttcgacgctatgtgtttcgaacgcttccagtcgcgtggtcttggcggtaacaccattgaagcaattagtctgatgcttggtgtcatatcgttcttcgcgctcaaaaagaaatgcccgcttgatttgattacggctagccagtggaagaacgcattcaaccgcagcatggtgctcaaggactattacgagcttcacaatctcaagtccaagaaaagccgcaaagctattcacgaatttgatgcgtgtctcattggcgcgtataccttctaccgacattcagggattaaaccatttactggcttctctcgcatcattgatgtgtatgtgcctaaattcctggcgtcacctgtactgtgagacaaacatggaacaaattgaactgttacgcgtagtgaaagagatcctcagcgaatatggcaaagttgagtttctgtcgcaaggtcatgttggcgtgaacaccgagcatcgtgcgacctatgaaacgttaatcactgtgacctcggatagcgagacagctttccccgaagcagatttccgcgctaagattgcggcgcagattgacgagtatcgtgtggtgggattcaaacgcacctacaacgagcagaccagagagtttgtgctgcaactgaccgaccctatattcacctatcgtgacccattggcgtgtccagcaaacggtaaaactatgtactcggtttccgtaggtttcccgttcgtgtccaccaattaatctgtaaatatccttacttggttaacgtgcgtgtgggatattgaaaatggcgaagttgaagaaagaaccagcggtcaaagtcaagaagaaaaaggctttgacgaccaaaacaaagaaagaaaaagcgaaagcgattcctatcagtgttgtgcaggacacacgtcctatcaccacttgtcctgaaatggaagagaagccgcagcctttcctgttccgtggccagtgtccaattgtaacctgccagtattgcacacgcgaaacgccgacaggctgcatggcgcttgaccgcaaagagtcggcagatcgttcaatctccaacaaggagatactctattataagaaaggtctcttccctgaacttaaagagatggatcagaaaacgctggacaatacgattcgacgcgcacagaatcgtacccgtaatgctatctgtcttactatgtttattgccggcattgatgattctgactgcgatcgctctttcaaatatgtagagggtcgttccaaactcgtcgatcaggtccataactatctgattcaaacgttcaacgattaccgtccgtggatgctcgcatacctcgatgacgagaaacgttttagcgacatggttggcaaaataaccaactctgactttaatttagttaacgcattacgattgactcctcgcaagtatcaaacgttctgccagtcgctacaaaatcttaaacaatctggagactctcatgagtaactttatttctctcgatcagtatcgcgccattctaaagcgcaatatcctgaaagagcctcagatgcttgtcattaatcagacgcagcctctgggacaaatcttcttccaatgccctggcgataactttgcgatgaaagatatcatcgtgcctgcttcgaagaacgcaatcgatctgactcaacaagctccgctggaaaatctgctggcgtgtagccaactgaaagcgctgctgcaaacgcaacgtctggtactgctgaaccctgaagaaatgccaacgcctggcgaaggtattcaacaacctgagttggctacacctcctgttgctggtgcaatctctgttgacggcaagactatcccgaatgcaatcgtgatcgtcgagcagaacggcaacgtgtggaccggcgcttctaacggcagcggtgtgttcactgtggacgtgtctggccttgaagaaggtgtgttctctatcactgtaactgctgatggtttcgtacctgcgcgttataacttcactgccggtgcgcagcctctgcaaccaatgcctgtgcctaccgtacacgctgtctttaaagagacaactgtgtcgggaaccactgttgcgaatgctaatatcatcgtatcggtgcagagcaaagagtttacaggtcaggctgatggtcagggtgcgtttagcattaacgttgacccactgccgtttgacattattcacctgacgatcactgctgctggctatctggataacgttgtcaatcacatggttgactctgttcccggtctggcgcagattaacagcgcgcctttcctgtctactgcactggctggtaaagcaagtccagaagctgaaatcgaaatcaccatcactggccagtccaatcagttcgttactgctgctgcaaatggcgattggtctgctgttgttggtgcggttaaaggtgaagtctctattcgtgtgctggagaaagatggctacgacgaagcgactgctaccatgcagcctaccaaactgcctgctcctgtactggctgtcgataacgccgatagcatcggggagaatcaaacagcattcggcggtgcaatcacaggcctgagtgcagaagcaaatgacgtagctgtgactctgactgttcaggctggtctgtatgaaggtactgttgaccttcaatcaagccactggtctgtgactggtgttgatgcaaaagctggtgtgggttctgtaggtgttgttaacctgacgtcggccttctatgaagacgcatcgactcagttcaacattctggaagagtttgctcagcctacgctgcaacaggcgcaggatggtcaaactgctgtggtcggtgacactgtagcttccgctactgttaaggtcacgatgggcggtgagactaaaactgcttcttcaaatcctcagggcgcgttctctgttgatggcttcaccaacgttgttcctggttcagttcatatcgaactgtcccgcgcacaatacaaacctgctgcgttcgatgtaacactcgtcgtgcaggcgttgggccaattggaccacgagctggctgtcggtgatgacacagctactggccacgctacaccagggtctacggtaactctgactcagggtagcatttctggcgacgctgttgcggatgtttctactggcgaatttattatcagcctgtctggtccgcttgtcgcagacactcaggtagagctgaaagtagaacatgcgaactacgttgactacactgaaaccttagctgtttctaatccttaatcttacctaaggggcttcggccccttgttgaaatacaattcggagaattaccatgtcagataaagcaagcactaaggttcaacctatcacgttgaccgcatacaacgaaaagtatggcaatgacgttacagcaccaatgtatgtcgctaaccgcactgagcctcgcggcaacgtaatgttcagcgcacaggacgacatgggacagccagttccagttctggtgccggcaacattcatccctgtcgacctgacccagcaggccaccaaagagagcctgctgaaatctactcacctgcgccgtgcgttaaatcgtaaccagctggtaatcatcgacactgaaagcgcagagcactacctgcgtaccagtgctatggctaagtccgagatgaagaacctcaacagaatgggcagcgctatcgcagccgagctgggtgaagaaggcggtgacctggcgcagatcgatctgggcggtaacaatcgtcgtcacgttcaattcgaaggtggtactcagtattctgaaaaccaattcgtcaacgcattcattgttcgtgctgcggaagacagcgaagaatctgatgacaacctgcaacgtgaattcctgtctcgcggtattaacctgcctgcgtcagagctgcaaatcctgcgcaaacacgttactcgtccggcaatcgttgaactgatcgttcaggcgcttgacgacgcgtaatcgaaagctacagaccaaaaaaaaaatgggagaccccgaaaggagtctcccatttttgttacgttcgcttattcgttatggctttaggtctagcccatcccaatgtctttgcaggcatgatgcacttcttaccgtgaatatctttcagtgtcatgcgtacttctttgatcaagttcatcggagcgttgtccgggtccagcttaatcagcttaccatcttcgtcatactcacgaggaagtttaaagtgcttgaccggtactggagagttcttttcaaactccgctttgattttattacgcagcaacttcccgccgccgtcattgtctgtcattgtgtagacgacactaatccctaacatctcaagcgttctgcgtttcgtttctccgaactgctctgcaccgagtacagctaacgctggaattccgtaagacaataaagcaagtgcatcacgaggaccttcaacaagaacgatatatcgcaacttgtatttcttcaaacactctttgactagaggtagtgggaacaagcctttctcttttgcccaatcaccattcgagttcacatagctggtgccgttcatttgcttgcgcagatacgcagcgataccacctatatatttcgaaccatgcttacatgggaagaagcacacattcgtgccttgacgttgtgcgttcagtaatccacccgcagcttggacaagcgctccaggataaccacgccactcaacatcaaccggccactccatgtaactgtttctgccgagagctttcatcagcaaaccgacagacgggtacgtaccaatcttcgtgctgatttgctcatacgttttgaacaacgcactcaggctgtttgtgttcgcgtctttaagcgcccagcctttaatttcctgtagctttgcgtgtgccgctaatttgttccaaccacccttctctccacatccgaagcagtgaaagaagccgagaggtatctccataccaacagaagtgtaaataccacaactaggagtcttatcgctgtggaatggacagcacaccataacagtgtcaccgttgtatttcttgtcgcccggcaatttgcctatttcgtcaagtattatttgatgaacatcttctgccataccatcacctgtttgtttcgtaatttgagcatataagcatatttacagaaaaaggacaatagaatgggcaatccacatcgttacgtgcatacggcacaacgtcgttactacggcaaacactggattggcttttgcgatctgattcgcgtcgagcctcaaacttacggagcattcgacaagcaggacgatatgattggcctgtcgctcccacgcaattttgatgtagacgctgcaacaaagagtctgcgcttgatttacaccacgaatgacgagaacgtagaagtacgctgctacctgtttggtactcgctactataggttcgtattcttcgagcaaaccattgccgttagcgaggactcccatgagaacgttagcaaacataccagcgcgagctaatgacacgcgcaacttgtctcgcatcggtaaaatgattgacgctgcccttgacgtaaagaatcaagaaaagcgttggccgaaaaagcgagtcagtccatctatgttccctatctgccctattcaagaggcagccaaacttatttaccagaagcataacaactgcatgaccggtgagtcaggtacgttgctgaacatctttgcgaaagctgggaccgggatgcacgaatcattgcagaatgctctgggtcatagtggtcagatggttggtcactggaaatgtacgaacgataaatgcgttgagttcccaaagactaaaggtaagatggtcgatggtgagtacgtcaaaggcaaatacacgcgaactcgaagcacgaacaatcgttgtccgtcgtgcgataaacccatggcttacgcagaactcaaagtcctgtacaagtcactcaaggggtatgtcgatggcctgattgataatctggacggtacgtacagcctgatagatttgaaatcgactatggtgaccaaagctgctgacggatctttcttcgttaagtatcaccgcttccagattgcgacatacgcatacctgctgaaaaagcgttacggctataacatcgttgattacaccctggtctatgttccacgcgacaaccctaaaaagtttgtcgagaagacctttgtctttgacgaggctgagtctaagcgcgccaaagactttatgatggaacaaatacgcgcatgggatgctgcggtaaaatcggtacgcacaggcgacttgctgcccgctattaagcggaagccttgcaagagtgccgagtattattgggacgagttccatggatatgatacatgcccttttgttgactattgctttattcaatcacacatgattgacttcatgaagaagttagagcagcgaatcatggccaaccccgagctgacttatatggaaatcgtaagcacaggtcggaaaactcaacaacaaggtctgctaccggacaagcctaagaagtctggccgtccgaagcatatcgtaaaaacatttgagctatgagcatacaaagagattatgaacgttccctgcgccggcttaaggagtctgtctatcgcaaagagcaactcggttatgtagtcccgagatgcgttgatgttgttctctcgaaattgagatcgccagagcatgtagtatcgaggaaatatttggtcatgctgatgttgtttagtcagacgtgcgaacaactcggtaccgctcttgctctacgcgaacaacttgtggtcaagatggctatccttagtcgcaagcatccaacgccggacattcagcgtaaaattagacgcctcgaagaactggtaataagtcaggacagaaacatcgagagccatcgtctgcttctcgactatcgtgccagcgtgttgattgatatactcgacggcaaagaacctaattcacgttacacttgaggtacttatggaaatgtatgtaagcctgagtcaggacagtacggataagaaccgtagcaaggtcaccagccctgaatcaaacactggccgagtcgatgtgtcagaatacgcatctctggaaaagaaattgcgtctgacagatgaagccaaagacaaagagaagttagctcaaaaggctggtggcggggattctgtaaagggtaagaaaggcgcgaagaaaagtagcgcagaacccaaggatgacgacactgatacggacgaagaccctacattagatgatgaaggtgacgcagatgattcagatgactcttccgatacagatggagacgactccgatggagactctaaagctaagaagtcaggaaagaaatctgacaagtctggagcaaaagactcagcggacgcagaagaccctgacgcagacgaacccgaaagtgatgacggggatgcagatgttgaaggcgctgatgacgaggacctcgaataacgatcctgtcgatgtgcctaagactcatgacgcgatgattgatattctgatcgctattcgctacatgtgcaccaagcgtatgatcttccctgtcgtagtcgcggccatcgaacggcgtaacgactatctggtcatgaacaagctgaccttcaacatgaagcctggcaagttcctgtctgctgttcaggatagcaactgtgaagtgaacgtgtgttggcttatgcgagccttcacacgtaccgctctgcattttgacctgaaacctgtgattgctgatcgcagtggcgaatttcagccgctagttagccgttacttcactcaggatgatcctgacttcgcctatcgtcgtcattacgacattcgctacatgactgcacttactgatatccgtaagcctcgcatgtatctgcttaatggagttaattatggcgtacaagtcactcgccaagaaaccgaagaagtcgaaagctgcgaaagaagccgagactcggaacaaggcgcacaagcaagctcgccgtgggaagctcggtcaggctgttaagacactcagcgctgcctcgaagaaatcccgccgcatgacaaaaggtgagaaacgtgcaattcaattgcagccgttcaaacctcaagtcgtaccgcagcctcctaaaactcctttgatggagaaaggcctttcgttaactgcgctgatcaaatcaacgccacgtttgatgaaagagaacgctatggaatgttatgtcaatagcgttaagcgcggtaagacgaacaaaggtctgccgatgattatggcaaacgttcgtcacaaagatccactgcgtcctaataaaacagtgcgcattcacaagccgatgattatcggtctggatgacccgttcaagcctatatcaaaacaaaagcgtgtactggtcagttgtccctgcgagaacttcgtgttcatgtgggagtatgcgaacgccgaacacggtgctgcgcgaatcatttacggtaacggcgagccgccagacttcactaatccaggtcacgcgccaggtctgtgtaagcatctgatggctttagccgatcaagtcaaacgaaacggagattaatccgaatgttctttaacaaccctgctccgggagtaatcccaaactacccgattgttcactctatccatgagatgaatcgtcgtgttgcggaactcaacggcgaactgattgccgctggttgcaccgtcgttcagaactgtggcgacatgctgatcgaagtacctgcgggtgctgctgcaaaagttgacgatatcatccagcggcacgttgatatgttcaatggccctgttgtgagtaagcctgctcatttgcagattggaggcgaagatgcagaagcagaaatttaatcctgaaacgcatagcgtgtcgctgcacttcggacggcacattgttcatggccatgcgcaagaaagcgtgtttggtgatatcatgcagacgttgttgctgcgtgagatcagtcgcaccaccaaagaagttatggagcaaggtatcgaagttgctcctcctaccattgagtgtaaaacaactgatgcaagttcgatcctgagcgcactcaagcagtggcaggaaatcatcaatgctcaagaacctcagaaagagttcgagccatgctctatcccagactggatgcgtcctggtctgaaagagaagggaatgacagaggaggagattgataagatcttgatcactggcatagagccttcgtggggcgatagtcctggcgtcattttcaaaacagtcaccatctaatggggtgtgctggctgtggccgtcgtagctcgcgcattagttacaacggcagctctgctcctcagacagtaatcgaagaggacgatacgttaagcgctgcgcgtttgacacctcacggctgggtacgcacctgcgttaagtgtggtgctgtctccgagccttcatcttttgcagagaacatagagaaaccgtgtgactgcaaaacagacgagtgatcatgatgaacaatctcgttggtaccgccgtagctttagaccattgtcgcttctatgcggagaacatggtaaacattcaattcgagcaacctctggccgctattccgcctgaaccttcgtacaacgaaccgattaaccctcgcgttctgcactctctgattgacggcatccagactgcgttcgacaatgcaatcagtcgcactgatctgcaattcccttacgcgccgattctgtatcgcttccgttctatctacggtgtgtactgtaatcagtatctggacgaagcatcgatcaaacgtgctaagtccgatcgtcctgctttactgactgtatcgcagcctgttccagttcgtgttgaagacgagcacgacagagagtttgcttcacgtttcctcaaacacactgccgaccaagtcagtgcgttcttgtatatggtgtgtctcgaccaatacgcccgtgaacaaacagactgctggctacccgcacctccgacgccattcgatctaccgaagaacattttcaatgacagccctatcgcattcactgctacgcacaatgttttgatcaatcacttgatggaagcaatgttgcagacgcatagcgatacgctggacattcatgtgtcgttgcgcgattacggcctgtcagtgttgttcccgcttgtggcggaatgtcgcaatgtgatttacgctgcatggccgatcacacgcgaatcgttccgtcatcctaagttcatggataaaggcgaacacgtaatgttcgacgacttccctattgatgatgacagggaagagttcgagccgattcctacattggggcctacgttcgaacgtcaggctgagtgggttactgtagcgactgaaattgcgcaggtattcaatctgcaagcgttcgcagatgatggtgattcttcgttcatcttaaagcctgcggtgtaccgaagcggtgaagacttcctgttctggtctgagggtcaattgacaggcaaaagcattctcgatatagccgtgagccctattaagggtcaagcgtatcttgatctcgaagtgctgctgcgtagcgtgagcgcaacaattcgtgaccgcgcagagcagaacggttgccatgttatcacacgctacatcgatcaggaagaccagaccatcggtgtactgattcgtgttcgtcgtgacgttgatttcccaggctccgctctggacgtagcatctcatgtggagtacgcacaatgacagaccaagtaatcactttcgaagatcaacagagctgggaagacttcggcagcgcggtctatgaagaatttcgtttgaacacgatgactggatccagcttcgcctctcaggtacccgaagtcggtccgaacgaaggtgttaaacacgccatgacatatcacaatatgtcagagaagtccgataaagtcgtgttggacattcttatcaacgaagtcgcattggccgaaggtgagtcgcgcaattacgacgcagccgagctggacgctgctgtgcgtaaagtcgtagcgctctaccaagcgcgagcgcgtgacctcaaatgtcacattactggtcagtatctgtcggaagagaacaatgtggtaggtgcgctgttgcgtgtctaccgcaacgatgacttcccatgtactggtcaccctgaactgctgctcggcaaaccaatcggtatgtaccactgcgataagtgtcatgagatgcaagtcgcaggtacattccatctgccgctggagaacgacaatggttaaaggtgggttatggcgtgtcttccctgactatgactcggaagagatgctgatgaagctcggtgccgctatcggcattgagcacgacgaagacgatgtgcctggagaactgcacgttactcttgcttacgacgaatctaatccaaacgtcaaggcagagcagaacgatgcaggccagttcttcgcagtcgttaaagaagcaacgttgtttggtgaaggtcaggataagattttagttctggtactcgaatcacctgacctgtgtgctgaacacgaacgcattcacgcatgtggtgccgctaagtggtcgcacccaacgtaccacccgcacattacgttattgaagcaagcccgtgatagtcaggctgaacatctcaatcagatcattcagcatccgggtcgccctccaatcactctgcgttttatcgaagaagatcgtaaggtgctggagaagcgtaactaaaatcctagcggtggccctgtgctgccgcttttgttattctggagatatttctatgaaaatggtcgtaagcctaagccacgaaattcgcgtagagaagcaggacagtgctgctaatgaagcgcagactcagggcccaaccgatgcgcagcaaacagctctcgatatccaagagcgtgggcgtattgtagaagaatacggaattgacgcacctaaggacgaagtggaggagaaagagaaagaccgcattgagcgtgagcaggaaaaggaagatgaaaagcgcgccaaaccacctgcagatttaggtcagcataagcctattgaaggcaaagaacttacggcgaccgatattcaaaacgagcatgatctcctgacgaagatctagaaatctgtaaataagagtcaaagcaactaacaggtgtatttgaccatgaacaataagtcgaatctcacaggcggtcagatagaaagcgtcatggacaccatgttacatgattgcctgtgtgagattgtggagaacacggacatattcgacgtccagcttacctacttactgggtttggttacgtcgaataagaaacgaaagccatataacgctgagacacgcgaccgggcaataagcctactgattagagcactctctgtacctcgtgatcagaagatggttttcatccgcgaacttaaaatggagcgtaacttcatttacgtcttcctggaaaatgtaattaaacggtactacacggcgtatgttggattgtatcgcgcattcattactacgcaggacccaatcaagcgtgttgcgtattcaaaacgactcgacgtgtatgtgaaaatgtttggcgcagagtcgcgctcgaagttatttgtcgcgctctgccgtttgaatgatctactaccgcagttcatggaatacttccactcggtagttgctgacttctatcgtctgtgcagcaagcagaccaagttctatgttgataccaatcgtggtaaactctacgatagcaaagacgtgcgccagaacttcctgcgcaacgttatcattgcaatcaacaagtatgactcgtcgcgtggtgcgatagtgagttatacgaagtggtggattctgaacgcacaaacctgtagcagtagcgagcacgaatacggcatcgcgtacactattccccagactcaacgtaagaaactggcgacaggtgaagataccacttctctgaatttctcggtaagtctcgatactccaacgaacgaatctgatgaaggtgcggacgcgtcccttcatcaaaaggtgagtgaccatcatcacctagaagatcacgttgatagtgaaagacgtactgaaaaactgagactgcttatcaagcgcgtagaccctctcggtgtcgctcgactaacgatggacgttggcgaggagttcgataagtttgaactcgatctcatgcgtagacatatgcaagctcaagggctagcctaaaactgtaaacagtgcatatcatagcacaactcaatattgaggaaatataatggcacgtggatttggtgacattcaggacaacagcaaacgtgatagtctgcgtgagtccgaaatctttgaaatcttcccgctctcaaagaaagcaaacggtaactgggtatcaatccgcctgttagatctcgacctgcttccaatcaagaagcactggatcaagatcatgggcggcaaagacaaagataaagaaatcaaaatcccgcgcatgtgcgttaacttcgatccggataatcagggtaagcctctgaacggtatgaagtgcccgtactgcggtattgcacacggcaacgacgaatctggcgcgccagcgcagtacgactataagtggtatgcgcaagcgatcattcgtgacgaacaagcggccgcgcctcgtaaaatgcctaagctctctaagaaagagcagaagactggcaagaaagagatgggcagcgaatcttggaccccggttcagtgtattcctctgactaactctctggcgcagaagatcaaagacctgggtgaacgtaacattcacacagtcaaagataaaaagtctggcaagaagtcaaagcaggcgttccaagtgaaccatgcgaagtacggttgtgatatcgaaatcaaatacaacccgaaaaaatctcctgccgaacgttacacaatcgaacgtggtgatcatacaccactgaccagcgatgaaaaagaatatctgacctgggacttcgacaactggaacgaaatctacgacatgctgggtcgtctgaacgaagaagccgctatggcagacttcaaaaagatggacgttatcggcgttaacaccaacgactctgacgatggtgatgacgaagacgatgaagatgacgacatggcgctgggccgcaagaagaaaggcggcaaggcagacaagaaaaaacgtcgcagcgatgatgacgatgacgacgaggatgatgaagacgaagatgatcgtccatccaagtctaaaaagtccaagccgaccaagtctcgcaaaatgctggacgacgatgaagatgacgatgacgacgaggatgatgaagacgaagatgatcgtccatccaagtctaaaaagtccaagaagtctgctaagtccagcaagacctctaagtcgtccaagaagtctaagaagtcagatgatgacgacgaagacgaagacgacaagccagcgaagaagaaaaagaaatcttctgataaggtaaaatcgtccgataagaagaagaagaaaaagtcttctgatgatgacgacgacaagcctgcgaaaaagaaaaagaagaaaaagtaattcgtgtctcggggtagcttaggctgccccttcttctctcaatctggactatcccacaatggcgaaagcgaacaacaaggccgagaaaaaggccgagaagaaagctaaagttaaagttaagaaaggtaaagcagaagcagtagcgtccgacgatgttggtggcgtagaactgctgggctttgaccttgcaagtctgatggacgatgtgcttgacggcatcgaaaagaaaacgaaagtaagctcgcaagatgcggcgcgacatgcaccacgtatttcgactggctgccttgcgcttgatatgtacctgtccggtggtatcgtacctggcggatggtatacgttcagcggcggtgagcagtcctgtaagtctacaatgaccatgagtatcatggcgagtctgattcgtctgaaatactctggcattagcgtagtgttcgactacgaaggttcaaccgatgcagagtacgttgctggtcagttgaaaacgtttggcgttaaggtcgacccgaaaactatcttcggtgtgcgtgacgacaaagacggtagctggatcgttaagcctcagatccgttactacgcaccagacaacggtgagcgcttcttcgactacatgtccatgttgcgtcgccgactgcctgacaagatcgttgagaaagacggcaccgcgtactacatctttgagaacaacaaagagaacgcgaagaaggttgctggcaagtacgataagaaatggttcagtcgtaacaaccagttcaaagtgcctgcgaacgatggtcacatgcaggcgatggttatcgttgactcctatcctgcgatgatgcctgatcaggtcgatgatgacgacggttcgaaagcaatggcgctacaagcgcgtatgttctctgacggcatcaaacgtttccgtggcggtatgcgtcgtaagatgatgactatcgttggcgttaaccagttgcgtcagaaacctgctgtgatgttcggcagccctgagtatgagccaggcggtgatgcgttgaagttctattgcttcgaccgtgacactctgattcgcaccgaccacggtgtattgactgcgcctaagatcaaagcgctgttggacgctggcaccgaagtctctgtagaatcgttcgacggttatcagaaaatcaacggcgcatggcttgtcgatgacgcaccgttcccgttcgaattgaacgctggtggtcatgtgtatgttggctcggcagaacatcgccagttcactctcatgcacgacctgacggccgaaggtactcctgtactgcgtcctgagtggaacacgcttaatcaactggcccagcatccagaagcgcaaggtcagtatgctggtctgcgtgtaccgccagttaaggaactgaaagagaaagttcctgatgcgttcgatgcggccagccagcgtatcaaagaactgcttgagtcttcggttatcattgataacatccctatgactctggctacttctgacggtaagttactctgcggtcacatggctcaactgcctgaagagttcgttggtcatgttagtgatttgctttcaatcggcatcttcgcctacgttgataacaactctgatgtttgggttcctggtctgactgctgatgatattctcgatgcagtagcgcaagacgaactgggcgcgtacttgggtatcagtttcgatgcaacctgccgccaacgtcagactcaaatgctgtcggtgattgctgaccacttccctgagctggtgcgttacgttctggactatcagttgtgggcaggcgaagacaaaatctatctggcgcctgagaacgactttgcgcaagcgcttgacctgattctgcataaagagatcgctggctacgatgacatgtacgacctgctgatgttccagctggcgtatgttgatgactggtacaacttcgactctgcaattctgcctgtgccgtttacgcttcgtgcgctcgacgagcagcgtgagttctgggatgtgaacgttgaagaaactgcggtagttattaccaacggcttcgtcagtcataacagtgatgtgcgtgtgcgtctggcttcccgtgcagtacctgaaggttggccgaagctgaaagacgctccaggcatcgtcggtgagaagtctgttaccgtcgaagggggtactgaccgttatcgcttcattgctgctaagaccatcaagaacaagatgggcggtatcccgaaccaacagacgtggttacgtttgtgggaagctgatggtaacggcgaagcgcgtggctttgacccagtgttcgatacgtggcactacctgaaaactctcggtctggtcaacggcacccgtaagtcgttcaaactgaaagcaccgtgcccgctcgcatctgatgttaagatggattgggatgacttccgtactcttatcaacggcagcaaagaacaagttgtcggcgtgtgtaagaaactgaaagtcaaaccatcaggcctgcgtctgtggtgcttcaagttcgttcagtctgtcaaaggtaacgacatgctgaaagctgctatcagtaagtctgccaagaagtctgatgacgacgacggcgacgacgagtaatccccgggcgggcttcggcctgctctcctttctggagaaagaaatgcgtactcaaatctacaccgctgatattgttaatctggagaccgttgtcgttgatgacgaaggtcaagagacacgtagcccgacaatcgttcccaatctcgaaggcgaacgtgacctgactgttagcactctcggtacaatcatggcgaccgtgactgctgaaccaaacgctgatgctcgcatgatcgttctggtatctcgcgctctggttcctgctttcgcagaccctgaaggtgacttgttcgatatctttgatccaatcgaacgtgttgctgatgttgatgctgggaacgtcggtagcgttctcggtatgcaggtagtaatcaacgataagtcagacgacaacgttctggccatcgctgatgttctcgacaatgaagctggcgttaccattcgtacctacggcgcagctatcattcgcgtttaagtaaaccttgtgcgggagaatgccctctcgcacaatccaactctcgataggcaatacgccacgagaaaacaaatcactcgataggcaatacgccaggagtaatgtatgaaaaagattcaacacgtagttcttccgaccgatgccctcaacggactcattcatggttattatcaccacagcaaaggtacggacgaattttgtaagtcactgttctacattgacgtgactgatcgtagcgcctccgatgcgctatactctattcttaaacgagacaagacctcaggcattgttcctatgggttacgatagtcaaaaagatgcgaggggtcacacttctcctgcgtctttggctgttgtgctgtctaacaatttactgcatctggatgacaataaaatgtccagaggcattttaaccatcttctctgctctggctagaaccacgcacaccaacaacacacaaataactgcgtatggggagcctggcgtagacaagattctaaacatagtgcgtagcgttgactacaaggactatattgaaggtgctggtgaaggtacagatgtggtgcttggcgactttgatcttgagtcaaacatgactatagaccatttcgttcacatggctatcgagcctaagttcgaagacgctattcgcaactcgcctgcgacagagtttaaactgggcgcaaactttatgttcatgcacccagacgaactggctaaggttgtccgcttgattcgccgttgcagtaagatctgcatcatgcaccctgacatacatcgctattactttgagaacgtaatctgtaaatactgatcaacaaccgaacacattgctgtgtgtagtctagcctgatttgggcaggggagagcctgatggcctccccatttttttttatctacagcagcaggagaacaacatgtctaaaacgactcctcaaatcttcctcgacctgtttatcaaagacgttagaatctttctgcctaagttcgacaaaggtctggacgcgtacttcttgaaatgtaaaggcaagcctggtcagtctggcgtgtcgttgcatcaatatctgaagtggctgagtcctatagcaaagcatccagagaacgcgggcaaactagctgtagttatctctgggtatctgcattacttctggcagttgtctaaaccaaactttgtgtttgaatcgacactagttaatcatttggcagactctgaattgcctgataggttgccgacagagatcttgaagaaactcccttactggtgtcagtgggtaacattgcctatacatctggagaatgcgttcaggactttgcatcttgacttcgatggtgcttttgttgggtactctcagatagacaataggcctgtactggttttatgtgctccctttacgccaggtgatgaaagcatcaagtcaaataacttcacaccgtctgtaacgtcattcgtatatctggacgaacctgtcgacccttggtcaatgctaaagaacatgcacctgttaaatctggttgatactcttgaggacccagactttcgtgaactgatgttcagcgtataccactacctgacaaaagttatgtgttgtgtgatgtacatctgttctcagcaggaagcgttatatacagaaggtcatactcagcctaagcctcaacgtttaggcaagagctatcgtatcactccgcctaagtcagatcgcatgatcaatataggttcggagatgatgcaggtcatcaaggacttcgaagcagaagtcgaaacgtgtactcgcgcttttaacggtcgcaaaccgcatctgagaaaagcgcactaccaccacttctggacgggaccgaaagctggacctcgtaagctcgtttgcaagtggttgccgccaagtattgttcgcggctctgtcgtagagcaataacttttatctcaactccacgtatgggcgttatgcccggaggctattatgaaatctcgtgtacaaactctatggattcctgatatggaatcgtatgaaccttacgttcggtctctgtgtcatatggcgcgagcactcgaaaataacggcctgaactacggcacgatgaaacgtgttgtaatcatcggtctctccaagcgtagtgtagaatcctatgttaagcagttgctgaactcaaatacattgccgaacactctcgtatgcttcggcattgatgaaccgccgagaagtcatagtgaattttcattcatcggcgcccacgttgtgttgatgcacgatctacgttacgcctgttccgactcaatgggacgtatagctggaagggtgttggatataatcgacagtctgaaacagaaagacaccgataaagaattgaagaacggcgcactatctctcgtctaccaggtaccaatgctttggacaaacattctggattatggcacaaacagtttcattaacctggaaagcaaacacgtagagtaccgcagcggcttggtatcgtctatcggcattgatgcgttgatgaagtgtcacgataacaaagactaccatgaacttcatgctgaggtgatcacaataggtcaggagttcttgtgcgtccagaccgacgagctgcttgataaggtgggcaacctactgtggtcactcgcgtctactggtagtaagtttgagaagacacacaaaattgtcttccatgagcacttccgtcacttgttcttcgaagaatacatcctaagagacttcaagggcttttaagaatattcttagcctgctctctaatttcaatatgttggcaagtagtgctgacatatcgttattggagaataacatgtgcggacgtagcctcgttaggttgaagtacctcgcacggtcatcgaactggtgcaataataaagtaaacgcttgtagtgagcggaaggcgaagaatgtgcaatgtgaggaatttttggcagcgaccaagaattgccgcagcgaacagaagtcgtccagtgtagtttctttcttcaaaggtcatgagcttgttggtcaggctatatggcatgagattgaaggagacagcacacttcaattccggttgctacttgcttaacgacagagggcctttcagattaacatctggtgggccctttcttctttatatgctaattttccctgttattaacacacaaacctatttcggggtaatactatgtctttgattaaaatcgaaggcgtccaatcattgtctgcgcccaccaaagctcagaaagacgccgctgtttatatgtttggctccaagggccattcaatcgttgctgtgcttgacaagttcagccgtgcgaaagaagtgcgaaccgcacacatcgacggtctgctcaagctgatgaaagatggggacgatgaagaaatcatcaagttcactgcatctgctccaggcaagaaaaccatcgcggctgcgaagcaattcgctgtagcaaaaacactgaccgctagcatcaaagcactgaaacttgtgcgcgttccgatgaagtggatcgatggtcactcggatgccgctgctgctcgtattaccgagacaaaagaaatccgcgcacgtaagagtgcgggcaacaagcctgagaagcctgtcaagctcgacaacccacatgcaccagaagcagagactgtagataacaaaggcacaaaagagccttctgcaaaagaagcgaaagcattcgccgcaaacttaactaaatctctcggcatggagttcaaagtagttcgtggtgatgctacggaagaagacccactgagttatgaagcaacaaacccagatgatcagtcagccgttgcgagctttcgcattactcctccgtttgacggcctgcccgacgatatgaaatctaaagataagcctaagtggcgaatcgcaatgtcatatcgtgacggcaagatgcgcattgctgtcttaggcgatacgttcaaagccgcttctgcaaaacgcgttatcgccaaagaaaatcaggcgcgtgtgaaaggtgtcaccaaaacaacaagaggcaaaaccgctgcacagcttgcttcgcttgttgagtctaaaacagccgcatccttggacaagctgggcactctcgataagaacgctttcttctctggcctgtctggaacagtaggcaagaagttgggtaaaggctatgttgttaccccaagtggcaatggtcttgttctgcgactggacgacggtaatcgtggtgcccgtgcttggctcgctctgactaactctggttggacgttcacttctgtcgaacaaggttctggtggtaagcaggaagaatcgttaggcagcaagttcaagatcgctgatcttgtgaaacgcaccaaagcgtggctcaaatctccgaaactgaaagcggctgcaccagcgacaaccccatacacgcctacaggtaagtctcctatctcgctggtggatgaactggcggaagtaactgcccgtaagatctcagccaagcctctgcaggagcgtgaagaatactttaatgcgctgcgtacggtactccagaacaacctgcctaagcgtgaagtgtctgcaacttccactggtgttgtgattggtggaagtaagctgcacaccttacgtctggacaataacgcatggacgttacagacaggcgttactggtaagattaagaagatcggcgccacgttcgatattgttgacctactgggtatgatggacaagagcattctgcgtcctaaaggctaatagcattaaatcaaaaggggtggcttcggctgcccctttttgcgtctatatgtgccgtacatctgactaactctgcatataataggttgaaatagcggtgtgcgcatatcagtcaaaatgatacaatatagtctctagcgcaacaacgcgcataacactgccgaggggcaaaaacaatgactatcaaatttaactctgtttacgaaatctttgaagctatgaacgtgtgcgccagcgattcagctttcaccaaacaatgcggtttcccttatcctgaggtagaaattttgcagtgtggtttgcaggaagatttaggtgtgtatgcgtcaatgacagacggcgtgaatttcctgattgcagatacgagtgacctgttttctgaacatcttcaaggtgatggtgaaatcaccgtttgtcgtatcgaaacacctaacggtgagatgttcgacgagccagaagctatcgttacgcagctggggatattcaatgattttgatgaagcatacgcagcattcactacagccgtaaacgctgaactcaacaaataataggtcaaaagcgctatagcaatatagcgctatttatcgtactatataatctctagcgcaatgatgcgcacctgaacactgcaatcccagctctgtaacgaacaactgactgcggggttacggccccgcttatatgacaactcgccaagagaacataatcatgaccagagaagaactgactacactgattcgcaactcactcacacgcactgacttcgcagtaatgaactgcgtagagcctgatgactacgaacttgttttgctgtatgaagtagacagcacgggtgaatcgcttggcgagatgggctatgaagtagaattgaatgatgacggcacattctcgcttcactaccttgagatgccttggtctcctgagccgttcccgtcgttcgctaaaacttcgaacttcgacgaactgatggcagcgataaacagtatcgagtttcacgtttcaggcactaactaacaataagaggcaacaatcatgtcagagaaacaaatcatcatcgacgtaatcgcagacgtagcatcgccaacagaagttgtgtttgaagatggcgagtcttctactcaatggctcgcaccgttcgatctgcgtttgactgtggcccaggcctgcggtccggccggcgtaccagaagtgaacatcatcggcgatgaagataacctgcgccgcttcttggccgtgaacgatcagttcgaagacgctgagatcgtagacgttatctaacaaacaaagagcggcgcttcggcgttgcttttctatttctgcctgagaaagctgctatgaaaaatcaatatctcattattcgcatgaacgccgcaaacttctacgacaaacagtttctgatgcgtggctttaacgccaagcgtatcgagcaggtcattggcgttatcgttatcataggcgatgaacatacatactcgctgaaagacagcatgtatcatttagcaaaaattcacgtcgaacagcttacatctgatacacaacaaaacttagttaagctgcgctggtcgagcgtagacagcaagcgcatagaagaaggcttgacgcgcatacccgctgacttgacagacgccatacgtgcgatgcgcaacactcgattgtattatgaagtcgatacgacaatcccacaggcgtttcgtgaatgccacactgaatttgatatacctactggcgctcaaatgcgtgagcgcataaacaaacgacaacgtgaagacgaggcaaagatcaaacttgttgaccgctcgcacgtaacgaaagcgcttaacgattgcactgtggaagaaattctaaagcacctgaaagagcgcacgggcgctgagatcacaatcaagctgtaacaactaatcaatgtgtggcgttacggcgccacatcatcacaacttaatagagagaatcacatcatggctatcgtaacttttttcgtaaaacgttcttatgcttcacttggcgcaggcaacttcgctatccctgcctcacaggtgcaagagctggcagaagctgagtgcttcatcgtctacactaacacgggactgggtaacacgttcgctgtgcgcaacatcacgatcacaccgctcgatgaaaacagcgtggctgtttcattcgaccctctcaccgatgttcacgcgctgcctgcttcgattctccctaaagagattttgaaagagtcagtcgagcgtatcgtaatgccagaagaagatatgcgtgaagtgccacgcttctatatcgcaaacgaagcaaatggcaacaacccgaacctgcttgcgcttgatctgaactgccgtcaacgtttcgtgcagtatcatggcggcctgtgtacactgaccgatcttgtgctggcgctgtacgagacaggcattcatatctctgaaatttctccgcgcgtgaagcagaaaagcaacgttgctgccgtactcgcacaatatccccgtaccgtgtttgagcttaacaaagataacggagttgtgaacgacaacctacccttgttggcgcgtatgaccgtactaatgtaaacaactatcgcctcgcattgagcggggcttttctatttggagaatgttatggtatacgaacgcgaagaactcgaagtcatgcctctcgatgcactttatcatctggcgagtgccaaaggcctgctggacgatttggacgatgatgacgatgcacctgatcgtgaagtgctggtgggcatgattcttgatgcgcagaatgaacaacaggagactggtagtgacgccaactgaactcaatgaatatctgcatctggtgctaacgcctgtagcaatggcgtggcgcgagcagttccctaagaagaagcaggtgatggcgtctgttaagacagcgtactcctgccgaatcaaattcgtcgaagaccgtgaagttgaaaagcagtggcaggcattctgccgcacacatggtctcaagaacgaagaaacactagaaatctaaacaacaaggactgtcgcatcggcagtccactaaccaaaaggagatttagatgaaacgcaaagtgattctaatcacaaccgaagagttccacagtcgtaagatcgtgtcaccttccctaatcgatctctctgacgtagacacggttgtgtttgtcgttggggaagacgcatatgtgccaactgatgtgaccgtcagttacgcctctaacccactacgtcaggtgacaacgttcaccgagtatcagaagattgcaactgagccgaagatgctacgcaacttcgcgcatgttggcgatcactatgacgatgaagtggatcaatcaccacaaactaaaatcaccgtccacgaataatctaaagggctgccattgctggtggccctttttcatttctgtaaatatcacgcacacaaacaacaatgcgagatattcaatgcgccgctttctgacagtctttaacgtcactcaacaggagtttgacgaccgtcgctttttccagcataagctgaacatcattacgaccatgcgccgaactcatggcgtgttgttagctattcgtgagacaggtaaagtattcgtagcctctaccgcctcatatcaaagggcagaagaatacgatctgcgtcgtgtggacttctctgctcctagtgaggttacgcacgaacttggtgaacgtttcaccgaactgaaacaggcaatcgctaacaacctgcaggacaaaagcattcgctacttcggccgcacgttgtcgcttaacgatgttcagcaggctctgtatcgcacacaactggagattatctcatgacaacaatcgcatctctaggcgctcgattcgccgcttcatcctctgatcgttgttctgctcgtaaaaagaaagacccaaagaacaagacgatcacctgtgcaggcacgaccgccatgtataacgccgtagagagactcgcaatcaaactcaacgtgtcccgctcccgtgcagtagagattgccattgaacagcttatggagaaacacggaattgtcgtggagggtaccgatgacaactgatacgatctactgtcgtctatatggcgttcagtatcgtctgggtgtcactggcatcgacttctcacaatcgcctactgtctacacagtacatgcctgtgacctgctgcgtatgctgccgagtatacatgtcggggctgcctacagcacgtacacaccgtaccgtgtgctcaaagccggccgtgctgacttcaagatcaaactgattgagaagataagtgctgacgagtggcgctactcatttgttgacagcacaggcagaccattcaacactattctgaaacggagaaagtatggccattggtttgatcaaagtcttaggcctaaaagacaaggcaccaaagggattcgatcttgatatcacaccagtctcacgcgatgatgattggtggtcgctgagtcctttctatctgggcccgtgtcgtactcctgacggtatgatgttcctgaacatggagaacatgtggcagtacagcaaggtgtacgaagaacatcttgttaattcgaacgacctgtttcatggagagatatccagcgagtggtgggagtggcatttgaaaggaagtacaaccgaacaggcgcatcgctatccagcggggaagggtcgaaaggctttattctcgaaatggggcgacttgcgcctttcgtacattcccgcacgaaaacaaatctacgtgccagaatatgcgaagctggtgatccacaagcctaagttcaaacgcttgttgaaggagtataagaaaggcgccaagatagtcctcagagattatgacacctacgatattcaaaaggcttatccagattctcgcagtccgtggttgaccgccatccaaaacgagaatgcaaagtttggtcatgcgtttgtcattgcactggccttgatgtttcacgaacgaccactatggtacaatcaatgggtaatctaaagtacgaagcctgcattgaattgagtacacgcgaaggcaacatcaacatgccagaactccctcgctgtgatctgcaatgtcatcttctcgatagctacacgcagatcaaggtgcctgtgcgtttcgattgcactaacatagttaaggtgtttagcaagacgtgtggcagcctgcaactaatatctgccgctaatctgatcgtctggtcatcgttcgaacctggtcgttttacgttgtatatcgaacgcgcctcaagcgagagcacaagcgcccagcgagctgctgaactctgcaaataattggctgaaatagccattcagtcagatacgctcctatgatatactatatgtgagcgcgatgctcatacaactaacgcttaggagcgtatcatgactactttatctatcgctgatttgaaaacccctgctactttcactacgaaccttactttcggtcacatggaagaattgcgggccaacctcgaacgcgccttgaatcgccctgaccttgaggtctatgtagattgtgattctaactacacaatcgaagaagcaaacaccgacggtcctgatcagctggtgggcgaccatgaatgtattaacgttcacgttcgttactcgggtatgtcgtttgatgaatcaacggctaaaggtgtgtgggatgttttgttgcagaccccacatgaagataacagtataagtgaatggtcgaactcatacattatgtatatcacggacgacaacatggacctgttagaggaggtaagtattgagaacggaaatccacgcatgtatgaaacattcgttgaccgtctgaacttctggttacctaagctgtaagcgatttgtgaagggcatttgcgagtgccctttgaaaatcctaaaccctaagctgaggagcttaacatgtcatcatctactactttgactttcatcttcccagaactgaccactctggaagttaccatcggtaacggcgttgttcctgctcgccttgaagtagcagagaacaaaagcaaaacgttcagcgatattgaagcgctgcgcctgatgcaagattcaaacgtcaacggcgtaatgtctggcttcgacctgtcgctgttgaatctgcttatcgaccgtcacaacaatcgtgagcatttccactgtcaggaatgcgtaatgtctggggcaacgtacttcccatcgacgggcctgtacctgcgagtgtcacatcaccgctaagatttgtgaagggccttcgacgagggtcctttgaaaatctaacccataagctgaggagcttaacatgaaacaatatccacgccgtggccaagtgtacttcatgaaagaaatcgaaaacgagctggagttgcgtgatagcccgttcttgcgtttcgtgccgcagaaagttcgttacgaacacgaggtatgtgcaggcattcaggtcattcagacctcgtcagttgctaatctatctgacattgaaggttgggcagatacgcagtggtcatacgtgcgcgagaccgaagagtggattccgctgttccgtgctgttgacgacgcggcgattgaagcgctctgtgttatcgagcctgacacgtctgagtttcgttcgggcggcggtatgcacatctatccgaaaggcaccgtgtgcaatcagcataagccgtacgatgaaaagctgcacggtgatatgcttgtgagggtatcatgaagggattaatgaatcttttcaactgttgggctacgcgcctttctgagcgtacaatcaaaattgcatattgcgtatatgtcgcattgtttattttggttgttttcctgacaagtccgtgggtgtatgactcgcctataggcatgtggatattctgctgcgttactgtatgcgttgtgacgccgatgttcattgctgttctgattcgctctaagacttgctaataaaacagggatgctcacaatcgtgcgcgtcccatttctcatttaaggacaatttccctatgataccagaactcactcatatctttaacgtaatgatgaccagcctgaaagatattcgcagcgttgatcgtctccatctcattaacaaaagtgctgtgcgctttcatctcaagggcaaacagttcgacgttcgcggtaagtttccgttgttgtccgttcatgaagttgaaagtcactgcctgtcttattcgaaagctgccaaagagattgaagcacaactcaatggtgaccctatcgaagaaatcgaagacaatgcccacgacgctgctctggacgaagtgttaatcgctcacgtagatagcatggaagaagatcgtgttcgtgcgtacaacgaagaatgtggcggccctgatttagacccgatcaatatgcagcgcacttggctaaagacacattttctgcatataggtcacaacacgcctgaccttctcgaaacagttctgatgatggaaggtcaagagcgccatgacgcgctggcaggcgccgttaaggggacattatgtttctagcgtggattaaatacctgcgcagtagaaagaaccagcagtttatgattgaagtaacaacggcaatcggtaagttaaaccagcgtgaccgcgacctactatgtcgtgtattcaatctacctgctgatgcagaaagtttgtttacgttgtctaacatgaagcgtaagcaattggccgagcaatgcaacatgtattatgccagcgtgtctggtaaaaactgggacgtgtatgatacgttcctcaaagtcttacacaacgcgagaaaaggaaagtaaaccatgaacgaaatagatattctgatccgtgagtatgaccgggcgtatctgaaggcagaagcatcacctttcggtaacgtcgcatatcacgtacaagatcaaacggacggcctgaaaaacattgcactctatctgcgttttcgttctggtccgcaagctctttggcagcgtccgtgtttagtgctcgccacaattgatgttcgtgactcaggtaaaggtacgttcagtgagttgcttcgccgcacgaaagacctgtgccgtgaacgcgactggattcttcaagttgaaaacgttctgactcctcagttcagaaagttcttgcagcgtggtggcttcaagccattcggcattgataaagacgtaccgtacggaagtctctactggttccatgacgagacaatcccgcagcaatgctctatgtacccagagaggccacacccatgaatattccttggtacgttatgttcatgataggcctgctgccgctatctacgtgttacgttgtctttccgtggtttcgtgctgctgttaatcgcagactgacattcaagcctcttgactatgatgcacttgacgagatactgactggtggtatgcctgagcgtgttaccattacgtgcctgcaagccgcatacaggtctaacacaccagcacattctcatgtggatatctatccgcacaaagagaacgttgctgtgattcgaatgctggtggaccctaacttccctattgcacgaacctttcacaaggtcctgatcgataactatagcgcgttcgctgtgaagtcgaacagagcgcccctgatcacaatcaatcagtgcgtatatcctgttgttgagtatgagtatgacgatacgtacctgttgatttacgtcaagcataagtaaggaaacatcatggtcacccaacagcaactaacagagtttgcctcaatgcctgtactccatcgtaaagtggtactgcgcagtatgcaggttgagatgttgggtgccttgcctgagctgactgacattgtacgtgagatgctataccgtgcgattgtcgttgacgtagctcaagctgaacgggcactccttgctgctcgccagatgtgtgataataaggacactcgtaagagtattgatgacctgcttcaattcgctgcacgtctgcatgacgttgcaactgataactttctttctggagatttactatgaataagactgttggcctgatgattgatgaagacgtaatgaactggctggacatgctgcttgctggtgaactcagcaacgtcttaggcgcgttgaacaatattgtatacgcccgccgtcaggaactgtctgtcgaacgtctaacagaagacgaagacattgccgcactttctcacaaagagttggaaatcatcctgcgttacgcttcacctgagcatgagtacgacacgtccgtgctgtctaatgagcaactgcttcgtttggcgatggacgcacaagggatcatctcgtacacattgccatgccactgttcgcctatcatggttcaacgtgctttcgctaacggccagatcaaatcgttgttgggtagcttctctaatcgtgctgatatcgtcatggcagttcatcattgggaatgcggcctgactaacatctcacttgatgctattgttggaaatgatgtgcgcccagacgagcaggggctgtatctgtgttacgacgaacataaacaggtacgttacggtcgcctgttccgaaatgccaatgacggctggacattccatgaatcgtatgctgctggcggttcgacttcgtggttcgaagagggcgaaggcaaaggtcttgacgacgatgacctgccaatcaacctgctgtctaactgggtattcgtagcgcctgatcaatcaccgtcaatcattcgcaaagagacggacattaaacgtctgtctgaaacacaacgcatcttcctgtatttgcgtagcctgagtcctcacgtcaaagcagaaatcgttgcgcatttcgatggcgtgttgaacaatcgcgtattcacttctgttgagcagattggtcgccttacagaaactgactggcgcaatgctgctatcgctatcggtgaagaagaacgaggtcaagaaggcagacacttctgggatgaccgtggtgcttgggcttgtttcgttgctgtgctcaactctctgtgctatgacatggagacacgcgacttccaacctcaatacgaatatcaagctaacgacgacactctggacgacaacaacaatggctaaatcactcggtgtatacatgacttacattctgcgacacaagccgcaggatatcgggatcgcaatggacactcagggttgggtgtccattcaggacttcttggaaaaagcgagctacaagaataagcccatcacacgcgatcagttattggctgaggtagttgaagacgaaaaaggccgcttccagttgaacgccgcgcagacacgcattcgttgcgttcagggtcactcggttgagaacgtcatcatgaacctcgaaccatacacgctaatcaccgaccctgtgtatcacggtactgcggaaaagaacgttgcttctattctggcgcaaggcctcttgaaaggtaaacgcaagcacgttcacatctccgctaatgtggctacagcgaaacaagtaggtcaacgtcatggttctcctgttgtgtttgagatcgacacttacgccatgatcacgcacggatataaattctaccgtgctgagaatggagtcatcctgaccgaccacgtaccgtccagatatatcaagttggtgtagtatggagaagacgtatatgcgtcattggggatcgcgctatgtgcggtcctcctccggcaagtggtattcagttcatggccgtgagggtacgtgggtaacgaatcgctacggtacttcattctatcgaagcggctccgaagtatggcgtgacatgacccgcgctgaccgcgaatcgctagagcgtgagctggtcaaacgtacacgcgaagactttaaggagaataaactcaagtataaccactggggcaatatagtgagggctattgcccggcagtcagaagacgaaaagaatgagcatacggcagaacttgctgagatgctcgaagcgcttagacagactttctacggacagaaggtacagcaactacgcacaatgttggacgaaatagccgttaaagagtaggctcgttcgtgctataatagagatgaacgctagacagtcgtttagctacttacatgaggacatgtatatgaaaaagatcaaacacactttccgtctgaccgatttggttcatatctccaaacttcctgcaggtatgtccaaattccatgaaggttcggatgcgattgttgtcggccgtaatgaagatagcgaccagtatattctgcacgttaagcatgtcggtgagctttcatggtacgaaggtaaatcactgactctgattagccataacaatggcgaactgcttgatcagtgggaagcaggcgactacggccgtgacaagaaaaagaaacgcaagatcccaaaagaactacgtaacttcacggcaatcctgcctgtgacctgcaatgccgattgttcgttctgccctgagaaagagatggagcagaaagccaatcagaaagaatggcaagatggtttgattgcccaaatcaaacgcatgtacaagaaaacgaagttcgaccacgtatcaatcagtggcggtgaacctacgttgcgtacaaagttcctgtttgagacgatcgaccgtattcagaaagaaacgccgatcaagaaagtcggtctgacttctaacggtcagttccttgagaaaccaaacagcacgttcgacttcttagaccgtaacactacgcctgagatgaccagcaagctgtcgcatctgaatatcagtatgcactcgttcatgcgtgagcgggccaacaagatcatgggcgttaactacaaacagactctggaggatttagttcgcttccgtcgccagttgggtcgtgacgttagcttccacatcaacttcgttattaacgatcagacaggttcgattacggaagagttcaagatggccgcaaacttcatgcgagccaacccattcatcgacgttgtgttccgtgttgactacaacgatgttgaactgtcgaaagcgttgcgtgactacgccatggaatatgaagcgtggcaggaagcaagtcgcattgcagtagcaacgcgcaagaagtgcaaagtgaaagagccgcgcgcaccacacatcgttcagaagtttgatcgcttcttcggcggtcagaaccttgctgatgttgaaagcgcttggactacaggttgcccttcttgcttcacccatgcgtctaacccagtcaataacagtcgcgcatatttgaaagcgtcttcctacgaaccaaacgaagacgaagcagaatacacggagctggtgtatcatatggacggcgctctgtattgggattggactcgcaatgaccctgtgccgctgccacgcagtaaacgttttgacttcgagatgaaggaagagagggccgacaagcctatgcctcgtttgaaaagcgcgcctaaagcgaagactgtgaagaaagcaaaaaccgccaagaaagaaactcctacaacgagttccggaagctgtcactattccgcaccttgtagctacagccagggcactggcggttcctgtagtttccgtagcggcggttgcaactattaataggggaaaagaacacatggctaagaaagaacaagtaacatcgaaagacctcgaagaactctactctgttgttatggagtacgaaggtagcgagcgctatcgtctgtactcaatgctgactgtccgtaagttgcaggcgattcactacggacatacaattcccgccgacattctgcggctgacgcacggcagtaacgaatatgatttgcaggaagctattgctctgctggggaaaatgcgatgaacgaacgtcgaaacttttactatgatagtccgttctattatgggcttatcacttggcgcaaacgtctggccgttgtcagtgcaatgctaatcggtattctgatttatcacggccgttctgctcctgctgttgatgatatgtggttctggacaggaatcatcttcggcctagttggtggtgtatgctacattcgcatgtggtcctatgagtgctacctactcgctgctatgggtcctctggacaacagcactgttattggtagtctgtcgttcgacaaacttgagcgtcgtcatgaactctggtacgagaagaagttcgggcacaaacctcctaagactaacacatggagcatcgactaatggcactcatgtttactgagaagcatcgcaaacaattcggacgtgacagcaaagacccgcagtatcatggagatgcgtgtgaggccgtgtacaaccatggcatggaattgttgcgtgagcataagcgtctggcgttgcttatcggagcgaaacgtagaacgcgcctagataaaggtgcgcctataaccaagtgctttcgcaagcagtggattgaagataagaaactggcgaacgaagacactcgccctattgctatgttgattgctcgctttaaagaagtggctgtcttattgaagctggcgcgtatgaactataccgacctacatactcgtcgtcacggctttactcgtcctagctacttccactggagagactaacatggaaaagaaattctgcaaactggtacacgtcggtgctgacgtgattatgcctgctatcctgtacgcattgaacgaaaagatgcaggcaggcgtcaaagtagatctggccgaagcgtatactttgttgaacgatacacaggctgtgtatcttactctggcgagcggtcagcctgatcgctattacgatcaactcacgccaaccattcgggcgcttctggcaaagtatgaaatagagtgggcactcgaccacgcagcgcttacgaaatactgtcaagcgtatatggagagcaagggcttcactcatgctggaaacgatgtgtattcatatccagaagttgttttgtacagcaactatgaccgagtgttcctgcgctcattgattagtgacgcggaccacaatctactggaagctgcaatacaggacgagatggccgttgcggcagagatggacgagattgataagaaactcgaccgagtagaagacggctgctgctccgagtgcggcaaagaacttgaaccagatattgatggtccgttcatgtgcctagcatgtgacgaggatgatggagaataaaaatggctgtaggcttcgtaaaagatgatggcgttaacgacaccatcgaagctaacctgaacaacgagattgaccgtgcccgtgcagagctgttgggtaatggcactacgcattgcgttaaccctgattgtggtgcagagattcctctcatgcgccgtgtagcaatgccgaacgcacgttactgcgtacagtgtcaatcaagccatgatggttctgcgctgagcctgtacaatcgtcgtggctcaaaagattctcaactgaggtagaaactatgttaagcaaaatctggactgcaatgggattgaagtacccgtcagtggatgctgctttacgcaagaacagaaagtgtgtgcgcattagccaagacggctattgcgttcgttctgcttctggttttgcatctgcgctgtcgcatcatatgtcccgtgattacgttactcttagttcgaacgaagaagctcgcgccaagatcattgaacgtgcgaagacgctggaatatccgtgcgttgtttggttcactggtgcctcttttgatgtgctgcctgttgatgatactaatctagagtaccctgtacaatgaagctgaacaaatggaaaatgaagtcggtgaagaaataactgatattggggaaacacgtatcatgacagaagaagaatgcagagtcttcctagaacgtttgaaaaatcgcggggaagaacgtaagcctaccatcgaatgcgaagactgccgtacttctctggaagaaggtgaagtctatggcgactccgtatacctgtgtgagaattgctgtgccgatcgtgaagacgaaggagagtcaatatgaagaaagtaactgcttctgtacatgctgtacatggcgaacgtgttgtccctatcttctttggtgaagacgatggtaagccatacataggcaaagcgttttgggatagcctgtgtctgcgtgatgacttgtttaaagagcctgaaacgcagcaggttcttcataatgatcagcggatgaatagaacggagttcattcgcgtgtctactttccctgacgtgattcaagcattgcgtcgatgcacaaactacatccgttactttgagtatatcagtgacgaagacattgaagacctgagtgaagctctcagtcactgggtaaacgaggacgaataaatggaacatcaaaagcatttagaagcaatcaagcaaatctccgtcaaccagattcaatcgttcagctacgtggctgcaatcatccacacgcaggctaacagtcagcctgaagtgctatccgaagtatggcagcgtcatatgtgtaccacgctaggcctgacttacgagcactggacgtactacaacgagcttgctaactacatggaactcggtatggttccatacatgcctgtgttgcaggtagccgtaactgctttcgttggcgcagacgttcgtgagacactggatcgtttctcttatcttgacaaagagctggtagtgtctgcgtatgaagtaggtaacgagtggctgttggacaatcatcgtttgatctgcacctgccgcgcaatcgactccctgatcagtctgtactctacgcacaagctggagatagacgaacaggaagagaatcgttgcatcgcctaccctgggatgccgaatatgccgcatcagtttgttgagatgtacaagctgatcgaagaagctcgtatgagtgtggccgggcactggcgaacacctatgcgttacttccactccaaagaacgtgactatctgtggaactatccaccgaacatgtccagtatgcagaatgttatcattcagacagacgccggtaccatctatctgactggcgcacctaagcgtggagatactaacgctaaccatctacgctctgtgtgaactgtaaacccataacatcgacctgattgaggtgttgagacatgattaagaaagtgacagcgttcatcgctaaagatgaaatgaccgtagagcaaatggcggagaaacttaacctgtctagctacaacgcgattcatcgtggtggctatactgtagtttgtggtacagacagtcaaggtgatcgtatcagcttggtctgcggtccgtatgtattgcagcaaagtatctggggtgttcagaagatgctggacgcagggtttagcgagacagatgcgctgctggccttaggtctaacccgttctgcttacaccgcgctcaagaagaaagagcgtgagcaaaagaaagcggccgagcaggctgctaaacaacaacctcgtcgcggctctgtcgtgtctctcgatgacctttaaggaacaagcaatgaaacagttattcgtaggtagccacccaaacactgtgaagttttctgaccttgacggacgtgaccgtgtttgtgagatccgtgtcatgattgctgcggcgtacactatgctgcgtgatgcaatcggcgagcaagcaaaagttgagggaaatactttccacggtccatggcttgtgtttcgcaatctcatgaacgagcaccctgctgcctgtcttgaagagtatcgtcacgcttcgatttatttcgatgcagacacagaaggcaaggtaactgaaatttgcgaactgatcgaacagcacattgaactgaccagacagacactcgacctgcggggcactcacaaacatcaggccgatgtgatggttggtatcgcaagcactgccgattcaacgcgtggagtaacgcttgtgcgtggactgggtaaatctcgaggcgatgctgtgcttgagactgaattgcagcacaacccacatcgtgccctggccgatgacctgcgcaagtatctcaatcatttcaaagaccgtaacggcgtctttgagttgtgtacgctgctgactaaacgatacggcaagccttcattcgatgactatgctgacagcacggtagatgaaatgattgacgaaacgtgtcaggctgttcagtcggtcaatgagcctatcgatcaagtgtacgacttggtttgccgtgcaatcctttcattcggtctgcctgctctccctgcggatgcagacgacaaagatgaccaggctgctgacgatgaaaactacgctctcgcaccttaagcagtactggcgcgaagcgatgatactgactgtgttggttattgtcgctatcgctcttccttttctcgaagtatgcaacccaacgttggtgatgcttgttgctgttatcgttgctgcgtacttcattgctacttgggcatgtaagcctatatacggacctgacgatgaagaagaaaaatgaaatcaaactgagcgctgcggatatagcaacgggtatcatctgcatcaacgaagctctggctaagcacggcctgtcgtgtgcagacggcgatgttggttacgaaactgtgtacactgacgagcatggtgaaacgcagggtggctggtacgccgagtttgataagaagtctcgtgagaagctgcgccaatctaagcaggtgcactggcgcaatactggaatgctcggcggtgatacgattgacgagattcttcgcacaatcgcaggtctcaagtttcgcaatcacgccaaagagccgacgccattgcagttgaagaaagcagagacggctttgaccaaagaagaggctactaagaaggcactggagatctacaactctgcattacctctgtctgatgcagacttaaagctgtgtatcgatcacttccgtacgctggagaagatgattcgtattgacccaatgttaaagctcgcgcagccgtacgttgtgaacaatctatatcaactcgaaaactatttacacgcacgtaagtgtaagtaaccaatcagggagatccttaactggatctccctctgtcgtttctggagcatttctcatgcgatttggtttcgcctgcaaactgattgacccacaaggcaaacagccgtacacaaacaaaagtctaagctataaacatttctctgccttatctgcacctgaccaacatgacaagctcttggacgtcgttacgcataacctgacttcactactgtctatgatcaaacacgttggtcagttacgtacggatatgcgcatgttccgaatcacaagtgagctgctgcctctatacacgcaccctaaggtgtttcacatgtacatgcgacaggacgttgtgcgcctgactgaaactatgctggcgatatgcggcaaagcagcaagacgacacggtgtgaggctttcatttcacccaggacaattcacggtgcttgcatctgatcgacctgacgttgttcaaaactcgattgctgaacttgagtaccacgcgtactgcgcctatcacatgggatacggtagacgctttcaagacttcaagatcaacattcacctgagcggtagattaggtgcagtaggattcagagcagcctttagcaaactctctacccactgccgaaagatgctgactgtggagaacgatgaaatcacttctagcattgaggacgtactgacactatccgacctgtgtcctatcgtgctggatatacatcaccactgggtaatgactaacgagtatatacgaccagaagatgatcgtgtgcgacaggtcatagactcttggcgagatgttcgacctgtagcgcattactctgtgtctaagcctgagtttgttccttctcgcggtctgcctgatcaaaacaagctgtctgctaatcgtatgcagttacgagcacactctgattactatcacaatgaagacgtgaacgagtgggcgctttcattcactgattttgacctaatgtgcgagtcaaaagcgaagaatctagcacgtacaaaattggcatgtttttcaggcaactctgcaaataactggacaaaatgaggcttgtatctgaacatagccctgtgatacactagatatgagcattatcgctcgtcaaaataactagaatcgaggaatcgctatgttcacaactactatgactcaaaagaaacctgcaatgtctctcacgtactcacggtctaatcactatgagacacgtaatagaatctcttgcatctggcctggtgcgctggacgtacctatgccaatcaaacgttggtgccgtgctcacgaaatcatgatcgatctcgacgcttacatgcgtgttcgattcaggggccgacgccaagatatccttacgttgattgctaatcacattgcagtcaataaccctgaccttgccactcgcatcgccgcgacaatcactgaggcttaaaatgaaacttcaacctgtggaagctgtttacggtgctcacaacaccaacactcctctagtggagaaacgcggctttcgttctgtcgaatcgcagtacgtcgatggcacggaggttagattacaacggctcgcacatgatatacatgaacgtgtggttgtgggctacgatcaatttggtcgggcagtgtacggaacacgcgtaccacaatcaacgttcgaagtgcgtgacagcaaggaaagcgaaccgaataagacggcgccctagcaagctcacaaccagaagccatagaataacaataaccaattcatgcgctgacctaccgtggggtgtcttaaaatgatcgttatatgtaatagctcgaaagaattttcagccgaccgtttggctcatggggacgcatttgtttttgggaagacacgcatgttgttacgtgcggacttcatcatcctgacagacaaaaacaatgcagtcttcgtagtacgcaaatctgatgttgtttggtctcccgagcttacgggtgcaacgcatgtgattaaaatccgggcgttcgcccagattaagccgtttgaactcaacgcagcatgtcctcaatttaacagtcgtgtgttcggaacaatcgcattccgtaacccacactttgagcaccgtcttggtagcttgaaatatgtagagacaatcttcggaggtttacatggcacggtatcatgtgtttagtgcgacccataaatactacggtgaagcatacgaaggaacttggctcaaagagataactcttaacgggcaccaagttctcaacgcagaattccctaacttcgaggccgcgaaagaatgtgccgacaagttgcatgaggtttgcgatattgggtggatcgtgtataacgctttttctgaacgcgctatgtacgatacccgcacggtacaaggcgagtctgtaaacaactaacaggcccgccagtaatccctaatcgtgatgctcacgggcgtcacacaaattcataatacgaggctataaaatgaaattcaccgcaatcgctatcgcactggttatgtctgcttccgcttctgctgcaaactacgtggcacccgcacctgccgctggcatgaaatcttctggcatgactatcagcgacaagctggacgatagctgcctgaagaaacttaatcaggcgatcgacctgcgtcattcagtgattgactttgctgtatcgaaagatgctatcgacacggtagccgcttggccgcttgtgtgttcaccgactgttgagtccgcgtcggttactattgaacgtatcggcagtgacattacgatcacctacgtcaataacgacaagtcgctggcgaatcttagcctcgtgttgcagcgtgtagaatccactacagaagacgatgcgcctgcgtatcagatcgttcagattggtgacctgaatgctatgggctatcaagaacaaactgacgtgaaagagtggctgcttgattgttatgcggctactgtgcaggacgacatggctgtagtgaggaactgatgaaaggaaagaagctaaacgtattcttgcagcaacgaacggcagtaaacaaagttgcgtccagtccacaagactgggagacgtacaaagaaatgctgctaaacatacggcttgccgtagcggtcgatccacgccccgatgctgctattcgccatttggctcgtacttggtatgctgaatcaaagtacgcgcttcctgtctgtcaggctacgcttctgaaactgatgacgttgaagaaagcaaaccaaacgcttgaagaaatgatcgcgctttatattgaccttgaagaaggaactgagaaatgaccgaagcagaactgaacaacgactacatcgttaacgcagcaaaaactatcttcacctcaggtacgctgcaacaacgtgatgccttgcgtactatcgccaacaccgtactgtctggcaaagctgcatttgcctacgaagaacgtgcgttggatgttgaaacaacgtatcgcctgctggaagaaatgcaattcactggcgacggtaagcagatgctgcctgccgatgaaatcgtagcgctggacaacatcctgcgtaagaactggcgtaaagacttcttctctgctgtgtcgaacatggcgctgactatgtactgtaccgaccctgcgacatacggtaagggcttctggccgaagaatcaaagcgattgtgtgttgttgatcaatcgcgcattcatatgggtggttgctcaacagggcctggtaaatcttctggaaaaagattgtccgagcgtgagtcatactcgtctgccgcagtttatcatcgccttgcagactgttggtaaagatgatggctatgctcgtcacttctcactgtacgagccgcatgaagattccggtaatgtgaattgcaccaacctgctgcctgagtcatacaaagcggcgctggaagaggagcgtatttcaaagcgtcctgctgaatatgaagcagtacgaaatatgaacttcgacgctctggccgatctgtgcgagcgtttgaacgtcattggtccaaattcaactaaacctgttgtctgtcgttgtgaccctgacgatgactgtggctgcgaagaagacgaacaccacacgcgggaggacttcgacaaggatgacgacgaactgcgcgatgtgttctatcagaagtttggttatccagatgacgatgacgaacctatggaagacgaaagtatctggttgccagatgtatcgttgatggaagttgatgttgatcttcctacagtaactcttcctctgcccgatcagcctgtacccaaacgtggtatgcctaagtctcgtgttaagaaacccatgtcttcacgtaaagtaaaacacatcttgtctccagcacaacaaatctggcacgaactggacagcaagcacgagtttggtgatcgtcgtttcgctatcacactcgtttctcgccacacatgcggtgttaatcgcgcagtcgctacgacccgtgaagcgcttgcaatagctaccgcactgatggatgtaagcaaatagctggtcagaatagcgcttcttcgtgaggcgcttctatgatataatcatagatagagcaataacgctctcaacgttctatcaaccatacgtttaaacacgggattgtcataaaatgtcacgtactatttcacgcaagaaagctctcgaattaatgtctaaaacttacaacgccaagcatcctgaatatctgccacgcctgatggcggaagatatggattcttccagcttgtttgaattccgtgaagatgttgttgcccagattcgtgaaggcaaagatcccgttgctgttgttgatgctatgatcgacaacgcgattcgtgtgaccttggttcgtcgtcgtaccagtaacgattataatcctaagatcgccgatgtgcttactgatgaaattcgtgacctgcttcgtaacttataaggaataaaatgaaaagctacggttacttctatatgttgaaccatatcgcaatggccgtagacgcacccaacaaggaagttgggtttaaatctatggttgagctggacatgttcaatcgcgcgtctatattaactcgtcctgacgctgagcctcgtgctgctcaactcgtcaaagacctgacctctgcaatctatcctgtcggtgattgtagcccgactattgaacaacgcatgatgcttgttcgcgctctgcacgatcaagagctggaaaagattgtaggctcgattcgtttcttcgtgccgttcgcatacacgaaagaagaactgtgcgacacgttcggcttcttcgacaacggagacacgttgagcattccgtatttcttgcgtcatcatttcatggacgaccaagccgtcttctgtgaaggtaagctaaccagcttcgcctactcatgcactcatggagaagtgtcacagactgctcggcagtacggtctgttccctgcatacgcttacggtaagaacgatatacctgagcaattcaaacatctgcctctgttctaggagcttctcatgggagtagttaaaggcataaccgctaccacgttcccgtcaagaggacgtgacgagggccagaagattgctctcaaaactcgctggggaattttccccgcgtctgttgttcgtcaagacaacgattatccacacaacgagatatggaagattgacgccaagaacttaccgcgtcgctacttctcggaagacgcagacctattcgtgtcaagacagttcatcgagaacttcccgaagcgctctctagtgtgcgctaagggtgaaagtgaaaaccaattcgtggacgttgtgtttgaccacgacacgcagaatacctgcgaaggcgttatcgtgacgcatcgtgatctgttagtcgtcatcttgattacgacgggccctcatgcaggccgatacgttacaggcaaagaatgccagtacgcacctaagccgcgtaagattaaggagctgatcgatgaaagttgataaaggtaatttccttgagcgtttgaagtcaggcaaaaccttttacatgcacgttagcggcaagaagaaaggtcaacctcgtcaaggtgtttcgttgggtcatgatgctcgctacaaagacctgatgatggccgtaggtggagttgcattcactcacgggtataagaacgttcaggtatcatttagtcgcaacatcatggcagatgctgatggtgttgtggtatttcgtgttaagcaatcaatcaccgttaaagaagaaaggacgtactaatgcaattcttaatcaagcctgaagatcgtttcccgaatttcattgcgcctaagcgcgccacagctaaagctgctggcttcgacctgtttgcgcaggaagatatgatcatcaccggtgacacagagttattcgatcttggcttccgcactaaggtaccgaaagaccacgttgctgtcatcttccctcgcagtggtctgggtgctaagtttcaggtgcagttggcaaacacgaacggtgttatcgacgaagactacacgggtatctggatggcagcgttgcatctcggcggtaaaggtactcaggtgcagcaactcgattggttgagcgcagcctacgagcaatcaagtcacaaagaaatccctgacattgacgacgacgaagaccagaaagcattgttgatcaaacgcggcgatgcgttcgcgcaagtgctgttcttcccagtgccagaagtcgaagtggttatcacgcacgaacctctgcctgaaacagatcgtggtgacggtggattcggctccacgacgaagtgatttacttctggctgatctttgcagcgtactacgttgtcggcattgtcgtattcgttcgggacctgagggaatcgacagatgatgtaatgctgatgcgccagttcaatgatgaactgaatcgcatgtccaatctcgaactcgtttgggatgcgacaaaacttttgctgttcgtggtgttcattcacattccgtgctggattctccgcgtatagtgatatcgttcacacaaggagccttacgtgggctccttattatcgtaatataaatgctatgggaaagaaaacttatctgctgccacgcgaacgccctagccctctgccgaacttacgtgcctatctcgcgtatctcgcccggaagcctaacgctaaccgcgaagtattagaaacgtattgtaatgcaagcctagctcaaatgcgccgcgaacggtttttcgtcggtaagctctttgcctacaaagtgtatacgaaatcgaacaagctcgcgtacacggttgtgtggattgacccatacaactacgactgccttgttctcaatcaccaaaggagatgtgtagagttcaaaaacttatacggcctgctattatagttgggtcctagcgccttcacactaggggaaatattccgatgataactgtccttaacaatcgtaccgacgaggtaatgaaacgcctgaacgtagcagtatgggtatgcgtggtagttgcgttcgctgtcttaatagcgttgcgtatctcacctgcattcgccagtatgtctacaggctctgacaacgccattgatatgtcctccgccgtgtcactcgatccctccaatcgcgtggcgacaaaatacaaggagatagaaaaggcagtagcagtcaaagacgaacgaaggccaaaacgctatgtaacacgcgagcgcctccgacaactttacgcgcacttgccccacccgtctgacttaggcaagcagattgatttggccgcagagaagtatggagtagacgcaaaactcgttctctctatctgtgtctccgagtcgcatcttcgtgcaaaggtcaggaataagtctggtgctactggcatgtgtcaaatcatgcctgacatgcacggacgttctgcacgggaactcatggactaccgagtcaacattgatcaggcagcccagattgttgcgttactaaacaagcagtgtaagggacgacgcgcctgcgttatccaaagttacaacactggttggggagcatacttaaaaggtgtacgttcaccacaatacttagcgaaagttcagaccgagtatcgccgcaagcatactccttcttcctgatagaggatataataatgagcatgaatatcaccgcactgtacaaaatgcaattccagttgttgaagccgctgtctccacgtcaagagtatgcactggtagtgctgctatgtgacaacattgttgatggtgacgttgcagcaatggcagaagtgatcgtccgtgattacccgcacgttgcgcgtctgtatgatgcgtttgctgcggctaaccaatacgagaacgcagtaccgttcatcgtacctgtgttgaactccgaagaagttacagaagaaatcttctgcattcgtgaccatgcactcgtagttgcacctgacctgcgcgaacttctgaatcaagctctcactcgcgttattctgatgcgtgaaacacctgatgaattgctgatacgtgaaggcgccgagttgctgctctgtgaagatgcactgccgtttgttctaggtcagttcatcgacagtatgctcgatgcttacaactgcggtgtgctcccaatgatcgtgcgcccttcgaaagagcaacaggcaatgcgccctgagcgtctgctctctttcgatatgctgcgcgaacataacatgttctctggaagtctggactttactaaagctctacagccgagcgctaaagcaaaggtgattgctgcccagcttatctctcgtctgcatagcgtcaaagccaaacaaggctttgatgcggtaacacaataaactcaacgggagaccttaactggtttcccgtttttcatttctgcgcaaattttaaggactacacagatgaccaaaatggttgcactgcctttcgcttcttctgaacaacgcaatcgcttcttcgatcaacgcgtgggtgacctaaaacttaacgccgtctggaactacgttgtatcaaacaacaatccgaactggaaaggcgatcctctgctgcaccacatgcactaccattcgaccgatcatatgaagcaggtaactgctctggctctctggcttctggataaagaagcgcaacagccgtggcaatacgatactggagccttgcctcttgctgtggcctgtatgttccacgacatggaccactcacttggtcgcctcaacgatgaaagtaatattcgtctggcgcaagaggctttcaagaagtatctcaccttgtgtgaggatgaacgtattaaagatcacgaagcaatcatcctagacctgattgacattacgcgcttcccgtacatgaagaaccgtcagccgaagaatctgattgagcgttgcattcgtgatgcggacattctctacggcctgcaggatgatgcactggacgtagtgatgtttgctctacgccatgaggtgaatcgtagcgtcaatatgaatacacgctacaaccaagaacagtgggcacaaggccgtgttgacttcattcgcagtgttgaaagttactgcccgactgctgacgcaatgatggactggctactggcggaagacaacgaccacaaccatcaagataagattgacgactggatgcgtcacgaagtcagtttccgagacacgtccgcgcataaactcaaagccaatgacgtgctgttcatcgacacgcaggaagacagcacaccgaagcgccgtctgattgaacgtgtcgaaacagttcacccgtatctcaatatctactttgacggaggcgaagctatctcgctgcgtgatggcgagagttgtgtggttgtcgaacgtcgcaaataataggctgaaataggcatgtactgactaggtgcctatgatataatacgcataggcactcataatagagagaactcgaatgatacacataaagcgtctgcacctgaactccgacaccaacttctttgcgattaacggaatcgtaataccgatggctttctactacatggacgttaccatgcacacagcagatcgcggagacagagaaatgaaaatcggtgtgcgtgtgaatccacatgttgcccgtgagtcttatctgcgtggcgtggactacagaacatttatacctgttctggcctgtcatccttcttcggacgaagaattttatacagagcttggctacattgatgttaacagtcgattcttcgacatgcaccaccagaagcgttcgcacttggcgtatcttggtgtgctgcctgatgttgccgagtcggatgtgcgggactcacgatatgtaacaccgattgatgtgtatcaagtgcaactgcctgaacgcgcccgcacctttgctaaggtgtacggcgctacgatacgcacggactacctacgcacttccgcagtcaataagattgacgatgatatgtgggaagcgttgcgtaccgtagatcatcctaaaggcgtatcgtggttccgcttcttagatgaagcaacgtcaggccgcttcacgccgcacgatgacctgtctaactgcttagaggcattcgatcaagagtacatgcctgagcatatctttaaacgcattcgtctggcccagttcgataaacgaggttaatcatgatgcacgatttgtataaggtgagtgctatcctgttctacacgctcggcgctatggctttccttgcacatatcgtaggcttcatgaagaactggatgaagattcaggagatgcgccaaaaagcaaaagcgaaagctgctaaggtgcgctctcctgttgaagacattaaacgccgtctgcgtaaagcagaagaacgcgcacggcatcgcccacgtaaattgagagactaatcatggctgaatcaacgcacgacaacaatctggcagacaaagtacaacgtgctttggagatctgctgggaagaaacaacgaagcgcaacgaaggcgaacacacctatgcgtttctcgcctccgagtttgctgctaacggtaagaacttgtttgatggagaattgcggatgctgaacgttatgctacgtgacgccgttaacatcaacatgtacggacgttatgttgcgactgtctatactggcaacaggggcatcatggttgcgttccagcctgttgctgatttggaagatatcatcgagatgaggttctagcatgaaccagattgatatgtttgaaacgtacggcgctcatgagatctctgactacactcaacttgagtatgagcgtctggctggtgagtacatagcgaaatgtgatcgtagagtgcaggctgccttcggcgacccaattcttacggcagagtctctggagaaatacccgatgcttatgcctggcaaattgaagtttcgtaagaagctggttatgatccaggagttcgtgctcgttacacacgacaagctcaaggcgagcctactcaagaaacagggcaacgttcgacagacaggtaatatcgacccgcagtacctgatcaacgtgtacaaccacaacgaaaagctcgcgctgttcatgagtgacttccaggacttcatgggcgacttcatgaatgccgttcacctgttcaccgttgctactgtgtatgatggtcgcttgcttgtctacgcagagaacggagagcctctggttactaccaaagaaacgctggcgatgctcaccgagatagagcacttcatcaaccgcagcaaagtgtatcgcgtacactcacaaaacgccatctaccgtacaatttaacctgagcgcttacgggcgctctactggagaaacattatgtcattcgatcttcgtcaaaacttactgcttgttcgtgacgctgccttgacaggcaaaccgctgttctatttctacaacgccatgggtagagagatggcactcactggtgacgtgctgcgtgagattcttgagcgtcagaaagaaggtacgctctgcaccaacacttactggggttttgctactgacccaacactggaagtttggtcgttcgatgctaacaatgacctaatgcttcaccatcgcgtaggcaagtcctgcaccacattcctgccttacgaaatgattgcaaatgcccatgacggattcaagccaatcaatggtctgttcattgaagacagtctgcgcactatcattcgtattcatctcaaggcgacttgccgagaagaacaaaagattacgtggttcgctgacctacctgagcctgagatgcgtagcatgttgctctcgtttggtctgggccctctgcgcgtatcgcgtgaagataaagaaggtctgatcaaactgcatgaccggtggctggaagacttcgacgacaaatacaaatatacgcacaacgcaatcggcgtcgaggccgacgagaagattcctgctgactatcgccctgaacgcattcgtgacattacgaagcgtatgatgcacaacaccaagactcagaatatgatggttcagactctgaatgacctgttacgtcagtgtcgtatcagaggcgatatcccaacgcccggcgccaactttaaccttcaacagttgatctgctactacgcaacacacttaatctttgcgcatgacgcagacgaaaagctgcgtagcctaattgatagcccgcagttcgtcgtcaacttcatctacggctggtacccagactattcgtggattgcggtcaatgaagaagcgttcgactaccagcaatcactggtacgcgccgcgctgatctcgttaaagcgtcatgtagagaatgaaatcggtacgtacaaaatcgttcacggcatggttaagttcgcagacggttttgaccctcacgctcctgagaaggtagaagtcgaagaagaggagttcgacgaagaggaagaggaagaggccgaaacggacgatcaagagaaagaagtcatcgactacctgcgtaccaaaagcgaagatgaattacgcaaagttgcgacaagaaagaaaatggcgcgtcctaataagttgaagtctatggacaaagaagaattgattgagctgtgtgctgactactacggcactgagatgcctgaagacttcgacgaagaggaggaagaagaaaaagaacaggagcgtgtgcgcattgcccgcaagttcccagtagtgttgcgttatgatcgcatagactatgattatgttcatcgtgcattagttaaaatgggcatagttaaaaagaacaagacccgcaagcagatggacaaatcacagaagctgactgttgctcaacaacacgctgcactgcttgtcacactcaaagaagctgtcttggactcaggtcaggacgttctatctaagctggacgaaataacgttgtaccagctggccgcctgcatgacgaaattgaaagaaggtgatagctatcctcgtgacgctgagtacctgaaagaactaattaaacacgcggtcaagtaagacctgcgtaaacaatacctaacattgacgggaaaataaaatgaaatttgaacaaaacattcttgtagtaaatcgcattgctcttatcatggacgacgaattagttcagaagtggggcgaagctgcaaatgcaaatcgtgacgctactgcgtatgcgacggccattattcttgccaaactccagcagaagattatagccgcagttgctgaggagaatccggaagcctgtgttcgtcctgagatattgtggacagactacggctctatctccatcaacggcttgtttatcattgcgtcgggtgcggatgctgagttgttgaatcacgtagaagaccacgattacttgaaccacctgcacaccatcaaacgtgttgctgaggagaatggattcaaactgacggttctccctgtgaagcatctgttcccattcaccaacactgaaatccctgaatccatgaagtgaggtgccctatgtcgcacaaacaaatcttgatgaatgatgttgctatcgttctgactatgactgaacgccgtgcattcttaggtcccaaagcagacggctttgtgtatctgccatctaaggatgctctcacgaaatttgaggcgcatatcaagaagtatggcaatcgtgatgactatgcgtttattgaccatcgtgagctacattctattagctctgcgggcattgtcgctattgcccatgctgtcgagtctgattctgagcagccgtggctttggacgaaagaagacttccgcgtcaagctgtggtaagcataaaactggctaaaatcgtggtatcagtctgaaccgtcctatgatataatagaagcgtagcttgtgctgcgcttttttaacatatgtctaaggagacaacaaaatgctcgaagaaatcaaaccaaccccaaccgacttagaactgcaagaccagatggtcgatgcggccgcccagaagattatcgaattgaaacctgaatgggttgacgtttctgccgcaggtctgcgcctgtatctgtctgtgtgtgaacaacttggtggtcctattcctgaattgcgtttcgtccacaacgccaagccgtgccgcattcggttcaacttgaatgaagtacctgaaggtacagagttcgtagcaaatgaaatcgacaaagaaaagcaaatggcgattgccgacgaaatgctgaaaactgccgaagcatgtccgaacggtcactcgctgctggatatagctatttgctctggtcgcctgttcatgattggttatgacggacttgcaggtactctcgataagatctgcattcgttgtaatcagaagaactacaccatgaatctggttaaaggtgaataacatgaaacctgaatacactttacttaaacgtagcaaggtcgatgttaaccgttttgctttcgtacatgacggcgagatactagctaacttcaccgccggccagttgtacagaacattggagaagctcggtcgaccgacatcctttaaggacgttgatgtgatttggagagacggcactcgcaccgtcgaagagctgcgagtgactgagcgccgccactttgttcgctttgatacttgcgagtacgatcatgcaatctgtctgatgatgcgggcgcaaggtctgcctgtcgaactctctgctcctgtagacgtgcgtaagctgtttgacgagcacggcccgcttattacttcaatctgtgtgccctgtgaactcgcagatgacctaaagcccgcacttgcgcgtttcatcccagacgaagatgacgacgaagatgaagatgaagatgacgacgaagatgaagatgaagacgagtgggatgacttagaggatgatgtagacgaagatgacttcggattccgcccagaagatttacgtcctcaactgagtgacttcggatatcgtgccgcggactgggttgtcactttgactgatgatcaaatcagcgatgtgcatagtcttgaagtcggtatggacccagatattgaactgccgcgtgccgatgacgcgaaggaagaatttttctaatgaaaacgattaacgaacaggtcaacgaattgaaacagcgcggcgtgcttatcatcgaagaacaccagaagcatacgctgcctgatttaaccttcacgcttgattgtctgtgtatcaatcacactaagcgggaagtagagacaaccacgcgcggccgcgttgttaagattcgcctgacaaacattcattaactttgtggtcttggcccgcccgtccagagatgctcacccccaatgaggtgcctcgcgcagaggtatgacggtcaccgggtcctttttagagcgcactacccctagtacgctgtacaaagtaaaacactcaacaggaggctgttatgaacttcaacgaagtatccaaagaggcgcaagtcgccctaatgtcaagtgccttggctggcgtaatcgaagcgttcacgcgtgaagatggagacgaaggtcgcaagattttagtcttagcactcaagcaagtcggtctgactgtagacgagttcggcgctcttatctctgacttgtcgccagaagttgagcttgaaattgtcagtgttatggaagctgccgatgcagagccggacgaagatgaagacgacgaagaacctgctgacgacgattctgatacagacgcagacggctggcagaacctgcatgaagatcgcgtgtgtcttgtatgcaaccatgaaagctgcatctgtcactaatctgcataaatctggacaaaacgatggttgtgtcaaaacagcgtccgtgatagaatatagatgtagggcgcatatcgtgaggagtgcgctctatatgcgaatgacgcgattcgcagtacgagagaagttcttgaccgtgtgttttcgttttccccggacacacggtcctttttcaagtgccttcgaagtttgagggtgcttgcgaaagggttcgataccttttgagcgcgtcgggctttacgcggtttccgccttacgtgctctcatgctaaaccgcaaaggaaatagatatgtcaaactcaaaagctgctgctaaacgttcaacgccgcgtggtccttcatctgttaagcctcgtcagttgcctcccggctacggctacaagtctaaggctacaggtgaacgttctggtggcttcacgcgtgatgaagttattatgcacacaagcgcgcctaagattcgtgacgaggagcgtgtgtacaatctcgtacatgcaattctgagcgcgtggaaagctgatgttggtcatgccgaacacacggccgcttctgctggcatcatcaaagtatcgcgtcgtaagattgaaggtgccttgcgtgacctcaagaatacgcgcttcactaaaatcccgacacttattaacgacgtcctcgtttataacgaagtctgcactgagttcgggcagtgggtatatgtcgagcatgacagtcctgattggattttcgtgcgtctgcctgaaaacagcacacccgtgattcgtgctgatgtcagctacgacaagacaggcgaaacgtctgcgtctatttcgacctcaagcgaagcgctgctggaatcgttcgattcccgtgacgacgaaatcgagatactcgaatgtaacgatcaggatattgaagacctcgaatctgctgagatgcgcaagcgtctgatcgatgcgaaaatcatcaaacctgaagctgcctcgaagctgtcacacaatgacttaatgaagctctgcgcgtactacggcaagtaagcaataacgagcaggcagtctacatgctgcctgctatctgtgaagtatgcagaaaactggacaaaatcgtggttgttatctgacggccacctatgctataatagattcagacgcaatagtgcgtcgcaaacaaaacacttatactgaggagtattaaacatggcacgtatcgaaactaacactaatctggttggcaaaactatcgttctgctggacggcaccaaaactaaaatcgaagatgcaatcgcgtctggctataaagtgaagggccgttcaacgaaagttgcaacccgctgtgttatcaaagaaggcgctcactttaaagaaatcgagcgcatgaacatgagcctgctggaagataccggcgaaggttacgtgaagctgaaagacgcgaaagctgcgaaagcatcaaccaagaaacctgatgcgaaagagaagacgccaaaagcaagcaagaaagctgccaagccagcgaaagaaaaagaacctaaggttcgtcgcaaatcttctaaagagaaagaagacgaatatcaggacttggctcacgctatcatcaaaggtggtaaacgtgcggcgcctgttgaaatcgctgagattgacggcgacctgacagactgcgttgctcaacgtctggtagacgtgctgaataatagcgaagttgcgaagctgtgcgctgataacaaaacgccgatcgcaaacgcagttgaagttacgtacggcgctgagttcgcccctgagaccaacgtcatgcagatcacgctgagcctgcaatacgctaagcctgttcaaacgctgtcacgtccgacgctggaaaacgcagaagctatcgcgttacgtgctaagaaaatggcggcgcctaagctgtcgatgaaactcaagaaagcgattcgtgaagcattcagcctcgaagacgcgaatgaccttgagctgggaactgtgctgctgtctgacggcgctgaatttgtttacttcggcgaatctgcgaagcatgtcggcaaagcgctgctgtatgttgtggagaccgacaagttcaaatctgtgctgggctctacgctgggtgagtacgaaatcccagacgcagaggaagaagaggaagaagttgaagaggaggaagacggcgaagaagaagaagaagacggcgaagaagaagacggcgaagaagaagacggcgaagaagaagacggcgaagaagaagacggcgaagaagaagattctgccgaatacgaatacgttgccgtgaacaaagatcagctcgatatggtcaataagaaagtgaccgctaagtatcacgctgcgctggccgaacgtttcaacacgaccgaagaagttctgattccgggtctggtactgacagacggcgaaacaaccttcgcgtacctgggttgcgatagcaaaggcggtctgctggtaatcgactgtggtgatgacggcgaaggcgaagacgtgctgatgtacagcaagtctgatatcaagtctctggatgacttcaatcctgtgatgggcgaagctgacgaagacggcgaagaatctgataacgaagatttagacgacggcgaagaatcagacgatggagatctggacgaagaagacggtgaagaagaagacggtgaagatgacgacttcgactttgacgatgtgccagaagctgatatcgaagatctgaccgaagacgaactgcgtgaccgcgtagtcgaagccggcctgaccactccgcgcaaagctgagaacatgaatgaagctaaactgcgcaagctgctgaaaagcgcataacgaactaccgtaacatcgaaatagtgtgcggctcttactgggccgcatatttgacaaataaagctgattgaggaatcacactatgtcaaacgcaaacaaaattctgcttaacgctcgtgtacgccgtttagacggaaccattactcacatcaacaaagtgaacgctaacggttatagcaccgacgcgaaaggcccgcaaatccctgtgaagcgcattgtgttcgcaggcaaaactctcaaagagattgaagcgccgttcgagaaaggcgagtatgtcattttacagggcgttgcagtgaagctgaacaagcgccagcaacgtgaactcgcagacaagacgctggatgagaaagcgctgcgtcctgactttgggcgtctggcgttcattgaccgcgacgacgacaaagcaactgacggtaagaaagtgaagccgaaagctgcgaagaaagaaagcgggttgaaagcgactcgtaagcagaacggcgatacacgcacaaagaaagagcgtaaggccgaagctgctgccgctgctgaatcgctcgacacaatcagatcaacgccagttgatcgcaagggcgagctgatagcgaccatcgacgcgaccatcgaagacgcgacaagcaaagagcgccgtaggttgttgtctgaatcattcgacatggactggaaagacattaagaagcacggcggtaagggtgtcgttaaacatctgggccgtaaagctgcgcaatctgccgtaagcaaaatgcgcgcgactgttacgcaggacgcattcattaagcagatgcctgctgagttgaagcgcttgattcaagatcgtcggctcgtactgaacaagcgccagattgaagctgtgctctctgcgcttgggcttgatgtgaagttctataacattgccatgcagacgttgcttggcaatctgtctctggctgtagacgacacgctggctgacgataaagcagataagaaagtgaagaagctaaaaaagcataaagcctctaagccgcagtatctgtcggagaaagaccagcaacgtcgcatgaagaaaatgaaagtgaagctgctggctcctactgagaaaggcatgaagaaagccaaagcgaaattgaagcaggcgaaagttacgcttgctgacaagctgggcatctcgccgaaagaaatcaaacgcggtctgattgcatatcgtccgaacggcgttgattacatgtttgttgccagtgatgctcgcggcccaatcttcatcgacaaagacggcgacccgtgcgtgtatacttacgagaatctcgaatcgacattcgacttccgtctgactcaaccttctgaactggacgctactgtatgaccaacaatgagatcatcctgactggtgttttcgcccaactgtattcgcggctagtaatggccgctatacagcgcgtccatgtatactactctgatctcgctcctgtggtgtttggtgtgcagttcactcgcgtagggaaagcgcagtacaaagcactggaggcgctcattgccgagacgatgcgcctcgatattcaaaacggcaggccaccacttgcgtccttatacgtgtcacgcgcaaacgacaccaagaaacctacccagtcattcttcaatgagtatctcaaattgactggtaaatatctttctgatgatgaatggttgatgctcgttgaacatgtgtggaaacaatatacaccagaccttcgggagccatcatgaaaaagtcaaaagttgaaatcagtcgcggtgggtatcgacccgtctcgccggaagaggcaaagaagttggttgttgaaatgctgcttgcttcaatcggcgttaacccaacgattatgagccagcagatgttgctgaacattgcgaactacaattacctcacgtctatcgcagacacaggtaagacaaatacagcgaaccagatagttctacataaaactgtaaaagaacttaatgcgttctgtagattgcacaagattcctctgggcttactaattatgccccatacatcggcgagcgattactccggtgacgaggttgtagcgattccctgggagtctgtgcgcaagaatgcaccgagccagtccgctgtcaactccctgttccaaacagtcgaagctgatggctatccgcagtttgtgactgatgcgaaaacagtagaggactacaatgttttatgatcacgtattcagccctgacgagaagcaacttctcttgtctgtagctgagtctaaatatctggtgcggcttgattgccctgagtatttgaagaaatcaaaacactcgattgaaattcgtcatacagtgaccaaccgtggcgaacaacgtcgaagcggtgttatcaatacaacgtttgtgccgcgtattcatgcctcaactgtgcagcgcctgttacgtgagattcgtgacaacgcaactatcagttcggctaacagcctcgccgcgttatttgaacttgggcttggcgtgccgaagcaacgtgatattgcaacgtacttgcacgactactctcgggagaatgacaagaagggtgtgggtatcaagtacatccgcaaactgattaacgagtatcaccgcaagcaccgtcatagttttgctggcagtcgctggatgatgcctgctgcgtatacggcgaacatgttgaacatgcagtctttcattcatctgaaagaaaacggttacagcaagaaagtgaaagtgcctgacggtctgcctgttgttctaatctatcagaacacgagtcacgcagaagctgagttctctatgtgtgacgccttcgctattagccctctgggttatccgatgccgttcgcccagattgcgatgcgtcctgagttcaaagctgcgccgaagacgtttcaatctaaagcgctgcgtgggcaaggcatgtatagcatggtcatgggtatcgttcactgggacaaaggtgacgcactgacgaacatacgcgaactgaacgccattgacgacgagccgtatctgacgttgttgtgtgacgaacaatacgcagatcgtcgttcgccggagtatcagaagctgctggacaaacgtgctgagtttgctgaacagcggcatgagtggtcagaagtgattgcgaagtatggtaacacaactcgcacactcaagcctaagcagttggagcgactggagcaggcagagaacttcttcaaagaacgcaaaacgtttatggacgagtttgataagttcgagaagaaagagaaccaccaggctgctaagaagtttgcagtagccagtgcgaagttcgctgccgttgattgtggaactattgctgaccgttcgacgtatatgtccgtagcgtcgggcctcgacaaagtgaataagattctcactaagtggggattcacaacggttgatactgttaatagtagtttgaagaagtctatccttacattcgacccaacaaccgctactcgcgtgtggtcactgtaaaccttttatctgaggagataacgtatgtcggaaaataacctgggcgctgctgcaaccttcggctctgagactcaaaagcaattaaacgaccaacagcgtcgtgcgcattcttctgagtccggccacgtaaacaaatgtaccatcgtcgttcttactgcgcttaacgcgcatggtcgattctcttacctgactgctgacgagcaactgcgtgagcgttcaatcgagggtaaggtgatggatcgcctgccggatctgattggccgggcatcgggtccttctactgatccgaacagcgcgtaccacatcctgcatccaaacaatggtgtgcctactcgtatcgacgagcgtatcaaagttggcgaagcggattcggtcatcatttcatatactgtaaataaagcagtgtcagagatgtatggcagtttatcgctggcgctgtttagtgctggtgaaagtgatatcgctgatttggcggctgagtatggtattcactccatctcaatcgttgaagaggcgaaagcgcctgactatatcaaagctcttgctgaacaggtagaagctctgaatattgtaaatctcactagcattgatgaagctgacggtgcttttgagaaaccagtaatcaactacagcgccctgccgggtaatccaatcaacgtactgtccggcgctgtgcgtactttcattatgcaaactctaaacggcgaagtattcgctgcgattccaaataacggagaactgaacgtgaaacaacctactaacgcaacgccggtcaatctggacgaagacttcgattcagaagacgaagtggttgatcagcagggcggcgaaagcgacgacgacgaagaagtaacaggcactgacctgttcggctataaagctgaaacactgaccgtcgcgcaaatgacagaagctcttgaagctctgtcctacgatgttagcgcgatggacgaagcgggcatccgtgagtcgttcgaaactgaacagcaaatctggatggaaggtaacgacgccgccgaagaagacgccgccgaagaagacggcgaagaagaagatgccgaagacggcgaagaatctgatgatgaagattccgaattcgatccttctctgtatctgggccacctgctgtctgctgaccggctggaccgttccgcactgaaagttctggtgcgtactcaagacctcaaagtcatgaagtccgacaccgaagaaacgctgactgcgaaactgcttgaactggtcgaaggtgcaaccgagcaggaaatggttgaactgatcgacaccttcgtaggcgcgctgcaggagcgtgagatcgattgttctaacctgctggccgcgcttgcgtctgacgaagacgaagaagaagacgcggaagagtcagaagaagatgaagaagaatctgaggatgaagaatccgaagatgaagatgattctgattctgtgcaagaccagatcgatgccgttatcgacccgctcgactacttccagttcgctggtggttcgctgactgctgaacagcgtgttgctgctgtcgaagcgatgggcgaagacgttactggcctgaacatcgtgcaggtaatgaaagcgttctctcgcattcagggccagactaacgaaatcgacgttgacgcagaagaaagcgaaagcaacgttgccgaactcgaagcgctgctgggccagtacgacgatgctactgtgcaacacgtcgcagaaagcctgggcgttaacgttgacgaatgcgaaaccgcagaagacatgatcgaagccattgccaatggcggtaccgaagaccagttcgctgcggttgtagaaatcgcaactagctacggtgttgacctgtcagaagttgctgacggcgaagacctggactttgttgacgcggttctgtctgtgctgccgtccttcctgtctgacgacgagcaggaagaagatgaagaatctgaggaagaagaatccgaggacggcgaagaagaagatgaagacgagcaggactctgagatcgattcttctgaaaacgaaagcctgaaattcatcaagtctgttaactctgacaacgccgttggtactctgctggcagtcgatatggatcagactgtagttatcaactttactctgactgacggcgatacttacagcgctgttgaatctgagctggtcgatatcaatggtttcaactaccgcttcccattcaacctgggcaaagcgtctaaaggtactgcgccgggttcaatgctgctgccagctcaatctctgctggacattgttgagcgcgtgaacactactcgcttcctcgccgatccgaaaacgttcgacattggcgcatgggctgaaagtctggaagcaacgctggcggaagaaattcctgtcgcgctgtacgcagaccgtattgaagacggcgttgacccaagcgaagctggtctggttgtgggtgacttcctcgacgaagaagaactggaagccgcaactgagctgggtcacatcgacgctgacgatgcctctgaactgaacggtgatcatctgccgctggcaagcctgtataacgctcgctctcgcgttcgcccggttcgtgtagacagcgcttacgttgcactacacaccacagtgatgaacgttgcactgcctggcttctggagcgaagcacctgtacagcgcatgattcaggcggcagttaaccgtgtcatcaatctggctgaatctgttgagaacgttaaagtgtatgctgcgttcaccatggagtctgctgcactgctgaacaacggccgtctgtttgaagcgctggcaactctgcgtgagtttgagcacgtccagtcttactctgctgctgacgctgctaacttcgacgatgccgaagacgtgatcgaagtagccggttcactcgacacccgtgacctgcctctgtctgtactggccggtggtctggctggcgcatcgttcgacaacggcggtgacctgacaattctggttccgtgcttcacgcaagaagaagacgcggacgaagaagaagaaggcgacgacggcgacgacgaataatatcgtctaaacgagtggctcgaaagggccactccctttcttggggatctgtaaacatgacacaagaagtagaccacggcgcaaacatcatcaagatggtaagtgaccgtgacgataaaatccgcgaactgaccgcagaacttgcagaagctattggtgataagaaagatgtggaaaacgtcttagaggatgaagtacgcggcaacactgtgttgcgtgtcgcactcagacgtaaagtacgcgaacacgccgcggagattgcactgcgtgatgaacgcattaaggaagttgttggcttctgcaacgaacaagcggttgaagtgaagaacatccgtgatgaactcgaatgtgtaaaacaaaagagtgaaccggctgctgcattgccattcgttctgcaattgataatgtctgctggtgtcgcacactaccatacgataatcgcacaatgcgctattgctactgccaacaaagcaacaaataaagttgcccgcgaactgcgcgaaatttatgatattgataatgtagtgaagcatccttcactttatcgtgtcgctgtccgactgtgtactcagctcggtgtttcgccaccatctcgcgccgaactatcagccgagattaaagagtatgtggaccagaacatcgacctgtacatcaaagacccgcagtacgctacatctgaatccgccttacgtcagattatcactgcgttgaaaagtcctgcacacttaggctcttacgggcgtgacgtgtgccaaatgttcgactggcttccagcactgactgctggcctggacgacattgaagatgactacaacgatttggtggaacaatctgtctatcaagtctgtcgtaatctgattaatgatagcttttcataatctgtaaaagttacctgtaatcgaatctgtaaacactaattgaagttcgaaccgagcgacaagctcacacttataaaatcccggagcattacaatggctaaagcaattaagtcctctaacctgtcacctaccctgatctctcgtattcagaaaaagtctggctccatcggtacttctaaagctaagccttctgaactgccgcacgacattctgatcgaaacggtgcaggctgttgagctgattggcttcattactgaccgcaccgaaaacagcgtcaccattcgccacaaacgtggtcatggttcttctgcgcaagttgtttctaccttcggcccgaatcaaactctgtccgtgctgggcgaagctggcggtcacggtagcgtaatcgctctgatcaacgcgccggttcgtgagtacaagggcttcaccatcaaatacaaaggcgcgaccatcgttgctacctctgttgagactggcgaagtgattgaagtgaacaccgcactgcctggcttcaccgttcgcgcaaccgtgaacgaaactgctgctgctaaaaagtacggcacgcctgctcctaccaaagctaagaagctggacaaaggcgacaaagctggtaagactgcgaaagtggcaaagaaagtaaaaaagtaagtaagtctgacgaagacttctaactttcgaaatctgtaaacattaagtatgcagcgagataaaaatgtttcgctgcctgtctctcgaaatctgtaaatcttaattgaagcaacgtcgcttctaatcaaacaggaaataaatatcatggctaaagctaaagcaaccgcaaacaccgcagcaaccgttctggctaaaatgctgggcgtcgtagtcgaaaacgccagcgctgctgatattgcagcaattctgaaagaggccggcctgactgttgttggcggtaaagttgttaaagctgaaaaaggcggtaaagctgctaaaggcaaaaaggccaaagcacctaccgttgctgaaatcgtcgctgctgctaaggacgaagaagaactggacatctccggcgtaagcgaagatgacctgcgcgccgcagttgttaaggccaagctgtctaccgctaagaaagcgaaagcgctggacgaagatgatctgcgcgaactgctgaacgaagcaatgggcgtcgagtcagaggatgacgaagacgaggacgaagacgacgactccgatgaagacgaagacgacgactctgatgaagacgaagacgacgactctgatgaagacgaagacgacgactctgatgaagacgaagacgacgattcggacgaagatgaagacgacgactctgatgaagacgaagacgacgattcggacgaagatgaagacgaggacgatgaagacgaactcgacctcgactcactcgacaagaaagagctgttagctctcgtcctggaacacaagctggccccggccaagaaagctaagaaaatggacgaagatgaactgcgcgaactctgcgaagaacacttcggcggtgaagacgacgaagacgaagaagacgaagacgacgaagacttcgacgactctgatgaagacgaagacgacgaataagtcctgatctgaaccggcagcccctctagttctaacgaaggagcgaggggcaaataatcgaaaaaatatctcgattattttcgtaaaaagttttaaaattcctgttgttgtatgttgaacataataatgtatgactacaggaacacaaacctgaacaaatttatcttttcatccagcggtgaaaacgccgcatcaaatataaagtaaggaatatcgtatgtctaagaaagcaatcagcggcctgaacaaagaaatcaaagccctggaaaaatctgaaaaagctctgaccaaaacttctgctgaaatcaccaagcaggctgaatccatcgctgaacgtcgtgccggtctgactgcccaggttgaagcgttgcagaacgacggtgctgctccggctaaagcagaaaagtctggcaaaaaagccaaagctgaaaaagctgaaaaagctgctaagcctgccaaagctgaaaaagctggcaagaaagcgaaagctgaaaaggctgagaagcctgctaaagctaagaaagccaaagcagagaagcctgctaaagctgacaaaaaagcgaaagccgccaaagctgaaaagccagctaaagcagaaaagtctggcaaaaaagccaaagctgctaagcctgccaaagctgaaaaagctggcaagaaagtgaaagcggataaagctgctaaggccggtaagaaaagcaaaaaagatgccgaagacttcgacttcgatatggaataagcaagcgccgcgcaatagcggtacttgatctaaaagggcagcgctgacgagcgtttgcccttttgtcatatctgtctcaaattttgaggtaaaccgaatgtctgctgaacatttgcttaacgatgacctaccggacgatactctctccacgaaagcacccacccctcctgaaaagcccaactactacgcgttaatgactctgcgacttgaagctggcgctcgtcttgctcgtgctctgaaaaccctgaaagatgccaacgtgttcggtgatgataataccgtgaatggcagtctcatgttgactgaggctctgaaggttgcagaagctaactgggcacatatctgcatgggatacacgcctgtaaaagattctaatggcagagagtctctgcgtgataaccttcctgcctgcatcgaagcattccgtgttgtcgtaatggaacatgctcaacgcgaagcattggagcgtgagtgcaaactcatgatcagccacgcagaaggtttcaaaattctgacacagcctcaaacactacagattgagccactacacttctgcgatggaaactgcgaccatgacacaaaaactgtctgagcaaatcaaccgctattttaatctcatggagaaaatccgtgagcaactgttccgtgtgttgaacgtgtccgatcgctacctgtgcatcgtgagctttaacacccagcatcaggcaatgcaatgcgacctagttagtcgtgaaagcctgctccctgccaagctactcgaaggtcttagtggtcaggagcttgtagtgtatggtaccattactgcccagattgagaaatgggtagcagacggtatgagcgacgacttcccgattgcgcaagacgccgatacctacgcgcagtatcgcaagctggtggaccctgagcaagagcctgctatctctgacgctaacttggcagagcatgttgcctctctacctaagtcagatgccctgaaatacgttgaccctctgagcaagtacgagcttgcgattatctgcaaagcatggggacttgagcaagatgccagcgagactgttatgctgtctctcgtcaagggctatattctgcgccgtgactcgtagcttgaactctgcaaatagttggacagaacgtgggtagcgtctaatactttagtatgatataataggcgtaggacaagtagtgtctgcatatgctaatatcgagtagtaatgctactcataggagatcacgaaaatggccaaagcgccgaaagctgccaaagtaaaaaagaaaacgggtgatgcttcccaagaaggtttcgtaattcacgaaggcttatcgggtatcagagaaaaccccggcatgtacatgggtcaacgtggcgaagacatggcgtatcgcgcggtaaaagaacctgtggacaatgactacgatgaatacatcgctggacgtaacaagttgatcgaagtggtcattgattacgacaacgacttgaacatcgtagctgaccaagctggcggcatccctaccgacttcaagaagttgaaagacggtacgaaagaaacgatcatgaccgcagcatttagccgcgttcatgcgggtggtaaatttaacgatcaggcgtataagacttctgctggtacgcacggtgttggcgtcgcggcactgaacgccatctccagtcagttgcgcgtgtggtcaatgtacaaaggcggctgcgtctatcagatgtggcagtgtggtgaagtcaagtcaggcaaagaccctaagaaagtcaagaccatcgacaaagacgttatgagcctgctgcgtgataagaaacacagcaagtacggtacagtggttgcgtggacgcttgaccagacagttgtgtctgctgacgttatgcgcggtaagaagctgccgaagaactatcgacacgcagcgccgaaccctgctcaactgggtgagtggttgcgtaacatgtcgatgctcaacccaggccttgagattcgtttgacgttgatcaagaagggcaagcgcaaagagttcaccttccacaacaagaaagacctgaacttcgttgtgaagacgatgtgcgaagaacgtgagctgggcactgtcggcaagccgttcatcttcaagtcagataacatcactgctgcacttgtctggactgatcacgccgacactgataacttcctgacgttcgttaacaccagcccgacagttgacggcgggtggcacgttgttggtttccgtgacgcgctgtttgatgctatcaagccattcatgaaagaatcgaagggcaaaggcaagaagaagcagaacttcaaacaggaagatttgcttatcggtctgactggtatgttcgattggcgtatgcacggtgcgcagtatacgtcacaggtaaaagacaagctggctagccgtgtagagaaagacgtatacgcagagctgaacaaggcgtttgtcgattacttcaagacgaacaagaaagttgcaacgacgatcattaagcgcgccgaagcaatgaacaagggacgtgaagaactcagcgccgtcgtcaagtctatggctgacacgaagaagaagctgaaaggtaacgcacttcctgctgacctgatcactgcaaacaagtgcaagcctcatgagcgtgaactgattgtcgtggaaggtgactctgctggtggtactgcacaggatgcgcgtaaccctgactatcaggaagttatgcttgctggtggtaagccgctgaacggactgaaagcaagtctggctgatgtgctcaagcacaaagaagtgcagggcctgttagtgagtatgggtgctgacttgaaatcgctcgacccgaaagcagacgcaccgattctcagtacgaagaatctgcgtatcggtaacttgctgctgctgatggatgctgatgctgacggcttccacatcgcaacgttgttccttggtgttatctatcgcctgctgcctgacatgttccgcgaaggccgtgtgtggatcgtcgatgcacctctgtataacgtcgtacacaaaggcaagcactacggtggcatgacgtttgaagaatgccgagcgctcgcaccatcgtctgtgaaagacaaagacattgtacgcgccaaaggttggggtgaagttgaacctgacgtgctggaagctatcgcattcgatccgaagacgcgccgtgtcattcgcgtgaatccattcgaaagcgtagagcaggaacgtttcttccgcggtgttctcgcagaagatgccgtacaccgtcgtcgcttactgggtctggagagctaacatgttcaacattgcaaagttgcctgacggaacgcaggttcgttttctcgatatgcctgacgtgcagtacccaccaatgactgacgaacaacgtagccaatgtgaggcgctgtatggtaaagcgcgtgagctaacaaagaacgttaccgtgtctgggttcactgtagttgacggactaccgaacgaacgtgtgcagattcaaatgcgccgcacaactctcgataagatcaatgcgattgccaaaggagaacagtaatggcaattacgccgaagaaagtgaaagtcaaaaaggttaagccgactgctgtagcgaaagccgctaagcctgcaaaactcaaagcgaaggccgtatcagtcgatgatatcaaaaagaagaaaaagaaaagcaccgacgttgcagcatcgaacgctgttggtacttcgctttatcctctgcttgggcaggacccaaagctgattcacgatgaaggcctgtctgactatactcgacgtgcgctgtcccactatggcgcatacgttgttgaagaccgtgctatcgctgactatcgtgacggcctcaagcctgtgcaccgcgcgctgctgtggtcgctgtctgacttgggcttacgtccaagcgctgcgttcaagaagtcggctcgtactgtaggcgacacgatcggtaagtatcacccacacggtgacgctgcctgctacggtgcgatggttacgattgcgaatacagtacctcctgctgtagcgggtcaaggtaactggggcaaccctgtgtctgctgctgctgcgcaacgttataccgaagcgcgtatgtcaaagttcacaggctcgttcctgcttgaccctgactatctcgaagttgtgccgcgtgtgcctaacttctcgaatgaccttgagattcctctgtacttgcccgcgttgcttccgtacatgttattcaatagctcggtaccagcgccagcgtatggtgtgaagtgcggtaacccaccgttcagctttagctccgtcagcaaagttgtgtgtgacatgctcaacggcgttcaatacgatgcgaagaagctcgctaagacgctcaagatcgtccacacgtatggctgtgaagacgtgacgactgacgaggagatgctgcaactgatctctacaggcaagggcaaagtcacgtatcagccattgatgcacgtcgatgaaaagaacaagctggtcatcatccagacctacgtgcctgctggtatgtcgaagctcgacgccatcacgaagaagctggagaagattggcgagtggaacggcgttgtgtctgcgcgtaacgcaagcggtaagaagaacaagcactctggtccgtatggcgctgcattcgaaatcaaatgccgaggcagcgaagacctgttgtatgagactgcgaagaagatcatgcgggaagtgacttcgagcgtcaactatacgctgggtgtaaccgttcgtcgtgctgatgcttcaaacaagttcatgtacctcgactacctgaagtatttcaaagcgtggattgcgtatcgcattaagctcgaaactgcgatgctccagaacaagctgacgaaagcagagaaggcattgcacttacagcaagtctacctctgggctgtagacaacatggacaagctgctcaaagtgttgccgaaagtgttggtcgctgctgaccctgacgcgatgcttgcgaagctgtgtaagattcctgttgaagatgcgaagatcatcctcgaccgtcaggtacgtaaactggcgaaactggaacgcagtggtctgcttgctaagattaaagaaatcaaggcagagattgctggatataaagcaggtctgaaagagccaggcaaatacgcggcagaaggtactgcggcgaaagttaaggcgtatatgaaatcgcctgacgacaagatgcctgtcaatctgtaatagatctgtaaatacaactcagcatattctaggacgaaacgcggttgtgtctgtatgtcatttatgttacaatgacgtgtctgtgggtagctgtctgttcgggagatagacagctactcgaactcataacaggagggtacgttagcgcagcaaatattcactcaggaaaaataaacgagcctaaaaaggccaaccagcctgactgtagattataactacggcagagcaatactataatcgacccacgtaatgctaatatgttagagcaacattggcattcaaagtgtcgctagggccggcaggatatggtcctcaactcttaaagaagtttggaaatccatacatgaaaaatcaggtagccaacctcaaagctggtttggagaaagtcaatgcagttctgacctctctgcgttcaggaaagaacttgaaacgccagcatgttgttgattcattaggtcaaccgacctctgtcttagctgatctcacgaaggcattaaaaagtaatacctacaagtcataccccgatgtaatacagttgcgtgactcagttcgtgcaacctgtacttcctgcctaagcctgtcagagcaagtggtcgctcgtcgtatcaagccacgtgaactgatggaaaagctcggagaaattgtgaagtcgttcgacgccgacgccaagttggctaagtcgtgtttgggctacctgcctgaatcacgcaaaactctcagtctcgatgatctcccagaagacagcaaagagcgcttagaagctctcaaagctatcgacaaagaggtgtacgagaacgaagcgaacgataaagctatacgccgtgagcaacgcgaagacgcagcgactgccaaaacaagtcgtgtgctacagcgcctcaaggacgcttactctcacaaggtcccgagaacgttcaacaaagctattcaaataatccaacttcctgtgatggcacgattcggtacactcgccatgagtcctgaatcgctctctcgtatgggcttcaaaatcgaaactgctggtctgcactcaacccctagttcggacttaggtatcgtctttgaaaaccaacttctgctgttcttccgtatgtccgacgcgaaaggcatggcagaagaagctgcgaaagatcacaagatgcttgatggaactctcgtcgaacgcaaacgcctccagaaagaacgcaacgcagaacgccgcgatctcaagaagctgaacaagctcctagaagaatcgaagtcgctcaaagctcgtcgtgctctccgtgaacaaatcgcagagactcagacagagattgacgacattacggcgaagctcgattcgatggagtacaaagtgcgtgagtcaggttcccgcgagcgtgtgtatcgtcagatgaaaacatctagcgatcatgcgatgctggattatcttaaccccattgtcgatatgattaacgagaagggaagttccacgttaggtctgtttactaccatgccgttacgcggtgtgatgaaggattcagacgtgcattgtgcttggcttatggagaaatcagcgatcaacttgttgctgcgccacactggcggcgatatgaagttgcagaactggttcctgccgtggactaatggctaacgagaaccgtttaccggcggtgcagaagggtgatttgtcgcagtgtatcatctgccagaaattcagtagatcgattcactaccatcacaccattccccgctcactgggtggcgaagatagtcttcaaatccctatagacggtgactgccacacaacgcttcacgcaaaagcagaagctgtggtagcgaagttagcaggtaaccgtaagcaaccaatcgggacgttttgggataaccctgagacagaacgacgagcacaaacgtggctagacattctagttgatgctatgcttaacccaccggtgcagcccggacagaaagaagtgctgctaccgatgatcaaggttgacatggaaactagacatgctctcgaactcttgaagcgcgacacgcctggcattactaatatgagccaagtgttgcgatattgtattgagacaacattaaaagcgaaggggttaaaaaatggcgaatcaaaaagtacgcactctggacatcaaagcactcgtaaaaaacgaactgacctgtggtgattgccgcggtctgactcgtgatgctcttttaccgactgcggagaaaccgtgtgctacgcaaggtcagttggctgattctaagatctgcaaacactatcgctcagacagccaatcgctgaccgagttgatgaccgagcatggtgattcacttgttgggcttttcaatacgttcaaaaacttcacagacaaagacctgcgcgttgtcgctggtatgttgttagctgaatcgaaaactcgccgccacggtgtgcgcatggggcaagcagtattcgtgcgctatcaagggcgcgagacacgcaactacctgaacaacttcatggcagcgcgtgtgttggatgtagacgacgatacgattcgcctgatcagtgagaagggtgacattgtgttgacgtatgcaaacacaggattcaatggtccgtccgtatatactaagaagcaatttgctaaactgcgtaaagagatgatcagtgctggcaagctgattgaccctgaacgcgagatcaagactgccaagcgcaatctcccgcaagaagacaacgttaacttctccgcaccgagcgacctcgatgggttctctattcctcttatggaagacgtggccaaaggccgtggcggtaagcgtaaaggtaagaagacccagacgttggtcgatattgtgagcatgatagaaagtggtcatgacatgggggcggagcaagacgagtccggcgtaatgtcactcggcggcaacagctatcgccacaagaagaagaaacttaacgtcggtaagaatggcgtggttgaacttggtgatatgtaagttaaggtctacacagcaaatatacttccaaaaacaatacgaataggatctcggaaaaaatgatcacaacagaagaatcaggccttaacgaatatctttcacgccgtctgggtatcgaggagaactcagaggaattccgtcaagtatacgctgcaacgatacgttacataggcagcggctataaatctatcgcggattatcaccgtgatttgcaagcagcaattgactttaagcagttcgaatttactgctcctgacttgcgtattgatatatcttccgtgtgtcgcttcacgttgaagatgcgttactttgtgttggctgtttgtctgcacaaagacccagtagcaacagttaaaaaatatgcgtcgtatggcctgtctcaccgcgaagctgtccttgcttggaacctgattctcaagcacgacaatcaacgtaagcagatgcgccgtacggctaaagcgcgagcgaagacaaaaggcggattggatatcacaatggtgtccagccgtgaactacgcttgcgtcttgatcaaacgactagcctgtttggtgagttgcatcgtaacgccaagcgtctggtcagaaagaatttgcagtgggtgtcggtcagccataacattccgattgctgatctgacttgcgatatcatgtgcaaggtgttgttgtcgtactatcaatccttgcctaatcgtttcagcgagggccaccagctcaactatcttcgtgcatcattgacgaaccgcattaacaacatgaacaactactacggcgcagagaagcgcaagcgtatgaagaaagttggagaagacaagtatgagattgtggttatgtctgacaatcagatgtggcacaatccagacgacgacagctccaactcatacgaagacatgttgggtgaggacgctcgtgtgcataccgagcagatggaaaacaatctgactatcaatcgtcttctggaagaggccgagggcactaagcgccacaaactgtatcagactgttctcggacgggattgcgccgagttcactgaatatctgcgtgagaacgggttactcaaacagaccatgacatgcgccactcagtggatcatggctaaacctacgaagttcatacgcaagaccttagccagttggttgcaggtcagcgttgacgctatcacaggcggtctggaaacgttacgcggttcattacaggtagcatgagaggtcaccgtatagttatgcagcaggcaatcattaacactgacgtagagcgctctgcactcgcgctgttcagtcgtcctcagttggatgaggactataagcgtaccgtgttgtatctcgtgtataagactgtaaatcgtaatggcatgatgcaagtcaatcgtctgctgttcgaattgagccagaagtatgaactcaacaaagaagatgtgaagtctgctatcggtgcgctcaaagctccgtacgcattcaacgcgctctctgtgtttgtacctcgcgcagatacaaaagcaaatcgtgtgtgtcgtgtgaactccacactggcaatcgaaagttggattgcagaagtggaacaaacccgtccacatatcgcacacttgttgcagtaggggcataaatggaa

SEQ ID NO: 2 - DNA, 262141 bp, unidentified
  source 1..262141: mol_type = genomic DNA
atggaaatgttttcgcttggcctggaagttcgggccattcgaacagtaacgaacccaaagattaaagaagcataccggacggccatgatgggtcgtctgggtccttctcactttagttcggaagtcactcgcaaggcattccgccgcataactaagctggtggaagtcaagagcgaaataattgaatgggacgacttgctggaagaccctaacctgagtgaggagttcagggatagtctgcgtgaagcagaagaaactccagcaaagaccatgaaaggctttgataagatctacgacagtctggagaagtatcgccagcgtcgtgacattatgaacctgggtaagatgattgccaaagacttcggggaagctgacccggaggagttcgacgagcatgagtatatgcagggtctggctgataagctcgggcaagcgcagcgtggcactcgaacgactgagaaggtttggacgtttggtggcaagaagtcgaacgcaacaaagttagcgaagcaggtaatcactaacccgaaagaagtgatgtacaagactggcttctcaagctacgacaagaagaacggcggctggccgacgactggcgtagtgttgttggccggttcgacgtctggcggtaagtctgtgctgtcaatgaacatcgcagatcgcatggcgaagatgaacggcatacactgtttgaaggtcactctcgaaatgaccgccgagcaggaaatgaagcgtatgctgtccatgatcagtggcatcgacttctggaagatcaagcagggcaagctgtcgaagcgtgagcagaaagaactgctgaaagctgcgaagaagtacgacaagatcatgagcaagtcgaagggacgtaactcgttcacttcacctgagcgtggcatgtcgattgatgacgttctgtatatgtcgattccgtatggcgtacacgtaacgttcattgactacgttggtctgcttgaaggtatcgacaacgacaaccagtggcgcgaactgtccaccgttgttcgtaaagcgaaagtacacgcgtctgctacaggtcagcttgttgttattctctgtcagttggatgaccagtctggtcgtattcgttattccggtggtatgcgtgaacacgccgacgtggtatgggcatggaactactctgaccctgagatccgtgaaggcaaaatcattcctgttcaggtaatgaaagcgcgtgatggtgaactgttcgagatgcctctgaaagacgtgtttgagaaaatgcgtgtcgaagatgctgacgagggcacagaggtaccgaagtcgaaagccatgtctgctgacgatatggaaggtggagattccaagaagaaattcggaaaaggtaatttcaagaagaaaggcgataagattgagattaagaagtctcgtcgtggtgctgctgcgttccttaattcaggtaacgatagcgatgacgatgatgacgacgacctgccgaagaaaaagaaaaagcgcaagtcctatgacgtagcttaggagtcttcatggacaatatcgaatggctcgtctttgatgatgaagcccgtaacaacatagacaaggattatgtctatcacgtccgcaccaaggagggtgcggagtacagtggtatgtacccgaacggtaatggcttccactgtcagaacccaggtgaaggtcgtaggactgatatgagtgatgttactcactattcggttcagatgacctttgacgatcatgccgaccagttcgtattcaaacgtgggtaagcaattcgaaggcccatacggacttgttgagtctgattcccttgtcccacgttggacgtaccctgttaagcatggacaggtgcgtcgtgtagaagcgtgggaactagataagttatcaaacaccacaacgcaagtgcgtatggtgaatgatatccatgcgattcacagcacgccagtagaggactacgatgatgacgcactcgacctcgacgaagaagccgcagcgctctcaaaaactgagtcccgacttcttatcaagcctcgactcaatgaagtcagagcccgtaagaacaaaaaccacgttggtccagaaaacgtcttcaccgtcgaaagtgaagtaattgacggtacgttggatagcgtcgatgaacacgctaagaccttccgtgactatttgctgcatcaggtattcagcccgatacttgggtttgatattgcggccggtgaagtggaagcgatctcgaaagactgtctcaaaacagacctagagattgatagcgagcttgtgccttatatcgagcgcgtagggcttgctaacatcatcggtgtgatgctctcaaagtctcaatcggtaccagagtcggtgcgcagtgatgtactgaaagactggctgatcaaatcgtttgacgatgtacgcgcagagcataaggcgaagacgggcaccaacacgttacgcgctcagatacgtcgattgatgcacggcaatgatgatatgattgctaaaggcgttggtataggaacaacgcgcggttacactgaacacaggaagaagcagaacgagaatggccaagcctaaaaagggcccagctttcactatacgtccaaaacgaatagctgcgtttgatgcgctgcttggtgatgacgtaaacgtgaaagcctcctctgacgatgaagattttctgtcagagaatagttcgagtgcgattagctttctcgaaaagggcgaggtcaacattgtcgatctcgttgaaggcgctttagaacaacgcacacttgtgccgcgtgacttgaagtttgatgacagtgcaatgcccaaggcgaaacacttccttgagtggtgtacgagtccagagttcttgaaagcagacccgtatctcgaacaggcccttattggccttcgtctattcggcgaaatttgtgtacgctgtagtcctaacttgcagtggatgtacacagagaatcatgagccacaagaaactacagccgcgattgagaagcacctgcacctgttacacaatggtgtgtgccctcattgcggcgctcgtcgttctgagatgattcgtaacggtgagatgaacttctataacgaactggcggtgaacgccggacagcgttgtgtgatagcgtcaactcctgttcttacttctcgtggcatcatgcccatcggtcacatgatgattggacacgacagtcctgggttccacaagccgcagcgtaacttcaatgcgcacaacggtcgtgagatcaagaacgtcagccaagtctatgtgtctgatgaagcacccaccaaagtcgttacgcttgcaaacggcatgtggattgaagcaactcatgagcaccccgtgcgcactgagcagggcttcaagaaagtgtccaagctgcgtggcggtgagcgtattgagattaagctcggtacaaactcgtggggcaagattcaacgtcctgtcagtatctatgatgctggtctgtctacccgtgaagaagcgttgcgttatatctccgaacgcagtgtgcctcttggcgagaagatgcagtacgttaccgaagacgttgacgcacttcaaatggtgtggtcgattcttatcaatgctggtcacatgccgcagatcgttcacggtacgcgtatgtggagcttggtgtatgacttgaccgagaagcctgagtgtcgttctgttcacgtcgaagtaatgtccgttgacgacggtactcctcaggtaacgtatgatttgcagatggaaggtctgcctcaattcgtagccagcggtatgctgcatcataacagcggtaagtccgttgtagtagcaatgatctcgacctatctgacgcacaggctgcttatgtcgcagtcgcctacaggcattctgagtatcgacaacacaaccgtactgcacggtacgttcgtcgcactgacacagaagcaagcggcagatacactctggactccatacttcaactacattatgggaagtccttggttccaagcataccacgatgtgattcgcaaacacgaacgccgttatggtatagaggtgatgaagattcgtgacacgttcgttctgtacggtcatcgtaactttgttatctaccctgctggaccagatggtcgtattcttcgtggtcgaacccgtgtgctggcggtaatcgacgaagtggcgtacttcgacaacgacgcccaatcgaagaagatcaaagtaagtgctggtgcggtgtatggtgcacttgaccgttcacttgcaaccgttcgcgctaaagaaaaacgccaggtcgaagctggttatgatgaagcgttcacaggttacttctgcaacatcagtagccctgtacacgcccgtgataaaatcaacgaactgcttcgtatgtcagttggttcgaagacgctgcttgggattcacgctcctacatggaagatgaacccagacatgccgcgtaactccgagttcctgctcgaagcgtttcgtcgtgaccctgtaggtgcagcccgagattatggagctgaggcaccgttgtctgcaaaccctttcatcacgcagcctacgtttatcgcagatgctattcgtgcgaaaggtcgttcgatgtgtacctatacccaccacatcattcgacacaaagatggcgaacgccagcgttatggcagtctcgtcaaagcggcaacgacaaccaaagcgtcgatacttgcaattgacgctggcttctcaaacaacagcttcgcactcgtcacagggtcacgcgatgatgcagggattatcagtgtcgattgtcttgtggagatcgtaccgaagccaggcataccgctcaactataccctcatatttgacgaactcctaattccgttgtgcaaagcgcgtaacgttcgcgtaatgctcgccgaccagtggcagtcactcaagctgctgcaagatgcgaaactgaaagtggattcaattgaggagtccgaccagtatagcctgaagtatcaggatatgtggactgtcaagacgatgttcgagtcaaacccgagtcgtatcagtctgccccgcatggttcatgcagagacgattgctgacacactgaaatacgacggcgacgaataccctcagtgcttcgagaacaaaccaacagagcacttgatcatgcagttgcagacggtacaagataccggacgcagcgtaatcaagaacacaggcgcaacagatgacctgtggcgagcaatggcactcatggtatatggctttgagtgtggtgagtatgacgagtatctgacgaaagccgcagaggtgactgttaaccgtgacccgaatcgcttgggccgcgtagcacatcgtcttaactcaggcactgccggaagctcacgtcctgcgctgacaggtggtcgagttcttggttctgctcgtacccgaatgattggccgtaaataagctaatttagtagagtacagtaatcacaaggaacaagatcatgagcaagcactataacccgttgctaaacaataactctgtaaagtcagagtctggagcaaactctgtggagagcacaagcggcgcatttgttgttgcgtctgctaacgtctgtcctaagtgtagctctactacagtgccgactaaactgctttccggtgaggacgtaatgttctgcaccggttgccgcgtaagtctcgcaatccctttagagtgaggtaacgatgggtattcaggttggtcgtcgtcaattgagcggcgcaccctcggagcctgcaaagaagaaacaaaattctctcggcgcagcctccttaccgcgcgagataggcaaagcgatccgcagtgagagttcacgtcgtcatacagacttcgtatctcaatctgcgggtggcgcaggaatggctgctggtaacatgcagattggttctgtacctctggatatcgacttagagccgatgatggaaggtatggactatgatgctgacgaccgacagctattcaatgtctaccgcgatatgtaccacttcgacccaatctgcggttcctacgtagacttgttctcaacgctgccattctccgacgtgagtttcagtggtgcgaaggacagtgtgcttgagccgtactacgaagtgaacgagcgtctgtcactcaccaccagcatgccgaacatcacaactgatattcaggttactggcgcgtttgttggcagtatgatctacaacaaagaccgtaagaagttcatcgacctgatgacgcaccgttacgacaacatcgacgtaacgcctctgccgtttatcagccaagacccgatgttcgagctgcgcattcctcagtacgtgaagtctgctttcgctaaagaaggtaaacgtattgacgcgctgaaaaaagaactcggctctggtttcgttgataagttgatgaacgacgtgacgatggaactcgaccctatcggcacaatctatattccacgtaagacgttcagctttggtgaaggtatctcggtgttacgccgtgtgctgccaatctggctgatcgaaaagaacctgtatcgtggaacgctgattgagtccggtcgtcgtcaacgcggtatcttacatgcccagctgggtgatggtgatcagtgggaaccgtcgcaagaagaaatggactttatgaccgaccttcttctgtctgcggatagtgacccgattggatctatcatcacaactcgtttgggcgtcaacatcagtgagttccgtcagggcggtgacttctggaagattacggatatctgggaccagactgcgcaattcaaaatgcgcgcgatgggaatcagtgaagcgttccttagtggtgaagcgaactatgactcaggtgctgctggcctgacgattttcgttgaagcgatgcgagccttccgtgatcatctgacgcgtaaagtctactatgagaaagtcttcccgcttatcagtatgatgaatggccttgctgttcagcgtaacggtaagatcatcaagaagaacaatctcatggaaggtggcctgaccgaagtaatgtacaaactgaatgacggctctaagctgtttattccgaacgtgcattggtctaagcaactgcgtcctgacgttgaccaagcgatgatggaaaacttacgtgcgatgactgagctgggtgttccagttccgttacgtgctatcgctgctgctggcgggtataacttcgaccagattcttatggatcaggatgaagacctcgcaatgcgccgtaagctgatggcctatcgcaaacgtcagtctgaaatcgacgctgagtttgctccgcctgagcctggtgctggtggggatggtgacagctttagttctgtcagtagcatgtctgctgatcgtgacctacagcgtcgccgccgccacatcgcgggcattggtctgtcgtctgctgttcttggtggtgagcaacgtaagctgcttaaccgtgacttcggtgagcgttctgaaatcttcgagatcggtaagaccggtaagaagaagcacgtcttccgtcagtcggtggcaaacagcaaagcgaatgatgctatctggaaagcctcaaagaactatgaagccaacaaaacgatgcctcttgataacggcaaggtatcattccagccgactcctcaggagcttcgtgcaatgtcgagacttcgttaatgtacaacgtgtcaacgtgttccattgacggcgaagaaaaggtggtggtatatcgccaccctatctttaccgattacgggataggcttgaagattgaccgtagtggcgaaatgacttccgttcagtgtaacattgttactggctccatagacggacagtctaagctggaggtcatcacggaccacacggcacctctcgaagtacaggtgtggtgttttacgtgtatgctgactctgcgggaatctgtaaatatgcagagcctatcattagatgccttattcccaaacaacgggggcatcgtatactacaaccaaaatcaggagagtacatcgtgagtggattattcccgcatcgcgttatcagtgagaaagaaggtttcgtattcatcgttcagcctgctgacgataacgatcctgatgccgtggacgcggcaaaagaggttgaagaagttctgaaagaagcgtggcctactgcgccgtcagaactgactgtcgctgacgtgacagaccccgaagaagccgaactgatctacgctgacgttgcgcaactgctggaagaagcagagcgtgaagaagcgaagcagatcgtaatcaccagcatcgttatcgttggcaatctggccatcgtcaactgtatgctgaccggcgaagatatggaagaagacgacgaagacgaagacgatgattccattgaagccgacgaagaagagttcgattaacgtctgccgtgaggaccttcgggtcctcatgaatctcgcagataccaacgttgcttatgcagcgaagttccttaccaacaagacagacgacgaagcacgtagtttgcttgctgcgctcaaaaatgaggaagtagaatcactgtacgacttcttggtgacgtaatggaaacaacatcattggacgaaagtcctaataacgcaaggcatcgcatcttttacaagcagccgaaacgagtacctcccttcgatacagctttcgttcgttcttccaacaaagaaggtctgaaagttctcctatcggctgctcctgaacattgtcagattattttgtttacggacggtcccggcgctgcttacgccatgaaacgcctctttaagcgcaacttcaaactctgttcgcaagctctccaacttgacctaagaactctcacgttcacaggtcaggtcgtttttcagttcgttcgtggtggtgcagtcgtcgatccactttctcgctacttctgtgctggcgaaagctatttgcatgagctggctcagacaacgaagattgctcaggttgatacagatacgattgatctattctgttgcggcctagggtttcatcgtgcgttacttgagcgtggtcgaggccgttctctcgtattcgcggaggaagaatgagtagatcgtttgccagtatcggaaggaattccgcacctggctcagtgccgaagatgaagatcaagtacggcaagctgccgatgcttcacattgttgatgcgtcgaactggatgtgccgtgcttacttcgccacgcagaaaagtcctacgtatgcaaaagatggtacgcctacgtatggtctgcgtcagtttatgtacatggcgaaagacctgattgacattgcggctaaagaccctaatggctcctacatagctttctgctttgacccaagcagtagcgaaacgtggcgctatcgtgctctccagcaatgggcctcagagcataagaagaaatacattcgacaggtgttcaagaagtctagcgactacaagggtaaccgcgaccgttctttgacccaagagcttggtccgcagatggctcttgctcgtgagatactgagcatggctggctactacgttgggctgaaacgtccatacgaatgcgatgaccttgtcggtacgttgagcgaccgctttaagcatgactatcttatcaagctgtactcgcgcgataaagactacgtgcaacttgttgaccacaagaacgtggagcttatcatgcaggcgcagtcgaatgctccagagcgtcgattcgatctcaaaacggcacagggcttctttggtgttccgccggaccgagttgttgatatgctcgcgctttctggagatagcgtcgataacgttcctgggattcctggacttggcgagaagacttctgccgagcttattcgcaagtggggcggtgcgttaggcatacgcgatgcgctgctcagtggtaagctgaaatcaaacgcaggttgggcgaaagcacttaccatgcagattccagcaatggatattgaattgcaaatggagcttgtaactatcgaccgcaacgttccgacgttacctcgtaaactcgaagcgttcgcaccaggcagacctgatataaaagcgttgaaagctactaagaaacgcttggctctgcctcaactattacacgtctagtagaggacagcatgacggaaaagattacgcagttggagaaatggtttgacgcggcgaaagtcgcgtttaagatgggcacacgcaatcctgccggtgacattgctctcgtactcagcattcacaagcgtctggcaaagaagctgaacgatgccaaagacgatgcagagcgcatcagtgcggaacgtgaactcaacgagtttcttgatgacttggctcaaccgtgtgttatgtacgagctgattcgcaagcgcttcaacaccgacctgtaccccaacattaagattggtgaagacgttaagatctatatcgcgcttatggcagaaacaccaggtagcgcagtaatggcaatgacgtacctgtatctcgctcgctgctatacgctgcaagatatggtagcgaacttcctcccgaatggctatcctgcctctgacgctctcggtcttacgtggagcattcagaaaggaaacagttctagcttcactggaaatctggtggatgatattgaaactgtaaatagcctgtacaataagatgtatagctcgggagagaagtaatggatttatctgcaatcggttacgccccgaagcagtttcgagtaatccccgttgagaagggcaatctcgttactgacttcattgaaggtaagtttcgcgttattggcgttgaatgtaacgctcgtggtgcttacggtagtcctatccaaaagagtattgcacgtcgcttccccgaagttgtgcgccacgtcgattcaatcgactatgagcacgaactgacaatcggtaagacgcacatggtacgtgttagcactcgtcatcgtcgcaatctgtttgtggctaacatgcacattgcgcgtggcttcggtctaggcctcaacggttctgctgagggttttcacaagcccatcaatcgtttcagtgagaagttcctgacgcgagcttttgaggacctgctggagcagtgtgcaaaagaaaacattgcaccagacaggcagattgcaatccaacgtttctacggcggattaggcggggtttcgtgggaagaagtatgtgcagttctggacgctatctgcgagaagcaccagttcaatatgtatgcctatctaccacgcaactacaacactaactttgtgcggggcgtcgctcaataactctgggggtgtattgatgaatacaatacgcggatttgattggctcttttacggagatggaaccgatagtggccaacactcaattttaagcgtcgttgttgaacaagcaacgaaatcagtgcaggtggaagtgaagccaggaatggcggtgcctgtaattcaagcgattcaggaaaatgaagtcctgtacgctcaaacggactctggcctgtatcgcattcgctatacttgttcgttccgttcactggatgctaacgcattcccgaaagacaaaacaaccttccgcttgaagctgattgcttgcgattttctggcggacgtaacaacgcacgataagctgtcggagtacgtgccatgatcactgtacagaaaattgaagcccgtttaaaaagactggactatactcggccctcaccttcgcgtgagatgcttgagggacttatgcaagacgggcgcactcgcattctcaagaagtctgagactgacttgtgtgccgactcagatcgctactttgagttttgtctttcacaggtcggctctttctgtactgccgcatacaatgctgtggagatcggtctgtctctcaacattcaaccaatctatattgcggctgctatcaatctgcatggcggcgactggcagtatcgctttcttgaattgaagcgtttcggcctgttagaccgtggcgataacactgtgtggcgttctgctgattcgtggtttgggttgggtgaagcacgtcgccgtttggtacacgctggtgcctcgtctgaaatctctaccggtcagtctattctgcgtatggccgtgcgtaagggtgatatggaaaagattcgtaagattgcagaaacgaatccgcatcgcatgatgtccattctcaacatccgcaaagagcctatgtacaatgaccctcgcactcttgccgcaaagaaagtgcgtgagaaagcgaaatcggatgctgcggctgcgggtaagaagctggtggagaaaggtgcgttcaacgatttgggtggcgtgttcaataaaacgatcacaaaagcagacccggcacgtcctcgcaccgctgatgagtacacaactgctggtggcagaaagtacaccatgtaggctacgatccaaggagaagattttgaaaatcgaatacatagttacgcagattgaaaagctcgtacacaatgagtacgataccgtcaataaatatagcggtatgacggctagcgaaatcgccaagacagaaggcaaacttatcttcattatgaacaatacatttgttcacgataagctcttgtgtctgcctgatgaccatcgtggagcttttcgtcctgtagagaatatggaaacattgcgcacgggtcttctcggacatgtgcataacatgcctatctacagtgactggatgcacgagccgcattcgagaaccggcgtcaaccgggagcctcgggtagctgttgttgatctggaaaccaacgcaatttttcgaattgaagcagagaaatttgtttgctgattttctgcgaacggtaatttcgacaggtcaaaacaaataacggaaacataatcatgagcaacgttgatacaacaatgcctgaaggtaagtgggagttcaatgagcaagttgctgctgtgtttgacaacatgctgcaaaactcaatcccatcttatgatcgtatgcgtgacctgacgtatcgtttaggtcgtcagtttgttacaccgggatcggccatcgttgatttaggtgcgagcctgggccgtgcgattgagcctttcgcaagagagttcggtcagtatcagtggcatcattgccctcactcggatgggcctgatacagagactggtaatcactacagcctgtacgagatcgctcctgcaatgcgtgagcgtttgatgactaacgagttgttgaacagcgtgaacgcaaagctggaaaaggaatctctggtcgatgtagacaccttccgctttagtggtcaagttgattgctcactgattctgagcgtgttgactctccagttcacccctatcgaacatcgccagcatattctggaaaaggtatatgactcgctacagaaaggcggcgcgttcatcctgattgagaaagtgctgggtgatgacaactacctggaccgtctgctggtaagcacgtactatcagatgaaaggcgataacggttactcgcaggaaagcattgcgacgaaacgtaagtcacttgaaggcgtactcgttcctgtgaaagccgcatggaacgaagaactgctgcgtaaagctggcttcgaccgcgtagagtgcttctaccgtgacctgaacttcgcaggttggattgcaatcaagtaaccgtgtgggtggcttcggctgcccactgcttttgagggaacaaccatggctaatgtacgccaagaacgctgcgcacgaatgatacgcgagtcactaatcgcagaaataaaaaaggctcgctctaaacgtccttacgtcttcctcagtggtggcgtagattcaaactgtattctgtttgctgcactggctgctggctgcaagccaatcacactgagcttccacatggaaggcgttaacagtcgtgacttccgtgctgcacaagctatcgctcaggagtttaatcttgagctgatcgaagtcgttcttcctaacagctatgagaagttgaagaaagatgtgctgctcatggcagagcgttatgcctgcattcagaagaacgaatttgaatgttcatggccgatgctctacagcttcttccacgttcgcaatcacgcggcagagaatggcatcaagaatcctgtgacgtttaccggacagggcgccgacctgatgtatctcagtagcaagaaggcgagcattcactataaagatcgtccagacgaatggcgtaaagaaggccgcgctaacccacatcgtactcagggccgtatcttacctgtgattgcgcgtgatgctggtgtgcgtaacatcaagccgtgggacagcgaagaaatcctggaagcgtttctcggcacaagctgggaagacgttaacaagcctcgtcagaaagagccgtctcgtatggctttcgaagaagacttcaaacgtattcgcgtatacaaccatcagaacttccaactcggtgacacaggcatcgcagagcattttgaaaagctgctggccgatcctgagatgaatcctgatcttaaatacaaaagcgtcgtcggtgtttacggtgagcttgcccgtaagtatcagggaatcgaatcatgattcatatcattgatggtggtgttggttgtgattacgtttctgaaaagctgcgtgacgctggaatcaactgtcgtactcatgcgccaaacaacccacgcgttcgcgctgcatacgcaccttatgcctcgctgtccatgggctttagcgtagaagaaattgagaagcatatcggtaacgtgcttggcacatatcgtggcctatttctgattagcagttacataggctcgctggtggcacgtagcatgattgaccaatgcggccaaagccataacatcatttactgcgatgacttcaagtgcggttctctgcctgtcgttgcttcttctatttctgtaaacacctataagaagcaacggcaactcggacgtattgctggacgcctcaaacactttgaccttgaccacgaatttattattgcagataaggcagtgcgatttgcggcaggctcagagtttgatgaacacgaagcgcgtagcgaactgaacaaccatgcgaagttcctgtcgagtccgtccatgattgttgcagcacacaaactcggtgtgcgtagcagcatgtatcataactatgcagggctggtgaaagagttcattgagaatcgccagtagcagtaacgagagggcacgatgattaatcgctttcagttaaaacgagttccagtgattgaagcctgtcagtggaacggagagaacgttgaggagatgaatcagtttctcaacggaggtggttacgttgtaggtcgttatgtccagattggtgtgacggacaaacagggtaacccaactctggctaacgtagcagtaggcaactacgcagtgaaagacgaagacggcaagtacggcgcaatcaccgcatcagagttgatggacctttacgtactggcggattgaggaacacatgaatcttttctctattttaaaacagcaagtgaagaaagcgctgtctaccgaagcgaaccacgaaccagaaattcgcgctttgtttgactggcgttactcagttgaaatcaaaggtcagatgtatatcgtcggcaagacaggagcaaacacctgcttctatatcgagccgggaacgtctgaacctatcgcctgttaccccgatgcgttactggacaagatcgaccaatggggttcaggcaagtacgtgtcgtatgcgatctacttcaaacgcttcgaaagccctgttgctgagaacatcaaaagtctcgaaaaggcaatgacaggtaaaccgaagacgtttaagaaaggttacttcatctgtggcgttacgccgaaaggcaagcgcgtcaagctctatcgtctgcaacagggattgagcggaatgcagtgggtagcagtggaacctaaaaagtaatcacggactgtccgtgtgaggagcaagtatgattagtgacattacagtcggccatatctataagtcacctagtgacagaccatttattgttgactgcattgctgcgcacggacaggattgctctctacctatggtcgtctatcgtaatcttgaaaagacgttagacaaaccggcaggtaccgtatgggtaatccctgagtcgttgttcacaatgcagttctctgagtatgaatgtggagaacatcatgaacacaacgaacttgtatcagcatctggcgtcaagggggttcgatccttctttttatcattgctgggtgagtgaaacacaaatgaccgtacctctgtttgcgtttgacagagcgatgcgtggtctacaggtctacacaccagatgcaccaaagcacgacgctaacccgaaagcgtgtcgttactttacgcgagcattcggcggcaagcagttggtgtggggatcggaaattaaacctgaacgggtcgaccgtattcttaactgagtctgtgttcaaggcatgtgcattgcatcgtcttggacttaacgcttggtctgttcttggttctgatgttagtgaccatctttatcgtcagttgcgtcttcttggtcttcggttcgtttgtctcggcgataacgatccggcaggacagaagtttagtcagacgtttgggctaggcgctgttagtcgtgaccttgatgaactgactgatgaggaacttctcgacctaactctaccattcgtaaggaagtaaaatggaaaacaaacacaagatcatcatccgcatcttaggtgatgtaggcagcggtaaatctgctgcgtattgtcgcattgcttcgatgctgaaagacagcggtgctacggtcattcacgccgacgagcaggcgtggaagatgttgcagaatgcgggcgaagctgaccgcgctcaggaagacctgtataccttctctccgcagatcactctcgaagaagcctgcattcgctctgatgctactctgtcgaaaaatcagatcatgcagtatttcgcatacgcccatctgcccgcccatctgcaacgtgttagcaagccgttcgcactgctggctcaagagatggatcagtatctgcctgacggtgctgagaaggctgcgggtctgcgcaaacttctcgaagcgaaagactgcgctgtccgtgcgttagtcgcaaaatgatcgtactgtgctttcgctgtctcaaaacatacgacattctgaaagcacctttgaccaagaccaaacggctgcgcgtcaaagagccagagtgtcctcattgtgggtgtagggtttacttctcataaggaggcaatcatgaacgattggttctacgactggtaataactcaaagggtggcctaatggctgcccttttctgatcttagacaagtaaaataagccattagggatagcgaataaccatgcgtaaggcatataaaaccatgtgtaggcagcgtagaaacaccacctttttcttgagcagtgggaagcgcttaaaatctgtaaatacagctcagataccaataactgcttctgagaagaataaaaatgagacctgagactattgctcgtacatataaagtcccaagccaaactttggagtccgttcacaacatctgtgagcgtcaaggcgtaaaactgtccgacgttgttcgtcgctatgttcaattcgtcgttcgcacccgcggtgagtttctgcgttccgcgcctcgtcctgagtcggctcagcttaacgtgcgtatgcctttcgacttggcgcattcgtttagtcatgtgtgcaaacaatctggatcaggcaccagcactactatgaccagtttcctgaatgagatagttcaactcaatcgtattcctgatgaactgttgcaggagaccgaagaagatgtgcgtgagtatatccgcaaagaacgtgctcgccttgatttactggaagctcaattcggaaaacaataatgacagtaataagtccaatccgctatcagggcaataagcgaagtcttatccctctcattctggagcacacaccttctgtgcaagattgtccacgtatggttgatgtgtttggaggcagcgctactgtgtgcgctaacatgcctcagaaatttcgtgtctacaacgaactgagtccgcaggtatttgaaatcgtcaagatgctagtcgaacaagacccgaagaaaacattgggtcaagtcaagcgtctggtaaaacattggtgcctgacaaacagcaacgaagaaaactacgatgcgtttcgtactgtcgtccaaaagaagcgaacgcctattctgcattacgtggcgcaccgacacgctcactcgaacatgctgcgctttaatcagcagggcatatataatgttggctttggcgaccgtggtctgattggcaagttcgacgaactggagcaagaactcactacgttccacagtcacatgcagggtgtccacctgacgaacatgaagtatggtaagttgttgagccgtcttggtagtcaactgaactgcaacacgttctgctatttcgacccgccgtatcttgcctcaggtgctatgcagtatggaaagtggacagaagcgaacgagcgcaacctgctggcaacgcttgagcaactgaatcgcttaggtgtgccgtggatgttgagcaacgttactgaacatcgacacttctcaaacgacttgttgaagcgttggctaaagaaacatgcaacgactgtgctctatccaaacaaaagctatgcgatgaacaacggccagagcggctcgcacggtaccgttgaaattctggcaatgaactactgaggtaatcatggaaccaccagtcggtacaaacatgaagttgtggagtattctcggctcaatcgttcgtgagcttgaaaagattaacgccactgcttggtacttgtcgaaagacccgaaagatacctgcggcgttatttgctgcgctatcccggattacacggacgccactctaatcaaagagattgagatgcgtgtcggtcagattgaagaacgcaaacgctacatcgctggtctgcaaaatggtgaagctggccatacctttgcttgtgagcaacgtgccgacgaactctaccagaagtattgcggcaagcgttaatctgtaaaacaataacataacaatcttttgactacacacagcaaggatataaaatgaaagagttcctgtctaagtatttcgatctggaagagtacgaccgttggccgctcgctctgcttttcgtgggcgctgtgtttgcaatcgcaagtgacttcctgtttgcctacgatgcagtctggccgatgttcgttgtcttcgcgctgtataccgtagcggtcattctcgatgtgcgcaacatcatggagtcaggcaacaccgcaccgtcgtggggctggctgttgttcattcctgtttatctgtggaagcgcgacactcttacgcaaaagaagaatcgcaacatcttctatgcgtggatgattctgtgcattctctcattcggcagtagttatctcgcaatgaaccgcgataaccacgagctggtggaacaggatgtgtgtcgtgtgctcgatacgattgactcattgcagtccaacaacatcacctgcgtccgtgcgtacaacatggaagagcagtatgacgggtactggaaaggcagtgcccatctgtccaataaccgcgacgttaatgtaagcgctgattacaacaaagataaagacagcgtgtacgttcaaattcatagcctgttaggagagtaacgtggaacaagaacaaaatcccctcgatatgcctgttcatatcgttaacggttttcaattccgagaagaatctgcaaagctgatggcttatgcgctggacatgaaacgtctcggtgctaacatcgacgcgaacttctgggacacgcgcattctcgacgacgaccagaatattgacatgattcaacgcctgtctactactggtcctgtgattaatcgccgtagtttcgacctgttcgaatctgctgaccgctgccgccgaaatgccgccgttgtgttcgaagcgcttatctacggctttgacctgatgatgcaggaattccgtgaagcgttcctcgaggagtccggcgtatcgccgtggattgatcgccacgataccaacatgttcagtcgtgaactgttgcaatatctgactcgtcctgcagaagaatcagacttactcgatgtgcccacgtatcgtcgtcaggcggctgtcctgtgtgacgttgaacctgtgctgcttacgctgcgtgtgcataacgaaattcagtacgtctggaacggtgagtggcgagcgctgacgaatgcgccaatcgaaacacgtcgccgtcaatgtgttaactggtactacaaccacgcgttcacaattcatcgtctgcgccacatgctgtcacgctatctgtaccacaaattccctgagcagttcggaggcaaaagtgcgtaacatcatcgctgtactgaaaatgcgttacatcgaacaactgcgtgacggctacgaagacggcccgattttcgatattgtttactttgacggcgaaacgaaagaagcaccgcattttgtgcgtactcgtattgccgatacgctgttcccaaacagtgtcgaagattccgctgttggtggttacgactatttggtgctgagtgtgcgtgaccacgacaacgatgttgaactcaagcctggtgactttgttgtgttccgtgaaaacagcagcttcacaactcttcgtggttttgatacagcagaggtgattgatggaaaactccgtcttagttgatctgcgtgggcgtctggtaaaggcggtcggcttgactgtggtgagcagcggccagtctgcctgttacgttgaccctgaaggtaaccctatgggtctggtgcgtgaatggcgtcctgagtcggcagagaatattctgctggtgatcgagcgttacggtctgtgtgttgaacgtacagttgaccctaaacataaaccacgtccgggcgaagaagataagattgtgtggcagtacaacgtgtggtcgcgcaatccaatctaccgaacgttgtccgtggataactttgctcgcagtcgtggtgcgcgcattgtcggacccgacttgaagacggccgtgtttacgtgggcagtgcttcgagccgagcgtgtcaaagaactgcgtgagtctaaagtggacgcgaagctctataacttcaatgtgctccaggagaaggtgtatgtatcaccagctcagtgataatccaagttccgatgaactacgccagtattatgagcaggtccacaaagaagccgaagaaatcatgcagcaggtgtgggcgcttcgcggttggactgttcgctgggaatggcataacggtatttgtgacgattgccagttcctgtttgacgcatcaggcaagtgtcttggtgagaaacatgcggctatcccacaagatgcaggcatggcaggcaagattgactcactcaagctgtctgtctctcataccaagaaatctgtaaagatcagtaacaagagcgctgataagccagttgagggaaaaggtcgtaatctaaggcttgcctacctcaactggttgctcaacattgaaaagcagaaagctgaggagaaaacgtgcgctgtcccttaaacgaattaccgatgaatctcgatcaggctgaacacattatggctagtgtgtttacgcttgccggttcctcgaagtccaaacgtcgtgccactgccgctatgctcgttcactttcatcacggcttcccgactgtcatcagtagcggtgtgaacggtacgcagcctggtgaaagcaacgttatggagaacgacgacctaacgctctcgctcgacactgttattcatgcggaggtgaactgcctcaatcgcatggaagaatacagcatgtgggctgacgagaaggacatcctgttctgtaccgattcgccgtgtcctaactgcttggctgatctcgaagccgaaggcgttaagactgtagtgtacgcgcgtgagtatcgtctgacggaacatctcgacgcatcgaagatcaagatgttctgtcttgatatgaagtctgtagaactccgtatgcttcgcggcatcgagcgcatgaaagaagtaatcgcaacaacaccagtgtctaactaagaccaataactgagaggctctcaacatggaaaacaaattcgaatcaggttttaaatgccaccctctaactaaagaacaacaggacgaggcgttccgtgcgttcgatagacagcaacaaaagtcgcttgagcgtcttgctcagatgattgaatctgattccgtgttgagggcccagcacgaagctgcccgtcgctatgaccatgagcagaagtttggtagcttggacttctctaaactcgaagacagggttatggctaatgctgtcatgggtcgcatgtcttcacctagcagcaacagcgaagaacgtgtagctggtacgtttgaacattcatctggtgtagttcgtggtgtagttcaacgctatccacgcatgtccgacaatctgcctcgtgatggtcgcattaaagttgaagtagtaccagggaaacgtatgctgcaaaccgatattcatctcggcgatgtgaagacagaagacctgtcgcttgctatggctgccgttgcattcggtcttagtggtgaacagcttggcgtcattcctgctccgggtggcggtcagttcgttgagccggaaacgaagttgagttacatcgacgaagctccatttattccaaatcatctgcctcagcactacctgcaatctgatacaggcccagtgcctgcgtgtggtcgtgctttgcgtatagctccgaaagattcatggtctgccgagcgccgtgaccgtgctgcgacgtctgcacctgctcgtaagaaactccgtgcccgtacacgcgcccagaagaaagcgcgtcgtaaacaacgctgaggtaacagcaatgagtaatgagattaaacaggcctcgatggagagctacaacgcgcttggcctgccgagtgattttatgaatctcgtatcagacgaagatgccgcagacttcgtggctaaactgtctgacgagaaacgccgtaagctgactgtcggtctggcgctgcttcatctgcaaattcctgatgcgattcgttatgagttgttgacgaaccacatcgacgaaactgagcgtctggttcacaatgcgttccaggacctgagcgcttcgctggtaaacaagctgtcgcatgaaggtagcgctgaaactaaatcaacactcggtagtgttcgtctggcaatgctgatgaacattctgggctttgatgatgctactcttagtggcgtcttgaacgaccctatcctgacacgccgcgcaagccttgttgctgtgactggcttgaatgagatgggtcagaaaatccaacaactgtacgacgagaaaaacaatgagccaacctaacgtagcaactcaatcagaagaaatggatctggatgcaatccctggtctggacccagatgcagtagcaccgaacggtgttgatgcagcagcatctgatgaaggttgtgaaggcggcgcctgcaaaatctaattcatggggcctagtgccccatttttcgtttgaggataaaaacgatgcaaacagcctatcgctgcaaacactgcaagtatgtccacatcggcaaagtgtccagttgtgattgtcagggcagtaagaaattcgaatatacgttggtgcaaatcatcgacgtgcccgagaacgaagaccaagtacctccgttcaaagatctcaaacactctcgcgctcaacgctacgtgaacgttaaagacggcacgtacggtaatggcatctatgaacttcgtgagaagcgtgatggtgagcgctactggtggacgcatctcggtactatgcagagcgggttcgatagcactgatatgccttaccagttctgcgaagacaatcgtaaggcgaatgttttactggctgccgctggtcctgttatgctcgaagcgctatacatggcgtatcagtatttccatctcaagcgtgaggttcagggcagttctattaagaacgatagccgactgtccatcatcgccgacgcgattcgtcagggtactgacctatctgtgttcgatacacttcaaatacctaaggaataaccatgttgattgatgcgttgaaagcaattcctgcgatcatactctgctatatagtgtggcgctatttcctgaacaagcgtgaccacgatcgtcatctgattaaggcgcaagagcattacaatcgtggccacctcgatcgtggtaacgcctggattcatttgaagacgggtcgtccttacaccgtgctgtggttgaccaacacgggtacgtctaaggcaggctgggaaatcaacgtcgtatacacgcatgacttccagcaaatatatagccgcccgttcagtgagttctgtcacaagtttcatcatattagtcgtggtgagaatgaacagcatttcgaagcgttgctagtgactgagcagatgctcaacaatactgaactacgtcttcctaaggaaggtgagatttggtttgaaggtactgtccatgcaacaccgccagaactggtgaagcagggtcatgcacctcaagtcgtgtctcaacgtcgtgcgcacattgatatggtactggctttaggtgaagcgcatccagtcgtcgtatttactgtaaatgaaaagcagacagcaatgttgctttcacagttcattttcatctatcgcaaagaggtgtccttcgatggaacaaccagctcttgtgtttaaatacgtgatgttcgtccgtacgcgcaccaaagagcgtgacgacggcgtttacttgcctgtgatattcccgacgcatatcatgcactctgatatgtcagacgaaatgcgcggctacggtatctccaacggttttcgggagaatcgctatcatcagcgtatcgatcccatctcggctggctttatcaatctgcgaacgcttctatgcttcggtgaatctgaatctctggaactgaaatctcgtccagaagatagcaccatcatcgcagagtatatgaagacccagggtaaaggcgcagaagctcctccagaggatgatgaatgatggacattctgagatcaatctgggctagccctttctgggacagtcctgcatctgcatttgtgcctacggcgcttattatcgcattctttatctacaccgaatggcgtgagcgtcgtactctgcgtctgtctcgtaaggcattcgcagacggctgggacccgaagaagaatactctcttccgccacaagtggttcccattcatgacttgtcgtgtggacttttattcgaatagcccgaatgataagttcacgccgtcagtgtttgtgcaaaggaatggtgggcgttatgtagagatgcctgcctatgtgttacgttaccgctataatgagattaaacaatgacaccagcaatcctctttagcgagcaggcctgtgaactgctgaaaaagatcttcggcaacaacaagcctttctttgttgtgcgccgcgacacaatcatcgaaaacgataagcagttcggtgagcgtgtgtatctggccaatggcgcgcatgtcattaccgtgcctaacgtacagggcctcgatctcggagataagctctatctcgcagaagacaatgaggtgtacgagtggcatcctcatttcgaccgccccaaatacgaagcaagcaacaatcaaaaggaagctctcgcttttggtcttcatcctatcgtccatcataaagacagccggaactcttaatgaacaatcaacctctcgatctgcgcgatcccaatcagtacgaactgtattctctgcattgcgtggatgaacagtacatcaatctcggcaatgcaattctgatgcacggtactgacgaaacagatcccggtcgtaccgaagacacgtggcgcactctgatcggtattggctttcaattgaccaacacgctgatcgctttccctgcgttgctatctgcgcgtaagaactggttcgcagccgttgatgaaatgtgctggatggctcgcggtgaaacaaatatcggcagtctcaattccaaaatctggaacgagtgggcggacgaagatggcgagtgcggtcctatctacggtctgatgtggcgcatgtggcctgatatcaaaaccttcccgactattgagtcgatgaaggagcgtcagattagcgatgctgaaatcgagcgtatctccaaagagatcaatcgcatgaaggccgctggttacactgaaacggaaatggctgacggccgtgtgtgctacgaaggtacaatcgatcagtttgctgatgctctgcgtcaggtaatgaatcgcagtcgctcacgtcgcatccgtgttcaggcatacaatccagcgtatctcaacatgcagggtctgccgccgtgccacactgagtttgagttcaatgtgactaagcctacgctgtatgaaacggctcagatggaagcacgtcagatggcgcctgccgaagactcgctgcacatcacggtgaccatgcgttccaacgacacgcttctgggcagaccgttcaacatcatcggctacagcgccatgcaccaaatgatcgcgaagtgggcaggcatgaacgtcggcagctttacgctgaatactaccaacacgcatctgtacactcaccacttcgaagcgttcaaaaagcaaagtgagcagtgggcagttctcgcagacaacatgaaacgcactggcgaacctgttgtctatcctatgctggaaatcagcgacgacattcttggcctgacgccggaagagttgcttgataacgccaatgctgaatggttccagcttctcgattatgcaccagcacaggcagtcaaaggacgggtgacaaagtgaacaacaacattcttctgatcaagcgcgtttcttcttacctgtatgtaggctattgcgaaaatgcaagtgacattccccgtcgtggtgttgagatgctggacattgttgtgccgagccctgtaagtggtgactcagacaacattctcgatatgaaagcgcgttgcatctatcatttgccacacaactgtttcctgctgcaacatgtagatggtgagttcgagggcaacgaatacccggcgtggacgaaaaagcattgtcgggataacatggaaatcttccagcgttcgtctcatggccgtgagcaggcagcgattgaactcatgctgaatgaactgcgtgatgcggaagttgagcatccggaatggccggaagaagcaattcatgcaggctccattctcgtggaagaagcgggtgagttgctgcgcgattgcgtgtccttcgatgaaacaggtgacgataagctgatcgttaatatgcagatcgaagccgtacagacaggtgcaatggcattgcgcttcctgaaaaatctgtccacgtcgcagaagcgcactatcccgcataatgctctgcgtactatcttaaactcagagatgactccggaagagcaactggcggagatgcgtcgtcttatcgatcacggagtacgctaatgcgtttactaaagtatatcccaagtgcaggcatcacgcacacgccaccagccggcggtgagtatgttcgtgatatggtaatcgactttggcgatcatccgaagcctgacgtaggtcaccatgatgaactctgtctgttcgatctgcgtctgaccaatgtggatgtgtatcacgaacaagatagcgtccacatctgcctgcctgacatgagccacatctacgccaacttcgatatggagatctgccgctcgcaggagtatcagttctggatgggtgacaacgctcatgctccttctgctgatgctatcgttcacgcacatatcgttaaaggtcatcttcctaatctgcacaaagacttcgatgcgtttgtcgaatggctgtttgatcgtatgcgtgaaattcctcgtctcaacatcgatcacatggtgctgaaaggcaaaggtcaaatgtacgatgcaaataccaaaaactcgtatgacctttggggcatgttccgctactggttgatgctgggtcgtaatctgactatcgggtattcgctcgacaatcagataacgctcaacgatacacacatctctgagaagggtgtgcgctggtggttgattgagcacaacaaacaactgatggaagtcgcgcgtgagaacgatctgctggctgcattcatcacgtttggctccgatagccctggctctgaggacgagtatgcgtatacgttcgttggcaaagaaggcaacttcatgcgcagccacgtagacgttagcgagttcatgcacctcgctgttcacggccacttccctgaactggtctgcgattcgagcggcaagaacttcaacgtgacgtttaacttcgcgcagtatttcccggaagagtatcacgcgtaccaaaactatcgcggcggtgattaccatcgcgctctgtctcgcttcgtctgacgggcttcggcctcctgtcagtaatttgattgtctaacaggagagccgacatgaactacgatccaaagaaagatttccacccgtttcaatatctgggcgcacctaaagtcccgcacacaggcttcttaggtaatacagtgaacttggttgagaacgacgtaaacatcggcagcgatgaatgcacgttcgagttcactgtagctcagatgaacgcgatggacagaggtactgttacgttcagggcgaaagactctggcggtggtatcgacattaagaaatgctcagtctcaggtttgaaaatggtaattaagctggacagaagggtgatcgagttcggcaaagttcaagtcgaatggcagactactcctcgccactactattactgaatctgtaaagacagagaaagagcaaccgataagagatacgacaatggcaaaaactgctatcaaaacaaaggacggaaagaagaaaaagaatgatgggctaaagttcgagttgaataaactcagctccgtcaatcaattaaaaggcgcagcgtataacccgcgtttcattacagacagtcgcctgaaagcactcgaaggttctttgggtagcttcggcgacttgtctggtatcgtgttcaacaacaacatcaaatctggtgtgttgatctcaggccaccagcgcttgaagtcaatcgaaggctggaagactcgtatcgaggtccagaagtctgttgataagcacggcactatcggcctgggttatattcacgcaacgcatccgaagaagtctgataaggtgatcagcattcctctgcgtatcgtgaactggaccgataagaaagcagagtacgctgcaaacatcgcggcgaacgcccacggaggtgagttcgataacaagaaactcgccaagctggttgagcaactcgacctcaacacaatcaagccgcagttgcttggccttgacccgttagagattcgcggtctgcaagccaagctgaaagttcaggctgttgttcaggacgagaaacgtgctggcaagacaactggccagatgaacggcagtaccggtaagttcaatgagtacaaccctgatgatgtgggtgaagctctgaactgcacctgcccgcgttgtggattcaagttcgagggataatatgatcatcaagccgcctactatgaaggaaatcaacaagctggataaaccctggcgtggtatgagtttcttcgcaggttgcggtgggtcttcgaccggtcacaagatggccggtatcgacattgtgttgagcaacgagtttgttgactcagcacgagagtcctacgaagcgaaccatccgacaactaaagtgctgcctcatgacattcgccgcttagacccaggcaagctgttgcgcttcgctggtctgaacaaaggcgaactggatttacttgacggtagtcctccttgcttcaccgaagacacgatcattcatacagcagacggcatgaagttcatttcggacatgaacgtcggcgatagagcaatgaccagtgtcgggcagtatcatcccgtgtacgacacgatggtgcgaccttacgtcggcacgatgcacaaaatcgaaacactgatcagtagcaacaaagcaacgcctgagcacccgttctttatcagacgtccacttgcggcgggcggttactctgaaccattctggtgtgacgctaaagacgtgcaggaaggtgatctgctcggtacacctcgtgttacgcctgaccagcctgctgatgtgtaccacaatcagatgaatcaattgccgaagatgattcgtcagtgggtaagcattcctgagttctggtggatggtcggtcactggtgtgatcgtggttcaatcgaaactatcggtggcattgaagcagttagcttcgagtcgcataccagtattgaaaacgcgatgattgagcaggcgtttgacgcgcttaaactcagcagcctgaatcgcatcgaaacaatgacagcgcaacgtagaacgttccgtactgttattgatgttgagctggtgcagtttctgcgccgctttatcagtcacggcaacaacacgttctctcgtcgtctgcctgccatgttgttccacatcaacgcggaactgaaacagcaattcattctgggctgtgctggcatggattatgtgactgctatgggcacaggcattgctatcacttctgcaagcaagcgcttcctgcttgaactgaattacctgtgctgctctgcattcaatcgtcctttgtttgacggactgacttggggcgacctgtatttcggtagttcgttaacgcctcgtgaacgtaacagtgcgcgtgagcatatcggctacctgttcttgcaggacgagcacaacttcttccatgagttcagcaaagaagacccgcatctctggacagaagtgattgagaacctcgcgtatcaagcaacctgtgacgtctataacttctctgtcgaagtggacgagacttatgtggcgaacggtgttgttgttcacaactgcaaaggcttctctactgctggcgtgaaagaagaaggctggggcaaagaagttaagtacagcgataacaagtatcagcaggttgatgacctgttcgatcagtattgtcgtatgttgaaaggcatgatgccgaaagtgttcactgcggaaaacgttagtggtcttgttaagggtgcctcgaaaggttacttccttgagatcatgcgaacgtttgacgagattggctattacgtccgagcgccgctgcttaatgctgcatggcttggtgtgcctcagtctcgtgagcgtatcatctttatgggtgtgcgcaaagacgtagcacacgctctcggctataagagcaatcaggctgctgtgcctgatgtagtgccgtgcgatacaatggccttccttgcagatgccctgcctcacattcagcggtataagtccacgaagaaggatatcatcacataccttcctgcgatgaacggaccgatgccgacgatcactgcggctgatgctatcgcgtatgagacagcccgtttctcgtctgctgggttcgtcgaggacaacaaaggtcatcgtcgtaagttgaccatcgacgaactgaaagttgtttccggcctgccgtcagactataaactgaaaggcaagtttgaagaacagtgggagcgactcggtcgtatctgtgttccggcaatgacacaggctgcgtcgaaagctcttatcgaacacgtcctgctgccttatgctaagaagcgtaagaagaagcctggcgaaatctttaagtaagggcgtctatgttctacgtaggattgggtttgggtatcgtgataggcatcatcctcacgctattctgtctgtggtttttcttcttgaaggacttcgcggtattcaggccgtgatacaacaggacaaggaagtcctggagaattgaaatgtcttattgtttagttcgtgcaatgatggtcgcccacgtgcaggatggccaactggtttgttctaagtataagatcaaactcagtgcgagtaactccacccaagtgcataacttcatgcaccgcattttctttgagttcaatggtcgcatcttattagaagatgaacaagaccgcgatgctctgccgacgctcaactatcgtaagcaggctaaagtcctcgaaggtaatggcagcgtattcagccgcattactcagcttggccagaagcacggcatcacttgtcatctggtgaacgcgtttaagtcgcgtctggacgaactggcttacgtgttctatctggtgcagcctactggcgttgcatgtcaggtgctcgataccgacaaagaagaactctggggcaagacgctgctagtgggcgctgattctgatgttgattacgcaggccgcaacgttgtgccagtcttctgcgacgaaaactgcaatgttgacgacaaggtgctggggaacgaactgttctctctgtacgacgacaccagtaagctcatggtgatggtcgacaagtaaaatgatacgctacctgataatattcatcgctacatggatgctggtagcgtactcattatcgacactggatgtttcgcctgtgtggtgtgaaagagtaggcatagtatctgccgccatcatcactcacatcgaaatcaaatggcagcgctttatacgagaacactcctgatggacgaactcgataaatttgatcttgaaattttaaacaattttggctatgagatcgttaacggctatgttcgccaagtgtatagtgacggacaaagggaatcgttagtctttcaccttaacgagattcgccgagtagaaatccaaaacgtgccagtcatacgcaaagacggatcgttcgatagaggatatcgaatgtatatcacgctcgccagcgcatggtacgtctggactgtccctctcccaccttcccgtgaggacgaaattcgagcactggttcaagcatttttaagaatgcgagatattgcgcttggatttgaccctgacgtgaagtaccttattcgagtagaaacgaagtcactcgatagctcgccagtagttaactggtaatctgaaatggtgtgcggcacaaacgtgactgcaccctctacctaaaaggtatgtactatgtctaagaaacacacgtcttataccagcgctttcgcaatcggtgaaatggctgttctgtctcttgatcgtttcggtcaaaacaaagtgccgtatggcgttgttgaaggctgcatgatttatggcgaccagcgcatgtatcgcgtatcgctgtttgtgaacgacggtcctgctaatcaaccgtcagcatttctgcatcaaggtcgccctgttgatggcttccttgcagatgatctgaaagctatcaccgactatcagtatgcagaccacatcgggcacatcggtcgtttcgaagatccgaagcacgaagtgattggcgactctaagttcaaagtcggccagctggtggaggttgatgttgacctcgaacgcgaaggcgagtacgacaagttcaacatccctgtgatgattacgggtgtgcgctatgaagaaggcaagattttgtacgacgtaagcattcaacgtgcgtactacgaagacggccgtattactggtggtcgtttggtgcgcgatactctcaccaatattgatagcgtcttcatcaaacctgccggcggctggcctgagactgttgttaatctcgaaggcgataacggtcagtctgttattgtgaagggtggttctgtcacaatcaatagtcctaagatcacgctggacggcgaggagctgaatgttctcacggcagatacggcgcctgaagaagaaaaagttctgctcctcaatgatctgtttgacgctgcatacgaggcacacctcaatggtgtgtcgtgtggtgaaaacaacaaggaggcggcgcgtaacttccttgctcagtatattcgtgaacaagataagctgctgcaaaaattccgcgctgtcggttctgcgactggccgtatctctggtcgtgtagaaaatacgagcgctaaacctcgctcagagtaactaatgtgggtggcttcggccgcccatttttgtatctataatctgtaaatatcagacaggagggtaacatggataaagataaacttagtgtcagagagttgaccgactatgttgtcaaacgcgttaatgaaaatgccagtgcgactctgactgacattgatgaagatgcgtggcgtagtcatgcgcgtgatgtggttgagggtgtcatgcgttcatgcgccgagcgttctgagatgggtgttcgtgttgtatgtgacgactcaaacaatcctcaatacaacatcgacaataacattctgtccattgatgtgattatcaatgacccgacagtccttcgtaaacttcgcataggaaacgacaatgctaaaacgtctgtttgcgttcttgttcagaaagaagaaaacgctaccgatcaaaaagacctttgagcaaaagctcgatagtctaagcgatcagattcgtcaggacgacgaacatctgcgccgtgtattgcacactggtcatcagcctgtgcgcaagaaagagcgcgtcactgttacagtagagccgccaaagaaacgctatcagactacaccgacgcctatgcctgagcgcaagaacttcaatgggcagcctcgtcgtggcatgacagtcaatcaggcgtcttccagtcgtgctcagacagacgatttaatgctggcggtgatgatgcagcagacctacgttgcacccacaccaagtcgttcgcacgatgatagctgtcgcgtagaccatacgccaagctatcgtcacagcgatcctgacccaagcccgtcctacgagggcggttctgattctggttacagcggaggtagtggttgtgattaaacgtctaatgaactggataggcttgatgcttatctcagacgcaaacaagcgtaagctccgtcaacacgaagcaatgatgcgcgcctgtaccgatgtatacgattggtgcggtgctgacttgcctcagacggcagaagctgttgagtacgttcgcacacgcgcattaggttatgagaaccgattgaacgtccacaacggtaaaatcatgacgccatacgaagcgcacaccggcatcagcaactggcgtgacgctatgcgccgtaagtatctgcatagcgaagtgaactttgacggcaaggcgttcgcagcaccaaaggcagattctgtaaactaaaaacacgaacaacatataccgagaaaaatatggaacgtaactcagacgaaaagattgtggtactggacgtagatgtgtaccgcaccctcgtacaatacgcagaatgcggtgaacgcgactgcgggcctaacttctttggaaaatccgtgaaagaactcgaaaaacatgcacggcactttaatccacatctacgcgcaccgtttgagcagatgttgactaacgagcgcttgggtaaagctgaacgtcgtcggctggtgaagaaagcacgtcgccttagttcgcagcgtgagcctgtacgcttcctcgttgaccatcagcacaaggtaatctatccgattatcattactggtgtgtcgtctgacaatcaactgcgtttgaagtatcacgcactgtctgacggctgggattcggctgctatggttgatcgcatcttcgaaacaccagaagaactgcctcagtcctatcgtatgctcaaggaaggggagaatgtctgatgaaagcactgtctattcgtcaaccgtgggcttggctgattaccaaaggtcataagaagattgagaaccgtacgtgggacacaaagaaacgtggacgctttctcattcatgcgagttcgaaacgtcctagtgacgacgacatgcgtgtggccaaagagatctgcgacggcctgaacatcaagctgcctgagaagcatgagttcgagctgggagctatcgtgggctatgctactctgtgtggtacgacaacgcaatctgacgacccgttcttcttcgggcctgttggtctgcaactgaaagactgtcgtgataccgagcctgttcgttgtaaaggcgctctcagtttctttaacacaccgtactgtgtcgtaggcggtaaagtgattcagtcaccgcgatgaggcccatactggttgttcatggaggcaaagttctgcccgctcaactggtaaatgaagatcgtaaagacgtgtactttgttcggcacatgacgatcagaggacaaaacgtgtacgtcgcaggattggcaccagttgctactgttgtgtttctctatggctactcgcctactgttgatgactatgaagttgtaaaacagatgcgaggcaagtaaatcaagggtggcctaacggctgcccttttcgcgtttaaggagcgttatgttaccgtttgcacctaagacccgcgtagtcagtatgcgtaacggcaataaggactacgatgttcgtattgatcgtgagactaagtggggtaacaagttctatatgaccaaagagactgtggccgaacgtgaccgtgtgtgcgatgaacatgagatagacctgtggttaaaaatctacagtggtgagatacgcataggtcatttgcttgaactctacggtaaacgtcttggatgctggtgtagtccaaagcgctgtcacggagacgcgttagctagagcggctgagtgggcatacaatgcaaactgtaaatgggaacgtataaaagccacttacaggaagcgtcgtcgtgcagcaaacaaagccaatagcaagaaaggtaggaagaaagttcctcggaagtagcccgtcgatgaaggctatgaattgggaagtgtatatcagtgcattcagcggcagagcttacggccagttcgctgttgcatggggcgcttctcacatggtgattcatacgctcgatgttaccgagtgtgtacgcaataactgcgaccagttatacatcgacaaactggacaagatcattgagtgcctaaatgcgttcaatggtctgcttggtacgaccaacatcggtcattgtcgagagtggctgaatcctattgagacaggcgctacaggcagtgtggcgttctgccactacgtcactgacaaagaagccaacatctatttcgagctggcgtcctgcaccgagaaaattcgcttctacccagcaccggcaggcaaacataagctgcgtaatctgaaaaccagccttgttcgtttagagcaggagctggtcaaacacagacaggctatgcttgataccatgagtgtggtcaacgaaacacgcgctatgctaaatctgtaaatatagcgtataccacatatacctagaataaggaacttggcatggccatgactcaaacgcagtacgctctttctaaggtggcagaagaagctaccgagatcgcaaaagagtgccacaagatcatgcacttcgggtttaactcatttgacccgaatgacccaaagcgcgttaagaacattgaccgcctgattgctgaactgcatgatctcgaaggcgctctcctgtttctgcgtgataactcgggcggtgagttcgagtttatcccagatacatgcactgcgttggctaagtacgataagattgcgcggcacatgggctacgcgattgagtctggtaatgttgaacctttcgatttagaagacgaggatgaataatgagttactctttcgttgttgagtggaacatccgcttaaaggccgatacgcctaaagaagttatgagcatgttgaaagcgtggcacaagcacccgcatcgcttcgacgcgtttttgaatctcggtgttgacgttagtgcagcattgggttgtggtctgggttcaatcgcaggtatttactacgagagtaacttcattcacggctccggcgtcgttccgtatatccgcacctgcgccaacttcacgcgacgtagctcaggcactgatcgtctggttggtttcatcaactggctggagccatatatcgatcatcgtgatgaagtcatcggcatcgttcgcggcgaagacgatctctattgctacgacgatacgcgtggctatggcttcggccttattcctgagccgcatccaagcaaaacgttctacgaaattcgtatcatcaacaaccgcgcacaaatcgaatataagcgtggtgatcttcataacctttatccgtgggtatcttatgcttactaacattgctcgtctcgttgctacacaggcacactctggtcaggtacgcaagtacaataacgaaccgtacatcaatcacccgctgcgtgttgcacagtggctgtctcagtttaacgttggtgaactgatcgaagcaggcgcaatctgtcacgatgttctcgaagataccgacgtcggctatagcgctctggaactcactgtcggtacacctgttgctgacctcgttcgggaagttactaacggcgtctatccggcaggcacttctcgcgttcagaagtactggggtaatatctccaagctactgaccgccagtcatcaggcgcaaacgctcaagtgcggtgatgtgtatgacaactgcaaagacgtgtacgatctggacccgtcgtatgcagcgcgttacatcgccgagaagttcttcctcgtgcgtctgtttactcgcgctcagtctgacgtgcgcaacgcaacgttgaacctactgtcgtctgtatacaacggcatgtctgacgggcaccgcatctactgtctggattacatgcagcaactcgaacgtgagtgtccggacgaactgttgattcacttccacaacgcgctggtagaagccaacgaacacaatggctgtactctgcgtatcggagatgcgtatggaactgaaactgcctccgtttaaaactcgcagcgtactggtagagaacatggaagttcgaaacaaacacgccacagccgttgttgccgtcagtgaaacaagctggtggggttatcgcaaacgtaacctgcgcgttgcaatgaagtgcgacaagatcactcgtaaggagatcgagtggtcggctctggtcaaatgggatgatggctatattgttgctcccatctgcaaagacagcgacgtccttacagtcgcaaacaacacactccgcgatatgcgcaacatgaacttgcagcgttatgagcaactgcttgcgcatcgcctgaccattcacatgaggaaacatcatggccgcacatgcagtttatctgtttgagaacgtggaagatgaagttgctttcaccgaacgccgctttcataaaagcattcttttcatgaagggcatcaataaaaacttgcctatggtggaagaaagcaaagaagtaacgttcgccgtatacgaagtgggtgacaccaaaacgtatgctgcaactgtcggtcagcctcttcctgaaaatctgcgtctggcactgaacctcgaaccggttcgtatgtggcgtctgattcgacgtaaagacgatgtgttctttgtcggtgaaaactcagaagctatcgttgcagatagcgtggtgcctatggagattcgtgttgaaggagcgcaggatgcagaacgttgctggtcacgcgcttgaactaacagcgaaggacgttgaggcttattggcggggacgtgcgtatattgaagcggctcgtattgcgcacaaccatcaggaagacccgactgcgtacactctgacctttcagctcattgagccgtatcttcctcaaggctgggaagttgtcaacccaatacgtgagcagcacgaaggtgaattgcctgatgccgtgtttgagccaggtgaaacccttgagccacgatttgtcgttatgcttgcgctgatgatcgatagcgataagactcatgtgggaggcaagacaataaagtctatggcgcacctgtcttctgttgcgcgtgacaaacgaatcgtgttggtgcttaacggtcacgacacagcacttgcgcggcatcttgcgcttgaagctgggtacgaagtgagtgaagcaggtctgattgatatggccaaagctatcggcgataaagctatgcgccgtgctgaacacactggcttctttgaacttgatactccacgcgagcgcaaagagcgtgacccgaatctcgacgctgtacgacacaagcacaatcgtgttggtcgccactcaggcaatcaacgatttaatgccaagccgcagcgtcagaatttcaaaggccgtggccgatgaaaaacgaaacatatgcgattgagtatgtggacaacgtaccactgcgcgtccatatctttcggccagaggcaagccccgagcaaagtgattatcaggctctggtaagcattgacgcgttcgataagcgtatgtgccttgcctgcaagaaagacccagcagttcgtcgcttctggcttcaacgtaagcacgaatgggaacatctcgtggagtctgatcgacgcatgatgcgtttgagaatgtctcctacattcatcaatcttccaaagcagatacacgaagacctctggacgttctaccgtgaagtcggctgggactataaaagcaaacgattcatttgaccaaaaatccactatctctgccgctgtctgctgtttgcattcttgcggtatcgacgcgcacgggagtctttctcgatgtgcttaataatgaaaagacaccagtaggccaatgtatcagtcgtgttgtagatgctgtccttgctgaggggagttcttatggacttgaaagactggttgatcacaacggagacaatcgtccacaagatggttgttgaccccgttgagggtacggctgctgggctagtcgaaactgtttactacggaccgaaacgtcttggtcgtcgtcgcattcagggcattagtcgttcgtgcatctgccacgatatttatcgtcgtcaggcagtttggatggacgtcaacggcatggacgaactactgccaaagtacaacacggccaagtcattgtgtcgtagactacgcacagaaatcaataaactcgtagcagagggtaaagtaaatggtgagtccattagcaaaaatcaacatcggcagcccattgcctgatagcggcgatctgatctacaaacagattcttgatggtagcattgagattctggacagcacactcgatctgcatcggcagagcaatgtggtgctgcgtaacaccaaagagctgggtattgatatactcaatggcgtctggacttatactcctaagtacacgtatgaaaacagacaccctctggcgtatacgttcggtcaaatgatggctgatccaaacagcacgtatcaggacctggcgaaggagcttacaaccaaagcggagcaagatatgttctacgcgccgctgcgcaagctccgtgcgttcataatcaaccatgatacagttactggtaaaactgatttgcgtatgccggacgcgtggatcgtaaacatcgacgctgcgctgacaatgcgtgacttcatgggcgtagttgaaggctacgttcaatctaagcagcgtcaggaagttgcggatgttgtctttgagaagtattacgccacaggcgaaagtacaaagaactccaaggcgcgcctgttgttcagtggtggtacgttagttatggtcgacccggatcgccatatagctgggactgccaatatgttcgatatgacgccaatcttcaagttcgtgtcgcgtccgtggaatcacggcctgacgcagaatcatctccgtacctatcgcaagttagtaaatctgtaaatactaactgctaaagttactctatcttattcagactatctttcaactaacataaggaaacaagcatggcttctaaagaacgtgcgggcgttgtggacaattctgctaagtccgctaaatctggtggcagcgcgggtaaacgtgttactgctccgatctacaacggcacccaaacttctgcgcatgtcgcatccgctgcatctacttctgtgctgcctgtctctggcgtgtctctcgctgcgcaaatctacagccgcgcggacagtctgcgttacgccacttctgagttatctgaaacgttgcagcgcctgggcctgtacgaaccggctccttcgaaaggtgaagatctggcaagcgctgcccacgataacgtgcttcgtgttatcaacgaagaactcaacggcgcgatgcgtttcgccaacaacgttctgttctcgtctgttcacggcgacgatgaagaagaaatcggcgaagactgcgacactgaaaaagaaacccagggcgctatccacaaaacgcagttcggccgcagtatttacggtgacgcacaggcagccatctcgcgtctgctgagtattcagagcctggccaatcgtgtcaatctgtctctggttggcgttgaaggccctgctgactgtcgtgctgctcaggtgaacgatagcgttcatggctgcctgtgcaatctggccgatcacatcgacgacaccgtcactactctgcatcgcgttaatgcagacctgatgaccaacctgttgggagttaacgggcaatgatcgacttcaaatctgttaagtttgacgaagaccgtaagccgtacatcgttgaacgcggcgctaagggtaagttccagcgccgttatctgactgacgcagaacagcaggagcacaaagagtgggacgccaagcgtgttagcaaactgaacgcagccgctgttcgtccggctcgtggccagactgaatctttccagcacgtcgatactgtcggtactgatcgtgcctcagcacgtaactctactctgcgtactggctacggtttagctgacggtcctaccggtcctgttggtccgggaccatgtcctgtcggcgctgaccctctgattccgtattctctggaaagtggctctgatcaggacgtcccggtcggccagcgcgtagctcgtcgctctgttaacctgatggacagcattgcgcatctgacgctggctctgtatgagttcggcgctatcgacaatgcgtgtgttgctgatgttcgttcgcgcgtcatggaccttgcagaaggtcttcatgaagacgaagactgtatgcgcattcaggcagaagacgagctggtggagccttactactacgttaagtctatggctgcgctgctgcacggttcgtatactcagtcgcgtactcaggctccgttgaaagttgttggctatcatgctgctccggttattactctgacgcagtacctgatgggtcttgtcttccctgaaggcgatatggcacgtcgtgctcagaccggtaacctgctgcgtcgcggtgacgaatccgtgcgtgatctggcgctggacattatgaccgtgtacaacaacattcaggctgacattagcgaagctggtattcgtttgctgggtgagatgccggaagaaatcggcgggttgaatgtaggtctgggtgagctggcgtctctggacgtcgttcgcgccgttgacgaaatgctggagtatctggtgattcgtattgacggcctgacgcagatgctgcgcgaccaactgtaatctgctgtagaaagcaaaaagggcgactctcaatcacgagggccgccctttttcgttatagcgctaaacctatgccgatagctgctgcaatgcgagtcaaccacaattgaaaatccgcagacttctgatcttcaatacgcgccttacgctctgctgctaaatcatcggatagtccattcgctctcacctcttcggcttgagccaaacgcaatagcttgttgcgttcatcaatggtcagattgagcacatcgagtaacttgtttcgttcctcggtgcggtctttccctgactgatacagattaatcaaatcaaccattcccttgttatcaagcactgcaaccttcttgtcttctaccactttgatagtgacagtaggcttgtcaggaacggcttccttttcccactcaactttgttgatctgctgaatatcttgcatggttgttttcttggttgcgtcgataccagataacgaactgcaaccagtcactagcaagcacaggagtaacgtgattattttcatagcttattgtacctgtccaccagctcgtccatgctgtcatctttacttggaggcttaacgtcagtctcaggcttccgcgtattcagatctttcaccgcatcgttaacagtcttgctgtcttggacttggttctcgattgctgcctcacgcgtattgtcagcggctttctgctcacctgtagtagtcgatgggcttgcctttgggcgacggaacaacagcgccgttacgacgagcacaacaacagatgcgaaaaccttccagtatttcataaacacttcaatagccttagacataatcacgctctccactattctttatctgtctcctgcttctctgctttagtcgtctgcatgttgactaggttctcaacagtaaacgcaagggagaagtaggtaagatggtcggtctgaccattcatcagcaagccaatgaacataccggtagacacgaacactgcggcgacggaggagattggattcagcgtccagtactccttccagtttaagccttctcgcttagtcttgaccacatagttcatcaagacaccgccgacgtatgaaagaaagaaggctacgatttggattgtcggcatttgtgatattacatcacccatgttgcaatactccctattagacaaaagaaagggagagccgaagccctccctatagatcaaagttgctcagaggtaatctgaccatcttgatacagttcgcgcttacgcgctttccacgttgaagaaagttcagagaagaactctctcgcacgatcatcgtcaagctcaaacggttgctgtacgccgtacttagcgcacaggccattgaacgttgcattgtactcggtctgcaaaagcgatttgtctgcgctctcgctgatatactgcttggccgacatggctactgttagttgcatgataccatcctcttattatctactcgcataaattatcatgcgaatttcaaaacgaggtcgttcacgataacagccttggactggtcagtaggcgtggtgttgtttgcatacactttacctcccaccaaacgtaagtctgcattcgacacctcgctgccaacactacacacagcaagaaatgcagcgcctgcatcgttgttgcctgtctgcaagttgatcgtgtttgagtacgcaccaacaacaatacaccaagtaggcgtagcgtctttcaggaaataactcgaacggttatcgctgtacgagacagcaaggcgcatgttcatcgcagacgcaagcagcacaggcacgttattggcaagcagtgatatagcagccttgttgcctgtaacaccaccaacatagtcagcaacgcgggcattcaacagaggcccgatgcgcgtgtacactgcgctgttgcctgccaattgagtagcctcggcaagcagcgcctgtacttctgctttagtaggcatcgtgcctgtataaaacagaattgagttggtagttgtggtgaacgaggtagggaccgcgcccccaacaagaccgttgtatgcactacgcatcatcgcattcgctgtagcaggaagcattctcattacgcaccctccacaaagttgtcagctatacgaatggtcagatcagaaacagccatcatgccatactcaccaatagaagtcgtacccagtgtaatatctgtgcctacatccagcaccatgccgaagtagtcctcagttgtagagcctaggtaggcttgagttgtactcggcacacttcccgtcagtggtacaagcacaacgtgcgtcagagcagcaacaacaaagtcactgcctttctcgacatacggagtgaatgacaactggttcgtagtagacgtaccgttcatgctcaagcgtaacttacgcgccagaatattcagaccatcattcatgcctgtagtgacagtgatacgcgtccaggccagagttgtcgggtcttgatactcaaggcgaatgttaccggcattgattacgttcgcatttggaataaagaacgaacggaagcgtagagtacggccgtagtcgtattccactgtatcgttcgcgtcccacgcaggagcaacaccgacagctacgtcagagcaagcagcaacgttggcaagcacctgttgtggtgtcttgctccatccggcgcttggcgtataacgagaatattcaggaaacacagcatacgtctgaataggctgtttggtaatggggtcgattgtaacacgaccctgaccgtagccgccaatcggcataagactgcgtgccttgctgtactgacggcataagataccgttagcatcggcgacctgagtctggtacttgatctccacggcagcacgagacgaagcgacaaggtcaaccaacgtcttaggaacgttgttgctactaccgtttcgaaagaacgctgcccagccacttgcgtttgtagaagtgcctacagtttgcagtagctggtagagcgcttgtttttcagagactaacataatgcctccttagagtttgatacgcatatcagcaacacgcagaggctgaccagcaacaacagcaccgcccaggattttcatatcagcagtagagttctcgtcaccaacagtaccgacgatgcagttatacaggttagtgcctgtagtaaagcctgaccacgtatcaatggtcgtacccgcagaacactgacgcagcatgaaccacgtaggcgtaccagaagcagcgatgttgaaaacgttaggctggctgctcagtggcagattcagtacgttgttatcgtagtccatggcaggagtgaacgtaccaagagatacgttgcctaagaagtttgctgtggttgcgaatgcagaaatggcagcggccgaccacgtagtttgagtgctcgcagtcgtcaacagagcctgtagttgttcatcagttggcggagtacctgagaacaaagcaaggtgagtcaagttgccgccaacagatgcacccggcagcatacgagtgcagatagcaatctgagactgtagtgtgttgtaggctttagaaacgcgcatgttagtatacctcagttgcgacaggtttataagttacagtgaacgagctaatagcctgttcctgcgcagggtaaacagtggcgtcgttaataacgaggtcgtagttcgctgcctgtttcagatcgtcagtgatagatacgccatagtgcgcaaagtaacgaccaaatgatatagccgccagattgacggagaaggatggtgttgtccacacagctccgtaggcgaaaggtaccatgacggcgtgctgaatcttgcccaaaacacgcggcgaagtaccagaagcataatcaccgtagaagtgcagagcgaatacaccgacgccgttagggaatgggtttgccgcagctttcgatacgatgcggaagcgacgggcctgaacagtagctggaagctggaagaacttctctgagttcagggcagtagcaggcagattaacagacaggttagtgacgtctacccacgaactgccttgctgcatctgtaagaacaatgcagtggctgcgctgttgataaacaggttattcgtactgtctgtctgcgtgaaccctgcaagagagttgataaccacttcggcgccaaagtcatactcagcaaacgtccaggaaccatcagcattggcctgcttcactgccggaatagaagcggtcttagccagtgcagcacaagaggtcagcgttgcgttttgagtagatgcacaacgatgggccatgatagtggcaaagataacatccagctgggaaccgaactgagacaggttacctactagatcttggtagaccgtgctgtatgcggcgaacgtcacttttggcagtacgcgcttgccgcgataaccctgaactgtagtccacgcaggagcaggagatacctgatagttggagacagttgttggaagggcctgatgttgggagttacccagttgagtctgcaagaacgcacggccgcttaccatgttgttcagaacggtttgcagatcgtagttcaacgtggcgggaagattcccttccataaatgcgccgaacactactaggggagtgttctgataaatcggtagaattttcatattcatgcccttggtttaaagacagttcaaattaatgacgtggcagccgaagccaccacgtaagtattacagttgaatggtaagatcaaggaagcgataagcctgacccgtcttaatcgtaccaccaatgaactgtagttccgcatcagacccttgatcgccgacagtgcctatccagaaaggaccagctatcgcagtattgtatgcaaagccagcccacgaggccacagtgttcgaagtaatgctacgcgcaacatagaacgtaggcgtgccgtcagcctctccggtcaatgtcgaagataaacccccaaacggcaaagtcactgtacgagcgaccgcattaactatgggcgtcattggagggcaggccatatctccgagatagtttgtctggagcagaccgagatttgatacaacgcttgcccagttgagcacactacctacaccaccatgaggcatcaagtccagcgctttgctgatcttaggtgcagtgcctttgaataacgctatgtgcaaaagcccgttggagatctgaaccgcaggaaacgcagcattcatctgagcaagcgaaagacctttattgctaatcatacgcccctcccgacgagtgcatcttgcttaatacggaacgtcggcacaggtgcttcaccgaacgttatgctgtagtttgtgtccggcataacgatatccgtactggcacctaacttgagatcgtcagtgacagtaaggtgtgtcattccaaagtaacgaccggcaacagtcgcagcaaccgcaggaagattgaagttccacggcgtactgtttgcgtagctcgcattcgccatcaggttcagtatagacatatgcttgtacttacctaatgtgcgtggcttcgttcctgtatagttgccgtagaactgcaagctaaacggatagtgccctgtagtagaccacggccatgctactgttttgttgatcagacgccacttctgcgctttaattgtcgcaggtaggctgtaggcgacaggcgagtagttgctggtggtacgaacgtttgcgtaaatatctacagcatcagtccagacatccccgataagagcttgcagcacagtgccttgagtaccgagaggcataagtgaagcaacaccggcgcctatgttcacaccaacaagtcctttaagttccatctcagcgccgaagtcatactcggccatcagccagttacctgcctcggtaagactgtattgaggactcagatagttgcctgtgtttactgagaactgcgtctgcgtcgtgcccatcttgtgcgcgagaatggttatggccacgctctcattatacgcattgacggtagtggcgaaacgcgcatcaagcgcaggcagtcgtaccttaggcacgattcgcatcaacgcattaatagcggcaccgtatcccaaagagccgctaaactctacccacgcaggatagaagttcgtgctgagaaacgtcgatgcagttactgggttgaactgccaacgaaacggcgcagtgcttgcaggctgcttttgaaacaagcgaatggcaatagcatcgttgaaggtgctatgaataccacgctcaccatttgcaggcacatcggtgtcatacaacagacccagcgagaacaccgaagcaatgttcgccgcttggtacgggaaaagttccatagcgcgtccttagctgaatgtgatgttgttaagaatgatagtgccattcagattgaacgtaccatcgttattgtccgtgagagacgcacccatagcaatcagatcctgagctgtgaactcaacaaccgtagcaactccaacagttgcaggagcgagtgtagtggtggtctgactaatgaacagatacatgcgattgaaaggcttcgcataggagaagcgaccaagcagactattcaggtcaaacatgcgcttaccattgcctgcgttgacaacacgcaaagtacctgtcgaggcataagcagtgtccatcacgcatcctggaacgttagctgccagataagtacgcagagagttcaggctaaacagagcttgcgcttggttagtccaggtgttatcaggcaccgcatctcctgaggagaacacaatcgcggcagcaggctcagcagagacatgcgtaccaccagcttgcatcgcatttgccgcattgtatgcagtgactgagctaggcatccacggagcttcaacaacagcagccgcagatgaacccaaaacatcgccacgcatattgagcatcgctttagagatatacatcagctactcctttgagtgaagcgaagtttggggcagtacatcatgttcttctgattaggataaacctgatcagtcaacttgaatggaccctgcgtaccgacagcaccggcagtaaacatgatgttgtcagagtaatcagtatcgccatgcgtgaacgtattgcagtgtgcaagagccgcccacgaaggagaggtcacggcgctggctggtggcgtgtctacagaactaagcagaatacgcatagcagtaacagaggtcgcagtagaacttttatagcggtagcgcttagacgcaacaggtgcagataaagccagacacgtagagtcaccagcaatagcagccgcgttgcccaacgatacttcctgcccctgatcatcaacagcaacaagggagaagatagagttaggagttgtgttgtacttaacgtgcgtcacagtcaccggagtgtcgaactcaaagtcaatatcaactccacccatacgagcagcaggaacggtgccgctacctgatcccataatcaacgtgacgtcgcgatcagtaatgcctgaacgagtgatacggtgaggcataagctgagataccacagtagcagcagtaccaacggtcccatagtacgatacccctttggggatgtactgagattggagagcaagtgcaatcacgttgccattctcaattccagtaatagggtttcgcacaaagccgattgcctgattgtacatatcggcaagtgacttattgttgaaggctgcatcaaagccttcttttgacgtaggcagcttaccactaaacgcaaacagattccagcccgcccctgcattagggtcattgagcatggttgcgttattcgcgtttgtgccaacgactgactgcgccatgatgcgtgtgttaatgatcttcattagctcaccaccggtgcaacagatttattattcgctttcgtgtcagacagatcgagcgtaggaacagacacacggaacacaatgttgtcgtacagaggttcaatcgtctggtctgttacgaatgcaccactaacaagaggagcatccacacgaggagccgctgggttcgacacgaaagtacgtggcgtaaacttcgactgtacctgagtagcagcaggactgttgagaacaatctggtctgcgtcagatacgcgctggttaagaatctgcgtccacgtatagataggcaggtaagcagacagagaagacgtaacacgttcctgagagaatgcggaaactttctcgttggtcgtcggcttcacaggctgagatgcagtgcttatctcaagctgagacataacgaacacgtagtcagcaaagagatctgggtcatacgcaataactggtacgaacattagtagactccttgacgaatgctgtagtgatcgatgatggccgtgcatgaggccgacgcaccagaaccgtaaccaccagtaacagtgaacgcagcgctgttggacattttcatcacgtacacaaaggtatcaacctgagtgccgtcaatgtagatagtgtgcgtaccagtaactgcatcatacacgtacttgaagcggacaggcacggtagtttttaacgcagcatacggagccatatcacgcacgactttcgttgtaccgctatcgccaacgttgttgcgcactacaaaggctttctctgtggtgcggtcaaacgctaagatgctgcggttggtcagagtcgaatagtaacgcaaaggctgccattcagcaaagtccgtgtctgacgtttgggcatagtcacactcaatggtgaatgacttgcttacgtcaacgatgttgctgttattgtattgcagcacaccggtggtacccatgttgataccattagccacaggcttaacgtcaccagacatgccatattggttgccgatgtaatcaaagaacgaaccagtattaaacgcattggcatcgaacgcagttacttcatttcccggcagccacgtagcgagcgagttctcaacccacatgttggaaagaggaatgttaaacgacaggatagaaatctgcgtcttatatccgttcgggtcgtacttaacgttcaggtcaggatagagcagagtcacatccgttcctacggtcaagcacacaggcagaatgccaccgagaattagatgcgtaggtacaccctcagccgtagcagtaagagcacagtcagacactgtaatcttcttacggtcgattgtgcggacgcagtttgtgcctttagcgatcacagtgcagatgccagtagaagcagcaagcgccgcgtcaaacatataacctgcaccagtctgaggctggaagttcaggcacttgtttaagtctgcttcgacgtaacctgcattcagcttaaccaagtagcaagacttatcgtccgcagttgattgagcaaacagacgcgctaactgaggcacagcagaagtaccaaagagcttgtaatccatgttatacctcggtagacagacgaagctgggcaaccgcagcgaactcaccaggaccgagagatgtagtcatcaactcgataggcttgccgctacctatagcaccaacttcacaggcaaagtaagtaggaatgtagttaccgttagcaagagcaccgtagttagtgtcctgaataagaaccatagcccacttaattgatttgtatgcagcgttacggccaacatcagaagcagtaacaggcagcacacgacgagtaccagaggtctgaatgaaacggtagcgcttagactgcggaatagcggtagcaatcacgttaccttcttggttcgcagcaattgaccacgaaacagcagtgcctaagatacccagctcgtcgataggtgcaatcgtgccagcacacgcagagctaatgtcaccaacatcagacaacacgccgtcaatagtaacagcgaagtcatacgtcaggtcagtagacgacagatggattcccggcataagtgcgtcatgcggaacacctgcgtaatcccacgggcgatagccagcaggaccgataccccacagtgctttgttacctgcgtcgttactcgtaagatatgcagtgttaatctgcaccgcggcagcaccgttgtacccgacaggacgtgcctttgacgggtagtgaatggttgcaccgttcttgatctcatacacatgaccagaacgcgctttccatccttcctgttgatctaagagaggcaacagaccttcagttgtaggacgaagcacaagacgcgtagcagcaactgcgttatcgaacaggttgcgcatgtcatacaggtgctgagagaagttaccctgagcggccaagtcagtatcgaagaagaacacgttaacggtctgcccgttagacaggttcgacgcccaacctgaacccaagttgagcacactgaacggcagtaagttgtgtcctaagatgcgcattagaactccttagagtctttaataacggtggcgaggaacttaccgttacgcaggttagatgacgacagaatcaagtcggcacctgaacccgcaccaccgatagtcagaatcaggaagccaccataaggcgtgcttgcaatatctttgttgaagacaatcacgttgtacgtgttcaacaagtcggcgatagagccagcaaatgtgccttgcagtgtagcgctcagacggaacttatatttgttatcagagccatgaatccagcgcacagggttaacggtaacagaagtcagatcaagcaccgcagttgcaccgatagctgtctgcactgtagtgccatcggcaacaacaatgtttgcagggtctggtactttagcgaggcagattgtcttctgcatatttgacaggccgtacttcaacggaggatcagtagctggacgtttgcctgcatctggaatcacaataccgttggcgaccaaagggaacgaaactatttccattttgtatctccagttaactcgctataaattactgacaagtcgaatcgcataggaagtcaaaacttgtcttacatcaaaaaccgtcgctttatcaccacagcgtcgtaggcattcaatgttgcagcaggcacttcattgggatttatgtctgaggccgcattgaaatcaacacccgctttggatagaacaacgtacactggagcgtcacgctcgaatgctatcggcatcgctccccactttagtgcataggcaggagtatcgtcatgggtgccttgtccgaagtatgccccgtcaggctctgaggcagaactgccgagagaacccgctgaatacgacgtggtgtaagaccagcctccaccggagaagtagtacgagccataagttgatgaactgaatggttgaaacagtctcgggaagatcgtatcagggaaggtactctgattgtacggagaacccgcatacaacgaactcagagtctgcacgttaatcgttacggtggctatatcggcagttacattcaacgcagtgattcccacgttttgcagataagaagatcctgtccgtgtccatcgccctatgccactacctccgcctccagtgatagtacctccatcactggaagtcacactggcagatgttttaggtacagagtaaagagacttcgtaaacgctgagccgtcgaatgcaggcagaaccatatcagaataagcgggtacgctaggacttccgttaccgtacgaatcaagcagactgcctgtaccttcctgagctgtaccgatgccagagtctaacgtacctatagcatagtagcgacggaacatgtcaatagcgctgacaacgcgattaccaccagtctgagaaaaccccgacttacggacagaaggcacgtagttatagaataggcgattacctttccagccagcaccacgaacgcattgcatttcattctgagcattaacaagagcgcagaatgaacgagacttattgatcttgttaatcatctcaggataagacgacttactcgttggaggctcaacatcatcagagaaaaggaacatgcgacgacgagccgtctcaatcttcttctctaagatttgcgctccgtttgaaatgaaaagcataaccactccttagcaaaactttattcggttcacataagatagagtgtcttggaaccgaaagggttttcagcttcgatgctcaatactgcaacatcaccagtgtccgcaggtgcggtctgtataatgtcttggccgatcttggcacgaagcatatacccttgaccattgcacttgaacatcatcatgcaagaagtcagagttacggcaggcgtgtttgtcttgcctgtgaccgcagtgcgcatagaaaatgcgtctgcaccacgagtgtaaccactaacaccatttgaggtggtcggggcttcccacgcagtgaactgatttagcccactgtagctgtagcgtttgcctacaggtcgaatgaacgtaatgtgaggagcattcgcatcccgatagacagaaggaatgatctgcaccggagaggaggtagtttggatgtatgagtaagattgagcgccggtctctgctcttgttgagaggtcaagagaagcattcataaacccagcatcataaccactgtacgttccccaaaagctgtcaacatttcgagcgtactgattgcctgccttagaactgtatgattcaatctgagcggactgtctcatgttctcaggaaagacgagcatacacgacgaaggccaatagtaccctgtctcgcatgtgtctcgactcacaccgttccagccgttaaacacggggttgccgttagaccactgctggccattgccctccgccgtgtcgtatacacataagtaacgctcggcaacagctttatacgtctgcactgccgtatagctattgtgaggcgcagcgttgcctgagataagattggcgctacgtgctgggtagaagtagttgtccttaacaccactcataggactcaaggtaatctggtcgccccgtgtgtctgagctattaccccaagcacgaacagactgcacctttgagatgtagtgttcttcgtccaaatgagcgtcagatatatccgtctgatcgtcaaagtaaagcgcacgatgtactgccagcttggctatcgtgttcgccttgttattgtggtacgttgcgtatagcataaactgtccttaagccctaatgtgtggcttgctaaaaacaccgcctgatgcggtcacgcccatgaggattattgttcgcttacacgcttatcacttcttcaaatggcaactctatccgtgacatgctaatcgttggagtattcccagactgctgcgtcgaagccgtgtagtctttcgattgctccggcttgaacagcttaacttcatttccccacagcattgggataacacagtacgacagatcgacacccgactcaggaacaccgatagccgcagttggaaccgtcggcagtacagtgccagatttgtagggcaactgaaatctactgttacctgagataaccacatgtccacaccataacagtaacaccgagccagtatcagcattgatgttgttgtagacaggacgggttgtagggctagagtcagattcgtgttgagatactgtcgggctgacaaacacgtccgttgttgtgcgcaacagagctatgccttgcgtcatgattccgccgtacgaagtggactgccctcgtgcaatatctgaatacatttgaggcagtacccagttagcgttaggtataggtgaattaccaacacgactaggaatcagactcgcgatggttccgtttgtaatccacggcttacccgcagtggacatggtaaacggagtaacactgtcattgcctacaagcccttcgttctgaccgttgcatcgaccactagcattgaagccagtaggtataggcaacatagtctgagcgaatgcggcctcagatttgaagtcagggatagcgcctaagtttgatatgcgtgtgagttttaattgactgcttgtacctaccattacaggcgtcagcttcacctgattgttatcaacgatggtctccacgtgagttcgtgcgttacgcatatagtccatgatgcctgcaacagtcatcgtagaaaatggacgctcggaaaacatcgcatagagtctaatatctttcctctttggtatgacgagttgcatacaatatccttgataaagaacttgtctttgcggacatatgcaaaaacagagcaaaactctgataaaaggtaaaagggcccgtaccattacgatacaggccatttcagttacaccagcagacgacctgcgatagtgattgctacaccattgagagtggtgtcagcagtgtctggtgcaacaacacgaagctgatctccagcaaccagaatgatctcttggtccagataggcagcaagaggagcaaacacaccagtcttagagccagcgccaaacgtaacagtaccgagctgaataacagcttgggtggcactgtcataagcacttactttgaatacagcctgagccgtagcagcaacatcagcaacagccatagagccgacaaagtttttgatgatcgcagtagtacgcacagataggtaacgagcgatctcttgtccaccagcgtagcgcttgagaacactcatacccacgtcatatggatttacagactgtagctggttgacccacttggtgcgcacggcagagtagacatacaggccaggctgatttgcgccagacacagcagtcaagttccacacacggccattagctgggttagctgggaatgttggaccagacgagtttgggtcgcccggcacacgaacgatctgcgcgttttcacctgcgagttgaataccaaaagcgtacatattttttctccttaggcgattcgcacatgtcccgtaacagcatacgggaatgttactttgaccgtgttcttatcaacaatgataacgtcgagtggcagcacttgatggagtttaccatcaggcatgttcacgcaagtagtcactgcgacttcacggccgaagttgtgcgtaatcgcccattcagcggcagcctcttcctgtaggaaggtgcgccccattgaatagttgatcatagagacctcgttattacagattatagagtgccgcgggtctgcgaactagagaaacggtgtctgcgaaactgccttgatagacatttcctggaaccatgtcgctgggaactgtgaagtcgtttgcatccaatagatacatcagaagatcgtttgtacctgtagagacaacaacagcagcccaagacagattcacagattcatcggttgaagcagtgatcggcagacttgcagtacgtttgtccgtaggtccacttgtgacattcgggtagcttgtcgttctagtcgcattgttaaacgtaatgccccgcagagtttttgtgcttactgtaacacctgcatttatgctatagtattgatacctaccgctaaagttttcgtaggtttgcccaaaagcagcaggctgtgcgtttgatgcgtcaaagtggctgactgcattcatggccatagtggtgtatgtaggataagagcttgcatagaagaaggatgttactcccactgtgggtatcgagacacgaacacttatatccaaagcgcgaacggcatcaggaactagatagatcgcgcttggtgtattagcaccgaaagtaactccataaccaccagcccaagagggtccaatgtcagtcaagaatgcactggaccctctgcgcgtggactccttcttaccgccctccattggaatagcggttagagagaacagatcgtttgaactgaaatccacatcacctgacatgtatgacattttagttaggtagtacgtgctacccaatcgacctctgattgggttaagccgaaatgttctccctgacatatcgtacactgtagtgcgggcctctccttgcttcgctctccagtcagcaagagacctaatgtcctttgtcgttgtttcatcgaaaaacgatgcgtatcgcagaacattatcagtagacaggagtgccatctgcatatgctacctacctaccttagtacaggatgaccgtaccagattgcggcgtatcgaacgtgatagtgagctggctggtgctgtcgtgtacgatagacttcggctgtacttctttgctgccctgatagatacgaacagcagggttatagcctaggttatgtacaacaacccactgcgcttcatcggtgaaggtagcggtgaatgcgacggtaggagtaggcagaccgttttcgacaccagacagcagcacggcagtaccggcaactggctcagggaacagaaccacggtagtgttcgcatcctgagagtgaatggaggaaggctgaacaacgtcaccattttcatcgtagcattgtacgattggcgtagcggtgttcatgttgtgcgtaatctcccagcgagaagacgcggaaggtttcgagtaacggtacatcgtcatctgttgagtcagaggtacccaaacaggcacatcgccaagttcgacgcacagcatcaaacgcttatccataagaatggccatgccgggcttagggtcagcaggccagtcggtagcaacgtcgaacacgaagttcttaattgagccgaacgttaagtcgagcgtcccgaggactttcataaatcttctcctgaaaggtaaaaagggcaggcagatgcccaccctttcattatgctactgaatcgaattacgcttctggttcaacgtaggcgttagtaccagttacgaatgcgattgcgactttcttcgcagtagtcagctcgacgcgcaggctgtttgcgtcaatgaacacgacttcatcagggatgatttgatagccggtgtcatcaacaacggtaacagtaccgtacttcacaccagcgttgtgcgtgaaggtgtgcgcagttgcagcagcgtcgccgccagcagttttatcgtactggtacagtttagcagcagcgccgccagcagagctggagatagcatcgtcaacatatttcttgttgacagcagactcgtcggtcagcgggtcggtgccagtgatggtcagcgcagcaacttcaccaccagtagcgtcgatgaagccgccagcagttttaaccgcagcaacgtcaacgatgattttgctgttggtagtgtcctgtttcaggccgttacccagggcagcagcagcgatctgctcgtaacccacaccgccgtcagcaactgcgataccgtctacagtgcgagacagagtagtgccatccagtttaacgcgagtagaaccagcgttatcttccagaccaccagcagcatccagcttcgcagtaacagcgttagaactgatctgaataccagcaccaactttaacgttaacgacgttgccagatttttccagaccatcaccagcgttgaactcagaagcaccgccgaaggtagtccacacagtaccgtcaaagcgacgatactctttgatcgctttaacccaggtcactgcaccgccagcttcgctgtcagtcgggtcgaatacgattacgaacttggtgccgtcgtaacgcacgatcatgttatcaaccaaatcggtgatagaaccaaagttcgggttgatctggtcagcagccagaatgatgtactgcttgccagctaccagctctgggtcgagagtaccatcttcctgaatcgcgtcggagtcgtgcagccagtcgataccagcaacggcgttgtcaatatcgatcttacgagcagcgtcgttcgggttagcaggagcggccaggttagcaacggtatgaccgttagcgtcgaggtcaccagagagctggccgttagctgagtccagcttgcctgtcagaccagtttcaacagtaccgactttaccgtccagtgcagtgatctgagactgaatgttagaagtcgcgccagacacatagcccagctcggtagcagttacgttgctggtagccagttcgttatcagcaccagcgataacaacaccgttttcagtcaggccagtgattttgtcttgcttggtagcagcaacggtttcgacgtgtttcttagaaacagcagcgttgtcgccagaagcagactggtcaggaccagacagcagaaggtcagcagtcatcggcacagagccgtcagccagaacagcaccttctaaggagccgccaccgccgccgaaatctttgatttcagtaccgtcgaagtatttgtacttcgcatcagtgctgttataccagatacgcgcagtttgcgcagcaaccagatcgcctacagccgggtcggcggtcaaaacttctggacggaagttcttaatctgaccgctgagcatcagttcaatattaccagtacgcattatctttctcctgagtgcgtgggattagaagaagttactctcgcaatcatcaaggctacaacgcagcgcttggtatgcagagattctttcttccgttaaattgatatatttatcatcaatattgtacttcactcgaataggcacatcgtacccatcaagcaagccgtgacgttggtagacttcaaggcgaagtacgggtgagctgacctgagcacgttccataatgttcaggtcaatcttgtcggcgtagatgaacgggcgttctctcttacacaagatgtaatctatctcatgcaaattaaagagtgtgaaattcatatagccaataataaactcggcaatgagtttaaatgactcgctcatgtccgaccgaaactgttgtgtgagaatctgatcgacgtgtggcttgactgccatacgcatctcataccagctctcacaaaacagtgcggggaaatcctcagggtggtgggccataagacccaacacgtctttttccgtatctgcgaaagagtttaaaatgtcagtggcatcaatatccgtctcgacgccacggccagttgaaatgaatcgacgctcaatgtctctcaaccaagactctgatgcagataggtattgaagcagtgtttctcgtgcggcagccgtgaactcatgcctgttagagtctaagacttccccaagcataaaggctttcgctttgtagaaatcactatagcgttcggcagtgaatcgtctgaaccctatgttattcttcaaatagcccatcatcgcaatgccctcaaatcattcaactccgagttgccttgagcattaggagttgtataaagagaactggatatgctctgcaaacgcagaccgagcttctcaagttcctgttggctcccacctaacttctcaagcacttcgcgcataagctcgacggaaacttgatggtcctgggattgttgagagatgattcgttcgaagcgctgcatagcacggagaacggaattcaatccctctttcatatccaaattatccactggcgcagagtcagagattgattgaagcatcctcatcatctgcgccaggtcagcttgcagtacgtcgctgtcggggttgacaacggtggcagccgcttccagttctgcgttccgctccttcaattgttccagttcttcaagctggggcagtatcttccaccaaacataggcaccgcctaggattagtagaacaacagagaagacagtcgcatagttggacgcaagcaacttgtataaaatatccgcccacattatattcaacccttacaggtgttatcgttcagatcaacaataatcctctcggcacctggttcgtttacgtcagtggttttgtacgtgtgcgccatccgaggcttgaactctaagcaactctgtccataacgtccatcgacaacacaaatggcagacaagcagctcacatcttccttgagtatcaagttttcaggagattcgttggcactcctaacagcagtgatcacgaaaccaaccacagcgagggaaatggcaacagtaatcgcaatcctaagtcgcttggcttgcatttcgggttatacctcatgatccttttatctgcttgaaattagcgaaccactcgcatctaggaggttattcctccaagacaccactaatttccgcaaacatgttcttgtagaccaaagaaccatccagcttgtctaggcgttcaggaagaacgtatagcttaggtgaagtacgcatgttcacccaagttttctcattacgatcaagtccaccaagtatcggaacaatgaccatactgaggtttctattcgctctaacaaagccaatgtcaatatgcttcctgttaatgcttatgaacagcttgttgattgcgtccaaaccaacaggcctattgaattccgtatcgctaactgtattgaccaagctaatgagaatacccctgtctctgctttctatatcaaacaaatcagacttcaaatcagcaacggtcgatgcggagaagtaggagacgtcatgcccatagtctttgagacaagcaccaagcgcacgggctgattcaatatgtgctatgttgtcgtctcgcagaatgtaaactggagcgtcggcctgatacgttctctgagtcattaggttgataagatcgcaagagggcttgccaacagcggccaagcccttattcgcaatgtaaaacttgtcgcggtacacatcgtacacgtttggtggcatgtacttcatgtaatcgtcgtccagactaagtatcatgcgaggcttagtgagctggacgacaagttgcatactacgaagcgatgctctatattccgtgtcagacagcacacgacttatcggaagatactgcacaactacgaatcggtcatcaatggaatcgacaaccgaccgtattaacgtactgcctagcgttggcccagcagagaattgggtaacgatcattaagccgttttcaactaagcctttcgactctgatagcgtcatgccgttacccgtctgctttaccgcgcgctcccacgttattgagggttcgtctcgctgatcggcatgtacattaactgcgccaccccagagacaggctccaagaaggtaagcagcaacacgttgtctggatcggcttctgctggattgaccgtgtccggccatagcacttctcctctctcgtcagtgacgtaaggaatgccggagcccttgcccaatccatgacgcaaagcccatacggtgtcggcattctcctgcacgaacactaaccctttaactgttgcttcatctgtagcctgttccagaatctcaacacgcgcactaagaagctgagtgtcagactggatggtacgaatcgcagcaaggttagagttaacgcgctggttcatgttgttaaacatggtgaagaacgagttgttcatcgaagtgcgaacgccgtccgtataggacttaggaatcagttcatcgttgtcgtagacggtgacgcctgagcgcacgagaactttaccggtaagacgtccaccacttgcgctgataatctgaggcgcaggcaaatcagcttcgtcccagacttgaacagtggtcatcaccgtattgtagtcagtctcttcctgccacgtatttttgtagggagcagtagcagttttggacttacggcgcatcacttttttatagttagcgctcgttccgtccgcgatgatccagagaccgtttagtggaaagacgtgagtagtaggctcagcaaacgcgagaataatcgtaacgtctgcaccaaccttatacacaatgttgttcgacgctgacagaccttgctgctgggcaagactaatcaacgtgtccacgtagttagtcaactgactcatccgagactcctaacgattgaagaattgtagaacttacatcggagaaggctttagcgatcagtttggccgcagccttatcgacgacgagtgtgctgattttccctttggtgttacacacaatagtttgtggtgcgtattgtgcgagagccaaagcgaatagcagatggttgccgagatcaccagtgatgcttacctctacgtcaagttcaggcacgtagatgttctgattgattccggcaacaaactgcgccagcgcaacagggtcgaagacaggaggcgctgtgtcgtaatcctcagcaagatcaatttgacccgtctcaggatagaagcgaaaggccgcagggtcactgatgattctgccaaacagttcatcactgacttcaatgcaatcgttgcctgtcacttcacgaacacgaccaacaatagcgttggtcgttaggttgattcgaattatcggcatattaatcacctaccgcagtataccagaagtcccaaccagcagtgttcgtgccagtagacttgatggtgaaaccgcctaacaaggcgttctcattcatcgcgctcgtaccgtccagattgtagagctggtaggtcttcgcttggttgagtgcagcgttcacgaaggtaatctgaatgctgatacaacggttgatgaatgccgtgttaaacacaacgtggattgtatcagtagttgacgcgttcacgactcgacccatgttctgagtaaagccagtgttcatatcgcggttactaccaatccatgcgttcggtattacagcgccggtcacagggttaagagcttgtgctgtacgatattcgtcgatagcagcatctcgaccaggactaccggtaggtccagtaggtccagtaggacccacagagccagtattaccagtagcgccgacaggcccagtgttacctgtcggtccattacgacccctcggaccacgagggcccgggcagccgtcttcaccgtcacgcccgtcacgaccgttagcaccaggaagaccacgcagaccttctttaccctgtttaccttcgcgccctgacttgagctggtcggcagtaggcagtccgataacactagactgactaccatctggccaaatgactgttagagtacctgtagttgtgtcgaactccacaccctgagagccgggaatcttcgcagcttctgtagggtcaataaactctacagatgtgctagtcttcttacctaacactttaccgatagggtacgcaccgccgtcgataagtgaaggattaatctttgtaagagacatgggctaaactcctaaccagtcagtgttgtccaatcaggttggcccgcctgtccggtttctggattcttgactttcgtgttattgactgtcatacgaacccaacgcacacttccgtctgcatcttgaaatcgaaccttcgttccaccgtaagctaaattagctacccatctgtctctgcttgggtctttgaatgctaaacgtgcataagcaggcatatgaatctccttagtgcagaatctcgtcaggttcccagcacaggataggtctgcgccatacttggaacacaccgattggtgacgcgcgagcatcatcaatgaagcaatccatggttcgtccaccactgttaccgcttttcatcaacgtctgcaagtcagacaaccaagaagcacggccaccagagtcagcttcgaacaacccttcccagaccatatcgaatgcaccattccatgcgttaaagtggtgagacgaatacgcaccatcactgactgtacacagcaccatgtactgataatctttgacacaagggatcatgtagttgttcccgcgtggcacagtggtactgttattgttgaagatacattcccagcccgtgcggtcagcagaacctgtagtgagatacaacggtctacgaatgatcatcataataccgttctcaccgccacggtcgctagacttctcgcagtacgcattgcagcgcagggaacggtcaacagtaaacgtggtagagttcgagaagtcacgggtgtagtagttcgatccccacttcggcagatactctgctggtgggacaaagaaatgacgttcagccagctcaagttcgccgtaacgatcatacgagaatacgatatactcataacccgcatcaatctgaatgttatggccttgagagcctggtccactccacttccaatgcacctgccagtcgtttgagtcacgagcaggtacgccagtgatcagattgtatttgcgctcatagatatgccacactttcccttcttcggttgtattgatgtacaacgagttcgggtcattgatgttaccattttcagtgccgcagtagatcttatgagacgcaccagcagagttatagatagtaccgccaccgccgctaccgaacatctcccagttcatcatcaggtgagaggtacacatttcgttctggccactaccatcggaggttgtgatcagatactcattcaagtctttgaacgggtacttaacgtagcggttgttcgcacgattgacgacatgcacccagtcatgggactgaaccagaggcttaggcgcgcacgggttttcgacagatataacgaacgtctttgtctcatacatcggcagcttcttgaatcggttgtcacggaacgttgacgtgtatttggcgccaaagaatttgctcatgtcaggcacgtcaagagtcttaccgtagcgaatgcgcataccacgtccgttctcaagtgcagcttggttaatctgcgtctgaggagtgatagcattcgtgcctgtcacatacggccaaccattaccgtcgaagtcaaaccctacatcgaacgtagcattagggtcattatccttttcgcccttgagcatctcaactatggcgttaccttctccgagtccaggactgccgaagcagcaataagcagcacgatagtagaagttcggaccgtcaaagatacggcgtgaggcaccgatgcgatacatagcagcttcaaggccactagctttgcggttgtaagacgcttcatcgaacatcgtaatcagcacccaataggcactgctaatcgagttcaagtatgcagccatctgaccggcattaaccagaccactcccctgaccctcaccgccatcaccatgcacatcaaactggcgacgctcaacaacctgcaacgacactttatcaatcttgtagactgaatagcttcgcgcttctgcgtagcgagtaccgttgatgatcgtatagcctgggttggtctgaggcgtatagcctgaaccggagccaggcacaccatagcctacagcgtggaagaagatacgaccacgattgacgagcgactgatcggtgttgttataccacgagatactatgcgtcttatttgcaaggccagcagcccagttatcaggcttggacgggaacgtgtacgcatcgaagttggcttcgtatcgcgtccctgggtctacgcagcatacgtcactaaagaacggaggcgtatatgcctgagtgtcatcgttaatatcgacagtaccacaccagaacggaatccatgtgcccggctgccccgacattgaagtctgacgagcaccacctgtatcggtgaagcgatagccctgagcactacggaaaccctgcgtaagatgaagctggccgacttggttccacgcaatatgatcaccgtactgagagacttggcgattacgcgctgtcttggtggcaacaatgcttgtggtcttctgcgtactaatgccaatctgagagaagatggcgttaaagttagcagcaccttcaccaggacctttttgaagcacaacaaacgagataccctctttgatggcattagcaatcgcgttgcacatctgcgcaggcatcgtctgagaagtcgccgataaacagaaaatggtgagagcaaactgtttaaagtattgcttgtcaccattgtagccgaatgcaccggcctgtatttctgcgagtgtgtgactgtagacgttgtaacgctcacgctcaagatagcgagcgaactggccccagttgttataggctttcgtctcagtcacagaagcaccgtcggacatgagtagaatatcatacccatgagtgaagttgcagttcatatccatcatcaggcggatatggcgcagcgcaccaacagcttggttgaactgagtgttgttgaagttaccaatccagccgtaaccctcaacgatgttaaacgaatatggcgtaacgaaatcgccgttcatgaatgcactaccgaagccacagatgtagcctgatgcgtgtccatcaactgcgatactcgttagcgttgagaaatctgggctcatgcctgcgtcagcggagccagggttattcgaggctgaccccgaataaccgctggtgattccacgcagatatagacagctttgtttcagcatatcttctgcatcctgttattgatatacgacctcaacgttgatacgaaggtcgatgtactgctcgccgctttctggcgtgtacacagtcacgatgccaatccaaccgttagccgctgttggtacctgcacaagctcagtctgatatacggaaccagtccaagtgtacgaagtcttagcgcttacgattgtacgatcaccgatgctagtgccccacggctcatactcaagcgtaccccacaagtcgccgtgtttcgtttcgttcgtcttctggaagtaaccaccagttgctgcaacacgaggcgtaacgtcacggccgtagccagaagtaacgatacgaataccatcgtcggtgcagatacggaagttgaagttaacggtgtggtcaacgttaccgtagtagcgcagaacacctttgctcaacgtccaactgctggaaacatcatcaacggacagacagcgatatggaacaagatagtcaaccacgtcaaacttaggcggttgaatcgggcagtatacaaagtaagaccaatcacatccgataggcgctgtcgctctgactgttatgttagagcgtaacgtgtgctctgggtacttccagaactcaagagtacctgtcttacctgccgctacatattcagtatcaagcaggttcatgtcttggtcgaacacctcaaacttggtgtcaaaggagttcgctacgcagacgacaagaacagcgcgttgatcagtttgtgttcctaacgcaaaattatcttctgtcgttgggtggccggcagagtagacgctgtaactttcacaagggtgcatgtattcacgcgcaccacgttcaccaggacaatacaggctgtagaagcaactcgcaagtgacgcagcgttaccgaagtctttgctgactacgcgcaccataatgtcacaggcaaccccctgtgggtcaaagtagaagtacagataaccttcacccgtcttcgcgtcaagcgttgttgcgatacgacgccctgcctgatacacctcgatgaagtcaaacgtttcccacgaggtgtagtcgagatacatccagcctgctgtccagccaatgaagtgatagtattcaaaggcgttagcgttctgaatacgttcagcgataggccaaacagtagcgtgacacggagcagggaagatagggctgccgatgtagtcaggatgaataacgtcagggaagttgataacgtcatatgatgcctgactgtcgagcgctaacccaccacggtcagacggtgctgcaagacgaggcggatagacttcgagactccagccatacccctgagttgtacgcacacgcaccatgatacgcatatcagcagcatcagggtcaaactgaaatttgatacgagagcgtccaatcagtttaccacacgttgaagcaacacgctctcccatgtgatacacgtcaacgcttgctccagcaggcgcatacgaggcaatcatcagctcaacgtagccttcaatagcaggcatcgcgtatactgtctcggtaatcgttgcgccacgtccatgaacagacgcatacggcacgttagggttagcataggtgcctagccctgcgcgagaagcaacaccagaagggtcgtatgattcgatggtcttgatgccgggtcggttaatagatcgaccagtaggaggagcaaaagagttgacgagaccgaagccagtgcgaccagcatcaggtaagtcgaaccctgcaggatagcctttgagtatatcgtatttctcacgaccgccactccctatcccgttaccagaacccttggttgttgatgtaggaccgccgccacacgcgcccgtgtcaagattagagcacgggtcatcgtatgtagggtcgaacgagtcatcaataagatgccaacgctgaccccattggttacgcacactaaacttctctggagttaaaggcgtccagtctccctctcgtgtgcgtatgaacatgggcgtgtccacacagtcatgccaaccgttattcgcagcgttacgaacgcgaaaacgagccatgatttctccttatggacgtacccagatggcgcctggtggaatctcttgttcgatagcagggtcggtatcttgaacaaatacggccacgacaccaggattacccggagcaccagtaggacccgtagggcctgtaggaccagcagggcctctgttacctacccagccttgcttgccttgcagaccatcattaccacgagggccgggacagccgtcagtaccacgacgaccatcgttacccatgagaccgtcaataccgtcacgaccagatggacctacgccaccggcaggaccgtaaccgatactatgaatcgtaggcagcccagaaatttgcagcttgccaatattggggatgttgattgctaacagaccggtaagctgatcaaaagaaccggtaagctggctgtcgtcttctgacgtatcaacgttaatcccaccttgagtcgcaacaacaggaccagatgcgttggccttgataagcgatatatcaaccttctctaccataacaactcccttatggccaagttatattctgatctttggtcgggtctacccagatggtgccagcagcaacgttccctgggttcgtagcacttacgatgatagacagacgaccggcaggaccggcagggccagttggtccggtagggcctgtagcacctgttgcgccagtaggacccgtaccgccacgagggccagtagggcctgtaggacccattgggcctgtgcgaccgtctgggccagtaggaccgacaggcccgggtagaccatcacgaccatctgggccgggaagaccctgctcaccatcaggtccgatattaccgtcacaaccctgctcacctggactgccgtctcgcccatcacgaccatctttaccatcagcacccgtttcacctctgcctccctgtcgtccttcaggtatatccgcagcggttgggaacccacctactttaatcgactgcccgttagcgaacttgagagtaagaataccagaagtcgcatcaaacgaggagtcagcagttacctctgagggcacatcggcatcgtttgggtctatcgaaagaactccagactgagcgcgaattgcagcaggcgtagacgaagaaccagcctgaatgagaccggtcttaactttaatcagactcattactttttctccgctttcgcaacaatatccgtgttgtgtgcgagtacatcaccaacgaagtagcagtcaaatggatcgacgtcaatatcaacagtctgcaccaaatcgtctacacgtcggaactcataaacagacactggtcctttacgacctagcactgtatgtcctggctctacttctcgcgcaggaacgtaacgccacacggattgatcatatatcaacactggatgctcgtgtgtgaacttctgtccgttgataatgaagtagtggtcttcctgtccgtacttgagagcagtcacagtagcgtttaccagattgcctttcaagctcttagaagaccaatcacggaactctttcggctgattagagaagctacgcaggctatcacctacacgcaagttctcaacagccttcggtccagtaatcgtttccacctcagaaccaaacacgatacagccagatgttgaagtgttgacagggttacgtgccacaacggttaacgcagaactcacggtaacagtagggcgcgacgtttgacccatatcagttactacgcagcggatagtgcctttgattgtacgatcagcaccaagtccgagacgcagatagaagttaacaatacacgttgaggtagtagtcgcatcgagcgttacgccctcagtagttgtgatagtccactgatacttgtatggacctacaccaccacgcgcattgacaggaagatatgcgagcgaggtaaacacatcagagccttgcacggcacgttggcctaccatgtacaagctcgacactgacgcagcaagaggtgttatcgtaggcagaggcggagcaggcgtcacgttggcagtagggtacaaccacacgaatactcgaccatctgtaggctgtgcagacgatagaacagcagtagtgattggcgctggtccagtgggacctgtagctccagatatacagcttgctccagtagcaccacgaggaccgagaacgccgggaggaccatcaggaccgtcgggaccagtagggcctgtaggaccctctcgtccagtatcacccgtctgaccatcagggccatcacgtcccggttcacctacagggcctgtcttgcctctattgcctacagggccaggacaacccggtctgcctgtctctccatcacgaccatcacgcccgtctcggccaggagcaccgggagcgcctcgacgtcccggtttcccttcaccaaacatagctacagtcggaaggccgggaacgtttactacattcccgttcttcttgatgaatactaacacacctgtcttgctgttaaaccttacgctggcaatctgagtatctgtcgctaagtcgctcgactcaaacccgacactaccatcaacaccaaccagcgatttaccttcatcgttagcagttgtttcgatttgcgaaagttttaactgtgttgtcatttcggttcaaccttaatgcacaagttaccagacagtttcgaaccatagctagtgatctgcgcattggtgatacgcaccttagctataatgtcgatgaagccctgaggctggttctctttcagtacggtgaacatctgcgtcaggctaacgtttgagtaagcaatcacctctgtgagacttgcatcagaagtaacaacgttaaagccagcgctgcccgtgcctttaagaccacgaccatactcagcttctgaggtgcctggcgttttgaatgacaggacatactcgatatgctctttaccgctggtggccgcaaagcctgggcccagttgacactggaagtcagcgatacaagtaagcatcacaccctttgtgaactcgattcgttgaacgatggtcagttcttcggaatcgccaacagtctgctggatgttatacatgttcttcgggtcagcttcttcggcgagagcctgagtgttactgatcgtaatctccggccacgtgcctttaatctgaataccttcgccctgaatgatagcaggtgttgcgataggtacgtcgataggcggcagaccttgacgtttgaacatgtagcctgtcggtgttgggatagcatcaatgatgacgccatctaccgagctgtctttcgaacccacagccataacgttctcaaagattgtgatctcaatgagtgtatcggcagggataggagtcagcgttttcagcgcattaccagcaacggtaaactcttgcgtgtgtactgtcaggccactcattgccataacgcagtgcgctttattcagcggagtagtaggcagaacaaatgtatcagcatcataaggcaggcgatactgagcaacacgaatacgagtagaccagttggcgcgttcttcatagcgagctacatagaaagtgtatttctgaccagatgggattgcttcggtaagcgtgacgctattaccattcgtgagtttatacacggtggtaggctgccacgtactaccgacaacgcagaagatcatatcgacgctttcaatcggcttgctgccaagtttaaacaaagcagtctggccgtcaccgacaccttcatacgtttcaaacagaacaacgtgaccctgcgatggttcgatacggaactgacgcatatcaagctgcatacgttgctcagggtaggacgaaagcagaagctgatcgtctactacgctatatgccgtgcgcggctggagaacgccagacgtaccaagcagtaagtcagttgagctatcgagaatctcggacagcgtgtagcgtaacttatcaggcgttgcagtggtcacaacggaactgaacagcatcttgcctggaggtacaaacagcgtgcctgtagtctgacgagcaccaccagcaacaggcccccaatatggctgcaagtctttaccgcgatacaacgcccatgcttctggtacatcgttgttgagcggccacggtatgccagcagtcggagttgttgggttagtgatacgacgccaaacagcaattgttgtctgagcgctcacgaaaggaatcgggtcgtccatgttaacgaactgacctttcgtgtatttaaagtgacgacacgcaccagagcctgtgcctgagattgtctgaatcagaacaacctctccctctttcacgctggtgatacttgcgatcttgaaggtgtttgcgttgatgaatccagatgcagtaatctgcccgctgaacacacggtcatgttcgctgaatgcccagtagaatgagccagcaccgtaacgataggcaatacccggagagcgagtgccgtcagagttaacgtgcatatcaagaaccgacacggcgttgaacacgttatcgttcaagctcggcagattctggagtgtggcagcacttggaattgaagtgtaatccgccatctttacagcaagaattttttgaatgtcctgctgaatatgtacgagaaggctaacgcggctgatagagtttggcactgcgatgattggctcttccaaaacaacgtgaccaaaaggtcggttgtctttgagcataatcaatagctcaccaacacgtttcagcgactcacctgcaacgtaattgactttaatatcgaagacaaagcgggcactgttctcggtaagaacctgaacatacgacaaagcgcccgacgcaagctcgttgccaagtaactgctctggaaccacagacgggttagagcctacaaagtcacctgctttaaacgacactggctgaactgcaagtccaccagagttagcgttcgcaacggcctgttctccctgaggcgttagacgcaatgcgtcaacgtagatagattcagtggccatcaaagaactccttgggttttaactgttctaaattagcgtaaaacaaaaagggagccaggaacatagcgctccggactccctttattttactgatagcgcactgtgataactgaggagccaaatgcacgagcgttggtgcgataaatcaagacgttttctgtcaggttatcatacaccactttccctacaatcggacccttcttgccgttatctccagttacaggccactgagcaccgtcgaaaccctgccaccctttgtttactgttcccgtaccgtctgcggctgctgagaatacagcggtaccgtatgactgtctgacgacaaagtaaccgtactcgtcttgtttggtagacaacacgaactggccacctgtcttagaacgtaaacgcgttggcaactgagcaagtgcaatactcacgccagtaatgccgaaaggcgcaacaccgaagcgtggataagatgacatggctttcatgaagtgcgtctgcgtaagcgtctgctgtccttcgatatagatagccttaacaccaaagtctgtatcgttaagcaacgaggctatggtcagtcgtccagtttgagcattgatagtgatgccttgaacatcaaccacatcgcctttactgttggtgatctgccacagacacttggcactaacatcatccttaacgaacgtacccgtacggccaagcaatgcgttcatctgcattgaactgtcgtctcgcacattcgtatatccgcctactgtcaggtcttgtgggaagccaatgcctgggcaagtgatttcctgaacgagactgatttcagtacgctgctcggtgatgatacactccactttaaccttctgcgggtctttcgatgcagggaagcggaaggtaccgtcctgagcaagagtaaagccactgacagactcaatgatgttccacttgaacttcacgctgtttgcatcaggcagacggcttgagccagtagcaccagagcggcgcgtatagaacgcagtgaaacgatagtcagtgttcggactgatattgccagcagggttctcgatgtagccgttgagaatcgtgttctgcgtttgaagctcaatggtgcgcgtaccgataatggtttcatcagcaagtgacattgggttctgcttggtaaacacagcgcgtagattaataacaccgtccgacaactgcgactgaccaatgaacagatgaccgttcagtggatcgattgatacgccgtcaacgtttgtctcgtcaccaatagaccagatagcgtcagtggttgtgagttcgtcatcaggctcgatgataacacgcaggctgtaaggaacgtaccagcgtccgttttcatatccgatagttgggttacgatcagacacgtcccacacaacatcaggaccaacgatgccaatctgacggagataggtgttagcctgcacgagaaacacaagcaacgtcttctcaatctgatactggtcgcacgtaaagcgggcgcggagcagcacagcaccgttgacgttctgactcggtgtgagtgaaccatcggcatcaatctctgcaatactgtctgttgttgggataagcacaggcgtattgtttggaccatcttgcgtgtagtagctctgcacgactgcccattcagaatcgacttctaggtcaaacgtctttggtgtttcctcagcgtaagagccatcaagagtgcgcattacgccaccagtcttatacgtgttgaccagagtgtatgactcggacagcacatcagcactgatttgcgttgcaccttcaatacggctgttgacgatattgttgatactctgcttaggtgcaggagaaacgaccaggtcaatcttgttgctcactcggaagaatgaggcaataacctgagtgtaggtgtcgtactcatattgcagcttgcccgtttgcagaatagcaccgtcgtaatacgctttgttcaggtcagcaatgctaccaatcgcgttgaacatcggcagtttgctaacgtccattgcacggaagtctttgtagtcgcttggtgtgcggccttcgatgatctcaacgatagccataccactatagcgaccgggcgagaactgtaagaacttatactcgtccgtgtctttgtctggccagttgcctacccactcagcggctgtcacatactcttgactaccatcagcataggttgcaagcagacgaacaaaggtgcgcgtcttctcgtacatcacgtctggacattcaatggtgatactgtccaccagcgctcgtgttggaatgagttgcaggtcacggtagtttgagagtttcgttccgtcgtactcatactccatgctaatacgcgcagaaccatgcaggtctccttgatagtaaagcacatactctttcacgcttctgcccatgattgggtcatacaccgtgttgttgctcaggctgacgttcagcgttacccagcgagcatagtcaggatgatcagggtcgaactgacttgggtcttgtccttgttcgactgcctgttgttgcagcctaattgtacgctgtctcgcttcttcgatagcagagtccgacggaatatactcgactttcacagcagccgcagcagcataagacaggccgttattccacagacacacagtaggcaacatcaacgtcgcgccgctactgatagtaggagacgagcgcaggtcaatcgacttcggaatcatgatcgtatcgttaacgagaatgattcggttgaacgtcactgtagagttaccatcaatgaacgtgaagttcagggcgtacttaacagcatcaccactgaccagaggtgcttcaaactcaccggtttgcgtattaacaaaaggtattgagtcaacaaacgttgctttgtctgagctactgaaccaaatgccaaacacttcggtataagcaaccacgatcgatgggtcacgcgcatcaatttccgcttgagtagcagaagcaagaacatagagagccattgcttttggtcgaacaatatcgcgctcgacaacagtggcaggaacaacgagatcaatcgttgccagtttaatctcaggcgccttcatcgttacttgctttacagcctcaacaggcgtaacttcaccaaagaccgcgtagatggaagtcagataatctccacgcataatcttagacttgaggacgttctcaacgatctcagtatgctcgctggtggtacgagcctgagcggtacccagcttggaagtaccgtcattgtacgtgattgcgtacttgagttcgacttcttcaccctgaggcacttcatcatccacgatgatacgcaactctgttggcaccaaatctttaacactgcgattgacgtcgaactcctgagtcttggacatatcgaactgtccttgataggagacgcttatatcaatcttggaatctgcttcgacactaggcagagacagcgttgtgccgttgaagatacccagagtagaactgagagctatcataccactgtcagttaattctttggtcgcgcctgtagcgagatacttaccgtagactcgcaccttagcactcgcattaccgtacaacgttgggcactcaatagaaagctcgtcaggatcaggctcaacccccatagggtagatgcgagactcaagcgcctgctgagtaccattgtaggtaagagtgaggttgataacagagatggccagaggctcattgaaacgaacagcattaccatcacgctctgcaatccaagtagagtcttctacccacacctcaactgtctgctcggtgccgtcgctgtatttgacgatagcgccaaacgtagtccactcaccgccgcgaataaactcaggctgaatgaacgagatggacttctgcaaaggacggccgacgttgaaacgcttaacaggctcaacaacaacgtgagcgccgagatacaacttagcacccaagttaatagcagcgtacacaccttcgagaacttcttcgataggcgcccattgataaaacaggtctgcgattcggcgatagaacattgcgctacgtgcggtgtactgctcaacgtcgttgttcacaggctcaaagccaatgtgattgttgaaccagtcttccgcttcctgttgcgtcatgcctacttcttgcagtgcgttaacaacgtctttctctgcatctttggtgatagtcagatctaggccgccatcaatcaaatgtgcatctacttcgagattgaccttgttcgacttataccacgtaccgccgtcttgaatcagagtaccaagaggagtaggcacaaaggtctgatagtcagcggtatacaggcgagaagaatcgaactgaccgccgagtaacatacccacgaacttaggccactgagttgtaccagagacttgctgccagtcaggcaagcagtcgataacacgtttcaacgaaggtaaacgatactgcatcaggtcacgcgtgatattgatgccgagctggcgaatacttgcttcggccaactcgtcgtttgtgtcaccgctgatgcgacgaatattcaacagttgctcaatggtcttgaggttctgctcgtcgttgtgtgcatcgagaatctcgaacaactctgcccatgcttcgttagcttcaaggaagtcaatgttaaaggctagagtgtttgatttcactggttcatcttcctttcgctataggtgatattgatgcgaaggttacgcagcgcaacatattccagcacggtgttagggatgatatcctgaacagggctttcaatgttgcagtaatcgacttctggtcgacgcgcaggacggtctgggtcagtccagtcatacagaacacggtctgttatgtcagacattgcgagacgtttacccagcagacctggacgacgttcaaacagtttaagcaccgattgctcaagaacggcctgattagactcacgcgtaccaggagcatcggcataaagagccacattcagaatgcagtcgatttgcagcttatcagggttccatgcctgaacgtcgagcgggctattgaattgagccagccagttcaggaatttattccattgcgcagagcttgggttagggttgatgcctccccaggtgcttgtgttacgaggcagaacagcgacgcgcacaacaccttgccactctttatcgttcggtgcaatctctgcctgaccctgaactaccacatcagcaacgtcaggataaagcgcaatagcagccttccattcatcacgacgaatcagcttcttgcgactgcggccaacgattggtgcatagttacgatagtagtcaacaggcgtttcatcagagccacctaagatagcgctcactgtcttaccctgtagctgagagttagacaggcactgtaccttcaggcctatactgtctgtgttgccactagcgccaagcgacttgataccctgcaccttcatcgtgtagccagctggtggctgtgctccccactgctcaccaccgaactgaatctcaacgtcaccttcatcggttgttacatcgaggaagatttgctgttctgcgtatgcttcgaacaggcatttgttgaaacgctgatactcaatcttagtgccagtcggatgctcaaaccaaacacgtaagtcatcagtcagttggaaattctcagtgcccagcttaatcgacatataatcaatcggctgaggaacaatttggctgaacgtaaacacttcaccaatgatgaagtccacgttctttatttcgcccggctcccactgcgttacttctgccagcagtgcattgaagttaccgatagtgaacggtgtgtttttatcgtatgactgtttcactgaactcaggttaacaacagccgcagttaccgtagacacagacttgcgaccaatatccacaccaagataacgagcgttagcaaggatagaggtgttgcgtcgagccaaacgactaaatgcttcacgcgcagcaatcagggaagcataggcattcgttacaccaaggtcaccaagtgcatcggcaagtaacgcagtcagtgagcttacctgactgtccgtccaatagctggacttattgatacgactcaggaagtctttcgcaaactcctcatgagtcgtgtatgtgttaagcatggacatgttactgtgccctcattgcaaacgtaattgattgtttgtcttcgagcttaggacaacgccatgtgattacacacacgtaggtctgctcgtattgatcgctcatggtgcaggctgtcttgacgctggttacgtcctgcgtaagaccgttgtatgggtcttctaaggcaagacgcatgtacgttgcaatccagtcagccgttgtttgatcgaacggctcaaacagatactgatatacatcggcaccgaagttctcacgccatttgcgagacttcttacgcgtaccgattaccatcagaatcttctggacgatgctgtccatgttctgcacgttatcgcgcggttcaagttgaatccacgcattaatatcacaatagatgcgctcgctaatcggcacatctatcagacgaactccgattccagccattagccaaatctcacattagaactaccactcgaagctgtgtcgccgcaactgttagcgtcaccagcacgttgcgcaggcttaccgttgacacgcacactagaacttgaagtagctttcccgacatgtggaggcttctttggtttccagtgaggacgataactatcgccttgacgaacactcccttttccattcacaagcacgttagaagatgcctgagcagggacaacaggaaaataaccattgtgtccagtagacagatctgtgcctaaacgaatagctttctgacccatgttaattctcctctgttaggcacaaattagcttgttatgcagtagaaacgaaaacgggcaacccgaaggccgcccgttttctttgcttggatttgtgtcgcttaactccctcacacccgaagcgagtgctcggtagccgaagccactaagccggagttaatggccgagagtgaagccgcacggcgcggcaacagcatgtgactctcgggaccagatagcaagcgaccaagcatcgcaattgctatcaacgacacgaagaacaaaatcatgtttgctcctgtgtctttactgtaaggtaaaacatttgcaaatgtcgatcaagttacttcaagttgcccttcgcccaacttcactagggtttcaactctctttctctcgttaccgcctgggttgcggagaccgcgcacaagaacaacgcttcaacgatacgtgggcaggaagacacgtaccgcattcacatcgctcaagcgaaggaggttacccatcggtgatctgcggtggttaatacactctttaacaatcgctcttgttgtgcattagatcgtggtaggaacgcgattgaccgctaacaagtcctatacgatatttcactacccgagaatgggtatcagctatggcagcacgtcaacagcagcggggcagcggacacactccattaagcattgttaagggcaatgctcaacaggctgtgaacagctttgaccaaatgcagagtcgctcgtcgcccgacttcacttgagtatctcgtctgcactcttttactccctgaataccgtacaaggaagacggcacccatgagggtctgcggatgtttatcacattaagactctagccaacttaatcccgtacgcagtgtgttgagtcgtccgctggatgacacactacataccccctcacgttcgtgcataagtgggatatagctggtggaaggttgtcatgaagattgcatcgcctggaggcttgccgttcttcccaatgcacacacggtgaaaggcatatgtgcatcaggcagcgtagctgcaaactgctatcccgataagaggggccacaacgttgagagtacgttccgcctgtcttacgcgcctagaggcaactgccgtgccatgtctgaaaagaatgaaaaacgctgggccttgtgagcgtcagcagcagagcagcagtctatcgcgtgggtgctggggttaatcctcacgattacagagcatcacactctaaccagctggaggcttgcctactgtggaacgcagcgacaagtttacagtcaaacaacgtccgctaagtacgccatctgactgggacaagttgatattactatctgcaatttttatttacagattttagaacgccttacgctcaatatttgaataaagagtatcgtaaggttctgagtacagttcaggtccgcgttgtgcgcgaatcgtcacgtagcctgtgtgacggttgaacgctgtgatttcgacagtcggctgtttaggcttgatagtcgcataaatcggagcattcaacgttggctcgtctgtctgaatcttatttacagattgcaatgcagcgccagagatagcaggcagattaaaacgcagttcagcacgtttctggccgaatgccgcgcgaatcataccgttctccaactctacaccgttctgcttgagatatgcagcgatgcgacgtccgataccagtaagctgatcgcgagtgcgcgggtcaaacgtgccttcgaagctgattgcttctgcgggctgacgtacagacaaatgcaggcctgtgttgaaatagccttcggtcagcagacgcaggatttctttcacgacttctttggtgttcgtcttgatagcagcgatacgcagttcaggaacgtccactttaatcgggtcacgaagctcggtctggttgtccatatagccgagtgagatatgcttcgcattggcatacgtgtgttgcagcacaccagtcgcgcgaatcaatacagagccaccttttgcaaggtcataaagttcatcgctggtggttgtgctgaacaggtaatagtccgtaggtacggccatgcgattaacagcttcaatcgctttggtttgagcttctttgacagttgagccaaagactacgcgactacgattcggctgggcagcagatacagggaagaacgcaccatagacaacgctaacgtttttcttaatcggacgttcagactgaatcttcttaccgccaggcagagaaggtagcttaacgcccaccagcttacctttgacgatagctttgttctctttgaccggcttgaggctgtcaatgagtttcgccagatcagcaccactaagaatcttctccagcggaacagcgaggttctgcggcagatagtgtttcttgcggaacatatagataacggtgtctttcttgatctgcactggcatagccatgttgcgaccaataacacctaccggctggaacgtgtttgctttgtcatcaccgatagagccgaactgcttagtgaactcagtctggccgatgatgttagcagcgcgtaaatgaccacgaatgatgaacacgattttcgggtcatctttcatgcgcaactcgtagcggtcacggttcagataaaccatgctgtacttgtcgcctttctccagctccagatcgtactcgtcgttagcgtcatcaacaacgactttcttacctacgtaggtaccgtacgtgcgctggccagcagactcagaagcaatctgcaatgctttgccactgttagacagggaggcagcgaagtccataacagcgggcatcaggtctaaagacgatgctacagcgtatggcttgcgcttctcaccaagatgcaaatgaacagcgctactgctggacatgaacacggttgtgcctacatcttcgtgtgtaccagcgaagtgcataccgctaatacgttcgatgatgtttgcgttgagcgattggaagtttacctcgcttcctgcagtgaagtcataaatttcaccgttacgccacgcataggcaacgttgtttgagcttagacccacgaacgcatcacccaactgacgcacggtcaacggcatgatgctcaggtcacgaataatcgaggactgcttttgaatgaggttcatataaatccctaatacgaaacaatgcggaaggcgttctgcttgagcaggttgagattacccagcatcaggctatacgcaagagtaccgtgctgttcaatcagactgtcaggtacaattgacccgaagtaaagagccttgtctggtcgaacgttaatctcttcgccggtagacttcattgcgtcagggacaacgaagcaccacggttcagcaacgtacttacctttgacgtactgaatcctataaccaacagccatgtgctggtctttggtaggacggtacgcgaaaacatccgtgttctgcttacgcgatttgcggaccgagaacagagccatagtgaggaagcgctgttcgaactgcggtatgaacgcattgtcttcgcaaatcttttttagtaccgcctcttgtcgtgcgcggggcatcgacgcgtagaggtttagattcatgacagcttggcgagaatttgacggacaacatcagacaccgaattaacctcagtgtcgataatcaaatcgaaaccaccaggtacttcgaggtagcgttggttgtattgctcatacacttctttggtctgacgcttctcaatacggtcttcaccgccaatgcgaatcttccgacgctcgatagaagtttcatagctacacgtcagcagcacggtcaggcggttctcaggagcaagtgcttcccaagtatgctggtagatgtgtgcgttaacgtcggactcaccagcctgataaacgtaggttgatgggtacccgcgatcggcaataatgatcgtgtttggttgattgtcgaggatgcgctcatacgcagtcatcgttgaggagcgcgcggcaaggaacaggagcagttcagtacgggggtccatgtcctcgttaagagggttcgagttggacagcagaacatcacgaatgtgttcagctaacggcgtaccgcccggctcacgtaagcgcaaagtattaatgccacgctgcgtcagtatttcagaaagagcagtacatacggtagacttaccaccgccttcgccgccttcgattaaaacataggttggtttcataatgcgattccttaggcaaatcgcccaccacgccatgcggccttaatgagcaacttcgccacgatttcgttcttcattgtctttcgcttggcattgcttctgacaaatgcagagccgaacttattcacgacaatcaaaccgcaaccaaggtccttgatacggtcaatgattttatcgccatgagattcaaacagccgttcatcaatgatgaagtacatacgcatacagaaaggcaaatacttgtgccacttcttatcggtattgaagtcagcccagcaactctttacctcagtgataatcatatcgcatttggtattcaggcagaacacgtcagcccttaagttaccgtgcttaatcagtccaagttcaacgtggcatgaatagcgtttgtcaatccagtagcgttgtgcagcttcggtaagaaaggccgtcttatcaggacggctcattgatttaaatacagcggtctgaatgggttcagctttgcgccgcttataggccatacgagtcgataatgtccagggcttgctctacgataggacgaagtttcttatccaatttacgcagagccttatccgctttgaaccatttgcgttcacgcgtcaaggcttcgtcgtactcggtcagcatagtcttgaccttcatgacgtaccattcaacgtgttgctcacggccggtcttgcctttgacgtagcgcataatgtctacgaagtcttttggcttaccgaggacaccagcttcttccatggcctctttcagagcactgtccagtggagtcattcccttctccaccccgcctttcggcagaccccagttaccagcgtgagtggtacgaatcaacaacagctcaatcgtaccatcacttctttttctgtatggaataacgcccgactgtttgcgaggtttcttctcgcttggcagtttagcagacaatgatacgttgatcatcataatgaatcgagtccccgtggcaggtcaacatcccagctaccggcattgtctttccacaggccctgatcttgcaacgttctgtaggcatcaaacagagttgcacgggcttgcacagagacttcatttgaaccggcggcacctaaactatagctgtacatacagccagggaagtattgtagacggcaggactcaaacgtgtcaaacacaatttggccctctgcgtcagctacaacgcagtgcgatgccataccaccttgacccagaacaacgatctgatagtcaggatgtttgttgtagactcgctgaataaactcggctgcttctgcaaacggtcgggctacttgcgcagcacggtgacagttctgttctaccgcagactcagaaagagagcgagcgccagtcagattcatagccgaggcaaagataagagttgtgagcgcttcaggctcaacagcagtggggaaaaactttgtgccccacgcttgagatagcgaaagcatggacgtctccttatacgatagtctcagctaaattagcgtcagtcgtgcggacagttaagcacttgcttgcgattctgcataaaatcacgcggagccgggccagagattacgacagcatgtttaacacgatgcttggtcggtttctttgatacattgcagcccgcatgagacagcgcatcaaaagcgtcagtagcggcaggaccagaaataacgagcatatgagcaaagaaaggcttaccaactttcttcattgttctgcccatcagttcgtagatatgttgcgcttctgcaacagacggcacagcaccacaccaaatatcgaacgtcatttagtgttctccttaatcagaaggacaccattgaaaataccgaacttatcagtgaaatcgccgaggacgttatagagactgccgttatcaccagggctgccgtaaggatcaaaagttgcgacgtcgatttgcagatgtgatgaactgacggtatcgcgtcccttttccgaaagaaagatggtatggtcagaaaagcgctgcttatcagtaatgaacacacccatgttatgccacgtacgggaagaggtttccagcacaaagacagacgcttcgaaaaagttgcatcccagctcaggcttgatctcttcgatgtagtgtgcatcttcatgatcagcaacaacaacgtccaccgtaatgtaatcaatcgcatcgcggcggtttcgcagccagatttgcatacagcgttcaaagtagtcagccatcgcacaacagatgcaactaaagttggtcgggtttttcttggcgcggggtatggctgtaatgctgcgttcatcaaatttccagctaatgtgatcggtaacaagagtaccgccctgcatctcaacgtcttcgtcgttaatgaagaagattttggtgcgttgcatagcgatgttggacatgacgtgaagtgcgctgccctgcaggcccaacgggtgctgaatcataacacgagcagtaacgacacgaggaactccgccgtccaaataagcgaagttcattacacgttgtaacacggtgcgcataatgcgtcctttagttcaggttgattgtctgtccatttacagatacatcttgacctgcttcaatgctaacagcacctttcacatcaagcacgtcatcgcctttaacagtgaccttgcggctgccgccaatctcaacagtctggttgcctgtaatcttggtgtactgattaccaccatcacccttcgcagtacctttaaacttgatacgcttcttggggtcaggcttgagattcttaggcgtcattgttgggtcattcagaatgtagtcaggaatatcattcttcgtacctgtgatgatcagttgctggttgccaacaatcgtttggttaacgtcgcccataatcgtcatgtgaaaatcaccagacgtcacgaggaagtgttcgttggtcatacgatcaatgataagctgggtaccggtggacagacgaatacccatgcgatgtggatagttcacctgaaactcaggtaacatgtcggcttgcgtcatgcgcacgtcagtagtatagataccttcatgcaactgaccagtaggaaatttaacgccgaccttaccgccgcgagtaggaatgaactgagcgccaaatacgacgccttgactcccacccttgagtccttccagatgaccaacagccgggcgaatccacggaatagactcgtcaggaatatcgtcagtcagacccataatacgcgcacgaatctggcagattttctgagggtcgttattgtcgataacgatagcctcatacaccatctgcgggtcgatgcctttctttgagttaactgtattgagtggaatcatttgttcacccgtggtaaatacatttcaagtttctcaccgtcaggcgtaccattcttaccagagccatcaacagtaccatcaccgagagagcacaggaagttacgcaggttctcttcctgttgacgaatgagttgtgcaaggttggtgcttggtccaagcagcttgctaatagagaacgcgtcgagacacttatcaggcagagcgtcatcgagcatacggttcatgtcctccagtctgttactgacacagcgctggttgatttgaggaccatctaggtactcagccggaatatcaccgttagctatcaggccgttcacgtcattagtgaaaccaccgagcatgttttccatgctatcaatacgcgaggcaagcgcaccaagtatgctgcctttgtagttgattgccagattgacactcagcttctccagactgttcagagcgttacagatgccagtaagatacttggccatgttgaactcttgcatcaggctattcagatagtcagcgccttcgccatacttcgcagccagctcagggaacttgaacatctcactatcagtctggaactggtcgagcataacgtcaagctgtaggctatgtgtctgcgctaaccagtcgatagggttcgagccatcaagtgcctgtttgatgttcgagttgatctgaaatggacgtagaatattcgcaacagtggacaatggcgtttgaatgatgtttgagccaccgccaatgtttgacgtgccttcaacaggagtaaagttgcgactcagcaggaaggcttcactgtacatgccaccaacgtaaacgcgtgtacgaccaatcacaagccacttgcctgacagcttaatgtcagtctcaacttcacgcttaccgtttatcacaccagcagatacgtcaacaatatcaaacaggtctacctcagggcagccgccaagaacaagagcgcgagcagtctcagtatacgccatagactgacgtttgttcgagtagtatgcctgcatgtacttgtcgtggatatttatatcgttggtgggtcgggcatacgctttacgtgtcccagcaatatcaccacgaacgtcgctgttaatgttcagaggatcgcggctcttaacggtcacggttgcaagctcattcgtcttgccactcgaatcagtccacagcagcttctcaccgtagttggacataccgttaaagataccactcattgacttcggacggaactcatgcagattgtacagaggagattcgccaataggcttatggttgaacagccagtacgccttagggtcttcgtcaaagagtttgtttatgtcacgcacgaccatgcgcttgtctgccgtaatgaacatcttcggcaacgcttcttccgagatccacatatgctgttcgatctcatgcgcaaacttcttaggcgagcacgttgcagatacccagttcatgatatccgacgtttgcacatcaccgaagtcaggcgttaagccaccgaacgaggcaacttgtttcagagcgtcaatggaggttccgcgaatgctaaagctacgcgtatcgaagatgaaggcgggagcgtcgagaatacacaacacgttaagcattggtgttccgccttcaccgtactccctgactgcatagacagagaacgtaagcgtagacgctgactcctgatcaggacccatcaccattgttatcttcgtgccgtctacaatcgcgtgagtggatcgtaatacgttcgtctggtcagagaatatgatcagagcgcagggcaatgcaaatgtgttttcgtacacatgaacggagcggataaggttaggcatagacggcggtgctttgccgtctaacagaataccgaagtaaccttgatcctttacgccaccagaagtagcttgatcagacatgattaaccctcagcgtcaagctcaatcgcaatggctttcagcttcgcagcgagcagcttaatatcggcagacttcgcttgcatgttaaagccaccacgaccgggcttgatttcagaatcgttcttggtgttgtaccacttacgcacttccacgacacggttaccggcatcgtcattgacgagatctacagacaggaagccatgtgcgccaatctgaatacgaaacagctcaggctcagaagtctctacacgagttttcttcttggccttttgcggcttctcttctttcttggctttcttttccttaggacgcttgagttcagtgtctttctcggtaagaggcttagacttctttttcaaactgtctttgatcttctttgccttagcgcctacgattttgccgttaaccattgccattagatttgcgtcctcttaactttcttgatagcagaactcggacgcttctgaggtatcgccatgagcatacctgcctgcatctcagatggatgaagcagggcgttcgcaataagcaacaacacccagttagcgttcgagccatatgtaatgtgcgacaagagttggggattgccctccattgaggcgtcgatgcgagttggcgtggtgtacagcgccgtgtctacatcctcaaacaccttcatacttagagggtcaattccccacttgtcaatcacgcctattgtttcagccatttcttcaagtcctctcgcgttacagcaaagtagctactgacctgcaggatgaagtccacgctgatagggttaccagtaccatcttcccacacgttatcgaagttagcgctcacgctatcaacaacacacggactcatggagaagaaattaccaatatcaacgaagaacgcctcgctgtcctctaagatgttacctattgcagcgttagccgcatcagcacccccgccaccagcagccagtgtgagtgtttccatactgactgattttaacgggcttgggccaggaggcatcaacaggccgccgttctcagaaggtgcacatagcgacagcaggttgatggtcgtatcaacaacttcgcttttagtgtcagagtaggcatcgacgaagataggaaggtcgattgatagataactcggacctccccatacgcgagcactcgccaacttgtgcatagaactggcgccagcgaatcgcagcgctttatccattgcaccagcattgttgccgatgaatgcaccggcggcacccaacttaccacctacagttgacagagcatcaccgcctttagcggcaacgtcagcaagtgaagtgttagcaaatggtgcgtcccactgagaagacaggctgaacgagaagtctggtggaatgaaaccagtgaacttgattgtaccactcttgttgtagatcttcacacgatacatgttatcgacagagataatatcgtcacgcgaccgtgtgctacctacagcagtggcttgcccaccatcggcaggcattaaatagttagccacacaaactccttatcacatgtagcccatagtaatcatgttcatcatcggatcatccataaacactggaattgagtcgagcgaatgtgagttactaggacttgcgttgcttgaaccgctagagcttggacgagacacagcgccacctttcggcatctcaggcgcaggtgcttgagctggtggtggcggagcaggtgcttctgtacgagcaatatcaccctcagtaacgagtggctgtctcgcaacagtttcttccggcttgactgtaggctcaatgcgtttaacatcaggtgcagccgcggcaacaaggtcattcaagcgacgctcatgctcttctggtgaggacttaggtgctacaggtcctctacctgtgaagtcaggcagcgaattgggatcagtttcagaatacgtctgaggttcacccttaggcaggtctgggaatcgagcagcaatacgtgcatcctgctccgcttccgtttcagccggcttaggagtatttacagctttcttctgacgatctgcctcagctaccttgagcaatacgtccttctcgttctgcgctcgcgtggcaacggactgccttgtctgagcatcagaggacttgaagtatttgtcagtcgttgcagctttataatcctggatggtcttaatcagttcatcgtcggacatgctgttaacgtctttgccttgcagcgcattcgagataacgctggtgcctgctccgtactgaacggccgtgctatacatcagctctttaacacctgcgccacgcttcgtcaggtcaacacctacttcgttctgcatcttcgcagcaagcggcgcatagtgagtacgcgtgatatagtcagactgcgctttatcaaaagcctcaccctgagtgtttgccacatctttatatacggagttgaactgagacgttcccggagcaaggccaccgaagcgttctaagaacggtttaccttcagggctgttcaggaagttcatcatactgccgttgtttgtggctagctggtgcttaccatacgacacaccgccgtagtcacctttaccagtagatacagtgctgacgcctcgaccaccagactcgaactgctcactaacagaaccaagaccgccctcagcaatcgctttgttggcaatatcagttacctgtttgctgtcatatcgcttggcaggctgcgctcgcatcggtccttgatactgaccaccaccgcctccgacaccagcacccattcccatcatacccataaagctgaaaggtgagacagtgggctgcgggaacttggacttgttctcgttctcgtcagtggtcttgttgtaatcctccatcttctctttacggtctttctcgccgtcagcaagcatcgtgtcggtttcatcagttatcttgtcagcaacgtattcgccgacagagttaccgaagtagtcacccaagatgccccccaacagactgccaagagcagcaccggcagcggtaccaacgacaggaacaactgaacccagcgtaccgccaatccacgcaccagcaatagcgcctgttgtaccaccagcagtaccgccaatagctccgccagtcgctttcttcttctcgtgcgccttctcagcgtcagtaagagtttcgtctgcgtcgatgtgctgcatatcattcgcaaggccgatactgttacctaaagcaggaccgatgacaggaatcttcttagacgcaccagccagcaacattgaagcgccagctacagcagcatcttgtgcttgtgaaggaggctgaggcgtatcacccttagcagcttcttcggcacgttgaacttcttggggctgtgctacaggctgaggctgggccggagcttctggcatacctgcaccagagttctctgcgttgtcctgctcaaacttctcttgtgatctttctttcaaccacaagccaccagcagttgcagcaccaataccaaccagtgccattaacgcaccagctttgcctctcagtcgcgggaagcgagaacgtgggagattgcgtccgggtcctctacgattaccggcgcctctaccgtaacgtctgccacggcgattacgacgaccggtacggcgacgacgattatcgttaccagaatcaccgagatcactaccgctatcattatccgggccgttgtcgtcatcattagcacccgtgttaggaccaccagcaccaggctgttgtccatgtggatctgacttagcgcgattcttctctttgaatgcctcgcgcttttcccactcaagccaatcttcgagagctttctgcgtcttggtagagactgcattgccttctttgattgccttaacaatatcgtcaccagacttctcgcctgcaatgaacaggtcttcgagtgctgactctacttcgcgggaattaggttgttgtgctacaggacgaggagatgttggtatcgcttcgctatcattgacatagcgcacacgctgattggccatcttctcgcgcatagctttcgctgcacggttcttcgctcttgatccaggaccgacgtagacaatttcttcttcgtacatctctgggtcgtaatcgcgttcgtaatcagcctgcgtaggataatcattcgcagccttacgtttgcgacgagctttaggcatacccgctacagaaggactaacgctgtccgcatgttcgatcattagttcgagtgcggacaactctttttcttgtggcttagccattatccacctctacggcctctctgcgctgctaacgcaagtgctcgctgttcttcggctttgttcttatcgtgaacataagcactatgccagtaaagcaatttgttgatcgttatatcgtctggcacgtagatgttcttggcgctggcgaggtcaagcgtcatgttcatcattgacgtgtcagagaacacacggaagtagccgagaatatcaattggacttttgtaggtgtatgtacggaagcaacggttgcacttgtgggtggtctccagttcgcaactcacatacacgtagttactggcgttaagcagttcgattgggtctgcatactcaagtgtctgcgcaagaggaatatcgctgtcgatatacaccgcgttcattacctgagtacggttctcatgctcagccagcaactctgcatcaatccaacgctgaacagtaggatggcgcaagccctttggaaggtcgcgccatttgtgctgaactattctttgtcgcatgacttcttcggtgttgagcaggccgcagtctacttcaacgaacttgcagcctcttggcctatcgtagtaacgctcaccacgcatatcaacaaagaagggcgtggtgcatcgccattcatacagacgatgcgattgcggccaactatttctgtcgaacattgccagcatatagcggaagtcttcgaggtacatctctctgaccttcacgttggtgaatcgctgcaacgtatcaacaaagagttcaggcagtttgtgtttctgcgcgttaaacagactcgacattgcatctgccgttatttggctgatacgacaatctgacctgcctgaagggagatagatctctaacattagttgacaaagaccgctgggttaagatcccatgcgcgtgtgctgcggcgttggcagtgcgggcacaggagttcaatatcagtcagcaggccatgacgggaagcacgtacccactcagacagttcaagccagagagtcaggtcggactgttcttccagacgcgctacgttggcatcgaagttacgacccatgtgagctacgtgccagctaaacatatcttccgacgcacgttcatagtgacgcatacgaggaaggtcaaagtgttcgtgctctgcgttaagcattgcgattgtcattgacgtttcatcaatcacgccaacgttgtttgcatcgcaagggaacgtattgataacgccaccttcaggacgcaactcattcacaatgccgtcggaatattcaaacagcggcttcttgcagttccagtatgtacgcagtggcataacagtgttcatccacatacgctgctggaagaccaaagcaaacgcatcaggcacggtcagttcttcgagtttgatattgagacacggcgccagagcatcgagcaggatgtacttcatatcctttgcatcaatagccttagcaatagcacggttctctttaccgccgaaacgacgcatctcaaaggctgtaggcagttcagccttatagccacgagaaggtaaactcgctgtttgaatttccatagttgttatctcacatcattggtcgggaaacatcaagagccatttgcacagaccacatgcctctaccgccggtgccgttaagctgaatgctttgaccaccgataggccagcagttgcgtagctgttgttcgccaaccatttgcccttggttgtcgtatagctcaatgataaggtttttcttatacacagacggcaaacggaagccaccagtgtacggattctgaatcagactctgccacgcattgaaatatttcatcactgcgagcttctggtcgataccaaacagcagactgaatccgtcaacgctcgaaccatgtggccagttgatttgcaccgtggccacttcttttgatttcgattgatagacggagaatggcaagtctacttcttcacacgcgaacgggcttaacgatatattaccaataacaggaaattctcgcacacgccacttgtcttgcatgaagggatcgtcaaggccaggagcagaagaatcattcaggtcatcaagcgtcggcagcggcatgattagtcctctacaataacaagcacaggcctaacggcatcgtcgaacttgaggaacgtagcaccaaccagatagccaccactctcaatctgcttaacgactgctttctcgtagtccgtttcccacttgtcacgctgattggctttgtagccatcaaacgtttctgacgcgtcgtagtagttatacgttccgccagttggcattgggattcgagcaaggaactcaatacgaccagcgttcttaaacttggccttacgtagctcttgagtcagcttcgtgttctctgctttagagccaggaacagctttgaatggtttctttggttgtggttctttcggtgcagcaggaagtttctcacgcgctggagtattcttgtcactcgccttcttaatgcgaatgccggacactgtaccagtgaacggacgactgcggccaagcaacgaacgtgctgtaggcgcatcgacttcaaacactactgacgggtcatccttatgcagcacatagaacttgttgcgctttgcagccaagataccgaatacatctttttcctcgatatcggcttcatgctccttgttctcaatgcttaccttgcgcttaccttcgaagcgataccagtcgcagtcttgaatacctacggcaggtgtcttacgtgcgctttcgctcagtagaataagcatagtctctccaaaacgaaaaagggccagaacgaatcttggcccttgtgtttcttacgatgcgagttcggcgtagtcgaaggaccattcgattgataccggaacagcctgtgcagcaccagagaactgcaaatcaggaacctgtttcggccacacaccgtagatgttgtactcagcaactacagaaccgtccatatcgaagatacggaagattcctttcgttgcgtagtctgccttacgtgcgcccagctgggtttgagtgttacgcacaaactggtgccactcttccagttgtttgtacacggccatctctgagttttcgttgtactcagtggacagagcgtgagagaagatcttacggccagcgtagttaagctggtggccgaacgcttctttcagaacttcttcgagcgttgaaccaggcttaacgccagtcttacagaacagacgcagagtacgcgcatagtccgtaccaccgacaggcgggttagggatcaggaactcgaagttgtcatcgagtaacggatctttcgtagacgcaaattcgtcaagagttacctttggcatctaaaagctccttagagtgcaccagagttaatcagttgcagcgcgtactgaatatcaccgacaggcggtacgatagcagttacgtgaatgcgtttagtgtagcgagtcgggtcaaggaacacgtcgatgatcagatcgccacgcgcttcgtcttctgcggtgttgttcttgtagtcacactggactgcataccaacgcaaaccacgaccggtcttaatcggttcgaggattgcttccatcgcagacttctggcgctgtttcagaatgtcatcgttcggttcgaacacggcactcaggttgtttgcgcgagcagaagcatgaagcattgccaacaggcgacgaataccgatatcctgcagcgggctcttagtggtgtacgttgtatcagcaccccacatgaagatgccttcgccgtcgaatacagcaatcgggttaatctggttgtctaccagaacgtcacggtcgccttgtttaaagcgatagcgcacgtcagtagcgaagtccagcttaccgcgattcagaccgcctggtgctaaccacgatgctacttggtcagcagtcaacatgcagtatgccatacagacagatgcaggcacgtagtagtcacgcgcattgtcgttgtcacgggccttaacgtcagcattcgagatagccgaccaagaaccaatgatggagaactctgcttgctgatacggtttgttgccacggcgatacgccacagcattgtcacgcgcttgcaggctgacagggacgccgtgagtagcgatacagtccatgcggctctcagccagttcatcgatcttgttcgcaatcacaggatgctcaaggccaccagcacacagaatgcctgcctgaacgtcttcccagtctcggtagttatcccacgcagtcaacacagcagacagactctggttagcgatagtcgcatcagaatgatctacgtcgataacagcgccgtcgctaccgccagtgaactgaccattaggagcagtcgggttcgttgggtcagccgggccaccgccgatggagttgataaccacatagttcgggtcttccagcagcttatagtggttttcgttcagcttaacgcggatgtacttggagttaacgttgatcacgtcttcgaggaagaactgattgcccgcttcgtctttgtagtagcgcgtagtcacggtatgagactcaagaggagtcaggtaaccgatacggtacactttgatgatggacttaatgcccagcgcatcagtcacgtcaggttcaaacgtgatgtacatatcgttcgccgctgcgtactgagacattgcatagaccaaacaaatatcacgatcagagaaggcaatctgctcagggtctacaagtccagcgtcacccagagggcggcaggtggcgaagttgttataagttgtgatatacacacctgcgtatttcacggagagagcgacacgcgtaatgttcagcttggttgctttcgtcatcagaagttttgcgttctggacgttgttagcgtactgccccgttgctggaccaaaaattgcgtcgatctcatccttagaggtaacagttgtgttaacacccacaggtccgcgagggaatggcagaaccagagtacacatgccgtactgcacaagtgacgcttggttgctgcgatcattctcctgcgaatagacccccggagaggggtgattaggttgtaacatcgtgaatctccataagaatgggcatcgtgtaacgactgtatgaaattagcgagaactcaatagcaaaccagattaactcgctgatccacgtcacttaccagaacggattgtgccatcttgcctgtaagtgtgaactgcccttcgataaccatctgaccaccagcgaactggaggatgattggctctgcggtatcaatgtacagcaaacctttaatctcaggcagcgcatatcccttagggccgacgatgatactctgcatctgatattcaccatcaaggggaatacctacggcgtgtgattgtcgttttaggatagagttctggttagaagtgacagcacgtacacgactatcaatgaccagagtacgatccagcttacgatacttctcgcgtgtgtacattagtctacttcctcctcgtcttcgacagcgttggcgcgaggacctaagtccatatcgatctcaacgttatcggtgatttcaccgtagttgttgatcttcgcctgctccatattaaaaccaatcttggtatgaatcgtaattgggatctcaagctcgaagctacctggtgtgctgccgtcatcgaggtcatcaatgttaggcagagggatagagtcatcgagtttaacgcgcacagtccatttggcggtaggcatctcgatagagaagctcatgagatcagtcaggcctgcgataagagcctgctgcacaaacagcaaggcatcgtcgatgttcatgaacttaacgaacaacgaaccagtgagtgtcacaggaaagtagtagttcgtcacaacgatggcgttagtatcatcgttgcctaatgcccagcctgagccgtgtcgtgcaatgttcttgatcggaacagactcgtcacggttgaatgccattgtaggcaacttgaaccatccatacggatagtcagtgctttgattgttcgttgcacgaataccctgtttcgggttgttatgcacagaccaaacaaaacgctttaagttgaacccttggcggaactgacgttgaaagccaaacaaggtagctttcagtgacgtactgttcttgagcatacctgcaaggttagcgctcattttcttgctccagatacgaaaaaagggcggccgaagccacccttttggttacccttaatcgggtgttagtcgagtcgtaaacgaatcaatgaggaaggggcggatgaatcggattcgattgcatcatctgcatcgtcctcttcttcatcactaagctcgtcttccaattcgtcttcttcgtcgctatcagagttaaggctgataacttcgtcgtcacacaacgacacggctgtttcttcctcggcattaagctctaaagcagcggataacgcagcgacggattcgttcagtccagacgcgttgctcacagagtttaccaagcaagaagcctggaagttatccgcgagttcgcattcgagaaagtcctcagcgtccggcgcatacgcagcttgcgagagcaaacgcgcaacgtcagtccactgtccttcacgcgccgcgacgattgccagtgcagctaaggaaccagataaagtcttcatgcttggtcctcagtagtgagggcagcataagccaccctcggcaatcaatcgttaaccacgaacagctttagctacagagcgcacgttcgccagagtgaaggagaaggtgctagacagcagccagccgcggtcggtgttaccctggttcgcgccggaagtcggggtagactgggtgccgccacgagtggtgtacactgcgtggtagtcctggtcagccagaacgtacagttcgccgtcgtgcagtacgcggtgttccggagcgcggaagccatcagttaccagttccatacccagcagggtacccaggcgaccagtggtgatcaggtcgtatttgcttaccgggtccagagcagaggagaactgatcgttaccaacgatatcgttccagtagtcctgcgccatcacagcggtgctaacaggcagcggccatgaagacacagaatttttcagagtagacagcagacgcggagtcaggtcgccgtgtacccaggtgatcgggttagcaacaccgactgcctggtcacaagcgcgtttccacagacggtcttctgcaaccatgatagaagacaggccgtcctgttgagcgcggtccagcagatcgccgttgatttggtccaggtccattttgctaacacgaatgttagatttcagttcgaactcagcaggcgtgtaaacacggccgcggaattgacggtaaccgaagtcagtaggaccggtcgcgattacagcttctgcctggtggattttcagttcgatacgagcaatgtcgccctgacgaacggtagcgcctttacaaactttgcgcagcaggcccgcacgttcagcacggtcttcgatagatgcaacgatagaagcacccagagaagcccacttctcgccgctgctatcagcaacagcttcctgaatcagctcaactttctcagcgtcggtcagaccgttctgagcgccggagtgtgagtgaacgatgttgccgttggcagcttcttccatcagacggctgatgttacgcaggaggtctttgttcgagtaggcgttgatttcgccggtgctctcactcagagccagatcgcctttaccaccgaagcgcaggtcttcgattggggcaccgttacgcagagttactttagcgccgcgcattaaggaattgttcattagttgctcctgagaataatctcgtagtttcagttcaaacagttacggtgcgcgacgattaggcgccgtaagaggaagacatttcgatgacaaggaagccgcgctcagaagtaggcgcttctttgatgatgcagcctttcagctcggtaccagcaccgccgatagtcagcaggccgtccgggcccaggctcgggtgcatcacgttgtcagcagaccagtcagcagtcgggtcaaacatagaggtagcgatgttacccagtttgatataaccgatacgaccggcgatattagaagccaggccgccgataggggcgtcagcagtgtaagaacgcgcttcggtaacagtcagctcgtaaccatactggatgcgaactttcttacctacgtcgtcagcgtggaagtacaggtcagcgccctgcacaccaactttaccggcagcagatgcagaagcggtagcttcctgctcggctttagcgccgtcgactttaaccagcatagcgccagcggtcggtacgcgagatgcagtgaactttttggtagagtcaataacgaactcttccacgcggttcatgtgcgaaggaggcatagagcgagccagtgcgaagccagcgaagacttcttcggcagcgccagtagacagacgcaggtaggagtgaccgccttcgcgggcccaaaccagtgcaacgccttcttcgtggattacttcgcccggcagcaggtcagcttcctgggtctgtacgatatcggtagcattttgaaacagcatgatgtttctccaataagagagattaaaaattaactgtcgtgcaggccgcaattacatgcggcgcagacgggacagcttatcttcgaatgagccagtggaagctgaactctgggattgaacaggtacgtcgctctgagtcagcagttcagcggcgttgaccggagctttaggctgcgcggctacaacttgctgttgaacaactggagcacgttctgcggtaacagtaccagcagccgcgtcgatagactcagagatttcgttctgcgcgacttcggacttattcatcaggtccatcgcttttgacagcgcggtcgtcaggaagtctttgccgtgggcgatgaatgcgcgttcgactacagcgcgtggttctttgatgcctgctgcggacagcgagctaaccaggctttcgacgattgggttacgcacatcaccccagaagtttttggtaacgcccagctgggatgcagacagagcagcgacgaaacgatcagtgtatgctgaggtcgcttcttcgatagtgcccgtaacgttcgcagtagcttcgctaatacgtgcgtcagattctgccaccagcagtgcatctaccggcatttcgatctgatacggcataaagccgaatgcttcacaagtaccggtcacgccagcgctgttaagcgagtgtgatactgcacggatgaaattatcagatgcgaaagatttcgcagcgttttcttcgccaactgcaccagacacagaagcgaatgttgcgcgagcaatcggctggccgtcatagtacatatgtacagtgtcgagcttaccaacagcgcggctcaggctaaccagctgagggtcgagcgtgccgtgttgtgcttgcgcggtagacaggctgttgaagacgcggctgacggatttgctttcagaatcaaaatcatcttcgtcatcgacgtcgagatcatcttcttccagttcttcctcgtcgtcgaggtcttcatcatcgaggtcttcatcgtcctcgtcaatgtcgtcttcttcgtcgagatcgtcgtcagagctggattctgaatcgaagtcctcgtcctcgtcttcttcttcgaggtcgtccaggtcttcgtcatcttccagatcttcatcgtcaatgtcgtccagatcgtcttcatccagatcttcatcgtcgaggtcgtcttcgtcatcttccagatcttcatcatcgttagacgattcagagtcgaagtcttcgtcctcgtcatcagacgaatcatcttcgtcctcgaggtcttcttcttcgataatatcaatgtcgctatcgtcgtcgccagattgggatgcaatcggctcgtcgaccaacgcggcagaacaatgcgcacagaacacaggctcttcatcagagcttacagtgaacggctgttcgcagttagcggagcagctatagatgtgcgcttcgacttcgccattggcgacgttgctggacagagcagtgatagcttctggagcttcctgcgcttcgcagttctcaacggcctggccggtgtacgggtcgaagtttacggtagtagcagcgttgaagctaccagtaccggacagtgcggtaaacgcgtgtgcgttgctcaaagccagagcgaagttgcgttgtgcagcttcggcagtctcgccggtagcaaccagaccagcgtgttcaatctgttcgtcagcagaagcggattcggccaggaactgagtaacacgttcgtcggtgatttcggacaggtcagcagagcacgatgggcagcagccctgaaccagcgcggcagaatcagagataacgtggctaccacaaccatcaagacagatggtgtaatgagctttcacatcaccagcagaagactgcgactggacttcggctttctcaaccaaatcaggatgctccaccagcagttcttcaccgccgttcggattgtagaggtcagcgccactttgcgaagcaaagcctacaccttcagtagaaccataaatcatcaggttctgaccggttgcagtgcggcgaaaattctctactgcctgattatggttttgaccgacacacaggatacccgcgagttgggtaatctttggcatggttaaaaccctcatagaatttagtcgttgaatcgacaggttgaaattaaaatatgcagaaaaaattcaggtatttttaaatttttctgctatcaatgtcagtttgaggaatatatctgttttcgaagtatttcgagacaatttcaacaccatttaaggtatatacgttgcgcagactatatccccaaaccatcagctccgcaagcgttgcgaagtgctcggcgggtaccgaactaatggttcgcgcattaagcgaatctggatggattttcttacccttgatagcctgatcgaacttcatgcggtcaacgttacgaatcatcgtatggtccacaaaatgggccagttcgtgagtaataacgtgagccatactcagactattatagccaccaagtagatgtaccaactgcgcaggatggattgaaatagcgccatacaggaagccgtgtacgcgatacgttgcgatatggctaccaccactatccgagttagcttttaacaggccaacatacagacgtttgaatggcagtgctatgttcagaccaatgccaggcatgacgttttcctgaatgtctttaagaacataatcaggaggactaacgccgttcttctcaagcgtaacgccaggcacacgcaggtcatccatacccattatttcaagatgcactttaccgcacttcttaacaggcttggtggcgtagttgtttggcgtaccacccggataaattgctgaggcatattgcagtggtttgaaattaccaaaatcaggcatatcgccaacacggcgctgaatagcctttaatgaatcaggtgtgtcttcctcagcagagtcctcaacaggtgcttccggctcaggttctggtgcaggctttttcttaatagaaactggtttgggttttggtgctggtggcgcaggcttcttctgcttctcctcataaggagtgaagtcaaagccaggcttaaagagcgcatcaggttttgcagtgaatgggcgactgttctgaatgagcttgtcaccgtcttctccactgattgcatatgcctgatcgtatttaggatgggctatgtagtacaggtcgctgttcactttgagaaggccaatgacctcgcgcggttccatgtggactccgtttgagatcattgccgcctgaccgagatagcgatagtacgaatagtcagctattgctaaaccttgtggcatcaggccatccttaacagatgttctttgtacgttgcagcacacgcgaacgctgggtcgtccacgctactacactcaaagcctgtcagcatcttacagtcacggtagaccaagcggcctgtacgcgcatcaagatacgttggtttgttgaacgccgtatgcgaacagaagttacgatgtttaggcgtaaccaactgaccacagatactgcacttatacgcacggtaggttgtgcctttgctgtacgtgttcagttcaccactcatgatacgatcacagcgctcagggcaacgagaacggtcgaaggccagcagcaacgtcagacgcgcatgatcaccacggaagttcttgagcttagacaagttactgtcgaagatcatgcccatggcttggcgatagtctttgttattgtgttcgataaacgtcggcttaccaatgaatgtctgatatgcaagacggccctggtcagggttgaacgttaaccactcctgcaggctaaacgcatcaccattcgtgttcggcagttcagtgatgtttaccggaacaggcacgatgatgtagtcgcggatgttgcgtgatgtgttatacatctcagccgctttgggcagccacacgttcacgtcaagattaaaagagcctgtctcgataccgaaacgcgacgcatccacacggatagacttagctgtacggctaacatcttccttgtgcatatcaatcgcgttcagtccgacgaggcccatgtccgaggtatcaaacgactcggagcgaatggactggtccatcgtgtactccctattggaatttgtcgatattgctctgcgtattggttaaacgcacctgaccttcatctgcttggaagcagtcgaggccattaacgctgttcagccagtaacgtaagcggccattagaaattactgcactttcgacaaatgcgggaatttcgaagccttcttttgtcttcactaatacttcgacgcctgggtagaacacatcgaaggacttcgtgctgaatatcggtttaacgatagcagattcacaaacagggtgctgggcgtagcggctgcttatcatatagatcgcctcttccttaccgataaggatagagttgatagtgccccgcaaaatacacggcgaacagtgctccgaaggaatttcgaacgaaacaatgtcgcctatgttgtaggcaaaagagaattgcggcatgttaacctcgcagcgcaccacgcgcccacgacttagcaagagccagagtcatacgcgtcggattatgaagtttgacttcacctttgtggacggcagtgaacggctcatgaggattctgactgcggccagaacgataggcagcttcattgaatccatcaaacagcgtcaccacccagccagtagatttgtcagagcattcaccacaggctttgtcccacgcaatcttaccgcacacacgaccaccagcgttaatcgcatagctgacctgctcagtgcctttataaatgtcagaggctttgagcgttttgaaggtcacacgcgacgatgactcagaacgtggcatcatcttttctttgattgcttcaacatccagcgaaccccagaaagattcaaacagcgcggcaaacttctgctcaataggaagttcgattgcgttgatttgtgcgatagtgctggagctgtcttccagcacacgattaaggaagtagccgcctaagatcacaggcatctgagtgccttgtgaaccagcagtcaggccagccttcttacagtagatttcagacaggccgatagccagacgcgcaagagtcatgaacgtctgcttctcggttgagttagcaatctctgtgtagatacgcgcagcgatggcaggaacaacagtacgtttcgccacgctcagaatatcttccggcttaataggctggccgagctttttacgcgcagccaattcgaaagcgttaatcaggctggctttgttcgctgccgtcaacgactcgcctaacttgatagtcgtcagctccgcgctgctcactataccctgttgaggcgttttctccagtcggcgtactcccgacgtcgatctcaccaatcgcttcactgtcatttgtttgttcctgagtagcaggctgctgcatgtacgcgagcaggccagagttctgaattgcctcattcaaatcttccccacggtgcatggagagttgagcgaggtagttgagagcaggttcaaccataccgagattacgacagccccaataagctgtttcgtaacataggtctaaattaatagaggtctggtcaaacaagaaactttttggattctgcttggtcgcttcgatgccttgaatagccatgcccacagcattcatcatatcgttgtggcgatagaagatgtcggcaagcataccgtagcactcgacgcgatcaggacggaacgcaatcgcacggtaacacgcgaagatagactcctgcgtgaaaccctgtttgaatgttgctttcgccagctcaatattagcgatagccacatagtcagcccagcgagcaatgccggcgaggcgatctacttcacgacgagcatcgtccagcaggtcagcacgatcaccgtagcacacggcatagcagagttcacgcgcatagtagaaactgcaacgatcatcatgtggataatcacccacgtccagaccaagctcaagcagataaccgcgcggctttgtgttgtcagggtagtggtcagttgcgaacgttgcctctacagtacgcagacgctgatcgggtttgcgcgacgacaggacttcatgcgcacgatacttccagaagtaagagcgacgacgatacgctttcatctgctggtaatgactgtcaccgttacgcatcagaatccaaacagcttcggcatgtttgatgtgtttggtattgcgaagtgtctcaacccaattagggtcatcgaaacgttcgtcaatgtcaagccacacaacgaggtcgtcctcggagaacggcgtagcggccagttcacgactcgcacctagattgcgttcctctgatacgtcgaacacatgatacaggttagggtgcgtgaacgccgagatgatgtttgtggtttggtcttcgctaccagtgtcaacgatactgattgcatcagcaccagcaacgtgcttcaaccactcaccaatgttcttttcttcattacggcaaatagccgctacgcagattctcatacatgcctcatttgggttatactaaaatgttgccgctatcccaccactgcttgccgtaaatatcagacaggcgatagtcaagaataagtggctggtcaagatcgacttgcgttataactcgcattaacgaaggactccaaactgttttctcctcagtgtagagtctaatctccagctcaatgtcgccttgtgtgttcttcggtacgaacggattggagaagtctccatcaaagcccgcaccaagagagtcgtcaaaataagtgtacgcacgaatttcttccgcactgttaatcacggtaggcgcatacgtttgacggttgtaataggacgtgtaatccgcaacagttgattgaagaggcacacgtcgcttatagatacgcgttacacctttgctgtctgtctctgcgcggtactgattgtaataccagtttatctgcgcaaacttaacaggcttcaaagtctcctgacctgcggcgtacttcatgaacggcttcgcagtgaaacggtggtatgtcttctgcgtgttcaatcggtaaagcagaatctggtacgtgtaccactgataaacatcaagggtaatcgtacctgagtcggactgctgggtaccgttggtcaggatgtaggagaagcagtcagcaccaacgtaaccacttctcgggctgtagataaacgcttcgttgaaagtgttcagccgcacagtgcctaccatagggtcattgaccttaatagcagaaaggcgccaacctctttgagctggcaccttatcaagcacaccctcagtcgggctatgcagtgtcacttcatcacgagcgccctgtaagatcttttcgagtgttatctcagtttcacctgagttacgcacccgcactgtcaggttcggagccagtggcttatagttacgccagtagtcgaacgtacaaggcaaagagagcataatcactccagtttgtatttgctcttgaactccgcaatgctcataacaggaatgcccttgtcaatcgctttctgtagcttcgcggaaccagagccagggtctttagcgatcagtatcgtcgtatcagctttcatgctgtcagacgccgtaccgccaagttggacaatacgctgcattagttctttgtcgcggatgccggtgaatgctacgttaatccctttcagtttggcgctaaccaccttcaccttcttcggagcaacgagagtcacttccatctcaacagccatcagataagacttaatggccgcatctgcgatctgtggcgccagcttatcgacgccgtgcatactactaatctttgttgctagatcagcagtattacctttcttcaaataagattctaggttaggcacagcatcaacaaccttatcaaacgttgtgttagcgccgcgcatgaagtatgaagcggtagctttaagccacgtattcatcggcacgccagctttcaacgctttcaggtctttggccagctgacgaccacgagagtcaccaacgatctcacgcagcgttgccataggagtcatgaacaattgctgaggagttttaacgccagaagcaacaagcagcttacacgtactcggtccagtgttcgcaacgtcaagccctttcaagaacgagccaagcatacgagagtcagcagcactggtcttcgtcttagcaacgaactcaacgccattgatcttgtactgtacgtcaggcagcttaggcttcttagcaggcttgagaatctccatgatgtatgggattaccttgccgcttcgaatcaacttaaccttagcacctgggccaagaggacgcttaggtcccatgacagcacctttcttcttcggcttgagatagccgtgctcaacgtagaaaccgttgtgcgcagaagcacgttcaaccgtaacaccgccaggcataacagtaggcgggaagattgcaacaggagccagcacaccgtacttggactcttgatagattacgtctttgacagtcacgataacagtgtctgactcaacgttcatcttgaacttgaaagcgtgtttaggattgctcgcagtagctttcggcgtaggaacatcacgggtcattacgatgccgtcgagttcatacttcgccttagcgatgcgtttgtccagccacggaatgagttcttcttccgactcaaaacgcatagggccgaagtggcgaactacttcgaatccccatttctccagcagcttgaactgcgaagactgtttgagcgtagcacctttaccgccgatgataccgaagcacaccatgtggacgtacttgaactctttggctgtttcgaagttacgaacaagacccgatgcagcgttacgtgcggctttgaagcgaccaccagcagactcatgcagctttgccataaaggtcttgtatgggattaacgcttcacagcgtaacaccacttggcccttctcagagatcttctgaggaatacgcatagcaggcagatgctgcgacacgtctttaccatgagttgcatcaccacgagtaagcgcacgaacaggtacgccaccttcgtagacgatttcaatactcaggccgtcgagcttgtcagtcagaatccagtccacgtcttcggcgagagcttttgttaattgcttaccaccgagtgtgaactggtcaagacttgccattggcacaggcagcttaacgtcagagtcatcacgcgcaccgactttacgagccagcttagacttaggccagcgcttgtctatgtatgtacggatgtaatcgtacaccgcgtccgatatcagaccttccgaatcagtgtggaacgcatcatcaagatgcgccacaagtttcgttgcctgcgtcaaattgagcgtgtcgagaatcttatcaggattcttttcgagccgcttcaaagagatttgcatgttattctccattcgtcagtaacactggtatttacagtctagctggcgattgggtctttgttgacgggataatcttcggccatgtcgagcacacgattgaacagcttaggcgccatatccttcacatgttctgcatagtcaaagaggttctgtttacgcgcacggttaacacgtacctgacgcacttcatcaggactgttggtaatatcgtacagcgtatagataacgatgttgtcggacttggagtgagtgctaacacgcagcacaacccaatcacgtttcaacttagcgtcagcgcggaactggagcacgtcgccttcttctgcctcttctgcgcgagcgcttggagtagatttgttggcagcagcgattttcttcgctgtctctttcgattcctgctcggcggcagcaacatcagagtccgtgtcttcgtcagcggaagtttcgtctactgcatcagatgcgtctgcatcatcctcggcatcggaggtatcttcgtcgctgtcgtcaccttctgaatcagctcctccgtcgtcggcatcgtcatcatccacggattcgtcgtcggagtcatctccctcatcagaatcgtctgtatcgctatcgtcagagtcttcttccacatcggtgtcttcctcttcttcgccgtcatcttcggaagtgtcttcatcttctgaaggttcttcttcctcatcctcttcttcggccggagcaggcgcagctttcttgcctttagcacgaaccttaggcggaggtgtatcttcctcatcctcttccggttcgtcaatatcagacaggtcgagggaaggttcttcgtggtcttctgagtcatcaccaccaaacagtgagcctacagaatcttcgatgttgaacgcatcgccagcgaatggactgcgagacagaatatcttccagcttctgctcgtcaagatcaagatcgatacctacttcttcgatctcgtcatccagaatttcttcttcaaccacacgaatacgcttaccgcgacggtcgataccatcttcgtagacagtacgcacttcggctttaggtgcttcgatctcacctgacttaaccttgttacgcaggtcacgcatttcagcagaacgctctaaggctttcttacgcgcttctttctggagttctttgcgttgttgcttctgctccagaacttttgcgttgttggccaagcgtgttgcttcttcctgctcttcttgagaacgacgacgagcacgacgaacaacacggcgataagccttaatcgtatctacgtcaactgtacctttcggccagtcgttcattggcagaatgttggtgtcatgaatcagcaggtcatactgtgcatcatcgactttgaggaacatgccctcagagttaatgacgatgccgcctttaccctgacgcaagaaacgaacaccaatcatatcgttcttgtacagcttggtgatacccttagaagtcttcacagggtattcagggcttgcaaccatacgccactggtagttgtcgaagtcgatgccgtaaacagcttctgacttgaccttacgtgggctgaaacgtgcggcatcaaactgagagcgcatcaactgacgctgcaacgtctgtgcaccagcagtcttggtgcgcttgccttcacgattaacaacgtctggcactttacgcagtttagatgcgcgttccatcaggaacaggccagttgctttatcgagcgggaagtcaacgtgcggcatatctgggaaaatgagagtgtagcgtccgccatttctcagcggaaggatgccgaatatatcgccttcacgaatcatgcgcttatgcgttcgttgtgcgacttcttttccacgaggacctgtatacttcatccacgcgtacttcgacacggcatcctgataagatgcagatacggagagtaccatgttattgtctctatgttgtacaaacacacgatgaaattagcttgcgcaaggtaaagcggggattaacccccgcttaaatatcctctcgcggcacaggacatagaaccacaagattcttcgcacacggtaatctgcgcccaagtccagtaaccattaggctgctggatagcatataccacagaaggatcgaagccccagacctgagtagcgttttgtagcgcctcaagttccgtagcaaaatagccctcttcaagaggcttatcaatcgaaccgtggttaggctctacagtccacgcctcaactacaggcgcaagaactgcatagactttactgttagccttacgcgtcttctgaatctcaacacgaataggcttaggcgtaacaggattacctgcctgacgagcaacagcgatgaccttgcttgagttgatctgacgtcccttcatctgatcagtcttggcggactgacttgtaccgatgttctgaccttcgatcaggtgacgatacacgatagggttgtcatacgcagcaggaccatacgcctctacttgcccagcaatcagcttcgtctgataccaatcgccttttgccgtatctaccttgtaccacacaggatgctcagaacgctcaggcgtcgaagggtccagatggtagattggtgagataggtgcgcgacgcacaaacggaatctcaggcaagaacagaacaatcggatggtagatagggtcaacatacgcagcaatcattgcgtctactttgtatgtcggtgactctgctatccattgaggtcttgcccacccaacatgatataccgcagctggtggaacataacgcgcttcggtcatctcttgtgaatacacaccaccaacagatgcttggcgtggcacaagtgggtcaacatgattcaggcccagatccgtaacgtatctcggcacaagaccatcagcaggataaacacccttaggctgcgtgtacttcggcagtatctgatcagacttagccttgatgccggaacggtactgaggcttacgcacttcgaaatactgaggtgcttcatccagatgctcaatgaagttgttgatgaacgtgtcactaacaacgtaaagagcctcagtgaagtcaggccagaacgtatctgagacgacagcaggaccttcgattgcctcgaacagtgggaatgagtctggcgtatcaacagtgccctgcgtcagttcaaacagagggaaggtgtctgaggtaacgctctcggtcttatcgacaaacgcaggaagaggtgtcgttgtaataacgtccttctggccttgcgtaagctcgaacaggtcgaacttgtcgagtacaatatccgagcgggcaataagatcaaccatgcggaagttatccacaaggtatttatgcccagtgatgaactcaggacctgcaactgtctgaccgatgatagcagaatcactctcaaccgtacagccagtagaatccccaacgtgcgtctgcgcgtcttcgaactcaagccattgtagctgtctgtcaagctcagggtcatacacaggcgtgacaacaaccacagcgctgccttgcgcttcatacgatctggtggcgaacgcatcgaatgcctgtgctacaccatcgacgtatgaggcatcgaactcttgaacggagtgttcagcgtaagcagtgtacgacggatcaaccgtcatatcatacagccagccgaacggtgcattgccaaacattaacgtgtgcggttgatcatgtgacggcagcccgtatatcttgagcagtgtgtcggcacactcgaacggaccgatatgcaggccctgctctttgtacacaccacgcgaatcaagttcctgttcgacacgcacaccatcgacgtcaagcaacatacccgcaggaacggtgatgtacgtccagaagttatctgggatgttatcgacaaacaggtcaccactatcgcccatgacataacgctctgcgcgtttagtaggagctggcgtaccaagccactgagcatcagcccacacgtaccattcatagctatactggtcagaatggaatttaatcgtgtactgcttattctctgtgggcgtgaacttgatgttggtagtgccgttcacaggcagggtaaccgactggccaccttgagcgaactctgcatcagtcgtgtcgattgtcagggtcagagggattgtgccagtgttcttgaacacatccgactgaacttgcttaccgacaggcatatatgcccaatgacgacccacttcaatctgcgcttcgacaacggtaaacagaccaaagcgagaactgccctgacctaccgttacatcaatatgcgtggtgtcgttagcgtggagaacttcaaagcccagcttttgattgttgcgaatgaacacaggcattgcggcttgcacaccatccacataaatcttaactcggtcatagtcctctacaccatccaccagcacagatacaggcacggacacgttgatgccactgatggtaacatcttcggtgcggttccatgtatcattgtcgatgcctaagatgttctgccacgcaaaagcgctaggcgtatcgtcagctttcatctcgaactgataaacagatcgaccgatagaaatcgggaatgacgtgctggtgatatacgcatggctcagcgtgatagtaacttcctgaccgtcgaacactttcgttacaggtacggtcgtggtagtcgtaacctctttgccgtcaacaatattagtcgtggtaacatcaatcgttgcagcaacggtcacaccggcaggcgcagtgataggaagaccgatatcagggtcaccagcgtcaacaaccactttgaacgtaacagtcgggcctaagttgatagcacttaggtcaggcaggttcaccgtgtaatcacggatagcgatatgcttcaagccagtagtaggacgcgctgcataatagaacagacggtcatacgtatcttcctgactgtacggcggcgtcaggagttcgatatacggccaaccagagcgcgtctgagtaggcgtatcagcagtagtgaaatcgaacaaagcattgctgccgttcgtgtccataccagcaactaacttaccaccggctgaggtccatgatgcagtcgtgttaaacacaacgaggtcattcgccacaagcggacgagccgctacgttctgtacgttatcgcgcaggttgaactgatagatgttcgtactatcatggccgaataccagcaatgaacttgggacgaactgataccagaagactgatgcaggtgcagcggcagtgttaccgccaatcagtctaccatcaagcgttgaaagcacatcgtaactgtcagagccgttaacgtagaagtagtctgacttaacagacgtttcagcaaacgaggcattcaggtaatgcgcacgtccttccttgtcaaacgcaacatagctatcaacagtgtttgaaccaacacccgcacgacgacacacaacacggttgacttcatatccgagttgcttaggttcaccgaactgcgtcatcgcttcatcaagcacgtcaatctgaccggactcgtggaagacaacggcgctacgcttacctgtagagtcgtaactgatcttatagcctgcaatatcaacgtcgtacatgccgccgaagattttcgtattcgacacgtcaccgtcagtgtggatgtaatacagagtacgagccgcacggtcgtggacgattgatacaggcttggttaaatcaaagaacgtggaatcaaagtccgagaacttagccacgctgccctgttgcatgtcctgcacggtagggattcgaacacccccaccaagtacaagcccgccgtaggtagggttgacagcagcgcccaaaggcattgcatccatacctttcgtcacaagacgatagtccagctctttcgtctgtggtctgacgaagatgcgagacagtgaatgcacaagcacccacaaatcaccgtccttgtaatacagcagaacaggttgcgttgcagaggcagagaccgttactgtagcagcgagagcaacagcatagtcagaaccagaactcggcgcgatatccttttcggtagtcgaatcagcaaacgtaccgccagatacacggaacgttagtgtatcagtatggcctggaacagatacgttaccagaccaggactgaacaccggtagctgatacaacaggaatcatttcagccattgttcacctcacgaaacagaaactaaaaagggcgcccgaaggcaccctgtgaggattaggctccggcgccttctggggctttatagccttgcaggaagaagatacgcataccggtgttgttcggactgttagcagtcagagctttgtaggtacgcttcttcgcagtgctgccgtcgtcttcggtctcgttatagacctgaacgtcgatcagagtaccgttggagataacgtcagcagacgcataaccaaccatatccatttcgtacggatagctatagcgctgagtgttgaagccagcaggcagacggaagtcgaagtggttatcttcggagaacggaaccatctgatacgggttcagcacagcagagctatccgcgctgtggacatgcgcaggtgctggcagagtcggtgcgttcacatcagactcacgcacggtatagcgcatgatctgatatgaaccggggctgtccgggacaggacgcacttcgtcgttgttgttcatggagccaccgccgttcacagagaacatgcagaacagaggagctttaccatcgacaaccacagtaccatcggagttaatagcacgttgaattaccagccacgcgccgcggcagccatcagagtcacgaccttcaatctgaatgtgaatcgcaacgccgtgatcagacaaagcgatgtggtacgtgaacggagtagcttccgggtcagcaaacactaggctattagagctggtctggccagtaggctgagtagtagcaggaggatatgccatggtgcctgcgtagtacgtagtgttaccctggttggcgataccgcgatgccagaagtacacttcgttgtcaccagaactggcgttgaactggctgctggtagaacgcccaccaatctggccagcgtattcgttaatggtagtgccgccaatgttcacagcaccagtcttagagatgatgcccatgtcagagatctgctcaggcgcagcacagaaaagctgagtacgcttctctgagcctttcatcgccagacgccagcgctgttgacctgcaccagtaccagcgatcgggtcgatggtgttagtagcctcaacaacaaacgactggaggtcagtcgaagggatagttgaagaaatagtgccgttgacactcaccagcttgaagccgttatcaaccaaatcctgcaggattgatttccacattttcaggttgctggtgaagccagatttcacgatcagtttgttcatgagttgttatccccttaattaagccgcgtcgcccaggccgataggaagcatcagacgcataccacggttgtctttaccgttagcgttcatgcccaggtatttggttttgttcgttgctttcagagggttcaactgcacttcggaaccagcggagagaacgtcagcagacgtataacccagcatgtccagtgtagcgaagtacacatagcgctgagtgttgatcatctgcgggaacagaacgatagcacggttgccttctgcgatcataacctgctggagagggttgatgataggagcagagtcaggcgtaggctgaacagcagacagtggaaccgtagcagagtagataccctcttcgattacagtgtagcgctgaatagcttctggcttgatggtgtcagggtcaccaccaagtccgccgccgcaggagaagatggcgaacagtgggctgtgatcgccaggcgtagtgtcgctagcctgtacgccacgctgaacaacaaaccagctaaatgcagtaccggtgttgtcgaagccttctgcgttgatatgcagagcaataccgtggtcggtagtgatgaagtcatacgtcagcgggtatgcagacaggtcagcggtcgcgtccatcttccagtcattgaccagatcgatgaagaagttagcagccagaccagacttggacatacggcccacttcaacatcagcggaacgtttcgccgcagtgtagttagtctgattgacctgattgtcaggcagaacgttgattgccagagttttaccggtgttgtcagcagagaggatgattccccacttctgagtttcgaacagcgggtcaactgattccgaggcttccagatagaaggccttagaggtcggcgttactgtgcttcctgctttgccgtcaacgccaatcagcgtgaagccagcagtaatcattttgccaaccagatcgcgagtcagagcttccagacccacgagcttagtggcagttacacgttgaatagccatatggttatcactccattaccagataggttacagtgagtttcggtttcgacggtgatgtgccgatgttcttcatacgccacgaaattgtaggcgtgttgtctttgttagacaagaaggcatatcgacgcagcttactaatgacaggattgccttcgctatcctcgtcagtaaacacaccatcatcttcgagaaaattagcagcggaacggaatatatacgggtttctgtcgtctcgaagtgaactttgatacgcggtaagttccacgtcaaaagcattgagcttaacagaaaggagcataaccgttttattcattgccagatcgaaatcaagctgttgaccaggagtgatatagttggcggcttcgtactctacagtcttacgcacaccagcctgttcattaccactcatatcaacccagaacatcgtaccgttagaaccagacatgagggtcatacccgcatactgaggttcaggcacttgcttactagggtcgaggcctacaattgtcagacctgtttcatccacagcagtcacgaacggcgactcgaacttatattcagagccaccgaatttcgcttcttcccacgttacgttatctgcaccaagctgatacatcgtcttggtctcagtgacgtagcacaacatcccaggctttttattgccgacagacattgtatcacgatcattgagcgtaggcagacagcgcataccccctcgaagatatttatcctcaaggaggtacgggagtgctgcggatgcgggcaacaggaacgaagtcatgttaaccggcatcctattctccttacgcgataccagaacctgggttcgatgaaccgtaggtcagtttaaacgtatacgccagattatcgaacgggaagtcgttacgatagataacgtaatcaacaccgttgatagtcacttcggcaggaccagcaaagttgaagtcatcaaactccaacgcaccatcccatgaaccagcaaagccctgtactgactcaacgaagtaaccgtagccgagagacttcggccacgcaacgtagaagaacacgttgttcgttgaggtactggtgtttgcaggacagttcaggagctgttgtccagtcgtagtcagcgcggtttgcaggccctgtacgaacgcagcatcatagccagctacagacttaatcttagagtgagagccgaagcgggcacccaagtcagaggactgttgcggtttgagcgtaacgtctttggttgcagtaaccgtcttaccgttcttaacgtaagtcacggtgatagttaccacagcatcagcagtcacagcgttggacttcaacgaaccgccagtaacgctcaggccagttgcggtgccggacttcacaaccaccgcccacgttgtgccactatcagcagtcacgtcaggcgtagtgccgtcagacagcgtagcagtcgcagtgtacgcggtagtcacaccaccgatgattgacgaaggaccagtgatggtcacagagtcaggagtcgcaggcgctggcgtgttcgttacagtcaggttcgcagtttgcgattggctgttgtacgaagcagtaccagtgatgattgcgctctgcacggtgcttaccgtgttaccgatgatggtgttgttgccggggtacgtgaacgctgtagtagaaccagagctacgcgtgataacaggcgtcaggtcgaccgtggtgttatcagagaacgtcaggcgaagaatgtaggtaccagtctcacctttgttcacagcggcaggaccaatcagctcgcgcttagtgatcgttgcagcctgattgataagcgtaatcaccttctcaggagcataggtcttaccgtcaacggtaacggcagcagcacggagcgtagcagtctggttctggctaatcgagttagcaggtacggtcagcttcacgcgagttgaagtagaaccgacagacatagttgcatacgcagcgccctgaggcagtgaccacgttggcagagaggcatactcgtttgttgcacccgacaggcgagtaacacgaacgaagtaatcaccagacacagtgccctcagtgatagagtcatcaccgatgatttccactttcgacacgtcatcggttgggccaacaacggtgaactggacgttaccggtcttcgatacagtaccaacagtagcagctacgttgagctggaaggtcagagttccgtagaagccgctcaatgctttcttggtgcgaatgcgccagccagttgttccaccagcaacgatctcaaagtattcttgagccgcggtggacagcgtgtaagacagttcgccgctagtaccctcacgagtagtagagtcagagaacgtcagaacgctatgcaggtcgcgagtcacaccgacagcagtaccgaagtcatacacaggcgatggcgcttgtggctgaacggacagcaggctgataacgatgatgttcttaaccagcacggacttctgggcgttacgtccgtcgtaggttgcacgaatcagaacagttgtgtcctgagtcacttcaccagcagacagcacaccagtttgtgcgatgcttgcgattgcactaccctgaatcacagaccacgtcggtgaagctacctgacggtcagtaccatcagagagaatttcccacgcggtgtattgcgcagtagtgttctcgttcatcgaatcgttaccgcgaatctccagagaggtcacagtcggtgggttaccaacgatggacacaggcagagatgcagtcttcgtgatgccgttttcagtgtacgacgcatagagcgttacgctggtgttagcgataggaacagcgccaacaatcagttcagacttatcaaacgtcgcatagttcgaagcctgctgcaaacggaaatcgttcgggctgatcgttgcggtgtgtccgtcagagtaagtagccagcaccgtatacggagtggttgtcttctcttgaacagacgtcgggccaacaatcttgatgctcgacaggtcaacgacaggtacaacattcacgattgtaatatcgagcgttgcagacttagtgatgccgttctccgtgtacgttgcagacagcttcacaggaatgtcagaagacactttgcctgcgttgacggtcttgttcacgatagtaacaatatccagtcggtcagccgtaaacgtagtcgggtcaaccagcttggtgtggccgtcagagtacgtagcgaggaacgtatagttcgcgctctcttcactgcggatagtgttcgcaccctgaatagcaagagaggtcagcgttaccgcagcagtctctttcaggatagtaacgttcttgttaccagtgacggtctgatctgccgtgatgtacgtcgcagtcaggacgatgctgcggtcctgcgttgtctctttcttcgcagtcaccacgttgccactgatagtggtgtacgtagtcggtgcagcaacgaaagagttcggcgtaatcatttcagtgtcgccattcgaccacgtaatcttaaacgtgtaggcttcactttgctgagaagcaatggtggaagaacccagcacttcgagcagcgtgatcaactgagctttaacggtaacgttcttcgtcgcgctaaaggtcaggccgttgtactgataggtcgcagtcagtttaaccacggtatcagtagagactttcttcgcagtaccctgcaggccgacgagagacagagcgttcgcgttatccaccgtgaagttcgacggcatgatagttgcgacgttaccggacttgtagcgagcagtcacggtgtaggtctctttctgcttatagatcagcgtgtcagcaccaacgatggagatagataccagctcgtcgtcagggatgaatgcgttcttgatcagcaggtcgtaggtagcagttacccagttgccgtaaacagggtcacgcttacgcgccgtgactttcagtacaacgtcagcagctaggtcaggcgcagacacagtaccgtcttggtcgatagtcacaccgataacgttctcttcgatggaccattcaacgccagaagggttgtgctcaatgctgtttgaccactcagcgtcgatgttcagtttgacgctactgttatccgacatgtagctcgcgttgccgggcagactaatacgcaagttaatcaggtgaggtgattcccactcgacgttatcggcgttgggcttgacccacttaccgatatacttgttcgggttaacagggtcctgatcgacaatcgccagaacatacccagcctgcggttcgttagagcttgcgacttcaacgaatgcagtggcgttcaggcgaatcatggtacgcgcataatcaggatgatcgtgattagttggataacgcgcatcagccatacgtgggtcagagcttgacacagcgataggcatatcagggtcagtcgggtcagtcttagtgacaacactacccagacggctggtggtcgcatgtgcgatttccagatcacctacttcgatacccaggtcagcggcattctctacaacgaaacggaagaactgtttctgagcaaacaactgcgcgtagtcagtcacggttacccaggagccacggtggttgccgtcagatacagcagaggtacgacgcagcacatactggtactgagggctaccagtgttcgcgtcaatccaaatcaggttgtacggcttctcagaaaacgatggctcagtcagagacacaacaacctgatgcacttccgtttgatcgttcgcgttaggacggaacaagaaagtgattgggttacgtggcgtcagaccgcgagtacgagccagagcgatatactgtttagcaaagccgtcgatcgtggttacgctcattcattattctccagaatgtcggtcgcaatcagatggccgtatgatgctttcacggacgtatcagcgatgaaggtagaaccattgtcgcctacatctgcgtccatgttcactttgtcctgcacggtcttcacttcgaccaaaggcttctcggcgtgcatttcatcgtgaggcagtggtgtgcgcttatcggtgttacgtgggtcagagacagacacgaacgtaggacgaccgacagtagcaggctcagtggtcaggcgagcaataccgtattcgtcaacagacgcgttaggaatatcgctaccaccactaatgtcagcaggatcataatactgcggagcccacagagagttgaagttcttcacttcttcccacgtatttttgtagccaccagcaggctctttggatttacgtgcaaggaacttgcgatagaacgcgctgttcacatccatgcaaagccacacaacgttcatcggcaacacaacaccaacaggctcggctgaggcggtgatgaacgtacaactgatgttgagtgtcgggttaatctgacgaacgatttggtctttcgacgtatcatccataaagcccgtaacagccaacagagcagcagcgatttcattcagtgtagtcataaccgctccgttagtcagtaggttggccgagttcagattcacgtaccttacgccattgaagcgtattgtcttcaagtaccataacctgattcacagcaggaaccagctggtctttgataggcacatgttcttcaccgtagctaccgttgatagagatcatggtagcaggcttctcagggtgtgtgtggtctttcgggtcacgattgttagacaacgtttcatcgccctcaagcataacacgcgactcagcctctgggtaagacagatagccgataccacgagtaatcgaagtagcaagcggaggcagagtctggttgatgattttcagatcgtttgggtcatacgtctggtctcccatggcatcgtcatagaagtacagcgcagtccaaacatctttgtacgggtcagccaggtctttcgttgtgcgcttaaacgcagtgcggaaagtaggcgactcagggtcgtagtcaatccagatcgcattgatcggaaggactacataacgtggaactgcatacgagcagtagaacaacagacctaactgcgaaccatctttaggcagacggaacatgattgggtttttgttctgctggtggatattcgtaagcaactcaacgttactgatgaactgttcaagtttcagttccattgtgttctccgtttaccagaagcggtggttaaaattatacagggtcgcctgacttaggactggtagaaccgtatttaatacggaacatataatccaggctatcgaacgggaagtcattgcgatagacaacataatcaaagccaccgagactgacttccgctgcgccttggaagttgaagtcattgaactccatagcgccatcccatgatccagagaatccctgcgcggtctcttgaaaatatccatagagcaaacgctttggccatgcgacgtagaagaagcggttgttatcagacgtagattcattcggtgggcaagtgattgtttgaggactcgattcaccgagaatagtagtcagagaacggaagaaggtatcgttgtagtcttgaatcgacaacactttatcgtgtatgccaaagcgaggaccatattcaccactgaacggcacagacactctaaccttgttcgacgtagcattgagagtggtgctgacgttatacgccttagccacaaggtcatgctcgcctgtatcaaaaggcagagtgaagtcgaaatatgcagtcgttccagaagtaggcaggtcaagtttcttgagcactgtacccgctgcattctcaatctggagtgtaccacgcaaaggcggattatccattgcgactaagaatcgcagttctttgttacgcagcgagaaacagtattccaagttaccttgaatggtcaaagtaagcatagaacctcacaatacgaaaaaaggaggaccgaagccctcctcattgattactgactcagagttgtggaggtactgcctgtcgggttgatgttgaaacgatagatcagacgcttcgtagtacgcgtcgggtccaacacgatatccagaatcaggtcgccattggcgatagtctggttggtgttgttgttctcgtcacagacaacctgatagccctgagaaccggagctaccactacgcagaccacgagccagtttgatctcttcgagaaacttctcgacgatacctttcagatagccacgcaggatgctatcgttcgggtcaaacaggccaacgcggcaagtgcgctgacagacttcaagcacgtagcccaccatacgctgaatctgaatctgctggaaagcagagttctgattgtactgagtgctcgcttcccacaccgcatagccaccgcccataatatcaggcagcttacggatgtagttgacctgctcgcgcgtcattgcatcacggtcgtcctgatcatacttctgagcgatagcatggaagtcgagaggaccagatgcagtgatacccgcaggtgcgaaccagctaccacggttattatccgtgtaggcaaacacagcacaaatctgaccaacacacgcagtccacaggtagcggcctgtgtcttcgtcgaagattttgatatcaggcgtatacagagccatgttggtgtcgttgacgttcaacgtctgacggcgataacgaatcgctttagacacagactgctcggacgacgggatgccacaaataacgaagcagttaacgtgcgcagcagccgcagctttcatgccgcggtggatgatgtaatcctgagtaggactaatcagcagcgtcacacgaacttcttcagggtcaccgaagtattcctgatacgctttcgcaaagtcatcagaagtgcaggtatcaccgtcagcaccgccctggaagaagatgaagtcggtggtgaagaagtcgatatcggtggtgaagtacgggttgcgcacgaagcggaagttggagctttcgttttccatcgcgtgatcgatacgatactggcggtcaaactcatccgcataatcatacaggctgcactggtaagagtttaccggattgctgccgttctgatagttctcgtactcgtcgatataaaacagcttcgtgttatacgacttacggtcgtcaaatgggtcgagacccttaggacaggccggacgaatctgtaacgccatctgattgttccagtcacctgggttttccagaataacgtaaccgatgatgttatcgttcaacgggtcagtaggcaggaagcccagctgatcaggagaatctacaccgacgatgttaccatcttgatcggtatatggggtgatacgcactacaggctgaacagcagacgcgtcatcgacagtaaccacaccgaccgcgtattttgcgttcttagtgatacggacgaatttgagctggttagtctgtttagcaacaggcagagcgagatacaggcctaggccatacttgggatcttttgcaccgaagatgttcttcaaatcatctttattacgcacatcaacacgctggtttacagggccgcgacgagcctgaccaacaatgcctactactgccgtagataaagacgttgcaccaacggagagatcccgtacaccagtataaacaccagcagaggaatgcgttgagttaacgggcatgatttgtctccttatatgactgtctgaaattatcgtataagagactagaaacgcaaaaggggcagccgaagccacccctttgttttaacaatcgcaacctacggaatcgaagtccaatttcagtcccggatagagttcattaaactccgtcagaggcatattgaaacctgcggcacttggatgcccgtcaccgccacgagtacgcgcaatgtagcgagcactgcctttgtggccttccggatatccttgagaacggcagctaacatacacacggtccgggtcgcggtgacctttacgcaccagcagcactgtttggaagtgcggatagttttcgtagacgtgtgcgccagtttcagacgcgatgttcttatcgcaaggcacaactgcatgtttaacaccgaccagctcgttaggctcagagaagttgctgttctcgtcgatcatgcggcgaatcttcgcatcacggtcagcgattgcagcttcaccctgtttgataatctgctcaatatcaccagacaagataatcttatacgccttacgtacagtcggaggcatatcggtgtagatgataccacacttctcaacgtcgctaaacacgtccttagaataaccttcgtagaaagcgaatgcgcgtttgttagtacgaatccacagatcgcggtcagacaccagttgggcacagcggatgatgttgcctgtgcaggagtattgatgctgctggaactcaccgacatgcgacatgtaggccagcagtgcgccgctaccgccggcagcaaatgtcagagacacaggagaaacgtcgagcgcagcacattcggcagcatacttctcctgatcgcgaacatcgtgatggtcgagaactttaaagccaccagcgccgaagcgtttagtgaagatagccatctgcttttcagtcagagagaaatcaactacgacaacgcgagtataacctttgggatctttgatgaactcacctttatcatccttgatgccctcaagaccaggcaggtcttgcaacagtacaccgttagcgtcaacaatatcgccttggttttctgcatagacagcaggatagaagtgaagcgtatcgttgggatacgcgagtgctgtgatggccgcagcgaaactgccatcagcacatccttgatgatagacaacaagtgtagtcatgactaaacccagtggttgttagaattgtttccagtttgggcagcgcgagcatgttcaaccatctgacgcaagccctccagcgtccgttctaagtgatcgcgatagtgttcgtcggcaatgttcacaccgtgatggaatgctacagtaaacaattgccattcattcgattggcgcagtgcttccattttacggtaaagaatttcacgacgctcgcgggcacgtaacaaacgctgaattaaattaagtggatcgtgagattttgaagcaagttcaatgtgaattgcatctaaaccctcatagtccaaacgagccaaagccagctttgcgttcaggaacaattcgcggcgccgaagctgttcttcctgaggcatacggcggcacttatctgggtgcgtcatacgtgcaatagctttgtagattgccttacacttcttagcgaggacggcacgggaccacttctcatgatcggcctgctggtctgcatcaccttcgttatcacgcacttcgtggtcagtgtcttcttcgaagttatcgtccaccagcttctgcaagtcttctgcattcgctttgtcttcgaggtcgtcagactctgccatgttgataatgatggcctggagttcggcgttgagtcgctcaatctccataataatcggcttgttgtttttgttcagcttgtcgattactttggtaacgcgttcacaatcagcactgtagcggagttcgagtgcggctacttcttcgaggacttcttcaagcgtttcgccgccttcctcttcaaactgcgccagttcctgtgtgtccaccaattcagtggactgagctaacagtgctggaagttgagggataaccatcaactgagtatttgtcatgggcgagtaagctccgagattggtttagccaccagctctgcaatgcgcggcgggcactgagggttgcgttttaagttcttgtgcaaccactgcaagttgttacctgacgaagacacctcagcgcgaaagctgggcagtttaagttcgtcacggtgtttggccagcagcgcattcagttcattcagcaacattgtttttccttaaagagaagaagtcatcagttcgagaacatttgaaaccacatgcgcaggaccgatagagataccagtgtgcgcctgcaggtgaatacgtttcgtaaacagttcgagtgggtcaggcccaccgcctgtcactacgatgcgaggtatcttcgggaacatctcaaggatgtctcgcagtcgttcaatcttatagctggtgctgtccatcgttacgttggtcaacactaacaatgatggtcgcttgcttttgagttgttcatagtcgaagcgatcaccgtacaacgttacccagcgaggcttgagcgctgtctctacgctgtcttctacagcagcgttaaagatattcagggctgccattttcgctcgatagtcattcgggaaactgctaatcaccgtgatacgcgggtcagactcaaacggattctgaatcatcttcgcaaggtgagtaagctgtttggctttggagacaacacgacctttgaagtaaggcgacattggcttatagtcctgcgccgcttcaactacatcaaaagtctcacgcttgccaaacagtagctggggatctacacccagcgtttgcatttgctttgccgcagcaggttcaaaatcgaatgttaacacaataccctccgttgttcatgtcaggtatttacagatttgggctgcgctgccaaacaacgaatctgacattcagagcacgatcatcacgcaaggctgtttcgcggggatcatggcgataggcgtatttctgcaaatgctcaggcctttcgtgatagacgactgccgcatgagcaggattgggcacagattcataggtgtgactttcaatcactaccagattgtcgatacgaagaacaccaggaacctcgaacacagatggcagattgccaggcgtagttgcagtaccaagaactgtctcatgatactccacaagcgctttaactaacacacgaccaacagcagtagtgagcgtcagattatattcggttctaaattccatggtgttctcctattattacatcagtggcatttctggatcgacgtaggtgtacaagaacaccacgttccaaccagaggcagcttcagggttgttgtggaagcgatatccatagaacatcaggatgcccgtactaccttcacccagtgttgggtcatagatagtgaacgcttcttccaacttgagcgcgtcagcaatgctgatagcccagttatccaaatcaaacggaccttctggaacttcccacgaatacgaatgcttctgccagtgttcggcttgcatgtcagtatctttggaaatccagtcgagatgtttaagtcccatgtgcagagcgacagcgcgtggaatgccgtgctcgttcatgtaacgctgcaattgatcaagacgcattgcatagttccttaatggtgcgtgggaagactgtcacattaatgcgcgtgtgatctttgtgttcaggatgcggtaggcattcatgagacacaagccagacgttcgtgcattcgagtttatcacgcatcaccattaacaggttggacatgacagacacgctatgcacaaagttagaataatcgagagtgaggaccattacttcactcgtcggttcttcatcgccttggttccacaggctaacgttcatcgacaggcgggctgcttcacttctcaacatatccatatcgagagtgtgcggtaaacgctctttcatttaaactccttatagcttcaaaagagacagtctataaattagagagcgagacccttaagcagtaaacgcgcactggtcaggaattgacgttgtttgttttgaggcagcttacgatagcgctggaggatatcctctaacgaggcgtcttcgcctgtactcagatggacgctttcaatcgtgccgagttctcctttcatccagttggctttggtgacagttaacaggaaggtgccgcgatactcttccacgatacgaccgccgggcccgccaacagggttacgaactttggtgtgctcgatgtttgcgatacgctgaatcgctatgccgtcagggaattgcgcaaacacctcagacagatcaatatctgccttgttgtccggcgcaggagatttagcaacgaatgttacacggaacgtttcgccgccttcaacgtcgtactgaccatcatagatgatcttgtcgttggcgcgcagcgtgtcagtaatcagtttgaaaatcggatctgagaacatgctattcctcaatgtagttgacgagcataccgatatgatttgtaatcattgtcttctgctctgaggttagctcgctatatgcagggatgtttgggaactggcccttcattgcgagatagattgtttgaatatttggcgcttcctgctcgacgcgaccgcgatgaataatacaaccgcgatagatgaatgcagacgcagggctggttggtgtgagatgtacaggctcaacatagtcatatgcaaccaacacaatcgtattgccgaatacctctttcagcatggacagaggctcgtctgggttatcactttccagatcatatgtctcatacgtcgcgtcaacgatacttgtcgcagcaccacaaaggttgatgttcagtcggaggtccatcttcgtgtgaacatcacgcatatcaggatgcggtgtgagagtaaagcccttctccttaagggcttgacgcagcatttgggacacttcgatactgcccggtttatgctgcggtgtgttttgcaactgcattagaatcgcctcatgcctaagttagagggctggcctttcactttcgcttccggttcgaagtagtcaggcaactcgctatcaagcgcttcacctctcgacacaactcccatccaatcacgcagcttcttcggtgtacgcttcgctttcgcgtaaccaaacttccagcacatcttgagaacggaacgagcacactgcatagagcggtccatctttggatcaatgaacatacgaatcacaggtgtgcgcttgttttccatcggcgtcagaatacgacacgattcctgtttccagttcggctcgttgttcatcggcatgatgtaatacagcgtgtcccacttaggaacgttcaggccgcgctgcatcagcttacgcataccgacaacgcagcgtatcttaccttcacgcgctgcatcaataatcggcttacgcttcttcgcttctttcgcgccaccaaggaacacagcagcaacttcgtccatgtaatgctcattgatacgctgcaccaaacgacgcgcctgatcagtgaacatgattgggattgcgatacttcgaccggcatcgaggtctttgataatccattcaaagatcttatcgttgcggtctggatgattcgcaaggaacttacagaatcgaacccaaccacttttgttgttgtagttcgctttcgactgcactctgtttgaggtcttatgcagcgttactttcggcacaagctcctcaacaaacgcctcggcaatcacaggcccgaaaatagattcaatcaggtagtgacgtccgtctttacgtttaggcgttgcagtcagaccgaagcgatacttcattttcagagaggccagtacgcggctataacagcttgcgttaccagcgtgacattcatcgacgaacagcgtaccgtagttctcgttcagcaacttgagtcgcttcttcgagttcttactgtcagagatcagagactgataggtcacgaggatgatctggaagttcttatagtcgtccagagtcttcgggaatccatacagcttcttaccgtgcttctcttccagctcaggcaagttcgtcatcgcttcgatagtttctaagaaaccatcaaggaagtccttctggtcagccataatgactgtacggaatccagagtgacatgcaccagcagtaccgataactgtcttaccagaacgaggcggtgctttgaatacaccacacagttcgccgaacatcttctcgaacggctcttcctgatattcacgcagcttgcctgtgaacttcactttgtagtcgtaaggcacacgcgacgtaccgttaacgaacttcacttctttcaggcttaaccctgctgtcttttcgaaacggtgcatctcaccataaggaatcgacacataacgcttacccttaatgtcagagtatttcgccagcacggttatatcaagcagaccgccctttgaacactggcggcattcatcggacggtcgtatagaacgaaactcacagttcttgcacacggcattttcgaactcatagtgagtcatcttcttgatgatgttgtctgcgtccacaaccttaactggaatgtgcagacggctatcgaccaatactttggcagtcacatctatttccttgagttcggcagaccgtactcacgctgattgatgatgttcatcgtatcgacaagtgctctgtatgcgaagccgcacttatcaatgtccttgatatacaggtcaagctcttccttgagcaactcaagctgatcagcgtagcggtagtattcggccataatgtttctgacacaacgctcgcgttctttcgcagcgccgacggctttcagatcttttgcatacgtgaccgaggcgtaatcctgaaaccgttccaacatatcatttaacagtttcgaggctgtatggatatgcgtcataatctcagtcatacggcttcggtacgattgatcttgaattatcgactcggctactttgttcagtgcctgcgggtcagagatgtttaacgttctgaccttacgcatcttaaacagtttacgcgcttcgtcttgcagctcggccaaaggttgctgaaaaatatcgttggtcttataaatatctctcagcttcttatagcgcttgtcgttcttgacctttattcgaatgcgctttaggtcgtccattaatcacctttgtcagttacgagaataggactctcaggagtcttgtgtggcatagcaaagaaactaccatgctcgtctcgataaattagcagacccccagaaggaccttcgataggacaggtgaagttgtatagtttttcgagcggaggcatgtagcctacagtcactgcgttaaacgtacaccacttcgcggagacttcaagcagtgagccaacaacagtgtcggctaggcgcagatacgattgcttgaagtggtagctatgttctataggcgcaacgctatcaatatccagcgagtcaccatacacagctttataaatcagacagaaacgacgacgcccgcgcggggcattaggtatttcatacagaacatcatgtatgagcgaacaaacgtccccaatgaggacgtttttcttaatagccagtttggccagacgtgccgtcatgctggcagatacccaaagtacaacagcgtgtgcgtgtcgaacttatagttcaggctgaatgcgttcaggctattgatgttcgcaccatggaagcccatgttgtgtcgttcttcacgcccgatgttacgcagcaactcacggatgatacgcatgtcaagcgaggtactaaactctttctcaacaggcttcgccagcttcaagctgtcctgcacactaccgctatcgttaccaaacttgagtttgaactcttgcttcttaactaggagcttcgcgttcgtgttacctttcttctcaatcaacgtcgagatgttggcgaacggtgcagacaggtcacccttaatcacacaaccaatcagcggcttgccgagctgtgcaatcatgttgtccatgtaacgatagtcttcatcgcttgcctgaatcggaggcagtgtcagaacaaacgactccgcttcggctgcgaatgaactgctgtctacgtggaacgttaccttctcttctccgcagaagcgataaatcaaatcgaacatttcgccagtcagactgaaacggaacggcttcactttctttttcagtgcagcgcgatagcgagatgaagtccagtgaccaggactgacgaggctcaggctctcaccgtcacagataacacgacacatcacggtctggcctgtgattgtatctttcaaccgagtcagcttaacgccctgagtcatcgcgtcgataacttcacgcgtcatctcatggccaccttcgatatggtgatgcagaccctgttcgaccattggaatctgctcggccgataccggacgcagtttcacttctgctttgtacttgcctttctgttcgctgatgttcaacgtcttaccgtcaaactcaatgttcagctctttacgcttgctgatcagaccggtcaactgaatcgggtcgatgttcattaccgtgtcagcgtcggcggtcgcgcctggaacgagataagcaacgaaggtatcaggagtacggcccagaacgaacacgtcggacttatacgtcaccagcaggtggatgtgagtcagcttgtcgtccgactcagagaaacgcgttacgctatcaacacgtttaagaatatctgacaggaacgtaccgttcagcgttaggctgcatttcttagcggggttcttcggcaatcgacaagtcttcatctctatcctctaaaacaaattgtagtgtgccctgtatatttacagcattgaggcgtttgccggatgctgcaatcaggccattcagaacgccaacgaagtcagcgctgtaacagtcaggtgctatctggtgaacataaatatcatcaggcacgtcacccgggttaagctgccaagcagtacgcaaggcagcacccatgaatgccggacgttctaccagatgcttgttcaggaatgaacatacatcttcggccgtcatcattttttcgcaatccccttaagagcagatttgagcatagacttactgagtttgattttcttcttaggcgcggctccctctgtagatgcagcggctttcttcgcagcttcttccgctttgtacttctcgaacgttttaatgttcttcggaagttctgccagccactccttgatgttcttcttgtccttgttggtgagaggattaactttgtccatgctacgaattttaatatcgttagcccaaagctgtttcttcatccaatcggacatgagatgatactggtcttccataatgctgtccagtgtcttctcaacatcgaggtctttctcacccagctcgtcacgcttaatctcaaggccgtctttaatgagcttcctgagttgaacgtaagagaagttccaaccctgcacgtctttctcggacgcaccgatttcaaagtcaatctcaggcacggacgtgaacgcaaacccttcgtgacgcttctgcacaacttcgaccactgcgctggtcatcgcacgttcgatcatatcgagcgcaaggaagatccatttgtaatcgcagtcaacggtcaaggagtcgtgtacagatacgttcatgtcaaagtcagggtactcgccgttcgctttccaatactcatacttcatacggtccagaatacgaatcgcggacatcatcaggtcagaaccgaagccctgcactggactgtttaccgcacgacggtcacacgctgcatgaaccatgttagcttcacgatgcgactcgggcaacatcaggccccagagatgacgacgacgaccaaccggcgactcaacaaagaagttctcatgagcaaacttctgaatcttatcgaaccacttcaagcccacagggaatcgtttaaggaacttgcttttgatctcttcaatctcaccgacttcacgtcctgtggacttcgcaagccctttattgccctgctgatagatcaggccgaagattacggtcttaaccgcgttacgtacggacttggttacgtccattacgtttggaatgccgaagaagtaagcggcgttgattttgtgaacgtcaccctctgcttcgacgcggtgctcaatccatggatcaggtactgtacggaaacgatgacgcagcttacggccttgctcaaatacgtctgcaacgccctggtcacctgagatgattgaccaaccacgaacttcgtgcgctgagtagtcgaccttgataagcaggcgattcttacgcgcaatcagaatacgtttgatcaacttacccatctcactacgagacggtacctgctgcaagttcgggtcagacgctgaggtacgacccgttacaactccaagataaccataagtcggtctgattgaacggtcatgtttgaagtcttctgattcaccccagagcttgagcaggctgttaacgtaggcgttcttgagcttgtacgctttaccaagtttggtgtagagagacacaagcggtatatcagcatacgctgcctggaagtccttgtcgagcttgcccgccttcttgccgttctcacgtaactgttccccttctttcagaggcttgagcttcatcacatcgaagaacagaatctgtttgtgttccgacttcgacatatcgaacttggtcacttcgactttgcccataagacccatcttaggaacattgtcgtctttgcaaataaccttgttcgcagccttaacctcagggctgttcatgaactcacgctctacgtttcgaatttcttcgttgatagggctgttcggtaggttgagcttaaacaggtaatcaatgtctgcgcctgcacctgtcgtttcaagaatcgagaacgcatgaatctggtcggagatttgctcactgaccatcgactcatacttcttgtatttaatatcgttggctcgcttttgctgttgctctgcaatacggaacggaacgataacgtcgagacccgcatactcctgcaccgattcgtcgaggtcaacgtctgcgattgtcgctcgcatctctttaccgaacgacacttcgtggtacacctgacaaccaaactgcatcgtcaggttagccaagttataataaccgctaccggtaacgttcaacaacgacttggcgttttcatcgaacgcaaactcacccgcctgaatatcccaaacgtttgctgcataactacgaatgccgaagttagagcgcattacgttcaggtcgaacttcgcgttggtgtagatttgatacttgttatcgttgtcctcgaaataatctttgaacaactcacttaccctacgcagttctttcggactgaatggactgtcacggtgatagataggaacaacatacgccttctgaccgtcagatgataactgcaccgtcaagattttattcttaatacgattcaggttctctgtttcggtatcgactgcaaccttcttggcgcgcttcatacgcttcaagattttctcaagttgcttgaccttcgttacatacacgaggtcccagttacgcttcttaccacacgtaacttcatcgatcttatagcgcatccccttgttaagccacggcaacatccagcgagccatgtagcctaacgtatacgatgaacctttgatgtgcatcgggttcaacacggtgtgatagctgacgttcggcacatggataaagctgtgcttcttaccgtcgtacttcaccttcgttggaatctcaacaccgtaccagtgctcgtagtgatctttcgagaactgtattttctcgctgttcagtgctttgaacggcgctttgccgaaagtcagaacatagtctggcttgtactcaacaatcaaatcacgaatacgatccgcaaacgcttggtctgcgtcttctttgaactgctcgcccttgtcatacgtcttgaacatgttgtacgagacaacaaggaagttccagtcgtcaagagttgtcttggtcggaaacgtatcttcaagatactgcatctgattcaggaacaactcaccttccgtactactgaatattttgccgctacgcaaatcttcggtaggcatatggtctaggacgagaagtgctttaccacctttggcacttttacttatgtgttttagtattcgaacaccgtcatacgtctgctggtcagcaaactgttcaggtggatcgaagtcaagagctacgtgcttgattttcaccatctagtcctatcagagtgtgtaacgcaaatcgatggctgttatttacagatttagaaatgaaaaagggcacccgaaggcacccttttggttaaatattacagcgtagatacggtcgcacgaaacacctgatacgcgctctgataatcagagaatgtacccagctgctcaaatgcagacttaggcagatcgctcggtgcgcccgcggacgaatcatacttggcaacagtgaacgtaccacgaccacgagcctgtttgatagagccagtcattgtcgcagtcggtccgaacacaacacccgtcttgctaccggcacccatcacaaggatgcaatcttcatcaccacccatgttagcaacggtagcagtcacgctacgtttcggcgcaggcagttgcatggctttgaacatagctcttacgttctcaccatcaccatccttcatcagcgcagcatacaggaagtcatagccgttagcgctcgatgcgttgctggtgctaggcattcgaagttcagcggcagtgcgctcgcctttcttagcggccgcagcaatctcagcgtcagttgcatctttggtggccagcagtttgatgacgtttttgattgaacgcagttcgcccagatgaatctgaaccttcttgacctttttaagatggtcaccgacgaaggtcatcaaccagcctttctgctgcatgacaacagccacttccagtttcttatactggaaagagaactgcttgccggaagcatataagaacttaccagcacccgcaacaggctcaacagcgcggatgaagtcaggcgcatagtcacgcgcatcgcttctgatcagactggagtacgcaggagagaacgtgcctacgatagttaccggagcctgcggcttcccagcacgaggcttagcgacgactttgttcgggtcagttgctttgatcttgattgcacgaagaccgttaatggtagccaccagcgtcttggctttatacaggttcttcatggcggtgacaagattcttgccagcagctttcttcgcaagagcggtagtcgccgctgagtcgttcagcaggtcaaggacagcggacagcttcgcagtgtccagctctttgattttaaccagctcgtcaatcttcttaacgataagttttgcgttcttaccgaaaaggatttcagcgttggcgatctgcgttttgttcgcagcagagaccgacacaacagtgccggacgggagagtgatttcgtgcattgctgttccttaacgtttcttgttggtccagttgttctgcttaacaggcgcaggtgaggtgttctcttccgtgatttcgtcgtcggcgtcttcttcctcttcctcgacgtcatctacttcctgctccggctcaggttgcggttcagcctgtttaacaggagtagtctccatcacagacgcagcgagaggtgcctgagacacagtatttacagtagcaaccggctctgcctctacggcctgacgcgctttagctacttcaccaacagcgtgttcgtgaataacgtcagtggtaagcaacgcacccttatccttcaggattgcatctgctttctcttgatcccattgatcccacaggatatcaagagtcttgtagccatagttcatgcccttcggcagcttaccgcgaccattgaacggcagcccattagaaggagtagctggctcgaactcgtccatcatctcccacttacgtttagcctcgatacacttcgggccccagacgccatcgcaggcaccgtcgtacagaccaagcatggtcatgatgacctgtagcttctgatagaatttgttcagcataacgtgttgtcctattaaagaaggaggggccgaagccccttaccttttagactgatttgtttttcgacatggtcaatttcaacttgtcgagtgcgccagtgaccttcttgatgttcgtgacggtgtagcctgctttcacgatcttattgatacgtgcttttgcagtagccgcattcttcacgaacccaatccacatacctggcgcctggtcgaacgtaccgaacttacgagtgttcgggattttcgtgccgacgaagcgtttcatctgcgggttggtcttcaggtcgaacatgatacgcagtctgtcttccatgatcatcgggtatgccttgacgtgtttcttatcggaggcagacttgtgacgaacgaggaagaacttcggcagttgctcttgacctttcgttgccagcttgacgttgaagcccatacgcggagtagactcgtcaaagaagtccagtacgaactccagacgcttctccgacatacggtcgaattccagcttcttcttaacttcgatgaagtccagcatcgcttcaaagtcagcgtagtacgcacagtcgtagtaaacgtaatcgccgaactcaacgaactcgaagtccttgagtgctttcgcatcagggtcagtcgcgttcgcatacagtgccacaaatccgttgtacacggtaggagtcagctccagtgccatatcagcaccagtcgcttctgcaacagctttcgcaccaggcttcatacgagtcgtagtgttagccaaaggaggcaggtcagcagacttacggcgacgaactttcttggcagcttcttcaacaccttcgttgattggcttaccagtctctttgttcgaagcgcgtttggcagcacgggcagctttacgcgcctgagcttcaaccttcttctctgtctctttcgtatcagccgtctgcgtttcatcagcaacggtgtcttcaacttcaacacggttagcttctgcgtttgcacgtttgcgatctttctcgttcgcccacggcttacgctgttcaaagaaacgtttcaggtcgttcttgtctaccttagtggcaatgtgaactttggtcgcaggaattgcaacggtctcaccagagccagccagacgaacacgaacggtactgataggactatcgccacgcagcttgccgtcaaccatacgcacagtcacagacacgacaacaccgttaccgaactcagtcacgacaggtgcacgattcagagaatctttcagcccttcgccgctagtgaagttacggttacgcgcccaatctaacagacgctcagtgccccagccattacgatcagggatcttctggttagcaacaagcggagtctgatccatcacgcggaagtcagtcagagccggagtagctggcagagcctgcattgctgcaaccgttgtacggcgcatctcctggaactcttgagattcgatttcgttcaggtcacgcttcgcaaggaagtagtcaccgaagtcttccatcgtgttgttgtcgatcagcagcttcgcgctcattttgatcgggtcgagcttgtactgatcgagtgcttcgtaacgctggttgcctttctcgtcgaagcgagtcttctccagagttttccacatcagacgagcaaccttaccaacctccaaggtcttgttcgtcataacccagtcgatgaacacaacttcacgagccatgtcacccggcttaccgttctcgtccagcttcgcagcagcaacgtcaggacggaagatacgcgcagtagactgatcgtaagtacccggtgaccacggagtatcgcagcggatgatgcggctacccatctgcatgttgtggccttcggagattgcctgctcgttcgcaatcagaatctggacgttgttgtcagttttgaatgcgtcgaggttagcatctttgttctgacccagcttaccaacttcaccatgatacaccacagcaactttcttatagttggctggcagtgcgttgtagatggcgtttgctgcacgaacgtaacgcgtaaagacaatcaacttgccctgtacttctggcttccagtagtccggatcgtccggaggcggaaccattgaaggcggcagcgcttgacgcttgaactcttcggactgcttacgtgccagatacttctgaccgttatagacagcaatgtccagttcacgcggctctacgcctggcttccattcgaagatctgttgctcgccgatcatgcggtcgcgttctggctgcacttcgaagtgcttacgaatacggtcgatgatggtcagcactttcgcagaaacgaagttggtaacgccagcggcttcaaacgtcatgcgagcaacgtcatcacccatcgggtcagtcagcatcatttccatgcgctggaagtacatgttcaggtcagcgttgcttgccagcagtgcgcctaaatcatcaccctcttcgatctcgtcttcgtcaatatcgtcagcggccgtggcttctgcaccaccagcttcgtcgtcatcgtcatcgctgctaccggctttcttcttcgcagacttggcagcttcgtccaacttctccagcacttctgcgtacattgcgttatacacttcctggtgcagcgcagagtttggaactgacggatcatcgatctcaacctgaatgaaggtatcaatcgggttcggcagcatgaacgcccaatgcttacgcttgaacgagatgaacgctgtatggtttgccatacgtgagtgcgcacgacgaatcatttcaatgtcgtctttcgcgccgtcatatgcaacgtccagtgagtcaccgaacatagcaggcgtcatcagtgcagcctgaccaacaatatcacgcacacggtcagttaccagcgtaccagtagcgatacgtgcatagcgaacggacggagcagtgaacaccgctttggtgttgaagtgaacctgagagccagcctgaccaccagagaagttcttcactttatgcgactcgtcgagcagcacatagctgaacttgaagcggttaacgaactctacagcaccacgcacacgaacacgcacaccgccaatgtcaacgttgaacgtaccagtttgcaaatagctcaggccgacgatgaagatagtgttacgaggtgactgagagatcacgtcgtacatacgttcttcgccccacgtgttcacggtatcagcagtaataggcactgcgttccagccgtcaacgattttgtgtaggtcgtcacaccagttcgctacgaggttggaaggacagatgatcagagggcgaatgccttcttcacctaagtcatccagctctttgattgtggctgcaatatcagtcagaccgatgattgtcttaccaccgccaggcgcgataaagattgttgcaaagcgcggacgacgacgcagagttttgtgcgcttcgacctgatgcggcagtaatgctgcaccgtctttcagacctgggatgcgaatatcatcaatggtgataccgctgtcaggtttcaggcgttcgatctcagtctcggccgattcgaaaatctcaagagacttaggaatcacatcgctgtacatcgtagcgaatggcaggatgatctgttgcagacgacctgagcctggagcttgttcgctttcaatcagagaactaaacaatttcttgcgatcggcgcgtacaagcgactgcgccatttcacggtacaccgcaccaccgaagtagttgttaaggcgtgccatgtcagacagcttggacttctcacccatcacaaagtagtgggtgtgagacggcagtgattcggtggcagcctgaatgcttcccatctcgctcatggaagttgcaatcaggttagaaccacgcagaccagcagcatcgttcagcacacgaatcatgatacgcagcatcgtcagagcagggcgctcgttagacaggtctggtaccgagaagtcgttagcgatcagattctcatagaggtctttgtccatcgggctttcagacagagccgcatcttctgcgtccatgccgattgctttacgtgcattctccaccagcgttttcaggtcaggaacttgtttgttcttgagcatgaactcgtaggtctggcaggtctgcgcgatgatgttcagcagctcaggcaggttagaaccttctgtggagttgtatttgatcgtggactcactcacactctcaaccaacttaccgctaccggactcaactttggcagcttcaatcagcgtgtcatacgacggacggaacagagccataccaccagatgcctgattgtgataaatgttaccaatcacgttcgcagcagaacggaagttaggcgcttcacccggctccgcaaagtcgtagccgagagcatcagcaacgtccagagagttaggtgacttcatgccgacagtacgagtttcgttaactgccagcccgccgccgttcgaggtgttcacgatcagagagaagtcagggtcgataccgatgcacacgtcactgaaacgagacagtgatttggctttcgtctgcacatcacggtcgaagtccagattaccgttctggatagcgaacatgttggtacgcagcgtgtcgtgctcagtagatagcggcacacctttttcgaacaggtcttcgaggacaccgttgagcgtggtttcgtaggtcttaaccatctcaatgtcaatgtcttcacgacgaggcagcacagccatcgtaccgttaggcatgatagtcataccgtgttcatcagcaaccacgtcgttaaccacgtagccgaatttctcacgcagctttttcaactcaggaagagaagtggcagaagtcacataacgcggaatacgagcagcacgggtgataccagtacgagtagaaccagcaacacggaagtagtagctcgcccaaccctggaaccaacgatacagacacatggtctgagtgtcagcaccctgagagatatactccaccagctctttttcgaagttaacaatcaggccaccttcgacacgaatgtcggttgccagtgctacttcgttgaaatcgacaggcgtatcgtgactgatcttcatcgcttgcagcttgcgatcaatcatctgtttgccggggatagagcggatgccgattgtcatgaaatcgcccaggccgtcaactacggatttttccaagttgcggaacaggtcaatatcaatgccgttcattgatgggtgaatagaacgcagagcagcgttatacacagaccagtctttgtcgagcgggatacgaatcatcttcgtatcgaatgcgttggcgttagtgcgctcagtgccaaagatatccttatagatagtcttcgccacacgaattgcagactgcgcaatatcggagctgtaggtacgcaggttggcgctttcgaagttcgcgtcgttatcaacacgaggacggtcgctaccctgattgttcagaacgttgaagttaccgttcgaagccagcgggctggtggggcacggagtaccagacatgataatgtctttgccgccagggaagcgcgtactgttttcgatgatagcgccagaagatgcagacagatgctcggccagagcggtcttgatctcacgactcagcttatcgccgttcaacatcatgttgattttcagcgaggacgcttcgacgttgttcttgatgcgcttaacgaaatcgtcaggagagacttccagcatatcttcgaactctgcaccgttagtaacgatgtagttgatcaggtcgaaggccgcgtagatgcgagctacggtagaagcggtgaatacagccagcgcctcatagttacgacgggacttccctgtcgcgtacatcttcgacgtcttggcgtcgaattcgggcggcaagggcttgatagcaagtgcctgattaaacgtatcggcaatttgctgggtagccgttgctgacgtactaatcatctgattcatcattcacccagtttggtatagttgtcaatcatagactgccacacgctcggtacaggcaagcgacggtctgcggcgatatccgatagcacaacggctaatgcgtaagcacgaagaggactaagcccttcgaacttgtcgcgcgtaaacacagacgtgagttgttcgttggtcagtgtctgatactgcgcacgatactcggacagatacgtgccgtacttaccgtcatcaaccggcatggtatcagggatgctctgaatagacaacaatgctttcgcaagagcgtccataatcagaagcaggtcagcctgatcatacggtgtgatatccggcacgtttgaacgacccagcagttcgatgactgactgcggaagttggataggctctcgcgcttgagagatggacttcatgattccttcggcagcaccagcatacagcttaccgctatctgcgatgcccttcaaaagagtatgaagccgcgagtttacgtcaatcacggttcttctcctaaataaaaatgctcttgaccaaagtgttgagcctcttctccacagcatgacgtttgtacgtggacaggaagcaggttagcctgcgcgattgcagatgcagcgcaatagcgttacccttaacccgcgcacagtcaactcccaaatcaatactccacggatgccaagcacgaggcgcaagcatcacttgttgaattgttgggtaagtgtctggcacaacaggcagaggagactttgccagtttcttcgtcaaattatcagttttgaacaaggctttaggctgtttgttcgaaaaccagtaaggaacctgcttgtgcagtatctcacctactttcggaataccaccacgcgttgtctgcggtacatacaccagataaatatcgatcgtggtgttgatgcagttagcaacccgattgtagtcgctgttggttcgactatgcacctcagccagcctgaacttattgctgaactcaatacgttgcagccatcttttcaagtcagcctgttggaccttgagaagcgcttttgcctgctcaagagagtgcttggtgatcggtgggataggacgtaacaggtacgttgtgctgctacgagccagagaagaaataaacccttctacaacgcgctgcataccaagaggttgtggtagcgaatgaaagaggtcaaccgctgtttgtgttgagatgtacgcaccccaagcctcgatgtactcagggctaacgcagtcaggaaagttgcgtaagtccaatcccacgtctgagccatatttctgcaaacgactcaccgtctacctccatgcagcagtcttgaaccacgtcggttgttactgccgatctgattgttatcgcagtcatagcaaagcagttcgaggttatgtttcatattcgaaccaccctgcgcatgaccaactttgtggttgagaatgagttgtggagtacgagtaccacagcgctcacattgttgtccacgctcgtcgatgatgctcattttgagacgtgtccaatcactcctgtccatgcgaacgtgagtaccagcgcgagcacgttcaaatcccgtaacaccagcaagacgttgagaagtggacatacttcttccacgaccacccatagttcttgctgcaataccgccttttggtctgtatgccatgatgatctcctaaatacagttctatttacagacttaggcgctcgcgctaaatatctgaactgtcttcgatagacccgcctgataggcttgctcaatatctttcgcagcgttacgaatgatcgtttgcgtctgattctgcgcaccagcaatcatttcaacaggcagattctttttattccatgcgttaatctggtggaatacgccaaccagaattgtaccagcagactcagcgaaaggtcccatgacttcttcgttgagaatctctgccagttgcgacacgtcacgcagcgcacgaaggtcagcgataatctcacgcatctggttatagagttgcatcagtgcgtaaatatcacggctctgcttcttgtccttataggcgtcttcacagatacgtgccattgactgacactgcttgaacatcgtcatgtactcggcaatctggtcgttctcttgtttgataacgtcaggcacatcagccataacctcaaggaactgaccctcaagagcaaccatatcggtgctcaaactccgtgactctttcttcttctttttctttttgatggtatctactgcattctctttctttttcttagctttcttgggctttggttcatccagagactgcattgccttttgagatgctgcaatatccgaatagaagtcatcgggatcaatgtgtttaggcagcacgtctttcgaagggtcggacttctttttcttcttgaccttaacgcctttgctaactgtcttagctttcttgacggtggtcttagctttaactttcgctttactctttttcgcagatgcttttgcaggctgggcgaaagagccaatgtcatccaagcttatggccgccatgtgaaaatcctcagtagaaacgaaaaagggaaccccgcgaggctccctttagggtttgtttagaagctgtgacctttgatgatagcagcaatcttgccgaagtagtccgggctgtagcggaacatcttggcatagtagtccagcagcttgttaacgtcaacgccagcagcggcagacactgaatcaacctgcgggaagtgtttctcgtccaactcgtcgccagacagaacagctaccatgctcatggaagtaatctgctcttcctgaccctgatcgtcaacaacgatgaagctgttgtcgtcagttacgttagcagcaacgaagccaactttcaacgcacctgagttagacacgaagctaaccatatcaccgccaacaacgctggacagttccagattgtggcgagcaacggcctgagccagagtaggcatagacgcctgcaggttaacagtagccgcgcctgacacagaacgaatcatgtcgatcagttcagagttgtcgttcgcgttgctttcgcgtaccagaacgtcttcaccgctttcgctacggcgaacggcccacatgcgctcggacttgtccatgtacatgtttttcgacagagcctggaactcgtcacccatctgcgacacagggataacgtcctgcatacggctgaggatggtacgaacaaagctggtggttttaccctgctcgatcatagaagacgcaccttcaacaggcatgtattcacgattgcaggaagcgcttacgatggcgccgaagttgtctgcgatattctcgccgacgttgtgagttacttgcacgatggccacgctctggttgtcgttgagctggtcaatctgtttgatgaaagccttcattgtcatctcctgaatgtttcgacaatatgaaattagtaaacttagggtttagcctgtcacgcgataccgcgcattgacccagatactgcggttaccaacagtagcccatttggttgttgggctgtttgtgatgccgagcttgccaagtgcgcgagcaccgtcaatcgcaccagaaccctgagaaccatcaccgtcgttgattccggccttagacagtttgttcttcaagttcgtaacaggaccttgaatctgcgtttcaagtctgcctaaagcagcctcaatcgaaggtgttcggtccatgtttaagttgacgacttgccccgtaaagtcgaatgccatttgcccttctgcctgcaactgagcagcgagcgcatagtagcaactacaggtaatccagccatctaagattgtgccctgcatgttcgtgccactaaagccagtaacacgcgggccaatcatattgaacagcgcaagaccacgatagagataaccaatcaggtcagcttgcgtgtactccagttcaggaataacgttatgctgacgtgctttgttgatgtggtcttccaccagcgatgcagcaataagaacctgaggcgtcactgcccagagcttatatgtcagcatcttggttgtcttgcgtgtcgcagaggtgtagtgcgcgattaaactaatcggctcaaggcgacgagtagcaacccacacaggcacctgaaacacgcaggtctttgcacggttcacaatcatcttcacacccgcatcgccggagtcgatatcggatgcaacgatttggttattaagtgcgagctggaatctcagcttatcgccacgagtgtcaaagtggaacggcaacgtcagttcaaacgtttcgttatcaccgaacaacgtaacgatatccgtaacacggttttcagtcagtggttcaacaatgagttcctgactggactgcatgatcccttcttcggaatcataacgccatttgactgtcagacgtttatcgtccaccagccccatgttaggaatcgcaacatcagcagtccaatagccaggaacttctcccggcgttgcgactacttgagccagcaccgatttatcgtcagggtcaatgaggcttacgacaggccccatatcgtctgactgcggataaacgggctggtctagatcatcgaagaaactctcctcgaggaccagtacgttaccttctgttgtgcgcatatcagtctgccttagtgagtcccagatactcaatcagattgcgtagctggtcgttatacccaccttcgattagcgctcgcgccattgcgacgtggttcgagttaatcgtcctcaccactttagcctgatactcaggaacgttctgcatgttctgactcaggttgtagaagtaactacggacgaagttggttcgttccacgttgctcgcttccatatcgcttgtgtcctgcgtaggagttagcagcaggtagagcgcagcaagtagttccggactctggtcaactataggagataccaacgaggcagcaatcttcgtcagtcctttcgcaacaaaatcaaccacagtcttctcgatgaacgctgtaccagctttacctacgtttggcaaatacaagccaggcaggatgtagatgcagaagtaaagcggaaagtctttgcgcatcacgtcagagataagcatctccgagtagtctttccagatgttgacgttgaagtgccattcatcgtaaggcacggtacgcatcaggttcgacactgacagatctttcacttggttcgcctgagatgcaagatcgcgagcgctttgcgaagggccaagattcgaacttgataccagctggacgtagttgcgtgtaacagcaccaacagtgttgtacacaacgttcagcatttcaacaccattaccgttcagtgcaaagataaccgaacgaggaagaccgatagtgatgtactcgttattattgtcaacgccccacaggcgccagtaacgcccgcgaccgagttgagtcatcggctgcgggagaatacgattagcgcgaggtttcaggcagaacgtgaagcagataccgctgtcaatcatgatcactgaatcatcaggacgattcgaataacccatcgacatatcgttatccgtcgagtacacgttcaccagagtgaagttcagcgacttggtgaaaggcatctgagcttcaatcaaataggcgaggacttgacgaatgatagtatcaagcacataaggagaagcgctacgcatttgttgtggccgatactgaccaccatacgtattctccttgaatgtgcgatctaccttgaaatgcgttaacgccattacttgaccgactgtttcagcaggcgtttctgttgcgggttcaggcccataacatctgcaatctcgtcgatcttacgcagagtcaggacgcccttcgcagtaccaccagaaccggtcagagagatcttaacgaactcacgaccgttacggccgctgaccatctgatgcacaacgctgttcttaccaccacgtcctgcacgaagcgcagtagaggccatgcccaggatttcagtaacagcttctttcttctcggtcgggctgaggccaggaacgagacgcacatacaagctatcgttctggacgcgcacgttgtcgaagatttctttcttacgaccgcgaatggtgtgctgttgcagacccagcgtagtggtatcacgcaggttctgagtagaacggttgattggcttacgctcactgtagttcaggaagccgtcgagagccatcaggtggttgatggtacgcttcatttcaggagcagtagcaatctgacgacccatcgggaagctacctggaactttctcgtcaacgattgacgtcaggaagttttcgctgataccgttagcgaccgcgattgtggtagacagtaccagagcatagttcgggtagtgcataccgtcagagttcacgaagttgtcgatgaacacataggtctggaaacagattgggtcagtaccggacgcgatgaaagtacgagtacgaatcttcgaatagtcttctttattcagaatcttcgacaggtagttggcgatggttgcagccaacttggtatgttctttcggcgcgccgtttttaacgtcgatgctcatgagcttaaccagtttggtctgctggtctttcgcctgagtaataacgttgagcagagacttagcggctgcgttctgatctttgaatgcgctgaaagtcttgctgttaagaatctggtaggcaacggacagttcaccaattgcctgagacagttggcttacctgctggttgtattgagctttgctcttaacgtcagaaatatcgatcttagacaggtcgataacttggttcaggtcaatcgcttttgcctgtttgcctttgattgagccttcgatatcggaaagttcgatggccttagcgctgacggacaggagtttctgcgggattgtaactgacgtggcgtttgcgataactttatcgagtacgttacggaactctttcgctgtgcgggcaccacgtaaggcagtcatgttcccagagctatagtcaacagatgcgctgatactgctaacttcattgtttttggcagtcttagccatgatcatcctctactgggtctagtaatcatatcgaataaaaattagcgactcaggcgtgttttgtccgatatagtgttcgcactgactttacaaattttggtcgctataaacgcaaaaaggggcagccgaagccacccctttttgtttcgtagtaatgtcttaccgaccaggtcgattaaacagttactttaccttttttcttggtctttgctgcttttttcgcgccggctttctgagctgcggtacctttgtggtgtacctgcttctgggtagtttctttaccctttttcagacgcggcagcggtttcagcttcggcttaaccagagttactgctttcggagcgactttcggcgttaccagtttgccgtctttgatcatcggcttacgagctttacgcgcggccagacgagctttctgcttcgcaaccaggttgcggtagccggctttctgtttggctttcaggttgctcagagcgatggtctgacgtttcagcagcagcttacgtaccgcgccctgagagcttgcggtagttttcaggccggcctgatatttagccagacgctctttcagacgctgttcgatagacttcgctttgcctttagctttctgcttacgcaggtgcgtggcgcgctcgttgtcgaactttttgtccgcagtggttttcttcgcagcaggctttttagctttagcagctttcggagcctttgcagctttaggtgctttcgcagccttaggcgctttggtggttttcgcctttttggtaccagtagctttggtagctttcgctttcttagctttggaaccgcctttaaccggatcggtcggagatgcaagtttgcgttttacggccatgattatatcctcaagttacaattgaactttcgtcctgtggacattaagttttgaaatcagcatgtaaaaattagtatattccctaatactttcgtcaggaattttcctaaatctttttacatagcagcataccctatttcagataacaccgcgttaagttccttgcgagcacggatgcgcaaggactttttaatcccagaagccttcaggtaatcctttaggccatctcgtgggtcaatgtccgcaagcgccagctcactaacatcaactgtatctatattatcgagatcgacacgtttattcgtggaatttatttgggaaatgtttgggacgcgagtacggatatctgctgggatcgacacggtatctttaacaacaagacggtagcgaatcgcagggtttacttccagacgtgaccagtctttctgattttcaattgcaactgtttccaatctaaacccaggcttgctgtcaacaaacttctgttgtaccaccagctcacctttcttatactgcacacggatatgaatgaatcctttcggcagtgcttcgccaaacgttttctgatacggcgacccgcagtaagtgaaacgtttcttttccagaacctgatgcaggtggatgtgtccgctgattgtataatcacgcgggtctactttgatatccttctttgttttaagagggcgtccgttatcgccaagcgcgcctacagcttcaacgtgacagaagttgaggcaaggcttcttatgcttgatgctttctttcgcagggtgtggcaggaagttaacaacgatgccgtcaatctcaacctgctttggtcggagatagatatgcaacgacttgaggaagtcccattcgcagaatgtcttgatcaagtccatgctggtgctcgacatatcggcccagtcgtggttgccaccacagtaccacgtttcgataacgccttcgtatttgaggaagaactggagcagcttgcgctttgtctcgtcatccattttaaacttgtcggttatgtcaccaggaacaaagatgtgacgaatgccatgctctacagcgtactgataaatacggtcgatcgtttcaagctgacggtcaacgtgatcagtagggaaatgattagcaagcccctcgaagtgccagtcagcggtcaccagagcctctaacatctcagatacttttttctttttcatcaatacaatccacgagtttctttgactgctatttacagaatcaaaatgaaaacgggcagcataagccacccgttaggtttacttcattttagcgaggcgttcacgacgtgctttagcttcctcacgcatgtagacggcttcttcttttgcttctgcaagagctatttcaagcgcacgatcacagatggcttggatcacatgcttcggagattcatttggctcaaccagaaaattaccgctacgtgatagcacctcagtatcaggataaagttcctctctggcctgagttatacacagctcctcgtcgatgcggtagattaacgtggccagctctgtcttcttgaacttgttctccttacgctcaaacagaggacgcagtttagggtggaagtctctgcgagcatcaatagccacatacttccacccatcaaataccttctgcgcacattcatagtagcgagcatctacactgtccttgtatcgctcaaggcttgcgcgtgttgcagcagggcagataggagacatgttggctagtgagccgatggcgggagcaagcacgtactcgtctctatagctatcacctaccacgtattcttcgtctacatatttggtctgcacttcgcctgtattaacgcggcacgcattgtaccagaatgcactttcaggatttttggtatacttaacgaacgaccaaatctgcgagagtgcggcagggtatgaccagttctggatgttctcttccctgtttccgtagaagtccacatcaccaagattcgcgtccaagaagttctgacgtttagtgtgaggcagcttgtcaatgaagatttccatagctctaggcctatgcgtcaggtactgccacaacttgatcacagtcgggtcttcaacaccaagtgtatcaaaaactatatcgagatagtcgccgaactcttggtagtgtttattcacaagtagctcggtagcggtgcgcacataaaacataggctgcccccacttctcacgcgcgagcgcaagagcaatgctcggatatcggtccatataactccgtgcaatgtcttctccgtctttagtgcgctttgcagcaatcaaacgtttaacaaacgtgttgacgtcaccatgaataagaggactttcgagatcatagtcaaactcctcccagcggcgatctggatagagcttgctgcttagttcgtatatgcctttacgttcggttgttgcgaggaacggattgatgtgctcgtcaagccactcctgcagcacgtggacgaaaggcatcttagcatcaggataggcaaactcgaccagatagagagcgttcaccttttcagagcctacgaatcgatcggacgctttaatcttagccttcttttcaaagtaaggcttagctaggcagcgaccaataggcttgttgatgttcttgtctgatgggtcaatcagataggcaaccagagtaccaccagcgatatcctgtttgacatacttcttgttcgaacctgtcttcacgttcatgcagctaacccagccacgatcggtggacatacctgcaatgtcgtatgggtgcattgagatacaaatgagctgacgattacgcgtagcattcacaatagacttacgattcgggtcagagtcgaacatctttttgagttctggattgttcgataacacacgaccaatcttaacgattcgaccatgcttgtcctttcctgcacctgtcaggtaatcgacgagaacaatatctttctctgccagcgcgtctacgatctgaatcggcggcttgacgttttgcgcaacgtttttgatcacgttgtcgctctttgcgtctatatagatacgcatggccttgtggcctttcttaccgctaatcttttcgaaaagattgagtaaagtcgtattaggcttccaaccttttctgtacttgcggtacaacgaaggagggagagcggacagactgacttgaatttccattggggatctctgtgttcgggtgatgataaaaattagcgtagaaacgacaaacgccccttcaggagcgtctattgaattttagccagtctttccaccaatacgtaacgggcttgttttgcttgagcgcgtagtcaatacagttctgtgttcctgatggtgcaccacaacacaatgaaatcagacgatctgtttgatcaaccatgtagtgattgcgtttgttgagtgcgaagcctgcttgaccgtccatgtgaagccagtcttcttttgatgtgactattcttacttcgtggcttttattaagaagaccgtcaagttcaatcacgctactgattggccagcgagcattgaacccaggataaggtagacaggaaacaactttatgtccttgggatattgcggcagtcgctacagccatatcaaagccaagagcgcacccgacgtagatgattgcatcgtcgtccagtgcgagtaatctgcgatgtgcgaaagtatacaggcgatcttttgccttagggctgaatccacccaacgattgtgggcgatgaccagtgaaggatatcttttccatacagagtatttacagaagcacgtccgtgtgccgatacaattagaccgttacttcgaggtcatgatcgcctgagttccatacgagttcgcggatgttacgaggcatgatgatacaacccgaagaggcagtacccggagccttgatgctatcgccgtgcatctgaaatgcagagcgaccgaacatctcgttctcttttgctggagtcaggtccatagcatacggtcctgtcttctggctggtacgaggtttgttcagagtgtagcgacccacaggcagagggcccatgccgactacgttctgagactcgtgtttgtttttgtgttcgcctttacctgcgtagccacgagcgaccagctgatgttgagcgttgaacagttcacctgtagtttgtttataaatccacataaatgctccttatagctcagtggtgattggaaagaaactggataaatattgcatgttataagccttggttttttattgtggaaccacggcatagcacaaaagggcctacacctttcgatgcaagcccttttaagtgtcagactataactgtcttgatcacgttacggttcttctttgggtcgaaccatacttcttcaataatcttgcccatgccgaagttaatcatctgcaccgtgcgtcggctgacgagttgcagacgtttagactggaacatgattactccttaatcatcttgacgcgtgtgggatcaaagatgccgaaggtaggcacatcgttgtgctcaccctcattacctttaatcgagtcatacccagcaagtttgagtatcttgctgatctcggtatactcgtcccaccacatataaacccttttgtgttgcgatgaagggataaggttgctaagcgcgtctaatcgtttgacaagagttatcgcctcatctttgcccaccagatgcaactggaaggcttccatgataagttgtttaacccttctataaatctcagcgaactttacttccgtccacagagaacggaacttcaaggtagcatagcgaccagggtccgcatgaaacttgtagagacgcccaccttctgcatacagttcggcatacgcacgatctggagttacccaagtcatgtgttgcttcttcgcatgatcatctgaccagtcttctgcaagaccgcgatagtagatagtgggcgcactcagactgacaaagatctgcattacttacgcacacgcaatgcagggtcgttcgccttgtcatagcgatcaggtcgaacgataacaacaccggtaggtccagttttcacttccagcaagccaggaatttcaaaaccatcggcagtgtctgacacagggaatttcttctccagcagtccacgcatcttggtcagtccttcattggacttggcgatcttcccgcccttcatattacgaatcagaccagcactgcgacctacgttgaatttgaaaccaacagagttcaaaatcccaggcagtgctttatcgatctgagccgaagttacttttttgaagccaccttgcctgtaagaagttttgcacgttgctctttcagtgctttcttcttagaaggtgagtgggcaccggtgactgcgtttttgtttttagggaagagcttagccttctcacggtcaatctctgcctgagtaacagtctttttcttcgcacctggtttcaccttacgatcagatggagtgctggcattaccattgaccatcttttcagctttcatgaacttaggcttgaacgcaccacgcttaccagtaacaccgaactcggtcagcttggccgcacgaatagctttcagtgctttgtctgagccaacaccagttttgatatcggtagcggacagaggaagattcaaaccgcccagatgatgtttcttcgcgtgagagtttgcttcacgaatcagagctttcgcctgctttatctcagcactggctttggtcttctcggttttacgagtttccatcagcgcagtacgcttaggccctctaggcagttgacgcactttagtggcggcggtattcgatttaatcgaagcagagatgccagcgatagcagcggctttagctttcttcaacagaccaacaactgcctgcaattcagccttgtactcagtcgctacgatcagagtagtaacgccaccgacacgagctactttatatgcctgaggtttaatacgcgcagactcggacgctacggtctgattaacattgattttaataagtgccattttggattcctcaaaccagggctctgcctgggagatcgaagttcttaccagccgagtaatcacccagcgcctgataaagggagtcacgcagcatttgctgaatgatatccgagttatgtgccgaagcgtctttaaaagcaacctcgattgcttctgttctcggattcaatacagcataacgcagcgggcagatcttttgcacatcacaccacgcgtcgattctgatttgcaaatcaggcgtgattggaatacgaaagtctgatagttgaaacacaacgctctggataggaggaggtgatgactctgacttaacagtgtcagtgcctagcttctccatagccatcgccgcgttgtacacggaggagaacttggtcttcaacgtgttcgtttcgacgagcttatagctattagccgcaagtccttgacgacgcaacttggcaatcttaacaacataatcaccagagtcgtcagaagcaaatgcaacgtaagcgtagaacgcaaagccagacgcttcacgcagcaacttatgatctaaggcgcggtcgcctatgatagcattcagttgttgcaaacccatctggacttcgcgtgacagtgaaacgtagatctgcattagcgcaggcgagcgagagcctgtttagcttttgccagagtctgttcgtagttcgcttcgtcgtcgaactcaggctccatacgaatctcgatgccagagatattgaagccgacatcttcgtcttcatctttggtcaccatgccgaaacgtgcaacgccgtttttgtagctgatgaaacggaagtcgagaatatcttccgggccacccaggtcagacggcatgccgtcgtccagcagatcgaagaactctttcttggtcagcttgctgaacactgcattgatagcagaggcagattcggacttaacagcttcttccagattcagtttgataagggacatggttagtgtactccaacttgtttagtgattgtgataacacgctggtaccaaccatagatgttatcttcctgagtttcatctgcctttgcaatgttcttcaacttcgcaatacggcagccgttgtaggcataagccaatactttaatgtcgcgtactttgacataggcggcaagagcagccagcgtcttcggaccaacattcgcagcaggagtaaagtcagggtagagtttaccacgaccattcaagatgttcagttggtcttgcagttcagcgattgctgctggtgggcctgaattaacagcgtagtcgaatacccacagtgccagctcctggctatacttcgcaatttcatcacacttgcagaaatcccagaagttagcgctgtagatcttatacgcgatctcataaggcaggtcttgcatcgcacccttgtagccgtaggcgcgagcgttcttttcagtgacgccccaacgagtaggaccgccacggtcagcagcacggttagtgtacgtcgagccaccttcgcgatcaataacctcagcgatagcgttctttctaaacgtcaatgcgtccataataaagccctctgttagacagactaaaattagcgttagatgaacaagtttgtcttcttgaacttcatcttagggcgggtgcctggagcagacacgatagcatcaaaatcggtcgtatcgaacttacaaaacgcacggaactgaggactatagaagaatgctttgtccaacacaggagattcatctgcgcctgtttgagtctgagcaaatacaccatcatacgtcgggaacgaaatgcccggctgtccgttagcaccacttactgtagtagaggttgggagtcccatcatagcgtaaccaaagtttggtgtttctgtggctgcgtatgttctgaatgtacaagcaccagtagacccaccagctgaggcagtagtggccgcagtctcacctgtcgcccttacatatctaataccgatgaatcctgtagcatactgaccgtacggacagttaccgtcgtgcagattcataggaggcaactgtataggctgacctgaaatcattcctgttgtcagaaagacagttgttaaggtgctggagttaagcaacaaataagactgggcttcggcgatacttgagttaccgctcaatccccacgccgtattttgttgaacaatatcagtgtcgttggtcaaagaattggacgcagcgtgcatatacttcaaacaggtgaagtgatatttgtttgccttgcgaccacgaataggattgagaaagccgttgaagccaagcaccgctcgcgcggttctggcaagcgtgtttgctttcgtcatgtccgtaagcacggagaagtcggacggctctcgactgtcatatagaaagacgttaggcatagtgggtgagggcccagctaagccagcgaatgaagatatgtactgcatagtttctacctcaggtaggttgattacaaggtactgcgcgttgaggtaaaattagttccaagatcgacaaaaggggccgaagccccttagaatgtccaacgtgtcgcccaagcgattaagccggagagaataccgatgtgagacagatacgcgtactgcaacacgtaacccttcacgtagtgcttgagaccaccagcatatgcaccgtcataaatggcagcgattatggtgaacgacattacgtaggtgaatacgtgccacttcgtcatctccatcacctcgtaacagaacacaatcagaaagagagctacggtcatgaggtatacagtgcgtttgatttccgtcaggttaatacagagaacaacaggacgtatcagaaacgcagcgagtatcgacacccagattaacgtttcgtaatcggttgacatattagacaccctgattagcgagataggtatcggtgatgttcgaggtcttctctacgttaccgcgaatgtaacctatctcgaacacctgaacgttgtgtttgacaacagcttcaccaactgtctcacacgcaccgctattcaaatcaaggaaggcctgacacaaacgctctgctacaggcttggccaagatcttcatcagcgtgtgcttttggattgcagtcagcttgataggcagtgcgtcgatctcacgctcgatattcttacgaccgccgtgataaatccagcgacagatagttgcagtcaaaggcttttggtgagtctttgaaggcaacgtatagatgtacgtcatcagacgatagaacaggctgccgtcgattgcacgtttcttgaggtcatcaagatacttaccaacaggactcagcttgcctttctgcggctccatctgatcgagtttgagatcaacatcaagcccgtaacgacgcagcgtttcagaatgtccaaacacaaagacaatgtggtcaggcatatcacgaatagcaacagcattacggctatactctttctcgccgacaacgaacatgtacttacgatatttcttggatggatcaatgacaccaccaagtggaacgaaggtcacacgatcagcctgacctttctttctcagccagcccagcacttgctctgggctctgccgcgttactgcgattacaggcatcgttactccaccgtgttaagggcttgtgccgtgtactcacgcagagtacgttcgatattctgcgccagcgtcgggtgacagataagctgatgatctttcatgtatacacgcagcgaaggacgcatcaccttgcgaacctgtggatagagaccgaagattttatgcagaggtgtcttgtagtaaaactcctcctgctcgtccatgcagttaatgtttgccacaacttcgtacttggcaaagatagctggattgcgattgatgtacgcaggttcaatcggcacactgcctttctcgtgatcgctattgagcttaccgaagatcatcacattaccttacgcgttaacttagacacaccaccctgcttggtgatagtccattgattgtcagagaagtgctcaacgtccagaggagtaatccaataaacgttaggaatgatttgcttgagaatcgggaggaaattcttcacgatatgatcgcgtgtcgcatcactacatgagttctcaggttcatccagcacaataaagtttgtacggcgattagcaggaatgaatggcatgatcgcaacagcaaacaacaagcggaaacagtttgtctctgcaccactcatgattgcaatgtcagtcgtcttcttcgacaccagacgagtaacggttgcaccaacaccctgcttggtagtaaacagttcgaagtgcatcggctcagggaacaccagaccagagtattcgttcagcttcttctcaatctgtttgagacggccttcaaccgctttcagtttgagagcattattgctatacgccttatacaggacttcgaataccttgcgcttgtcgattagcggttgcaggtctgcgagcttgctgcgaagttcacgtaacgtttcttcgtagtgttcgtgttcctgaatgcgcatctggatgttctgtgccttgcgctccttcttctcaatgtctgcgatcagcttctcaacttcggcgctaacctttttgtactcaccatcgatcagatagaactcacggtcaggcttaccaacgcctttgattgcagcacgaaggtctttcagaatctcaagatccttgattcggttcttgattgtcttacgggctttcttaggctgcttaaccgctttaggtttcttgagcgcatcacgcttggccaccagcttctcatacttcttcgctgtctcgaactgttcttcgatttcatccagcttagtgccgactgcattgagttgcttttcaaggtctttacgtttatgcttcggcttcttgaccttctctgcctgcaattcagtgagctggtcattcagcttgtagtagtcgagagcttcgatgcactcgtcaatgatcgactgagctttcgttgcagcgcgagccatagctttaaggtcaacatcttgcccacaggtaggacatgagttgccgtcgtgatcgtgttcctgaaacgcacgatacgcctgaactattgctttggattctgcgcgggcatcttgtgcctcttcctgagttcgtttaggagctttgagcttagacagctttttactgagcttgtccacggcttctcgccagtcgtcgtactcttcctgttgttcatcgactttctccagtaacgcttcgaggctctcttcctcttttatcagtgctccgtgcttcttacgcagcttcttgttgtcaagcgccgcaacgtcaccgagtgctttgattttctttttgacttctgatagctcggactgatattcgtccagtgcttccacaaagtcatcgtaacggtcatgctcaatcaacagaccacgtaaggtattcagttcacctttgagatcgtccgtctcgatacctaacgtgtcgagttcatgcttgagcttctcgtacttcttcgcggttgtgcgctgagtacctagttcaatcaggagttccgacagttcgttacgtttggctttcatcttatccgactgcttgatgattgcagtcagcgtgttcttttcttcggcgtgaatcgacagcgcattttgtttacgctgtgtaacgtccagcatgtccgccagacctttcgattctgtctcggcatctttagccaagtccagtttcttcttcaacgccgcacggatgttatcgaacacatccagattgaataacgaggtcaggtactttaaacgatcagcaggttgcgcacgttggaagggatgcggtatctgcgactgaatgtaggcatagctgtagaactcgtctttcgacaacggccaatgctttgagatccacgaacgcgctacgtcctgacgacctaccttctggtcctcaccgttgtagtagactttatagctcttggctgtttgctcaatacgaacaataccacctaacggagattgccatgacagatcgataacgctgcccttactgagcatgttacccttgtctttctttttcagagcaagagggtcagcttcgtagagcagcgtaggtattgcaccgaacaggaggcttttgcctacgccgttcgtattgtctttaacgtttggactgtcgaggtttctgccgcagatagttgcgaagccttcactgtccaatgtgtcaatatcaagttctttgtacacaccaacatcgcggagatgaatctcttttaatccgatgccgtggttctgcttttgcttcgctttggccattagatatactcgaaggtttcttcctgaataagacctttaccgtgaatctgctcgaacacttcgatctcgtcatcggtatacggctcggctgcttctgcaatcacatcgtaactgacagattcgtctttgcggccttcaccgtagtaatgaacaggcttgacgatgcgccagacagggacttgtattagttcgcgctttaacattagtgaaataccgcagttggttcaacccacaattcagcagcgttatactttttacgcagctcgttcagtacggtatcagacacagggctggtggacgagaagatacactgaggcactttctcttcctgacctgttaccggattaatatcgtggtcgtgacgcattacgttccagcgtttgtttacgcggatattgatagtgtgttccatagttgtatgcccaggtttggtatgaaagatactgcttatttacagtttctaggcgtatagacaaaaagaagggccaccagcaatggcagccctgtctttagtagcgtcttggtttctttggcttcttaatcttgaccgacttaggacgcttgatacgctgcagggccttacgtgcctcagcaatctgaccagacagagtagcacgttgtttcttcacggcatctgtatcttggtcagtgcctttcaggttatcaaggcggttccactctttgaccaaacgatcaacgacagcagcacgactaacacgttgctggttggtacgcacaatatcctgctgcgtctttaccgagcgttgcgcttctaatactttggcacgtcctgactcaatgcctttcgtatcaccgtcagactgtttttcgttgagcgttttacgtgccacggttgctctgcgttgtgctcctttcagatcatcacgcgagttctctaaactgactttcgtttcttcaagtgggctggtacgcgcactcaagctaatgaggattttcataacggctccagaaatgaaaaagggcagccgaagccacccttttgtagaatggcgcgctatgcacccgactgttaagtctactacggttattttacctcgcagtagtcagcgaggagattgggatcacctcctcatgctgattgaagatcgacaacttcctcgtcttctatatcagcggcagaccacgaacgaagcacggacgcattgccgcgattgcccgtcagcatagatttaactgctggtttggcatcgcgctctgcatagtagttgctaagagcgttctcattagcgaaccacagaatggagtgaccacctttcgggcagatcaggaattgtgctggacgctgcggaacgttcaacgtcatataaaaatcaccagcaccagtaggacccatcataggcatgggtttcatgatctgcataaaatcgttggcatctttaaggcgagtatcgcctaacagccagagagcaccttcttcaccttcacgcacggcagacaatgtacctttgcgagtagtgattgaaccgaatacatcctgatcaaatcgagccagaccaaagataagcgatgcgagtttctttaaatcaggagtggtgcatgggctatcaattttcgccatgccctcagacccaattgtaatcttcgacagtgatacaaagatttccatttattgtcttccagagctgtatgattaattgtagttaaaattatcgttcagtcagacatttctgaaacaaaaatgggcagcactttggccacccatttttcacttatttatcacttcttctttttctttttcttcttaggctcgtcgtcttcttcgtcgtcgttgcctaaatcaacagtcaacttaccgctgtagatgttcgccatcacttcggtaattccagtctccagcataatatctgccggcaccgaagttgagttgaatgccacttctgcatcagccagagctttctgcaaatacaccaaactgaccagattgactttgatgttgtctttcttgatcatgttcatgaacatcttgagacccgcagactgccacttatttgtttcagcgtaatgccccaacacaccatgaataatccaacgagctttcgctacgattgcacgtgggttgtttgcttcccgcaggaactgaataacgcctatcaggtccatactgagataagcaccgatcatctgaacggctttggcttccatgtcgatttctggatcagcagcagccagttcagcaacgaggttcttatcaaagtcttcaccaccacgaacagaggcgtagatgttttgcagcatggtgattgcgccacgcatctgtccaccagcgtactctgctacctgatgaagtgccgcttctgctttatcacgcgccttgtctttcttcggcaggatatcaagctgaccactgatctcaatcaggcgtttatgaatcacgtcagttgcaatcggtctgatcggcagttgcgtcatacgactgatcatcgtgcctttcatcttctcagggttcgttgttacgaagatgaagactacgtgcgctggaggctgttcggtaatcttgagcagcttggattcagcagcactggacatgaggtgcgattcgtcgaagatgaacacacgacgtttgaacatcgggcttaacggggccgagtcaacaatcttctgtgagccttcaactttacctgcatcgccgcccatatcgaactcttgttcgtcaggatgtgcgccacggtcgtgcatctcacacgaacgacacttaccgcaggcagagaacgaatcacagttgatgtacttcgctaccagacgtgcgaacgttgtcttgcctgaacctagatgacctgtgatgatcattgttgacggaatcgttttcgacttctgccaacccttcatgatcttcacgatgtggtcttgaccaacgtaatcttcgatacgcttcggtcggaactgatctgcaaagttaaccgtggtcaactcaacagactcggaagaaccgcttttctttttcgatggcttatcgtcaccgaacgaacgcgacttcttctttttcttttcttctttcgccattttacttcgccctttattttgatgcgttacaccagtaatttacagattttagacaaaaagaaaggaccacatctcaaagtgagagggtccttatttataaggtgttggatgataacacatcggcagtgggcgctgacgattaggcaaagcacatttcccagcgtggaacaacgcggaagaactgcttaaagttggacggcggattcttcttgattgattcaagtttctgttccactacgtcataatcttttatgccactctctacggtgtgagtggtgaatgtaccgtcagcctgaatcaagtcggcgacaacacggtagcttggtttacgaagcatctattctcctgtgtaaaaattttctcgttcttctgaattatgtttacagtttactgcgagtagtcacacaaggataaagtcagacaaatcttaaactccaataggctctcaatcaagaacatattggagtccaccctagccagatgacggtctagccagggctttctccccgtgtctttcaattgcaccgacacggtagcgctcgcggtcttacgctctctgcggcttgcgaacatatcggcaggtagcagggttcgcagcctagagcagccgctttcggccattagcgataacgcggtgttacgctagttggcctgactctgtggccgagtctgtacaaaaaagagttcggcctatccccaaattcggcaaaagaaacaggccgaactaaacagtcagcgcaaactccctatgcactgttttgtactgtaacaaattagaaacatcctgcaataaatcagacaattcttagtctaacattggaataagattttgcaggaaatgctcacggtcaaacgacgaaattctgtgcggatgatcgatgtgcatgttccatggtttgttaaacaataggacgctacgaggcagcaccagttgctcaccgacgcgagtgaacttatcacgcacggcagtaacaggattatcatcgacaaggacgtaggtaccttcgccgtgtacttcgttcaggtacgcaatcttgtcaggatgctggcggctatccaaaacatgaatgtgatcgaacaatgacaggtgcttctccaaagacttgcgcgtgttgcgttcgcctttagggtgatatcctcggtgcgtacaaatgcctgcactgaaaccatcacgcaccaacattgcaactgtctggatgaagtagtcacgcatgttggcttcaagcataaagcggccgtcttccaacatatcaacgaaaggctcaagcccattctctggcgtgatgtaggaatcggtacctggatagattccccagttcatcagatagcacaacataaagttatgcgtgtcgaatgctgtgtcgtccatgtcgaagaaaatcttcttaatcattagtgcctcgtacttttgacaaccaaaggaatgtcattgatgaaagcgagagttagcaactcaccattatggcgcaatcgcatttcatctgcattcattacgacaacaatatcggcgagaggatctaccttgaacgttgggacttcgataagctgtgcatccacttcgctttcttcgtcgtcaacaacgtaatagcctccatacattaatacagtgtcacctgaatctacaaggtgaccaacgatacactcgtcaccatcaataaccatgtgcagtggttgatcgatgtagtaaccgttaccgtcatctgagtcgaactcaaagtcgaagtcctcgtcgcccataatctatgccctcaaatcaaccaagatagatgcagacaaatctcggagcatgtcacgaccgagaggtgtgtacattgtttgggaaactacaattcgttcaaggaagaggcgagaactgataacgtcttgccctgtgcgttgttgaacgaaatcaatgatggctgatggcggttgaatgaggaacgttaagatctcagcgtcatgtaggacgctacccatctctgtaacaggacgcatctctgtttcctgatcgagaatgtatgagatcacacggtcttcattaccaatgttgcgatgtgttttaaagaacttgcgagcagcactcacggtgcgcataaaatcgtagtccgaagaagtcggcatacggagaaagagtgaagctaagagcaggtttatttctaactgcgggccttgctcgatgtttaacatggcatgagaggtcagtaccacatctaacgagaagtcacgagtgtagagcgggtgagagttcgctgtctgatcgaagtagtcgagagccatgtgcagccctcgacgttttaacaggtgctctgccttgatacggttcaggcggtgcatcactcggcgccacgaatctctttgagggagttcttgatcgctttgcgcagcgtcttaccagtgtcgatgccgtcgatgtgacgagcgaacacattcgcaaacaacgtggtaggattcttcatgattgctttgtcgaggtcgggacgaccctcagcaatctgaatctcacccggccagagttcggcaactgcctgactgtcgttagcggcaatcagctccagctcacggaccgagatactgttctggcgagcaatcgtgcggaagatcatgtcaacgaaaggcagcaggtcttcggacacaacgttcttcacgtctttcgcatcaccagctcgctggaaatcttccagcagaccttcgaggtgagtctgcgtgatcttctggacgttacgcagtttcttgaacagcatcatccagcgcactttgcgtttggaactcagcaggtgagtccacactgattcgcctaaggcaatcatcagtttgttgtagacgtcaaccgacacgcaatcacgatcaacaaacacagtgatctcgtcatgccactcgtccttcttgaacttggttcggaaggagtgagtcttcgaccctgactgctggacgaagttgatttgcttgcagcgacgaatagcttcctgaaggccatacttagcaatcaccttcggaagtttcttcacggccagacgacaggctttagcgacttctgcttcgcgcccgtagagagcgaggcgaggcagaccaccatagacaggcattgatgcgtaaggtcggacagtgacgccacacacggacatacccggctcagggtctggacccaagaccgcaagcacgtcacctgccttaggactgaacttgatcgtttctgtttccggcgcaccaagcgtgttagccagaatgccaacagtgttgccggttgccagaacaagatgattcttattaccctgccttacgacaaggtaatcattttcactatgtttcataacggcctttaaaagattgagtcagcgatattgtaggtgtggacttccgcggtatgctgacggaagatacgaccttcggattgctcgaacgttgcaggacgccagtcttctttggcttcaatggagacgatgacttgctcgtcccacatatcaccatcttcgagagtcccggcgatcatacgaagcgcagcaggtcggtctttgccgagatgcgccagctccgcaatcatgacacgcggcttggtacgatcaccaagttcatcgagcgcccagccaagctcagacagagaacgaatctggtacgcttcgacttgagcgttaccacgatactcgtctggtccgaaataaacaatttcaaaatcgttgacgtcggtttgactgacaaagaagtgaggtgcgtccaccataatagaaggtgaggcgcacatctggagcatgcccatatatggattaggaatctcacgggcttctaccgaacaggacttcccagcaaaactttggattatgctgtgtgcgagattattcattgtaacctcagttctcaggagtaggtttggcagggcttggcgtatacataaaaccatagcccaccattttgttttgttgacgctttgcttgctgcttgcgtttgatctcggcgtcacgcttgtccagctcgtcaaagatacctacgcggcgagcataacgaaacttcggatgtacggagatatgtttgacgatagctgtcatgcgttattcctctatgttgattgctgttagtttacagtatcaatcactcttgcccatttggcgttcgagcacgtaagccagatagtcatcccacgtagcgaaaccatctttggccaacatacggtcaaactcgcggtcagacttagatcccttaggaaagcgaatcttgttggacaatcgttgcagtcggtcgtacatgaaccgagactgtttgacaatcgggttcttttccggcaagtgattttgcaacagcttgtaactgaacaccaacggaaaatctttgttaggtactgtctctcctagcaaacgatgcaccgtgttcaggtactgctcgatttgcgcgtgacattcctggtgagcgtagtaccagtcgtccagtgatgcaagtccataagtttcctcataaaccattgcgtcatacatgaccatgagaatcggcttctcttccttcttttctttgtacgcctgaaacaaaactgggcaagtcccatatttgttttgcagcatcgtttccaagattgctgcgaagcgtacaacttcatattcggtaagtaccttactcatacttcactccgagaatatctttttgtcagaaaacttcttgagcacaaactcggcacaatcgctcgtcacgctgtctccatcaacgcagagtagcgcaccgtcatgctcaagggaatacacacccttgacgttcggacaattaagaatagcatcgaacaaatacaaactctcccagccagacagcatgtggttgagaatgcgtttgtcaatcttcttgcctgtgtcgtcaggatcaggatcgtagttagatcctgtcgggcactggagtaccccatactcgggtcttcgtgcatttttattcttgcggaacttagaccgatacacgttaagcaattctttgatcgcaagatacagaggagtcatcctcgtgttccagtctaagatttcctctttcactctcgaagctggtacgaagcgagctaactctttatagacgttgctgtacttcgttggttcaagttgacctgccgaaaaaattgtaccatacaaacaaaccttggctgcgcgtctgtcaagtttcataatgcggctaatgtcgtcaacagaactaatctggtcgaacatcgcacacgcaataccgtaagcgtcaaactccctacgcaacacgttgaactgactggacttcatatcccagttagtgcctatcgtgtagcactgctccttcaagtccgaaggtaagttctggaacccaccaccgacctcgaacaagcgtccgccaatttgcgatagcctatacttcggccagtagcgaacgactagaggtttctcactaacgatctgaacaggacccgacacaatagtatcgagtaacgttttcacctgcaggtattgcttcttcgccttatgattagcaatcaacgatttgtcttctaaataagcaagtatagggtcgatgttcacttcattaggcatcagcttatcaagtacctgtcgataaagagcacggccactaagcaccttagagtttcctctgtctcggttgcgatcaagcgaactaagatcgtgcgtagggcgtttgaaaggcagcttagaatttttctgaatctgtgaccacactgtcacaccataatcctcccttaaaattttaagaggactatagaaacgaatgcggtacaaaatatcgtaatgcgactgcggcttaaaatgcccgtacatcccgtctaagatttcaggacgcatcctaaactcccgactaaggcccttttctttgttgtaaggcttcgtttcaaatacgttagccatcaaccactcaagggacctaccgtacgtgccttttttagacttggcatatcgcccgacagcaacattatcgccacctcgcttgtgtccgaagaccatcggtagcttttcttttcctaatgagcttggaaacggcacccagacccgtccaaacttctttttcttgtgtttacgtgcaggataaagactgcattgaagaatgtgccagaagaataagttcaattgagcacgaaactcagatcgctcgctctcggggccgtcgtagggacaggcatcaagaacatgttttcgcacccacaaaacaacttccttctcctggtaagaggggttcgtgattaatactggcccctgaccggaaacgattcgttttttcatgttcacatcatgattacctgatttttctatcgtttctttacagtttcagacaactcttaacccgaaagctactacagcgctaatgctaggaaggctaaggctacagcaggctagctacaacgctcatggcatgcttcaacaatagttctacaggtacatctttaggcggcacgtttcagagacatagaaaataaagaaaccatgtcctcagcagcccgaactatagtccatacgcactacaggcagcgatctagcggaaatccctaggtcgtctaaaccgtgtaaattttccgtcaaaaacagtccgttttttaaccaaacgccctttttgactctgaaaatgaggaaaatccgagaaaaatcaaggactttcccctcttttgaaacgaaaaatcagatcactttttctgtgaaacgcgttttccgagcttaatcccgatttgagtcagaattttcttaactgtttcgccgtcatgctcttccatagcagcggctaggcgttcgccctgttcgcgcgatagctcaggcataaccattttaagcatctgcgaacgcagttttgcgctctttgatttgcctttcgagacagacacgccttcattcgccttaagcgcactgctgatcgctttctgcacacgacgatcaccaaaaatgtcgccgaatatgtcaccgaacaggtccttgaacgacaatccgccgcccataatgtcgtctttcgtgaaacgaacaggtacacccagcgcattagtcttcgtacagtgcgtactttcaacctgattcgatgtacgtccaccggcacggaagttctcgtcagggcgtgatgccttgccctctgcaccgggcttagtgttgccgttgcgtaaatctggatcgccttcaacctgtttgttttgatcaaacatatcgtcggctgtttcgctttgatttgggtcgaacgggatcttacctgtcagcttgtttggatctggccagctatcaggaatatcggacgcaggctgtgccttgttcgtcatatcaccgttcgcttcaccactcaaactgatcttaatacgagtcatttgaatctcctatcgaattttatagcctttgaaaatgttatacgcaatctctttgcgctgtacgggacgagtgacgcacacccattcccactgatcgtttttcgctgtgcgtttcttcggtgcttccataactttcagcacgtagtttttgaaaggcagaacgagaatgtcttccggctcaatcgcgccgctgcgagcaggcagaactaccgtgatgttgccgacagtcagttcctgatcgtagttgagcacgtttgcttcttcgctgatgttgcctttaacaggcggaacacctaagtcaaagatcatggtgcagtgcgtgaatgcctcaatgcctttgacgcgaatcgttacatgcttgccgcgccagcgttccagattctctgctgtcagatcgacttcaacgccgttcactagcagcataggacgtgggaaagcaggaagcagagtttcattcagacgtatcgaataagtcgcctgcgtaaagtattttggaataagctgatcaaaatcagcgtagccgtctttacgtacctgcctgaatgttgcggggctggtggactgatcaagagtatagccagtcagctctttaatgtgatgatgcgtagcgatgttgtagacaaagccagtgctgataaagccgggcacaacaccctgacggaaacagataccgcagttcgcaacgttgccgccgtcccatttaacgtcgaactcctcacctgagtctacgcccatgatatcggctgcgtccataacggcgttcatgccatcatcaatatcgtcgagggttactgcttgacgtccaccgccaaacatgcccttgcctacggtatcgatcttaacgccgcctgacattgaatcagattctcggccaaggcttttcatgcctgccggaatattgtccataatgtcgttctcaaccttgttgcaactacaggtgagacccatcttcgctttcttgaagatgacaatatcggtggcgtcaaccgcaagcgcctgttcgactttggattgcacgaccttctgaatactgtcgaggcgttgctggacacgttcagtttcgtaggtcttgtgcctgtcataggtatttcgtggtctcccacgttcaatccagctcataaaagttctcctctgtgtgcttgaaattagtgactaagaatttaggaccttctgcctagcaaatacttatttatagcatgttaaatcacggagcctaacatgcgtattctttcaggcgacccgggaaaggttaacttcgcgttgtctgttcaggagtttaaggacaatcgcattaacatactcggcacccggatgtttcagcatcctattcaaaacctgcattacgatatgcgccagccggtcaaagagttcatgaaggaactcgaagacatatggaagcgctatggaccgtttgatgcgatgtgctttgaacgattccagtcgcgcggattgggcggcaacaccattgaagcaatcagtcttatgcttggtgtgctgtcaatgttcgcgctgaaaaagaattgcccgatcgatttgatcacggccagtcagtggaagaacgcgtttaaccgcactatggacctaaagggctattacgcggaatacaatctgacttcgaaaaagagccgcaaagcgattcacgaatttgacgcaagccttattggcatgtataccttctaccgacagacgaatcggaaaccttttgtgggcttcaacagaatcgttgacgtttacgttccgaagttcttggcagcacctgtactgtgaggcaaacatgaaacacgaacaactgctcgctctcgttaaagatgtagtgtctgaatttggcactcctgtatacctcgatcgtggtcaggttggcgagaacagccgcacgtatgccactatcgaaactctgatcaacgttcagtccgacgcacaaggcacgacgctgctgcaagatctgaaagcgaagatcgcagagtatgttgaactgctgcgtaccgaaggcacgacgcgctctattgacggagccgttcagcgcctggaacctgttactcagggtcagaagtttacctaccgcgacccgatggtaaacgaaattcccaacggtgtgctgtactctgtctccattggttttcccatgtttgtggccaattaatctgtaaatatccttacttggttaacatggctcgtgggatatagaaatggcgaagttgaagaaagaacaaaagacagttgtggctaaaaaacctgcgaaggtcaagcagtccaaagccgtcaaaacaaataaaggaaaagcagtagctattcatgttgttcaggacacgcgtccgattgtgcattgccctgaaatggaagacaagcctcaaccgtttcgttttcgtggccagtgcccgatcacaacatgtcagtattgcacccgcgaaacgcccaacggctgcatggcgcttgaccgcaaagaagctgccgaccgttcaatctctaatagggagatcgcttattacaaacgtggcctcttcccagaactcaaagagatggatcaaaagcagttggacaatacgattcgacgcgcacaaaatcgtacccgtactgctatctgtcttactatgtttattgccgggattgatgatagtgattgcgataggtcttttcagtatgtagaaggccgcagtcgcattgtcgatcaggttcataactatctggtgcaaacgttcaatgactaccgtccgtggatgctggcgtatctcgacgacgaagaacgtttctctcagatggtaggcaagataaccaattctgactttaatttaggtatggcactgcggttaacgcctcgtaagtatcagacgttctgccagtcgctgcaaaaccttaaacaatctggagactcaaatgagtgaaattttctctctcgatcagtatcgcgctatgattaagcgcaacatcctgagcgagcctcagatgctggtgaagaaccaaacccaaccgctgggccaaatctctttccagtgccctggtgacaacttcaaaatgaaggacgtcatcatcccagcaactcgtaacgccgttgacctgactcaacaggcaccgttggaaaatctgctggcgtgtagccaactgaaatctctgattcagttgcagcgcatcgcgctgcttaaccctgaagagatgccgcagccgggtgaaggtatctctcagccttctctgtctcagccgcctgtcgctggcgcgctgtctgttgacggcacaactatcccgaacgctgttgtgattgttgagcagaacggtaacgtttggaccagcacttctaacggcagcggtgtcttcactgttgacgtgtctggtctggaagaaggcccgttctctatcactgtaactgcgaccggttatactcctgcgcgtttcgactacgaagcaggtccgcaaccacggcagccaatgcctgaaccgactgtacatgctgtctttaaagagacgactgtttcgggaacgactgttgcgaatgctaatatcgttgtatctgtggcgagcaaacagttcacgggtcaggctgacgatgctggtgcgttctctgtgaacgttgacccgctgccgtttggcactatctacctgacgctcactgctgatggatatctggacaagcaggttgatgttgttgtcgatagtgttgccggactggctcagattgatgcaaccgcattcctggctactgacctgtctggtaaagcaaaccctaacggtgaagtcgaaatcatgatcgacggccagtccaatcagttcgctactgctgatgcacagggcaactggactgcaactgtcggcgcgattaaaggcgctgtgtctattcgtgctctggaaattgatgggtacgatgaagcgactgcaaccatgcaaccgaccaagcgtcagtttggtgcaatcgttgttgatgacgctgatgcgttcggcgagacccgtaccgaagtcacaggtagtattgctggtctgaatgccgaagcgaatgacattgctgttaccgtaacagttcaggctggcgtgtacgaaggtactgtcaatctggcttctggcactttcaacatctctggtgttgatgcaaaagctggtgtgggttctactggtgtggtcaacgttacctctgcgttctacgaagatggttcaacgtcgttcactattctggaagagttctctccgcctacgttgcagcaagcacaggatggccagactgtggtagtcggcgatacagccgcttctactcaggttaaaatcacgatgaacggcgaaaccaaaactgcgtcttcaaatgcgcagggtgcgttcagcgttggcggcttcactaacgttgtcccaggtccggtcaccatcgaactgtctcgcgctcaatatctgactgcaaccttccaggtcactcaggtagttcaagcgctggcgcaactcgacgctgatctgaaagctggtgaagagactgttgcaggtcaagcaactcctggctccaatgttaccttgacgcagggtagcgttactggtgacgcagtagcagatgcaagcactggtgagttcattattacgctgtccggccctctggttgaaggtcaggctcagcttgtggcgcaacatgctggttatgttgactacaccgacaccttagctgtcgcggcagcttaatccttttacaggggcttcggcccctaatagaaatgaaattcggagatttacaatgagcaagcaaaagactaccgtacagccgattactctcgcaacctataacgagcgctacggcaaagacacagttgcaccgatgtatgtcgctaaccgtaccgagccgcgtggcaacgtaatgttcagcgcgaaagacgatctcggccagccagtgcctgtactcgtacctgcaactttcatcccgatcgatctgacccagcaggctactaaagacagcctgttgcagtctactcacctgcgtcgcgccctgactatgggccagctggttatcatcgacaccaagagcgccgaagagtatctgcgtaacagcaagatcgctcagaccgagatgcgtaatctgaataagatgaacgcgtctatcgctgctgacctgggcgaagaaactggcgaactggctgcaatcgatctgggcggcggtagcaagaagaaagagatcctgttcgaagacggtgatcagtattcttctaaccagttcgttaacgcattcatcatgcgagcgcaagaagacagcggcgagtctgacgacaatctggaacgtgaattcctgtctcgcggtctcggcctgcctgtgtctgagctgaacattctgcgcgagcatatcactcgtccggcaatcgttgagctgatcgttcaggcgcttgacgacgcgtaatccaaagctacaaacaaaaaaatgggaggccccgaaaggagtctcccatttttattactgctgctgttctctcatgcgatcaagaaacgctttacctgcgcctggcacaagcactcgaggcttgaaaggaatcttattgattctgcgctgcatgttacggcgaaagcgttcacgtagtgcctgaacggtgtgttgcttaaactgtgatctgaatttcaaagccattctactttcctttcttctctattgcctttggtctattccacccaagttctttcgcaggcatgatgcacttcttaccgtgaatatcacgcagcgtcatacgaacttctttgatcaacttgaatggtgcgttgtcggggtcgagcttaatcagcttgccgtcttcatcaaactcacgaggtagtttaaagtgcttgaccggtactggtgagttacgttcaaattcatctttgatctttgtgcgcaacaacttcccaccaccatcgttatctgtcatcgtatagacaacactcacgccaagcatttcaatcgttctgcgtttcgtttcaccaaactgctctgcaccgagaacagccagcgctggtattccgtatgacaggagagccagagcatctcgcggaccttcgacaagaacgatgtagcgcaacttgtacttcttcaaacactctttgaccagaggcagtgggaacaggcctttgtcttttgcccaatcgccttgcgagttcacatagctggtgccgttcatttgcttacgcagataagctgcaatcccacctatgtatttcgttccatgcttacacggaaagaaacaaacgtttgtgcctgtatgctgcgcattaagcagaccaccagcagcacgaacaagcgcacccggatatccacgccactcaacatcaagcggccactccatgtatgacttacgtccgagtgctttcatcaatagaccgacagacggataggtaccaatcttcgagccaatctgatcatacgttttaagcaaggcactgagcgagttcgttcctgcgtcttttaacgcccagcctttgatctcttgcagtcgagcgtgagccgctaatttattccagccgcctttctcgccacagccgaagcagtgaaagaatccgagtggtatctccatgcctacagaagtgtaaataccacaactaggagtcttatcactgtggaacggacagcacaccataacagtgtcgccgttatatttcttctcgcccggcagtttacctatttcgtcaagaattatctgatgaacgtcttctgccataccatcctctgtctatttcgtaatttacgcatataagcatatttacagatatagggataactagaatgggtaaccagcatcgttatgtagcttcggtagaacgtcgcttttatggacctcaatggttggcgctatgcgacctgattaaggtagagcctcagacgtgtggtgcgttcgcaaagaacggccatatgatgggactgactctgcctaaagagtttgatgttgaagctgcaacaaagagcctgcgccttgtctacgcagtcaaggaagaagacgtggccgtgcgctgttacctgttcggtactcgctactacaagttcgttttctttgaacaaacaattgccgtaagcgaggatgattatgagaacgttcgcaaacgtaccagcgcgagtcaatgatacccgcgctctgtctcgcataggcaagatgatcgatgcggcactcgacgtaaaaaatcaagagaagcgctggccaaagaaacgcgtcagcccttcaatgtttcctatctgcgcgattcaagaaactgccaaactgatttaccagaagcacaacaagtgcatgacaggtgagtctggtacgttgctgaacatctttgcgaaagcagggacagggatgcacgaatcgttacagaacgcactgggtcatagtggtcagatggttggccactggaaatgtacgaacgaaaaatgccctgaatacccaaagaccaaaggtaaaatggttgacggtaaatataagaagggcaagtacacgcgaactcgaagcacgaacaatcgctgtccgacgtgtgataaacccatggcttatgcagaactaaaagtcctgtataagtcactcaagggttacgtcgatggactgattgataatcttgatggcacgtatagcctgatcgatttgaaatcgactatggtgaccaaagctgctgacggatctttcttcgttaagtatcaccgcttccagatcgcaacatacgcatacctgctgaaaaaacgttacggctacaacatcgtggactataccctggtttacgtgccacgcgacaacccgaagaagtttgtcgaaaagacctttgtgtttgacgaggcagagtcgaaacgtgccaaagactttatgatggaacaaatacgcgcatgggatgctgcggtaaaatcggcgcgcactggtgatctgctgccagctattaaacgaaagccgtgcaagagcgctgagtattattgggacgagttccacggatatgacacatgcccttttgttgactattgctttattcaatcacacatgattgacttcatgaagaagttagagcagcgaatcatggccaaccccgacctaacttatatggaaattgtaagcactggtcggaaaactcaacaacaaggtctgctgccggacaagccgaagaagtcgcaacgtccgaagcatatcgtaaaaacatttgagctatgagcatacaaaaagattatgaacgatcactgcgccgacttaaggagtctgtctatcgcactgaacagttaggttatgttgtgcctcgctgtgttgatattgttctctcaaagttgaagccgcctgagactgtatcgtctaggaagtatctggtcatgttgctgctgtttagtcagacctgtgacaacctacgatctgctttgacaatgagagagcaactggtagtcaagatggccatactcagtcgcaaacacccaacgccagagattcaacgtcgcatcagacgtcttgaagaactggtcaataatcaggataggaatatcgaaagtcagaggctgctgcttgattacagagcaaacgtcctgctggatatccttgacgggaaagaacccaactcacgatacacttgaggtactcatggaaatttatgtaagcctgagtcaggactctacagacaagaaccgcaacaaggtatcgagtccggagtccaacaccggccgcgttgacgtgtctgaatatgcgtcactggaaaagaaactgcgtctacgtgaagaagctgtcgataaagagaaactcgctcagaaggctggtggcggggattctgtaaagggtaagaaaggcgccaagaagaaaggcgatgacaaacccgaagaagacgatactgacattgataccgacactgatacagatggaggcgatgatgatacagatgactcttccgatgacagtggagacgactccgatggagacgctaaagctaagaaaggtggaaagaaatctaacaagtctggagatgcggacgacgaagacgcagaagaccctgacgcagacgaacccgaaagtgatgacggggatgcagatgctgaaagcattgatgacgaggacctcgaatagcgatcccgtcgatgtgccgaagacgcatgatgcgatgatcgaagttctgatcgctattcgctacatgtgcaccaagcggatgatctatcctgtagttgctgctaccatagaacagcgtaacgactttctggtgatgaacaagctgactttccagatgaagccgagcatgttctacagcgctattcaggatagcaactgcaaagtgaatgtgtgttggcttatgcgagccttcacacgcactgcactgcattttggtctgatgccaatcatcgcggacagaagcggtgacttccagcctctggtgagtcgcttcttcactcaggacgatcctgattttgcgtatcgacgtttctatgacgtgcgtaagctgccgtcagtaacagacattcgtaagccccgcctgtatacgcttaacggagttaactatggcgtacaagtcacaagccaagaaaccgaagaagtcaaaagctgcgaaagaagcagatactcggaataaggcacacaagcaagcgaagcgcggtaagctcgctcaggcagtgaagactctcagtgctgcatctgccaaatcgcgccgcatgactaaaggtgagaaacgtgcaattcagttgcagccgttcaaacctcagattgtgcctcagcctccgaaaactcctctgatggaaaaaggtctgtcgcttactgcgcttatgcgctcgacacctcgcctgatgaaagagaacgcgatggagtgttacgttaacactgtgaaacgcggtaagactaacaaaggtctgccgatgatcatggctaacgttcgacacaaagatccactgcgccctaataaaacagtgcgcattcacaagccgatgattatcggtctggatgacccgtacaagcctatctcaaaacaaaagcgtgtgctggtcagttgtccttgtgagaactttgttttcatgtgggagtatgcgaacgccgaacacggctgtgcgcgaatcatttacggtaatggcgaaccgccggacttcactaaccccggtcatgcgcccggtctgtgcaaacatctgatggctttggccgatcaagtcaaacgcaatggagattagttttgaatatcttcacatctgatacgcactacggagccgaacgcactcttcaatttagtcgccgcccatttggcagtgttcttgagatggataaaaccatgctcgaccgctgcaatgagatagctactgaaaaagatacactgtaccacgtaggtgactttggttcctatgagatggtgcaacatatctgtgcgcctgtcattttgatttgcggtaactacgagatcaatgacatgcacaaacagtttgcttcggacttcgatgctttccgtgcgcacctgatgcgtttgggttttgttgacgttgttcgagacagtctggaagtggatggaatgtatctcaaccactacccaactaagcgccgcgttgaccagttcagcctgttcggtcatattcacggattacagatggtcaaacgcaatgcgttaaacgttggcgttgactgtcatcattacgcgcctgttgatgcagagcgcctacagttcttccgtaatgcaatcgaaaatcattacgacgaagacgtgtttggttcataaggagattgcatgttctttaaaaatcctgccatgggcgttgtgcccaatcagccgatcattcactctattacggagatgcaccgtcgtgttgcagaactgaacggtgagctgattgctgctggctgtactgtggtcgagaactgcggtgagatgttgattgaagtacctgctggagcatccgccactgttgacggaattatgcagcgtcacatcgacatgttcaaaggcccgattatcagccgccctgcgcgtttgcaaatcggaggtgaagatgcagaagcgtaagttcgatccgaacgaaccttactcagtatctctgtcgtttggtccgcatatcgttcacggccatgcgcaagacagcgcgtttagtcaggtgatgcagaacatgttgctgcgcgagatcaacaaatcatgcgaagcgatgttcaagactctggctgatgttcctgtcgctgctgctcctacgtttgattgtgccgaagtagaggcaagcaacattcttgcggctgttcaacgttggcacgaaatgattgccaatgagccactcgtgaaagagttcgaaccgtgctttgtgccagactggatgcgtcctggtcttcgtgctaaaggcatgactgatgaacagattgataagatcgttatcactggcatcgagccttcgtttgaagatcgcccaggcatcgtattcaaaacggtgagtgcctaatggcctgcgctggttgtggccgtcgtagctctcgcattagctatcacggcgcctctgctcctcaagttgaaatcgaagaggacgatacgttaagcgctgcgcgtttaactccaatgggttgggtacgcacctgcgttaaatgcgggaaagtatctgagccttcaccctttgcagaaaacatcaataagccatgtgactgcactttagacgagtgatcatgatgaacaatctcgttggaacagcgtgtgccttagactcctgccgcttctatgcagagaatatggtgcacatacaattcggcagttctctttgtcctgtgtcgcctcaaccgccatacaatcaacctgtcaataatcgcaatctgcattcgtggattgaaagtattgaactggcgtttgacaatgcaatcagtcgtaccgatctgcaattcccgtacgcaggcattctctatcgtttccgttctatctacgggaactatgtggcccaataccgcgatgacatttcggctggtcgtcagtatcgtgcgaaagtaggaactccgttggatgcggtgccggagcggattgagggcgaacatgcgaaagagtttgcttctcgcttcttcaactacacggcaggccaagtgaccgcgttcttatacatggtctgtctcgatcagtatgctcgtgaacaaacagactgctatctgcctgacccaccacgagcattcgatttgcctcagaacatcttcaacgaaagccctaccgctttcacgaagacacacgacgttctggttaatcatctgatggaagcgatgttgcagacgcatagcgatacgctggacattcatgtgtcgttgcgtgattacggtctgtctgttatcttcccgctggtggctgagtgtcgcaatgtgatttacgccacctggccaatccctaatgccaaaggacaaaaagcaaatgtctgatgttattctgtttgacaatcagaaagactgggaagacttcggtagcgcggtctacgaagaatttcgtctgaacgtgatgacaggcagtagcagcgccagtcagattcctacagtcgcaccgttcgaagacgtgaaacaccaactcagttattcgaacattctgcctgagggtgagcaatcgcctatcgttgtgctggacatcctgatcatggaagttgaactggccgaaggtgaatcgcgcaactataatgcagacagtctggacgaagctgtgcgcaaagttgtatcactgtatcaggctcgcgctcgtgatctagactgccacctgactggcaacttcattactgccgatcataaagttaatggtgcgctgttgcgtatctaccgtaatcaggacttcgtgtgcaaaggccatcctgaacttctgcacggacgtcctctgggcatgttccattgtgacaagtgcggtgagatgcagatggccggagcattccacttacccaaagaggaaactcaaaatggttaaaggcggactgtggcgcgtcttccctgattacgactcagaggagatgctgctcaaactcggtgctgctatcggtatcgaccgtgacagtgatgacgtgcctgatgaattgcacgttactctggcttacgatgaatcgaaccctgacgttgaagcagagcaaaacgatgcgggccagttctttggcaccgttgcctctgctgaattgttcggcgaaggtcaagataagattctggtgctcgtactcgaatcgcctgacctgcaacaggaacacgctcgtattcatgcgtgtggtgctgccaagtttgcgcacactccataccgcccgcatgtgacgttactcaaacatgcaaaagacagccaagctgaatatctcaaccagatcattcagcatccgggccgtcctccaatcactctgcgcttcatcgaagaagatcgcaaggtgctggagaagcgtagctaaaacctagcggtggccttgggctgccgcttttgtcattctggagaaatttctatggaaatctatgtaagcctttcccatgagattcgcgttggtcgtcaagactctgatcaagctgttgcgcctgaaaccactgatggccagagacgtgctgttgagcaacaagagaaagagcgtattgttgaagaatacggcatcgacactccccaagaggaaattgacgaaaaagagaaggaacgcattgagcgcgaagaggaaaagcgcgacgaaaacaagaccaaagcaccggaagatttgggtcagcgtaagccggaatctgaactcactggttctgagattcaagaccagcatgataacctgacaaagatctaggaatctgtaaataagagtcaaagcaactaacaggtgtatttgaccatgaacaataagtcgaatctcacaggcggtcagatagaaagcgtcatggacacaatgcttcatgactgcctgcgtgagattgttgagaacacggacatattcgatgtgcaactgacctatctgttgaacatgattacgtcgaataaaaagcgaaagccgtacaacgctgagacgcgggaccgtgctatcagccttctgattaaggcgctgtctgtgcctcgcgatcagaaaatgatttatatccaggagcttaaaatggagcgtaacttcatttacgtcttcctggaaaatgtaattaagcgatactacacaacgtatgtagatctctatcggggtttcatttcgacgcaagatgctgttaagcgcgaagcgtattcgaaacgcctgaatgcctacgtgaagatgtttggggcagagtctcgctccaaactctttatcgcgttgtgtcgtttgaacgatcttctgccgcagttcatggaatacttccactcggtagttgctgacttctatagactatgcagcaagcaaacaaaattttatgttgatacgaaccgcggcaagctgtatgacagcaaagacgtgcgccagaacttcctgcgtaacgttatcgtggctatcaacaagtatgactcctctcgcggtgcgattgtgagttatacgaagtggtggatcttgaacgcccaaacctgtagtagcagcgagcatgaatacggcatcgcttatactattccccagactcaacgtaagaaactggcgacaggtgaagataccacttctctgaatttctcggtaagtctcgatactcctgcgaacgaatctgatgaaggtgcggacgcgtccctacatcaaaaagtgagtgaccatcatcacttagaagatcacgtagatagtgaaagacgtactgaaaaactgaggctgcttattaagcgcgtagacccactcggcgttgcacgattgacgatggatgtgggtgaggagttcgataagttcgaacttgatatgatgcgcaaacatatgcaggctcaagggctagcctaaaactgtaaacagtgatcacataagcacaactcaatattgaggaacaacaatggcacgtggatttggtgacattcaagataacagcaaacgcgatagtttgcgtgaatcagaaatctttgaaatcttcccgctggcgaagaaagcaaacggcaactgggtttcaattcgtctgttagatctcgacctgcttccgattaagaagcactggatcaagatcatgggcgggaaagacaaagacaaagagatcaaaatcccgcgcatgtgcgttagcttcgacccggacaatcagaacaaacctctgaacggtatgaagtgtccgtactgcggcatcgctcacggcaacgacgaatctggtgcaccggcgcagtacgattataagtggtacgcacaggcaatcattcgtgacgagcaggctgctgcgccgcgtaaaatgccgaagatgaccaagaaagaagagaagtccggcaagaaagaaatgggcagcgagtcttggactcctgtgcagtgtattcctctgtctaactctctggctggtaaaatccgcgagctgggtgaacgtaatattcacacggtcaaagacaaaaagtctggcaagaagtctaagcaggcgtttcaggttaaccatccgaagtatggctgcgatattgaaatcaaatacaacgccaaaaaatctccggcagagcgttacaccatcgaacgtggcgatcatactccactgacgaaagaagaacaggcgtacctgacctgggacttcgacaactggaacgaaatctacgacatgctgggacgtctgaacgaagaagctgctatggctgacttcaagaagatggacgttatcggcgttaacaccaacgattctgacgatggtgatgacgatgacgatgacgacgatgatatggcgctgggccgcaaaaagaaaggcggcaaagcggacaagaaaaaacgtcgcagcgatgatgacgatgacgacgaagatgacgacgatgatgaagatgatcgtccttccaagaagtctaaaaaggcgaccaagtctcgtaagatgttagacgatgacgaggacgatgatgacgacgaagacgatgaagatgatcgtccgtcgaagaaaaagaaatcttcgaaagacaaaaagtcctcgaaggttaagtctaagaagtctaagaagtcagatgatgacgacgaagacgacgaagacgaaaagcctaagaagaagaaaaagtcttctgacaaggtgaagtcttccgttaagaagaaaaagaaatcttctgacgacgatgacgacgacgcgccgaagaaaaagaagaaaaagaaaaagtaatgtgaaacagggtggctaacgccgccctttcttttctctaatctggaccacccaacaatggcgaaaacgaacaacaaggctgagaagaaagctgagaagaaagctaaagtcaaagccggtaagacaaaaggcaaagcagtcgcctctgatgatattggcggcgtagaagtagcaggctttgaccttggtagtctgatggacgatgtgcttgacggcatcgaaaagaaaacgaaagtaagctctcaggacgcagcgcgacacgcgcctcgtatctctactggtgtgctggcgcttgatatgtaccttgacggcggcatcgtacctggcggctggtatactttcagcggcggtgagcagtcctgtaagtcaacaatgaccatgagtatcatggcgagcctgattcgtctgaaatactctggcattagcgtagtgttcgactacgaaggttctactgatgctgactacgttgctggccagctcaaaacgtttggcgttactgttgacgcgaagaccatctttggtgtgcgtgacggcgacgacggcaactggattatcaaaccgcgtattcgctactacgcgccggacaacggtgaacgcttcttcgattatatgtcgatgctgcgtcgtcgtctgcctgataagatcgtcgataaagacggtagctcgtactacatctttgagaacaacaaagagaacgccaagaaggttgctggcaagtacgataagaagtggttcagccgtaacaaccagttcaaagttcctgcgtctgacggtcacatgcaggctatggttatcgttgactcctatcctgcgatgatgccggatcaggtcgatgatgacgatggctcaaaagcaatggcgttgcaagcgcgtatgttctctgacggcatcaaacgtttccgtggcggtatgcgtcgtaagatgatgactatcgttggcgttaaccagttgcgtcagaaacctgctgtgatgttcggtagccctgagtatgagcctggtggtgacgcgttgaagttctattgcttcgaccgtgacactctgattcgtaccgaccacggcgtgatgactgcacctgatattgcgcaactgctgaaagatggcgttaaagtttgcgttgaatcgttcgatggttatcagcaaatcaatggcgcatggaaagttgaagacgccccgttcccaatcgaactgtctgctggcggccatagttacatcggtagtgcagagcaccgtcagtttgttctggtacctggcgtaactgctgatggcacgaatgtgttctatcctgagtggcgtactctgaacgagatggctactggtgggcacgaaggcgtatacgctggtctgcgtgtcccgcctgtcaaagaactgaaacagaacgtacctgatgcgttcgatgatgctagccagctggtcagtagcctgcttgctaactgcgatccggtaagcgttcaactgcctctggccacgcacggtgatactacctatgcagcgaacgtgctgaccattgacgtagttggcgagagcactgattcttccgacttctcgttctgggctaagaagctgctggacattggtgtattcgcttacgctgacgaacgcggtattcacatgcctggcctgaacaagcatgagctggaagaagctgttgtgcaggatgctgacggtgcgttccgtggtctgtcttatgccgccacctgtcgtcaacgtcaaacgcagatgctgatcgctatcgctgatcgcttcccggaactgactcgctatgtgctggactatcagttgcaggtaggcgaagctaaaatctatctggcgccggagaatgactttgccgaagcgctcgacctgattctgcatcgtgagattgacgggtatgatgacctgtacgatctgctgatgcagcaactggcttacgttgaagactggtacaacttcgatagctctatcttgcctgtgccgttctcgctgaaagtgctgaacaaagaagttgagttctgggacgttaacgttgccgagacttctgtggttatcaccaacggcttcgtatcgcataacagtgatgtgcgcgttcgtctggcttctcgtgcagtacctgatgcaggctggacaaaactcaaagacgcacctggtgttgtcggtgagaagtctgtcactattgagggcggtactgaccgctatcgtttcattgctgctaagaccatcaagaacaagatgggtggcatcccgaaccagcagacttggttgcgtctgtgggaagctgacggtaatggtgaagcacgtggctttgatccggtgttcgatacgtggcactatctgaaagttctcggcctgatcaatggcacacgtaagagctttaagatcaaagcgccttgccctctggcttccgaagtcaagatggactgggatgacttccgtactcttatcaacggcagcaagacacaagttgtcgatgtgtgtaagaagctgaaagtcaaacctgctggcctgcgtctgtggtgcttcaagttcgtgcagtctgcgaaaggcaaagaaatgttgaaagcgtctatcagtaagtctgcgaagacttctggtgatgaagacgacgagtaataaacgcgggagggcttcggctctccctttattcgtgtaaggagaaccaatgcgtactcaaatctttaccgctgatattgttaatctgcaaacaaccgcaactaacgaagaaacaggcgaagagattgtcacacaaacaatcgtgcctaacgtcgaaggtgaactgacaatcagtgttggtgaactgtctcgtctgtctgaaagtctgagcgagcctaccgactctgactgccgcctgattgttatcgtgtctcctgacgcgacgcctgtgttctacgacgaagcgctgtccagctacttcgatccaatcgagcgtgtcgctgatattcaggcaggcaacatcggcaccatcaacggtctgcaagtcatccgcggcctgcagggcgatcacccttacgttgcagttgtcgaagtacgtgacgctgataccgtagagatcgttcgctacaacgcgtctgtagtaaaactgtaaatactgatcaacaaccgaacacaattgctgtgtgtagtctcgcccgacttgggcaggggagagccggatggcctccccatttttttttgtctgagaggttttttctatgtcaacattcatcgaagtacatgaggcttacctgcaggagtctgcctctcgtggcgcagcgcgatctaaaataaccgaccagtttactgcttatcttaaaaagagaaacggtaaactcccgccactaggaatccctatggacgagtttgtccgttggtctaacatgattccgacagagatcaaccctgacatatctcgtcagctaatgtttatttcgtcagcgacctacactcattacgtttggtcttttacgaaagcatcctttgtgattgagaaagaattgtggccacatctgattgagggtgatgctcctaaagtgcttcccacttccacactgcgccagctgcctcactggtcgcagtggattaattgtgtgttcacgcttgactacaaacacgcagcgaccggtaacaaatatacaattgacctagaaggattctgggcaacatacaccaactatctggaagcaacacatctcaatctatcctgcttgggtgtatacaatgatggtacgggagatcagatcatgtctctctacatcatattcgacattactaaagacatggagttgtctgatggattcgattggttcattcatctggtaggcgctagaggcgcaactgctgtggatattaattctgataacggcgctgaggttaatgaagctatcatggcgctcatgaagcctgtcgttaacgtgctgctatttgttgcatcgcaggtagataacatctataaaggaggaatcaaatcactcaaacctagacgtagcggtaacagctacaaaatcattcctgttcgtgatgttcgtgagtggaatgttggcactgagttgcttaatgaaattcgtacttacgaaagcgaagtgagatctcacgaatcaaatggtcgtcgtgctcacatacgtcgagcgcaccaccataactattggtacggccctctcaagggcgagcgtgagctaaaatcgcgctgggtaccgccatgcgttgttcgcggcactgtcgtagaataactctcaaacaactccacgtatgggcgttatgcccggaggtcaatatgtctcgtgtacaaactctatggattcctgatatggaatcgtatgaaccttacatccgctctctgtgtcatatggcgcgagcgctggaaaacaatggtctgaactacggcaagatgaagcgtgtcgtgttcatcggtctgtcaaagcgtagtgttgaatcctacgttaaacagcttctcaattcaaacacgttgccgaatactctcgtttgcttcggcatcgacgagccacctgttagtcaccgtgagttctcctacatcggttcgcatgttgtgttgatgcacgacctgacatatgcaggagacaacgcgatgggccgcgtgtcgcagcgtgttctcgaaatcatcctgagtctgaaacaaaagcctgaggatcgtgaacttaaaaatggtgcgctgtctcttgtctaccaaaacccgatgctgtggtcttacatcagggacaatggtgcgagtatgtacatgaacgccgcccacattcaatacgcagaaggtcttgtgtcgtctatcggtgttgatcaactcatgtcctgcaaagacaacgaagactatcacaaactccatgcgcctgtgattacgatcggccttgagttcttctacgttaagcctgatgaactgctgtccaaactctgcaacctgatgtggtctctcggatcaaccacctgcgagtttaaggacaactataaaatcgtactgcatgacgacttccgcctcgctttcttcgaagaattccttctcagagagtttaaggggttttaagattattctgagtttcgtcattaatttctccaagttagcaagaagtgctgactaaatagttatttggagaaataacatgtgcgaacgtagcctcgtacggttgaagtacatcgcacggtcatcgaactggtgcaataataaagtaaacgcttgtagtgagcggaaggcgacgaacgtacaatgcgaagattttttagcagtaacaaaagattgtcgcagtgtgcaggactcgtccaatgttgtttccttcttcaaagatcaagagctggtaggtcaagctatttgggaagagaaagagggagaccacatacttcaattccgactactactcgcataactttcctaatagggctatcagagcaatctggtggcccttcttcatttctaggagctgtcatgccgtaccacctccaactgcaagagaaacactttagagctattcaagatcacgcggaccaaatcatcggtctgtccgctttagtatcgaagttagctgaggacgatattgtcgttgtcaatgtgtccgtgtcgcgtccacaagacgcgggtgttcccattaccgttgttcgtgacggctgtgagcgatacttggaggtgcagagagcgccttggcccatctcacctgattcaccatctatagaaatagcaatcgttcaatactgacgctcaggctgccctcgttggcggccttttctatttctatgctaatttcatcttgcattcactcgcactggagagacactatggaaatctacgtttcactatcgaagcaggaagaaccaccgatagtaacagagatcgaccaaaaggcgcctcgcattaacgacaacagcaaagtgggccaagtattcgacgttcacgttctacagcaaatgagttacctcgacatgaagaacattcgtggtgacgcaggagcgaagtacgccaaagctattgctgattggctcaacagtcaaaggtcgatcgacaataagtttcgcgtatcaaacagaagtaaaatctcgattgctgtaaagaacacacaacagatggccgcgcgttatcgcaacatctacctgttgagtcctgagagcaataaagatcgctgctggttgctggtgggtgaaggccctcacgacaacaagcagactgtggagattggtcggagtcttcaaatggatgtgctgtatgcttccgttcgtactatgcttgcatcacacttaccgaccgacgagtggccaggcgataacacatacgaacatgttcaattggagttggacaaacggggcaaacatggtggtcgcgtggctaagcgtcattacacgtttgcaaaagaaaatgaaaatacactgatcacgatgatgcaggacgggttgtccattgcagaaatcaccgattgggttctgaaacagtaagaggaatctatgtccctgattaaactcgaaggcatcgcatcaacgtctgctccgaccaaggcgcagaaagatgctgccgtttatttgtttggctccaaaggtcattcaatcgttgcagtgctcgataaattcagtcgcgccaaagaactgcgcacagctcaccttgacggtctgctcaagctgatgaaagaaggcgaagatgacgagatcatcaagttcgctgcgtcggccccgggcaagaaaacaatcgctaacgccaaagcatttgctgtggcgaagactctgacctctgcaatcaaagcgctgaaactaatccgcgttcctgttaagtgggttgaggggcattctgatgcggctgctgctcgtgttcaggagaccaaagagattcgcgcacgtaagactgcgggcaataaacctgagaagccaattaagctcgataacccaggcgcgccggagtctgttgaagttgaacagaccaaaccgaacgccaaagtaagcaagatctggttggcaaaaaacttctctgcgtctaatagcgctacgtggtctgccctgcagaaagcattcaacgacgaatgcaaagaccttggtttctctgctaagttcattaagagcgagggtggtctgcgcattactgttccgggcgcgggctatcagcaattgcgtaacatgcacatcggtctggatgactcaggcaaaagacctggctggcatttatatgcagtctcaccgaccgacaaacacggcgcagatattgatgggcgctccatcggtccgcgtctgaccgttgcttccgtgattgctgctattcgtgactttatcgccaatggtgataagatcaagcagtctctgaatgcacgtatcgcaggcgctcaggtgtttgacaaagatctcacaccaagcagtggtatctttgacgagtatgaagctaacgaacgcaaagcacgacgtgatccagaagcgccggtgactcttgcgaagctgaataaaaacagcatcggtaaggcaacaaacggtatgcttggcggccttgctactgagataaacaaagtagtgaaagacacacctatctacgccacgaactttatgggcaaagagggtgcgtatggtctgaacggctatatcattgatatgcacatctctaaacgagataagccaggcaacctcgcaggcgttattttgatcccgccgcaggccggaactgctatcaaaggtgatacgtggcgcgctcgtggtatcaagattggccgcgaagaactgggtgctgaatacagcatcggtgccaagctgactgctgctggcgtaaacaaagcctacgctaagatcatcaaagaacctatgtttgcaaaggctgctgtgaaagaagcgtatactccgtctggtaaaactgacgtaacgctggtggacgaactggcagaagtgactgcacgtaagatcgctgcgaagcctcttcaagcgcgtgaagaatatttcaatgcgctgcgcaacactctgcactccaacctgcgtaactctgtggtcaacactacctctgacggtgtgacagtagctcagggcaacaagctctatacaatccgtctggccgacaatacgtggaccattcagactggcgctaccggtaagccgaagaaggtcggcgcaacgttcgacattgttgatctgcttggcatgatcgacaagagcattctgcgtcctaaagcgtaatcaaaagggtggcttcggctgccctttttcatttatttctgtgccattcgtaaataacctatctgcttccctagccagttctcctcgacacacaatctcttatcctgtcctgtatttcaaaacatctctatctccactggtactactcaaaaatgcaccagcgcctacagtcatcctgttctctaattcaaccttacagactcggtcgtctgtgttgtatttctcaagaggaaaatgtgatgattgaagtaaactgctttgctgatctgcgtacaaccaaacctgagaaagctggcgctctggctttactcgctcgctactacgacaaagacagtaagttccgtggtggtggttggttcatcggttaccctcagaaaaacgtaccagcagatgatggcggtatcattgctgtgggtaaagacgacaacggcaatccattcttctggcagcgtgtcgtcaatgaccctgaagagatcaacattcttcacttcggtggtaagtgtgacggcaagacagatgacagtgatgcgtatcgccgcaacttcatgtgggtgttcaacatgaaagacggtagtgacacgctgggtgttaagctgccgtcaggtacaactgtcctcaatccgatggacttcactgacttgggtgagattccggtattcgccatgtacggcgatactcgctgtcttaaaggctggcgccctcgtgtcaaggtcattagtaatcagggcgacaagcaggtaatcaaagtcaaggcgcgccgcaccgtaattcaaggcatcaactggaacggtcagtgctatccaaaagttgacggcaagaaggttgacgtggcgaccattgctggtgcagtaatgcctgagcaacgtagcaacaaccaaatcttctttgagaacatctgtgcgatgggtcaatacgtaggtgttcactgtttccgcgcagagaacactggcggctctgcactcaaatttcaggacactatcgacacgtcaatcactgagatctatggctcgaaaatcttcggtgctgtgattgaagccaagtggtctaacacgaaagaagcaggctggaaccactctactgctgtacgccttgagaacggtaacttccagtacggctacggtcctgctgtactcgatatgccacgcatgactcaagcgttcatgaagaacatttggatcgagcatacacgcttccccggtaatctgaatgacggtcagtgggtattcgaaggcaactctatcgaaagctctgacaaccctctgaatctcgccaacactcgttgcgttatcaatggcttctacttccagggcaaaggcaccatgactctggaacgcgctaagagtcctgataactggctgtcaggctacgagcgcggtaacatccgaactgagacatacggcatcatcatgaccgatgcgtgtttccgtccgggttactacactggctataaagtaacgaacacaactgatcaggacaagtggttctatatcggtgacttctcgttccctaaagtcggccagatttggcagatcgagttcctgtctaatcacaacgctcaggtacctaacgccaagctgcaacaaccagcagacatggaaggtatgggccgtcgtgttattactatgcaacgttgcacggtacctaatgcgaaggtttatgccgatatgcactgcatgggcaaagatgcaattgtcgatgttgtgtaccagcgcctgtgggatactcacggtaaggtgtttatcaaagtcgcagccaaagctggcgatgtgatcttcaacctgactactacaggcccgactcgtttcgaagaaggcatttgtactctttactctgatggtcctgttgagtgcgttggtgaactactgacagaaatgaccaccagcgttgaaaagaacctgaaagactacgctcgacctcaatctcgtttcagtctgcataacggactggcgggcattggcgcaaacgagcaaggcgtcatcacaatgcagaccaaagaaggctctgctcctaaagaccctaccaagcctgcaggctatacgacaatcaacatcaacggtgttgatcgactcgttccctactattgatcacacgaggggcgcaatgcccctcttttcattctgtgacttaactcaaacgcaatgctccagagatgcaactatgcaaataataggctgaaataggtctatatacgcacatgcgcctgtgatacactatatgcagacgctacacgtcgtagcgcacacaactcatgctaaggggcatacaatgaaagcagcaaactttgataaagcattcaacgcgaaagacgaagcaaccttgaacgcatacgctgatcgtattcagcaagcgcttaacgctctgggtcgttatgacctgaaaatcaaaatcatcttcggtactgacccgtttagcgagttccctgattttgtgaatgacccgaacggttttcgtgttgttcagaacaacgaagaagttttcgacatatacacgccgaccgagaaacatcttgaaggtgacgcgtcacaaactttcgtctacgcggcaatcggcggcgtagaggcctccaagtgggggaaagaggtttccgataatgatgtagaagaaattgccgttgacctgaacgaagaaatcgaacgtgcaggccgtgtgttttatgaagaagaccgcgcaatgctgcaagagattgccgacaagctcaattctcaaatgcagcgcaccgacgctcgcgtgatcgttacaaacggtgccgaagacaatctcattcttatggttgtcggttatgctgacggcgaagtcagtgacgagtacggtttcttcttagacctgccgtacactgacgaagacgccgctgatacaaactacgtcctgcactatgcaggttacccagatatgaacgatcacacgttcacttctgaatcgctcgatgaaatctcaaaagagatcgaaacactcgacctgctgtaatcgctaacactgactgcggggttacggccccgcttacttacttctatatagagacacgaccatgactatgcacatcactactttctttgttaaacgctcttacgcttctctggctgctggttcattcactattgcttcgaagcaagtgcaagagctggtggaatctgaggtcttcatcgtgtacgcaaacacggggttgggtaacgcattcgctgtacgcaacatcaccctgacgcctgttgatgaagcaaacgtgcgtgttgagttcgacccgctgaccgacgttcacgcaatgccgtctagtgttctgcccaaagagagtctgactgaaagcacacagcaatatctcatggcgccggatgacgtggccgctgcccctcgcttctgcgtatctaaccacgcatcgggcaacgagcctaacatgttgtgtctgaaccatgatgtgcgtgagcgcctgattcaatataagggcggcatgatcagtctcactgagctggtgctggtgcttcacgaccaagatatttcagtgaccgacattcatcaacaccgtcgcaacaaagagaagtacgtggcgcagatcacagagcgcacctcacacgttatcgaactgtcgaaagacaacggcgttaagcagcacgatagcgacttcccgttgcttgctcgcctgaacgtgtatctctaatcaacatagctttggacaaaagcgccattgtgctctaacgttcaatggcgtactatgtaatctctagcgcaatgacgcgctcaatcaagaaagaggcaatatcatgtcagagaaacaaatcacactcgatcttatcgcagacgtagcatcgccaactgaaatcatctttgaagatggcgagtcttctaacgactggctcaagccgtatgacctgcgcctggctgttacgcagactgtcggcccgaacggctatcccgaagttgcaatcatcggccatgaagatgatctgcgtcgcttcttggctgagaagctgcctgacactgacggcgaactcgaagacgtgcgttaatcttatggggcctcgtgccccatttctactttctgcctgagatacgactatgaaaaaccaatatctgatacttcgcatgagccctgctgatttatacgacaatcaatttctgatgcgcggcttcaatcgcaaacgtatcgaaaacgtcattggcgttatcgttgttgttgatcactccgacagcatgtatcacctgtcgcgtgttcaagttgacctgttgcagtctgacacacagcagaactgggcaagactgagttggtctagcatagatcgtgagagcattgacttaggcatgcgcagcctgccgcctgagctggctattgccattcgcgctatgcgaaacaatcgcatgtatcacaccgtcgatacaaaaatccctgtggcgtttcgtgatcgtcacactaacttcgcctacacgccgagcgccgtacgcaagattgctaacagagaaacgaagtcactcgacgacttcactgtagaagaaatcgtagcgcacctgaaacagcgtcttggcgttgagattgaaatcaaactgtaaacacttaaggctcacattgtgtgggctgtttctatttggagaatgctatgatttatgaacgcgaagaacttgaggcgatgcctctcgatgtgctgtataacctcgctggcgctaaaggtctgttagacgacctgacagacgatgacgatgcgcctgatcgtgaagcgctgactgatatgattctcgaatctcagtcgctcgaacagcaggccgatgaagacgacgcagccaagcgtcaggcagaagatgatcgcgacccgcgcatcaatcgtcgtgatggtcaagacggctcggatgattactgctaatgtcacctactgaactgaacgaatacctgcatctggtgctgacgcctgttgctatggcgtggcgtgaacagtttcccaaaaagaaacaagtgatcgcttcggtgaaaacgccgtactcatgtcgcatcaagttcgtcgaagaccaagaggttgaaaaacagtggcaggcattctgccgcactcacggcctcaagaacgaagaaacactcgaaatctaaatcaaagggctgccattgctggtggccctttttcatttctgtaaataactcgtacaacaatcaacgcgagtcactacaatgcgccgcttcattctcgttctcaatgtcactcaggcagagttagacgctcgccacttcatgcaaatcaaactcaacatcataagcaccctgcgccgagccgcctgtgttctgcttgttgtgcgtgagacgaaacaggtcatgtgtgtttctgaactgacctttcaaagtgcgtcaggcaatctcaagcgtgttgacttcgacgcacctcgcgatgttactgcgcacgtaatcaaatacaacgaactgatgatggctatggcaaacaacgccagagaccttagcgttcgtcactttggccgacaggtcgagctagacgcagccgacaccaaacgcctgttcactcaactggagattattgcatgagtcagtcattaggcgcctcgcttggcgctcgctttgctgttagctcacaagagaatatcgaacgccgtaagaagcgtgacccgaaaaataaaacgctgacctgcgctggcacaacggcacaatacaacgcaatcggagtgctggcaaacaaacttgatgtaagccgctcgcgtgttattgaaatggccctcgaagaactgttggctaaacacaatatcaaagtcggcggtgacaatgattgacacgcatatctactgccgtctgtatggtgtgcagcatcgtctaaagattaccgccttcaactttatgaagcagccgaacatgatcactgtcgattcgtctgatgttctcaagatgatgccgctgattaatgttggtgcagcctatgatacatacacgccgtacaatgtactcaaggcaggacaggctgacttcaagattcgtctgatcgaaagaactgatgcgcatgtctggcgctatgtgttcgaagactatcgcggtcagatgtttgaaacgttcttgattcggagacactatgaaacgcctagggattgtaacggtgttgtcattaaaggacaaacaacccaaatcatgtgatctcgatattgtgcccgtgtcgaaagacgaagaatggggctcgctgagtccctttcatttagggccgtgtcgaacgcctgacggtacgatgtttctcaacatggagaatctctggcagtacagcaaagtgtacgacgaccatgttatcaattcgaatgacctgttccttggtgagatctcaagtgactggtggcagtggcatttaaagggaagtaaatcacaacaggcgcatcgctatcctatgggaaaaggccagaaggctttattctccaaatggggcgacttgcgcctttcgtacatttcggcgcgtaaacaaatctatgtgcctgagtatgcgaagctggtggtgcagcagccgaagttcaggcgcttgttgaaagagtacaagaaaggcgcgcacatagttttacgcgactatgacacctacgatattcttcgtgcctatcctgatgcgcgtagcccgtgggtatcggcgatcgaaaacaacaatgcaaagttcggccatgcgtttgttatcgcactgtgcctgttattccacgaaagaccactttggtataatcaatggataatatgaaatacgaagcctgcatcgatctgttcacgcgagccggaaacatgaatctcccgattctgcctaagtgtgaactacaggcaactctattcgatcagtatacgaaaaagcgaataccagttcgcttcaacgccacaaacgtaatcaagatcaatggcgctacctgcggtagtctgcaaatcttcgactgtgttaatctgatcatctggtcatcgtttgatgttaatcgctttacgctgtatgtcgagcgagtacacaaggcagacgtgtcagagagcgcccagcagtctgtcgaactctgcaaataactggtcaaaatagccgttcttttcagtaccagtttatgttatactgagagcgagcgctattgctcataaaactcaagctgaggagcttaacatgtcatcttctactactctgactttcatcttccctgaaatgaccactctggaagtttctatcggcaacggcgttgtgccacaatatctgggtctcgcggaaaaccgagacataacattcagcgacattaaggcgttgcgcctgatgcaagactcaaacgttatcggagtaatgagtcgcttcgaccagtcgatgctgaatatgctgatcgctcgccacgaaacgaacgagcatatccgctgccgtgacgccattgagaatggcagcgagtatttcccatctacttgtctctacctgaaagtagcgcatcaccgctaagatttgtgaagggcatttgcgagtgccctttgaaaatcaaacccatgttctgaggagaacaaaatgacttctactgaaatgccccgtgacgcccgtgcttttgacgatctcgacaacaacggcttcctgcgtatcactaactgcctgtcgatcattctgtctcgtggtgatttagaactcgtcactgatattgcggaccgcaccgtcactgttaagtatcgcactggcgctgtgaacaaactcggacacggacacgttgttctgcgtttcccatctgaggtcattcagtctgatgttcttgaagacttcgaagtgaccgtcgataaagacattgtgattcttatcgaacgccagtacagttcggctgcaacgttccagcgcattgcaggcgtgattgaaggtctgatgtacaaactgtgattgttgctcgcaggttcttacgagagcctgctgtcaacataacccataagctgaggagcttaacatgaaacagtacccgcaacgtggccgtgtgtacacactgaaagaaattgagaacgaccttgaactgcgtgacactccgttcttgcgcttcgtaccgcagaaagtacgttacgttggaatgcctgctggtattcaggtcattcagcaggcgcacattgctgacctgtctgagcttgagggttgggcagataccaaatggtcttatgtgcgtgagaccgaagaatggattccgctgttccgtgctgtagacgatgctgcaatcgaagcgctctgtgttatcgagcctgacgtgtcgcagttccgttctgacaacacgttgttcatctacccgaaaggcactgagtgcaaacagtatgatgggtacgatgaagcagttcacggcgatctgcttgaacgcgacgaataacaaacagggatgctcacgctggtgggtgtcccattttacgttcagggaggtttcctatggaaatgtttgaccgctcaaatgtgataagcgcaatcatgcgcaacctgaaagacgtgcgtaagataaaagacctgcgcacgttcgacgacaaggtttactttcagcttaacgacaaaggctactttgtttctggcaaacacccagagttgaaagttgtctgtcaaggtcagtacgactacgagatgatggcacaactcaactttgtgtatcgtcgtaagatgaagcccaacactgatacgccgatgcgtcttgctcgtatcgctgtgggtgtgacgcttgttcaggtagccaaagagatcgatgtagatgcaggcaacctgagccgtatcgaacggggcattcagatcccggcgatggaggtagcagagcgcatcgccaagtatttcaacaacacaataacagccattcaaatttgtcatccaacttataagggaaaaactaatgcttagtcaaatcactcatatcatccaagtgatgatgaccagcctgaaagatgttcgtgctgtcgaagaaattcgtatcatcggagacaaagctgtgcgtttccgtactaacggcaaaacgtttgacgtgcgtggccagtacccgctgttctgtgtgcatgagattgaaggctcctgcatgtgtggatcgaaagatgcctacgagatcgaacgtcaactcaacggcggacctattgaaagtcaggacgaagaagccttcgcgcacgactcacacgaagaagcggttaacgatctgctatgcaatcacgttgatagcatggaagaagatcgtgtacgcgcatacaatgaagaatgcggcggccctgacttggacccaatcaacggtcaacgcgtttggttgaaagcacacttcatccatatcagtgcggaaatcccaagcatgttggagaccgtgatgttcatggaaggtaaagagcgctacgagcaactgcgtcgcgcaatcaaagagatttactcacctaaaccaaaagtagcctaagaggaagtagcaatgagcgaaatagatattctgatccgagagtttgagcgggcgtatctcaagtcactggaatcaccttggggtaacgttgcgtatcacgttcacgacctgcaccctgagatgaagaacatccaactgtacttgcgctttcgcacccagtttcaatgtctctggaatcgacctgtgctagtgttgtcaacaatcaacgtgacaaatccgggacaaggcgagttctcgaagttactcgcacgtaccaaagagatgtgtcgtcagcgtgattggattctgcaagtcgaaaacgtcctgacgccgaagtttagaaagtttctacagcgtggtggattcaaaccattcggcattgataaagacgtgccaatcggtagcctctattggttccacgacgaaacaatcccgcagcaatgtgcgatgtacagggagagaggtgtatgacaatctggtggccaactattctaatctgcttaacgccgctggctgcctgctatgccactatcccatggttccgcgctgctgttgataggcgcctgcgatttaagtctatggactatgatgccttgactgaaatctttgatgatggcatgcctgagcgtatgcgcatcgaatgtctacaggcaaagtacaacgcgcaccaagcggaccattcttatgtggatatttatccgcacaaagagggtgtcgcaactattcgctttcatgttgaccctgagtttcctatagcacgtatgtttcatgatgtgctggtgggcaactacaatgctctgggaatcaaaacaaagaaggcgccagtgataagcatcaatcagtctgtgtatcgtgtgcttgattttgagtatgacgatcagtacctgttgatttacgtgaaacacaactaaggcattatcatggtcacccaacaacaactcaaagagttttctgcattgccttctcttgacaggaaagtgtttctgcgtagtaagcaagtagagatgttgggtgccctccctgaggtcgaagcgatagttcgtgagatgttgtatcgcgctatcgtggtagacgtagcccaagcggagatggcactcctagcagcacgtcagatgtgcaagaacaaggatgtcagacaagccatagacgaactacttcaattcgcggcgaagatacatgatgccgcaactgatacccttttccttggagatatagcatgaataccatttctggcgcaatgattgacgaagacgttctcgattggctcgacaacttcaacatgcacaagcagaagaatatctgcgaagcaattaaccaactggcgtatgctaaccgtaccgagctgtctattccaaacatggactcggacgaagatattgcagcgctgtctcactctgacctcttcaaaatcttaacgctggccagcccgaacgcgaagtacgatcttactctgtctaacgttcaactgttgggtctggcaatgggtgcaatgggtgtcattgaatactctatgcctgaacttaacagcccggttatgatcgctcgcaagttcgcagacatgcgccgcaagaacatcatcggctctactggtgaccgcgataagatcatcaaggcgcttaatgagtgggtgtgtggcctgcgtgatattgatttgtcgaacgctggtgcagacgaaacgcctgagcaagcgggcatgtatctgtgcgtagacgaacacgaacaagttcgttacggtcgcctgtacccgaacagtagtgaaggtttaacgttctgtgaatcgtatgcagacggtggatcgactatgtggtacagcggtaacactgagcataccaccgaagatgacctgccgataacgttgctgtctcattgggtactggtatcagagtggcatagcccgaacgttaaagccgcgcagaaagttattcctatggaagtgcgtgacacacatcgcatctttatgttcctgcgcggactcagcccgcatgtgaaagcagagctggtggcacacttcgacggcgtactcgactataaagacccaacgtccgttgacgctatcggtcgcctgactgaacacgactggcagatggctgcgacaagtattgcagatgacaacaaacttcctgaaggtgcctcggcgtggaaagaagtgacagcgtgggtctgcttcgtagcgtcgcttgaatctttgggtttcaatttccaaacacgtcagtttgacccgcagttcgactatcaggcaaacgacgatgacctggaggaagacgacgaagaatgaacagacgaatgatcgctttgcttgcgctggtgatcttctgcttggtgggagcagttgcttccgccgaagcagcaaaccactacaacattatgttgtgccttggcctgacacttatgtttctggccggcttctttatctgtgtagaatgtttccgtaagacttcatgggaacaacaaaacaaaaaggacaaaaagaatggctaaatcattgggagtttatctgacgtacattctacggcacaagccgcaggacattggtatcgctatggacacgcagggctgggtgtcggtctctgacctgttagagaaagctaagtatgttaagccggtcactctcgatatgttagtcgcagaagtagacgcagacgagaagggtcgctttgagttcaatcgtgaccagacaaagattcgctgtgttcaggggcactcggtcgagcatgttatcatcaacatggaagaatggactgagttggctccactgtatcacggcacggcagaaaagaacgtgtcgtcaatcatgcacgaaggtattctgaaacgcaaacgcaagcacgtccatatcagcaacgatattgaaacggcgcagcgtgttggtcaacgtcacggagaacctgttgtgtttgagattgacgctcgggccatgatcactcacggctataagttctaccgcgcagaaaacggtgtcatcctaactgaccacgtaccgtcccgctatatcaagttggtgtagttatggaaaagacgtacatgagtcattggggatcgcgctatgtgcggtcgtcatctggccgatggttctcagttcatggacgtgaaggaacaatggtgaccaatcggtatggaacgacgttctaccgtagcggttcagaagtgtggcgcgacataaccaaagggtgggagatagctctggagcgcgaactgcatagtcgaactcgaaaggactttgaggcgattaatgagaagttccttcactggggtaagataatcagaacgatgattgagcaagggatcgcagagaacaaccagcatactcaagacttagctgagatgcttgaggcgcagcgcatcaaatcttacggacccaaaatcgagcaactacgcataatactggatgaaacagccattaaaagctgagtctgattgtgttataatagagatgaacgcgagacactcgtttagctacttacatgaggatatgtatatgaaaaagtcaaaagttaaagcagaagttgttgcacctactattgaaggccgcccattcactttgtacaacgcctcgcctattcctgaggtatcagaaacaccattcgctgatcgtgatacatttcttcctatgctacgtaaagttcaggacgctgctcaactggaacgcattcgtggtttatcctgctgtccgtattgccgtgagacaatgatgcttggtgaatacaccaaagacaactggctctggtcatactgctatcagcacatgattgagcaccacaacgtaacgccgtccgcagaatttattgcttacgtcgaagctgcttccaagtaacctgaaatttagctgaggatatgtacatgaaaaagattaaacacaccttccgcctgactgacttggttcgtattgccgatgaacttccttcgaccaagagcgctttcacttctggtgaagatgcaattgttgttggtcgtgatgaaacagaagataagtataaacttcacatcaagcatgaaggcgaatgtgcttggtatcacgcagagcacctgacgctgattaaacacaatcagagcgaattgctcgacaagtgggaagccggtaagtacggcaagaagaaaaagaaagagcgcaagattcctgacgaactgcgcaacttcaccgctattctgcctgtgacctgtaacgctgattgctctttctgtcctgagaaagagatggagaataaagcagatcagaaagcgtggtcaaacaatctgattgctgcgattaaggcacatggccatcgcgttgaccacgtatcaatctctggcggtgagcctacacttcgcatgaagtacctgttcgaaacgatcgaccgcattcgtgctgaaacaggtatgcgtaaagtgggtctgacttctaacggtcagttccttgagaagcacaatcaaacaatgacgttcctcgatcttaacacggacgagatgctggagagcaagctatcgcatctgaatatcagtatgcactcattcgaccgtgagaaagcaaacaagatcatgggcgtcaagtatacgtggacgattgaagacctggttcgcttccgccgtcagttagggcgcaagctgagtttccacatcaacttcgttatcaacaaagagaacatcgacagcatcgagtgggagtttcgtcaggcaaacgagttcatgaaagcaaacccgtggatagacgttgtgttccgtgttgactacgacaataagaaactaagcaaagaactgcgcaagtatggtcaagctgtacaggctgcgcgtgaagaaaagcgtccgcgtgataagagcatcaagtatactcctaagaaagtcaaagaacctgaactgattaaactgttcaactctatctttgacggcagctattacgacgaactgacggaagaaactctgcctggtttcggtgacacgtttactacaggctgcccgtcctgcttcacgcatcgtagtaccgatctcggtaacagctttgcgtatctgaaagcgtcttcatacgaaccgaacgaagacgaagaagaatatactgagatggtattccacatggacggcagcctgtacttcgactggtcgcgcaaagagcctgtaccagaagtgaaagcgaagaaggctaaacctctgcctcgtttgaagaaagctaagaaggctgaaccgaaaggttatcctgatagctgcgactttggttcttctcgttgtggattcactggcggtaacgggcgttgtggtttcggtagcggcatgtgctaataggaaaaactaaaaatggctactcaattagaagtgaacaagttcctgaccgagtttgaaaagaaattccgtcaatctatcccgctgcttgggcaggaagagttctttgcttgtgtgcttgagcaaaccaatcgtgaaagctacatcgtgtgtcttgaggacgaatcgcttcttgagatgtttgagcaggaagagtctggcccgttaagtggtttcgagttccttgaaaacgaactagatcggatagaagctgagttggaccaagaccctggcttccgcgttctgcgtattgcgtttgcaaactgggcaggaacaaccaaagagctggagaacattatgctctgtgttatggacgagatgggttttgatctggatgatcatcctgaacttattattgaacctgtggttgaaatcaaactgaatgcagacgaattgaaagcactgttctcggtagttcaggaatatacaggacccgaagttcatcgtctgtatgcgatgtatatcgttcgtaagctggagcgtgttgctacaggccgtcctctgctagagaagttcgcgtacctcaataagtctagcagtgaacaggaactcaagaccgttcttgctgagatgggagaatagcatgactcgtaacttttactatcacagtccgttctactacgggcttatcgtatggcgcaggcgcctcgctattacaggcgctatgctgattgctattctgatcatgcacggccgttcagcgcctgctgttgaggacatgtggttctggacaggcatcatcttcggtcttgttggcggtgtatgctacattcgcatgtggtcttatgagcaatacctgctcgctgcaatgggcccgcttgataacaacactattgtgggttcgttgaacttcgataagatcgaacgtaaacacgcagtctggtacgagaagaagtttggctgcaagcctcctaaaactaacacatggagtatcgactgatgcctcgcatgttcactgatacacaccgtaagaaatactttcgccgtgctgatgacccgcaatatcatggtcacaagtgcgagggcatttaccgtgaagcaatggcgacgctacagaatctgcattattacaagcaagccattggtgcgatgcgtatgcgcgagcgtatgactgtagatacgtctcgaaagtttcaagagtgggaacgtctcggtacgttgattaaaggcaatccgagttatgaggaattgcgttcagcggtcaacatgtgtgcgttcaggctcaagcgtcttcgcattgaatataccgaagagcattcacggcgacacaatcaaccactgagttttgaagtgagagatgcggacaacaatcgcgttgacgtgttcgtgactcacgaagcagcgagatactgcaaactgcactctggtctcggtgcaaacatcattcgttatgaggaacagaaataaaatggctgtaggctttgtgaaagacgatggcgtaaacgataccatcgaaacaaacgtaatgaacgagattgaccgcgctcgttcggaacttcaaggcgtaggttctgattactgcgtcaaccctgactgcggtgaaaagattcctgtgatgcgtaagctcgctatgccgaatgcgcgttactgcattaactgtcaggcaagtcacgatggttctgctcatgctggctacaatcgtcgtggctccaaagactctcaattgaggtagtcatggacattaaagctagccctgaagaacgcaaagaaccgtattcccgctgcactgactgccgtactcctctggctgagggtgaagtgtatggtgagtgggatgacctgtgtgaaaattgctccgctgatcgtgaagacgaaggcgaatcaacctgaataaggagaacaccgtgggcagtatcattcaattcctcatggacgaggacgaagtgcaagacgcacttactgcataccgcactgacccgaccgaagctaataagcgtcgtgtgattgaaacgattcttgcggaacgcgaaacggcaaaacgtattgagcctgatttgcctgtagttaagcctaagcctattcatcggtatgtgcttataccgaacgtcaccactatctataaacaaaacgtgacgagtacagggaagggcggcactacaatgtcacgcaacatagacccggaacgtaagtcgatagctgctcttgctcgacgcgccgctgatcacattcatcagcttggaggttctgctgcctacgtccgttttgaatttgacgaatggcaggcgctgtttgagaacgaaggtcacgttggcacagtcaacatgttcaacaacatccaagagtacgatgacttggataagatagctgacttgctgaatacttttattgcgcgacttggtaacgtcgatagccctgagtacggagcaaaacttctgcgtaagatgtacgctgtagcacagggtaagattgatgacactatcggcaaggcgattattcgcatgatagatacgtcgggcaccaagaacgtacccagcgtactgtaaagaacagacagtcgaataacgaggataataaaatgatcagacaagttcctatcagaatctccagcaaagagcctaacacttcaatcgaagaagttgctcttgttcgcggcttcaaaaactacaccgttgttgttcgcggtccgtggcgtcttattcgttgtaccgatactgttgacctcaaagtcgtgcttatcggtccctacgacgtaatgccgaacattacaggctacgagattctgacctctgccggtttctcgtcagtcgatgctgcgttagctcttggtgcaaaacactatgaagttaagacgtggcagaagcaacaacgcgctcgcctgaaagcagcaaaagcacaaccgcgcctcggccgtactaacgcactcgacgatctttaaggagaaagcaatgaaacagttattcgtaggcagctacccgaacaccgtgaaattctctgacctcgatgcgcgtgaccgtgtgtgcgagattcgtgtcatgatcgccaacgcgtacactacgttgcgcgatgctatcggcgaacaggccaagaacgaaacgaataccttccacggaccgtggttagtgtttcgcaatctcatgaacgaacacccggcagcgtgtctggaagaatatcgtcatgctgcaatctacttcgacgcagacactgaaggccagattactgaaatctgcaaactgattgaacagcacatagacctgactcgtcaggctctcagtctgaaaggtgttcatcaacatcaggcagacgcgatggttggcattgaggcaactcccaccacccatgaagtaactatgcgcgtcggcgttggcaaaacacgcagtgaaggtgtgtttgactataagctgtcgggcaataacccgcatctgatcatggctgatagcgttcgcaagtatatcgagctggccgctgagaaagaatcagtgtttgccttctgcgttctgctgaccaagaagttgaagtcagattgttatgaccgttacgaagatatgactcaggaagaaatgattgagtgcgtacgcggtcttattctcgcttcatcccagagcgtgaagtgcatccgcgaacatgttgagtccgccgccaacgaactctctatgccgtatgcgcagttcgttgctgacgttaactctgacttcgacgcagaagatgaccgggcggctgacgatgaaaactacgctctccgcaattaaacgttactggcgcgaagctctgatacttgccacgttgcttgtcattgctatcgcgcttccttatttcgaagtacgcagcccagcactaaccctgctggtggctattattgttgctgcgtacttctttgccacttgggcatgtaaaccgcgttacggagataacagtgaaaaagaatgaagtggtactgagtgcaagcgaagtcgctgacggcgtggataaaatcaatcaggcactgctggaagttggtctgcgttgtaacatcggtgatgttgggtacgagccgacatatactgatgacctcggtgaaacacaaggcggtcggtacgcacagtttgataagaagtcccgcgacaagctgcgtcaatcaaagcaggtatcgtggcacaacactgggatgattggcggtgatacacttgaggagattctcaaagtgatcgcctgtcttaaattccgtaatcacaagaaagagccgaccttggttcaagttgaaaaggtaatgtacacgatgactaaagaaggcgccacaaagaaagctcttgaagtctacaactcagccgcgccgttgtctgacgaagacctcaagttgtgtatcgatcacttccgcactctggaagagctgatcaaagttgacccgatgttgaagctggcccagccttatgttgtaaacaacctttatcaactcgaaaactatctacacgctcgtaagagcaagtaataatcatgggaggcccttagcggggtttcccttttgtcatttctggagcattttcgcatgagattcggattcgcctgcaagctgattgacgcaaacggcaaacagccctacccaaacaaaagcattagctacacccacttctctaaacttgacctcgacgcacaacgtcaacgcctgcgcgagatagtcacggtcaacctgacttcactttacgatatgatcgcacacgttgcgatgctgcgtactgacatgcgcatgtttcgtatcacaagcgaactacttccgctctacacgcacccgcatgtatctcacctgtatgacgagcgcgaactcgcctcgtacattgaacactggttgtggaagtgcggtagtcttgcacgtagttctggcgttcgtctttcgtttcacccaggtcagttcacggtactcgcatctgatcgtcctgatgttgtcgtcaactcgatacgcgaacttgagtaccacgcgtactgcgcctaccacatgggatacggtcgtcgctttcaggacttcaagatcaacattcacctgagcggtagacttggtgcgaaaggcttccgtgctgctcactcaaaactttctgaccactgccgtaagatgcttacggtggagaacgacgagattacttcgagcgtagaagattgcttggagctggcggacctgtgcccgatagttctcgacattcatcatcactgggtaatgacaaacgaatacattcaaccagacgatgatcgtgttcaacgtgtcattgagtcttggcgcggcattactcctgttgcgcactactcagtttcaaagccagagttcgtgccgtctcgtggtctgcctgatcaaaacaagctgactgctaatcgtatgcagttacgtgcccacgcagattactatcacaacgaagacgtaaacgactgggctctcagcttctctgaatttgacctgatgtgcgagtcaaaagcgaagaatagagcgcgaatgaaattggcgtgttttacgctcaactcagcaaataactggacaaaataaggcttgttttcgaaggttgccctatgatacactgtttatgagcgctatcgctcgtttttctcatataagaagacagaggaaataagacaatgttcaatacgacaactatcgcaacgaaagcaagcattgcaccgaccgttaaacactcttttggcatcacgggtcttgcacccactaatcgtatctcctgtgtttggcctggcgctctggaagttccgctgcacattaaacgttggtgccgtgccaacgaaatcatgaatgaccttgacccgtacatgcgtgttcgctttaaaggtcgtcgcgcggatattctgaatttggttgctgtccatctggcaccaaataactctgagcttgcggttcgcattctcgcaactattactgaggcctaaaatgaaagtccaaccactggaagctatgtacggtgctacgaacaccaatactccgctgatagaaaagcgcggcttccgtcctgtcgaatcaaaatatgtcgatggcacggaggttagattacaacggctatcacacgatgtacatgaacgtgtggttgttggttacgatcaatttggtcgtgctgtgtatggaacacggacaccgcaatcaacgttcgaagtgcgtgacagcaaggaaagcgaaccgaataaaacggcgccctagcaagctcacaaccagaagccatagaataacccaaacaataaattcatgcgctgacctatcgtggggtgtcttaaaatgatcgttatttgtaatagttcaaaacagttttgtgcggatcgcctagcacacggggatgcttttgtttttgggaagacgcgcatgttactacgcgctgacttcatcgtcctgaccgacaagaacaatagcttctatgtagtacgcaaatctgatgttgtttggtcgcctgagcttacaggtgctacgcatgtgattaaaatccgggcgtatgcccagattaagccgttcgaactcaacgcagcatgtccacaattcaacagccgcgtattcggaacaatcgcgttccgcaatccgcactttgagcatagactctcgggtcttaaatatgtagagacaaacttcggaggtttacatggcacggtatcatgtgtttagtgcgacccataagtatttcggcgaagcatatgaaggtacgtggctgaaagagatcgttctcaacggccagcaagttaccatcgctgagtttccagacttcaacgctgccaaagaatgcgctgacaagctgcatgaggtttgcgatatagggtggatagtctacaacgccttttccgaaagagcgatgtatgatacccgtacagagcaaggcgagtctgtaaatacatagcagcctcgcctgcacctttttcttaccgtgaggcttacgggcttcacataaattcatatcaatgaggttcaaaatgaaattcacttcaatcgctatcgcactggttctggctgcttcttccgctaacgctgcaaactacaaagcaccagctccggccgcaggtatgcagtcgtctggcatgactatttctgatcagctggatgatagctgcctcagcaagctcgctgccgccagtgacctgcgcgaagctgttgttgacttcgctgtgtcgcgtgatgctatcgacactgttgcactttggcctctggtctgttcgccgactgttgaagccaagtctatcgacgtcgagcgtatgggctccgacctgacaatcacttacgtcaacaaagacgcgtctgtgccaaaactcactctggttctgcaacgcgtccgctctgagaacgaagacgatgctcctgcgtatcagatcgttcaggttggtgatatgaatgctatgggctacgaagaacagtctgctgttaaagactggctgctcgaatgctacgcgctcaccgttcaagatagtatggcggtggtgctgaactgatgaaaggaaagaagttagacatattcctgcaacaacgcacggcaataaacaaggttgcttccagtccacaagactgggagacctataaagaaatgctgctgaacatacggcttgccgttgctgttgacccacgccctgatgctgctgtacgccacttggctcgtacatggcatgcagaaaagaaatatgcgctccctgtctgtcaggctacgcttctaaaacttatgacgttgaagaaagcgaatcaaacgcttgaagaaatgatcgcgttgtacattgaccttgaggaaggaactcagaaatgatcgaaaagaatgaacaactggccgatgcggttcgccgtatgtttaactcaggcagcgttgaagtgcgtgatgcgctacgcgcagtagcaaacactgtgctggctaaagatgttgctctgccttatgaaggtgacgagccgtccgtagagacaacgtatcgtctgctggaagggatccaattctccggtgacggtaaaacgcttctgccctctgacgaaatctacgcgctcgataaactgctgtcgaagaagtggcgtgatactttcttctctgccgtgtcgaacatggcgctgactatgcactgcaccgacccacgcaccgcaggcaaaggctactggccaccgaataacagttcctgctgtgagctggttactcgtgccttcatctggactgtagctcaatacggtctggacaatcttctcgaaaaagacacgtcggttgtcagtcacacgcgtctgcctcagtttatcatcgcgttgcagaccgaaggcaaagacgaaggctatgcacgtcactttagtctgtatcatcctcacaacgatacaggcaatatcgacacgaccaactactggccggacgagtacaaaattcagcaggaagaaaaacgcatcgcaagtcgccctgctgaatacgactccgtccgtcatatgggattcgacgagctggccgctctgtgtactcgtctgaatcttattggaccaaactccaaagttcgctgtgattgcgatgaagacgaagaggagattgattgcgattgccagcctatgatggtggaagacttcgatcaggacctcgacgaactgcaacaagtcttctatgacaaatacggtgacccggacgaagacacggacgaagatgaaagtgagtggattactggcgtgtctgttatggaagtcactatcgatcttcctactgtgcgtctgcctgagcctgctcaaaacaaccgctcacctctgcctcgtcgtggtcagaagaaagcatatgcgaagccaatgccacgcaaagtcacattgactcacgatcagcaaatctggcatgagctggacagcaaacaagagttcggtgaccgccgcttcgctatcactctcgtatctcgtcacacgtgcggtgttgatcgcgctatcgctactaaccgtgaagcgctggcagtcgcgtacactcttatcaacatcgacaaataactggtcaaaatagcgcttcttcgtggggcgcttttctgctataatagcagctagagcaacatcgctctcaacgtcatttttaactatacgtttataacgggaattgtcatttatgtcacgcactatttcacgcaagaaagcagtaagcctcatgtccacaacttacaacgcaaaacatcctgagtatcttccgcgcctgttggccgaagatatggactcgactcacctgttcgagtttcgtgagatggttgttgctaagattcaggctggcgaagacccgactaaagttgtcgatgatatgatcgacacggcgattcgcgttactcaggttcgtcgtcgcaccagcaacgattacaacccgaagattgccgacgtgcttactgatgaattgcgtgatatgctccgtaaactctaaggataaaaatgaaaagctacggttacttttatattctgaatcacatcgctatggccgtagatgcacccaacaaggaagttgggtttaaagctctagtagaactggacatgttcaatcgcgcatctattctgactcgccctgacgctaacccgcgcgctgcaaagattgtgcgtgacctgactgaggcgctttatccctctgcaacggatattcatccaactgtcgcgcaacgcatgatgctggtgcaagcgctgcatgatcaagaacttgaatctatcgttggcagcattcgcttcttcgtaccgttcgcgtatacgaaagagcaactgactgaccagttcggtttctttgataacggcgacggcttgaacgtgccgtacttcttgcgtcacctctttatggaagatcaagcagtcttccttgacggcaagctgaccagcttcgctaattcgtgcatcaacggagaagtgtcgcaaactgctcggcagtatggtctgctccctgctcaggcttacggtaagaacgatattcctgagcgcttcaaacatctgcctctgttttaggagacactcatgggagttgttaaaggcataaccgccaccacgttcccttctcggggacgtgacgagggccagaagattgctctcaggtgtcgttggggaatttacccagcaactattgttcgtcaagacaacgatctaccttataatgagatcttgaagatcgatgcaaagaatcttccgcgtcgttacttctcgacgactgacgacctgttcgtgtctcgtcacttcattgataacttcgcaaagcattcgcctatctgtccgaagggtgagtatgaagatcaattcgtcgatgttgtgtttgatcgcgacacggagaataaatgcgaaggcgttgttatgacgcatcgtgatttgcttgtagtgattctgattactacaggccctcatgcaggccgctacgtcactgacaaagagtgtcagtacgcgccgaagcctcgcaaagtaaaagaactaatcgacaattaaggatgtagaatgcaattcaaagtaatgcctgacctcaatcgtttccctgaatttaaaatgccagctcgcgcctctgggcaggctgccggtgttgacctgttcgctcaggaagacatgatcatcaccgaacagacaactctgtttgagctgggcttcaaagctgccgtgcctgagggctacgtaggcatcatcttccctcgcagtggtctgggcgctaaattcaactgtgaactgtctaacactctgggcgtcattgatagcgactatcgcggtcagtggatggctgctctgcatctcggcggtaaaggtacgaaaggcaacgcactcgaagatgtgcgcactattctgcgcagtgttgcgccggccgttgcttctctcgttgaaggccccgatacacaactcggtctgcatattaaacgcggtgaagcgtatgctcaggtgttgttcttcgaagtgcctctgatggaaatcacgcaggtagattcactggacgacactgaacgtggtgagggtggcttcggttcaaccacacctgctcgtggctaacctgctgtatgtgctaatcgcctactatctggtaggcgttattcagttctttcgtgaactacgctccatcccaaatgacgatcccgtagtaactcagttcaatcgcagtatggataatgaatccaacctgcaggtactttggatagggatcaaactcgctgttactgtgatattcattcacattccgtgctggatatttcgtatatagtgatgctactcacacgaggagccttacgtgggctcctcattatcgtaatataaacactatggcaaagaaaacttatctgctacctcgtgagcgaccaagcccgctgcctaacttacgagcctatctcgcgttcctcgctaggaagcctaatgctaatcgcgcagtattagaatcgtattgcaaagcaagtctggcacaaatggctcgcagccgtttctttgtaggtaagctctttggctacaaagtgtatacgaaatcgaacaagctcgcatacacggttgtgtggattgacccatacaactatgactgtcttgttctgaaccatcaaaggagagaagtagagttcaaaaacctttacggcctgcttttatagttaggtcctagcgccttcacactaggggaaaacttccgatgataactgttcttaacaatcgtaccgacgaggtaattaaacgcctgaacgtagcagtatgggcttgtgtcgccgttatgtttgctgtgtatatcgcagtaacgagcaacgcaaacgccagtatgtctacaggccctgacaacgccattgatatgtcttccgccgtgtcacttgatccctccaatcgagtggctactaaatacaaggagatagaaaaggcagtagcagtaaaagacgaacgaaggcccaaacgttatgtaacgagagagcgcctccggcaactctatgctcacttgcctcacccgtctgatttaggcaagcagattgatttggccgcagagaagtacaacgtagatgcaaaactgcttctatcaatctgcgtgtccgagtcgcatctccgtgcaaagatcaggaacaaatccggagctacaggcctgtgtcaaatcatgcctgacatgcacggacgttctgcgcgggaactcatggactaccgaatcaatgttgatcaggcagcccagattgttgcgttactaaacaagcagtgtaaaggcagacgcgcctgcgtcattcaaagctacaacactggttggggagcatatttgagaggggtacgtgccccacaatatttagcgaaagtccagactgagtatcgccgcaagcatactccttcttcctaatagaggatataataatgaacatcaatatcaccgcgctgtacaaaatgcaattccagttgctgaaacctttatcgcctcgtcaggagtatgcgctcgttgtcctgctctgcgagaacatcaatgaaggtgatgtggctgcactggcagaagtaatcgttcgtgactacccgcatgtagcgcgtctgtatgatgcgtttgctgccgccaaccagtacgacaatgctgtaccgtttatcgttcctgtgttgaactcggaagaagtcaccgaagagatcttctgcattcgtgatcacgcactcgtcgttgcaccagatctgcgtgaatctctgtgtcaggctctgactcgcgttgtgctgatgcgcgaaacgcctgatgaattgctcatgcgtgaaggcgccgaagtgattctggttacagatgctataccgtatctgcttggccagttcatggattgtatgctcgatgcgtacaattgcggtgtgctgcctatggttgttcgtcctacgaaagaccagcaggccatgcgtgatgatcgtctgttgtcgtttgagatgctacgcgacaataacatgttctctggaagtctggacttcactaaagctctacagccgagcgagaaagccaaagcgattgctgcccagcttatctctcgtctgcgcactgtcaagcctgcacgtggcttcgatgcggtaacacaataaacccaacgggagaccttaactggtttcccgtttttcatttctgcgcaaattttgagactatgacaatgaacgaacaattcgcatcaatccctgctgataaaaccactctgccgttctattcttctgttgcactcaacacctacttcaatgatcgtatcaagcgtcttggtctgactaaggtttgggaatacgtcgaacgcaacaaccgtcctgcgttcggcgatgatcagataatggaagctctgcattaccattcgacgatacacatgaagcatgtaactgcgctcgctctttggttgctcgactgcgaagccgttcacgattggcagtacagcaacggcgcagcatcgttagctatcgcctgtatgttccatgacatgaaccattcgcttggtcagaaagatgatgcgtacaatgttcagcaagctattgcagctctggagaaagctgcgcaccacgaactggccgatgccgtgctgatcgataactgcgatattgcctctgacctgattcgtgtcacacaattcccgtactcggatgatcgtaagccaaagaatatgattgagcgttgcattcgtgatgcggacattatttacggtatgcagccgttcgttatcgactacgttatgtatggtctgcgtgacgaagtgaacagcaaccctgaaatgccttacccgttcactcgtcaagactgggcctcgggtcgtgttgacttcttgcatggcgttgagatgtttacgcagacaggtaaagacgctatggattggctgcttgatgaagaaaacgatcacaaccatcagtcgaagattgaaaactggatgaccgacaacatcgagttcgtcctcaccagtgcgcgccatatcaaagcgaacgatgttctgtttatcgacacgccagaagacacgttgaaagctcgtcgtttggtcgagcgtgtggaagattgttaccccgatatcaatctgtatttcatgggtggcacttcttgctcgctacgcaacggcgagcactgcattcgcgtcgaaagaaacaaataatcggctgaaataaccatgctgtctaaagtgcgtctatgctacaatatgcgtagacgcactaacaaagagaaaacgatatgaagccattaaaacgaatccctctgagttcagatacaaacctgtttgctattaacgccatagtctatatgaccgcatttctatatctggacgttactgtgcattccgaacatttcggagacaaagaaataatgctaccagtgagggtcaatcacaatgtgtcgccccatgaacgtctggctggtgtacagtatgccgcttatatacctgtgttggcgtgtcatccgatatccgacaccgagttccatacagagcttggttacacggaagtgaatgtcaaacacttatccatggactataccaaatgcagtcattgggcatacatcggccttctgcctgacgtggctgagtctgatatgcgagacaagcgttatgtcgcgcctcttcgtgtgtatacagttccacatgaaatgggtatgcctgatatatacaaacggcatattgctcgcggtgcagcgatacgtcctgactatctgcgcacttcggctctggacaatattgacaatgaaacctgggaacaacttcgggctcgtccagatcgcggtacctcgtggtcggacttcttagacgcaatcactaacggacgtctgacacctaaagacaatctatccgaatgtcttgaaagcatagatcaggagttcatgcctgagagtgtagttaaacgtctgcgtcaggctcagattcaaagacgcatgagaggttaatcatgatgcacgatatatacaaggtaagtgctgtcctgttctacctgcttggcgctatggctttccttgcacatatcgttggcttcgtgaagaactggatgaagataaaagagatgcggcagaaagcgcaggcgaagattgccaaagtgaaaacgccgcacgaactcattaaacgccgtctgcgcaaagcagaagaacgcgcacggtatcgcccacgtaaactgagagactgacaatgcctactattactcgtaacgacacactggaaaagaaagtacaacgcgcactggaaatctgctggaacgaaacagtaaagaacaattcagggccgacgacttatgcttttctcgcttcttcatttgctgctgatggtcgcagcctgttcgaaaatgaattgaagatgatcggcgtcatgctgcgtgacggtcttaacatcaacctgtatggtcgctatgcagcaactacctacacaagcaacaagggaatcatgatcgcattccagcctgttgctgatctcgaagatattgtggagatgactctataatggaacagattgatttgttcgcgtggccagactgcggccgtacaatgtacgaagcacacacgctgctggagccagcagttcgaacgcctgacttcgcagtacgtcagatgcgctacactcatgcggccttcggcaatagcggggcaattggcggggcactctttccgcagaagctgaacaagaaaattgtcagcctgcacgaatttatcatcggcccaagccctgcgtttcagcgtgagataactgctggctctggtgatgtagcaaacatgatggacccgcagtatctgtacaacctgtatctgcatacagagaccgttgcaattcgtgtgtctgagttccataacttcactgaacggggtccgttgtctgcgctgcacctattcactgtagcgactatttatgagatgcgcctgatcgtttactttgcagatgacggcatcgaaactgatcgtgaccgtgaagattggttgcagagcattcgtggttacttctcgaaccgcagcaagttccgtatcaaagcagaaaaaactttattcactaaataaccgcagcgcttacgggcgtcgcacaggagaaacattatgtcattcgatatgcgccagaacgtactcatggttcgctctttgattagcggccaaccgttctattatttctacaacgcagaaggcttggagttcagcctgtctggttaccagctcaaagagatttatgatcgtcactttgatggtcgtatgtctgctgtcactacttactggggcttcacaaacaagccgaactatgagtctttcgagtttgcggataacggtgacttgttgtggcatgtttctctgaatgctgtgtgtcacacgtatctgcctcttgagatggttatcggtcatgaaggcttcaacgtgattaacggattcatgatcgaagatcacaaacgcatggtgatgaagattcatcaaaaagctgtcgggcgtagcgttgaaaaacttacatggttccatgatatgtccgaagagcgtatgcgggaaatgttgaatgctctcggtcacggtccgctgcgtattgaacgtgctgaccgtgaagaattgattaagattcatcgggactggaagcgtaagcacgacgaagaatttaaatacacacacaacgcctgtggtattgacccggacgacaaactccctgctgacctgtacgacgatcacggcaagtggttgcgccagcggcacatggcaaaaggcaaaacgcttgagatgatggccagcgaacttgcgaacatcgtccgcatctttgacctgtacatcggcgatgatgactttgaccacatgaatccggattgggacgaaggtctgcgtcgtgttgctcaagcattcatctacgggcctaacgccaaagagcgtttcgatgaagtgaagtataatcctcaattcgttgtcaatggtatctatgcgttggcgaaagacttgaactggattcatgttaacgaagaatctcaggactataaagagtcgttgattcgtcgcctgatgcaagaactgaaaaacgaagtagaacggccggacggggtgttcgttcttgaagacggtgtagtaatgttgaaagctgccttggcagtagcgaacgcagaagaggaagaagaagaagaggacgatgattcttccgctcgcgcagaagtgcgtacctacctcgaaggtctcagtgaagaaaagctgcgtacagtagcaattgatcacaagctggccaagaaaatgaagattgccaagatggccaagagcgagctggtggacttgtgtgctgactatttcggctcagactttcctgaggacgaagaagaggaagaagaacacgaatagcctgaaagaactaattaaacacgcaacactttaatcttccaatcatacctaacattgtagggaacaaaaatgaaattcgaacaaaacattctggtagtaaatcgcatcgctcttatcatgaacgacgaactggtgcagaagtggggtgatgcagcaaacgctgatcgtaatgctacagcgtatgcaactgcaatcattctcgccaaacttcaacagcgcgtgtccgtcgctctgcataccgagaatcctgaggcgtgtgctcgtcctgaattgctctggacagactacggttctatttcggtaagcggcctgtttatcatcgcctctacttcggataaagaggtgctcaatcactacgaagaccatgactatcttaatcatctgcacacaatcaaacgtgtagcggaagagaacggatttaagttaacggtcgttcctgtgaaagcgaacttcccgttctctaatactgaaatccctgccagtatgaagtgaggtgatctatgaagcgtgaacacattccgatgatcgatgccgctatcgttttaacgatggaagaaagtcgtagctttatgggtcaacgccctgatggctttgtctatctgccgagcaaggaagcactggagaagttcgaagcgcatattcagaagcaccgaagctatgacagctacagcactatcctgcaccgcgagcttcacgctatcagcgctgagggcgtcgatgcgcttactgctgatattgagcgcgattcaagcaagccctggatgtggtcagacgtagactaccgtatcaagctgtggtaagcaaataactggtcaaaatgacggtagtatctgaaaccgcattatgatatactagaagcgtagcgactgctgcgcttttttaacttatgtctgaggagacaacaaaatgctgcaagaaactcaagccaccctgtccgatatcgaactgcaagaccgcatggtagatgctgccgcccagaaacttatcgaactgaaacctgagtgggttgacgtttgcgctgcggcacttcgtttatatctgaccgtgtgcgaacaactcggcggtgaaattcctgaactgcgttttgttcacaactgccgtccgactcgtttgcagttccgtctggcggaaagtgttgagggtgaggagttcgttgccaacgaactcaacaaagaacaccagatggctatggccgaagcaattctcgatgttgccgaagcaaacgaagatggccactcgctgatggatttagctatctcctctggtcgtctgttcatgattggttacgacgggcttgcaggtacgcttgataagatttgcttccgtagtcataaaaagaactacaccatgaatctggttaaagaggcttaacatgaaacaggaatacactctgcttaaacgaagcaaagttgatgttaatcgttttgctttcgtgtgtgatggcgaggtggtagccaactttactgctggccagttgttcgtgacaatgcaaaaactcaaacacgccgacgctattaaaaacgtcgatgtgctctggcgtgacggtacgcgcacagttgaagaactgcgtgtggttgagcaacgacgatttattcaattcgatatgctcgaatatgagcattcgatttgcttgctgatgcgagcacaggggctgcctgttgagttgtccgttcctgttgacgtgcgcaagctgtttgataagcatggaccgtttatcacagaaattcgtgtgccgtcagaactcgttgctgatctgcatcctgctttagagcgcttcactccagacgaagacgacgatatggatgaagactttgatgaagacgacgaagcggaggatatggatgacactgactttggcttccgtccagaagacattcgccagcagttaggtgattttaactatcgctcaccggattgggttgttactatgactgatgttcaggtggatgaagtaaatcaccttgaagtcggcatcgaccctgacattgaacttcctcgtgcggctgacgcgaaggacgaatttttctaatgaaaagtacaaacgatttggtcaaagagttacgcagacacggccagcttactattgacgagcgcgagaaacacttgctgccagatttaacgttcacgcttgattgtctgtgtatcacatacaagaagcgggaaatagagactaccaagcgtggtcgtgtcataacgataaagttgatcaacgttcattaacaatccagagtttggcgcgcccgtccagaaatgctcaattccccaagtgaggtgcttcgcgcagaagcatgacggtgcgggtcctttttgaagcgtactaatcgagtgtgtttcacaaagaacccaaaacaaacaggaggctgttatgaagtttaacgatgtgagtaaagatgctcaggtcattcttatgggcgctgcacttgctggcgtgatcgaagcgttcggacgtgacgacgaagatgaaggcaagcagttgattgaaactgcgttgcgccaagtcggtttgacgttcgacgagttccgcgtcctgatgaccgaaatcccacctgaagttgaagcggaagttgcgtctgtccagacagtagttgctgatccggacgatgacttcgatgacgaacaactggacacaatggaagaacgtccaggcaatctgaacgatgatgggcgcactgatgaaaatggctggcaagatcttgacgaagatactgtgtgccagatgtgcggcaaagaacactgcgaatgcaatcgcatagggtgatcaaatgagccgacgcccaacgcaagatgaagtgaacggccagatagctgcctcagaagaacaacgctatagcgaacgtgaggcacaatacgctgattggtcagatgacgatttgcgtaatgcgctgttggagaacggtctagtctttgatgacgatgacttagacgactacagccgacaagactgtctcagactgcttctgggcagcggctactaagcataaaactggacaaaatgacggttgtgtcaaaacagcgtccgtgatagaatatagatgtagggcgcatatcgtgaggagtgcgctctatatgcgaatgacgcgattcgcagtacgagagaagttcttgaccgtgtgttttcgtttttcccggacacacggtcctttttcaagtgccttcgaagtttgagggtgcttgcgaaagggttcgataccctttgagcgtacagggctttacgcggtttccgccttgtatgctctcatgctaaaccgcaaaggaaatagatatgtcaaactcaaaagctgccgctaaacgttcaacgccacgtggtccttcatcggttcgtcctaagacagcgcctcgtcctcttgataaagacgctgtgccgaagatgcgcgatgacgaacgtgtgtataatcttgttcgcacaattctgtctgcgtggaaagcagatatcggacatgccgaacatacggcagcctctagcggtatcatcaaagtatcgcgccgtaagattgaaggtgctttacgtgacctcaagaatacacgcttcactaaaatcccgtcgctcattaatgatgttctgaccgatatggaactctgcaaagagttcgggcagtgggtgtacgtcgaacacgattctcctgattggattttcgttcgactgcctgaaaacagtacgcctgtattgcgggcagacattagctatgatcgcacagggcaaacgtctgcttctgtggcgacctcaagcgaagcgctgctggaagacctcgatgaagaagaggaagacgagattccagagaacgttgaatatgacgacgaagatgaatctcatgttcaggaagaagaggaggaagaataatgacctcttcaattcgtccagcctccgagacagccgcaatgatcattgaaaacgtcactctctattctcaagagaagggacacgaccacacgctgccgcgctttaaaatgcccgacactgcgatacgtcgaatctctggtcatgctcgcgttctgcctgagagttatatcgaccaagtatctatcgaattacaacaactcgactggatgatgatgcgatacaatgcaggcgagttcctctttctgcattttgatataccgaagaactggacgcgattgagcgcgaagcgtgtcgtaccaaacgacgaccctagcgctgagtacgacacgtggacattgcctgagctacagggcttcgttcaacgtaacgacttcttgcggccagacgaagaagggtttcacgatagagcgtcattagttcgtgctatcttgcgcggcgagactcactaagcaataacgagcaggcagcacgtagactgcctgctatctgcgaagtatgcagaaaactggacaaaatcgtggttgttatctgacagtcacctaagctatactatatgcagacgcattgagcgtcgcaaacaacatatcacttatactgaggagtattaaacatggcacgtatcgaaactaacactaatctggttggcaaaactatcgttctgctggacggcaccaaaactaaaatcgaagatgcaatcgcgtctggttataaagtgaagggccgttcaacgaaagttgcaactcgctgtgttatcaaagaaggctctcacttccgcgaaatcgaacgcatgaacatgagccagctggaagatactggtgaaggttacgttaagctgaaagaagcgaaagcgtcaggcaagaaaactgccgtcaagaaagaagcagctacgtcgaaagcgtcgggcaagaaagctggtggtaaagctgcggcgaaagacgcgaagccgtcgaaagacaaagagccgaaagttcgtcgtaaatcttccgaagagcagtccgaagattatcagaatctggctatggctatcatcaaaggcaaagccaagccggctgttgaaatcgaagctgttgacgaaacgctgaccgatactgtcgccaaacgtattgtcgatcacgttctgtcgtctgatattgcgcgagtgtgcgctgacaacaaaacgccgatcgctaacgacctggacgtgacgtatgaagccgaatacgcgcctgaaggtaacgtgattcagattacgatgaacctgcaatacgccgcgccggttaaagtgctgtctcgtcctacgctcgaaaacgcagaagctatcgaagcccgtgcgcagaagatgatcgcgccgaagctgtctaagaaactggcgaaagctattcgtgaagcattcagcctcgaagacgctaacgagctggaagccggtaccatgctgttgtctgatggtgctgagttcgtctactacggcgaatctgcgaagcatctgggcaaagcgctgctgtatgtcgtagagaccgacaagttcaaatctgttctcggttctactctgggtgagtatgaaatccccgacgcagaagaagaggaagaagtagaagacgaagaggaaatcgaagaagaagaggaagaagaggaagaagaggaagaagaagacggcgaagaggaagatgccgaagaatcgcaaggcgccgagtatgagttcgtcgctgtcgaagctgaccagctgaaactcgtcaacaagaaagtaacagcgaagtatcacgccgctctggcagaacgcttcggtgttgacgaagaagcgctggcccctggcctgatgttgactgacggcgaaactactttcgcttacctcggttgcgatagcaaaggcggtctgctggtgattgacctgtctgacgatgcggacgaagacgacaacgtgctggtctacagcaaagccgatatcaaaacgctgactgactttagccctgtgattgacagcggtgaagaagaagcggatggcgaagaagaagaagacgacgccgaagacaataacgctgacttcgaagaagaagacgaagacgctgacgaagaagaagaagacgaagacttcaacttcgacgacctgccgagcgaagatctggaagacctgtctgacgacgaactgcgtgaccgcgtagtcgaagccggcctgaccactccgcgcaaagcagacaaaatgaacgcgtctcaactgcgtaagctcctgaaataagttcgacctgtaatacaaaacactgatgatagatgcggttcagacagagccgcatctctgacaactaagctgattgaggaatcacactatgtcaaacgcaaacaaaatcctgttaaacgctcgtgttcgtcgtctggacggtactgtaactttcatcaacaaagtaaacgcgaacggatatagcaccgacgcgaagggacctcagatcccggtcaagcgtctcgtagtcgcaggcaaaactctgaaagagattgagtcgccgttctcgaaagaggagcacgtaatcgtgcagggcgtatcagtcaaactgaataagcgccagcagcgtgaacttgctgatggctcgctcgatgttaagtctttgaaccctgactttggtaagctggtcttcatcgaccctgaaacaggcaaagcgactgacgggaaagccgtgaagtcgaaagcgaaagcgaaagataaagacggtgtgaaagcgggtgtgaaagctactcgccagcgcaacaaagatacgcgcactaagaaagaacgtaaggcagaagtcgctgcgtcaaatgacgagctggacatgttgccgtctgataagattgatcgtaaagcagagctggccggtatcatcgacgcgactgtggctgatgcgacaaccaaagaacgtcgcaagctgttgtccgaagcgttcgatatggactggaaagatgtgaagaagcatggcggtaaaggcgtcatcaaacatctgggccgcaaagccgcgcagtctgctgtgaataaactgaatgctaccgtaacgcaggatgctttcattaagcagatgcctgttgcgttgaagcgtctgattcaggacggtacgttgacgcttaacagagcgcagattgagcgcgtactgagtgcgcttgacctcgacgtgaagttctacaacattgctatgcagacactgttgggcaatctcaagctgtcactcgaccagtctgtcgctgagccgaaagctggtaagaaagtgaagaaggtgaagaaagcaaaagctacttacgcctcagagaaagagcaaaagcgccgtgttaagaaaatgaaacactcgctgattgctccgccgaagaaaatgctgaaagaagcgaaggcccatatgaaagctgccaaagcggctatcgcacaaaagctgggtatctcttcgaaagaagttcagcggggtctgctggtgtatcgtgcgaacggcgatgaactgatgtttgttgcctgtgatatgacgggccctgtgttcatcggcaacgacggtgaagtggcagtgattgcctacgcaaacgtagagactgccttcgacttcactctgagcaaaacctctgaactggacgccactgtatgacaaacaatgaaattcttttgtcaggtatgtttgctcaactgtatgcgcggctgatgacggccgctgtattgaaaacccacgtgtactactctgacttggcgccgattgtgttcggcgtccaactgtcggtgattagcagtgcgcagtacgatgctctgtggtcgcttgtaaaagaaaccatgagcgtcgatatagctcacggcaggccaccgcttgctgcgttgtatgtatcaagggcatctgatagcaagctgcctgctaagaagttctttcgtgagtaccacaagctcacgggcaagaatttgtcagaagctgaatggcaagcactcgtcgaaaatgtgtgggaacactatcaaccaaatcttcggggtcttgtatgaaaaagtcaaaggtcacaatcagtcggggaggctacaaaccctcctcgcaagaagaggcacaaaagctggtggccgagttcattcttggtaccatcggtatcaaccctactgttatcagtcagcaaatgctgttgaacgttgctaactataactacctgacttctatcgccgacactggaaaagctaatcaagcgaaccagagcgcattgcataaaactgtaaaagaacttaatgcgttctgtagattgcacaagatctcgctgggattactaattatgccgcatacgtctgccagcgattatgctggtgacgaggttgtagcgattccgtgggagcatgtgcagaaaaacgcattgagccagtcggccatcacatctctgtttgaaacagttgaagctgatggttatccgcagtttgtgactgatgcgaaaacagtagagggatacaatgttctatgatcacgtattcaaccacgacgaaaagcaattgcttctgtcggtggctgagtctaagtatctggtgcggttagactgccccgattatttgaagaagtcgaaacacgcaattgaagttcgtcataccgtaaccaaccgcggcgagcaacgccgtagcggaacaataacaactgcgtttgtgcctcgtattcattcagcaaccgtacagcgtttggtgcgtgaagtgcgtgacactcaaagcaaaagcgcgtcgtccagtctcgctgcattattcgagcttggacttggtgtaccgaagcagcacgatattgcggtatacctgaaagactactgccaggaaaatgataagaagggtgtgggtatcaagtatatccgcaaactgattaacgagtaccatcgcaagcaccgccatagttttgcaggtagtcgctggctgatgcctgctgcgtatacagcgaacatgctgaacatgcagtccttcattcatctgaaagaaggtggttactcgaagaaagtgaaggtacctgacggcattcccgttgtgttcatctatcagaacacgaaccacgagaaagcaacctttactttgtgtgacgcattcacgataagcccgctcggctatccgatgccgttcgcacagatagctttacgacctgagttcaaagctgcaccgaaagagttcaagtcgaaagcacttcgtggcagaagcatgtacgcgatggttatgggcgttgtctactgggaagaaggtgatgcgcttgataacttccgcgagctacaggaaattgacgacgacccgtatctgacgttgctgactaacgacaagtacgctgatcgccgtagccctgagtatcaggaactgctggaccagcgcattgcgttaaacgaacaggcgccaaagtggaacgagattattgcgaagtatggcaatacaactcgcgtactcaagcctgagcaggcagaaaagctggagcaagcaaacgacttcttccagcagcgtaaagagttcatggatgctttcgacaagttcgaaaagaaagagaaccatcacgctgcgaagcaatttgctgcggccaaagctctgtttgctgccgttgattgtggcactatcatggaccgcacaacgtacatgtcagtgtcgtccggtcttgacgatgtgaacaacattctcaccaagtggggattcactacagtcaacactgttaatagtagtttgaagaagtctatccttacttacgaccgtaaaggcgcaagtcgcgtctggtccctgtagacaacatatctgaggagatagtacaacatgtctaataataatctgggcgctgctgcatcatttggtaccgagacgcaaaagcaaatcgctaacgaacagcgccgcgctaattcgtccgagagcggtcatgtgaacaaatgcaccatcgttgttctgactgcgttgaacgcgcataaccgtttttcgtatttgagcgcggacgaacaactctgtgaaaagccgattgaaggcaaagtaatggaccgtctgccgaacctgatcgaacgcgcatctggcgcgtcgaccgaccagaacagcgcgtactacattctgcatccgaacaacggcgtaccgactcgcatcgacgagcgtatcaaagtgggtgaaggtgacgcggtcattatttcatatactgtaaataaagcagtgtcagagatgcacggcagtttgtctctcgcattgttcagtgcgggcgaaagcgaccttgcagacctggccgccgagtttggtattcacgccatctcgattgttgaagaaagcaaagctggtggttatattcaagcgctcgccgcacaggtagaagctctgaatattgtaaatatcacaagcattgatgaaactgacggcgctctcgataaagcagtaatcgactacagcgcgttgccggccaatcctgttactgtgctgtccggcgctgtgcgtactttcatcatgcaaactattagcagcgaaatcgttgctgcaattccaaataacggagaactgaacgtgaaacaacctaccaactcaacgcctgtcgatctgaacgaagacttcgacgcagaagacgaagttgttgatcagcaggacggcggtgaagacgaagctgcggtcggcacggacctgtttggctacaaggctgaaacgctgagtgtcgagcaaatgtccgaagcgctcgaagctatcgactacgatctgtctgctatggatgaagacggcatccgcgaatcgttcgaaactgagcaggccatctggctggcaaaatctgatgacgccgctgccgacgacgcggacgacgccgaagatgaagaagaggaagaagaggacgacgaagacgaagaaggcttcgacgctgttcagttcctcgcttctctgctgatggccgaagacttcgaccgcgatgcgctgaaagttctggtccgtactcaagacctgaaagtaatgaagtcggacactgttgaaactctgtctgctaaactgctggagctggtcgaaggcgcaaccgaagaagagatgtttgaactgatcaacaccttcgtcggcgcgctgcaagagcgtgaaatcgaatgcccgaacatgctggcaactatcgctgaggaagaagacagcgaagaagaagatgccgatgaagaagacggcgaagacgaagaggaagattctgaggaggaggaagatgaagactccgaagaagaaaccgaagaagaagacggtgacgaactgcaagaccagatcgaagctgttaccgacccgctcgactacttccagttcccgggcggcgctctgtctgctgaacaacgcatggctgctgttgaagctatgggcgaaaacgttgaaggtctgactatcgtgcaggtaatgaaagcgttcactcgcattcagggccagaccaacgaaatcgcggtagaagaagacgccgagctgtctaacgttgaacaactgactgcgctgctgggccagtacgacgaagcgaccgtgcagcacgttgctgaaagcctgggcatcctcgttgacgaatgcgaaaccgttgacgaaatgatcgaagcgattgcaaacggcggtaacgaagatgacttcgctgctgttgaagaaatcgcaaccaactacggtgttgacctgtccgaagttgctgacggcgaggagctggactttgttgacgctctgctggcagtgctgccgtcgttcctgaacgatgatgaagttggcgagcaggacgaagaagaagacagcgaagatgaagaagacgctgacgacgaagatgaagatgaagatgaagtcgaagctgctggtgatgccactgctgagaacgatcatctgaaattcgttaagtccgttgatacctccaatcgcgtcggcccgatgctgactgtcgatatggaccaaacgctgatcatcaacttcactctgaccgacggtgatacttacgcaccgattgaaagcgaactgtctgacattaacggcttcaactaccgctacccgttcaacctgggcaaagctggtaaagcaccgggcgcgatgcacctgccggcgcagtctctgctggatatcattgagcgcaccagcaccacgcgcttcatggctaacccggcaacgttcgatgttgcagcctgggcggaaagccttgaagcaactctggaagatgaaatcgcatcctctctgtatgccggtcgcatcgaagaaggtctggaccctaccgaagccggtctgattgtcggtgacttcatcgacgacgaagaaatgcagcaggcaagcgaactcggttacatcgacgctgaccagttcgacgagctgcaaggtgatcatctgccgattgctggtctgtacagtgctaagtctcgcgttcgtccggtgcaggttgatactgctcacgtcgcgctgcacaccactgtgatgaacgtcgctgttcctggcttctggggcgactctgatgtttctctgctggtgcaggctgctgttaaccgcgttatcgctctggccggtactgttgaaaacatccgtgtgtacgctggcttcacgttcgaatctgccgcactgctgaacaacgaccgcctgtttgctgcgctgaccgctctgcgcaccatggaaggcgtacagtcttactctgctgctgacgctgcaaacttcgacgatgccgaagacgtaatcgaagtagcaagtgcgctggacacccgcgacctgccgctgtctattctgtctggtggtctggctgctgcaacgttcgataacggcggtgacctgactgtgctggtacagtgttctccggaagacgaagagtccgaagaagaagacgaaggcgacgacgagtaatatcgtctgattgagtggctcgaaagggccactcgcttttcttggggatctgtaaacatgacacaagaagtagaccacggagctaacatcgtccggatgattggtgagcgtgacgaaaaaatccatacgcttactagcgagcttgcagaagccgtaggtgataagaaagacgtggaacacgttttagaggatgaggttcacaacaacacagtgttgcgtgtcgcccttcaacgtaaggttcgccaacacgccactgaaatcgctctgcgtgatgaacgcattcgtgaagttactggattctgcaacgagcagaccgaagaagttcgcgctctgaaagctgaactcgaatctgtaaagagtaagcaagaagcggcaaacccgctgccttttgctctgcatatgataatgtgtgctggcatcaaccactactacacaatcgttatgcaactcgcacacggtactgtaaatcgtgaaacgaatcgggtagcgcgagaccttgccgagcagaacaagttggacacggtaggtaaacagccttcgctgtaccgctctgttgcaatgtattgctctgctgctggcactgacgtaccaacgggtgcaacgttgcgtgaatcgcttaaagctcacatcgaagcaaatattgacctgttcttgaaagacccgcaattcgaaatctctcgctcaatgttacgccttgtgtgggaagcgaataagaaagcggctcatatgggtttcggtgcgaataacatctgccgctcattcaactggatgcctgccgcagaagttggcagtcttgaaacactggatgatgaagacgactacgaagaattgttctgcgagtcgcttcaaacaatttgtttcgatttgattaatcatagcttttaataatctgtaaaagttacctgtaatcgaaactgtaaacactaattgaagttcgaaccgagcgacaagctcacatttataaataccggagcattacaatggctaaagcatcaaagaccacctcactggcacctaccctggcttctcgcatcgctaaaaaatctggttctatcagcacttctaaagttaagccaactgacctgccgcatgacattctgatcgaagctgttcaggctgttgagctgattggctttatcaccgaccgcaccgataacagcgtaaccattcgtcacaaacgtggtcacggttcttctgctcagatcgtttctaccttcggcccgaaccagttgctgtctgtgctgggcgaagctggttctcacggtagcgtagttgctcaaatcaacgcgccggttcgtgagtacaaaggcttcaacgttaaatatgtcggcccgatgattcacgcgacctctgttgaaacaggcgaagtggttcacatcaacaccgcactgccgggcttcaccgttcgcgcaactgtaaacgaaaacgcggctgctaaaaagtatggcatcgctgctccggccaaagccaagaaagcggacaaaggcgacaagtctgcgaaagtggctaagaaagtaaaaaagtaataaagtctgacgaagacttttaactgactttctgaaatctgtaaacattaagtatgcagcgagataaaatgttctcgctgcctgtatctcgaatctgtaaatcttaattgaagcaacatcgcttctactcaaacaggaaaaacaaatcatggctaaagctgctaaagcaaccgtaaacaccgcatctctggttctggctaaaatgctgggtgttgtagtggaaaacgcgactgataaagaaatcgctgcgctgctcgcatctgccggtctgaccgtgtctggtggcaaagttgttaaagctgacaagggcggtaaagctgctaaaggcaaaaaggccaaagcacctaccgtcgctgaaatcgtcgctgctgtgaaggacgaagaagaactggacatctccggcgtcgatgaagacactctgcgcgaagcagttgtcaaagccaagctgtctaccgctaagaaagctaaagcgctggacgaagacgacctgcgcgatctgctgaacgaaaagctgggcggcgagtccgatgaggacgaagacgaagaagaggacgacgaagacgaggacgaagagtccgacgacgaagatgaagacggcgacgacgaagacgacgaagacgaggactctgatgatgaagaagaggacgaagacgacgaagacgaagacggcgacgatgaagacgaagaggacgacgaagacgaggaagacgaagacgaagacgaggatgaagacctcgacctcgactccctcgacgaagacgaactccgcgcgctggtaatcgagcacaagctggcgactgccaagaaagcgaaaaagatggacgaagatgaactgcgcgaactctgcgaagaacacttcggcggtgaagacgacgaagacgaagaagaagacgaagacgacgaagacttcgacgatgaagacgaagacgaagacgacgagtaataacttctgatccggcgcgcccctctagttctgctgaatgagcgaggggcaaatattcgataaaacttttcgaatatttttgtaaaaagtttcaaaaatccttgtagacctatgttgaatataataatgtacgtctacagggaaacaaacctgaacaaatttatctttcatccagcggtgaaaaacgccgcatcaaatataaagtaaggatatcgtatgtctaagaaaatcatcagcggcctgaacaaagaaatcaaagccctggacaaatctgaaaaagctctggttaaaactgctgccggtctgaacaaagaagccgaagcgattgctgcacgtcgcgaaggcctggctgctcaggttgaagcactggcgagcggcggtgacgctaagccggcgaaagctgctaaagcgaccaaagctgaaaaagctgctaagcctgctaaagcagaaaaagctggtaagaaagcgaaagctgaaaagccagccaaagctgaaaaagctggtaagaaagccaaagcagaaaaacctgctaaagctgagaaagccgcgaaagctgaaaagcctgctaaggcagacaaaaaagctaaagctgaaaagccggccaaagccgacaagaaagctaaagctgaaaaagctgctaagcctgccaaagctgaaaaagctggcaaaaaagtaaaagctgaaaagccggccaaagctgataaaaaagctaaaggcgcgaaagcgaagaagcaggaagaagacttcgacttcgaaatggaataagcaagtaatcgcgcactagcggtcacttgattgaaagggcagcgctgacgagcgtttgcccttttgttgtatctgtatcaatttttgaggtatttgccatgtctgctgaacatctgcttaacgacgacctacctgacgatactcgcccactgaaacccactcctgattctgccaagccttcttactttgacctcgtgtctctacgcttagaggctgctggtcgtctcgcacgttctctcaaaactctcaaagacgctaacgtattcggtgatgacaataccatcgccaaagatctcatgttgaaaaaggctctggagatcgcagagaactactgggcagagatctgcatgggtctagtccctgttaaagactctagtggaatagaatcactgcgcgacaatctgcctgcgtgtgtcgaagccttccgcatcgtagtcatggaacatgctcaacgtgaagcattggagcgtgagtgtcgtaacaagattgaccacacaggtggcttcaagctcctcactcagcctcaagtgctgcacctcgaaaacaaacacgtctgcaatggagattgcgatcatggcccagaagctgtctgagcaaatcaaccgctatttcaatctcatggagaaaatccgtgagcaactgtttcgcgttatgcctgtatctgaccgctatttgtgtattgtcagtttcagcacgaaccatcaggcgatgatgtgtgatctcgttagcaaagaaagcctcatgcccgcaaagctgcttgatggtcttaccggacaagagctggtgacgtatggcagtattaagcgagctgtcgaagactgggtagctgatggtatgcaagctgacttccctctcagtcagagcgatgacgtatacgctgaatacaagagcttaacacgcgaacctgacataaactaaactctgcaaatagctggacgaaatgcgggtatataagaataatcttatgtgatataatagcgtcagacaagtagtgtctgaacttgctaatatcgagtagtctacgctactcactcaggagaataccaaaatggccaaagcgcctaaagctgccaaagttaaaaagcaaacgggtgacggttctcaagaaggcttcgtaattgccgaaggtcttgatggaatccgaatgaacccgggaatgtacttgggtcaacgcggtgccgatatggcttatcgcggagttaaagagcctgtcgataacgtttatgacgaacacatcgcgggacgtaacaaagttctggaagttgtgattgactacgacaacgacctgaacgtagtagccgacatggcgaaaggtattcctaccgacttcaagaaactgaaagacggtacgaaagaaacgatcatgaccgcagcgtttagccgtgttcacgctggtggtaagtttaacgatcaggcgtacaagacttctgctggtacacacggtgttggtgttgcggcactgaacgcagtgtccagccagttacgcgtttggtcaatgtacaaaggcagttgctcttatcagatgtggcagtgcggtgtcgccaagtcaggcaaagacccgaagaaagtcaagtctgttgataaagacgtaatgagcctgctgcgcgaaaagaaagcgagcaagtacggtacgattgttgcgtggacgctcgaccagactgttgtgtctgctgacgttatgcgcgggaagaagctaccaaagggttatcgtcacgctgcaccagaccctgctcaactcggtacatggctgcgcaatatgtcgctgcttaacccaggcttcgaagtacgcctgacgcttatcaagaaaggtaagcgcaaagagttcacgttccacaataagaaagacctagcgcacgttgtgaagacgatggtagaagaacgcgagcttggctcagtcggcaagccgtttatcttcaagaacgacaacatcaccgcagcgctgacgtggacagatcatcctgacactgacaacttcctcagtttcgttaacaccagcccgactgttgatggcggctggcatgtagtaggcttccgtgatgcgttgtttgaagcaatcaagccgtacatgaaagaaacgaaaggcaagaagaagcagaacttcaagcaggaagatttgcttatcggcctgaccggtatgttcgactggcgtatgcacggtgctcagtatacctcgcaggttaaagacaagctggcgagccgtgtcgaaaaagaagtatacgagatgctgaaagaagcgttcgtgaaatacttcaaggacaataagaaagtcgcaacgacgatcatcaaacgcgccgaagcgatgaacaagggacgcgaagaactcagtgctgtcgtgaagtctatggcggacacgaagaagaagttgaaaggcaactcgcttcctgctgacctgatctctgcgctcaagtgtaagccacatgagcgtgagcttatcgttgtagaaggtgactctgctggaggtactgcgaaacacgcacgtaaccctgactatcaggaagttatgcttgctggtggtaagccgcttaatggcctgaaagcaagtctggctgatgtactcaagcacaaagaagtgcagggcatgttagtgtctgtgggcgctgacctgaaatcgttagacccgaaagcagaagcgccaaagctgagtacaaagaacctgcgtatcggcaacctgctgttcttgatggatgctgaccctgacggcttccacatcgcaacgttgttcctaggtgttatctatcgtctgctgcctgacctgatgaaagagggtcgtgtgtggattgtcgatgcaccactgtataacgtgatgcacaagggcattcactatggcggcatgacgtttgaagaatgccgagcgaaagcaccgtctgctgtaaaagataaagaaatcgttcgcgccaaaggatggggtgaagtagagccagaagttctcgaagcgatctcattcaatccgaagactcgtcgcttgattcgcgtgaacccgttcactagcgtcgagcaagagcgtttcttccgcggtgtgctggcagaagatgcagttcatcgccgtcgtctgttgggtctggaggattaagatggacttcaatatagctaatctgtctgatggtactcagatccgttttctggacatgccgtctattcaacatacgccgatgactgccgatcagcaggctgaatatgacagactgattccgaagctgcgtgaactgtcaaaggattgtattgtgtctgcgcacactgtagttgacggccagccgcatgagcgtgtgctggtgcagatgaggcgaactattctcgctaagattaacgcgattgccaaaggggaacagtaatggcagttaagccgaagaaagttaaagtcgaaaagaaatcgactgcggtagcgaagcctgcaaaggttaagttgaagtcgaagtcgaaagctgttgctgtcgatgacctgccgaaaaagaaaaagaagaaaggcgaagtagttgagacgagcacaggtacttcactgtacccgatgctgggtcaagacgagtctctcattcgtgacgagaacctcgccgactacacacgacgcgctctcttccagtacggctcatacgttgttgaagaccgtgctatcgctgactatcgtgacggtctcaagcctgtgcatcgtgcgctactctggtcgctgtctgacttgggcttacgtccaggcggtgcgttcaagaaagctgcacgtactgttggtgatgcgttaggtaagtatcacccgcatggtgacgctgcttgttacggtgcgatggtaacgattgcaaacacagtgccgcctgctgtagcgggtcaaggtaactggggtgacccggtagcacctgccgctgcgatgcgttacaccgaagcgaaaatgagtaagttcgcgggtagcttcttgcttgaccctgactatctcgaagtaacgccgatggtggataacttctcgaacgatatgaagctgccactgtatctgcctgcgctgctgccgtacatgctgttcaacggtagtgtgcctgcgccagcatatggcgttaagtgcggtaacccatcgttcagctttacgtcggttgcgaaagtcgtgtgtgatatgcttaacggcaaagagtacacggctaagaagctcgctgagacactcaaagtcaatcatgagtatggctgtctcgatgtaagctccgacgaagattacctcgcgctgatgacgacaggcaagggtaaggtcacatacgaaccgcagatgaaggtcgacgagaagacgaagaccatcacgattcaaacgtatgtgcctggcggcatgtcgaacaacgcagcgataaccaagaagctggagaagattgcagagtggtctggtgttgtgtctgcatcgaatgccagttcgaagaagaacaaggacgcaggtccatggggcgcagcgtttgctatcaagtgtcgcggtagcgaagaccagttgtatgagattgcgaccaaggtgcagcgtgaagtaacctcgtcaatcaactacgcgttgggtgtgacagttcgccgtgctgacgcatcgaacaagtttatgtacctgtcgtatgtgaactacttcaaagcgtgggttgcatatcgcgttaagctggaagtggcgatgctcaagaacaagatggccaaagcagagaaagccttacatctgcaacaggtctacttgtgggcagtggacaacatggacaagttgctcaaagcgttgcctaaagcgctggtggcaaaagacccggacgagacgcttgcgaagctgtgtaagattcctcaggaagatgcgaaaatcatcctcgatcgtcaggtacgtaagctggccaaactggagcgcgccgggctggtggccaagattaaagaaatcaaggccgagattgccgagtataaagccggtctgaaagagccgggtaaatatgcagcaaacggtacagcggctaaagttaaagcgtatctcaagtctcccgacgacaagatgcctgtaagtctctgattaatctgtaaatacaactcagcatattcttggatgaaacgcggttgtatcagattaatcttatatgatataatggtactgttgagtagcgctacttagtgggaaataggtggtgctactcgaattataacaggagggtaaggtagcgcaacacaaaccaattcggaaactcaagggtaaaataatccgagcctaaaaggccaactctggcgaggtattctctgggagagcccctcgacctatactataatcgacccatgaaaatactaatatgcacaagcagcatttggtatttcgaagtgtcgctaggactggcaacaatggtcctcaactcttaatgaagtttggaaatccatagatgaaaaatcaggtaagcaacctcaaggctgggttagagcaagttaacacactgttgaccacgctccgttcaggaactaacttgaaacgccagcacgttgttgattcattaggtcagccttcctcaattttagctgatctgaccaaggcattaaagagtaatacctacaaatcgtaccccgatgtactgcaactgcgtgactctgtacgcgcaacttgcaccacctgcctcagcctgtcagaacaagtggccgctaaacgcatcaagccacgcgatctgatggaaaagctcggtgagattgtgaagtcgtttcaagctgacgtatcgttagctaagtcctgtttgggttatctgcctgagtctcgcaaagtcgtaacgctcgacgatgtgaagatgaatgccgacggtagcaccgatttggattcattccagaaagttgcggaagagatctacgaacaggagacgaacgacaaagctgtacgccgtgagcaacgcgaagatgctgcgactgctaaaacaagtcgtgtgctcaagcgtctcaaggacacgtatggccacaaggtcccgagaacgttcaaacacgctattcaaatagtccaacttcctgtgatggctcgattcggcacactcgctatgagtcctgaatcgctttctcgcatgggtttcaaaatcgaaactgccggtctccactcaacccccagctcagacttaggcatcatttttgaaaaccagctcctgcttttcttccgcatgtccgacgcgaagggaatggcagaagaagccgtgaaagatcacaagatgcttgatggtactctcgtagaacgcaaacgcctccagaaagaacgcaacgcagaacgccgtgacctcaagaagctcaatcagcttttggaccaggcaaagtctctgaaagctcgtcgtgcgcttcgtgaacaaatcgcagaagcacaggaaacgattgacgagatcactgcgaagctcgacgcgatggacagcaaagtgcgtgagagtaattccaaagagcgcgtatatcgccagatgaagacctctagcgatcatgcgatgttagactatcttaaccccattgtcgatatgctcaacgagaagggtagttccacgctcggtctgttcaccaccatgccgttacgcggtgtgatgaaggacagcgatgtgcattgtgcttggcttatggagaaatcagctatcaacctgttgctgcgccacactggcggtgacatgaagttgcagaactggttcctgccttggactaatggctaacaacgataaccgactgccggcggcaacgaaaggtgacttgtcacagtgtatcatttgcttgaagtttagcagatcgattcactatcaccataccgtgccccgctcactgggaggcgagctttcgcttcaaatcccaatagacggtgactgccacacaacgcttcacgcaaaagcagaagcagtggtagcgaagttagcaggtaaccgtaagcaacctatcggtacgttctgggatgacccagatgcggaacgtagggcacaaacgtggctagacattctggtagatgctatgattaacccaccggttcagcctggacagaaagaagtcctgctgccgatgattaaggttgacatggaaaccagacatgctctcgaactcttaaagcgcgacacgcctggcattactaatatgagccaagtgttgcgtctctgcattgagacaacattaaaatcaaaggggttaaaaaatggcgaatcaaaaagtacgcactctggacatcaaagcactcgtaaaaagcgaactgacctgtggtgattgccgtggtctgacgcgcgatgctctgttaccgactgctgaaaagccgtgtgctacacaaggtcagttagctgattctaagatctgcaaacactatcgttcagacagtcaatcactgactgaactgatgaccgagcacggcgatacgctggtggctcttttcaatacgttccgtaaattctctgacaaagacctgcgcgttgttgctggcatgttgctgtctgagtctaaaacacgtcgtcatggcgtgaagatgggacaagctgtatttgtgcgttaccaaggtcgtgagactcgcaactacctgaacaacttcatggcagcgcgtgtgctcgacgtagacgacgattcgattcgccttatttccgagaaaggtgacattgtgttgacgtatgcgaacaacggctttaacggtccgtccgtatatacgaagaagcaatttgctaagttgcgcactgagatgatcaaagctggtaagctgatcgaccctgagcgcgagatcaaaactgcgaagcgtaatcttccgcaagaagataacgttaacttctctgcaccaagttcacttgatggcttcactgttccgctgatggaagatgtgactaaaggtcgtggtggtaagcgtaagggccgtaagactcaaacgctggtggacattgtgtctatgattgagaacggtcatgacatgggcgcagagcaagacgagtctggtgtaatgagcctcggcggtaactcctacaagtcgaaacagaagaagaagattcgtgtcggtaagaacggcgctatcgaactcggcgacctgtaattaagatctagcaccaagcaataacttcaaactatacgaacaggatctcggaaaacatgatcacagaagaattaggtcttaatgcttatctggcacagcgtctgggaattgaggaaacctcagaagcgttccaacgagtatacgctgcgacaattcggtatatcggcagcgggtataaatctattgcgggttatcaccgcgacttgcaggcagcaatcgactttaagcagtacgagtttactgcaccggacttgcgtattgagctatcttctatttgtcgtttcacgttgaagatgcgtttctttgtgttggctgtttgtctgcacaagaacccgaaagaaacagttttgaagtacgctgcgtatggactgtctaagcgcgaagccgtgttagcatggaacttagtgctgaaagacgaaacgaagcgtacacagattcgtcgttgtgcgaaagcgcgggcgaagtccaaaggtggtctggatatcactatggtcagtagcaatgaattgcgccttcgtctcgatcagtcggccagcctgttcggtgagattcaccgcagtgcgaagcgtctggtcagaaagaaattgcagtgggtgtcagttagccataacattcctatcgcagaccttacttgcgatattatgtgcaaggtattactgtcgtactatcagtctctgccaaatcgttttagcgagggccaccagcttaactatcttcgtgcatcactgacgaaccgcattaacaacatgaacaactactacggtgctgagaagcgcaagcgtatgaagaaagttggcgaagacaagtatgagatcgtagtcatgtctgataatcagatgtggcacaatccagaagacgactcgtccaactcatacgaagatatgttgggtgagggtgctcgcgtacacaccgagcagatggagaatactctgaccatcaatcgtctgctggaagattcagagggaacgaaacgccacaaactgtatcagacagtgcttggccgggattgcgccgagttcactgactatctacgtgagaacgggatgctcaaacagaccatgacgtgcgccacacaatggctcatggctaagcccacaaagttcatacgcaagacgctggccaagtggttagacgttagcgttgatgcggtgtcgggtggtctggaaacattacgtggttcattacaggtagcatgagaggtcaccatatagttatgcaagcagcaatcattaacactgacgtagagcgttgtgctctcgccctgttcactcgcccgcagctggacgaggactataagcgtaccgtgttgtatctcgtgtataagactgtaaatcgtaatggcatgatgcaagttaatcgtctggtgttcgaactgacccagaagtatggactgaacaaagaggacgtgaagtctgctatcggcgcgctcaaagctccgtcggcattcaactcgctttcagtgttcgtgcctcgtgcagatttgaaggctaaccgtgtatgtcgagtgaactcgaatgcagccattgaaaactggattgcagaagtagagacgactcggcctcatatcactcgcttgttgcagtaggggcgtaa

SEQ ID NO: 3 - DNA, 261095 bp, unidentified
  source 1..261095: mol_type = genomic DNA
atgttttcgcttggcctggaagttcgggccattcgaactattacgaacccaaagattaaggaaggattcaggacggctatgatgggtcgtcttggtcctgcccactttagttcggaagtaactcgcaagtcattccgccgtattacaaagctggtggagtcacgtagcgaaataattgattgggaagacttgctggaagaccctaacttgacggaagagttcagggacagtctgcgtgaagcagaagaaaagccagcgaagaccatgaaaggctttgacaagatattcgatagtctggagaagtatcgccagcgtcgtgatatcatgaacctcggtaagcagattgctaaggactttagtgacgctgacccagaggagttcgacgaacaaacgtacatgcaagagctggctgataagctgggtcaagcgcagcgtggcacccgtaagactgagaaggtttggtcattcggtggcaagaagtcgaacgccatgaagttagcgaagcaggtaatcactaacccgaaagaggtgatgtacaagactggcttcaagacgtatgacaataagaacggcggttggcctacgaccggtgttgtgttgttagctggttcaacgtctggtggtaagtctgttatctcaatgaacctagctgatgcaatggcgaaagtgaacggcattcactgtctcaaggtcacactcgaaatgaccgccgagcaggaaatgaagcgtatgctttcgatgatcagcggcatcgacttctggaagattaagcagggcaagttgtcgaaacgcgagcagacgcagttgctgaaagccgcgaaagactacgacaagatcatgaagaagtcgaagggacgtaactcattcacgtctcctgagcgcggtatgtcgattgatgatgttttgtgtatgtcgattccatatggcgttcacgtaaccttcatcgactacgttggtctgttggaaggtatcgacaacgacaaccagtggcgcgaactgtctacgattgttcgtaaagcgaaagtacatgcgaacgcaacaggtcagcttgttgttatcctgtgtcagcttgatgaccagaccggacgtattcgttactctggtggtatgcgtgagcacgccgacgttgtgtgggcctggaactactctgaccctgagattcgtgagggcaaagtgattcctgttcaggtaatgaaagcgcgtgatggtgagttgttcgaaatggcgttggaagatgcgttcgaaacaatgaccgtgcgtgatgctggcgccgatgctgaaataccgaagtcaggaaaggttatctcaactgacgatatggaaggtaagggagattccaagaagaaattcgggaaaggtaatttcaagaagaaagataaaattgagattaagaagtctcgtcgtggtgctgctgcatttctcgatgcgggtaacagtgatgacgatgacggcgacctgccgaagaaaaagaaaaagcgtaagtcttatgacgtagcttaggagtctctatggacgaaatccagtggctagtcttcgatgacgaggccaacctaaacatagacaaggattatgtctatcacgttcgcaccaaggagggtgcagagcattctggtatgtaccctaacggagctggctttcattgtcagaacccaggacagcctggtcgtgtagcaatgtctgacgtaacgcattatgctgtgcagatgacattcgatgaccatgcagataagttcgtattcggccgtgagtaacttcgaagggccgtacggactcgtcgagtctgaccagatgatcccacgctggtcgtaccctgttaagcatggacaggtacgtagagtcgaagcgtgggaactcgatactttgccaaataccacgcagcaagtacgcatggtaaatgacattcatgcaattcatagcacacctgtagaggattatgatgacgctctcgacctcgacgaagaagccgcaacgatctcaaaaactgagtcccgacttcttatcaagcctcgactcgatgaagtccgttcccgtaaaaacaaagaccacattggtccagagaacgtcttctccgtcaccgacgaagtgattgacggtgcgcttgatagcatcgactcttactctgaaactttccgggactatctgatgcaccatgtgtttagcccgatacttgggttcgacattgcagcaggtgaagttgaagcaatcgccaaagactgtctcaagacggacctagagattgacagcgagcttgtgccgtatatcgagcgcgtaggtcttgctaacatcatcggcgtaatgctgtctaagtctaactctgtaccggaacaagtacgtgctgacgtgctgaaagactggctgattaaagcattcgatgatgtacgtgcggagcataagtcgaaaggcaattctctgcgtgatcagattcgtcgtctgatgcacggcaatactgacctcgttgctaaaggtgctggtatcggcacgacgcgaggattctctgaatacaggaaacagatgaccgagaatggccaagcctaagaagggcccagctttcaccttacgtcctaaacgcattgcggcctttgatgcgctgctgggcgatgacgtaaaggtagaggcttctgctgacatggacttcttgtcagacaatagttcaagtgcgattaacttcttggagaagggtgaggtaaacatcgttgacttggttgagggtgcgttagagcaacgtaccatcgtgccacgcgatttgaagtttgatgacagttcaatgcccaaggcgaaaaacttccttgagtggtgtacgagtcccgacttcttaaaagccgagccgtatcttgaacaggccttgattggtctacgcttgtttggagagatttgcgttcgctgttctccagacctgcaatggcagcacactgaaaaccacgagccgcaagaaactacagccgcaatcgaggatcacttacacctgctacacaatggtgtgtgccctcattgcggcgctcgtcgttctgacatgattcgcaagaaggagatgaacttctacaacgagctggctgtgaatgccggacagcgttgtgtgattgcctcgactcctgtagtaacttctcgcggcatcatgccaatcggtcatatgatgatcggacatgacacacctggcttccacaaaccgagacgcaacttcaatgcgcacaacgggcgtgagattaagaaggtcaatcaggtgtacgtgtctgacgaaagcccgacaaaagtcgtgtctctagctaatggcatgtggcttgaagcaactcatgagcaccctgtacgcactgagcaaggcttcaagaaagtgtctaagctcaaagagggcgaccgcgttgagatcaaactcggcactaacgcgtggggcaagattcaacgaccagtatctatctatgatgccggtctttcagtccgtgaagaagcactgcgttatgttgttgatcgctctctcgcaatcggcgacaagatgcagtatgtgacagaagatgcagacgcgctacagatggtgtggtcgattcttatcaatgctggatatatgcctcaagtgttgcatgacacgcgaagctggagcgttgtatacgatcataccgcagagcctgactgccgctctgttcacattgaagtaaccgcagttgatgaaggtacagcgcaggtcacgtatgacttgcagatggaaggactgcctcagtttgtggcttccggccttgtgcatcataacagcggtaagtctgtggtagtagcgatgatctcgacctacctgacgcatagactgcttatgtcgcagtcgcctactggcatcttgagtatcgacaacactaccgttctgcacggcacgttcgttgcgctcacccagaaacaagcgtcagatacgctatggactccttacttcaactacatcatgggcagtccctggttccaagcataccatgacctgattcgtaaacacgaacggcgctatggtatcgaggtgatgaagattcgtgatacgttcgttctgtacggacacaggaacttcgttatctatccagcagggcctgatggtcgtattcttcgtggtcgaactcgcgtattggcggtgatcgatgaagtggcgtattttgacaacgacgcccaatcgaagaaaatcaaagtcagcgcaaacgcagtgtatggtgcacttgaccgttcacttgcgactgtgcgggcgaaagaacgaaggcaggtggaggctggctacgacgaggcattcacgggttacttctgcaacatcagtagcccggtacacgctcgtgataagatcaacgagttgttgcgtatgtcagtcggcagtgagaagctgttaggcattcatgctcctacgtggaagatgaaccctgacatgccacgcgattcagagttcctgcttgaagcgttcaagcgtgaccctgttggcgcagcgcgagattacggggcagaagcacctctgtctgcaaacccgttcatcacgcagcccacgtttatcgcagacgctatccgtgagaaaggccgttcgatgtgtacctatacgcatcacatcattcgacacaaagacggtgaacgccagcgttatggttctcttgtgaaagctgcttcgacaaccagagcgtcaatccttgcgatagatgcaggcttctcgaacaacagttttgcacttgtgacaggctcacgtggtgatgacggtattatcagtgttgactgtctggtggagatcgttccaaagccaggcatccccctgaactataccttaatctttgacgaactgcttatccctttatgtaaagcgcgtaacgttcgtgtaatgcttgctgaccagtggcagtcattgaagctgctgcaggatgctaaactgaaagtggattcgattgaagaatcagatcagtacagcctgaaatatcaggacatgtggactgtgaagacgatgttcgaatctactccaagtcgcatcagtctgcctcgcatgacacacgctaagacgatcatggacacgctgaaatacgacggcgacgaatatccacagtgcttcgagaacaaaccaacagagcacttgataatgcaactccagacagtgcaagatactggacgcagcgttatcaagaacacaggggcaaccgatgacctgtggcgagcaatggcactcatggtgtatgggttcgagtgcggtgagtacgacgagtatctgataaaagcgcaagaagtaacagtgaaccgtgacccaaatcgtttaggccgcgtagcacatagacttaactccggctcggctggttcgactggcagacctgcacttagtggtgggcgcgttcttggttcagctcgtactcggatgattggccgtaaataagctaatttgaatgagacagttcatacaaggaatacgatcatgaccaagcattacaacccactactgtcctcgaacactgtaaagtcagagtcgagcgacacgcatcagagcacctcggccgcgttcgtagttgagagcgctaacgtgtgccctaagtgtggctctgcaaatgtgccgacacaactactctcaggcgagggtgttatgttctgcacaggctgccgcgtaagtctcgcaatccctttgaagtgaggtatatatgggcgtccaggttggtcgtcgtcaattaggcggcgcaccctcggagcctgcaaagaagaaagaaacttctctcggcgcagcctccttaccgcgcgagataggcaaagcaatccgcagtgagagttcacgtcgtcactccgacttcgtgtctcaatctgcgggtggcgcaggaatggctgccggtaatatgcagattggttccgtccctcttgatatcgacttagagccgatgatggaaggtatggactatgatgctgacgaccgacagctattcaatgtctaccgcgatatgtatcacttcgacccaatctgcggctcctatgtggacttgttctcaacgctaccattctccgatgtgagtttcagtggcgcgaaggacagtgtgcttgagccgtactacgaagtgaatgaacgtctgtcactgaccaccagcatgccgaacatcacaaccgatattcaggttactggcgcgtttgttggctcgatgatctacaacaaagaccgtaagaagtttatcgacttgatgacgcaccgttacgacaacatcgacgtaacgccactgccgtttatcagtcaggaccctatgttcgaactgcgcatccctcagtacgtgaagtctgctttcgctaaagaaggtaaacgtattgacgcgctgaaaaaagaactcgggcctgggtttgtcgataagctcatgaacgacaccacgatggagcttgaccccatcggtacgatctacatcccgcgtaaaacgttcagctttggcgaaggtatctcggtgttacgccgtgtgctgcctatctggctgattgagaagaatctctatcgcggtacgttgattgaatctggtcgtcgtcaacgcggtatcttacatgcccagttgggtgatggtgatcagtgggaaccgtcgcaagaagaaatggactttatgacagaccttcttctgtctgcggatagtgacccgattggatctatcatcacgacccgactcggcgtgaacatcagtgagttccgtcaaggcggtgacttctggaagattacggatatctgggaccagactgctcaattcaaaatgcgagcgatgggtatcagtgaagcgttcctgagtggtgaagcaaactacgactcgggtgctgctggcttgactatcttcgttgaagcgatgcgagcattccgtgatcacctgacgcgtaaagtttactacgagaaagtcttcccacttatcagcatgatgaatggcctggctgttcagcgtaacggtaagatcatcaaaaagaacaacatgatggaaggcggcatggccgaagtaatgtacaagatgaatgatggctccaagctattcattccgaacgtgcattggtccaagcaactccgtcctgatgttgatcaggcgatgatggaaaacttacgtgcgatgactgaactgggtgttccagttccgttacgtgctatcgctgctgccggcgggtacaacttcgaccagattcttatggaccaggatgaagacctcgcaatgcgtcgtaagctgatggcctatcgccgacgtcagacagagatcgatcaagagttcgctcctcctgaggccggtgctggtgatggtgacagctttagctccgttagctctatgtctgctgatttgcagcgccgtcgtcgtcatgtggccggtatcggtctgtcttctgccgtacttggtggtgagcaacgtaagctgcttaaccgtgacttcggtgagcgttctgaaatcttcgaactgtccaagacaggtaagaagaaacacgtctaccgccagtctgtcgctaactcaaaagcgaacgaccagatctggaaggctgctaagaactatgaagccaacaagacgatgcctctggatgacggtaaagtgtcgttcaagccaacgccgggtgagcttcgtgctatgtcgagacttcgttaatgtacaacgtttctacgtgtccaattgacggtactgattcggtggttgtgtatcgccaccctgtctttactgacttcggtcttgggttgaagatcaatcgtagtggtgagatgcctgttgttgagtgcaacatcgtgacaggcacaatcgacggtcagtctacgcttgagaccatcagcgatcatactgcaccgctcgaagttcaagtgtggtgctttaccgggatgctaactctgcgggaatctgtaaatatgcagagcttatcattagatgccttgttcccaaataacggaggcatcgtatactaccgaccaaatcaggagagtacatcgtgagtggattgttcccgcatcgcgttatcacgcagaaagaaggtttcgtgtttatcgtccagcctgccgacgatactgatcaggatgccgtagaagcctctcaagagattgaagcgcttctggtggaagcgtggccgactgcgccgtctgagctgtctgtgaatgacgtgcgcgacccagaagaagccgagctggtattcgctgatatcatgcaactgctggaagaagcagagcgcgaagaagcacatcagatcgtaatcagtggtatcgttgttgtcggcgaactggccgtcgtaacctgtatgctgaccggcgaagatctggaaagcgacgatgaagaagacgaagacgatgattccgttgaagttgacgaagaagaattcgattaacgtctgccatgaggaccttcgggtcctcatgaatctcactgattcgaatccagcgtatgcagccaagttcctgacgaacaaaacagaggatgaagcacgtactctgctggctgcactcaataacgatgaagtaacatcactgtacgacttaatggtgacgtgatggataataccgtggacgaaagtcctaatagcgcaaggcatcgcattttcttcaagcagccgaaacgagtacctcccttcgatacagctttcattcgttcatctaatcgtgaaggtctgaaagtcctcctatcggctgcccctgaacactgtcagatcattttgtttacggacggtcccggcatcgcttatgccatgaaacgcctctttaagcgcaacttcaaactctgttcgcaagctctacaactggatttaaaaactctgtccttaactggtcaggtcgtgtatcaattcactcgtggtggagccgtgtatgacccattggctcgctacttctgtgctggtgatagctatttgcatgagctggcgcagacaacgaagttaggaagctccgagacagatacgattgacttgttctgttgcggtctggcgttccatcgcgttttacttgagcgtggccgaggtcgttctctcgtattcgcggaggaacaatgagtagatcgtttgcgtcaattggcaagacgcctgttgctggcgctataccgaagatgaagattaagtacggcgaccagcctatgctgcatgttgttgacgcatcgaactggatgtgccgtgcttacttcgcaacccaaaagagcgcaacgtatgccaaagacggaactccgacttacggcctgcgtcaattcatgtacatggtcaaagacctgatcgatattgcagcgaaagaccctaacggtcagttcattgcattctgtttcgacgttagctccgagtctacatggcgttatcgcgctatgcagcaatgggcagcggagcataagaagaagtatatccgtcaggtgtttaaaaagagtagcgactacaagggcaaccgcgaccgttctcttaccaaagagctgggtgtgcagatggcgctggcgcgtgacatactacaactggctggctactatgtagggattaaagccccttacgagtgcgatgacattgttggtacgttgagcgaccgcttcaaatatgattacctgatcaagctgtactcgcgggataaggactacgtgcaacttgttgaccacaagaacgttgagcttatcatgcaggctcagtctaatgcagccgagcgtcgcttcacgcttaaaactgccaaaggattcttcggtgttcctgccaaccgtgttattgatatgctcgcgctatctggcgatagcgtcgataacgtacctgggattcctggcattggcgataagactgctgctgagttcatcaatcgttttggtggtgctatcgaactccgagacgcactgctatctggtgagatgaagtccaatgctggttgggcgaaagcgctgacaatgcaagcgccttcaatggatattgagctgcaaatggagcttgtaactatcgaccgtaacgttccgggcttacctcgtaagatcgaagcgtttattccaggccgtccagatataaaagcgttgaaagcagttaagaaacgcctggcactgcctcaactattacacgtctaagagggtagtatgacggacaagattacgcagttggcgaagtggtatgacgctgctaaaaccgcgtttaagatgggacagcataatcctaatggtaatgctgctctgctgttgagtatcttagctcgcctgaacaagaacgtggaagtggctgcacctggctccgaccacgacgctgctgaacaggaacgtgccgagtttctcgacgatcttgcggctgaggtcaagatgtacgaactcattcgcaagcgattcaacaacgacctgtacccaggcattaccgtgagcgaagacgtgaaggtgtatgttgcgctcatggctgatcgccctggtagcgctgtaatggcgatgaccttcctgcaccttgctcgttgctacacgctcaaggatatgatcattaactttctcccgaatggctttcctggtgaagacgcacttggtctcacctggagcatacagaagacggacgctggcaacttggtggatgatattgattctgtaaatagcctctatactaagatgtataactctggagataagtaatggatttatctgcattaggttacgcgccgaagccgtatcgagtgattcctgtcgaaaaagagaacctcgttactgactttattcaaggtaagttccgcgttattggtgttgagtgcaacgcccgcggtgtttacggcaacccaatccaaaagagtattgctcgtcgtttcccggaagtcatgaatcgcgtcaacgccgttgattacgaacatgaattaactatcggcaagacgcatctgattcgcgttcgtactcaagcccgtcgtgatttgtttgttgctaacatgcacatcgctcgcggctttggtctgggcctgaacggctcggttgagggctatcataagcctgtcaatcgtttcagtgaaaaattcctgacgcgggcgttcgaacatctgctggagcaatgcgataaagagaacatcgcaccagaccgacagattgctattcaacgcttctacggcggactcggcggagtttcttgggaagaggtttgtgttgtgcttgatgctatctgtgagaagcaccagttcaacatgtatgcctacttgccaaagaactacaatactaactacgtgcggggctccgcacaataactctggggtgtattgatgaacacaatacgcggatttgattggctcttttacggagatggaaccgatagcggccaacactcaattgtaagtatcgttgtcgaacaggcatcgaaatcaatacaggtagaagtaacgccgggatgcgccgtgcctgtaattcaagcgattcaggaaaatgatgtcctgtacgcccagaccgaagctggtctatatcgtctacgctacagttgctcgttccgaacgttggatgctaacgtcttcccgccaaacaaaacagagttccgtttgaagctcattgcgtgtgacttcttggctggtgttactactcacgataaacttctggactaagcactatgatcacagcaaagaacgttgaaagccttttggcaaaaataaactatactcggcccgacccgtcacgggaagagctggaggaacttgtaagtcacggcagaactcgtattctaaagaccgcaggcattgacggcttctgcccactgtctcgaaaatactttgagttctgcttgaagcaagttggttctttctgcgcgacttcgtacaatgcagttgaaatagcaatgtgtgtaggcattcagcctatctatgttgctgctgcgctccatctttacggtagcgactggtcatatcgtttgctcaaactgaaacgctttggtcacctcgatcgcggcattcacagtgtatgggaatccggcggtgcatggttctcgcttggtgaatgccgcagtcgcattgtaggttcgcagattgtatctcatggtcagggtaacctgaagactgcaattcgtcttggtgacatggaacagattcggcaaattgttgcgctgtacccgcaccgaaccatgagcgtactcgcacctcgcataggacttctctacactgaccagcgtcgtgaaaagagtaagcgtgaccttgaagccaagaagaaagctcttgaggcagaaggtaagaagatggccgaacagggatcgtataacgacctcagccctgtcttcaacggctcgatatctaaacctaactacggtagggtataattgtggataaaaagataatcagttttctcgtggatagcttgagtagcgacgcacgggagcctgccgaaaagtatgcaggtaagactgctggtcagattgtcaaagaagaaacaggcattgtgtttatctgcaacaacgcattcgtcatggatcgtcttctctggttgcctgacatggagcatgagtggttcacaccagtcgaagctctggttcatctgtctagcggtcttattggtcatgtaggagatgtgcctgtctatagcgattggtactacggcagcccgtccgatcgccagcgtccttgcgaccaaatccctcaagtcggtgtggtcaacgtggcaaccaatgaaatttctttgattactgttgaacaatttgctcgctaacggtaatttcgacaggtcaaaacaaataacggaacactatcatgagcaacgttgatcaaacaatgccacaaggccgctgggaatttaacgaaccagttgctgctgtcttcgataacatgttgcaaaactccattccttcgtatgaccgtatgcgtgacctgacctaccgtctgggccgtcagttcgtaactcctggcagcgctatcgttgacttaggcgcatcgctcggtcgtgcagtcgaaccgttctgtgctgagttcggcgagtacatgtaccaccacgcggcagaccgtcctgagcctgattcagaaacaggcaacatgtactgctgttacgaagtcgctccggcaatgcttgagcgtctgcgtcagaacgaagtgctgaaagcggctaaggctaaaatcagtagtgagtcgctgattgaagtggacacctttagattcgacgagcaggttgaatgctctttgattctgagtgtgctcactctccagttcactcctatcgaacatcgccagcatatcttggagaaggtgtatgactctctccagtctggaggcgctttcattctggttgagaaggtgttgggtgatgacaacttcctcgaccgtctgctggtagatacttactaccacatgaaaggcagcaacggctattcgcaagagagcattgcaactaaacgcaaatcgctcgaaggtgtactggtccctgtgaaagccgcatggaacgaagaactgttacgcaaagcaggcttcaaccgtgttgagtgtttctatcgcgatctgaacttcgctggatggattgcaattaagtaacaagtgtgggtggcttcggctgccccttgttacacaggagattagcaatggccaacaaacgccaagaacgttgtgcgtcaatgattcgtgagtcgttgattgcagagatcaaaaaagcacgttctaaacaaccatacgtcttccttagtggtggtgtagattctaactgcattctgtttgctgcgcttgaggcaggatgccgtccaattactctttccttccacatggaagggattaatagtcgtgacttccgggcggctcaggcgatagcaaaagagtttgaccttgagctgattgaggtcgtgctgccaaactcatacgagaagctcaaaagcgatgtgctgcttatggccgaacgctacaagtgtgtgcagaagaatgagttcgaatgttcatggcctatgctgtatagcttcttccgcgtccgcaatcatgcgcgtgaaaacggcatcaagaatcctgtgaccttcacgggtcaaggcgctgacttgatgtacctgtcctctaagaaggccagcatccactataaagatcgtccagatgtgtggcgcaaggaaggacgtgctaatcctcaccgcactcaggggcgcattctccctaagatggcacaagatgcaggcattcgtaatatcaagccgtgggatagcgaagaaatccttcaggcgtttctcggtacgtcatgggaagacgttaacaagccacgtcagaaagaaccttctcgtatggcttttgaagattacttcaagcgcgtccgagtattcaaccatcagaacttccagcttggcgatactggtattgcagagcacttcgagaagctgttggaggattctgaaatgaatccagacctcaaatataaaagtgttgtcggcgtctacggagagctggctcgcgcataccaggacaaatcctgatgacaatgattcacatcatagacggctctgttggtggaagttacgtttattcaaagctggtggatgcaggcttcaatgctcgcatccacgcaccgccaaatccgagagttcgtgccgcatacgctacgcacccatcactttctatgggtcactcggagcaagaaattgagcgccatatcagtcaggtcttaggcacgtttcgtggtctattcctgatcagtagttacgttggttctctggttgcgaacaacatgattgacatgtgcggacagtcagacaacgtgattacctgtgacgacctgaactgcggttccattccagtcgttgcttcctcaatttctgtaaacgtatatctgaaacaacgcaagctggctcgcattcatcatcgtctaaagcactatgacctcgatcacgagttcgccatagcggacaaggctgttcgattcgcggcgggtgatgattacgcaaagcaggacgcaaagcaggaattgaacaatcacgcgaagttcctgtccagcccgtctttgattgtggccgcacacaaactcggtgtgaaaggcagcatgtaccataactatgcaggtctggtgaaagagtttatcgaaaatcgccagaagcagtaacgtgagggcacgatgattaatcgcttccaaatgaaaaaagttcctacgctcgaagcgtgtcagtggaacggggagaacgttgaggagatgaatgagttcctcaacggtcatggttatgtcaaaggacgttacgttgaaatcggcgtgttggataagtatcagaaaccaactatcgctaacgtgtctgtaggcaactatgcagttaagcacgaagacggttccttcgacgcaatgactgcgagtgaattgatggacaaatacgttctggctgattgagggcacaatgaatctgttttctattttaaagcagcaggtgaagaaagcgctgtccaccgaagctgcccacgagccagaagttcgtgcgatgtttgactggcgctattcagttgacgttaagggtcagatgtacatcgtaggcaagactggagcaaacacttgcttctacgttgagccaggtactgatgaacctatcgcgtgttatccagatgcgctgctggcgaagattgacgagtggggcgcaagcaagtatgtgtcttacgcaatctattttaagcgtttcgaatctcctgttttcgaaaacatcaagactctggaaaaagcgctgagaggtaagccgaagacattcaagaagggttacttcttgtgtggcctgacgccgaaaggcaagcgtgtcaaactgttccgattgcaaaaaggcttgtctggtatgcagtgggtggcagtcgaacctaaacctaaatcttaatctcacggcactgtccgtgttaggagcaagtatgattgacgacattatcgtaggtcacatttatcagtcatctaatggccatccgtacaaagtggaaggtcgtgctgaacacgggcaagacccagaagacaagtgggtgcaactccataacttgaccgatactcccttgtacgccaagggatataagtttagtgtgcgagagcctgtgttcaaggaagttttctctgtgtatacagaaggggaataccatgaacacaacgttaaggcatcatctgaaatgccgccacttcaatcctgcattctaccattgctgggttagcgaaacgcaaatgaccgtgccgttgttctcgtttgatagagcaatgcgcgggctacaggtctacacaccagacgcaccgaagcacgataagaaccctaaagcctgtcgctacttcacacgggcgttcggtggcaagcagttggtgtggggatcggaaattaaacctgaacgggtcgaccgtgttcttaactgagtcagtattcaaggcatgtgctctgcatcgtcttggactcaatgcttggtccgttcttggttcaaacgtgagcgagtacctgtaccaccagcttcgtctattgggtctgcgtttcgtctgtcttggcgataacgatagagctggtcaggagtttagtcagacgtttggactaggcgctgtcagtaatgaccttgacgagatgcctgatgaacagctactcgatctaactttaccattcctgaggaagtagaaatgtcacgagaagttattgtccgtatcttaggacctgttggtgttggcaagtcggctgtgtacgcgactttggttaatgctctgtctcaaatcggtgttagcgttaaacacgcaaacgagaaagtgtggaagtctttggagaacgctggtgaagttgcgatctctactgagactcttaacgaactcactcctgttgtgacgttcgaagaagttggtattcgtaccgacgctgctgcttctccaaatcagatcatgcagtatttcgcatacgctcacctgccgccacatctgcaagcggtaagcaagccgttcgcgttgctggcccaggagatggaccagaacctgccaaacggtcctgaaaagtctactggtctgcgcaagttgcttgaagcgaaagactgcatggtacgtcaactcgtagctaagtaatggaggctatcatgagcgattggttctacggcggttaatgtgcagtaactcaaagggtggccattaggctgcccttttctgatcttagacaactaaaataagcccaaaaggaccatgcagaaccgtgcgtaaacagtatagaaccatgtgtaggcagcgcagaaacaccaccttttttctaagcagcatcaagcgcttgaaatctgtaaataaacatcagataccaataatgccccttgagaaggataaaaatgagacctgataccatagctcgcacatatagggttccaagcaagacgcttgaactggcccacaacatctgcggacgccaaggcatcaagctgtctgacattgttcgtcggtacgcccagcacgttgtgagaactcgtggggagtttctgcgtactgctgtgcggcacgaaacgtcccagcttaacgtgcgtatgccctttgacgtagcgcactcgtttggcactgtgtgtcgtaatgcgggttcgggttcaagtaacgccatgtgtgatctcctgaatgagatcatccaacttgatcgtatcccagaggaacttctgcaagagacagaggaagatgtgcgggaatatatccgtactgaacgtgagcgccttgctacgttagaggctcaactcggaaaaatctaatgacggtaataagcccaatccgatatcagggtaataagcgtagcctaatccctattattcttgaaaatacaccacccgtaaaagactgtcctcgtatggtcgatatgtttggcggaagcgctactgtctgcgcgaacatgcctcagaagtttcgcgtttacaacgagcttagtcctcaggtgtatgagatcgtcaagatgctggtcgagcaggacccgaagaaaactttgggacaagtcaagcgactggtacgccattggtgtctgacgaacagcaacgaagaaaactacgatgcgttccgtacagtagttcagaagaagcgcactgcaatcctgcactacgttgcacaccgacacgcacactcgaatatgttgcgcttcaaccaacagggcgtgtataacgtgggctttggtgatcgtggtctgattggtaagttcgatgaactcgaacacgaactcacatctttccatcagcacatgcagggcgtccacctgacgaacatgaagtacggcaagctgctaagtaagctcggcaatcaactggactgcaatacgttctgttacttcgacccgccatatctggcgagtggtgcaatgcagtacggtaagtggaccgaagccaacgagcgcaatctgctggcgacgcttgagcaactcaatcgcttgggcgtaccgtggatgttgagcaacgttatcgagcatcgagagttctcgaacgatctgctaaagcgttggttaaagaaacacgcgacgaccgtgctctacccaaacaaaagctatgcgatgaacaacggccagagtggttcgcatagtacaattgaaattctggcgatgaactattgaggtaatcatggaaccaccagtcggaacgaatatgaagttgtggcgcattcttggttgcgtcgttcgtgaactcgaaagcattaattctcaagcgtggtatttgtcccaggacccgaaagatacctgcggctcaattggctacgctatccctgactacacggatgggactctgatcaaagagattgagatgcgtgttggccagattgaagaacgcaagcgttacatcgcaggtctgcatggaggtgagcaaggtcatcgtcgtgcctgtgacttccgtgctgatgaactctatcagaaatactgcggtaagcgcggatgaatctcgtctgctacctgttcgacaaaatcccagagtacgagaaagcgatctatgcgatggtcgctaagtaccattctgatatgggtgaatggggacagttagctccagttgctagaatggaaactgttcgccgtatcttcatcgcacgtactcggggtgcatattgtatgctgcgtcgttgcacaaacatcgagacagcgtatcgtgaaatcaaaaccctgttggccaaccctgttgctcaagagattgagttaatgtcggatgcagttatcaaccagaggtataaataaagtggaacaagaacaagatatgagtcagaaccctaagcacatcattaacggtttctctttccgtgaaggctctgcgcaactgatggcgtttgctctggacgtcgtgcgtctcggtggtaagattgaagaatctttctggaccgaccacatcgtcgagaacctcaaagagcttgacctgatggacaatctgcacatcactggaccgatcatcgatcgtggccagttcgacattttcgaatcactggagcagtgccgtaagaacgcacacgtcctgctggacgccctgatgtacagcttcgacctgatgatggaagaactgcgcaccagcttctgctccgaagagcgtgtgtctcagttcattgcgcataacaaacagaacatgttcagtcgtgacttgcgtggctacctgacgcggcctgtgcaagagtctgacctgcacctcgttcatgcttatcgtcgtcgggctttcgcactgaatgatgccgagcctgtgctgttgcacatcggtggcacggacagtcaccaatgggtctggaacggtgaatggcgagcgctgctgggtgcgtccgaagaaacacgtatgcgtcagttccagacgtggtactacaatcacgctttcaccgagcatcgcctgaaagcactcgtcaatcattacctgcactacaaattccctgagcacttcaaccgaggttaatcatgacctgtattaatgaattgcgtagtcgtctgggggccgcacttgacctagaagtgaagacggcaccgaacgccgacatagaatactatgttgactcggatggtctacctatgggcttagttaaagactggaggcctgatgtgcctgagaaaatcgttcaggtcatcgagcagtacggtctgcgtgtcgagcgtgttgttaagccaggtatccctaagccaatcgacgctgataacgttcagtgggtgtaccacgtctggtcacgtcaccctgtatatcgctcgctgtctgtcgataactttgcccgacgcgaaggccctcgtgtcgcaggtgaaacactaacgctcgccgtactgacttgggcagtcctccgtgcagagcgcatcaaagaactacgggcatgtcctgtgcagtccaagtcctacaacttcgaacgcttacaggagcgtgtgtatgtatcatccgttgggggataaagcaaccgactccgaagtacgtgcgtactaccagaagcaacatgatcgggcagaagccactatgcgagaaatctgggcgctgcgcggttggacgattcgctgggaatggcacaatggagtatgtgacgactgcgagttcctatttgatgaaacaggcaagcagatgtgcccgtaccatgacgcgattccgcagacacattcgattggccgttatattgagaagcatcgcctcaatgtgacattcacgaagaaatctgtaaaattgactaacaagcaagatcccaatccagttgaaggtaaagctgatacgctacgtcaggcatatctcaattggttacttgctcttgaaaagcagaaagctgaggagaaaacgtgcgctgcgacctgaaagaattaccactggctttagaccaagctgaacacatcatggcgagcgtgttcactctggcggcttcctccaagtctaagcgtcgtgcgacggctgcaatgttggtgcatttccataacggcttcccgatgattctaagtagtggcgtcaacgggacaatgcctggcgagagcaatgtcatggaaacccctgacttgactctttcactggacactgtaattcacgcagaagtgaattgcttggatcgtctcgaagactactcgctgtggacggacttccgtgacgtgttattctgcactgactctccgtgcccaaactgtcttgccgagcttgaagttgctggcgttaagaccgttgtgtacgcgcgtgagtatcgcctgactgatcatctggacgcatctgatatcaagatgttctgtctggacatgaagtcggttgaacatcgtatgcttcgcggcatcgaacgcatgaacgaagtgatcgcaacaacacccggcgtctaattaaggccaataactgagagactctcaacatgaaattcaagattcaaccacatcaagatatgtccatacctaccgatgcgcaagtgcagcaggttgctgatcacgaagatcgtatcttccttgattcgttgtgtgaatttgaaaacatgcaacgtcgcagcatggagcgttttgcagaaatggttgaatctaatccaaagttgaggttccaaatggaacaggctcgacgccacggccatgagcagaagtttggaagtttggacttctccaaactcgaagaccgggttatggctaatgctgtccttggccgcatgtcttcgcagcacaataacatcgaagaacgtgtttctgatacgtttgaacattcatcaggtgtcgttcgaggcatagttcaacgctatccacgcatgtccgacaatctgccgcgtgacggccgcattaaagttgacgaaataccggggaaacgtatgctgcaaactgatattcatctaggtgatatgaagacagaagaccggtcgcttgctatggctgccgttgcattcggtcttagtggtgagcagcttggcattatccctgctcctggtgacagtcagctcgttgagccggaaacgcagttgagttacatcgacgaagctccatttattccaaatcatctgcctcagcactacctgcaatctgataaaggctatacgcaggcactgggccgtgctttgcgtatagctccgaaagattcatggtcccccgaacgtcgtgatcgtgctgcgacgtctgcacctgctcgtaagaaacttcgtgcccgtacacgcgcccagaagaaagcgcgccgtaaacaacgctaaggaacaatcgtggaacctttcctgaaagaaatcaaagataacttcgcccgtgctctaggtatcgaccctaaagttctcgacgtgccagtagacgaagaggctacggcacgttggaccgaaatgctgcgtgaagatcgtcgcaagatcactgtcggccttgcgctgtgtcatctgcaaatcccagatgatattcgctacagcctggtgcatgatcatctggacacgactgatcgcttgctgcgggaggcgttcgaaaacctcgctgcccagcttgttgctgttaatagcactggcggtggcgatgaaaaacaagcggcgtctggtgcgtttcgtctagctatgctgatgaacatcctgggcttcgacaacgaaacactgaaaggtgtgcttaccgacccaagccttactcgtcaggctggtcttatcgctatgactggcctgaacgatatgggtcagaaaattcaacaactgtacgacgagagaacaaaatgagccaaccagaaaacccactcgccaaattctttgacgaagaagcattcatcccaggtttagacgaagcgcaagatcgcgtagagactatgcgtgacggtggaggtgagatcgttgaagcatccgacgagtgcgaaggcggcggctgtaagatctaactgtctaactcatggggcctcgtgccccattcttgtttcggagctgaaatgcaaacggcatatcgctgtatcagttgtaagtacgttcacgttgggaaagtcagtagttgtgactgcaacaataccaaatttgaatacacgttggtgcaaatcatcgacgtgcctgagaacgaagaacaagtacctaagttcaaagatctcaggcactcacgcgcccagcgttatgtgaacgtcaaaggtggtgtatacggtaacggcgtttacgaggtccgtaagattcgggataatggctccgtgatctggacacatctaggcaatatgcagagcggctatgacagtaccgacatgagctataagttcatcgaagacaatcgcaaagcaaactgtgtactggccgccgctggtcctgagatgctcgaagcactctatatgtgctatcagtatttcaatctgaaacgtgaagtgcaaggcagttcagtcaagaatgatagccgcatttccgtgatcgcagaagcaatcgtacacgctactgatatcagtgtgttcgacaagcagagggaactaccaaatgattaaacgtctgaaagataaactggctgcattcggcctggctgtacacaatcgtcgtcaggagaatcgtaaacgccttgctgcgctacgtgcaattcaggacaatgcaattcacggtggccaagtatggaagtcgaacgagaacaacgctgaatatcaagtgctgttcctgactaacctgtatactgacggttcgattcaggtagtatactctcggcactgggcatacatatcctctatgcctctggaagacttctttgacaagttcaagcatgttaaagagattgataactcattgccaccagcgtctgacgatctcatggctatggcaaccaacatgtttggacgtagcacagtgcgaaagcctcaagaaggtgaatactggtcgcgtgttgatcgtgtacccagtggctttgatgaacaacgcaatcctgtattcatggacaataaagccacgattcaggttcgctctatcgtccatcaaactccgtctcagccgtttgtgttgtacaaagagaacggagaagacctagtgctgaacatgcaccaattcttaaatcgctacagtccggagcctgaataaaatgttgattgattttctgaaagcacttccagcaataatcttgtgttacatcatctggcgctggttgctgacaaagcgggacaggcgtcgtcatctggaacaagcgcagtcacactacaactgtggtcgccttgatagtggtaacgtctggattcatttgaagacagggcgttcttataccgtgctgtatctgactaacacgggtgtgaataaatccaactggcgcaatgactgggagatcaatgttgtatacaccaacgatttcgagcaagtctggaacaggccgtttagtgagttctgccataagttcgcgcacgtcagtcgcggaggcaatgaagaagacttctctacggttctgatgggtatgcagatggaggcaaacacgcgcattcttattccgcacgaaggtgagatgtggttcgaaggcactgtccatgctactcctcctgaactggttgctcgtggacatgcacctcaggttgtgtctcagcgccgtgctcgaatcgacatggtgctgggtgtaggagaagcgcaccctgttgtcgtatatactgtaaatgaaaagcagacagcgatgttactttcgcagttcatcttcatcttccgaaaagaggtttctttcgatgggacagtcagctcttgtatttaagtatgtgatgttcgtccgtacgcgtaacaaagaacgtgacgacggcgtccacatgccagtcatcttccctactcatatcatgcactctgatatgggcgaagcgatgataggctacgcaattcagaacggtatgatcgaaaacaaatactatcagcgcatggacccggtcagtgctggctttatcgatctgtctgacctgcgctgttttggcgagtccgaatctctggagctcaaatcccgtgaacaggacagcgagatcattcgtgcgtacatgaagactcagggcaagggggcagagacaccgccaggagacgacaagtgaaagacttactgctgtctatctggaactcaccgttctggaacgaacctgttagcgcgttcgttgtgccagtgtgcgtcatctcgtacttcttgatcgaacattatctggagaaacgtgcgctgcgtctgtctcgtgctgtgtttgcgtctggctggaatcctgttaagggcaccgagtatcgtcatcgctttctgccttggcgtacatgccgtatgtgctacacgtcaaacagcccgaatgataagttcatgccgtctgtcgtgattgatgttgagcgtggtggtatcgtagagctgccagcacacgtcttccgttttcgctatagagagattgaaaatgccaactccagtgattctactcaagcagcagactcgtgatctgctgttgaagatgttcggtcagaacaagccgttcatcgtcgtgcgtcgtgatgccattgttgaagaaggaaaatcattcggagatcgtgtgtacttctccaacggtaccaacactgttactgtgccaaacattcagggccttgacctgggtgataagctctacgtcgcagaagacggtgacgtgtatgagtggcatcctcatttcgagcgtccgtacgaagctgtgtcaaacaatcagaccgaagcgctcgcgtttggtcttcatcccattatcttccatactgacagtcggaatatctaatgtcacaacctcttgatttacgcaatcccaatcactacgaactgtactccctgcactgtgttgacgagcagtacgtcaacctgtgtgacgcgattctcgcaactggtacgcaggagtcagacccaggtcgctctgacgatacgtggacaactctgattggtgttggcttccagttgcagaacacgcacatcgccttccccgcactactcagcgcacgtaagaactggtcggcggccgtcgatgaatcatgctggatgatgcgcggcgaaacgaacatcgaatcccttaactccaaaatctgggacgagtgggcagacgaatcgggcgagtgcggtccaatctacggtgagcagtggcgtcgttggcctgatatcaaagcgttccatgacttcactaagccgtctggtgtttgtccttctgccgatgctattcgtgcgcgtgacgaaatcttgcgtatgcgtgaagacggttacatcgaaacgcaaatggctgatgggcgcattctgtttgaaggtgaaatcgaccagttcgctaacgcactgcgtcaggttcaggcgcgctctcgctctcgtcgtattcgtgtgcaggggttcaatccaggctacgtgaacatgcaaggtctgcctccgtgtcataccgagtttgagttcaacgtaacgaagtccactcgttacgaacaggctcaggccgaagcacgtggtgtagctgtgtcagaagacagcctgcacatcactgtgacaatgcgcagtaacgactgcctgctcgggcgtcccttcaatatcatcggctacagtgccatgcaccagatgatcgcgaagtgggcaggtctgaatgttggtggattcacgctgaacactaccaacacgcatctgtacgatcatcaccgcgacgcgtatcagacgcaacgcgctcagtggatgctgttgcgtgagcgtatgcagaagactggtgagcctgttaaataccctgttctggaaatcagcaacgacattctcggtctgacgccagaacagttacttgataacgcaaacgtagactggttcgagctggtggactacagcccgcagcctgcggtcaaaggacgtgtaaccaaatgaaaaacttcatgctgattgagcgtgtcagctcttacctgtatctgggctttgcagaaaacatccctgacattcctcgtcgcggtgttgagaagttcgaagtgctaattcctgacggccgtgatggcgagaatgaccctattctccaaatgactgcgcgttgtatctatcatctgccgcataactgcttcctgatcagcattgcagaaggtaccgaaggacacgagtaccctacgctgatgaagtctcactgcaagtacaacatggaactgttcctgcgttctggccatgggcgtgagaagatcgcagttaagcagattctggatgaattgcatgatgcagaagtgcagcatcctcaatggccagaagaggcgattcatgctgcgtcaatcgtcacggaagaggcaggtgagctgctgcgtgactgtgctaccttcgaagaaaacggtgaccagcgtctgattgtcaacatgctcggtgaagccacgcaggtcggcgcaatggcagttcgctttatgaagaacttgcctacttcccaacgtcgtactatccctaacaatgcgctacgctcaatcctggactctgacatgaccccagagcaacaactgattgaagtgcgtcgcctgatgaatgacggagtccagtaatgcgtttactctcatacggagcttgtggcggtacaccatttcgtcgtctggtagttaaagacgacggtcagttcgaagtcggcgttcatcctaaaattgaagcgttcggctgtgtgttcactaacgttaacgtcggacgtattgctgacgatgccgttgagttcgatctaccggacgcgggcgactggtccatcaacatggcagattacttcctgtcgcctgagtacaagcagtgggttggtgggcatacgccacgtatcgaaactatgctggacgcccacgtcatcaaaggcaagctgcctacgctggtgcaggacttcgatgcgttctatgctgacctccagcagaagatcaatgcactcaatctgactgacattgtgtttgaacacaacacgattaagcagacgaacctcaatcagaagttcgatgtgtggatgctgtacaagtacaacttgatgcttgacggcaagatctctgttactcgttcgaacgtcggcgagctggtcttccaggaagacttcatctcagcgaaaggcacaacgtggtggctgcgtgagcataacaaaactctgatggaactggcccgcaggcacgacatgttggctgcgttcattacgttcggtacgtcccaccgaaatgagcgtgagttcttctactcgtttgtcacacaggaaggtgatacgtcacatcgtcctgttgacccggcagagttcctccatctgtccgtgcatggtcagttcccagagctggatatcaaggatgaaggcgaagggtatcgtctgactgtcaactacggtcaatacttcccgcaagcgtatcacgatctccaaaaagctgtgaacatcactatcggtagtaactacgcactgaacctcttgcgctttatctgacggccagagtctctcagtaatttatgtttcaacaagggagactcgccatgcaatacgataagacgaaagactatcaaccgttccgctatctaggaacaccaaaactgcctagcgtaggattcatcgccagcactgtcacactcgtcgaaaatgaagtattgatcggcaacgacgagtgtgagttcgtgtttactgtggagcagatgaatactatggacaggggtaccatgacgtttcgtgctaaagacatgggcggtggtatcacgataaagaaatgctcagtctctggattgaaaatggtaattaagctggaacgacgcgttgtgcagttcggcaaagtacaggtcgagtggcatagcaccagccgtaaatatctttattaatctgtaaagacagagaaagagcaaccacaagagatactactaatggcaaaaattgctaaaacaaaggaagggaaaaagagcagcgcgatgaagattgacttgacgaaattcaagacagcttcgcaactgaaaggtgctgactataacccacgtttcattacagacagtcgcctgaaagcgctcgaaagttctttgggtagctttggtgacttgtctggtatcgtgtttaacaatagcgttaaaagcggtgtgctggtctctggccaccagcgtttgaaatccattgacggatggaagacacgcatcgaagtacagaagacgactgataagtacggcactatcggtctgggttacatccacgcaacgcatccgaagaagcctgaaaaggttatcagcattccgcttcgtatcgttaactggactgacaagaaaaccgagtacgctgcgaacatcgcggcgaatgctcatggcggtgagttcgacaacaagaaactcgccaagctggttgagaagctggacttgacaacaatcaagcctcagttactcggccttgacccgttagaaattcgtgggctgcaacaaaagctgaaaggtcaagccgccgttgtcactcaagaacgtgtaggtaaaactaccggccagatgaacggcagtagtggtgcgttcaaagagtacggcactgacgaagttggtgagagcctgaactgcacctgcccgcgttgtggatttaagttcgagggataatatgatcatcaagccgcctacgatgaaagaaatcaacaagctggataaaccctggcgtggtatgagtttcttcgcaggttgcggtgggtcttctaccggtcacaaaatggccggtatcaacatcctgttgagtaacgagttcgtggactctgcccgcgaatcgtatgaagcgaatcacccaacaaccaaagtgctgccccatgatattcgtcgccttgacccaagcaagctcatgcgctactgtggcttggctaaaggcgaactggatctgcttgacggtagtcctccgtgctttaccgaagacactctcattcatacagcggacggcatgaagttcatctcggatatgaatgtgggtgaccaagcaatgacctcagtcggtcgttacttccctgtgtacgacacgatggttcgtccgtacgttggcacaatgcacaagattgaaactctaatcagtgcaaacaacgcaacgcctgagcatccgttcttcatcagacgcaacactgctccgggagaatacagcgaaccgttctggtgtgatgcgaaagacgtgcaggaaggcgacttgctcggcacgccgcgaacgacacctgacatgggactcgacgtatatcagtctcaactcgaccagctgcctaagcagattgcagagtgggttgtgtttcctgagttctggtggatggttggtcactggtgtgatcgtggtacgattgagtacgttagcggtgttgaagtcgttagctttgaatcgcattcaagcctcgaaaacgctatgatcgaacaggcgtttgacgcactgaaaatcagcagcctgaatcgtatcgacacgatgacctcacagcgcaaaacgttccgtattgttatggacgcagagctgttgcagttcttacgtcgatttgtcagtcagggtaatgaccgcttctcgcgccgtctacccgcgattgtcttccatctgacacctgagttgaagcaacaattcatcttaggctgtgctggctacgactacgttaccggcatgggaacaggcctgtctatcacgtctgaaagtcgccgcttcctgattgagatgaactacctgtgctgctctgcgttcaacaggcctttgtttgatggtctgacttggggcgacgtttacttcggtagcccgatgactcctcgtgatcgcagcagctctaagccacttattggctatctgttcctgcaggacgagcacaacttcttccacgagttctctgatgccgacccgcatctttgggtcgaagtgattgagaacctagcgtaccaaactacgtgtgacgtgtacaacttctccgttgagacggacgagacatacgttgcaaacagcgtggtcgttcacaactgcaaaggcttctctactgcgggtgtgaaagaagaaggctggggcaaggaagttaaatacagcgataacaagtatcagcaggttgatgacctgttcgatcagtattgccgtatgctcgaaggcatgatgcctaaagtgttcactgcggaaaacgttagtggtatggttaaaggtgccgctaaaggttacttcatcgaagtcatgaaagagttcgaccgtcttggctattacgttcgagcacctatgttaaatgcagcgtggctcggtgttccccagtctcgtgagcgtatcatcttcatgggtgtgcgtaaagacgttgcacacgcactcggatataaatcagcgaagactgctgtgcctgatgttgtgccttgtgagagtatggcgttccttgcagatgctctgcctcacatacagcgctacaagtcaacgaagaaagatatcatcacttatcttcctgcgatgaacggtccgatgcctacgattactgctgccgatgcgattgcgtatgagactgcgcgtttctcgtctgctggctttgtcgaagataacaaaggtcatcgccgcaagttgactatagacgaactcaaagtgatctctggcatgccgtcagactacaaactgaaaggcaagttcgaggagcagtgggaacgtcttggtcgtatctgtgtgcctgctatgacacacgctgcgtctaaggctcttattgaacacatcctgattccttatgcgaagaagcgtaagaagaagccaggcgatatcttcaagtaggtgaatcatgttctggacagggcttgtattaggtatcgtgataggcgtagtggctacactcggcttcgcatggtaccacctcagaggcttttcagtatttaagccttagcgacaatctgtgtgatactctccgaagcggtcgcgatttaaaggccagaatgtttctggctaggagatatcactatgaaaaacgaaaactggtatgaagcagacgacgagcaattgaccgtagagcaaatcgaagctattcaacgaaaagcgaacgaagacgctatacggtcaggcaagcctctgcctgacgcagatgacccgtgttgggttcgtttgttctaacctaacttaacaaacaggacaaggacgtccaggagatttaaaatgtcatactgtttgattaagaatatcatggtggcgtatgtacgcaacggccaactggtttgtgcgaaagtcaaagtgaaattgagcggcgatgattctgtcgtgctctacaacacgatgcaccgtattcatcatgatacgtgcggtcgcattctgcttgagcaagaatctgatcgtgacttcctgccgacgattctctatcgtgaacgtgcggaagtgattgaaggtcagggtggtgcgttgaaacgcatcgagcagttcgccaagagcgttggcctaggctgccgggttgttgacctgttcaaagattctgtgttgagcatcggctgcctgttctacctgaaccagcctaacgctgtggtctgtcagatcattgagacagacaaggaagaactcgcgggtaagacgctgttcattggcgcagaccctgacgtggcttacgttggtgcgaatgttgttcctatgcttgtcgatgaaaacttcgacgttgacgacaagctgttgggcaacaaaatctactccctgaacgatgaccagaacaagatgttggtctcggtaggcaaataagatgatacgctacctgatcgttttcttcgctacatggattctggtagcgtactctctatcgacactggacgttccctctgagtggtgtgataggcttgcgttagttagtgccgcattcgtcacgcacttcgaaatgaaatggcaacgcttcatcaaggagcaacaatgagcaagcgtcagaaggcaattgctgtactgaaagagttctactttgaccaccagcgtggcttcattcgcttctcccgcgagaacaactacctgtcttcgttccagttccatctggacgagattcgtgaagtgaacattcatcgtgggtcgggcatcaataaagcggacggcagcctcgttacagttgctcgggtgaacatcgatctaattggtggtggtagtgctcattcatgtccgatgcaccctgaaaaagatttatcagatttgaagagccttacgtccgcattcttgctgctacgtgatgctgcgtgtggtctgccttacgctgaatacgaagcgcgtattgttgacactgagttctacatcaataagcctgtagttacctggcctgttgaaacccccgccgaataatcggcattcggtgtgcagcacaaacgtgattgcaccctctacctaaaaggtatgtactatgactaagcaacacacttcctacagctctgcgtttgctatcggtgaaatggcagtgctgtctctcgataactttgggcagaacaaagtaccttacggcgttgttgacggctgtatggcttatggcgaacaacgtatgtatcgtgtctcgctgtttgtgaacgatggtcctgctgataaccctactgcgttcttgcatcagggccgtccagtcgatggcttcattgcgtctgacctgaaagaaatcaaagagcagtacgttgatcacatcggtcatgtaggccgtttcgaatcaccacaccataagctcggcgactctgtgtttatgtctggccagctggtggaagttgatatcgacctcgaactcgatggtgagtatgacaagttcaacatccctgtgatgatcaccggcgttacttacgtcgaaggtaaagtgctgtatgaagtgagcatccaacgagcctactataatgacggtcgtgttaacggcggtcgtctggtgcgcgacacgttgagtaacatcgacagcatctacattaagcctatcggtggttggcctgagacagtccttgaagcaaaaggagaggcgactctgactgtcaagagcgatggtgctatcactattgactctgaggctgacgtgataatcacagccagcagtatcgcactcgaacctgtagtatcaggcagaacgtcgggactcgtagagaaccaaagcaacgttcctcgctctaagtaacaacttgtgggtggcttcggctgcccctttttgtatctgaatactgtaaatatctgacaggaggacagtatggaaaagaaagtagaagaattgaaacagtatgtactaaggcgtgtcaacgagaacgcaagccccgaacttaatattagccctgacgctatacagagtcatgcgcgtgatgttgttcaaggcataatgaagtcactggctgagagcgataatgggattcgtgttgtctgtgatgaatcgaataacccgcagtacaacctcgacaataacatcttgtcgttggatctgattatcaccaaaccgtcagtagttaaaatggtctttgagaaaggaaacgataatgctaaaacgtctgttggctttattcagcaagaaaccatcgtcccaaaagacgtttgaagaaaagttggagcgcttgaaaggagaatcacttgccgatgaaattcgccgcgatgatgaatcattacgtcgggcgctacaccctgggcatactccaagtgctaaaccacagctaccgcctgatagttctttcgaccgtactgctgtacttgatgctcatggcaatctgcgttacgccaaagatgcagcaaggcagaagcctgttaagcaatatgcaccaccagccaaacgtcatatgcagaaaactcgtcgcggcatgacagtcaatcaggcttcatctagtagggctcagacggatgatatgatgttggctatgatgatgcaacaaacaatcattaacacgccaagcgctctggatgatacttgccgcattacgccaagtcacggcggatacgatacaagccctagcgacggtggcagttcaaacgatggcggtggtggaggttcatgtgattaaacgtctgtgtaactggataggcttgatgcttatctctgacaagaacaagcgcaagctccgtcaacacgaagcgatgatgcgcgcctgtactgacgtatacgactggtgcggtgccgacttccctcaagcggccgaagctgttgagtatgttcgtacaatggcactcggctatgatggacgcctgaactataacaaccacatcatgagtcctcgtgagtgtcatgtaggtatcagcgattggcgagaagcaatgcgtcgtaagtatctgcgtaccgaactggactttgatggtaagacattcaaggcaccagcgggagagaaggactgaacgactaagagcgtttctgtaaactaagaacacaatcaacatataccgagaataaactatggaacgtaattcggacgatacagttgtggtgctggacgttgaagtcttcaacacgcttgtacaatacgcacattgcggtgaacgtgattgcggggaaggtttatatggaaagtccgtgaaagatattgagaaacatgcacggcattttaatcctcacttacgcgcggcctatgagcaggagctgactaacgaacgtctgggtaaagccgaacgccgtcgactgattaagaaagcacgtcgtcttagctctcagcgtgagcctgttcgtttccttgttgaccaccagcataaggttatctatccgattatcattactggtgtggcgtcagacaaccaactgcgtttgaagtatcacgcgctatcagatggctgggactctgctgcaatggtcgatcgcatcttcgaaacaccagaagagttaccgcagtcatatcgtctgttcaaggaaggggagaagacagaatgaaggcactgtctatacgccaaccgtgggcatggctgattgttaagggatacaagaagattgagaatcgcacatgggacacgaagaagcgcggtcgttttctcgttcacgccagctctaagcgtccgtcggatcacgacatgcaggtagcgaaagaaatctgtgatggcctgaacatcaagttaccggagaagcaggagttcgtgctgggctccatagttggttacgctactgtgtgcggtacagtcacgcagtcagacgatccattcttcttcgggcctgtaggcattcagttgaaagactgccgtgctgtcgagcctatacgattcaagggcgctctcagtttcttcaacacaccgttctgtgtcgtgggcggtaaggtagttcagtcaccgagatgttaagacccatactcgtacctcagttaggcaagctcgtcttagcacacctcgtcaatgaagaccgctcggatgtttacttcgtgcgtcacattactgtcagaggtgtggctatgtgtcatgtcgggcttgctcctgtcaaaagcgtaacgttcctgtacggctacacacctacacccgacgattacgaaattgtaaagcagatgcgtaaataacaacagggtggccttcgggtcgccctttctcgtttaaggattaacatgctaccgttagctccaaagaccagagtagttagtatgcgtaacggcaataaggactatgatgttcgtattgaccgagaaaccaagtggggcaacaagttctacatgaaccacgaatgtgtcgcagaacgcaatagagtgtgcgacgaacacgaagttgatttgtgggagaagatcgagaacggcgagatactgctgcgtcatttacttgaactctacggaaagcgacttggttgttggtgcagccctaagcgttgtcatggggatgcgttggtcagagccgctgaatgggcatatcagctaaactgtaaatatgagcgtatcaaagctacttacaggaaacgcagacgtgctaataaaaccagagcaaacaatatcaagaagaaagtttctcggccgtagtccttcaatgaaagccattagctgggaagtgttccagtctcaacgtggcgatggtgtgtacggtcagttccgcctagcatggggtgctgactgtattaccattcatgctctcgaccagacacgcaaagactatgagtacgagtatctggagaagctggataagatcatcgaagcactcaaaggctatgcaccagtacttggtacaaagaaccacgcatcatatcgtgaatggcttaaccctatcgagacaggcgctacaggcagtctggcatatcactatgatgtagtgtcgcctgagaacctcatattctttgaactggcctcatgtgacggtaaggtcagaatctatccccatcattttgggcgccaaccactgcgtaagatgcagagctgtttggatgccattcgtgtggagctagtcaaccacagggcgtcatttgtgctgttaatgaaagccatagaatctgtaaagaatagctatacagaacaaaacaaggtggtttgactatggctatgacccatgtgcaatacgcactgaataagctggcagaagaattgacagaggccgcccaagagtgtgccaagattgctcagtttggatttgactcctacaatcctacggacgaatcgaagaccaccaaccttgttcgtctgcttaacgaactgcatgatgttgaaggcgctaaggcattcctgaccgaagtatctcggggtgagttcgagtttgtgcctaacacgattcgcgctctgaataagacggataagatcaaacgccatctcgcaatttccatcagcatgggtcacgttgaatcgttcggagacgaagaagaagaggacgaataatgtcatacacgatgatcgttcagcacaacatcaagctgaaatctgatacacctaagcgcgtactaaacaagatacgtgagtggcacaaagcgccgtgggctttcgattaccttgaccgacacttcaaaatcaacgttgccaaagcgctcggcccgggctgcggtggtgtgtactgtaacttggagtgcaagcgcatcttcaataccggtagcggtgttgtcccgcacatccgcacaactgcgatgtttaatcgtggtaacgaaggcgcagaagtcctgcaacaattcttcgactgccttgccgattacgtcgctaacactgacgaagtgattgcggttattcgcggcgaggataatctttatgaccgtaacgaagggcgctccaacatgtttgaagcgatacctccttcatacggttactatgaagtgcgcatcgtaaacaaccacgcgaagataaaatgggttgtcaacgatctctatgaacaattaccttgggtaacctatgcttactaacattgctcgacttgtcgctacacaagcacacgaaggtcagttccgtaaattcaacggcgaaccctacatcaatcaccctgaacgtgtatcagcatggctggcgcagttcaatgttggtgagttgatcgaagctggtgctctctgccacgatgttctggaagactgcgatgtgtcgcacaacacgctgtctctgctggtggatatgcctgtcgcagatctggtgcaggaggtgactaaccgcacttaccctgaaggtacgcctcgcatcaagaagttctggggcaatatcgttaagctgattacagccagtcatcaggcgcagactctcaagtgcggtgacgcttacgataactgcaaagacgtatacgagaaagaccctgtatacggtgcgcagtacattgcagaaaagttcttcctagtctgcctgttcacccgagcacaagctgatgttaagcaagcgctgttggacctgcttaatgatatttaccataaccgcatgactgacgagcatcgaacttatgcgtgggaatatcttggacgtttagacgccgagtgccctatcgagtaccgccagctctacgaagaaacaagtcgtgaagctcgcagtctgtctcgcgcagggcttgtctttggagatcacaatggaactgcgcctgcctcagtttaaaactcgtagcgtgttagtggagcacatggaggtcaaacacaaacacgctaccgcagtagtcgatgtgaccgaaacaagctggtggggttatcgtaaacgccggttgcgtgttgcaatgaagtgcgacaaggttaatcgtaaagagcctaagtggtctgcacttgtgcgctgggacgacggctacatcgttgctccaatctgtgaggacagtgaagtcctgacgatagcaactaatacactacgcgatatgcgcaatatgaacatgacacactttgatcagttgctcgcacatcgcctttcaatccatttgaggaagcatcatggccgctctctccctgaacctgtttgaaaagattgacgacgaaaaggctttcaccgaacgccgcttccataaaagcattatgttcatgcacggcgtatcgtccaatagtccttacgccaaagacagtttgcctgtaacgttcgctgtgtatgaagtgggtgatactcgcacgtatgccgcaactgttgggcacaagctgtcggagcagttgcagtacgcaatgaatctcgaacctgtgcgtgtttggcagttggttcgtcgcggtagcaacgtttactttgttggcgagagttccgaagcgattgttgctgataacgtagtaccaatggagattcgtgtcgaaggagggcaagatgcagagcgatgctgggctacatcttgaactaacggcgaaagacgttgaagcctactggaagggacgtgtctttattgaagcggcccgcatggcgcacgacgcgcacgaagataagcaagctaacactccgacttatcctgagattgaaccgtatctcgaacaaggccgcgctgtcattgaccctattcgtgaacagcatgaaggtgagttgcctgacgccgtgtttgaagagggtgaaacactcgaacctcgtttcgtcatcatgctggcgttgatgcttgaaagcgaaaaccagcatattggcggcaagacgattaagtctatggcgtatctgtcatcggcggcccgtgataagaagatcgtgttagtgctcaacaaacacaacacggcgctgtctcggcatctggctattgagtctggctttgaggtgcgtgagtctggacttgtcgaagtggcagaagccattcgagataagatgactggcttcttcgaactggacacgccacgacctgttaaagagcctgatattaatctccgcgctgtcaggcagaagcacaatcgtgtaggccgcaattcaggtaatcagcgtttcaatgcgaagccgcagcgccagaacttcaaaggccgtggccgatgattcacgaaatgtatgcgattgggtacgtgaataatgttcctactagcgtccacgtatttcggccagagaaagacacacagcaatctgattatcgtgctctcgtcagcatggacgctttcgataagcgtatgggtcaggcatgtgctcgcgatcttacagcgaaacgcttctggttgaaacgcaagttcgaatgggaacaactggtggagagcgacaggcgtatgatgcgcctacgccattctcctatttgggttaatcttccaaagcagatacacgatgacctgtggtcgttctatcgtgcggtcggctgggactacaagagcaagcgattcatttgacaaccaaaccatctctgccgtgtgaagtaacgagcttactcacggtatcaacgcgcagcgggaagtatctcgaagtgctgaataataacatcacaccagctgggcaaagtatcagtcgtgttgtcgatgccgcccttgctcaggagactgaacatggatctgaaagactggctgataacaacggagacagtcatccataagatggttgttgatacaaaagacgggaccgccgttggtcttgtcgagactatctactatcgtcctaagcgtttgggtggtaagcgtcttcacggcaccacactgtcctgcatttgtcatgatatctaccgtcgtcatctgacgtggacggacgttaatggcatggacgagttgatgcccaaagataatcgtgcgaagtcactttgtcgtcggctgcgcacagaactgaataaactcgtagctgagggtaaaatcaatggcgagtccattatcggaaatgcaaataggcagtcctttgcctaatcacaaagacctgatatcgaagcaacttcttgaaggtcagattgagttcctgtcaggtattgctgacctgcacgaacacagtgccgtacaaatgcgtaacccgcgcagtctcggcctagacgtattgaacggtacgtgggtgtatacaccacgatatatgtatgagaatcgtcacccactctcgtatacgtttggccacatgcagcatggcggtgatgaagaaggctatgttacgctgcttaaaacgctggcgcagaaagcagagcaagagttctactacggcccgctattggctgtacgcaagttccttattcagcacgacaagattagtggtaagactgacctgctgatgcctgattcgtggtctgttgtgattgacgatgatctgaaaatgtccgacttcatgggcgtcatcgaaggctacgtgcagtccgatcagcgtcaggcgatttgcagcgcggtgtatgagcaatactatgccacgttgcgtagtcacagtgacctgtcagcaagactgatgtttagtcagaataaactgattctggtcgatgctggtgctgcgttggttggagcgggtagcctgtttgacttaacgcctatcatgcgcttcatttcgaaccctaaaggtcacggtctgacgcaagagattttccgtgcttatcgcaagctcgtaaatctgtaaatactgattgctaaagttatctgtctaatctaactatcaactatgtaaggaaaataacatggcttctgctaatggtggtgctcgcggtgcaggctctcgttctggtgttgtagataacagcgctaagtctgctaaagttactcgttccgatcgtcctatcgcggccgcatctgctgctcctgcttactctcaggtgaatacgcctatcgctgctggtagcgttgcggtctctctgtctgctcgtgctgccaatgtgggtgtagcgcaggaagacctggcggcggtattaggtcgtctcggtctgtacgaaccaactccggcaacccgagaagattttgcgtgtactgaaaacgttctcgaagtgttgacttctcaggtgaatgtcggtctacgcagtctgcaacgtatgctggaaagctccattaacggctctgattgcggcgagaaagacggcgaagaagatcaggaagaagcgacaggtaacatcgctcaaacgtcatacggacgtagcttctactacgcggccgatactgcaagcgctcaattgcgtgatgttcgtaacaagctggagcgtctgcgtacttctctgctgggtgaacgtcctactgccgatctgaaaactgcggcgcatgacagcacaggcagtctgtacgcggcagtctctgtcctgtgtgataacatggacaacaccgttaatcagattaacgaactgatcgctgaaatccgtaacacgctgctcggcgagtaatcgcggtgcctacacttaatcctgttggagaaatagtcgtgattgattttgaaaacactgttattcgtttcgacgaagaacgccgcccgtactacactgctcgtggcgctaaaggtaagttcgagcgcgtgtatctgaatgacgccgaacagcaagcgcacaaagagcacgaagtggaaaaacgtgatcgtctgaacagcgctgcggtagctcctgcttgcagcttccttaaaagtggtcccacaggccctgtcggtccgggcccatgtcctgtaggcgcaattggtgcagaaggcgttaccggcctgaacgtacctttgtctctggaagaaagcgttgcggaaactctgcctgttgctgattgcctggcgtcacgcactgtaagcctgattaactctatgagcaatctgtcgggcgctctgtacgcgttcggtgtgctggacaataatcacgtaggcaacctgatgcacctggtgctgacctacgacgagcgcaacgaacacgaagcggaagatgaaaacaacggtctggtatctgcctgcgcgttcactaatcgcattgcgtaccatatgtgggatgcgtaccgcgatgatcgttccgccagtccgatgtttgttgttgcacagcaagtaactcctgttgtgacgcttatgcaatacctgatgggtagcgcgttcccagacagtgacatggctgtacgtgcgcaacaacaaagtctgatgttccgtaagtcagatgacctacgcagtctggttgaagacttccacacagtctacaacaacattcaggctgacctgggctacatgggcgaaacgttcatcggtatcgtaccagaagagattggtggtgacactaatctaccggaagatctgtctaaaatcggtctggttcgcgctgtagacgaaatggtttcgtacttgattcgtcgtactgataacctggtcgatctgctgaatgcagaaatgtaattcgctgtagaaatgaaaaagggcggccctcaatcaagagagtcgccctttttgcgttatagtgctaaacctataccgatggctgctgcgatacgtgtcatccacagctggaagtttgctgccttttgatcttcaatgcgagccttacgctccgccaccaaatcctcagacaaaccgttagccctaacttcttctgcttgggccaaacgcagtagcttgttgcgttcatcgatcgtgaggttgagaacatcaatcagcttattgcgctcttcggtgcggtcttctcccgccttatataggttgatcaaatcaaccatacccttgttatcgagtacagccaccttcctgtcatcaatcactttgatcttaacagtcggctttgctggtaccttctcgggtgtccactcaactttgtttatctgttggatgtcctgcatggttgttttgtgttgctcgtcaatgcctgacaaagaactgcaaccagaaacgagcaacaacaggagtaacgtgattattctcatagcttattgtacctgtctaccagctcttccatgctgtcatcttcggacggtggcttaacagtctcaggcttccgctcgttcaggtccttcaccgcatcgttaacagtcttgctgtcatcgacttggttcttgattgcctgttcacgcgtattctcagcggctttctgctcacctgtcgtagtctcggacttagcgctagggcgacgaaacaacaacgccgaaacgataagcaccgcaacagatgcgaaaaccttccagtatttcttaaacaattcaatagccttagacataatcagcactcccgcttattctgcgtcttctttctttgctgccttagaagtctgcgtgttaatcaggttctcaacggtgaatgcaagagagaagtaggtcagatggtcagtctgtcctgcggtcagcataccgatgaacatgcccgtagacacaaacactgcggcgatagacgagattggatttgacgtccaatactctttccagttaaggccttcccgcttggtcttgaccacatagttcatcaagaccccgccgacatatgaaagcaagaaggctacgatttgaatcggcgcaagattcgttactacatcacccattttcaatactccgtatcgacaaaagaaagggagagccgaagccctccctatggttaaagttgatcagaggtaatctgaccatctttatacagttcgcgcttacgttctttccatgttgaagtaagctcagagaagaactctttcatgcggtcatcgtccagctcgaaaggttgattcacttcgtacttaccacacagggcgttgaacgtattcgcatattcctgctgtaggaatgatttgtccgcgcttacgctaagatattgctgcgctgacagggctaccgatacttgcatgatattatcctctatgtttgacttgcttaaattactaagcgaatttcaaaacgaggtcgttaacgataacagcttttgactggtcggtaggcgtagtgctgtttgcgtatactttacctccaatcagtttcaagtctgcatttgagttttcatcaccaacagagcacacagcaacgaaagcagcaggcacatcagtaacaccagactgaacgttgatcgtagccgctgcaccaccaagaacgatacaccaagtaggagtagcgtcttttgtgaagtagcttgcacgatagtcagaataggacgcattgatacgcatgttaaacgcagacgctaacagcacaggtacgttgttggccgcgagagtcatagccgctttgtttcctacaacgcccccaacgtagtcggcgattcgtgctgaggtcaaaagacccggacgctgatagattgcgtttccgccagtgagctgtgtaccttctccaatcagtgcctgtaactctgctttggttggcatcgttcctgtgtagaacaggatagcgcaagcgaccgtagtgaagtttgaaggtaccccagagtttacaaacgaactataggcattacgttgcatcgcatttgcagtggctggaagcattctcattacacgccctccaagaagttatccgcaatacgaatagttaggtctgggacagccatttggccgtactgaccgatgtttgtcgtaccgatagtcacgtctgtgcctacatccagcacaagaccgtaatagtcctcttgcgtctgagacagataggcctgagtactggatgggttggctaatgtcagcggcaccagcacaacatgcgtcaaggcggcagaaacaaagtcgctgcctttctctgcgtatggtgtgaagtacatgtcatttgttgttgacgtgccgttcatgctcagcctaagtttacgcgcaactatatcaagaccgtcattcatgccagccacaacagtaatgcgcgtccagacgagagtggttggatcttgatattcgaagcgaacgttacctgcattaatgcccgagacagatggaataaagaagctacggaagcgcagagttcgaccgtagtcatactcaacagcgtcggcagcactccagccgctacccacatcgttagcgatatcagaacaagcaccaaccatagccataatttgctgaggacttttgttaacattagcggccaacgtgaagcgactgtactcaggatagactgcataggtttggatattcgtcttcgtcgcagggtcgaagtaggtgcgcccctggccgtagccgccgattggcatcatactacgtccacgagagaacacgcgacagaacgtgctattcgcatcggttgtttgttgctggaacttgtactcgacggcgcagcggcttgtcgccaccaaatcaaggaatgacttgggtacgctactgctacttccgttgcgaaagaacgccatgaacccatgagtgttcgcagtcgttcccacagtctggagtagctgatacaacgctgatttttcagagactaacattaggtgtctccttagtatttgatacgcatgtctgcaagacgcagaggctggccagcgataacagtaccgccaacgattttcagatcagcattagagttctcgtcgcctacagtgcctgtaatgacaacataggcactacttccagcagcgaatcctgcaaatgtatctgccgcagaagcggccgcagtcaaacgcatcatgaaccacgtaggtgtacctgacgcagcaatggttgctaagttagcttgggcgctgaatggaagctgcatgacgttgttatccagatccatggcgacagtcataataccacacgtaacatcgcctaagaagttaagggcggaagcaaaactattaatggccgccgctgaccatgggatcgtctgaccagacgtggtaatcatagcatttaactgagcatctgtaggaggctcccctgagaacaaagcgatatgcacagcgttgactgccgtattgctgttaggtggcaatcgtggattaagtgctgtcattgccataaacgagttgtacgctttagatacgcgcatattagtatacctccagtgtaataggcggataggacactgtgaatgagttgaccgcctgttcctgtgctggatacgctgtggcgtcagttatcaacagatcgaagttcgcggcctgcttgatatcgtcagtgatagtgagtccgtaatgcgggaagaatcgtccgtagttattgacgttcattgccgcagacatagcgggcaggccataggcagtaccgaagccatgcggaaacatcactacgtgctgaactttacccagcgtacgtggggaggaacctgctacatagtcaccgtagaagtgcagagcaaacgtaccaataccgatgaagaatgggttggttgctgccgcagacttagacacaattcggaagcgacgcccttgaaccgaggccggaagctgataatacttctcaacgttacccgctgtctggaacaggttagttactaggttagttacatcaacccacgaactaccttgctgtacctgcaagaataccaagttagcaggtacgttagcgaacaggttgttattcgctgtagtctgagtaatactggtcagagcgttaataaccacatctgcgccgaagtcatactcggctaaagtccaggatccgtcagagttcttgttcttaacagttggaacagatgcccctgatgttggtgacgtacatggcatctgagttgcagaagttgttgaagcgcaacggtgccacagaatggtagcgaacaacatatccagttgcaactgagcacttgcaatcccagtatcaacaaggtcttgatacacttgactgtaggacgcgaacgttactttaggcagaacgcgttttccacggaagccctgtgcagttgtccacgcaggagcaggagaagactgcaagctggtggtgtttggaaccagagtatgttgggcattaccaatctgggtctgtaagaaggcgcgaccactgagcatgttgttcagcacagtctgcatgtcatagttcactgggttaggaagattcccttccatgaaagccccgtacatcacggtaggtgtattttgataaatcggtagaattttcatatcatgcccttggtttaaagacagttcaaattaatgaggtgacgccactacaaggacgccacccacttattacagttggtaagtcatatcaaggaagcgatatgcttggcctgtcttaatcgtacctccgatgaactggagctccgcatcagagccttgatctcctacggttcccatccacgcaggacctgcgagcaacgtaccaggagaagacgacagtacgaagttagcccatgaggctatacctgcgccaccagaagcaacgatacgagccacatagtaggtaggagtaccgtcagcaacaccagtcaatgtcgcagcattaccaccaaacggaagtgtcagtgtgcgagcacttgggttgacgataggtgtcatggcagcaaatgcaattgagcctaagaagttcgcctgtgtcaaccccaacgcggtaactgctttgacattccagcctgcaccatgggccagcgtgaagatctgattgaagtcaggcttagagcctttgaacagagcgatgtgcagcgtgttcgcaggaatcgcagtcgcaggaaatccggcgttgattgctgccagtgatgccgctttgttgctgatcatactcccctcccgataacagacgcgagttgcacacggaacgctgggacaggcacaggaccaagtgctgtgttgtacgtcgtgtccagcatattgatatcaaagttcgcagcctgtttaacatcatccgtaatagtgagatgcaccatagagcagtaacgactctgcactgtagttgttgcagctggccagttaaacgcccacgtggtgcctgcattataggaagcaagcgcttgtaaatgcagcacggtcatgtgcttgaactttccgagtgtgcgaggcttctgtcctgtgtatgttgcatagaactggatgccgaacggatagtgacctgatgtagaccaaggccacgtaacagccttgttcaccagtcggaacttctgcgctttgacttttgtaggcagttcgtatgttacagctacgttatttcctgtggtccgcaggctatcgtaggtatgaataacgtccgtccagataccattaacctgagcttgcagatacgtctgttgagtacctagtaccatctgagcggctacagttgcccctgaggaatagcctgctagggcacccagttcaatctctgcaccgaagtcatactcggcacacagataccaaccttcctgagtcaagttgtactgaggactcaagttgtttgtgatgctcgccagagggtaatctccagacaacactattcgatgcgaaagtatgcaggcggccacagcttctaagtacgtgtttactgtactggcaaaacgagcatccagcgcaggcaactttatcttaggaatgattcgcgtcttcgtggagaaagcactaccgtatccgttagctactccgtttgattcgatccacgcaggcaagaaacgaagggtatcaaacgccgatacggatacgggctgatactgccaacgggcagaaggtaaggcaaccgacgttctctggaacaggcgtaatgcaatcgcatcgttgatcgcactgtgcagagatttctcgccattttcaggagcatcagtatcgtacaaaagacctaagcaaatgttcgatgcagcgttcatgctctggaaaggatatagttccatgttagctccatacgatgttgttgagactgatagtaccgttgagcgtaaacgtaccatctccattgtctgtcagaggagcacccataccaagcaggtcttgcgcagtaagctcgatcacagaccctatagacgcagtacccgcagcgattacagtcaggttggtcccgagcataatgtacatgcggttgaatggcttagcatagctaaaacgtccaagttggttgaacaaatcgagcatacgcttaccctgacctaagttcacgatacgcacagttccgtttgagattggcgcagcatccatgacacatccaggaagatttgcagccagatatgtacgcagtgaggtcaggctgaacagagcaagcgattggttattccacaccgtgtctgtgatcgtatcaccggtagaaaacacaatagctgccgtgcgttctgcgctgattgtactgccgccaccttgtatcgtacctgcgttggctgctacagcgacgttagatgaccaaggtgcatcaatcgttgaggcaacgttagatcccaaagagtcaccacgcatattgagcatagcttttgaaatatacatcagttgctcctttgggtgaaacgcagtttaggacagtacatgacagtcttctgcgtagggataatatcgccgatgattttgtacggaccttgagcacctacagcacctgcggcatacatgatatcgtcagagtagtcaatgtcaccgtgagtgaacgtgttgcagtgtgcaagcgccgtccaagtagggacagtttgcgcagaggctggtggagtatcgacggtagacagcagtacgcgctgcgctgtggtggttgtaggcttagcgtatttgtagcgataacgttttgacgcaacaggagtagacagtgcgagacaaagggcatctcccgcgattgctgtagcagtgcccagagaggtctcggtctgaccgtcatccgacaaggcgacgagaacgaacgcatcccctgtgcttcccgtgaacttaacatgagtgacggtagttggagtgtcgaactcaaattcaacgtcactgacgaagcgcgcggccggaaccatcgtcgaacctgagcctaaaatcaacccgatgctacgatcagtaaaacctgaacgagtgatacgatgaggcataagctgataagccacagtattagcgctgccaatggtcccatagtacgatacccctttaggaatatactgagactgtaaggcaagcgttagaacgttcccagactccacaccgctaatcgggctgcggatcatactgatagacgcgttgtacaaatcagcaagtgacttgttattgaaggcagcatcgaagccttcttttgacgtaggcattttaccactaaacgcaaagatattccaaccagcaccgacattgggatcgtttatcagtgctgcattgtttgcgttcgtgcccatcattgcctgcgccatgatacggttattgataatcttcattagctcaccaccggcgcagcagatttgttgttcgctttagtgtcagacaggtcaagcgcaccaacagttacacggaagacgatattatcaaacagagggtcaatcgtctggtcagtagcgaactgtccgcttacaagagggaagtcgatacgaggtgtagccaaattcgaagtgaacgtcttcggagtaaacttacttaccacttggccaatcacattagctacgaacagcacttgatcgattgcagagacttgtctgcgctgaatccaagataccttgcttgctgtatatgccacttgagcaacgtcagcagtctggtgattaggcacagcggtgattgattccactgcccgcttctggggctgcgagtcagaactaacttcaatctgagacataacgaacacgaagtccgcgaacatgtccggatcatacgttacgactggtacgaacatggttaggctccttgacggatcgcgtagttattgatgataggagtgtatgcagcattggcacccgccgcatagccaccagtcacttgcatacctacagtgacaggcttgagcacggcatacgtgaacgtatctaccactgtaccatcaatagagattttgtgtgtagacgttgccgcatcgtattcatatttaatatgaacaacactgcctccccacatagctgagtatggagatatcgggcgaactactttaggcgtaccaccaccgccacccacgttattccacacgcatagacctttctcatttgagcggtcgaatgagatagtatagcggtcagtcagagaagcgctggaacggaacagcgtccattctgcgtaatcagcattgcctgactggtggtagtcgcactcaatcgtgaaggacttgcttgggtcaaacgtagaggacgcagccattgtcacggcgcctgtagtacctaagtcaacacccgagccgtcagcagcaaacttcaagttaccgctggtggtgcaggcattgcctgtcaggtcagtgaatgcgccggtattaaacgtacctacattgaacgcagcacgttcagtgccagtaagccacgcagcgttagcattctccacccacatttgcgtcaggctaatagtaaacgcattgattgtaacctgggtcttatatccgttcggatcatagcgaacaacaaggtcaggatagagcagcgtaacatcaggacctacctgcaagcacacaggcaagataccaccgagaatgagatgtgttggaacaccttcggcggtagcggtcaactgacagtcagagatagacagcttgttgcggtcaatagtacgaacgcagttagtgcctttcgccaacacggtacagataccactcgaagcagcaagagcagcatcgaagatatagcctgcaccagtctgagcctggaagtttaagcagcgattcaggtcagcttccacgaacccgctattcagcttaacgagatagcaggacttatcgtctgccgtagcctgagcgaataaacgcgtcaattggggaacggcagagtttgcgaataacttataattcatgttatacctcggtggacagacgaagctgggcgacagatgcgaactcaccaggaccgagtgcagtagacattaactcgattggcttaccgctaccgatcgcaccaacttcacaggcgaagtaagtaggcacatagttaccgttggccaaagcaccgtaattagtgtcctgaataactaccagcgcactacgcattgttttgtatgaagcagttcgaccaacatccgaagcagtcacaggaagaacacggcgtgtacccgacgtttgaatgaagcggaagcgcttagaagaagttgttggcgtagctagtacgttaccttcttggttagcagcaatcgcccacgcacgagcagttccaacattgcctgcgccgtcgataggagcaacagtaccggcgcaggcagaagtcatatcaccaacgtctgacagaaccgcgtcgatagtcacttcgtaatcgaacgtcaggtcagttgtggacagatgaatgcccggcgtcaggctatcatgcggaacgcctgcgtaatcccatgcgcgatatcctgcaggaccgataccccacagcgctttattgcctgcgtcattgcttgttgtgtaggcagtgttgatctgaacagacgcagcaccattgtagcctactggtcgcgctttcgctgggtaatgaatggtagcaccgttcttgatctcgtacacatgaccagaacgtgctttccatccctcctgcagatcggccagaggaacaagaccttctgtgtttgggcgcagaacgatgcgcgttgcagcaacagcgttatctgtaagattacgcagatcttgcaggtgttgagagaaatcaccctggtcagcgagtgctgtatcaaagaagaagcagttagcgacgataccgttagcagcattcgaccaccagccgctcccaagattcagtacgctgaacggaagcaagttgtgtcctaagatgcgcattagaactccttagagtctttaactacggttgctaagaatttaccgttgcgcagattggctgaggtcagaatcaagtctgcaccagaacccgcagcaccgatagtcagaataaggaagccaccatatggagtgcttgcaatatctttgttgaagacaatcacgttgtacgtgctcaacagagttgccaagtcacctgcgaatgttccttgcagtgtagctgacagacggaacttatacttgttatcttgaccatgaatccagcgcactgggttagtattggcgctagtcaagtcgagcaccgcagtcgcaccaatagcagtctgaacagtagtaccatcggcaacaacgatgttggccgggtcaggtacgtgtgcgagacaaatggtcttctgcatgtttgacaggccgtacttcaatggcggatcagacgcgggacgtttgcctgcatctggaatcgtaatgccattgacgaccaaagggaacgaaactatttccattgtgttatctccagttgactcgcagtaaattactgagaactcatagcgagtaggaagtggttgctataaagagaaacgttttggcaacacgacgggctcatacgcagtgaccgtgccactcaatatctccgtaggaagaacagggccgtgtacgaggactttctatcaggagcagcaacatccgatgaaaacagaaacatgcgctttcgtgctgtctctatattcttctccagtaactgagcaccgttcgaaacaaataacataccggctcctatagttcaatagtgtccgtgttatatatgacaggcatttctggcatagatagggagagggtcgcacccacatttgcactacgtggggagaagtcatcggcgttgtacacaacagctcgtatccctagaccctcatagataaaaattgcaaacttatcaatgctaatcgaagactctgcctgttcacttgaaccaaactgattagagcatggtgtaaacaggttggcgtccagcgcgtttcgtctggtgattgggcctgctctccagtaaccacctccgtataccatctccacataagcactcattgagaaagccatacagccaggtgcatccaacgcccagcttgacatgtttgtgcctgtgaagttatacgaccagctatgaggagttgtcagcgcttcgctgtaacctgtcgcagtgtagattcttcgtctgtgcctatacgaatctcctgtctgcctacttgcaccactcacctgaactgtggtgtcagggaacgagacttggtatgaggtaggcacagtgacattacctactttggtaggcactaagcagaacggtgatggtacccaggaaccgttgttgccgttgaaaggcgtattccctgcgaaggtatcagtcaaagacatttgagaacctttacgaccactaccacctttaattcctgttactaaaagagtccttataaagttttcgtcagatgtaaagttaggaggctctgacataatcgttagcttagagtaatacacacgagatcccgtaccgtaggcagcaatgcccataatagggtgcgtgactataacgttttcattctgagattggacagacgcccggctgtttcgtattagatctcgtagttcactcactgaactgaaatctatggcttgcccggagtcgaaaaagaatccgtacttacgcacatcatcctgtctaggaagtacgagttgcataaactttccttattacatctgggtgagagacttatctggaaatagttgtgtgctcgtcagagacaaagtggctatagacgctgttggaatagcgcccgcctgtgtgagatcttttccctgaccaatttcaccgcgcacaagatatttcaggccattcacttggaaggctgacatgtacgaagtcaggacaacatcatctgtgtttgccttgcctgtgatagcaactcgcatcggataggcttggttctcaggccgagtatatccagatacgccgttaccagactgtggggtgtacgtcgcacttgactgattcaggccgttagcagaatacctcatacccattgtgcgcacgaacactagatggtccaaagcggcgtatgtgttatgtagcgttgcctgttggtttggtgtacctgtggtctggatataagaatagccaacagggctagtctccataagcatatccaaacccaagccaccgttgttgaaacctgcatcgtagccgctgtacgttccccagaaagggtctgtgttacggctgtattgactacctgccttggagctgtatgtttgcagatgaacgtttgtgttacgcatacctgcagggaagataagcatacagttcgatggccagtagagagattccgacgtatcactcgaaggtcctgactgacctgtaaacactggagcgcccgcagcccatagactatagttagacgtgtccgatacagtaaagtatcgcgtgagtgcggcttccggtgtttgttgtgcagtgtatgacgcatagccactactactgactggagaattgcctaataggcaggcgcttcttgcaggatagaaaaagttgtctttgatgccgctcattggactcaaggtgactgcgctttctgtacctaatacagagttaccccaagccctggcacctttaacctttgagatatacttcgcagcacttacatgagcgtctgacaggtcagtctggctgtcaaagtacagagcacggtgcgtggccaatagagcgatcttgttggcctttatggggtgtggcgttgcaaagagcattatgctcctcctacagtaggtatttagacttagcattggcgtaagacataacttcgtcagagaagtttaggtcagcaatctctgctatgctgttgcctgtctgcctaacatcatttgtgcttgcatcaccgattgaaagaactatcaaacctttttcaagaggatattcgtatgcgatagcaccgaaagataaaacgcaaggaggactatctgccgttacatcctttagaggtacatacaggggttctgcaataccgcaatttgggaagtcagatagagttggcgagtaggagaaactggtatagcctccacctataggccagctttgagtctcttcctgagtcgatataaacatgacgcagggtgcagatgcagaatacatagcaggagctactacaggaagagtgttgccttgaccgtattgcttagtcgtgtctgtagtcgtgaggtttgtttgcgtctgcaacgtattagtcataggcaaatatgcaccacttgaccaatagagcgtgtactgaaagtttcgcccaagccacgagttagattcgtatttagtgatcgatagggtttgacctttgaaactcaagttggctcgaataccacctgtagcagaaacacgcatcgaggtaacaagcgtctcaggaacaaagtacatcctattgctgaacatactcgatgttgggtcataggctctacttttaccaacgccaaagaaattagacttcaaatcactcatggcaccttttgtctgtgccgtagttacggtaacatatcggtatgcttgagcatcggctgtctggttgtctctggagcttccgtagtagtaccaatccttgttgttgctattctggttgaaccccattaagtcggcagtgtgtgctatatagtgtttgttgttcttcacgccagatagggcagttgtcttcgccgtattgtcagagagtccccatgcagtaccacgacaatacggaatattcttgagcagattaactcttgactgtcggacggcagccacatctacggttgaatcaaatagaaacaatgcagacagtgcatccttgcgcatcttgccaaccttgacagcaccgactgaatgaaactgcatatacgccccttttcgactcaaaatcccagatacaaggtaaaacggcccgtaccattacgatacaggccatctaggttacaccagcaaacgtcctgcaacagtgatcgcaacaccattcagtgttgtgtccgcagtatcaggtgcgatgacacgcatctggtcaccagcaacaagaatgatctcttggtcctgatatgcaaccagaggtgcaaacacaccaactttagaccctgcggcgaaagacacagtgccaagctgaataacagcagaggtggctgagtcatacgcgcttatcttgaagacagacgcagcggtggcagcaacatcggctacagccatagagccgccgaagtttttgatgattgcagttgtacgcacagacaggtagcgagcaatctcctgtccaccagcataacgcttgagtacagacagacccacgtcatatgggtttacagactgcaactgattaacccacttgttacgcacttggctgaacacgtacaagcctggttgattctgacctgaaacagcagtcagattccacacacgaccattagctggagatgatggaaaggttgggccagaggagttcgggtcacccggagcacgaacgatttgagcctgttcacccgcgagctgtagaccataagttaacattgtttatctccttaggcgattcgcacttcgcccgtaacagcgtacgggaaagttactttgactgtattaacatccacaaagataacgtccagaggcagtacctgatggagtttaccatctggctgcatcgtacacgtagtcactgcgaccatacgtccgaagttgtgcgtaatcacccattcagcagaaggcgtttcctgtttgtaggagcgccccatcgaatagttgagcataagttcctcacaattcatatgtgtattttgacacgactgcattagacagctttgccgtgccgtttccattcatcacaggacttacttgcataaggtcggactcagcaagcagagctatatgcagcgttttcttttcatcaacgattgcagccataccccatgtaggaacagagacacctggtgtgccattcgtgatagcgtgataaagatttggtactccccaccacaacgagaagtagttgccgcctgagttgttgaagttcacgtttctgaccactacggcgtatgacatagcgttcgcctgtatggcattccctacgacgacgcgatagccattcgagttccatgaataaccatccccgctcacagaaagagcagcatcaagagatactggatagttatacatcaacatggaagtgccatacatactgctaccgacttgatcattcaacaacttgtctgacattataggctgcgtcttgtcaacaccttgagctgcaagcgaggttggacccgacgcctcgatctgcattaatgtcatacccaaagagtctgacaggtcgagagcaaactgccgttccatgtagcggtacgaaggaactgttggcgcattcacaggagctaaagaacctgttgatacgcccctgttgcttgtatacgtatggtggacagaacgtgtgtgtagccagcgccttgtaccatcagcactgataccggcagcaggattaagaggtatagttccgttgaccgcaaagtcttttgagctggtcacagacttctcggcacataacttaacgaagttgttccacgtaagagaactcatgtcaggcttagacgtagaggcctcgaataagaacagacttcgctctatcatatgcttttgtacactgcgatagttttgagcgaaaagcatatgagtgcctcttaatacagaatgacggtgcctgactcaggattatcgaatgtgatagtgagcagacttgtgctgtcatgcacgatagacttcggctggacttctttcgtgccttgcatgatacgcactgctggattgtagcccaggttgtgcgtaacagtccacacagcctcgtcagtgaatgacgcagtgaatgcaacggtaggagtaggcagaccgctttcaataccagacagcagcacagccgtaccagcaacaggctcggggaataacacgatggtagtgtttgcgtcctgagagtgaatggatgagggcataacaacgtcaccgttaccgtcgtagcactgaacgataggcgtaccagtgttcatgttgtgtgcgatttcccaacggcttgatgcagatgcctgcgagtagcggaacatcgtcatctgttgcgtcaacggtacccagataggtaggtcagcgatctcaacacagaacataaggcgcttgtccatgaagattgccatgcccggctgaggattggttggccagtcagtcacttcatcaaatttgaagttcttgatcgagccgaactctaagtctaaagtcccaacgactttcataaatcatctcctgaaaggtaaaaagggcaggcagaagcccaccctttattatgttacggctgtcgttgtcgattacgcttctggttcaacgtaagtgttggtaccagttacgaatgcgattgcaactttcttagcggtggtcagttcgacacgcaggctgtttgcgtcgatgaacacaacttcgtcagggatgatctggtagcccgtgtcatcaacaacggtaacaacaccgaacttgtggccagcgttgtgcgtgaaggtgtgcgcagtagctgcaacatcaccgcttgcagtcttatcatactgatagaccttagcagcagcaccgccagaaccggcagcgattgcatcgtccacatacttcttggtaggaacgctggtgtcggtcagcggatcggtaccggtcagagtcagcgcttcaacagaaccaccagtagcgtcgatgaaaccaccagcagttttaacagcagcaacgtcaacgatgattttgctgttatcaacatcctgtttcaggccagtgcccagagcagcagcagcaatctgaccgtagccaacaccgccgtctgcaatggcaataccatcaacagaacgagccagagtagcgccgtccagtttaacgcgagtgctaccttcgttgtcttccaggccgccgttagcgtcaagtttggcagtcacagcattgctggtgatctgaatacccgcgccgactttaacgttgacaacgttaccagctttttccagaccgtcaccagcgttgaactcagaagcgccgccgaaggtagtccactcagtaccatcgaaacgacgatactctttgatatctttaacccaggtaaccgcaccaccagcttcgctgtcagttgggtcgaacacgataacgaacgcagtgccgttatagcgaacgatcatgttgtcagccagaccagtgatagaaccgaagttcgggttgatggtatcagcagacaggatgatgtactgcttaccattttccagaacagggtccagagtgccgtcagcctgaataccatcagagtctttcagccagtcgatgccagcgatagcgttgtcgatatcgatcttacgagcagcatcgttcgggttagcaggagcggccaggttagcaacggtattaccgttagcgtcgaggtcgccagtcagttggccgttagccgcatccagctttccgcccagcgcagtttcgtttgcgttagctttgttgctgacagcagtgatctgagactggatgttagagcttgcgccggacaggtagcccagctcggaggcagtgatggtagagctttgcagttctgaatcagcaccggcgataacaactgcgttctcggtcaggccgctgatcttgtcttgcttggtagcaacaactgtctcaacgtgtttcttagaaacagccgcgttatcgccagaagcagactggtcaggaccagacagttcgaggtcagcagtcattgctactgaaccgtcagccaggaccacaccttctacagaaccaccgctaccgcccagctctttgatgacagtgccgttgaagtatttgtacttatcttcggtgctgttgtaccagatacgtgctgtctgggatgcaaccagatcgcctactacagggtcggcggtaagaacttcaggacggaagttcttaatctgggcgccgagcattaaatcaagattaccagtacgcattgtaaatctcctgttgcgtgggattagaagaaagtaccttcacagtcatctaggctacaacgtagcttttgataggctgcgattcgttcttccgtcagattgatatacttatcatcaatattgtacttcactctgattggtacatcgtacccatcgagcaggccgtgtcgcttataagcattcaggcgtagcacaggtgaactgacctgacagaactccataattgtcaggtcaatcttgtcggcgtatatgaatggtcgctctctcttacataagatgtaatcaatctcatgcaaattaaagagtgtgaaattcatatagccaattatgaactccgcaatcagcctgaatgagtcaaacatgtcaggcctaaattgttgtgtgagaatctggtcaacgtaaggtctgatctcggtacgcatctcgtaccaactctcacagaacaatgcagggaagtcttcagggtgatgggccataaggcccaacacgtctttttctgtatctgcgaaagagcttagaatgtcggcagcatcatcggatgcctcgacgcctctcccagttgaaataaaacgacgttcaatgtctctcaaccaagactctgatgcagacaggtattgaagcagtgtttctctcgcggcagccgaaaactcatgcctgtttgagtcaagaacctcaccaagcataaaggctttcgctttgtagaaatcactatagcgttcggcagtgaatcgtcgaaaccctatgttattcctcaaatagcccatcatcgcaatgccctcagatcattcaactccgtgttgccttgcgcattaggagttgtatatagagagcttgagatactctgcaatcgcaggccgagcttctcaagctcctgctggttgccacccaacttctcaaggacctctcgcattagctcgacagaaccttgatggtcacgggattgctgagagatgattcgttcgaaacgctgcatcgcgcgaagaacagagttcaatccctctttcatatccaaattatcgaccggcgcagagtcagagattgattgaatcattcgcatcatctgcgccaagtcggcttgtagctcgtcgttatctggattgccgctcataccgctttccagttctgcattacgcgccttaacttgctccagttcttcaagctgaggcagtagtttccaccaaacgtaggcaccaccgagaatcagtagaacaacagaaccgacagtcgcgtagttggacgcaagcaacttgtctaaaatttccgcccacattatattcaacccttacaggtgttatcgttcagatcaacaatgacccgttcggcacctggttcgtttacgtcagtggttttgtacgtgtgcgccatcctaggcttgaactctaagcagctttgtccgtaacgtccatcgacaacacagatggcggacaggcagctaacatcttccttgagtattaaattttcaggagcttggttggtactcctaactgccgtgattacaaagcccaccacagcgatagcaatgacaaccagaatggcaatccgaagtcgcttggcttgcatttttggttctacctcatggtcctttcatctgactgaaattagcgaaccacacgcctagcagaagatttattcctccaatacgccactaatctccgcaaacatattcttgtacactaaactcccatcgagcttgtctagcctgctaacaagcacatagagttttggagtcgtgcgcatgttagcccacgtcttttcgtttgtgtcgagtccgcccacgttcgggacaatgaccatgctaagattgttgttagcacgaacgaaaccaatatccatatgcgtcctgtttatagttctgataagcctattgattgcgtccaaaccaacaggcttgttgaattccgtatcattcacagtgttgactaagctaataagaattcccttatctctgctgttaatctcaaacaaagttgacttgagatctcctacagtcgtagcagagtagtaggacacgtcatgccctaagtccttcaggcaggaacctaacgcacgagccgactcgatgtgtgctatgttatcatcccgaagaatgtacatcggcgcatcgggctggtacgtgcgcttggtaaccatgtcgataagatcacaagaggggcgaccaacagtggccagccccctatttgcgatatagaacttatctttatatggcccgtagatattgggcggcatatacttcaagtaatcatcgtccagactaagtatcatgcgaggcttagttatctgaatgacgagttgcatggtacgaagcgaggccttgtactctgtatcggagagcactcggcttataggcaaatactgcacgacaacgaagcgttcatcaatcgaatcaactacagaacgaatcaacgtacttcccagcgtaggcccagcagagaactgggtaacaatcatcacaccgccttgaacaagacttcttgcaccagcgatagtagcaccgttacctagttgctgcgtagacgcttcccacgttaaggctggtcggtcgtctccgatatcggcatgtacataagctgcgctacaccagagacaggctccaagaaggtaagcagcaatacgttttccggatcggcctcggctggattgacagtctcgggccatagcacttctcctcttgcgtcagtgacgtaaggaatgccggcgcctttacccaatccatgacgtaaggcccatactgtatcggcattctcctgcacgaacactaaccctttgacttgcgcttcgtctgtagcagtctccagtacctcaacacgcttctcaagaagctcggcattggattgcagcacacgaatagcagccaggttagagttaacgcgctggttcatgttgttgaacatggtgaagaacgagttgttcatcgccgtgcgaacgccgtccgtataggacttaggaatcagttcatcgttatcgtaggttgttacgcctgaacgcacaagaactttaccggtaagacgtccaccacttgcgcttatgatctgaggagcaggcaaatctgcttcgtcccagacctgaacagtggtcatcaccgtattgtagtcggtctcttcctgccacgtattcttatacggtgcagtggctgctttggacttacgtcgcatgacttttttatagcctgcgttcgaaccatcagcaatgacccagagaccgttcagtggaaatacgtgagtaatcggttcggcaaacgaaagaatgatcgtaacgtccgcccctaccttgtacgcaatatcgttcgacgcagaaagcccctgctgttgtgcaagagcaatcaacgtgtccacgtagttagtcaactggctcatccgaaactcctaacgattgtaaaattgaagaacttgtatcggagaaggccttagcaatatgagaggcagcagccttatcgacaacgagagtgctgattcgcccttttgtattacacacaatagtctgaggtgagtacggtgcaagcgcaagggcgaatagcagatggttgcctagatcgccagagatagatacttctacgtccagttcaggaacgtaaatgttctggttgatttcagcaacaaactgcgccagcgccactgggtcgaattcggggagcgctgtatcgtaatcttcaacgagatcaatctgtcccgtctcagggtaataacggaaggctgctgggtcagagaggattctgccgaacagctcgtcactgacttcaatgcagtctgtgtccgtcttttctcgcacacgaccaacgatgctgttgttcgcggggttgatacgaatgataggcatcgttaatctcctactgccgtataccagaagtcccaaccgacagtgttagtgccgctggacttaatggtaaagccacccaacagggcgttctcgttcatcgcactggtaccatccaggttatacaacgtatacgtcttagcttggttggtagcggcgttaacgaacgtgatctgcaagctgatgcagcggttaatgaacggactgttgaagataacgtgcagggtatcagttgttgatttgttcacgacacgggccatgttgtgagtaaagcccgtgttcatgtttcgattactaccaacccaagcattaggtactaccgcacccgttactgggtcaagcgcttgcgacacgcgatattcatcaatcgcagcatcgcgtccaggactgcctgtaggtcctgttgcaccagtgggtcctactgcaccagtgttacctgttgcgcctacaggacccgtattaccagtaggaccgttgcgccctctagggccgcgaggacctgggcagccgtcatcaccatcacgaccatcacggccgttagtgcctgacagaccgcgcaagccttctttgccctgcttaccttcacggccagacttgagctggtcagcagtaggcaaaccgataacgtttgtctgactgccgtctggccagatgatagaaagcgtaccggtagtagtatcgaactgagcaccctgtgagcctggaatcttcgatgcttctgcagggtcgatgaatgcaaccgctgtcgaagttttcttacccagcactttaccaacggggtcagtaccgccgtcaataagtgatgggttaattcgtgttaaagacatgggtgagctcctaaccagtcagtgttgtccaatcaggttgacccgattgtccggcttctggatttttgactttcgtgttgttgactgtcatacgaatccaacgaacagttccgtctgtatcttgccaccggaccttcgtgccaccgtatgctaaattagctacccatctgtctctgctcgggtctttgaatgctaaacgtgcatatgcgggcataaattctccttactcgatttcactcggttcccagcaaaggataggtctgcgccacacttggaacacaccgatagggtcagctcggccgccatcaatgaaacagtccatggtgcgaccgccggagttgccgctctgcattaacgtctgcaagttagcaatccaagaagcacgacctccagaatcagcttcgaacaatccttcccacaccatatcgaacgcaccgttccacgcattgaagtgatgcgatgaatacgcaccatcgccaacactacaaagaaccatgtactgatagtctttcacgcatgggattctgtagttgttgccacgaggaacagtagcactgttattgttgaagatacactcccaaccagtacgatccgccgaacctgttgttaagaacagaggacgacgaataatcatcatgataccattctgaccgccgttatcgctagacttttcgcagtacgcattgcagcgtaaggcccgatcaacggtaaaagtagttgagttggagaagtctcggcagtagtagttcgaaccccacttcggcagatactctgctggtggtacgaagaaatgacgttcagcaagttcaatctcaccgtagcggtcatacgcaaatacgatgtactcaaagcctgcttcaatctggatgttgtgcccctgagtgccgacgccattccatttccagacaacttgccaatcgttcgtatcgcggtcaggcagttcagtgataagctgataaggacgctcatacacatgccacactttcccttcttctgtcgtgttgatgtacagagaactaggatcgttgatgttaccgttagacgtaccgcaataaactttatgcgatgcaccagcagagttatagatagtgcctgagccgattgaactaaacatgtcccagttcatcatcaggtgagaggtacacatttcgttctggcccgcgccatccgaagtcgtaagcagatattcgttcaagtctttgaacgcatagcgaacgtagttcgaaccagcacggttaacacgatgcacccagtcatgcgattgaaccttcggcacagggaagcatgggttagtgacagacacgacgaagtttttagtttcgtacataggcagtttcttgaagcggttatcacgaatcgttaccgtgtgcttcatgccataggtttgtccaccatccattccgcccaacactttgtagtacgactcatgcgcactcttggtgttttcgaacagaccggtaattcccaacgcaagtgtaccatcacgatctgtaccggtgcaataaggaacgttgcccgaatcgaagtcaaagcctaccgagtagtagctatcaggtgagcttgatttggggccccagtacagttctgtgtgcgctgaaccttcaccaataccaggctcgccgaacacacaatatgcagcacggtacacatactgactgccttggaacacacggcgcgaggcaccaatgcgatacatagcagcaggaagaccgccctgtacacggttaacgtcggctgtatcatacgacacaacgaagacataacagtctgtgccgattgagtttaggaacgcagcacaggcagcggcattagcaacgccagggttagtgccttccgcagatgcgtgaatatcaaacgagcggcgttcaagcagcgcaagatctgatttacgaatcttatagacgttcaggccgcgccagtccgtgtattgcgtaccgttgtagatcgtgtatcctctatcgccagtatcaaggtagtgttgatatcctactacgtgcgagaacaaacgactacgcgctgcaagtgactgcgcattctgattcgaccacgtgacagacacatccccagcagcaagacgagctgcccaatcatcaggcttgtatgggtaggtagtaacatcgaagttaacaccgtacgccgagccgggctccacacagcatgggtcacgatagataatagctgggtcgagaatcacatcatctggaatatcaacctgcccacaatacagttgtttccacgccccaggctgaccgccgagtgaagaaggtcctgctggaggagttgtattaaactgatagattgcagacgtgcgatagttaatctgattatgaagctgcggaacattcgtccaagcaacatggttgcctaatgcgttgatgctcttatcgtgcgcagcctttgtggagacgacgtatgcctgtccgttactgcgaatgcctagtgggttgaagatagcattgaagttcacgttaccttcatatgcgttcttctgcaatacgattaaactaacgccgttgcgatgcgcctcacggagcgcggtgagcattgctgtgggcatactttgattggtggcagacagcagaagcattacacagctaaactgtttgaaatacttatacgagccgtcatagccgtatgcaccagcgttgatttcctgccagctatgtgcaagcatatccaaaggcatacgctgcatgtaaccaacaagctgaccccaggactccatggatgtatcatcattgacaggagctaagtccgagatgacaagcatggaagtgccgttagtgatatttgaattgtaaccacgttgtgttaggaagtgacgcaacgcgcccatgttgttgatggtcttgtttctgtagttgccaagccacccgtatgaggcatccaccagcgggctaccatctcgcacgaagcgaccattcataaacacagaaccaaagccgcacacataagctaaagcgtgtccgtctacaacgaatgacgtaaaacgtgaggcatcgacacccatagcatctaccgcagcctctgtgccattgccaggactgccgctgaatactggagtgatgcctctagcatacaagcaactttgttgtagcatgttatgtccttaagatcggcaagaggggccgaagccccttcttttacccaaatactatttcagtgattgcaagataggtcaagtcgttcgagtcgcctctatctccgccgccatgataatacagccacacctcttcacctacagggatgttcgtatcaaacgtaaagcgttggagaacgttagacctactcgatacatcttgttcagcacctgcgccagcgtaacgttcataaatacttatgttatgccagccaccatttcggccatcatacacccagtcaaatgtgatacgcttgattggtcgagtaaagaagttattccacttgaaccaaccactggtgccgccccataagttcttgtagtcaccatcccacgaagtgaggttacttacgtcactgctgataccacgtccacctgtttgtgcgaacgtataacagtaccaagggaatgtgtcagactcaggaggtaacgcgctgcccccagctatagtcacgcaacgataaggtacagtgaagtcactcacgttgatgtgcggaggctgaatagggcagtacacatagtacgaccaatcacatccgataggtgcagtcacgcgcacagtgatgttagcgcgaagcacatgctcagggtatttccaaaattcgagtgtgccagtacgacctgcaacaacgattgctgtatcgagcaggttcatgtcttggtcaaatacctcgaacttcgtatcaaacgagttcgctacgcagacaacaagctcggcgcggatatccgtttgagttcctaacgcaaaattatcttctgttgttggatgaccggcagagtacacgctatagctctggcatgggtgcatgaactcacgagcaccgcgttcgcctggacagtacaagctgtagaagcaactggccagtgaggcagcattaccgaagtctttgctgaccacacgcaccatgatatcacaagcaacgttctgagggtcgaagtagaagtatagataaccttctcctgtcttagcgtcaagcgtagttgcgatacgacgaccagattgatagacctcaatgaagtcgaacgtttcccaggatgtgtaatcgagatacatccagcccgctacccaaccaatgaagtgataatactcaaatgcgttagcattctgaatacgatctgcgattggccaaacagttgcatggcaaggcgcagggaagatagggctgccgatatagtcagggtggataacgtcagggaagttgataacatcatacgcagcctgactatcgagcgctaacccaccacggtcagaaggcgcagcaagtctaggcggatagacttcgagactccaaccgaatccctgagtagtacgaacacgcaccatgatacgcatgtcagcagcgtcagggtcgaactggaatttgatacgagaacgtcccgtaactttaccacacgtcgaagcaacacgcacacccatatgatacacgtcaacactcgcacctgcaggagcatacgaggcaatcatcagctcaacgtaaccttcaacagcaggcatggcgtagattgtttctgtgattgtagcaccacgaccatgaacagacgcataaggtacgttagggttagcgtatgtacctaagccggaacgagaagcaacaccgacagggtcgtaagtctcgatggctttgatacctggtctattaatcgaacgaccagtcggaggagcaaaggaattaacgagaccgaagccagtacggccagcatcaggcaagtcgaagcctgctggatagcctttgagtatgtcatacttctcacggcctcctgagccaataccgttgcctgagcctttggttgtagatgtaggaccgccgccacaagcacccgtctcgacattcgaacacgggtcatcatatgtagggtcaaacgagtcatcaataagatgccagcgcttgccccactgattacgaacgctgaacttctctggagtcagaggagtccagtcgccgtcttgtgtgcgtatgaacatgggcgtgtccacacaatcatgccaaccgttattcgcagcattacgaacgcgaaaacgtgccacatgatctccttatgggcgaacccaaatagcgccggcttccacctcattgtcgatagcagggtccgtatcctgtacgaacaccattaccttaccgggattgccgggagaaccagtcggaccagtaggaccagtaggaccagcggggcctcggttgcctacatagccttgcttaccttgcagaccatctgagcctctaggcccagggcaaccgtcagtaccacgacgtccatcaccgcccataagaccgtcaagaccatcacgaccggaaggacctacgtcaccagatggaccgtagccgatgctgtgaatagtaggcagccctgcgatctgtatcttaccaatcgtagggatgttcagtgctagtacaccggtgagttggtcgaatgagccgctgagtgtgctatagtcttcttcggtgtctactgtcacaccgccttgagtggctttcacaggaccagaagcattggtcttgagaagcgcaatatcaactttttctaccatgattactccttacggccaggtagtgccttgatctttagtagggtcgacccagatggtgcctgcggcaactgctcccggctgggtagcactaacgatgatagacagacgacccgcaggaccagcagcaccggtaggacccgtagggcctgtagcaccagtattacctgtaggtccagtgcctcctctagggccggtagggccggtaggtcccatagggccggtgcgtccatcagggccggtaggtcctacagggcccggtagaccatcacgcccgtctggaccaggaatgccttgctctccgtcgggacctatattaccgtcacacccctgttcgcccggactaccatcacgcccatcacgcccatctttaccgtcagcgccagtctcacctctaccgccttgtcgcccttcaggtatatcagaagcagtagggaagccttgcactttgacagtctgaccattagcgaacttgagagtcaagattccgctagtcgcatcgaacgacgagtcacctgttagttctgacggcacctctgagtcatcaggactgaccgttagtgtgcccttagaggcacgaacggcagtaggcgtagaagacgcaccagcttgaatgaggccggtacttactttaatcagacccattacgttttctccgctttcgcaacaatatccgtattatgcacaagcacatcaccaacgaagtaacagtcgaatgggtcaacgtcgatatcgactgtctgcacttgttcgtctacacgacgcatctcatatacagagataggtcctttgcgaccaagaacagtttgaccagcttgcacatcacgcgcaggaacatagcgccatacgatatcatcgtaaatcaaaacaggatgttcgtgcgtgaacttctgtccattaatcacgtagtaatgatcttcttgaccgcgcacgagagctttaacagtcgcgtatacggttgtgccttttaggctaggcgaagaccatctgcgaaactcttttggctgattcgaatagccaagtaacgcatcaccaacacgtaagtcttcaactgctttcggaccaacgatagtgttaacgacagagccgtacacgatacagccggatgttgcagtattagtaggattacgagccacaacagtgagcgcagacctaacagtaatagtcggacgcgatgtttgacccatatcagttaccagacagctaatggtgcctttgattatacgatcagcacctaagccgagtctcaggtagaagttaacaatgcaagtgcttgtctcaatggcatcaagagtcacaccctctgtagttgtgatagtccatttatacttatacggaccgacaccaccacgcgcattgacaggtagatatgccagcgacgtaaacacatcagaaccctgcactgtacgttgaccaaccatgtacaggctagagactgacgcagcaagaggcgttattgtaggcagaggaggagcaggagtaacgttcgtcgtagggtacaaccacacgaatactttgctatcgagaggctgcgtagacgaaagaactgctgtagttataggagcgggtcctgtagcgccagtagcgccagctatacagctagggccatcatttcctttaggacctattggccctgtaggaccggtaggaccgtcgggccccgtaggaccgtctggccccatgcgaccagtatctccatcagggccgtcttcaccgtcacgtcccggctctccaactggccccgtcttccctctattacctacaccacccggacaccccggtcgtcctgtctctccgtctcgaccatcacggccaggacgaccgggagagccaggagcgcctcgacgccccggcttcccttcaccaaatactgatacagtaggcagaccagggacgttaactacatccccgttctttttgatgaagactaacacaccggtcttgctgttaaatcttacgctggcgatctgtgtcagtgttgccacatcggagttttcaaattgaacacctccgtcaacgccgactaaggatttaccttcgtcattctgcgttgtttcgacttgcgaaagttttaactgtgttgtcatttcggttcaaccttaatgcacaagttaccagtcagcttcgagccgtagctagtgatctgcgaatcggtgatacgcaccttagccacgatatcaatgaagccctgaggttggttctcaataagcacggtgaacatctgtgtcaggctaacgttagcatacgcaatcacttccgtaagattggcatcagacgtgacaacgttgaatccagcgctgcctgtgccctttaaaccacgaccgtattcagcttctgctgtgcctgggattttgaacgacagaacatactcaatgtgctctttaccgctggtggccgcaaagcctgggcccagttgacactggaagtcagcgatacaggtaagcatcacacccttagagaagtcgatgcgctgagtgatagtcagctcctctgaatcctctactgtctggtgaatgttgaacatgttcttcggatcagcttcttcggctaatgcctgagtgttgctgatagtaatctcgggccacgtacccttaataagaataccttcaccctgaatgatggctggtgcagcgataggcacatcaatcggaggcagaccctgacgcttgaacatgtaacctgttggcgtagggatagcgtcaatgataacaccatcaacagaactatcttttgagcctaccgccatgacgttctcgaagatagtaatctcaacgagtgtgtcagcaggaacaggtgacgttgttttaatcacgttaccagcgacagtgaagtccataggatgtactgtcagaccacccatggccataacgcagtgcgctttgtttagtggtgtagtcggcagagtaaatgtatcagaatcataaggtaagcgatactgaccaatacgaatgcgagtagaccagttggcgcgttcttcatagcgagccacatagaatgagtagcgttgtcctgacgggattgcttctgtcagcgttaccttgttacctgcgttgagcttgtagacagttgtaggctgccacgtactaccaacgacgcagaagatcatgtccacgctatcaatcggcttgctgcccaaagagaacgtagtggtttgaccgtcaccagtaccttcatacgtttcaaacagaacaacgtgaccttgagaaggttcgatgcggaactgtctcaagtcaagagacatgcgctgctcagggaaagatgaaagcagaagctggtcatccacaacgctatacgcggtacgcggttgcaagatacctgatgttccgacaaacaaatcagtcgagctatcgaggttctcggtcagcgtgtatcgcatcttatcaggcgtagcagtagtcaccacagaactgaacaacatcttacctggaggtacaaacaatgttgctgtggtctgacgcgtagagccaccaacaggtgcccaataaggcttgttgtctttaccgcgcattaacgcccatgtgtcaggcacatcgttattgtcaggccaaggcagaccagctgatggtgttgttgggttagtgattcgacgccatactgcgatagtagtctgagcgctgataaacggaatagggtcgtcttggttaacaagctgcccgccaacgtacttgaagtgacgacaggcgccagcaccagtgcctgcgattgtctgaatgatcacaacttcattcgctttcagagttgcagcaaggctggcaatcttaaacgtgttggcgttgatgaacccagcagtcgttatctggccgctgaataaacgatcatgctcgctgaatccccagtagtaggagcctgcgccgtagcgataggcaacaccgggagacttagagccgtcagagttaacatgtaagtcaagtaccgatacggcattgaacacgttatcttttaagctcggcagattttgcagcgtagccacactaggaatagaagtgtagtccgccattttaacagcaagaatcttttgaatgtcctgctggatatgtacgagcaagctaacacggctgatagagttcggtacagcgatgataggctcttccagaacaacgtgcccgaatgggcggttatccgagagcatgatcaacagctcacctacacgcttcatctgctcgccagcaacgtagttgattttaatatcgaagacaaatcgggcactgttctcggtaagtacctgaacataggacagggcgcccgacgcaagctcgttgccaagtaactgctctggaaccactgacgggtttgagcctacaaagtcacctgctttaaacgacactggctgaattgctagtccaccagagttagcgttcgcaacggcctgttctccctgaggcgttagacgcagagcgtcaacgtagatagattcagtggccatcaaagaactccttgggttttaactattctaaattagcgtaaatgaaaaagggagccaggaacaagcgctccagactccctttattttactgatagcgcactgtgattacggcggtaccgaacgcacgagcattggtacgatagatcaagacgttttctgtcaagttatcgtacacgattttgcccacgattggtcccttcttaccgttatcgccggtgacaggccactgagcaccatcgaacccaagccatgacttattcacaacaccagcactatccgccgctgctgcaaatacagcttgaccgtatgactgcctaacaacaaagtaaccatactcgtcggtcttggtcgatagcacaaactgaccaccgacgttcgagcgtaagcgcgtaggcaactgagccaatgcaatactaacaccagtaataccaaatggtgcgatgccgaatctaggataagaagacatagccttcatgaagtgcgtttgctgtaggcgttgctggccttcgatatacagagctttcacaccaaagtcagtatcgttcaacagcaggccaatggtcaggcgcccagtagaagcgttgattgaaatgccttgcacatcaaccacatcgcctttgctgttcgttatctgccacaagcacttagcactaacatcatccttcacgaacgtgccggtacgtcctagcattgcgttcatctgcatcgagctatcatcacggacgttggtgtacccaccgactgtcaagtcttgtgggaagcctacgccaggacaagtaatctcttgcaccaaactgatttcagtacgctgctcggtgatgatacattcaactttaactgtctgtgggtctttcgaagcagggaagcggaaggtaccgtcctgcgacaagctgaaaccactaacagattgaatgacgttccactggaacttaaccgagttggcgtcaggtagagaggacgatccaccagcgccggagcgacgttgatagtacgcaataaagcgatagtccacattagggttgatgttacctgcaggattttcaatgtagccattaagaattgtattctgcgtctgcaactgaatggtacgagtaccaataatcgtttcatctgcaagcgattgagggttctgcttggtgaacacagcacgaagcccaatcacaccatcagagagttgagactgcccgataaacagatgcccattgaggttatcaatagacacaccatccacgtttgtctcgtcaccaatcgaccacagtgcatcagtcgaaaggaactcgtcatcagggtcgatgataacacgcagagagtaaggcacgtaccagcgtccgttctcataaccaatagtcgggttacgatcagatacatcccacacaacgtcaggacccacgataccgatttgtctcagatacgtgttggcctgaacaaggaataccagtaatgtcttctcaatctgatactggtcgcaggtgaaacgcgcacgaataagcacagcaccattaacgttctgtctcggtgtcagagaaccttcagcatcaatctctgcaacaatatctgtcgtaggcatgagcacctgcgtattgttgggaccttcctgcgtgtagtagttctgcactaccgaccattcagaatccacttcgagatcaaacgtcttagggtcttcttcaacatacgaaccatcgagcgttcgcattacaccgccagtcttgtacgtgttaaccagagtgtatgactcggaaagcacgtcagcgctgatttgcgttgcaccttcgatgcgactgttaacgatgttgttcacgctctgcttaggtgtaggcgatacgaccaaatcgatcttattgcttacgcggaagaatgaagcaatgacctgagtgtacacatcgtagtcatacaggattttacctgtctgtaggatagcaccatcgtaatacgctttatccagatcagcgagactgccgatcgcattgaacataggcaacttgcttacgtccatagagcggaagtctttatagcttgttggtgtgcggccttcgatgatctctacgacggatgtgcctgagtaacgcgcaggactaaactgcaagaattgatattcatcagtgtccttgtctggccagttacctacccactctgcggcagtcacatactcttgagaaccgtcaacataagtcgcaagcagacgaacaaacgtgcgcgacttctcatacatagtatctgggcactcaatcatgatactatccaccagcgaacgcgcaggtataagttgcaggtcgcggtagttagtgagcgtgtgtccttcaaactcgtaggtcatgttgatacgcgcagagccgtgcaggtcaccctgaaaataaagcacatgctctttcacgctacgctgcataacagggtcatacacatcaatcgttgagaagctaacgttcaacgtaacccaacgtgcatagtcaggatgatcggggtcaaactgacttgggtcctgtccctgctcaactgcttgctgctgtaggcgaatggttcgtgcccttgcctcctctttcgcgctatccgacggcagatactcgacagtaacggcagcggccgcagcatatgagagtccgttgttccacagacacaacacaggcagcatcaacgacgaaccactactgatagttggagagctacgtaggtccacagacttcggaatcatgatcgtatcgttaatcatgatcgtgcggttgaatgtgattgcagtgctgccgtcaatatacgagaagttgagagcataaggcacagcgtcgccatcgacaagcggggcttcgaactcacctgtctgttggtcaacacgaggcagagcatgtgtgcctgtggcagtatcttggctgctaaaccagatgccaaacacttctgtataagctacgacaatcgcagggtcacgcgaagcaatctgctcaggagtagcagaggccagcacatacaaagccatagccttgggtcgaataatatcacgctcaaccacagtctcaggaacaactaggtcaatcgtcgccagattaatctctggtgctttcagagtaacctgcttcactgcctcaatgggaacacctgaaccaaacgaagcgtagatagacgttagatagtcttggcgtaataccttagacttcaagacgttctcaacaatctccgtatgttcgctggtggtgcgagcctgcgctataccaagtttggacgtaccatcgttatatgtgatggcgtagcgtaggtcgaactcctcaccttgaggaatctcgtcatcaacgataatgcgcagctcagtaggaacaagctcaatcacacttcggttaacatcgaactctttcgtctgggacatatcaaactgaccctgatacttgacgttaatgtcaatcgttgtgtctgcgtcaacactaggaagtattaacgttgtaccattgaacgtaccgagcgtggagcttagagcaatcatgccgctgtctgtcagttctttggtagagcctgtagcgagatacttaccatacactctgaccttagcgcttgcgttaccgaatagcgtagggcattcgatcagcagttcatctgggtcaggctcgacacccataggatagatgcgagactcaagtgggaaactggtggtattgtaggtaagagtcaggttaataaccgatatagcgagaggctcattaaagcgtactgcgttaccatcacgctcggctatccaatccgagtcttctacccagacctcgactgtttcttccgtgttatcactgtagctgaccacagcaccaaacgtagtccactcgccaccacgaatgaactcaggctggatgaatgcgatggatgactgtagaggtcgcccaacgttgaaacgacgaactgattcgacaacgacgtgagcgccgaggtataacttcgcgccgagattgaccgtcgcatagacaccctccaatacttcttcgattggtgcccactgatagaacaggtctgcgatgcgtcgctggaacatagcactacgcgccgtaaattgttcaatatcgttattcacaggttcaaagccgatgtggttgttgaaccaatcctccgcttcctgctgtgtcatgccaacttcttgcagtgcgttaacaacgtctttctctgcatctttcgtgatcgtcaggtcaataccaccgtcgatcagatgtgcgtcaacttcgagattgaccttgttcgtcttgtaccattgaccaccatcttgaatcaaaacaccaagaggtgtaggcacaaacgtttgatagtctgctgtgtacatgcgagtagtgtcgaactgaccaccaagcaacatgcctacaaacttaggccattgagttgtaccagatacttgctgccagtcaggcaggcagtcgatgacacgtttcaacgaaggcaaacgatactgcatcagatcacgcgtgatgttgatgccaagctggcgaatggcggcttcggccagctcgtcgtttgtgtctgccgtgatgcgacgaaggtccaacagttgttggatgactgccaggttatgttcgtcgttgtgtgcatcgagcatctcgaacaactctgcccacgctggattgctttcgagaaagtcaatgttgaaggctagagtgtttgatttcactggttcatcttcctttcgctatacgtgatattgatgcgaaggttacgcagcgcaacgtattcgaggaccgtgttcggaatgatatcctgaacagggctttcaatgttgcagtagtcaacttccggtctacgtgctggctggtctacgtcggtccaatcatacaggacgcgatctgtgatatcagatagagccaagcgtttacccagcataccaggacgacgcttgaacagttcgagcacggacgcttcaagtaccgcctgatttgattcgcgggtaccaggtgcatcagcatacagagccacattcaacgtacaatcaatctggagcttatctgggttccatgattgcacatcgagaggactatggaattgtgccaaccagttcaggaacttagtccactgtgcggatactgggttaggattgatgcctccccaagtgcttgtgtttctaggcaatacgcacacacgcacaactccttgccactcgcggtcattaggtgcaatctctgcttgaccctgaacgacaacatctgcaacatctgggtagagagcaatagcagctttccattcatcacggcgaatcagttttttacggctgcgccctacgataggactatagttgcggtagtagtcaacaggcgtttcatcagagccacccaaacaggcgctcacagtcttaccctgcaactgcgagttagacaggcactgtactttcagtccgatactgtctgtgttgccgctggcaccaagcgctttgatgcctcgcactttcaacgtatacccaacaggaggctgtgctccccactgctcaccaccaaattgaatctcaacgtcaccttcatcggttgttacatcgaggaatatttgttgatcagcatacgcctcaaacaagcacttatcgaagcgctgatattcaatgcgcgtaccagtcgggtgttcgaaccaaactcgtaggtcatccgtaagctggaagttctctgtgcccaatttgattgacatgtaatcggtcgcactaggaacaatctggctgaacgtgaatgtttcagcgatgatgaagtcaacattcttaacctcacccggctcccattgagttacttctgcaagcaacgcattgaaactaccgatagtgaatggcgtatacttgtcgtaagattgctttacactactcaggttagcaaccgaagcagtaacagtagatactgacttacggccaatatcgacacccagatagcgagcattcgcaagtattgaagtgttacgtctggccagacgactgaatgcctcacgggcagcaatcaagttggcatatgagttcgtaacacccaagtcaccaagtgcgtctgcaagcagggacgtaagtgaactgacctgtgcgtctgtccagtagctggacttattgatacgattcaggaagtcctgcgcgaactcctcatgcgaggtgtatgtattaagcatggacatgttactgtgccctcatagcaaacgtaacggattctttcgattcgagcttaggacaacgccatgtgataacacatacataggtctgctcgtattgatcgctcatggtacacgcggtctggacattcgtcacatcgtttgtcaggccgttagctctgtcttcgagagcaaggcgcatgtacgttgcaatccagtcggcagtagtctggtcgaaaggctcaaataggtactgatacacatcagcaccgaaggactcacgccatttacgtgttctctttctggtacctattaccatcagaatcttctggacaatgctgtccatgttctgcacgttatcgcgaggttcgagttgaatccacgcattgatatcacaatagattcgttcgctaataggaacgtctattagtctgactccgattccagccattagccaaatctcacattaggactaccgttagatgcagtgtcgccacaactgttgccgtcacccgcacgttgggcaggcttaccgttaacacgcacactcgaactggaagtagctttgcctgtatgaggagggctgtctttcttccagtgcggcatgtacgagtcgccctgtctaacgcttccttttccgttgataagcacgttagcagacgcctgcgcagcgactacagggaaatagccgttatgtccagtggacttgtctgtgcctagtcgaatagctttctgtcccatgaatattctcctctgttagacacaaattagcttgttaagcagtagaaacaaaaacgggcagcctaatggccacccagtttctgtacgcttggatttgtgtcgcttaactccctcacacccgaagcgagtgctcggtagccgaagctactaagccggagttaatggccgagagtgaagccgcacggcgcggcaacagcatgtgactctcgggaccagatagcaagtgaccaagcatcgcaattgctatcaacgacactaagaacaaaagcatgtttcgctccttgtgtcatactttaagagactacgtttgatcaactggtactttgctctgcccgtcgtccaacatcacttgggtatcagaacgtttctctgtttttaccgcctacgttgcggcaagccgcgcacgacactcacatatcaaggacactcggcggaaaggggaagttccgaatgccctaacaacatgagtgaagcgaaggaggtcccgtatcggtgatctgcaggggttcatgcacgtttaacattcgcttctttgtgcgttaaaccctcgaggacccgaatgccctgctaatcattcctcgaggatattgcacaccttagtgaacaaggtttcaagctatggcagcacgtcaacaacagcggacacactccattgcaatctgttaagggcagagtgcaacaggctgtgaacagctcggtcggaataggtttcgctcgtcgcccaacttcacttgagtatctcgacctaaacttttactctccacgcgaactacaaggaagtgccgcgcttctgtggcctgcggatgtttatcactctcagactcttagctcctgactgggaatcaacacgttgagtcgtccgctggatgacgtgttaactctcctcacctcgtagtgcgaatgccagaacaggtgccgatggaattgtcatgaaggaatccctggggtcatcgcttcccaatgcacacagggtgaaagcctatgcacatcaggcagcgtctgctgcgatactgctattccctattagagtggccatagcgttgagttttcgcttcaccagtctacgtgcctgaaggtatatgccgtgccaagtatgtatcagcatggttcctgctgggccttttgggcgtcagcgacagagcacatattcatcacgtgggtgccggggttgtcctcacgattacagagcgaactcaaaccggctggaggcttgtatgctcaagatgcacatacaagtttgcgcaggaggacgatggccgctatgacacatcgttcccttgagacatattgatattactatctgcaatttttatttacagatttcagaatgcttttcgttccacattcgaataataagtttcgtatgggtcagagtacaactcaggaccacgttgagcacgtacagtcacgtaaccagtgtgacggttgaacgcgatgatttcgacggtaggctgcttaggcttaatggtcgcataaatcggtgcgttcattgtcggctcgtccttctgtagcatatttacagatttcagagcttcaccagtaagcgtaggcagattgaatctgatctccgcacgtttctgaccgaaagcaatcttgattgcaccagcaggcatatcgacgccgttctgcttcatgtatgcgccaatgcgacgagcgatacccgtcaactggtcacgagtacgcgggtcgaaagtaccttcaaagctgatagcttccgtaggctgacgcacagacaaatgcaagcctgtgttaaaataaccctcagccagcagacgcacaacctcctgcacgatttctttcgtgttggatttgattgcagcgatacgcaaatcaggcacatcagccttaatagggtcacgcagttcggtctggttatccatgtagccgagggatacgtgcttcgctttggtgtacgtgtgctgcaacacacccgtagcgcgaatcaaaacggaaccagacttagcctgatcgtacagttcatcgctggtggttgtgctaaacagatagtagtctgtaggcaccgccatacgattgacagcttcgacagctttggtctggacttctttcactgtcttaccgaatacgacacggctgcggtttggctgcgacgcggatacagggaagaacgcaccgtagacaacctgcacgttcttttgaataggtttctctgactggactttaatgccaccctttagaggaggcagcttcatgcccaccagcttcccactaacgattgctttgttagcgactacaggctttaggccagacagaagtttctgcaactcagaaccgtcaagaatcttctccagcggaacagctaagttttgtgccagataatgcttcttacggaacgagtagataaccgtgtctttcttgatctgcaacggtgtagccatattgcgaccaatctgacctacaggctggaaggtgtttttcttatcgtcagccacagagccgaatgctttcgtgaactccgtctggccgatgatgttagcaacgcgctgatgaccacgaacaatgaagatgattttcgggtcgtctttcatgcgcagttcataacgatctcggttgagatacgtcatgctgtacttatcgcctttctccagctcaagatcgtattcatcgttggcgtcatcgacaacaactttcttaccttgataggttgcgtactgacgagcaggcgcggaggtcgaagcgatctccatagccttacctgtgttagacagcgcaacagcgaagtcagtcacagcaggcatcaggtcaacagcagaagcaacggcgtagctgttacgatgctcaccgagatgcagatgtacggcacttgaagcggacatgaatacagtgttacctgtgtcttcatgcttacccgcaaagttcatgccgctaatgcgttcgatgatgtttgcgcttaacgcagggaacgagatatcgctaccagcagtgaagtcgaagatttcaccctgacgccatgcgtaggcaacgttgttggagctaagtccgataaacgcatcgccgatctgtttgacagtcatcggcatgatactcaagtcacgaatgaccgagttttgcttttgaataagattcatataaatccctaatacgaaacaaggcggaaggcgttctgcttgagcagattgagattgcccagcattaggctatacgccaatgtgccgtgctgttcaagcaaactgtcaggaacaatagacccgaagtaaatcgagttgtctggccgaacattaatctcctcaccactagacttcattgcgtcagggacaacgaagcaccacggttcagcgatgtatttacccttcacatactgaatcctatagccaacagccatgtgctgacctttggttgggcggcacgaaaacacatccgtgttctggttacgcgacttgcgtaccgtgaacagcgccatagtcaaaaagcgttgttcgaactgcgggatgaatgcgttatcttcgcaaatctttttcagtaccgcctcttgtcgagctttaggcatcgacgagaatagatttagattcatgacagccgagcgagaatctgacgaacaacatcagagacagaattaacctctgtgtcaatgaccaaatcaaagccgccaggcacttcaaggtagcgttgattatattgttcgtacacttctttggtctgacgcttttcgatgcggtcttcaccgccaatacgaatcttacggcgctcaatagacgtttcataactacacgtcagaagcacggtcaggcggttctcaggagcaagtgcttcccaagtgtgctgatagatgtgtgcgttaacatcagacgcaccagcctgatagacgtaagtagaaggataaccacgatcggcgataatgatcgtatctggttcattttccagaatgcgctcataagcattcatcgttgaggaacgtgcagcaaggaagagcagtagttcggtacgcgagtccatatcctcgttgagagggttggtgttggatagcagaacatcacgaatatgttcagcaagtggcgtaccgccaggctcacgcagacgtagagtttttgcaccacgttgcgtcagtatctcagacagcgcattacacacagtggatttgccgccaccttcgccgccttcgattaaaatataggttgatttcatattgattccttaggcaaatcgcccaccacgccatgcggccttaatgagcaacttcgccacgatttcgttcttcattgtctttcgcttggcgttgcttctgacaaatgcagagccgaacttattcacgacgattaggccgcagcctaactctttaatgcgaccaatgatcttgtcgccgtgagattcaaacagtcgttcatcaatgatgaagtacatacgcatacagaaaggcaaatacttgtgccacttcttatcggtgttgaagtcagcccaacaactcttaacctcggtgataatcatatcacacttggtattcaggcagaatacatcagcccgtaagttgccatgcttaatcagaccaagttcaacgtggcatgaatagcgtttgtcaatccagtagcgttgtgcagcttccgtgagaaaggccgtcttatcaggacggctcattgatttgaacacagcttgaaggggttcagctttgcgccgcttataagccatacgagtcgataatgtccagggcttgcgatactatcggtcgaagtttcttatcgactttagtaagcgccttatccgctttaaaccatttgcgttcgcgtgtcatggcttcgtcgtattcagtcaacatggtcttgaccttcatgacgaaccattcaacgtgttgctcacggccggtcttgcctttgacgtagcgcatgatatctacgaagtctttaggcttaccgagaacaccagcttcttccattgcttctttaagcgcactgtcgagcgcagtcattcccttctccacgccgccttttgggagaccccagttgccagcgtgtgtggtgcgaatgagcaagatctcaatcgtaccgtcctttttctttctatatgggatgacgccagactgcttacgaggcttcttctcgaatggcagtttggctgacaatgacacgcgaatcttcataagtaatcaagtcctctcggaaggtcaacatcccacgagccagcgttgtctttccacagaccctgatgttgcaactccttatacgcatcataaagagaaacacgagcctgcacagagagttcgttgatacccgcggtgcctaagctgtatgcgtacatacagcctgggaagtattgtgtacgattggcttcatgtgtgtcaaacacaatctggccctcactgttagaaataacagcgtgggctgccataccaccttgaccgagaatgacgatatcatagtcggggtgctgtttgtagcagcgttgaacatactcggcgcagtctgcaaatggtcgagctacagcagcagcgcggttgcagttgaactgggcagcagactcagacagagaacgtgcgccagtcagattcatagccgaggcaaagataagagttgcgagcgattcaggctcaacggcagtggggaaaaactttgtgccccacgcttgtgatagcgaaagcatggacgtctccttatacgatagtctcaactaaattagtgtgcttagtcttctgggcagataagcacctgacgaccctgttgataatagctgtcgggtgctcgccctacaacgatagcgcgtttgcacataaatgcaggcttacgcagagcgacattgcagcctccgtgagataacacggcaagcgcttctgctttacagggaccagtcagacacagcatatgcgaatagaaaggcttctgcgccttcttcatcgtgcgtgatattaaggcacgaatacgctccgcttgttgtgcggtaggtgcatgatcgcagtacacagcgatgttcataatcagtccttaacagtcagaagacctgcgtaaacaccgaagcgatcagtgagtgtagcgagagcgccatgcacgtcaccgtcagaataactaaggcacacagcattagcattcgacacagatacgttgttcgcaccttcctcgtacaggaagatggtagccccgtcatgcttacgtcggtcagtgtagaacagaccgtacgaagtccacgaattagtgccgctttccataacatacacagatgcctcaaagaacagggattcgaaatctagagcattggcatcaatgaagttacggtcttcactgtcagacactaccacgtcgagagtgatgaggtcaattgcttctggcttggagcgtaaccagatcttcatgcaactgtctaagtagtcggcgatagcacaacaaatacagctacggttgttcgggtcacgttccgcacgaggtatagcagtcagaacacggtcgcttattttccatgagatgtggtttgtctcaaggcgcccgttatgatactcataatcctcgtctttgatcacaaacaggttggtacgctgcattgcaatgttagacagtacgtgcttggcgcggctaatcaagtcaggtgggaattgaatcataacacgcgcggaaacgacacgaggaacgcctttttcgatgtaggcgaagtccatcgtgcgatgtaaaagagaacgcataatgcttccttagttcaggttgatagtctgtccatttacagttacatcctgaccagcctcaatctgaatgccacctttcacatcaagcacatcatcgcccttgacagtgatcttacgactaccaccaatctctacagtctggttgcctgtgattttagtgtattgattacctgcatcgttcttggcaacacccttaaacttgatgcgcttcttcgggtcaggcttcaaggacttaggcgtcatcacagggtcattcagaatgtagtcagggatatcgttcttactgcctgtgacaatcagttgctgattgcctacgatagtctggttaacatcacccatgattgtcatgttgaagtcgccggaggtcacgaggaagtgctcgtttgtcagacggtcaatgataagctgggtgccagtagacagacgtacaccgatacgatgtgggtagttgacaaggaactccggtaacatgtctgcgtctgtcatgcgcacgttagtattgtacataccttcatgcaactgacctgtaggaaacttaacactgactttagcaccacgagtagggatgaatgacgcaccgaacgtcacaccctgattaccgcctttaagtccttcgagatgcccaacagcaggacgaatccacggaatcatttcatccgcaatatcatcagtcagacccatgatacgagcacgaatctgacctatcttgcgtgggtcattgttgtcgataacgatagcctcataatccatttgagggtcaatgcctttcttggcgttcacactgttaagaggaatcatttgttcacccgtggcatatacacttcaagacgctcaccgtcaggcgtaccgttcttgctcgaaccgtctaccgtaccatctccgagagagcacaggaagttacgcaggttctcttcctgctggcgaataagctgactcaggtttgtactcggacctaagagcttgctaatagacagagcatcgagacacttatcaggtaaggcgtctgacaccatgcggttcatatcatccagcttgttactgacacaacgctgattgatttgaggaccgtctaggtattcagcagggatatcaccgttagcaatcaagccgttcacatcattcgtgaaaccacccagcatgttctccatgctatccagacgcgatgcgagtccgtcgagtatgccacccttgtagttgattgcaaggttgacactcagtttctccagagagttcaggacgttacagataccagtcaggtactttgccatgttgaactcttgcatcaaagcatttaggtagtcaacgccttctccgtatttagccgcaagctcagggaatttgaacgcctccgattctgtctggaactgatcaagcatcacatcgagttgtaggctatgttgctgcgatatccagtcaatagggttcgaaccgtcgagtgcttgtttgatgttcgcgttaatctggaacggacgcaggacgttagcgacagtggacagtggagtctggatgatgttctggccaccaccaatgttcgacgtaccctcaacaggagtgaagttacgactcaacaagaatgcttcgctatacatgcctccggagaacacgcgagtacgacctatgacaagccatttgcctgacactttgatatcagtttcaacttcacgttgaccgttgattacaccagcagatacttcgacaatatcaaagatatctacctcaggacatccgcctaagataagagcgcgagctgtctcggtgtacgccatagactgacgcttgttgttgtaatacgcttccatgtacttgtcatggatgttgatatcgttcgtaggtcttgcgtatgctttacgtgcaccggcaatatcaccacgcgtgtcgctgttaatgttcagcgggtcacggcccttcacggtcacggtagatagttcgttcgtcttacctttcgagtcagaccacagcagcttctcaccatagttagacataccgttgaagataccgctcatggatttcggtctaaactcatgaacgttatagattgggctatcgcctgtgggcttgtggttaaataaccagtacgcctttggttcttcatcaaacagcttgttgatatcacgcacgaccatgcgcttatcggccgtgataaacatcttaggcagggcttcttcacttacccacatgtgctgttcgatttcgtgcgcaaacttcttaggcgagcacgttgcagatacccagctcatgatatctttcgtttgcagatcgccgaagtctgtagtcaagccgcccatagaggccacttgttttaatgcgtcaagggaggttccacgaatagcgaagctacgtgtgtcgaataggaaagtaggcgcatcgagagcacacaacacggtgagcattggactgcccccgtcaccagattcgcgtacagcaaacacagagaacgtgaacgtagacgctgattcagaatcaggtccgattaccaatgttattttcgtgccgtccacaatcgcgtgggaggatcgtaatacgttcgtctgatcggagaatacaatcagagcgcagggcacagcgaatgtgttttcgaacacttgaacggaacgaatgagattcggcatagacggcggtgctttgccgtctaataaaagaccaagaaagccttggtcctttacgccgccagatgtagcttggtcagccatgattaaccctcagcatcaagctcaatcgcaatggctttaagtttcgcagcaagcaacttgagttcagaagacttcgcctgcatgttaaagccaccgcgaccaggtttgatttcagaatcgtttttggtgttgtaccacttacgcacctcaacaacgcgattaccggcatcatcgttagcgagatcaacggacagaaagccatgaggacctatttgaacgcgaaacagctcaggagcagaagtctctacgcaagttttcttctttttctttgctggcgcttcttcgacaatctctttcttgaagtcttcccatccctcacggatagtattcttcttggatttcttttctttaggacgcttgagttccgtgtctttctcagacagaacctttggcgtcttcttgagagtgtctttgatcttcttcgctttcgcaccaacaattttgccgttaaccatagccattagatttgcgtcctcttaacttttttgattgcagcgctaggccgcttttgcggaagaacgacgagcatccccgctttaagttcagaggggtgtatcagtgcgttcgccaccagtatgaaattccagtagacgtttgagccgtagttatctactgataatagttgtgggttgccctcaatcgaggcatcaatacgcttggacgttcctgtctgcgccgcatcaacatcctcgaatagcttcatgctaagagggtcaattccccacttgtcaattacgccgattgtttcagccatttacgtaggtcctcacgagtaacagcgaagtaactactcacctgaaggatgaagtcaacgctgattgggtttcctgtaccatcttcccacacgttgtcgaagttagcactaacgctatcgaccacacagggactcatggagaagaaattaccaatatcaacgaagaacgcctcactgtcctcaagtatacccccaatcgcagcattagcagcgtccgcactacctccgccagcagcaatggtcatagactccatactgactgacttcaatggacttggtcctggaggtaagagtaagccgccctgctcagaaggagcacacagcgaaagcagattgatagttgtatctactacttcgcttttcgtgtcagagtaggcatcgacaaagataggcaggtcgattgataagaagctcggccctccccacactcgcgcactcgccagtttgtgcatagaactcgcaccagcgaacttgagagctttgtccattgaacccgcagtgttaccaatgaacccaccaacagcacccagcttaccaccagcacccgacagagcgttaccggcagcgccagcaacatcagcaagtgaagtgttcatgaatggagcttcccaagaagacgccaagctgaatgtgaagtcaggtggaatgaaacccgtaaacttaatcgtaccactcttgttatagattttgactcgatacatgttatcgacagagataatgtcatcacgagatcgagccgtacctatagcagtggcttgcccaccatcagcaggcattagatagttagccacacagactccttattacatgtagcccagagtgatcatattcagcatcgggtcatccatgaagataggaatcgcgtcaagcgtatgaccagcagcaggactaccgctactgttacccgaagaagacggcttagatacagcgcccgctttcggttgattggcaacaggttgaggtgcagcagaaggctgtggagtagcaggaggttctgatcgagcgatatccccaggagtaactagaggttgacgctctacagcagcttccggctgtaccgtaggttcgatgcggttaacatcaggagcagccaatgcaacacgttctttgagttgccgttcgtattcttctgaacttgaacgaggtgcttctggcccttttgctgtaaggtcaggaaggttctttagattcctatcgacagtagtgtctgcggtatctaatgcacctgaggtacctgagcctttaggcagatccgggaatttctccgcaatacgagcatccaatgcagcgtccgcatctggagtatttacagctttcttcttgcgctccgcctctgccaccttgagcaatacgtccttctcgttctgcgctcgcgtcgccactgattgttgcgtttgcgccgaacttgatttgaagtaacgatcagtcgtcgctgccttgtaatcctgaatggtcttaatcagatcatcgtcggacatggcgttaacgtctttgccttgcagcgcattggagataacgcttgtgcctgcaccgtactgtactgccgtgctgtacatcaattctttcacaccggcaccgcgcttcgtcaggtcaacacccacttcgttctgcatcttcgcagcaagtggtgcatagtgagtacgcgtgatatagtcagattgtgctttatcaaactcggcgctgttattgctcgctacgtctttgtagacagagttgaactgtgaggtacctggagcaagaccaccgaaacgctgcaagaacggtttaccttcagggctgttcaggaagttcatcatgctgccgttgtttgtagcaagctggtgcttcccgtaagacacaccaccagcatctccctgtccagtagagactgtaccgacgccacgaccgcccgactcaaactgttctgatactgaaccaagaccaccctctgcaattgcgcgttgagcgatatcggttacttgcttgctgtccatacgacgcgcgggttgtgctcgcatcggacctgcatatgtacctgcaccggagcccggcataccacccaggccacccataccaccaaagccaaaaggcatgatgacaggctgaggaaatttcgctttgttctgattctctgcggtagtgtcgttgtattcgtccatcttctctttgcggtctttctcaccgtcagcgagcatcttgtccgattcatcagtaatcttttcagcgacatattcgcccacagagctaccgaagtagtcacccagtatgttaccaagcagaccacccaacgcagcaccggcagcagtaccaactacgggtacaactgaacccagtgccccacctatccatgcaccagcaatagcaccagtcgtaccaccggcggcacctcctatagcagagccaccagctttcttcttctctttagccttctcagcatcggtcagagtttcatctgcgtctatatgctgcgcttcattcgcataagacagaccgtgacccgcgctgggtccgatgatagggatcttcttcgaggcaccagcaagcagcatactcgtgccagctaccgctaggtcttgcgtttcagaaggcggcttaggcaagtcacctttagcagcatcttctgcacgttttacctcaggggcgctaggcattggagtaggcttagcatctgaatcgggcgcagcgtcggtcttctgatagtccggtgtaccggcaccgccattctctgcgttctgttcttcaaactctttctgagacctgtgcttcaaccacagaccaccgcctacagcagcgcctaacgcaagagcaagacccagcttacctttgatcttaccgaagcgactacgacgaggcagtctacgacctggacctctacgttcgcctcgattgcgaccatagcgtttacctcgacgacgtgaacgacgttcatctgggccgaagtctccgcctccatcattgttgtcaggacccgggtcatcattagcagaatcaggtcctcctgctctgcccgcaccaggctgattaccatgtgggtctgacttagcgcggttcttctctttgaatgcctcgcgcttctcccactccaaccaatcttcgagagctttctgcgtcttggtcgaaacagcattgccgtcacgaatagccttgacgatatcttcgccagacttctcccctgcaatgaacaggtcctcaagagcagcttcgacttcacgaggattgggctgggatgctactgcccgcggcgctgacggagcttcttcactcgctgttggtgcatagcgcacacgagtgttggccatcttctcacgagcagctttggccgccctgttcttagcgcgtgaaccgggaccgacgtagacaacttcttcgtcatacatctccggatcataatcttcaacgtcatttgcagcacgacgtttacgctttgctttaggcatgccagctactgaggaacttacattgtccgcatgttcgatcattagttcgagtgcggtcagttctttctcttggggcttagccattatccacctctacgacctcgctgcgccgcaagtgcaagcgctcgctgttcttcggctttgttcttatcgtgaacgtaagcactatgccagtacagcaatttgttgatcgttatattgtctggtacgtagatgttcttggcactagcaagatccagtgtcatgttcatcattgacgtatcagagaacacacggaagtagcctaagatatcaattggacttttatacttatacgtacggaagcatttgttgcacttgtgcgttgtctccaactcacagctaacgtatacatggttgcctgcgtccatcaattctatggggtcggcatagtcgagcgtttgctccagaggcaagtcgctatccatgtacattgcgttcataacctgagtacggtcacgttcttccgcgagtgtttcagcatcaatccagcgctgaacggtaggatgacgcaagccttgaggaaggtcgcaccatttgttggacactacgttctgtcgcatgacttcttcggtattgagcaggttgcattctacttctacgaatttgcaaccacgtggcctgtcatagtaccgttctcctcgcatatcaacgaagaacgtttgggtgcatcgccattcgtatagacggtgtgacttcggccaactattagcgtcgaacattgccagcatgtatctaaagtcttcgaggtacatatctcggactttaacattggtgaatcgctgcaacgtatcaacaaagagatcaggcagtctatacttctgggcgttgaacaggctggacatggcgtcagcagtaatctgttcgatacgcacatcggacctgcctgagggcagataaatctctaacattagcgcacgaacatcgctggattcatgtcccaagcacgaacgcttttgcgtttacatgcagggcaagtgagttcgatatccgtaagcacaccgtggcgtgatgcagttacccactcagacagttgaagccagagtgttaggtcttcctgttcttccagcagagccacgttacgatcaaactcgcgtcccatgtgagctacatgccagctaaacatatcctcagaagcacgttcgaagtgacgcatacgaggcaggtcgaagcgctcatgttcagcagccagcagcgcaactgtcattgacgtttcatcaacaacaccgatgttgtttgcagcacacggaaacgtgttgatagctccgccctcagggcgcaattcattcacgataccgtcggaatattcaaacagcggtttattgcatcgccagtgagtcatcagaggcataacagagttcatccacatacgctgctggaagacgagcgcatacgcatcaggcactgtcagttcttcgagaggaatagacaggcatggagctaaagcgtcgagcaggatgtacttcatgtctttcgcatcaatcgcctttgcaatcgcacggttctctttaccaccaaagcggcgcatcgtaaacaactcaggaagctgcgctttatagccacgcgaaggtaaactcgctgtttgaatttccatttgttcttatctcacatcaaaggacgggaaacatcaagagccatttgcacagaccacataccacgaccaccggtgccgttaagcgtaatgctttgaccgccgataggccagcagttgcggagctgctgttcgccaaccatttgcccttggttgtcgtatagctcaatgataatgtttttcttatacactgagggcaatctaaatccaccagtgtatgggttctgaatcaaactctgccacgcattcatatacttcatgactgcgagtttctgatcgagtccgaacagcagactgaatccatccacactcgaaccatgtggccagttgatttgtacagtggccacttctttagatttcgattgatagacagagaacggcaggtcgacttcttcacacgcgaacgggcttaacgatatattaccaataacaggaaattctcgcacacgccacttgtcctgcatgaaaggatcgtcaaggccaggagcagaggagtcattcagatcgtcaagtgtcggcagcggcatgattaatcctctactatgacaagcacaggtcgaacatcattatcgagcttgaggaacgtcgcaccaaccagatagccacctttctcaatctgcttcactacagctttctcgtagtccgtctcccattgctcacgctgcgaggacttgtagccttcgaacgtttcagaagcatcgtagtagttatacgtgcctccagtaggcatagggatacgtgcaaggaactgaatacggccagcgttcttaaacttggctttatgcagttcttgagtcagcttcgtgttctcagctttagagccaggaacagccttgaaagatttcttcggttgtggttctttaggcgcagcagggagtttctcacgcgcaggagtattcttgtctgtagccttcttaacgcgaatgccactgaccgttcctgtgaatggacgactgcgacttaacagcgaacgcgcaacaggcgcatcaacggtgaagactacagacgggtcatccttgtgcagcacatagaacttattacgcttcgcagcaacgataccgtacacatctttttcttcgatatcggcttcgtgctctttgttctcgatactgaccttgcgcttaccttcgaagcgataccagtcgcagtcttgaatagacacgtcaggcttacgtgcgctttcgctcagtaaaataagcatagagtctccaaaacgaaaaagggccagaacgaatcttggcccttatgtttcttacacgcgctctgcgtagtcgaaggaccattcgattgaaaccggaacagcctgcgcagcaccagagaagttcaagtctggtacctgtttcggccacacgccgtagatgttgtactcagcaacaactgaaccgtccatgtcgaatacacggaacagagctttcgttgcgtagtcagctttacgtgcgcccagctgggtttgcgtagcacgaacgaactcatgccagtcttccagttgcttgtacacggccatctcagagttttcgttgtactcagtagagagcgcatgagagaagatcttacgaccagcgtagttgagctggtggccgaacgcttctttcaatacttcttccagagtagaacctggcttgataccggtcttacagaacaagcgcagagtacgcgcatagtccgacccaccgacaggagggttaggaatcaggaactcgaagttgtcatcgagtaacggatctttcgtagacgaaaattcgtcaagagttacctttggcatctaaaagctccttagagtgcaccagagttgatcagttgcagcgcgtactggatatcgcctacaggaggcacgacagcagttacgtggatgcgtttggtgtaacgagtcgggtcaaggaacacgtcgatgatcagatcgccacgcgcttcgtcttctgcggtgttgtttttgtagtcacactcgactgcataccaacgcagaccacggccgagtttaatcggttcgaggattgcttccatcgcagacttctggcgctgtttcagaatgtcgtcgttcggttcgaacacggcagtaaggttgttggcacgggcagaagcatgaagcattgccagcagacgacgcacaccgatatcctgaagaggagacttcgtagtgtaagtggtatcagcaccccacatgaagataccttcgccttcgaagatagcaatcgggttaatctggttatcaaccagaatgtcgcggtcgttctgcttaaagcgataacgaacatcagttgcgaagtccagcttaccgcgctgcataccaccgggagcaagccaagaagcaacttggtcagcagtcaacatgcagtacgccatacataccgacgcaggaacatagaagtcacgagcgttggtattgtcacgcgctttaacgtcagagtttgacagcgcagaccaagaaccgatgatggagaactcggcttctttgtacggcttgttaccacgacgatacgcaacagaagcatcacgtgcctgcatagttacaggaacaccgtgtgttgcgatacagtccatgcggctttcggccagttcatcgatcttattcgcaataacaggatgctcaaggccaccagcacacaggatgccagcctgaatgtcttcccagtcgcggtagttatcccacgcggtcagcacagcagacagactgcggttagagatgatcgggtctgaatgatcgatatcaatcaggtcgccatcgctaccaccagtgaactgaccgttaggtgcagttggattggttgggtcagcaggaccaccgccgatggagttgatgaccacgaagttcgggtcttccagcagcttgtagtggttctcattcagcttaacgcgaatgtacttcgagttaacgttgataacgtcttcaaggaagaactgattgcctgcttcgtctttgtaataacgagtagtcaccacgtgagtttcaagcggtgtcaggtagccaaccatgtacactttgatgatggacttaatgcccagcgcatcggtcacgtcaggttcgaacgtgatatacatgttgttcgcgtcagcgtactgagacatggaatagatcaggcagatatcgcgatcagagaaagcaatctgctctgggtcaaccagtccagcatcacccagaggacggcaggtagcgaagttgttgtacgttgtgagatacacacctgcgtacttcacagagagagcgacacgagtaatgttcagtctggtcgctttcgtcatcagaatttttgcactctgaacgttgttagcgtatttaccagtggctggaccgaagatagcgtcgatctcgtctttagaggtaacagttgtgttcacacccacaggacctcgcgggaacggcagaaccagagtacacatgccgtactggacaagtgacgcctgattcgagcgatcgttctcctgcgagtatacccccggagaggggtgattaggttgtagcatcgtgaatctccatgagaatgggcatcgtgaaacgactgtatgaaattagcgtgttatcagtagcaaatcacattaacgcgctggtctacgtcacttaccaataccgattgatccattttgcctgtgagcgtaaactgaccttcgatagtcatctgcccaccagcatactggaggatgataggctctgcggtatcaatgtacagcagccctttaatctcaggcagttgatagccttttggtccaacgataactgattgctgcacgaacaggccgtcttcaggaataccaacagcggtcttctgcgtcttcatgatagcattctgttggcctgaaacagatcgcacacggctatcgacgactagtgtacggtcgagcttacggtacttctcgcgggtatacattagtcatgctcctcttcgtcttgaacccgagcagcctctgcgcgtgggcccaagtcaatatcaatctcaacgttctcggtaacttcaccgtagttgttgatcttagcctgctcaaggttgaatccaatcttagagtgaatcgtgattggaatctccagctcgaagctacccggcgtactaccttcatcgaggtcatcaatgttgggcatagggatagagtcgtcgagtttaacgcgcacagtccacttggacgtaggcatctcaatggagaagctcattaagtccgtcaggcctgcaataagcaactgttgaacgtatagcagtgcttgattgacgtccatgaacttgaggaacagcgtaccagtgagggtaacagggaagtaatagttagttacaaccacagcgtttgagccatccccgtcggcacctagcgcccaaccactaccatgtcgtgcaatgttcttcacgttcacagactcgtcgcggttgaatgccatagtaggcagcttaaaccaaccatatggataatcagtgctttgattgttcgttgcacgaataccctgcttagggttattatgcacagaccaaacaaaacgctttaggttgaagccttgacggaactgacgttgaaagccaaagatggttgctcgcagcgatgtgctgttcttgagcataccggataggtttgcactcatttgtggtgctccagatacgaaaaagggcggccgaagccacccttttggttacccgcaatcgggtgctagtcgtcgaatcgtaaacgaatcagagaagatgtagcggcagagtcggactcaacagtaatgtcgtcttcgtcttccagatcttcatcatcatccagatcttcatcttcttcctcttcggattcggagttcagactgatgatttcgtcatcgccatacagcgacgcgacttgttcttcctcggcattaagcgctaaagcagcagataacgcagcgacggattcattcatacccgatgcggaactaacggagttaacgaggcatgatgcttcgaagttgtccgagagttcacaacagagaaagtcctcagtgtctggcgccacagcagcttgagcaagcaagcgggaagcatccatccactgtccgtcacgcgctgcgacgattgccagtgcagctaaggaaccagataatgtcttcatgcttggtcctcagttaagagggcaacattacgctgccctcaattgcacagtcaattagccacgtactgctttcgctacagaacgcacgttcgccagagtgaaggagaaggtgctagacagcaaccaaccgcggtcggtgttgccctggtttgcgccgctggtaggggtagactgggtgccgccacgagtggtgtacactgcgtggtagtcctggtcggccagaacgtacagctcaccgtcatgcagaacgcggtgttctggagcgcggaagccgtcagttaccagttccatacccagcagggtacccagacgaccggtggtgatcaggtcatacttagacactgggtccagagcagagctgaactgatcgttaccaacgatatcgttccagtagtcctgcgccataacagcggtgcttacaggcagcggccagcttgacacagaatttttcagagtagacagcagacgcggagtcaggtcaccatgcacgaaggtaatcgggttagcgacgccaactgcctggtcacaagcacgtttccacaaacggtcttctgcaaccatgatagaagacaggccgtcttgctgcgcacggtccagcaggtcaccgttgatctggtccagatccattttgctgacgcgaatgttggatttcagttcgaactcagcaggcgtgtaaacacggccgcggaattggtagtaacccatgtcagaaggaccggtcgcgatgattgcttccgcctggtgaattttcagttcgatacgagcgatatcgccctgacgaacggtagcgcctttacacactttgcgcagcaggccagcacgttcagcacggtcttcgatagatgcaacgatagaagcacccagagaagcccacttctcgccagagctgtcagccacagcttcctggaacagttcgattttctcttgctcagtcaggccgcctgcgttagcagaggtagagtgcaccagttcgccgttctggaatgcgcccatcagcttagtgatttggcccagcaggtctttttggctcgatgcgttgatctcaccagtggaagaggaaagcgcaagctcacctttaccaccaaaacgcaggtcttcgattggcgcgccgttacgcagggttactttagcgccgcgcattaaagagttgttcattagttgctcctgagattaatctcgtaagttttcagatactaaacagtcacggtgcgcgacgattaagcgccgtaagaggaagtggtttcgatgatcaggtagccgcgctcagtagttggcgcttgcttgatgatcagacctttcagctcggtaccggtaccaccgagggtcagcagaccgttcgggcccaggctcgggtgcagtacgttgtcagcagaccagtcagcggttgggtcaaacatagaggtagcaacgttacccagtttgatgtacgcgatacgaccttcaatgttagaaggcaggccgccgataggagcatcagcagtgtacgaacgcgcttcggtcacggtcagttcgtaattatactggatgcgaactttcttaccaatgtcgtcagcgtggaagtacaggtcagcaccctgaacaccgactttaccttcagcagtaggagcagcgttagcttcctggtctgctttagtaccgtcgattttaaccagcagtgcgccagcgttaggaacgcgggatgcagtgaattttttggtggcgtcgataacgaactcttcaacgcggttcatgttcgctggcggcatagagcgagccagagcgaaaccggcgaatacttcgtcagcagcaccagtagacagacgcaggaatgagtggccgccttcgcgaacccaaaccagtgcgaggccttcttcgtggattacttcacccggcagcagatcagcttcctgggtctgtacgattgcggtagcattttgaaacaacataatcagtttctccaatgagagattgtgcgattaactgtagtacggcttcaattagaagcgcatacgtgccagcttgtcgtcgaaggatgagccagtggaagctgaactctgggattgaacagactctttgtcctgattcaggagttccgcagcggaaggctgtttgaccggagcggtcgtaacctgctgctgaacaaccggcgcacgttcggcactaacagtgccagcagccgcgtcgatagattcagagatttcgttctgcgcgacttctgatttgctcataagctcattggctttggacagagcagttgtcaggaagtctttaccgtgggcgacgaacgcacgttcaatcagagcgcggggctctttgataccagcggcggagagtgaacccaccaggctatcaacgattgggttacgtgtatcaccccagtagtttttcgtaacgcccagctgggcagaagacagagcagcgacgaagcgctcaccgtgatttgcaacggcgtcttcgatggttgaagtaacgttcgcagtagcttcgctaatacgtgcgtcagcgtcagccaccagcattttgtcaacaggcagttcgaactgatgcggcataaagccgaacgattcacaagtacctgcaacgcccgtgttgtttaacgagtgcgatacggcacggatgaaattatcagtatcgaaagatttcaccgcattttcttcgcctactgcattagatacagaagcgagagttgcgcgggccagaggttcgccgtcgtagaacatgtgaactgtgttcactttaccacttacgcgactcaggctaaccagagacgggtcgagcgtaccgtgttgagcggtagcagaagacaggctatcgaaggtgcgactgacgacattgctttcagaatcgaagtcgtcatcgtcatcaaggtcgagatcgtcttcttccaggtcttcgtcgtccagatcgtcttcgtcgccgtcagagctagactcggaatcgaagtcgtcttcatccagatcgtcttcgtcgaggtcgtcttcttccaggtcttcgtcgaggtcgtcttcatccagatcgtcttcatccagatcgtcttcatccagatcttcgtcgccgtcgtcagagctggattcagaatcgaagtcgtcttcttccaggtcttcgtcgtccagatcgtcttcatccagatcttcgtcgtcgaggtcgtcttcgtcgtcgatatcatcttcatcatcgttggatgattcagaatcaaaatcgtcttcgtcgtcgatatcgtcttcatcatcgagatcgtcttcatcaacgatatcaatgtcgctgtcgtcaccgctgttggattcgataggttcatcgaccagcgcagcagaacaatgcgcacagaacacaggctcttcatcggagcttacagtgaatggctgttcgcatttagcagagcagctatacatgtgcgcttcaacttcatcgccagcagaagacagagccgttacagcttctggagcttcttgcggctcacaggaagttacttcctggccggtgtacgggtcgaagtttgcggcagtagcagcgttaaagctaccagtaccagacagcgcggtaaacgtgtgtgcgttgctcagggccagcgcgaagttgcgttgtgcagcttcggcagtttcgccagtagcaaccagaccagcgtgttcaatttgctcgtcagcagaagcggattcagccagagcttgagtaacacgttcgtctgtgatttcggacaggtcagcagagcacgatgggcaggagccctgaaccagtgcagaactgtcggaaataacgtggcagccacaaccatcaaggcagatggtgtaatgagctttcacgtcacccgcagatgactgcgactggacttcggctttctcaaccaaatcaggatgctctaccagcagttcttcaccgccgttaggattgtaaaggtctgcgccgctctgcgaagcaaagcctacaccggcagagttcccgaaaatcatcaggttctgaccaagtgcagtacggcgaaagttctctactgcctgattatggttttgaccgacacacaggatacccgcgagttgggtaatctttggcatggttaaaaccctcatagaatttttagtcgttgaatcgacaggttaaaattaacgattgcagaaaaaattcaggtatttttaaacttttctgctatcaatgtcagcttgcggaatatagcgattttcgaagtatttattgaccacttctactccgtttaacgagtaaacgttacgcatactatcaccccaaaccattagctctgcaagggttgcgaaatgctccgttggtacggatttcattgtcctagcgtcgagcgaatccgggtggattttcttaccacgaatggcctgttcaaacttcatacggtcaacgtttcgtatcatcgtatggtccacaaagtgagccaattcgtgggtcattgcatggccgaatgatcgactattatagccaccaaacaaatcaaccaactgccggggactcattgaaattacaccatacaggaatcctgacacggtataagtcattatatgagaaccaccaacgtcattgccctgtttaacgatacctacgtataaacgcttgaatggcagaggcacgttcagacctatgcccggcatgacgttctcctgaatgtctttcagtacataatcaggagggctgacgccttctaagtgaatacgtctaccgccaataagcaagtcatcggcacctaatacttcaagatgcacattgccacacttaggtatcttttggacagcgtagttatttggagtaccgcccggataagtagcgttagcatataccagagctttcttatcgccaaacataggcatgtcttgcaggcgacgcgctcttgctctcagggactcaggagtatcgctaccatctggtgtcggcgtaccggcatcttccggttctgctggtggtgcgggctgttcctgatcaggtttcgctttgactggcacgggctttggcttaggcgcagtagctattttcttcttctcctcataaggagtgaagtcaaagtccggcttgaagagggcgtcaggcttagcagtgaatgggcgactctgtgcaactaccttgtcaccgtcatctccactgatttcataagccatgtcgtatttaggatgggctatgtagtacaggtcgttgcttaccttgagcagacccacgacctcacgggtatgcagatgcaccccgtttgagatcgctacgtctggtcccagataacgatagtacggatagtccgatatgactagacttcccaccattacgccatccgcataaggtgttctttgtacgtggcagcacaggcgaatgccggatcatcgaccgagctacattcgaagccagtcaacatcttgcagtcacgatataccagacggcctgtgcgaccatcaaggtacgttggtttgttgaacgcggtgtgcgaacagaagttacgatgacgaggagtaaccaactgaccacagatgctgcacttgtaggctttgtacgttgtgcctttagagtacgtgttaagctcgccgctaaggatgcgatcacaacgttcttcgcagcgtgtgcggtcaaacgccagcagcagagtcagacgagcatgattaccgcggaagttctggagctttgacaggttgctgtcgaagatcatacccattgcttggcgataatctttgttgttatgctcgatgaacgtaggcttaccgatgaacgtttgatacgcaagacggccttggtcagggttaaacgtcaaccactcttccagactgaatgcgtcaccatttgtgttaggcagctcagtgatgtttacaggcacaggcacaataacataatcacgaatgttgcgtgacgtgttatactgctcggctgctttcgacagccacacgtttacgtccagattgaatgagccggtctgaaggccaaaacgcgaagggtcaacacgaatagacttagctgtctggctaacatcttctttgtgcatatcaatcgcgcctagtccaacgaggcccatgtccgaggtatcaaatgactcggagcgaatggacttgtccatcgtgttctccctattggaaattgttgatgttatctggcccagcgtttgcaagacgcacacaaccctcttcaacttggaaggcgttgagtccgtccatagtgcttagccagtaacgtaagcgtccatctgaaattactgcgttctcaacatatgcaggaacttctttgcctgaatctttcattgaggcaatgacttcgacgccagggtagaacacatcgaaggacttcgtactgaatatcggtttaacgatatcagactcggatacagggtgcatggcgtagcgactttgaatcatatagatcgcttcgttagcaccaatcagaatcgagttgatagtgccgcgcaatgtgcaacgagcactaccgtcgagagtacgcccgtggtagaacgtaacaatatccgcgatgttatacgcgaaagagaattgagccatattaacctcgcagcgcaccacgagcccatgacttagcaagcgccaaagtcatacggcttgggttttgcaatttgacttcaccattatgcacagcagtgaaaggttcatgcgcattctctccgcgaccagaacgatacgctgcttcattgaagccgtcgaataacgttacgacccagcctgtggatttgtcagaacattcaccacaggctttgtcccagctaatcttaccgcacacacgaccaccagcgttaaccgcatagcttacttgatcagtacctttatacaggtcttgagatttcagcgttttgaacgtcacacgcgcagcagactcagaccgcggcgtcatcttctctttcagtgcttcaatatcaagtgaagaccagaaggactcaaacaacgccgcaaatttctgctcaataggcaggtcgatagcgttgatttgtgcgatggtgctggaactgtcattaagcacacggttgatgaagtaaccgccgaggattactggcatctgtgtaccctgatctccagtggtcaagcccgcccgcttcgcatacatctcacacataccgatagcaagacgtgccaaagtctggaacgtctgcttctctgtactgttggcaatctcagtatagatgcggctggcgattgcaggaaccaccgtacgcttcgctacactcagaatgtcttctggtgtaattgattggccgagcttcttcttagcagcaagttcgaaagcattaatcaggcttgctttgttcgctggtgtcagagactcgctcaacttgatagttgtctgctccgagctgttcaccagactcggctgctgtggcgccttcagtctgcgaactcccgtcgttttcaatcgagctactgtcatttgtgtcttcctgattaggagcctgtagatattgcaacaggccagagttcataatctcctcgttaacatcaagaccgcgaagcgtagccaagttagcgaggtaattgagagctggttctaccatacccagattgcgacagccccaataggctaagtcgtagcacaggtctaaattaataggagtctggtcgaacaggaaactttttggattctgctttgacgcttcgataccctgaatagcttgaccaatcgcattgatgttgtcaccatgacgatagaagatatcagcgagcatcgcatagcactcaatacggtctgggcggaatgcaatagcacgatagcaggcgcacaccgcctcttgggtgaagccttgcttgaatgtagctttcgccagttcgatgttagccaaagcaacatagtctggccacttagctatgccagccaatcggtcaacttcacgccgtgcatcttccagaagatctgggcgctcataataactgaccgagtagcagagttcacgcgcataatagaaactgcaacgatcatcatgtggatagtcaccaacatccagaccaagctccagcagataattacgtgctttgtcgtggtctggatagtggtcagttgcgaacggcgcttctactgatttaagtggttgtcctggcttgcgcgaggccaggacttcatgcgcacggtacttccagaaataagagcgacgacgatatgctttcatctgctggtagtgactgtcgccgttacgcatcagaatccaaacagcttctgctttcttaatgccttgcgtattgcgtagcgcctcaacccaattagggtcatcgaagcgctcgtcaatatcaagccacactacaaggtcgtcttccgagaaaggcgtagcggccatctcacgactcgcgcctagattgcgttcttctgacacatcgaacacatgatacaggttagggtgcgtgaacgccgaaatgatgttcgtggtttggtcttcgctgcctgtgtccacgatactaattgcatcggcacctgcaacgtgcttcaaccactcaccgatattcttttcttcattacggcagatagccgctacacagattctcatgtttgcctcattgggttatatcaaaacgttaccgctatcccaccactgcttaccgtagatatcagacacacggtactcaaggatgagaggctggtccaggtcgacttgcaaaatgtatcggcctaatgatggactccacactgttttctcctcagtgtaaagccgaatctcaagctcaatgtcgccttgtgagttcttcggtacgaacggatgtgaataatcaccatcgaaacccgcaccaagagagtcgtcgaagtatgtgtatgctcgaacttcttcaccagtattgatgatggtcggcgcatatacctgacggttatagtacgaggtgtagtcggcaacagttgtctgccagacgacacgacgcttatagatacgagtcacgcctttgctgtctgtctctgcacgatactggttgtagtaccagcttatctgtgcgaattttacaggcttcaatggcgcttgccctgatgcgtatttcaggaacggcttcgcagtgaaacggtggtatgtcttctgcgtgttcaatctatacaacaggacttgatatgtgtaccattgataaacatcaagggtaatcgtacctgagtctgattgctgcgtaccgttggtcaggatgtaagagaaacagtctgcaccaacgtaaccgctgcgtgggctatagaggaacgcatcgttgaagtagttcagacgcaccgtaccaaccatagggtcattgaccttaatagcagaaaggcgccaacccctttgagctggcaccttatcgagtacaccctctgtagggctgtgcagcgtcacttcatcacgagcgccttgtaagatcttttcgagtgttatctcggtttcacccgagttacgcactcgcaccgtaaggttcggagctagtggcttatagttccgccagtagtcgaacgtacaaggcaaagagagcatagttactccagtttgtacttgctcttaaactctgcgaggcccataacagggatgcctttgtccatcgctttctggagtttcgcagaaccagagccagggtcttttgcgatcagtatcgtcgtatcggacttcatgctatcagaagcagtcccgccgagttcaacgatacgcttcatcaagtcacggtcacgaataccagtgaatgctacgttcacgcctttcagtttagcgctaactactttcaccttcttcggagcaacgagagtcacacccatattcgcagccatgtcgtaggacttcacggcagcttctgctatagagggtccgagtttgtcgatgccgtgcatagcgctaatcttcaacgtcagtgcatcagtctgtcctttctttaggtactgctcaaggttaggaattgcatcgacaactttatcaaacgtagtgttagcaccgcgcataaagaatgacgctgtagccttcaaccacgtattcattggcacgccagctttcagcgccttaaggtctttcgccaactgacggccacgagagtcgccaacaatctcacgcagcgcacccatagaggcatcgaacaactgctcaggtgttttaatgccagacgcaatcagcatcttgcatgtaccaggacctgtgttagcaacgtccagccctttcaagaacgagcctagcatacgggcatcagcggcagacgacttcgtttttacgacgaactctacaccactaattttgtaaggcacgtcaggtagctgaggcttcttggctggcttgagaatctccatgatgtatgggattactttgccacttcgaatcaatttaaccttagcaccaggaccaagaggccgtttaggacccatcactgcgcctttcttcttcggcttgagatagccgtgctcaacatagaaaccgttgtgcgcagaagcacgttcgacagtcacgccgccaggcatgatagtcggagggaagatagcgacaggagccattacgccatacttggactcttggtagataatctctttgaccgtaacgatgaccgtatcagactcaacgttcatcttgaacttgaatgcgtgtcgtgggttagatgcggtagcttttggggtcgctacgtcgcgtgtcatcacgatgccgtcaagttcatacttcgctttagcgattcgcttatccaaccaaggaatgagttcttcctggttgtcaaaacgcataggaccaaagtgtcgaaccacttcgaagccccaacgctccagtcggacgaactgcttagactgccggtcagttgcgcctttacctgcaagaataccgaagcataccatatggacgtacttgaactctttgggagttttaaagttacgcacaaggccggacgcagcactacgtgcagccttatatttaccaccagcagactcgtgcatcttcgccatgaaggtcttatatggaatcagagcttcgaagcgcatgataaccgtacccttctcagaaatcttctgagggatacgcatggcgggtatatggtgagaaacatctttaccgtgcgtagcatcaccgcgagtgaacgcctgtactggtacacctttctcataaacgagttcaatgctcagaccatccaatttgtccgtaagaatccagtcaacatcttctgccagagccttagacagttgcttaccgccgagcgtatactgatcgagactcgccataggaacaggcagcttaacatcagagtcatcacgcgcaccaaccttacgagccaactttgacttaggccagcgtgtgtcgatgtagccacgaatgtggtcatagaccgcatctgatatcaagccttccgaatcagtgtggaacgcatcatcaagatgcgccacaagtttcgttgtctgcgtcagattgagcgtgtccagaaccttatcagggttcctttcgagccgcttcaatgagatttgcatgttgttttctccgatcgtcatcaacactggtatttacagcattagctggcgatggggtctttgttgacagggaaatcttccaccatatcgtacacgcgattgaatagcttaggtgccatatctttcacatgctcggcatagtcaaagaggttctgtttacgcgcacggttcacacgcacctgacgcacttcgtctgggctattggtaatatcgtacagcgtatagataacgatgttgtcggaggagttgtgcgtactcacacgaacaaccagccagtcgcgtttgagtttagcatctgccttgaactgcaacacatcaccttcttctgcctcttcggcgcgagcgcttggagtagattggttggctgctgcaatcttcttagcagtttctttcgcttcatcttcggcggcagcaacgtcagagtcttgatcttcctctgcaccagcttcgtctaccgcgtccgtagcatctgcgtctgcgtctgcgtcatcgtcggactgttcgtcatcttcaccttctgaatcagctccttcgtcgtcagtatcggcatcatccacggattcgtcgtcgcttccatcggattcatcatccccatcttctgaatcatcactgtccggatcgctatcgtcaggatcttcttctgcatcgggatcttcctcatcatcagtgccagaagtatcttcttcctcttcctcctccggcggagcttcgacaggcttcttgcctttgaccttagcacgtactttggacggcgctacatcttcttcgtcgtcttctggttcgtctatatcggacaggtcaagcgcaggctcttcgtggtcttgtgaatcatctccgccaaacaaggacccgatagaatcttctatgttgaacatatcacctgcgaatgggctacgcgatagaacgtcttcgagtttctgctcgtcgaagtccaaatcaacttccacttcctcaatcgcatcatccagttcttcatgctcgatgattttcacacgcttgccacgtttgtctataccatcctcatagacagtacggacttctgatttaggcgcttcaatctcaccgctcttaaccttgttacgtaggtcgcgcatttcggctgcacgttctgcggcagtcttacgcgcttgtttctggagttctttgcgctgctgtttctgctccagaaccttagcgttgttggcgaggcgtactgcttcttcctcctccaattgagaacgcttgcggtgacgacgtacctgtttgcgatacgctttgactgcatcaacgtcaatctcacccttaggccaatcattgaatggcaggatgttcgtgtcgtgtacaatcaggtcaaactgactgtcatccactttgacgtacaggccttcggtattgatgactacgccacctttaccttgacgcaagaaacgcacaccaatcatgtcgttcttgtagagcttgatcatacccttagaagttttcacagggtattccatgctaggcaccatacgccactggtagttatcaaagttgataccatacacagcctcagccttcacagacttaggagcgaaacgtgcagcatcgaactgaacacgattgatctggcgctgcatagtacgagcaccggcagtcttcgtgcgagaatcacgctggacaacatcaggcactttacgcagcttggagctacgctccataaggaatagaccagtagtcttgtccagtggaaagtccacatgcggcatgtctgcaaagataagagtgtagcgtccgccattacgcagcgggagaatgccaaaagtatctccttcacgaatcatacgcttatgagttcgttgagatacttcctttccgcgtgaacctttgtacttcatccacgcgtacttcgttactgcatcttcgtgagatgcggacacggaaagtatcatgttattgtctctatgttgtactgtcactcgttgaaattagcttactcaaggtaaagcggggattaacccccgcttaaatatcctcttgcagcgcacgacatagagccacaagattcttcgcacacggtgatttgtgcccacgtccagtaaccgttaggctgctggatagcgtacacaacagatgggtcaaagccccagacctgcgtagcgttttggagcgccagcaattctgtttcgaaatatccttcttcgagtggcttgtctatcgaaccgtgatttggttcgactgaccacacctcaactacaggtgcaacgacagcgtaagtcttattgctgtctgctttacgcgacttcctgatctctactgcgataggtgcgcgtgtagccggagcccctggagtacgtgcaacaggtatgattctcggcgccttgataagatcaggctcaagaacatccgtgttgatctgaggagcaccctgaatgaacttaccctgaatcagatgccgatacacctcaggcgtcttagccccaagaggactatgaggtacaacaggcgcagcaatcaggcgcagttgttcgaactcacctggagcaggactcacaggatatttaacaagatgctccatacgcatcggcgtagatggggcacagtgataaatctgcgaaggctgcaaccaacgtgtgaacggtatctcaggcataaacagcacagcagggtggtagtcaggatcgacatacttcgccaccagcgtgtctgctttatacgtgacactaacagggcgccagataggacgtgcccaacctacatgatagacagcagacggttcaacatacttaccgcttgtcatctcctgtgggtacagaccgctgccagttgcatgacgcgggtcagtcattccctgctgatacagaccactagcatctaccttcttaccttcaatagcgttagcaggatagttacctttagtgtcagtaaacttaggcagtatctggtcggacaccgcttttatggtagtgcgatattcagggtctcgaagatcgaaatactgaggcgcatcatccatgtgctccacaaagttgttgatgaaggtatcgttgaccacagccacatcagtgaagaatgttggccagaacgagtcagagacaatactatcaccagcaatagcttcgaacaacgggaactctgaggcagtgtctacctgaccctgaataagctcaaacagagggaacgtatcggttgctgcaccttcattcgtaccaataaatgcaggcagcggcgtaaccgtgataacgtccttctggccttctgtcaattcaaacagagggaaatcgtcagatgctattgcaggagcgtctgtcagttcgaacagagggaagcgatcatagatgatatctgacttagcaatcagatcagccatgcggaagttatccacaaagtctttatgacctgtatcgaagtcattcccttttgtcatctgcatgacgtgcgtggccgcgtcttcgaagtcaagccactgtagctgaacatccagctcagggtcatacacaggagtgagcacaacgttctggtcagacgcagccacataagtcttagcgtcaaacacagacacggcatctgtagtagcatcaagataagacaagccgaacaactgcacagagtcagtgccgtacgcggtatacgtagggtcaaccgtcatatcgtagagccagcctgctttcgcgttaccgaactgcaacgtgtgcggttggtcatgagaaggtaagccgtagatcttgagcatcgtgtctgcgcattcgaacggaccaactacgaggccctgctctttgtacacaccacgactatcaagttcttgctcaacacgcacaccatcaatgtccagcaacataccagcaggaatcgtgaagtacgtccagaaattatctgggatgttgtcgataaagaacgtaccgctatcacccatgacataacgttcagcacgtttagtctgaggcaatgttcctagccactgattatctgcccacacataccactcataggaatactgctccgagcggaacttaatcgcgtactgctcgttctctgtaggagtgaacttaatgctggtggtcgcgccaacagcaagtgtgatcgtctgcgtaccgttggagaatacagcattggtatcagtgatagtcagcaccagagggatggtgcctgtgttcttcaacacatctgactgcacttgcttacctacaggcacgtaggcccaatggcgaccaacatccaactgcgcttcgacaatagtaaataggctaaagtgggaggtaccttgacctacatctacgtcaatacgggaagtatcgttctcatgcagaatttcaaagccgagtttctgattgttgcgaatgagcacaggcattgctgtctctacaccatcaacaaaaatcttcacacggccataatcttctacaccatccaccagcacactaacaggtacagcaacgttgataccactaatcgtaacgtcttcggtacggttccaagtatcgttttcgatacccagaatgttctgccacgagaatgcgtttggcgtatcgtctgctttcatctcaaactgatagacagtatgaccgatagcaacagggaacgacgagctggtaatgtacgcatggctcagtgtgatggtaacttcctgaccgtcatatactttggtgactggcaccgcagtaacagtcgtaacctctttgccgtctacgatatcgatcgtggtaacatcaatcgtcgcagacacagtaacacccgcaggtgcagtgataggcagagggatatccgggtcacccgcatcgacaagcactttgaacttaacacttgggcctagttcgatattcgtcaaatcaggccacacgatatcgtagttacgaatcgccaaatgcttcaagcctgtagtaggtcgagctgcatagtagaacagtcgatcatacgtatcggcctgagcgtacgggggtgttagtagttcgacatacggccaaccagcgcgtgtctgagtaggagtttcagcagaagcaaagttgaacagagcgttggagccattcgtgtccatacctgcgacgagcttaccgcccttatcagtccacgccgcagtcgtgttaaacacaacgaggtcattagcgacaagaggacgtgccgctacgttctgaacgttgtcacgaatgttgaactgatagatgtttgtaccgtcatgaccgagcaccaacagtgaactcggaacgaactggtaccagacgacagatgcaggtgcagcggctgtattgccacccaccagcttaccgtccagagttgacaatacatcatagctgtcagagccgttaacgtagaactgatcggacttaaccgaagtctccacgaaactggcattgagatagtgcgcacgaccatctttgtcgaaagcaacatagctgtcaacggtgtttgtaccaacgccagcgcgacgacagataacgcggttgacttcatatcctaattgcttaggctcaccgaactgagtcatcgcttcgtcaagcacatcaacctgaccggatgtgtggaagactacagcactgcgtttattgttcgtgtcataactgactttatagccagcgatatcaacattatccatgctaccgaacacttttgtattcgaagcatcaccatcagtgtgcaaataataaagacggcgtccttggcggtcatggactattgaaataggcttggtcaaatcgaagaacgtgctatcgaagtccgagaacttcgctacactactttgctgcatgtcctgagtagtgggtatgcgtacacccccaccaagaacaagaccaccataggtaggattaagtgcagcgcctagaggcattgcatccataccttttgtgataagacggtagtccagctctttcgtctgtggacgaatgaagatgcgagacagtgaatgcacaagcacccaaaggtcaccgtcgagataatacagcagaacaggttgcgtagcggaggctgagaccgtaactgtagccagaagactcacagaatagtcagagccagaactcggcgtgatatctttctctgtagaagcatccgcaaacgtaccgccaacaacacggaatttgagaacgtcagtatgaccagcagcagttacgctacctgaccaagactgcgcacccgttgccgatacaacaggaatcatttcagccattgttcacctcacgatgtagaaacgaaaaagggcggccgaagccaccctgtgaggaataggcttagccgcctgttacttctggttctttgtaaccctgcaagaagaagacgcgcataccagtgttgttcggactgttagcagtcagagctttgtatgtacgcttcttcggagtgctgccgtcatcttctttctcgttgtacacctgcacgtcgatcagggtaccgttagagataacgtcagaagacgcatagcccacgatatccatttcatacgggtagctgtagcgctgagtgttgaagcccgcaggcagacggaagtcgaagtggttgtcttctgagaacggaaccatctggtacgggttgataaccgcgtagctgtctgcgctgtgtacgtgtgcaggtacaggcagagttggtgcgttcacgtccgcttcacgaacggtgtagcgcatgatctggaacgagcctgggctattcgtagcaggacgtacttccagatcgttattcattgagccaccgccgttcacactgaacatgcagaacagaggagctttaccgtcaacaaccactgtaccatcagagttgatagcacgttgaactaccatccacgcaccacggcaaccatcagagtcgcggccttcaactgcgatatgcagcgcgaagccgtgttcagtcagagagatgtgataagtaaacggagacgcttctgggtctgcccaaatcaggctatcagggttctgctgaccagaactctggttagttgagttggtagggtacgccatggtgccgccgtagtagacgctgccattgcctgaaccgacgatgccgcgatgccagaagcatacgtcgtaatcgccagtggtaccgccggtgttcccgttaaagcgagcaccaatctgacctgcatactcagggaaagaagtgccgcctacagtaacagtaccagtcttagcgatggtgcctgtgtcagagatctgctctggagcagcaacgtacagattggtacgcttatcagtgactttacaggctacacgccagcgctgtttaccaacgccagtacctgccagtggatcgacagtcgcagttgcttcaacaacgaacgcagtcaggtccgtggatggaatagccgaggcaatagtgccgttgacactcaccagctggaagccgttatccaccaggtcctgcaggatagatttccacatcttgatgttgctggtgaatccggattttacaatcagtttgttcatgagtcgttatcccttaagattaaggcgcatcaccagtgccgacaggaagcatcagacgcataccacggttgtctttaccgttagcgttcatgcccagatacttggttttgttggttgctttcagagggttcaactgaacttccgaaccggcagacagaacgtcggcagaagtatagcccagcatatccagtgtagcgaagtacacatagcgctgagtgttgatcatctgagggaacaggacgatagcacgattaccctctgcgatcataacctgctggagcgggttaatgattggggctgagtcaggagttggctgaacagcagacagaggaacagtcgcggagtagataccggcttcgataacagtgaagcgctgaattgcttcaggcttgattgtatctgggtcgccagccagaccgccgccacatgagaaaatgcagaacagtgggctgtgatcacctggattagtgtcacctgtctgtacgccacgctgcgcaacaaaccaactgaacgcggtgccggtattgtcgaagccttctgcgttgatatgcagagcgatgccgtggtcggtggtgatgaagtcataggtcagcgggaatgcagccagatcagcagttgcatccatcttccagtcagcaaccagatcgatgaagctgttggccatcaggccggacttagacagacgaccgatttccacagttgcagagcgcttagccgcagagaagtcagtgtcattcacctgaaggtcaggcagaatgttgacggacagagttttggcggtgttatcggctttgaggatgataccccattgctgagtttcgaacagcgggtcaaccgattcagatgccagcaagtagaatgctttaccgtctggtttaacctcagtgccagcgacaccatcaactgctacgagttcaaaacccccagcaatcattttcgccaccagatcacgggtcagagcttccagaccaatgagcttagtggcagttacacgttgaatagccatatgttaatcactccattaccagataggttacagtgagtttcggtttcgacggtgatgtaccgatattcttcatacgccacgaaattgtaggcgagttgtctttgttggacaagaagctatatcggcgcagcttgcgaataactggattaccttcgctatccacatctgagaacacgccatcatcttcgaggaaattagcagtggagcgaaataaatacgggtttctgtcatctcgctgtgccgtagggaacgcagagagttccacatcaaacgcattgagtttaacagaaagcaacatcaccgtacggttcatttgcaggtcaaagtcaacctgttgtcccggagtaatgtatgcaggagattcgtactccaccgttttacgcacaccagcactttcattgccgttcaggtcggcccagaacatcgtaccgttagcgccagatacgagggtcatacccgcatactcaggctcaggtacttgtttgcttgggtcgaggcctacgacagtgagtcctgtttcatccacagcagtgacgaacggagattcaaacttgtagttggcacctccgaacttcgcttcttcccacgttacgttgtctgtaccaagttgatacatcttcttggtctcggtgacgtaacataacatcccaggctttttattacctacggacattatgtcacgatcagccagagtaggcagacagcgcatacctcctcgaagatatttatcctcaaggaggtatgggagtgctgcggatgcaggcaacaggaacgaagtcatgtttaccggcatcttattctccttacgcgatacctgaaccagggttcgatgaaccgtaggtcagtttaaacgtatacgccagactatcgaacgggaagtcgttacgataaataacgtaatcgacaccattgataacaacttctgctgggcctgcaaagttaaagtcatcgaactccaacgcaccatcccatgaaccagcaaagccctgaacggattcgacaaagtaaccatagccgagagacttaggccacgcaacgtagaagaacacgttgttcgaacttgtactggtatttcccggacagttcaggagctgctgaccggtcagagtcaatgcagtttgcagaccagcaacgaacgctgcgtcatagccagaggtagatttaatcttggaatgcgaaccgaagcgagcacccagatcagaaacctgctcaggcttgagcgtaacgtctttagttgccgtgacagtcttgccgttcttaacgtaagtcacggtgattgtcactacagcatcagcagtaactttgtcagacttcaacgaaccacccacaacactcaggccggttgccgtaccagacttcacagataccgcccacgttgtaccactatcagcagtcacgtcaggagtggtaccatcagacagagttgccgttgcagtatatgcagtagttacgccgccgatgattgaagcaggtccagtgatagtcacagagtcaggagtcgcaggagctggagtgttcgtcacagtcaacgttgccgtttggactacgctgttgaacgaagcagtaccagtaatcacagcggtctgcacagtgctaaccgtattacctgtaatcgtgttgttgccgttgaacgtgaagcccgtagtagagccggagctacgtgtaacaacaggcgtcaggtcaaccgtagtgttatcagagaacgtcaggcgaagaatgtaggtaccagtctcacctttgttcacagcagtaggacctaccagctcgcgcttagtgatcgttgctgtctgattgatgatctgaatagtcttctcaggcgcgtaagtcttaccatcgacggtgacattagcagcacggagcgtgacagtctggttctgcgtgattgagttaggtgcagaggtcagcttcgcacgagtcgaagtagtaccaacacccagcgtcacataggcagcaccctgaggcagtgaccaagtaggcagagaagcatactcgttcgttgcgccagacagacgagtgatacgcaccagataatcacctgacacagtaccttcgttcatcgaatcagcaccgatgatttccacagtgttcacgtcatcggtaggacctgtgaccgtgaactgtacgctaccagttttggacacagcacctacagtcgctacgacgttaagctggaaggtcagagtcccaaagaaaccactgagagttttcttggtgcgaatacgccagccagttgtaccaccagcaacgatctcaaagtattcttgagcagcagtggataacgtgtagctgagttcgccgcttgtaccctcacgggtagatgaatcagagaacgtcagggtactatgcaggtcgcgtgttacagcagccgcagtaccgaagtcaaacacaggtgctggcgccagaggctgtacgctcaacaacgagatgacgatgatgttcttaaccaacacagacttttgcgcgttacgtccgtcgaacgttgcacgaatcagaacggttgtgtcttgagtcacttcaccagcagacaaaataccagtctgcgcgatgcttgcgactgcgctaccctgaataacagaccacgtaggtgaggtcacctgacgctctgaaccatcagaaagaatctcccatgcagtaaactgcgatgtagtgttttcattcatctggtcagcaccacgaacttccagagaagtcacaaccggcgggttaccgacgatggttacgttctgcgtggcagtcttagtgataccgttttcagtgtacgacgcatagatcgttacgctggtgtttgcgatgttcaccgcacccgcgatcagattcgagtcagagaacattgcatagattgaagcctgttgcagacggaactcgttaggactaatagtagccgtgtgtccgtcagagtaagttgccagcaccgtgtatggtgtagtggtcttctcttgaacagacgacggaccgacgatcttaatgctcgacaggtctactacaggcacaacgttaacgataagaatatcgagagtcgcagtcttagtgatgccgttctccgtgtacgttgcagacagcttcacaggaatgtcagaagacaccttacctgcgttaacagtcttgttcacgatagtaacaacatccagacggtccgcagtgaacgtcgttgggtcaatcagcttggtgctgttatccgagtaagttgcgaggaacgtatagttcgcgctttcttcgctgcggattgtattcgcaccctgaatggccagagaagtcagcacaacggcctcggtctctttcagaatcgtgacgttcttcttacctgtgacagtctgatcagcagtgatgtacgttgcagtcaacacgatatcacggttcgaggttgtttctttacgcgctgtaaccacgttaccactaatagtggtgtacgttgtaggtgcagcgacgaaagagttctgcgttaccatctcggtatcgccattcgaccacgtaatacggaacgtgtaggttgcgctttgctgggacgtgatggtggaagcaccaagcacttcaagcagcgtaatcaactgcgctttaaccgtgacgttcttattcgcagtgaatgtaacgccgttatacacatacgtggcagtcagcttgacgactgtatcagtcgagactttcttaccagtaccctgcaggccaacgaggtccagagcgtttacgttatcaaccacgaagttcgtaggcatgatagtcgcaacgttaccagacttgtagcgagcagtaacggtgtaggtttctttctgcttatagaacagcgtaccagtaccaacgatagcgatggacaccagctcgtcatcaatgatgaacgtgttcttgatcagcagattgtaggtagctgttacccagttgccgtacacagggtcgcgcttacgggcagtcactttcagaacaacgtcagcagctaaatcaggagcagtgactgtaccgtcctgcgtgatagtcacaccgattacgttttcttcgatagaccactcgacgccagcaggctggtgctcgatacggtctgaccactcagcgtcaacgttcagtttgacactactgttatccgacatgtaacttgcgttgcccggcaggctaatacgcaggttcatcaagtggggtgattcccactcgacgttatcagcagtaggcttaacccacttaccgatatacttgttagggttaacagggtcctgatcgacgatagccagcacgtagccttcttgcggttcgttagagcttgcgacttcaacgaatgcggtagcgttcaggcgaatcctggtgcgagcgtaatcaggatggtcgtggttagtcggataacgtgcattactcatgcgcgtatcagagctggacacagcaactgtttcagcagtcgattctggttcatctttagtgacgacattccccagacggctggtggtcgcatgtgggatttccagatcgccaacttcaatccccagatcacctgcgttctcaacaacgaagcggaagaactgtttctgattgaacagtgcagcgtagtcgttcacagttacccatgaaccacggtgattaccgtcagacacggctgaggtacgacgcagcacatacatatactgcgggctgcctgtgttggcatcaatccaaatcaggttgtacggcttttcagaaaacgacggctcggtcatagacacgataacctgatgcacttccgtttgatcgttcgcgttaggacggaacaggaaagtgattgggttacgtggcgtcagacctcgagtgcgagccaggccgatatactgtttagcaaagccgtcgatcgtggttacgctcattcattattctccagaatgtcggtcgcaatcagatggccgtaagatgctttcacgttagtgtcagcgatgaacgtagcaccgttatcacctacatcggcgtccatgttcactttatcctgcacggtcttcacttcaaccagcggcttctctgggtgcatttcatcatgcggtagaggagtacgcttgtcagtgttacgcgggtcagtcaccgacacaaatgtaggacgaccaacagaagcaggctcagcggtcagacgagcgatcccatattcgtcaacagacgcgttaggaatatcttccgtaccgctaatatcagacgggtcgtaatactgcggcgcccagaacgagttgaagttcttcacttcttcccatgtgttctgaaagccaccagcaggcgtcttagacttacgcgcaaggaacttacgatagaacacactatcgcgtaccatacacaaccagacgacgttcattggcaacacgatcccaacaggttcttcctgtgcgatgatgtgcgtacaactgatgttgagtgttgggttaatctgacgaacaacctgctccttagcagtgttatccatgaagcccgtaacattcaacagagcagcggcgatatcattcagtgtagtcataaccgctccttagtcagtcggctggccgagttcagattcacgcaccttacgccactggagcgtactatcttcaagcaccattacttggttcacttgaggaaccagctggtctttgattggcacatgttcttcaccgtaactaccattgatgctgatcatggtagcgggcttctcaggatgggtgtggtcgagtgggtcacgattgttggtaagtgtttcatcaccttcaatcaggacacgcgactcggcttctggatatgacagatagccaacaccacgagtgacgctagtagccagaggaggcagcgtacggttgatgatttgcagatcgttcgggtcatacgtctgttcagtcatcgcgtcatcgtagaaatacaacgcagtccaaacatctttgtatgggtccgagttatctttcgcagtacgcttgaaagctgtaccgaaagtagacgactcagggttgtagtcaatccaaatcgcattgattggaaggaccacgaaacgcggaactgcatacgagcagtagaacaacagacctaactgagagccttccagtggaagacgaaacatgatcgggtttttgttctgctggtggatattcgtaagcaactcaacgttactgatgaactgttcaagtttcagttccattgtgttctccgtttaccagaagcggtagttaaaattatacagggtcaccggacttcggactggtggaaccgtatttaatgcggaacacgtagtcaagactatcgaacgggaagtcattgcgatagacgacataatcaaagccgcccaacgagacctcagccgcaccctcgaagttgaagtcgttaaactccattgcaccatcccacgagccagagaatccttgtgcagtctcttggaaatatccatagagcaagcgttttggccatgcgacatagaagaagcggttgttgtctgatgtagactggttaggaggacatgtaatttcttgaggactcgactcacctagaactgtaggaagtgagcggaagaaggtatcgttatagtcaagcaacgacaacactttatcatgaataccaaagcgtgggccatactcaccactgaacggcacagacacccgcaccttattcgacgttgagttcaggacagtgctgacgttatacgctttggctacgatatcgtgctcgcctgtatcaaaaggcagagtgaagtcgaagtaggcagtcgtacctgacgtaggcatatcaagtttcttgagcaccgtacccgcagcgttctcaatctggagagtaccgcgcaacggcggattgtccatcgagaccaagaagcgcagctccttgttacgcagcgagaagcagtattccaagttaccttgaatggtcaaagtaaacatagaacctcacaatacgaaaaaaggaggaccgaagccctccctttgtgattacagactcagacttgtggaggtactgcctgacgggttgatgttgaaacgatagatcagacgcttagtggtgcgtgtcgggtctaacacgatatccagaatcaagtcgccgttagcgatagtctggttggtgttgttgacttcgttacaaacaacctgatagccctgcgagccagaagaaccgccacgaagaccacgaccgagtttaatctcttcgaggaacttctcaacgataccctgcaggtagccacgaaggatagcatcgttcggatcgaacaagccaaccttacaggtgcggtgacatacttcaagcacgtaaccgaccatacgctgaatctgaatctgctggaatgcagagttcatgttatactgcgtactggcttcccacaccgcgtaaccaccaccagcaatgtcaggcagcttacggatgtagttgacctgctcacgggtcatagcatcacggtcatcctgatcgtacttctgagcaatagccaagaagtcaagaggggcagatgcagtaatacccgcaggtgcgaaccacgtaccacgattgttgtcagtgtacgcaaacacagcacagatctgtccgacacatgctgtccacagatagcggccagtatcttcatcgaagactttaatgtcaggtgtgtacagtgccatgttcgtgtcgttcacgttcaacgtctggcggcgatagcgaattgccttagacacagactgctcggcggatggaataccgcagataacgaagcagttgatgtgcgcagcagcagcagctttcatgccacgatggatgatgtaatcctgagtaggactaatcagcaacgtcacacgaacttcttctgggtcaccgaagtaatcctgatacgcttgcgccagctggtcagaaccaaccgtgtcaccgtccgagccaccctggaagaagatgaagtcagtggtgaagaagtcgatatcagtagtgaagtacggattacggatgaagcggaagtttgagctttcgttctccatcgcatagtcgatacgatactgacgttcaaattcgtcggcgtaatcgaacaggctgcattggtagctgtttaccggagcgcttcctgcctgatagttttcgtactcgtcgatatagaacagtttcgtattgtacttcgtgcggtcatcgaatgggtcgaggccacgaggcgtagcagggcgaatctgcatagccattgcgttgttccagtcgcctgggttttccagaatgacgtagccgatgatattctcattcagcgggtcatctagcaggaagcccagttggtctggagagtccacaccgacaatgttaccttcgtcgtcagtgtaaggactgatacgcagcacaggttgaacagccgacgggtcatctacagtcacgacaccgaccgcgtatttcgcgttcttagtcacacggacgtatttgagttggttggtctgttttgccacaggcagcgctagatacaagccgaggccatacttgggatcttttgcaccgaagatgtttttcaaatcatctttattacgcacatcaacacgctgattgacaggacctcgacgggcctgaccaacgatgcctacgacggacgtagataaagacgttgcaccaacggagagatcccgtacgccagtgtagacaccagcagaggaatgcgttgagttaacgggcatgtttcgtctccttatatgactgtctgaaattatcgtataagcagttagaaacgcaaaaggggcagccgaagccacccctttgttttagcaatcacaacctacggaatcgaagtcaagtttcaggccaggatagagttggttaaactcctccagtggcatattaaagccggcagcattaacgtgaccatcaccaccacgagaacgtgcgataaaacgagcactacctacgtgaccttcaggtaaaccacgagagcgacagctaacgtaaaccttggtggggtcacgatggccttggcgcacaagcatcactgtttgaaaatggtcatagttctcatagacatacgttcctgtctcggacgcaatgcctttatcacaaggcacgactgcgtgtttgacaccaatcaaatggttaggttccgagaagaagctattggtattaatcagaccacgaatcttttcattacgcgcttcgatattaacgaagccctgagcgatgatttcttcgatatcgccagacaaaatgatcttatacgcagcacggacggtaggaggcatttcagcgtagacgtgaccacacttctctacctctttgaagacgtccttaacgtaaccttcatagaaggcaaaggcacgttcattggtacgaatccacaggtcacggtcagacaccagctgcgcactgcgaatgatgttatcagtgcaggcatattgatgctgttggaactctgacacatgagccatgtatgtgagcagcgtaccactgccaccagctttgaaagtaagacccagcggagatacgtcaagcgcagcacactctttggcgtacagctcttggctgcggcaatcatggtgatcaagcaccttgaagttaccaccatagcgtttagtcatgacagccatctggcgctcggtcagagagaagtcaacaacgacaacgcgcgtatactcggagggttcaccgattaacttaccgtcggcgtctttctgcaaatcgctgagtttgataccttcgagacccttcatgtcttcgaacttagtaccatcggcagaaacgatatctccctggtcgttggcgtacacggcaggatagaaatggagagtatcgttagggtatgcaagtgctgtaatggcagcagcgaaactaccatcagcacatccttgatgatagacaacaagtgtagtcatgactaaacccagtggttattatgattcgttccagattggacgctacgcatatgctcaagcatttgacgcaggcccgccaacgtccgctccagtgatacgcggtactgatcagaagccacactctctccgtggcgcagcgaaagaatataaagcgaccattcttccgattgacgcaggcgctccattttcttggagagaatctgacggcgttcacgagcacgtagcagacgctgcattaaattaagaggttcgtgagattttttcagcaattcaatgtgaatcgcatccaggcgctcataatccaaacgcaacagggcctctttggcctcaaggaaaagtttggaacgacgcaatgcttcatccacaggaaggttacgacacttatctgggtgagtgatacgtgcgataaccttgtagatagccttacatttcttacgcagatgcgtcttcgaccattgttcatgctcggccatcatatctgcatctgcttcgttgtcctgagtttcatgctcagtgtcctcaacgaatgcttcttccatgatctttttgatatcatccgcgttggcttgatcttccaagtcatcggagttagccatttgcacgaccatcgcctgaatctcattgttcaagatttcaatctcggcgatgattggtcgatgttctttgttcaggccgtccaccagctttgtaacgcgttcgcaatcagcgccatagcgcagttcaagcgctgcgacttcttcgaggatttcgtcaagcgtttcgcctgtgtcttcctcaaactgctctaccgcatctaccagttcagtgggtgcggtgtgcggcacagggagttgagggataaccatcaactgagtatttgtcatgggcgcacaagctccgaaattggtttagctaccagctctgcaatgcgcggcggacactgagggttgcgtttcaaattcttatgcaaccactgcaagttattacctgacgaagatacctcagcacggaagctggggagtttgagttcgtcacgatgtttggccagcagcacattcagttcattcagcaacattgtttttccttaaagagatgaagtcatgagttcaagtaaatttgaaactacatgcgcaggtcctatggagatccctgtttgcgcctgtagatgaatacgtttcgtaaatagctcaagagggtcaggactgccgcctgtaactacaatgcgaggtatctttgggaacatctcaaggatatcacgcagtcgttcgatcttatagctggtgctatctagtgttacgttggtcagcactaacagtgagggccgcttgcttttgagttgttcatagtcgaagcgatcaccatacagcgttacccatcgtggcttgagtgcggttgtctctgagtcttcaacggcagcattgaagatagacagcgcggccatctttgcacggtagtcattcgggaaactactgattaccgtgatacgtgggtcagccttgaaagggtcctgaatcatacgtgcaagatgcgtaagctgtttcgctttaccaaccaccttgcccttgaagtaaggagaaatagtcttgtagtcctgtgcggcttctgccacatcaaactgctcttgcttaccgaataatagttgtgggtcaacgcccagcgtctgcatctgctttgctacagcaggttcaaagtcaaatgttagcacaataccctccgttgttcatgttaggtatttacagattctgtggcgcgctgccatactacgaacttgacgttcagggcatgttcttcaagctctgcctcacgtctaggatcatacttcggggagtgccagcgtgtatgatcaggacgttctacaggtttggtcacaaactgctgtattggatttggtacttgaaaatattcatggctctcgataacaactaagttatcaatgcggagaacaccaggaacatcaaacactttcggcaaggtgctcggtgtgagtgcagaccccataactgtttcatggtagtcaacaagtgctttaactaaagcacgaccagcacacgtagacagtgtaagattgtactcggtacgatattccatggtgctctccttagtattacatcagagccagttcagggtcgatatacgtgtattgccacacgatattccaacctgaggcggcgtctttgtttgggtgaatgcgatagccgtagatcatcagcttgcccttagtgtcaggttcaagcgtaggttcatactccagccatgctgcttcgagcttcaacttatcggcgatatctttcgcccaaccatcgaagtcgtaatcttctggtacttcccaagacagagaatgcttgcgccagtgttcagcctgcatgtcagtgtctttggagatccagtccagatgtgctacgcccagatggtaagcaatggcgtgtgcatagccatgctcattcatgtgacgctgtaactgatcaagacgcattaggttgctccttaaagcgtgggaatacggtgacgctaatgcgcgtagaacctttctcatactcacgctcactatgagacacaagtaggacgtctgtgacctccaaagtatctctaatgagagtgagcaactgcccaacaacggacagtggatggatatagttggagacaatcatattgatctctgttacctgatcaggattgcctacagcaccatttccatcccattcttctacgctcatacacgctcgggctgcttcactctttagcaggtccatctccagagtgaagggtaaacgctctttcatcataaactccttatagcctgttgaaaagagacagactataaattagagagcgatgcctttaaggaacgttcgagcgaatttaataaagatcttctgctttgcctcaggcagcttgcgacagcgctggataatgtcttccagtgaatcttcatcagtggtgagatgaacgccctcgattgtaccgacttcacctttctgccagttagctttggtcactgtcaataggaaggtaccacgatactcctccatgctacgaccaccagcaccaccaacaggattgcgtactttagtgtagtcgatattagcaatacgctggacggcaaaaccatcagggaattgcgtaaacaccgaagacagatcaatatctgctttattgtcaggtgcaggggatttagcaacgaactgcacacggaacaattcaccaccttcaacatcgtactggccgtcgaagatgatgctgtcgtgcgcacgtagcgtatcggcaatgagtttgaaaatcggatcgttgaacatgttacttcctcagatagtcggccagcatttcaacatgattacgaatcatcttcctctggtcgagagtgagcttgctgaaaggaggcaggtctgggtaaataccctgcatcgccagatatgttgtctgtatattgcgcttcggttcgggcgcttcgccaaccgcaaagatacagtctttgaataaatacgatggcgggcagccgaatggggtgtccataacctcaatgtggccgcatccgagtaacatcagacagttacctaaagtcttacgcacatcactcatacccaagacggacagcttttcgtaggtagcatcaacaatgctggtggctgcaccttcgatagaaattttgactgtcacgtccagagtcgccgtggacgcacctaatacggacttgggcacaagagtaatgccctcctccgcgagggcacgccgcaacaaagtttcaaggtctctgtgtggctcggattgcatttcattaagatccattagagtcgcctcatacctaagttagatggctggcctttcacacgcgcttctggttcaaagaagtcaggcagttctccatcgagcgcttcttctctcgacacaactcccatccagtcacgcagtttcttcggtgtacgtttcgctttcgcgtagccaaatttccagcacatcttcaacacagagcgagcacactgcatcgagcgatccatcttctgatcgatgaacatgcgtatgactggagtgcgcttaccttccattggcgtcagaatacgacacgactcctgtttccagttcggctcgttattcattggcatgatgtagtacagcgtatcccacttcggaacgtttaggccgcgctgcatcaacttacgcataccgacgacacaacgaatcttaccttcacgcgctgcatcaatgattggcttacgacgcttcgcttctttcgctcccccaaggaacactgccgcaacttcttccatgtaatgctcattgatacgctgcacaaggcgccgcgcttgatcagtgaacatgattggaatcgcaatgcttcgtcctgcatcgagatctttgataacccactcaaagattttgtcgttacgatcaggatggttggcaaggaacttacagaaacgaacccagccagctttcccgttatactgcgcacgagtctgcactttcttcgaggtcttatgcagcgttactttcggcacaagctcttccacgaaggcttctgcaatcacaggcccgaagattgattcgatcaggtagtgacgtccatctttacgcttaggagttgcagtcagaccgaaacgatacttcattttgagagaggccagtgtgcgactgtagcagctcgcgttaccagcatgacattcatcgacgaacaacgtaccgtagttttcgttcagaagtttcaggcgcttcttcgagttcttactgtcagagataagtgactggtaagtaacgaggatgatctgaaagttcttgtagtcgtcgagagtctttgggaagccgtacagcttcttaccatgcttctcttccaactcaggcaggttcgtcatctgctcgatagtctcaagaaacccatcgagaaagtctttctggtcagccataatgactgtacggaatccagagtgacacgcaccagcagtaccgataactgtcttaccagaacgcggaggtgctttgaacacaccacacagttcgccgaacatcttctcgaacggctcttcctgatagtcacgcagcttaccagtaaacttcactttgtagtcatatggcacacggcttgtaccattgacgaacttcacttctttcaggcttaaccctgctgtacgttcgaagcggtgcatctcgccgtaaggaatcgaaacgtaacgcttacccttgatatcagagtatttagccagcacggttatatcaaccagaccacccttcgaacattgacggcattcttcggacggacgtatagaacgaaactcacagttcttacaagcggcgttgtcgaactcatagtgagtcatcttcttaatgatgttgtcagcgtctacatgcgtaacaggaatatgcagacggctatcgaccagtaccttggctgtcacatctatttcctttgattcggcagaccgtactcacgctgattaatcaagttcatcgtatcgaccagcgcacggtatgcaaacccacacttgtcgatatccttgatataaaggtctaactcttccttgagcaaatcaagctgatcagcgtaacggtaatactccgccataatgtttctgacacaacgctcacgctctttggcggcgccgacggctttcagatctcgtgcataggttaccgaggcataatcctgaaaacgttccagcatatcatttaacagtttcgaggctgcgtggacatgcgtcatgatttcagtcatacggcttcgataagactgatcttgaattatcgactccgctactttgttaagagcattagggtcaccagtcacattcagcgttctgaccttgcgcatcttaaacagcttacgcgcttcgtcctgatactctgccagaggcatctgaaacaggtcattggtcttgtagatatcgcgcaacttcttatagcgcttatcttccttgaccttgagtcgtatacgctttaggtcatccatcaatcgcctctatcggttacaagcagtggactgtcaggagtcttatgaggcatggcaaagaaacttccatgctcgtcacgataaatcaacagaccaccagacggcccttcaatcgggcaggtgaagttaaagagtttttcgagtggtggcatatagcccacagacacatcgttaaacgtacaccacttcgcagatatctccagcatagagccaacaacagtgtcagccaaacgcaggtatgattgtttgaagtggtagctgtgttcgataggagcaacgctatcaatcgttaactcagtaccatacaccgctttataaattaggcagaaacgtctgcgtccccgaggggcattcggtatttcatacaatacatcatgtatgagagatgaaacgtccccagagaggacgtttttcttgacaactagtgccgtcatgctgggaggtaaccgaagtacagcagagtgtgcgtgtcgaacttatagttcaggctgaacgcattcaacgagttgatgctgctaccgtgaaagcccatgttgtgtcgttcttcacgcccaatgttacgcagcaactcacggatgatacgcatgtcgagagaggtggtgaactccttctcaatcggcttcgccagtttcaggctgtcctgtacgctaccgctatcattaccaaacttgagtcggaactcttgtttcttaacatgcagcttcgcgttcgtgttgcctttcttctcaatcagcgtcgagatgttagcaaacggtgcagacaggtcacctttgattacgcaacccagaataggtttacctagctgtgcaatcatgttgtccatatagcgatagtcttcatcgctcgcctgaatcggaggcagagtcagaacgaacgattcggcttcggcagcaaacgatgtgctgtcaacatggaacgttaccttttcttcgccgcagaagcggtagacaaggtcgaacatctcacctgtcatgctgaaacggaacgcaggcactttcttctttaactcgaaacgataacgagatgaagtccagtgtccaggactgactaagctaaggctcttaccgtcgcagataacacgacacataacagtctgtcctgtgatggtatctttcagacgagtcagcttgacgccttgagtcatcgcgtcgattacttcacgcgtcatctcatgaccaccttcgatgtggtgatgcagaccctgttcaaccatcggaatctgttcggcagatactggacgcagtttcacttctgctttgtatttgcctttctgctcgctgatgttcaagactttaccatcgaactcaacgctcagttccttacgcttgttaatcagacccgtcaactgaatcgggtcgatgttcatgattgtatcagcgtcagcagttgcaccaggaacaaggtacgctacgaacgtgtcaggcgtacggcccagcacgaacacgtcagacttatacgttaccagcagatggatatgcgtcaacttatcgtccgactcagagaagcgcgtcacgaggtcaacacgtttcagaatatccgacaggaacgtaccgttcaatgtcaggttgcacttcttagcgggattcttcggcagtcggcaagtcttcatctctatcctctaaaacaaattgtagtgtgccctgtatatttacagcttcaaggcgcttacctgttggcataagcagaccgtttaacaggccaacgaagtcagcgctgtagcagtctggagcgatctggtggacgtagatatcgtcaggaacatcctgaggattaagctgccaagcagtacgcaaggcagctcccatgaaagcaggacgctcgaccagatgcctgttcagaaacgaacaaatatcttcggcgcttaacgtcatttcttgctgatccccttaattgcgttcttgagaagggacttgctgattttgattttcttcggagcactttcaccagcagaggctgctgctttcttagcttcctcttctgctttatatttctcgaaggtcttggtgttcttaggaagctcggcaagccattctttgacgttcttcttatccttgttggtaagaggattgactttgtccatcgaccgaatcttaatgtcgttggcccaaagctgtttcttcatccaatcggacataaggtgatactggtcctgcaggatgctgtcaacagtcttgtcaacatcaaggtccttctcaccaagctcgtcacgtttaatgatcaagccgtctttgataagtttgtggagctgaacataagagaagttccagccctgcacatctttctcggacgcaccaatctcaaagtcaatctcaggaacggacgtgaactcaaacccttcatgacgcttctgcacaacttcgaccactgcgctggtcatcgcacgttcgatcatatcgagtgcaaggaagatccatttgtaatcgcagtctacggtcaaggagtcgtgtacagatacgttcatgtcgaagtcaggatagtcgccattagctctccagtattcaaacttcatgcggtccagaatacgaatcgcggacatcatcaagtcagagccgaagccctgtactggactgttcaccgcacgacggtcacaagcggcatgaaccatgttcgcttctttgtgtgactcaggcagcatcaagccccatagatgacgacgacgaccaactggagattcaacatagaagttctcgtgtgcaaacttcttgattttgtcgaaccattttaagccaacagggaaacgtgttaagaacttgcctttgatctcggcaatctctttcacgtcacgaccagtagacttcgcaagacctttatcaccctgctgatagatcagtccgaagataactgtcttaaccgcgttacgtacggacttggttacatccattacgtttggaataccgaagaagtatgcggcgttgattttgtggacgtcaccctctgcttcgacgcggtgttcaatccacggatctggcacagtacggtaacgatgacgcagcgttcgaccctgttcgaatacgtctgctacgccttggtcgccagagatgatcgaccagccccttacttcgtgggctgagtagtcgaccttgatcagtaagcgatttcgacgtgcaatcaagatacgcttgatcagtttacccatctcactacgcgatggaacttgctggagattggggtcagacgctgaggtacgacccgttacaaccccaagataaccatacgtcggtcggattgatctatcgtgtttgaagtcttccgattcgccccagagtttaagcaggctgttaacgtaggcgttcttgagcttgtacgcctttccgagtttcgagtagagagcaacaagcggtatatctgcatacgccgcctggaagtccttgtccagcttgcctgtcttcttaccgttctcacgtaactgttccccttctttcagaggcttgagtttcatcacgtcgaagaacaggatttgtttatgctccgacttcgacatatcaaacttcgttacctcaacgcgtcccataagacccatcttaggaacgttatcgtcttggcatatcagtttgttcgcagccttgacctcagggctgttcatgaactcacgctctacgtttcgaatctcctcgttaatcggggagttcggtaagttgagcttaaacaggtagtcgatatcagcgccagcgcctgttgtctccagaatcgagaacgcatgaatctggtcggagatttgttcactgaccatagactcatacttggcgtacttgatatcgttcgcacgaagcatctgcttctctgctatacggaaaggtacgataacgtcgagacccgcgtattcttgaacactctcgtccaagtcaacatcggcaatcgttgctcgcatctccttaccgaacgatacttcatgatacacctgacagccatactgcattgtcaggttcgctaagttgtagtaaccagcgccagtaacgttaagcaatgacttcgcgttttcatcgttcgcaaattcacctgcctgaatatcccagacgttcgctgcataactacgaatgccgaagttggagcgcattacgttcaggtcgaacttcgcgttggtatagatctgatacttgttggagttatcctcgaagtagtctttcaacatcgagctgactttacgcaactctttaggagtaaacgggctgtcgcggtgatagattggaatgacatacgccttcttgccgtcacaggaaagctgtaccgtcagaatcttattcttgatacgattcaggttctctgtttcggtatcgactgcaaccttcttggcgcgcttcatacgcttcaagattttctcaagttgcttgaccttagttacatacacaaggtcccagttacgcttcttaccgcacgtaacctcgtcgatcttataacgcattcccttgttcaaccaaggcaacatccaacgtgccatgtagcctaacgtgtacgatgaccctttgatgtgcattggattcaatacggtatgatagctcacgttcggcagatggatgaagctgtgcttcttaccatcactcttaaccttggtgggaatctcgacaccgtaccaatgctcgtagtggtctttcgagaattgaatcttctcgttgttcagcgccttgaacggtgccttaccgaacgtcaaaacatagtcaggcttatagctgactatgatctcacgaatacgttcggcgaatgctgcgtcagcgtcttccttaaactgctcacccttatcataggttttgaacatgttatacgagataacaaggaagctccagtcgtcgagagtggtcttgaccggaaacgtatcttcaagatactgcatctggttcagaaacaactcaccttcggttgaagtaaagatcttaccgctgcgcaagtcttctgtaggcatatgatcgaggacgagtagtgctttaccgcctttagcgcttttacttacgcttttcagaagtcgaacaccgtcataggtctgcgtgtctgcaaactgctctggcgggtcgaagtcaagagctataaacttgggtttgttcaccatctagtcctatcaaagtgtgtatcacaatatgatggcagttatttacagatttagaaatgaaaaagggcaccctaaggcaccctttttgtctagttatgctcggcgttgccgacgctggatatcggatcgttcctcagaacgagcatcagcagcgccgcgtttggctacgtcagtatgatcggcaatgaaagatgcgatgcctttcttatcagtgatagcaaacgattgaattttaggatttggatggaacttaccgctacttgcgatacgccagctatctccgatagattcaatgcggaaggttacgaaattaccacgattgagcacgaagtagtcagcagactcattcgaaattttgaagccagtgcgcttaatccctgtgtctgcaaagaataagtcagacattttgccctgacgttttcctttagacgtccgtgcttcttttttagtggcggacttaccgataacgtccttgacagccttagcgagagcagcagccgtaggagacttcagttcgttgcctacgtagataccacctctgctatctaccgcagacactgcccatttaattgagcgcatctgagagtggaacgcataaggcgggtcaatagacacgctcttgtaccctgctttaggattagttgcttcgaagacccacggactagactgaccgttagtctcctggtagatgggcaggaatttcaggcctgtagctttcgacaactgatcggcaatggcgtcagtttgtgcctgggtgactgtcttcatgaacgcaggagtaatgcgcgccagatcgactttaggcagttctgcgttttgattgacgcgggtcgccacaactctggcagacttgatacctatatcaccttttgtcttagcgacaggctcaggcttaacgtctactttagccgcagcatttggtgcagtcactttgactttgattgcacgtaggccgttgatggtagctaccagagtcttcgccttgaacaagtttttaatcgcagtgactgcgttcttgcctgctgctttcttggcgaaggccgtcgtcgcttctgtgtctttcagaatgtctagaacggcttcgagcttagacgtgtccagctctttgatcttcgtcagctcgtcgatacgcttgatcaacactttggcgttcttaccaaagagaatctctgcgttagtggcctgagctttagtcacagcggatagtgataccactgaaccgttgttcatcgtcatgttgtacattgctgttccttatcgcttcttggtccagttggagttctgtttgccctgctgctgcgtgttctgcgtgggctgttctgtgttttccatttcttcttctgtctcaatgtcatcttcttcctcgtcgatgactggcttcgcttctggcgctggtgcctgcgtctgcgtgttgagcgatgttgcatttagaggtgctgcctgcaacgtatttacagtagctacgggctcctgcacggcaaccttgcgcgcctgagcaacttcacctactgcgtgttcgtggaccagatcgacagtcacgagctgacctttctctttcaagatttcatcagctcgtgcttggtcccattgatcccaaagaatgtccagacctttgtgcatgtagttcatacccttcggcagcttaccgcggccgttgaaaggcaggccgttcgaaggagtagctggctcaaactcgtccatcatctcccacttacgtttcgcttcaatacacttcggtccccatacaccgtcacacaaaccatcatagagtcccatcatggtcatgatcagctggagcttttggtagaacttgtttagcattgtcgttctcctaagagaaaggggccgaagcccctagtctaattacactgccttgtttttggtagtggtgagtttcagacggtcaagcgccgtcgtcactttcttgatgttcgtgatattgtaaccagctttcacgatcttgttgatacgtgctttagcgccagcgacattcttcacgaaaccaatccacatgccaggtgaggagtcgaaagtaccaaacttacgagtgtttggaatcttcgtaccgatgaagcgtttcatctgcgggttcgtgttcaggtcgaacatgatacgcagacgatcttccatcaccatcgggtatgccttgacgtgtttcttatcggaggctgccttgtgacgaatcaggaagaactgcttcaactgctcttgagctttcaacgccagtttgatgttgaagcccatacgcggcgtagactcgtcgaagaagtccagcacgaactccaagcgcttctcagaaggcttgtcgaacaccagtttcttcttaacctctatgaagtcgagcatcttctcgaagtctgcatagtaggcacagtcgtaatacacgtagtcaccaaactccacgaagtcgaatgctttgagggctttcgcgtcagggtcggtggcgttcgcgtaaagagccacgaagccgttgtatacggtaggagtcaattcgagctccatgtccgcaccagttgcgtcttcaacagcggcagcaacaggtttcttacgacgggttgtgttatccagcgcaggcagatcagcaggcttacgacgacgaacacgaccagcagcctcagcaacaccttcgttgattggcttaccttctgccttgttctcggtacgtttcttggcgcgagcggtcttacgcgctacggccacaaccttcttctctgtctcaaccgtatcggcagtctcagtctcgtcctgaatggtgtcttcaacttcaacacgattcgcttcggctgtagcacgtttgcgatctttttcattcgcccacggcttacgagtctcgaagaacttcttgagatcagacttatcaactttcgttgcgatgtgaaccttagacgcagggaagctgacggtctcgcctgtaccagccagacgcacacgcacggtactgattggactgtctgcacggagtttaccgtcaacagtacgcacagtcacagacactacaacaccattgccgtattcagtcacgacaggtgcacgggccagagagtctttcaggccttcgccgcttgtgaagttacggttacgcgcccagtcaagcagacgttcaaggccccagccgtagcggtcaggaatcttctggttagcaacaaacggagtttgctccataacacggaagtcgttcagagcaggcgtggacggcagtgcttgcattgctgcaatcgtcgtcttacgcatctcttggaactcctgagactcgatatcgttcagctcacgtttcgcaatgaagtaatctgcgaagtccgccattgtgttgttatcaatcaggagcttggcgctcattttgattgggtccaacttgaactgatcgagtgcttcgtaacgctggttgcccttctcgtcgaagcgcgttttctccagtgtcttccacatcagacgagcgaccttaccaacttcaagggtcttgttcgtcatcacccagtcgatgaacacaacttcacgggccatgtcacctggcttaccgttctcgtcgagttttgcagcagcaacatcaggacggaagatacgcgcagtagactggtcgtaagtacctggtgaccacggagtatcgcagcggatgatacggctacccatctgcatgttgtggccttcggagattgcctgttcgttcgcaatcagaatctggacgttgttgtccgttttgaatgcgtcgaggttagcgtctttgttttgccccagcttaccaacttcaccgtgatagactacagcgactttcttgtagttctcaggcagagcgttgtagatagcgttagcggagcggacatagcgcgtgaagacaatcagtttaccctgcacctctggtttccagtagtctggatcatctggtggaggcgtcattgaaggaggcagcgcttgacgcttgaactcttcggactgcttacgtgccagatacttctgaccgttgtagacagcaatgtccagttcacgaggagtaacgcctggcttccagtcgaagatctgctgttcaccaaccatctggtcacgctcaggctgcacttcgaagtgcttcttgatgcggtcgatgatcgtcatgactttagcagaagtgaagctggtaacgccagcggcttcaaacgtcatacgtgcaacgtcatcacccattgggtcagtcaacatcatttccatacgctggaagtacatgttcagatcggcgttacctgcaagcagcgcacccaggtcatcgccttcttcgatatcgtcttcgtcaatgtcggaagcggcatcgttatcaccaccagcatcttcgtcgtcgtcatcgttggacgcagaggctttgcgtttcgcagcgttagcagcttcctgcaatttctccagcacctgctcatacatcgcgctgtacacttcaaggtgtaggcccgagtttggaacagatgggtcatcgatctcaacctgaatgaaggtatcaatcgggttaggcagcatgaacgcccagtgcttacgcttgaacgagatgaacgcagtgtggttcgccatacgagagtgagcgcgacgaatcatttcgatatcgtccttcgcaccatcgtaggccacgtcaaggttatcaccaaacatagctggtgtcatcaacgcagcctgacctacgatatcacgcacacggtctgttaccagagtacctgtagcgatacgagcatagcgaacggatggggcggtgaacactgctttggtgttgaagtgcacctgagaaccagcctgaccaccagagaagttcttcaccttgtgcgattcatcgagcagcacatagctgaaacggaagcggttgacgaactccacagcaccacgaatacgaacgcgcacaccgccaatatcaacgttgaacgtaccagtctgcaagaagctcaagcccacgatgtagatcgtgttgcgaggagcctgctggataacgtcatacatgcggtcttcgccccacgtgttaacagtgtcagcagtaataggtactgcgttccagccgtcaacgattttgtggaggtcatcacaccagtttgccactaggttagatgggcagatgatcagaggacgaattgtttcttcacccaggtcatccagctctttaatcagagcagcaacgtcagacagaccgatgatagtcttaccaccgccaggcgcgataaagatagtcgcaaagcgaggacggcgacgcagagttttatgcgcttcaacctgatgtggaagtaacgcagcaccatcacgtaaacctgggatacggatatcgtcaatcgtgataccgctgtccggtttcagtttctcaatctccacctcagcctgttcgaagtattcgagagacttaggaatcacttcgctgtacagcgcggcgaatggcagaatgatctgctgcaaacggtcagagccaggagccgtgtcgctttcaatcagagagctaaacagcttcttacgatcagacttagtgatcgcattggccatttcacggtagactgcaccaccaaagtagttgttcagtcgggccatgtcagccagcttcgacgtttcacccatcacgaagtagtgagtgtgtgacggcagcgattctgttgcagcctgaatgcttcccatctcggtgagagaagtagagatcaggttagaaccgcgcagaccagcagcatcgttcagtacgcgaatcatgatacgcatcatggtcagtgctggacgctcttccgcaatctcagggatcgagaagtcgttctcaatcaggttctgatacaggttctggtccattggactttctgccaatgaagcgttctccgcatccataccgattgcaacacgcgcgttctgaatcagcgtcttcatgtcaggaacttgtttgttcttgagcatgaactcatacgtctgacaagtagacgcaatgatctgaatcagttcgtgaaggtttgaaccttcggtgctgttgtacttgatagtgctgtcagaaacagcttctaccaaacgacctgcaccagactcagcttttgccgcctcaatcatcatgtcgttagacgtgcgataggcaggcatcatgccggaggactggttcttatggatgttaccgatcacgttcgacacagagcgatagttcggtgcttcaccaggctctgcaaagtcataacccaatgagtcagcaacgtccagagatgtaggagatttcataccaacggtacgagtctctttaacatcaaggccgccaccattcgaagtgttaacgatcagcgcgaagtctgggtcgataccaatacacacgttgctgaaacgattcagggttttagctttagcctgaatatcgcggtcgaagtccagattgccgttctgaatagcgaatatgctggtgcgcagtgtatcgtggtcagtagacagcggcacacctttctcaaacaggctctccagcacatcgttcagcgtagtctcgtagttacggaccatctcaacgtcaatatcttcacggcggggcaacacagcgagagtaccgttcggcatgatcgtcagaccgttgtcatcagcaacaacgtcattaactacataaccaaacttctcacggagtttcttcaactcaggcagagttgtggccgaggtgacgtaacgtggaatacgcgcagcacgagtgatacctgtacgggtcgaaccagcaacacggaagtagtagctcgcccagccttggaaccaacgatacagacacatggtctgcgtgtcagcgccctgagagatatactccaccagctctttttcgaagttaacgatcaacccagcttcaacacgaacgtcgatagcgagagcaacatcgttaaagtcaacaggagtgtcgtgactgatcttcatcgcctggagcttgcgctcaatcattgccttgcctggcacaggacgaataccgatagtcatgaagtcgcccagcgcttctgaggcagacttatccagattacggaacaagtcaatgtcgatgccgttcatcgcagggtgaatagagcgtagtgctgcgttataaacagaccagtctttatcgagagagatacggaccatcttcgtatcaaagacattgccgttggagcgctctacgccgaagatatctttgtacagagtcttcgccacacgaatcgcagactgagcgatctcggagctgtatgtacgcagattggcgctttcgaagctcgcatcgttatcaacgcgaggacggtcgctaccctgattgttcaggacgttgaagttaccgtgcgcggccagttggctggtaggaacaggcgtaccagccatgacgatatctttaccgccaggatagcgcgtactgttttcaacgatagcgccagacgaggcagacagatgctcggcgagtgaggtcttaatctcacggctcagcttatctccgttcagcgtcatgttaatgcgcatggtcgccagatcgatgttcgccttgatacgcttggtaaactcctcaggagcaacttccagcatatcttcgaactctgcaccgttgacgacgatgtagctgatcaggtcaaaggctgcgtataagcgagcgacggtcgacgcggtgaatactgcaagggtttcgtagttacgacgagacttccctgtagcatacatcttcgacattttaccatcgaacgcgggcggcaacgcacggatagcaagcgcctggttaaaggtgtcggcgatctgctgggttgcggttgctgaggtactgatcatttgattcatcattcacccagtttactatagttgtcgattacagacgtccacaccgcaggtacaggcaggcgtcggtccgcagcaatatcagaaagcacgatggccagcgcataagcacgaagtggtttcaatccctcaaacttatcgcgggtgaacaccgaagtcagttgctcattggtcaacgtctgatactgcgctctgtattcagtcaggtaggtgcgatacttaccgtcgtcaacaggcgtggtgtcaggagtgttttgcacatagagcagcgctttccccaacgcatccataatcagcagcaggtctgcttgatcgtacggcgtgatatcaggaacgttagaagtgccgagcagttcaatgactgactcaggcaattggataggctcttgggcctcagatatggactcaataatcccctgcgcagcacccgcatagctctttccgcttaacgagatacttgacagtaaggaatggagccgcgtatttacgtcgtgcgtcacggttcttctcctagataaaaatgctcttgaccagagagttgagtttcttttccacagcatgtttcttgtgcgtggtcaggaagctgcacaggcgacgggactgtagatgcagagcaatagcattgcccttgacgcgcatacaatcaacacccagatcaatattccacggatgccaagcacggggtgcaagcatcgcctgttggatatttggataagtgtccatcacaacgggtatcgcagacttcgccagtttcttggtcaaattatcagttttgaacaaagccttaggctgtttgttcgaaaaccagtaaggaatctgcttgtgaagcaactcgccaactttcggaataccactacgagtagtctgaggtacatagaccaaatagatatcgatcgtggtattgatgcagttcgcaacacgattataatcgctggtggtccgtgaatgaacttcggcgagtttgaacttattggtgaactcaatgcgttgtaaccactgacgcaagtcctgttgttgcagacggagcagagcgcgggccgtctcaagagaatgcttagtcacagaaggaataggacggagcagatacttagtgctcgtcttcgccagcgaggacatgaaaccttcaacaacacgctgcatgcccaaaggctgaggcagcgaatggaataaatcgactgcggtctgtgttgttatgaacgcaccccacgcttcgatgtactctgggctaacgcaatcagggaacgcacgtaggttcagtcctacttcggagccatagcgtttcaaacgactcactttctacctccgtgcagcagtctggaacctctgcggttcgcagtgcctatctgattattatcgcacacatagcatagcagttcaagattgtgcttcatgttagaaccaccattagcgtgtgcaattttatggttgagtataagctctcgcgtaggcttaccacaacgttcgcagtaatagccacgctcgtcgatgatactcattttgagcttggtccattctgctcgatccatacggacgtgagtgcctgcgcgggcacgttcaaatccagttactccagcaagacgctgagaggtagacagactccgcccacgtcctccttgtgctcttgctgcaataccacctctaggtctgtatgccatgtgcctattctcctaaatacaatgatatttacagacttacgcagaggcggagaagatctgtaccgtcttatccagtccagcttgatacgattgctccacgtcttttgcagcacgtcgaatgatgttctgcgtagagttctgggcagcagagataagctcaacaggcaggttctttttgttccaggcattaatctggtggaacacgccaacaagaatcgtaccagcagattcggcgaacgggccaagtacctctgcgttaagaatctcacccaactggccaacgtcacgcagcgcacgtaggtctgcaatgatctcacgcatctggttatacagttgcataagcgcgtagatatcacggctctgtttcttgtctcggtaggcaccttcgcatagacgcgccatgttctgacattgcttgaacatggtcatgtactctgcaatctggtcgttctcttgtttgatgacgtcagggatttcatccatgacttccatcaactgcccttcgagaacagccacatcggtaatgcctttcttaatcttatccttcttggacttcttcttgattgtatcggcagcgttttctttcttctttttcttcttcggcttttcgtcgatagaagatattgccttttgggtactggcgatatctgcgtaaagttcttctgggttaagaacacctggcatgatatctttcgaagggtctttcttctttttctttttgactttcacgcctttgctaactgtcttagctttaacagcggtagtcttagctttcactttcgctttgcctttctttgtaggctgtgcgtaagagccaatgtcatccaagcttatggctgccatgtgaaaatcctctgtagaaacgaaaaagggaaccccgcgaggctccctttagggtttgattagaagctgtgacctttgatgataccagcgatcttgctgtagtagtccgggctgtagcggaacacttgagcatagtagctcaacagcttaggtacgtcaacgccagcagcggcagacacgctatcaacggcagggaattggttcgggtccagttcgtcgccagacagaacagcaaccatagacatggagctaatctgttcttcgttgccttcctgatcaaccaccagcatggtgttgtcatcggtaacgttagcagcaacgaaaccgatcttcaacgcgcctgagttagacacgaagctgaccatatcgccgcctacagcagccgccagaaccgcttcattgcgcaggatagcctgagccaattcaggacgctgagccgagaagttaacagtcgatgcaccgctgacagaacgaatcatgtcaatcagttcagcgttgtcattggcggagctgtcacgcaccagaacgtcttcaccggattcagatttacgcacatgccacatgcgctcgctctggtccatgtacatgttcttagacagtgcctggaactgatcgcccatctgagacacagggatgatatcctgcatacggctcatgatagtacgcacgaagctggtggtcttaccgccttcgatcagagtggatgcaccgtcgactggaagatattcgcggttgcaggatgcacttacgattgcgccgaagttatcagcgatgttctcaccctgtgcgtgggttaactgtacgatggcaacgctctgagtgtcgttgacctgatcgatctgtttaatgaaagccttcattgtcatctcctgaatatttcgacaatatgaaattagtatacttagggttagccagtgacgcgataacgtgcattgacccagatactgcggttaccaacagtagcccatttggtggttgggctgtttgtgatgccgagcttgccgagtgaacgtgcaccgtcaatcgcattggcaccctgagaaccatcaccgtcgtttattccagctttagacagtttgttcttcaagttcgtaacaggaccttgaatctccgtttcgagtttgcctaaagcagactcgatagacggcgtacggtccatgtttaagttaaccacctgaccggtgaagtcaaatgccaactgaccttctgcctgcagttgagccgcaagcgcgtagtacgaagcgcagataacccaaccattaaggatggtgccctgcatattcgtgccgttgaaacccgtcacacgaggaccaatcgtgttgaacagcgcaagcccacgatagagatagttgatgatctctgcctgagtatattccaactcagggataacgttcatcgcacgggctttgttaatgtggtcttctaccatagatgctgcgatcagaatctgcggtgtaacaacccagagcttgtacgtgaacatcttcgtggtcttacgagtgttcgatgtgtgctgtgcgattaagctgataggctccagtcgtctgactgctacccacacaggaatctgaaacacacaagtcttggcgcggttcacaaccatcttcacaccagaatcaccgccgtcgatatccgaagcaatgatttggttgttgagtgcaagttggaatctcagcttatcgccacgcgtgtcgaagtgaaacggcaacgtcatctcaaacgtttcgtcatcaccgaacaggcacacgatatctgtcacgcggttctctgtcataggctcaacaatgagttcctgacgagactgcatgattccttcttccgactcatagcgccatgagagcagcaaacgtttatcgtccaccagccccatgttaggaacagcaacatcagcagtccatgcgcccgggatttccccaggcgtagcgactacctgtgccagaatcgatctatcatcaggatcaatgaggcttacgacaggccccatgtcatctgatagcgggtacagtggttcgtctaggtcgttatagaaactttcctcgactaccagtacgttaccttctgttgtgcgcatatcagtctgccttagtgagtcccagatactcaatcagattgcgtagctggtcgttatacccaccttcgattagcgctctcgccattgatacgtggttggagttcgctgtacgcactaccttagcctgatagtcaggaacgttttgcatgttctgattcaggttgtagaagtagctgcgcacgaagttcgttcgctccacgttactcgcttccatgtcgctggtgtcctgtgtaggtgtcagcaacaggtagagggcggcaagcagttcaggagactgatcgaccatcggagaggcaagcgaagcagcgagcttcatcaggcccttcgatacgaagtcaacaacagtcttctcaatatacgccgtgcccgctttacctacgttaggcagatacaggccaggcaggatgtagatgcagaagtacagcgggaagtctttacgcatcacgtcagagataagcatctctgagtagtccttccagatgttcacgttgaagtgccattcgtcgtaaggcacagtgcgcattaagttagacacggacaggtctttcacttggttcgcctgcgatgcaagatcgcgagcgctctgcgaaggagtcagtgacgaactagataccagctggacgtagttgcgagtgactgcgcctacagtgttgtagactacgttcaacatttcaacgccgttaccgttcaggccgaagataacagaacgaggaagaccgatggtgatgtactcgttgttattgtccacgccccacaagcgccagtaacgcccgcgtccaagttgagtcataggctgcgggagaatacggttagcgcgaggtttcaggcagaacgtgaaacagataccgctgtcaatcatgatcactgaatcatcaggacgattcgaataacccatcgacatatcgttgtcggtactgtacacgttcaccagagtgaagttcagagccttagtgaaaggcatctgcgcttcaatcaaatagccgaggacttgtcgcaggatagtatcgagcacatatggagtagcagaacgcatttgctgcggacgatactgcccgctgtatgtgttctctttgaatgtgcgatctaccttgaagtgcgtcaacgccattacttaaccgattgcttgagcaaacgtttctgcgcagggttcaggcccatcacgtctgcgatttcatcaatcttacgcagagtcagaacgcccttagcagtaccacctgaacctgtcaggctgatcttaacaagctcgcgcccgctacgaccacgaacgacctgatggataacgctgttcttaccaccacgccccgcacgaagtacggtagatgccatgcccaggatttcagtgatagcttctttcttctcggtagggctaaggccaggcaccagacgaacgtacaggctatcgttctgcacacgcacgttgtcgaagatctctttcttacgaccacgaatatcgtgttgagcattacccagttgcgtagtgtcgcgcaggttctgagtagagcggttgattggcttgcgttcgctgtagttcaggaagccgtcaacagccatgagctggttgatagtacgcttcatttctggagcagtagcaatcagacggcccatagggaaactacccggaaccttctcgtcaacgagtgacgtaaggaagttttcgctaatgccgcttgccaccgcgatcgtggtagacagcaccattgcgtagttcggatagtgcaggccttctgagttcacgaagttatcaatgaacacataggtctggaagcagatagggtccgtgccagacgcgatgaaggtacgtgtacgaatcttcgaatagtcttctttattcagaatcttcgacaggtagttggcgatggttgcagccagcttggtatgttctttaggagcgccgttcttaacgtcgatgctcataagtttaaccagacgttgctgctgggtcttcgcctgttcgatgacacttaacagagacttcgcggctgcgttctgatctttgaatgcgctgaaagtcttgctgctaagaatctggtaggctactgccagttcaccaattgcttggctcagttggctcacctgattgttatactgcgctttactgcggacgtcagtgatatcaatcttagacaggtcgataacctgattcaggtcaatcgctttggcctgtttacctttgattgaaccttcgagatcagccagctcaacagctttagggctggcgctgaccgacagaagtttctttggaatagtgactgaggtggctttagcgataactttgtcgagtacgttacggaactctttcgctgtacgcgcaccacgtaacgcagtcatattcccagagctatagtcaacagatgcgctgatgctgctaacttcattgtttttggcagtcttagccatgatcatcctctactgggtctagtattcatgtcgagtaaaaattagcgactaaggtcagttttacccaacatagttctcgtatagactttacaaattttgggctgtagaatacaaaaaggggcagccgaagccacccctttttgtttgtgtatcgtaataccgaccaggtcgattaaacgatcactttaccttttttcttggtcttagcagctttcttaccagctactttctgagccgcggtgccggtgtgcttaacggctttagcagtagtctgcttaccgcctttcaggcgcggcagtggtttcagcttaggcttaaccagagttactgctttcggctgtacttttggagttaccagcttgccgtctttaacggtaggcttacgcgctttacgtgcggccatacgcgctttctgttttgcgatcaggtttttgtagccagctttctgtttggcggccaggttgctctgagcaactttctgacgggccagcagcagcttgcgaactttgtcctgagaaactttggtagctttcaggccagcctgatacttagccagacgctctttcagacgctgctcgatagacttcgctttacctttcttagcctgcttacgcaggtgattagcacgttcgttgtcgaacttcttctcggaagaggtacgcgcagccttcttcgctttggctggcttggcggccgcaggagctttagcagcttttgctttcttcgcttttgcaggtttagcagcggctggcttggcagcttttgcttttttagctttaggcgctttcgcagccgcaggctttttggtcatctttggatctttggtgcttttcagtttgcgttttacggccatgattatatcctcaagttacaattgaactttcgtccttcgggacattaaagtttttgaaatcagcatgtaaaaattagtataatctctccaggattcctgaggaaatttcctaaacatttttacatagcagtataccctatttcagataacaccgcgttaagttctttgcgagcacttatccgcaaagactttttaattccagacgccttaaggtaatccttgaggccatcacgtgggtcaatatccgcaagcgccagctcactaacatcaactgtatctatattatcgagatcgacacgtttattcgtggaattaatttgggaaatatttgggacgcgagtacggatatccgctgggatcgacacggtatcttttacgatgacacgataacggatcgctgggtttacttcaaggcgtgaccaatccttttgattttcaatcataactgtttctaatctaaacccaggcttactgtcaacgaacttccgctgaaccaccagctcgcctttcttatacttggcacgaatgtggatgaatcctttcggcaacgcttcaccaaacgttttctggtagggcgagccgcaatactcgaagcgtttcttctccagcacttgagccagatggatgtgaccactgattgtatagtcacgtgggtcaaccttgatatcgtgcttcgctttaagagggcgtccgttatctcccaatgcacccacagcttctacgtgacagaagttgaggcagggcttcttgtgtttaatgctctccttcgcagggtgtgctaggaagttcacaactataccatcaatctctacttgctcggggcgtagatagatatgcaacgatttgaggaagtcccactcacagaatgttttgataaggtccatgctggtattagacatatcagcccaatcatggttgccgccacagtaccatgtgtcgataacatcttcgtacttgaggaagaactggagcagcttgcgctttgtctcgtcgtccatcttgaacttgtcagtgatatccccaggaacaaagatgtgacgtatgccttgctcaacagcgtattgatagatgcggtcgatcgtttctagttgacggtcaacgtggtcgacagggaaatgattcgctagtccttcgaagtgccagtcagcagtcactaaggcttcaaggaaggccgctactttgttctttttcattagtgtaatccgcaggtttcaatgtctgctatttacagaaaaatgggcaacccggaggccgcccatgtggtttatttctttctttctttctgcaaccatgggctgtattgcgagtctttcgactccagcaggctttcgagttcttcaacgttgatattgtgtttcttggcagcagttgcgctcaggtagtgagtcttgtcagtggtctggtcaaagaaagtcataccacctttcttgtccataggaccatacgccatagtcttcaaacgagatggtttgaagtcgtcgcccatgaacgctttcaggcctttcatgttcttagcgttctctttcttccgtgccgctttcagcacagcaatcatttcatcagcactaggtttcaccttagtgaaacggttcgcacgttgtgattcaagctctttggctttagcaggagtcttcgcaccagtcactgcacctttacgtttggcagcaatttttgcttcaactttctttacgccacgcttgacagcctctgcgtgacttggcttcttaccgctactggcaagaattttggcaacgtcaccgaacttaggcttaaaggtgcctttcttgcctttgatacgaacctggtcaacttgcgcagcgttaactgtgcgcagcgaacggcccggaccagtagtcagagtgatcgcagacgcaggaagcgcaagtgctagagaagacaatcctgctttacgcagagaagcggcagcagtacgcagcaactcttttgcctctttggcctcagcgcttgctttggctttcagagtcttgtacttggtgaccagctttgtcttagcagcaccctctgcacgggaagcctgactatgggctgtagtagaatcaattttcgctttaagcgcaccagcagcaagtttcttcgctttcttagccgaagacagagcagcagccacggtagctttgtgagacttgtcgatgacaagcgtagtagcaccgctgacctgagcaaagatatgcgcaggtgtcttagcggctgattcagaaacgatattgctaccgtcgagttttaaacgaatgagtgccatggtatgcctctaatgaatgagtatgctgtgactgaaaaattagcgactaccttcttttggtgtggtcttgatacgcattaaatcgtagccaatcattccacaaataagtcacaggtttagagtttctcagtgcgtagtcgatacagttctgtgtaccagacggtgcaccgcagcagagtgcgactagacggtcagtgttatctaccatgaagtgattgcgcttgttcaacgcaaacccagcttgaccgtccatgtgaacccaatcttctttcgaagtaacaatatggacttcgtggctcttgttcaacagaccgtcaagttcaaatacactcgatatcttccacagtttgttaaagccaggaaaaggaagacaggacacgactctgtgtccttgctcaatagcagcggtggcgatagccatgtcaaaccctagagcgcagcccacccatatttcggtgtctgtctcaaggcgcagcaatcgtctatgagcaaaagtatagaggcgacgttttgcctcagggctaaagccacctagatactgtgggcgatgaccggtaaaggatagtttctccatgcagtatatttacagatactacaggttagtgatgaagcctgcgttgaaggcgaaacttggtttagttccaggtactagaggactattagattgacctgaaactagaatttcattggcaacaaacttaatcaacataccatctacaggacttgtaatcgcatcagtcattgtaggagtttcatctgagcccacgttgtctatcatcatagtaacttctgcggcacgttgtataaatgctccgccatatccaggctgagtgtgtccagatgcgtagaagcctgtgatgattgtttgatcagtacctccagaaagattcagtgcctgtgtaggtctgttgaatgtacgtccctcatattgagaaggtgcgccggaatagactgtgtagttttgtggagtacctgaaccccgcataacagtcatgttgatgaaactgtcgccgggtctgtatgcaccaagctgaccaaattcaggataagtaacatcaatagatgtggtttcatttgtgtgcaacgcacttggcaccattgaacaaacgtttgggctgtatggcaatacatagtcagcactgagagaacctgaactgatattgtttgcgcccgtctgaggactatctatcttagcagcaaaggtagtgcctcctaagtatttaaagttggtgcagtaatacttgttgctcttgcgtccggaaacgacattaacaatcccttttcctacaatacctcgggccttaggtgcaaccgttttaagcgttgtcctatctacaatgctatcaatatcaacaccatcagctctatcgaacagaaagatttcaggaaagatatcagtcacagcaagatgatttgcagttgagataaattgcataagatattccttattagtcaggtcagggcctgcgtgaaacgcaagctcactgaactttggtgggagcacatccatgtgctatgtaagtgttatgctactacttcgagatcgtgatcacctgagctccaaatgagttcacgaatgttgcgtggcataatgatgcagccacttgatgcagtgccaggagctttgatgctatcgccatgaatctggaaagacgagcgactgaacatcacgttgtctttgttcggatcgagaggcatagcatacggacctgtcttagcacttgtacgaggcgaagtgataacgtacttacctacaggtagaggacctacgcctacaagattctgatcagcgtgtttattcttgtgctcacctttaccagcatagcctgtagcaatgagtctacctgtcttgtcatacatacggccagttgattgttcatatttccacataagtattgcctctacgttggagaaaaacaaaagggcctacacccctcgatgcaagcccctttcttataaaatgattgtcacgaactcgttgcgattcttcttagggttaaaccatacttcatctatgatctttcccataccgaagttgatcatgcacacagtgcgtctactgactaactgccaatgctttttacgatcaaacatcactggtccttaatcattttgacgcgcgtatgatcgaaaatgccgaatgtaggcacgtcatggttttgaccttcattgcctttgattgagtcataaccagcaaggttcagtatcttactgatctcggtgtactcgtcccaccacatgtagacgcgtttgtgcttactggagggaacgagtttgttcaacctatctaggcgtgatactaaggtcagtgcttcgtcgcggccaacacgcttatcctgaaacgcttccatgataagtttcttaacccgactatatatttcagcgaacttgacctctgtccagagagaacgaaagttcaggctggcatagcgtccagggtccgcgtgaaatttgtagaggcgcccgtcctcagcatacaattcagcatacgcacgatcaggagttacccacgtcatgtgttgcttcttcgcatgatcgtcggaccagtcttctgctagtccgcgatagtagattgtgggcgacgacagactaacgaatatctgcattagcgcgcacgaatagcatcgtcacgttcacgctcggccactttcattttctgcttagccgtctcaagacgcttaccagtagcaccatcacgaatgatgttatcgtacttggttacctgcttgtccagtctggtgatagctcgctcacgcgctgccggggtcatttcgctatagtcaacgccatcaagggcagcggcacgttttgctttcagctctttagctttggctggagtgcgggcccctgtaactgcacctttacgtttagtcgcagcaacaggtttcggcttatcgctcggcttagcgcctggcgtagattttttagcagcagcggaggcaccgatcttatcgaacttatcacctgttgcgaaacgaggtttgagtaacgatggactgcgattagcgccgctcgctttcacccaaaagctatcagccttagctttaccaatcttagacagtgtatagtctggctgagtcgtcgtaatataggatggacgaataggagtggacaaaactttcaagccagctttagcaagagaggcaacagcagatgcagccagcttcttagcggcagtaacatcttttttgatcttggcattgttggccttgatcttagcactgataggagctttcttttctgagtctcgcgttgacttcaacttgagtttcaacttcgcagtagtctgaccaagtttagccgcagccacacctaacgtcttcgcctgcttcaaggaagcagcagccttagcgacaacaggcttgtacttagagttgattacgatcatcggaccattaggggattgaacgatatgatacgacgatttctttgtagcagactctgaagacaatgtctgagccacattaagtttgattttcattttagtccttacaccagcgctcggcctgggatatcgaagtttttaccagcggaataatcacccaatgcgcgatacagtgaatcacgtaacatttgctcgatgatatcggagttatgcgcagatgcgtctttgaaggcaacctcaatcgaatcagttctcggattcactactgcgtatcgcagaggacagatcgtttgtgcttcacaccaggcgtcgattcgcggctgcaagtcaggcgtaatggggatgcggaaatcagcgagagcaaagatcacgctttgaattggtggtggtgaggactgcgacatgtacttgccgttaggactcaggcgttccatagcagtcgaggcttcaaagatcgattggtaaccttcaccgattgtggtaatgttactgagcttgaagctatgcgtcgtcagtcctttgcgaatgagtttggcgactttcagatcgtagtcacctgaatcatcttgcgcaaaacagacgaaagcgtagaaggaaaatccagagtcttcgcgcagcagacgatggtccagcacacggaaccccacgacactttgcagcgcctgtgaggtgatctgaattcccttagatagagagacaaagatttgcattaacgcatcgctttaagtgctttcttagcgtcggccagagtagagtaaaactcttggtcatcgttaatctcaggctcaatctggaagccgacttcgagaatagcgaagcctgcgtcttcgtcttcgtctgcaacaacaacaccgaaacgtgcagtgctgttcatgatgttgatgaaacggaagtcaagaatatcgttcgcgctaccgatatcagacggcataccgtcagcagtaagcagggcgaacaggcctttcttgtcgatgcttttgaagaaagtagtagcagccgcagacgaggtagacttaacggtttcttccagattcagtttgataagactcatggttagtttactccaacttgtttggtgatggtgataacacgctggtaccagccgtaaatgttatcttcctgggtttcgtctgccttagcaatgttcttcaacttcgcaatacggcatccattgtaggcgtaagccagaactttgatatcgcgcactttgcagtaagctgtcagtgctgcaatagtcttcggaccaatattcgcagcaggtgcaaagtctggatagagtttaccgcgctggttcaggatgttcaactggtcttgcagttctgcaattgcagctggtggtcctgagttaactgcatagtcaaatacccacagagccagctcttggctgaacttcgcaagttcatcacacttgcagaaatcccaaaagttagcgctatagatagcatatgcaatttcatacggaagattctgcatatcgcctttatatccatacgcacgagcattcttctcggtgacgccccaacgagttgggccaccacgatctgccgcacgattcgtgtacttctcgccaccttcacggtcaatgacctcagcgatggctttctttctgaatgtcagagcgtccataatgattcctcttggtcgacgtatcaaaattagcgtcagacagacaactttgaagatttgaaccgcattctagggcgtgtaccaggcactgcatcaaacggagtaaaatcagtgctgtcaaacttaacaaagcctctgaattcattcagataacaaaacgctctatccagatgtactgtttcatccaatcccgtttgcgtttgataaagaagaccatcgcctgtagtctgcgtcaatgtaggcgtgccgctggagctacctgttacacttgttgatatagcgacttgcagcaactggaagggcaaaccaactgaggagtatgagggtttaacttctacgaaacggcaggcagggactcctgtgtactgtgttgctattccatttagttgaatgcctccctcatgaacatatcttatacctatctgaggagatccagattgaccataaggacagtttgagtcggacagacgcacaggaggaaacacaagagtaccttgtccttcttgggtaagggagatcgaaccttcacctatatgcagagttgtcgccgaatcaagaccaagagcataggactgctcctcggcaatggaactaactccagacagagttccgtaccctgtctgcttaactatctcagtagttttctcaatcagagaagatcgtggttgggtgtacttcaaattgggaagatagtatttgttgtcctttctacctcgtacaggattgagaaagccattgaaggccaacaccgctctagccttacgtgcgacagcattagcagtagtaaagtctgtcaggtcgatggtctgattctcggagctatcatacagaaacacgttcgggttctgggcggatgacccagctaacccgaaaaaagaatgaatatattgcatggactgtgcctcgtcaatgaagggaatgttctacgcgcttgcctaaaaattagctccaagatcgacaaaaggggccgaagccccttagaatgtccaacgcgttgaccaagcgatcaatcctgagataataccgatgtgagacaaataaccgtactgcatcacacggcctttaacatagtgcttcatgccaccttcatacgcaccatcatacacggcagagatcatcgtgaacgacatgacgtatgtgaatacatgccacgttgtcatttccatcacttcgttacaaaacactatcaggaatagtgcgatgctcatgatgtacaatgtgcgtttagtctcggtcagattaataccaagcacaacagggcgcatcacgaaggacgcgaatatcgaaaccagcattagcgtttcatagtcggctgacatgctgcgtccacctgatcaggagtgatatgcgctttattgcgcaggtcgagtgccagttgcgccttacgtcctatgcgggcatacgactcaagatcatcatcggagtaaccgctcatgctttcgcgtacatgagacagctcggccatttggcgtggactcagttcgttcgaacgcgcataggcagtcgcatgatcaatgttacctacattaaggcctgcacaacgattccagataggctcggcattagggtccgtctgcaccatcaacgtaccgtgacgatcaacgtcatgaatgttacgactcatatcaaactccctggttagaaacgtaggtgtcggtgatgttagcagtcttctccacgttaccgcgaatataaccaatctcaaacacctgtacgttatgcttgaccacagcctcacctactgtctcacatgcaccgctatgcagatcaaggaatgcctgacacaaacgttctgctacaggcttcgcaagaatcttcatcagcgtatgtctctggacggcagacagcttgatgggcatcgcatcgatctcacgctcaatcgactttcgtccaccattgaatatccacttacagatagtggcagtcagtggcttctggtgcgtcttagatggcagcgtatagatgtatgtcattaagctgtagaacaaacttccgtcgatagcacgacgcttgaggtcatcaaggtactgacctacaggctgcaacttaccgcgctgcggaaccatgtcatccagtttaagatcaacatcaagaccgaaacgcttcaacgattcagagtggccgaatacatagacgatgtgctgcggcatatctcggattgctacagcattacgcgaatactctttcgcaccgacaacaaacaggtgcttacggtatttctttgaagggtcaatcgtaccaccaagcggaacaaacgtcacacgatcggcttgacctttcttcttcaaccaacccatgacttgctctgggctttggcgtgtcaccgcgattacaggcatcattactccacagtgttgagtgctttagccgtgtactcacgcagagtacgttcgatatcttccgcaacatcaggatgacagatcaactgatatcccctgataaatacgcgttgggaagggcgcatcactttgcgatgggaaggccagataccaaagaacttgtgcataggagttttgtagtacgtctccttatgctcgtccatgcaattgtggttggagactacatcatacttggcataaatgtctacgctctttttgatgtagttgaccgatacaggcatgctgtgcttttcatgatcgcgattgagctgaccaaagatcatcatatcaccttacgagacaggctggacgttccaccttgtttggtcactgtccattgattattagagaagtgctctacgtcattcggagttatccaatagatgttcgggataatctgtttgagtataggcaggaagttttcaatgatgtgctcactcactgctgggctgcaactattatcaggctcgtcgaggatgataaagttcgtgcgtcgattagcaggaatgaacggcatgatcgcaacagcaaacagcaagcggaagcagttagtctctgcaccactcatgataccaatgtccgtagtcttcttagaagtcatacgggtcaccaacgcaactacaccttgcttgctggtggatagagtgaagtgcataggctctgggaacacgagactgctgtattcgttcagcttattttcgatctgcttcaatcggctttcaacggctttcagtttgagagcgttgttgctgtacgctttatagagaacttcgaataccttgcgcttatcgatcaggggctggagcttggagagtttgctgcgaagttcccgcagtgtttcctcatagtgctcatgctcctgaatacgcatctggatgccttgagccttgcgttctttcttgtcgatatcgttacgaagttgttctgacttagcctcaatctttttgtaacgaccatcgagaatataaaacgggtcttctggttcacctacggccttcattgcagaagtcaggtctttcagaatctcaagatccttgatgcgattcttgattgtcttacgagccttcttcggctgcttaatcgctttaggtttcttgagcgctgctttacgtgcttgcagcttctccaacttcttcgcctgttcgaattgttcttcgatagcgtcaagctgtttgcccagcttcttgatttgtttctcaagggcttcacggtcgtgcttaggcttcttcaccttgtcgtcttgcaacgcagtgagttcagcgttcagcttatgatagtcgatagcctcaatacactcgtcaatgatcgcctgtgctttggttgcagcgcgtgacatagctttcaggtcaacatcctgaccgcatgtcgggcaagagttaccgtcgtggtcgtgttcttcaaacgcacgatacgcctgaactattgctttggattctgcgcgggcatcctgtgcctcttcctgagttcgtttaggacttttgagcttagacagtcgcttggtgagctttgcgcaggcttctcgccagtcgtcgtactcttcctgttgttcatctaccttctccagtagttcctgtgcagcctcttcctctttaaccagcttgccatgcttcttgcgcagcttcttgttatctaggtctgcaacatcaccaagtgctttgatacgcttcttaacgtcagcgagttcctgctcgtactcatccagcgcttcaacgtagtcatcatacttgtcgtgatcaatcaattgaccacgcaggtcattcagttcgcctttgagatcggttgtctcaatgccgagagtgtccagctggtgtttcagcttctcgtacttacgagcattgctacgtgcggaactaagctccagcagttcttcgttcaggcgattgcgccgtgctttcatcttatccagatgttcgatgatagcttttagcgtattcttttcttcggcgtgaattgacagcgcgttctgcttacgctgtgtcacgtcgagcatgtcggccagacctttcgattctgtctcggcatcttttgccaagtccagtttcttcttcaacgccatacgaatgttgtcaaagatatctaggttgaacagacgtgtcaggtataccagacgctccgacggagttgcacgttggaacggatgttgaatctgcgattggatgtagcaatagctgtagaactcttcctttgacagaggccagtgcttctgtacccaaccacgcgcaacgtcctgacgaccaaccttctggtcttcgccgttgtagtatacttggtacttcgtggctgtctgcacgatacgcacaacaccaccaagaggtgagttccacgacaggtcaatcgaactacctttgccgagcatgttccccttgtctttcttcttcattgcaagagggtcagcttcatacagcaaggtaggtattgcagcgaacagcatacttttacctacgccgttcgtgttgtccttaacgtttggactatcgaggttctttccgcagatagttgcgaagccctctttgtctaggccgtcaatatcgagttccttgtacacgccaacgtcgcgcaagtgaatctctttcaggccgataccatgttgctgtactttctttttggccattagaaatactcgacggtttcttcctgcacaagacctttaccgtgagtctgctcaaacacttcgatctcgtcttgcgagtattcggtggaggactcagcgataacatcatacgaaacggattcgtcgcgcgtatcagacacgacaggtttgatgatacgccacagaggcagtgcgattgggtcacgcttaatcatagacattagtggaataccgccgttggttcaacccagagttcagggttgttgtacttcgcacggagttcctccatctgatcatcagtcagaggactgtcggagatgtggatgcactgaggaactttttcctcttggccagtaacaggatgaatgtcacggtcattgcgcataactgcccagcgtttggttacgttgatgtggatggtgcgttccatagtgaagacctatgtataatgtatgaatgatactcgctatttacagtttttaaggctatagacaaaaagaagggccaccgttaggcagcccctgcgaacactttacgcaccccattatccagatagtggtctgcgtagaaaggtccgttttcattttcaataccaatacgacggcagagctgacgacgcaaacgcttaggccacaccatctcgtcatccagcagatgaataaccgcaggtagcgcttcgagttgagtcattgtcagatcacgaatcttatcgtcaatcctacaaacttccgcgtagtcctgttcaggtgtaggcacaggaagtttgggcttagataggtctacggtgagttccatcaatacctccgaggcttcttgattttcttaatcgtggacttaggacgtttgattgccctcagtgctttacgtgcttcgacaatcttcttggacaactcagagcgttgagccttaacagcatcagtgtcctgctcggtgcctttaagtttctcaaggcgattccactctttgaccaaacgatcaacgacgttagcacgagacacacgttgctggttaacgcgcacaatgtcttgttgcttcttcacggagtcacgagtgttattcacttcgtcccgcgcagacttcacacctttagtatcaccttcggactgtttgtcgttcagcttctttcgtgcaacttgcgaacgtcgctgggcacccttaagatcatctttcgagttctcaaggctaaccttcgtatcttcaagtgggctggtacgcgcactcaaactgataagtattttcatactgacctcaaatagaaaagggtgaccctaaggccaccctgtgtagaatggcgcgctatgcacccgactggttaggtctactacgattatttaacctcgcagtagtgagcgaggagatagggatcacctcctcatgcggattgaagttgaatgatttcttcgtcttcgatatccgcgccagaccacgaacgaatcacggatgcgttaccacgattgcctgtcagcatcgacttaactgctggacgtgcttcgcgttctgcatagtggtcgacaagagctttgtcgttgacgaaccacataatggagtgaccacccttagggcagatcaggaattgggctggacgttgtggtacgttcaacgtcatatagaagtcgccagcgccttcgggactcatcattggcatcggcttcatgatctgttggaagtcttttgcatctttaagacgcgtatcacccaacaaccaaatagcaccttcttcaccttcacgcacggcgctcaacgtgcctttacgcgtagtgatagatccgaatacatcttgatcgaatcgagccagcccaaagataagtgatgcgagtttcttcaaatcaggagtggtgcatggactgtcaattttagccatgccctcagacccgattgtaatcttcgataacgaaacaaagattttcatattgtcttccagagctgtatgattaattgtgttataaaattagtgtttgatcagacaattctgaaacaaaaatgggcggcacaaaggccacccgtttttcacttatttacttcttcttctttttctttttcgctggcttgtcgtcttcgtcgtcttcgcccatcttgactgacagcttaccttcgtagatatccgccatgagagtaagcactttggattccagcataatgtctgctggtacggacgttgagttgaaggctacttcggcatcagcgagtgcagattgcagatagaccatgctgaccagattaactttgatattgtctttcttggtcatgttcatgaacatcttgaggccagcagactgccacttattcgtttcggcgtaatgacctaacacgccgtgaataatccaacgagctttcgcaacgattgcacgtgggttgttcgcttcacgcaggaactggattacggcaatcaggtccatagacagatacgcaccaatcatctggacagctttcgcttccatgtcgatttctggatctgctgctgcgagttcggcaacgaggttcttatcgaactcctcaccacctttgaccgacgcatagatgttctgcaacatcgtgattgcaccacgcatctggccaccagcatactcagctacctgatgaagtgccgacgtagccttatcgagagctttgtctttcttcggcagtatggagagttgctcgctaatctcgaccaaacgcttatgaataacatcggtcgggataggtctgataggcagttgcgtcatgcgactgatcatcgtgttcttcatcttctcagggttcgttgttacgaagatgaatacaacgtgagctggtggttgctcggtgattttcaacagcttggattctgctgcgctggacattaagtgggattcatcgaagatgaacacacggcgtttgaacataggactcagaggtgcgctgtccacaatcttctggctgccgtccactttacctgcatcgccacccatgtcgaactcttgctcgtcagggtgtgcaccacggtcgtgcatctcacacgaacgacacttaccgcaggcgctgaatgtttcgcagttgatatacttcgccaccagacgagcgaacgttgtcttaccagaaccgagatgacctgtgatgatcatcgttgatggaactgtcttcgacttctgccagcctttcatgatcttaacgatgtggtcttgtcccacatagtcttcgatacgcttcggtctaaactgatcagcaaagttaatcgtggtcagttcaacagactcggaagaatcgcctttctttttcttcgacggcttaccatcgtcaaagctacgcgacttcttctttttcttttcttctttagccattttcaattcgcccttagttctaatgcgttacaccagttatttacagtatttagacaaaaagaaaggaccacatccaaaacggagggtcctcttacgtgtagcaataaagtttggaatgataacgcatcggcagtgggcgctgacgattaggcaaagctcaactcccaacgtggaaccacgcggaagaattgcttaaagtgggacggtgggttattcttgattgattcaagtttcttttccactacgtcataatcttttatgccactctcgactgtgtgagtggtgaacgtaccgtcagcctgaatcaagtcggcgacaacacggtagcttggttttctcagcatctattctcctgaaaacgaaattcttattgctctgaattatgtttacagattactggagtagtcataaaagaataaagtaagacaaatcttaaactccaatagggactcgttagaaatcctattggagttcaccctcagtgcgatgacggtcgccagaaggtgttctccccgtgtctttcaaatgcaccgacacggtagcgcttgcggtcttacgctcttgtgtgtgcagcgcgtcggcagcaggtagcatttacgcgcagcaaagagcagccgctttcggccattagcgataacgcggtgttacgcttaacggcctgtatgactctggccgagtctgtacaaaaaagagttcggcctatccccaattcggcaaaaagaacaggccgaactaaacagtcaacacacactccatgtgcgctgttttgtactgttacaaattagaaacatgttgaaataatcagacaattcttagttgagcatcggaagaagattttctaagaaatgctggcgatcaaatgagctaattcggtgaggatgtttgatgtgcaggttccacgccttgtcaaacagcaacacgttctttggcaggactacgttaacgccaacacgagtgaaggaatcacgaacggccgtaactggattgtcgtcaacaagaatccaagtaccttcaccgtaagtcgcattcagaaaagcaaccttgtcgggatgctcaacgctgtttaagcagtgaacatgatcgaacaatgacaggtgcttctccaaagacttgcgcgtgtagcgttcacctttctcgtggtaaccgcgatgcgtacagatgcccgcactgaatccatcacgcaccaacatcgcaactgtctggatgaagtacggacgcatgttcgcattcaacatgaacgtaccttcggcaagcaggtcaatgaaaggctgcttaccgttctcaggcgtgatgaaggtgtcagtgcctgggtagattccgtaattcataagatgacacagcatgaagttatgtgtatcaaatgctgtgtcgtccatgtcgaagaaaatatgtttgatcattaatgcctcgtgctcttaactaccagaggaatatcgttaatgaatgccagagtcagcaactcgctgttaaagcgcaggcgcatttcatcggcattcgtaacaagaataatatcagacagaggatcaaccttgaagattggaacctcaataagtacggcggtgtcctcggcttcgtcaccatcaacaatgaagtaaccaccgtacatcaaaacagtatcaccagaatcgacgagatgaccaacgattgcgtcctctccgtccatgatcatgtgcagaggctgatcgatgtagtagccgctatcatcgtctgccccgaactcaaagtggaaatcatcatcgctcatggttaggccctcaaatcaaccaatatcgaagcactcaggtctcggagcatatctctcccaagagaagtgtacatcgtctgcgctataactattcgttcaaggaaaagacgagaactattaacgtcatgtcctgtcttctgctgaacgaagtcgatgattgatgacgcaggctgaatgaggaatgtgagtatctcggcgtcgtgaagcacgttgcccatagccgtcacaggtcgcatctctgtttcctgatcgagaatgtatgagatgactcggtcttcattgcctatgttagggaatatcttaaagaacttgcgtaccgacttgactgtcgccatgaagtcatagtttgggttggtgggcatacgcaagaagagggaggcgagcaacaagtttatttctaactgtggaccttgttcaatgttcaacattgcatgtgaagtcagcacaacattcaacgagaagtcacgagtgtagagcgggtgagaggtcgctgtctggtcaaaatagtcaagggcggaacgcaacccctgacgtattaacaggtgctctgctttaatgcgagtcaggcgatgcactactcagcaccgcgaatctctttcaggctattcttgatcgctttgcgtagcgtcttacctacgtcgatgccgtcgatgtgacgagcaaacacgttggcgaatagcgtggtcgggtttttcataatcgccttgtcgagatcagggcgaccctctgcaatctgcaactcgcccggccagagttctgcaactgccgcgctgtcattagcagcaatcagttcaagctcacggacggagatagagttctgtcgggcaatcgtacggaagattatgtcaacgaacggcagcatgtcctcgctaacaacgttcttcacgtccttagcatcaccagcacgttggaaatcttccagcaggctttcgagatgtgactgcgtgatcttctggacgttacgcagtttcttgaacagcatcatccagcggaccttgcgcttggaactcagcaggtgagtccacacagattcaccgagcgcaatcatcagacgattgtacacgtcaacgctcaggctatcacgatcaacaaagacagtcatctcgtcatgccattcgtccttacggaacttagaacggaacgcatgagtcttcgaccctgactgctggacgaagttgatttgtttgcatcggcgaacagcttccgcaagatgatatttctcaatcaccttaggaagtttcttaacgcccatacgacacgcttttgctacttcggcctcacgaccgaaaagagacagacggggcaagccaccgtagacaggcattgaagcatacggtctgactgtcacaccgcatacggacatacctggctcagggtcaggacctaatacgcagagaacatcacccgccttaggactgaacttgattgtctcagggtctggcgtactaagcgtgttggccaatataccaacagtgttcccagtagccagtaccaaatggtttttgttaccctgccttacaacaaggtaatccttttcactgtgtttcataacgacctttattgaagttgatcagcgatatcgaacgtatggacttcggctgtgtaaccttgacggaacatacgaccttccgaacggccagtagcttgctcaaacgaaggaggagaccacgaagttgaggcttcgattgagataagaacttgctcgtcccacatatcaccgtcttcaagatagtcggcaatcatgttaagagcagcaggacgatcgaggcccagatgcgcaagctcggcgataatgagtcgcggtgcggtgcggtctttcatttcgtcgagttcatattgcagttcagcaagcgttgtgactttgtgagagtccgcacctgtcatgccagcatagtcatctggtccgaaataagcaatatcaaagtcagggatatcggtttgactaataaagaaatgaggtgcgtccaccaaaattgaaggtgaggcgcacatctggagaaaacccatataaggatgtttaatctcatgggcttctaccgaacaggacttcccagcaaggtcttgcttaatgctgtgtgcgagattattcatggtaacctcatttctcaggagtaggggtaaaggggctgtgaacaaacaggtttgtcttattgacatacaggaacccgaatgcgttttgtttgtaactttgacgcgcggccgattgcttacgtttagcttcggctcgttgtgcgtcctgctcgtcaaagatacctcgacgatggaacttaaaatcagggtgtactgaaatatctttgacgatagcagtcatacgttattccttatacgggcttaaggtttaggtgatgccacggaaaatctgctttctccaccagctcattggcggtacccatctccgagaacttgtcgaatacatgaccgtacatcgcggcgaactcagcgttctccaactctgcctgccagtcttcgtcttcggtaacatgtttcctccacacttcgtcgtgcaacttcataaatgtatcggaacgtttcgggtaaagcaaagagaataggtcacgcgcaaaacaaacgcgatatgtacctttatctttaagagcctgcaaagaagtcagtggatgcgctgcgtcaaaagccgcgagcacttctccatactgtttgaatagacgcttattctttacagcaatcaattctaatgggcagtctttgattagtcgcatcacaattttacgtgaacgcaactctggccactcagttggaggcaacacggcactttgagataacttgaactcaagccgaaacagaatttcaataggactcattctgcatcctctaaaaatgtaaggtgatcggagaattgcttcttaaggaataatgcaccgtcagaatgaaccgagtcaccgaccgtttccattaaagcaccatcatgctccagagaataaacgtgtttcacctgtgtgtcatctacgataagacggaacaggcactcagactctatgccgctgaaaatgtgattgagcacctttcgtctgcgacgttctgatattcttgctttcttgagatcgtacttaacgcccgatttgcacgttaaagttttttcgccatgcttcgtctcacggaccgagccaatataaatgtcggtcaactctcttagggccacgctcaaaggtatcgcgttgttattccatttgcgcacaaaatcaaatactttcaggaacggcatatgatgcgttagttcttggaagactcgacttttatacgacggaaccaattggcccatagaaaagagtgtggcataaaaacaaatcttcgtcgcagctttcggtagatcatttcttttcgctatatcgtcaacggaggtcacatcgtccataaacgaacaatgaatcccgtgtgcttcgagttcacgcaacagaatgtttagctggctgctggacatatcccagttggtgcctatagcactgcactcctgtttgagctccgcagggaatgactggaagccacctcccttctcaaataaacgaccaccaatcttagccaagcggtatacaggcatatagcgaatagtcagtggatgctcacgcacaatctgcacaggtccgctcaggatagattgaagactggacaaaacatgatggtattgaccctgtgagcgttgtgacttcatatacgacttatgctcaaggtacgccagaattggatcgattaaaatctcattcggggccagcttattaagcacggacgtatagagtttcttcgcttcacgatccctgttagaacatagagcggtgagatcgtgcctaggccatttgaacggcttcttcacggcttcatcgagcatgtccttaattgtctgaccgtactgctcattaaccagacgcaagggactatataaacgagttaccgacaacaagtctttgcttgtctgggggttctcagggtacatgcaacccagaaccccaggactaatacggaagcggcggcatatacccgacttacctttcttgaacaaatgatttttgtattcgagaacattttcgagcaaccaatcaagggctctgctaaaatgttggtctgttttcttaaagttaggcgacacaggaccgcccctttgagattttaccccgaacaccataggcaacactttacgtccgaacgttgaagggaaaggcgtccaaacctccccgaacttagcgttacgctgtttgctctttgttggcgtatagattgacaattgcagaatatgccagaagaacagatttatctggcgtctatactctggttcgagttttcgcggcccgtcgtacggacaggcataaactacgtgggtttgtacccactgtatcggaaacatctcttgatacgtgggattcttgactaaatacggagaagccattgcatactccagaaaaagtgcttcttgctcttgttttttacagttttaggtgctttcgaccattttcttttgctttaggtacaaaacagagtcacataacgacacaatcacctccctcaccatctagatccctgccacccaggagccacgccaagcaacccgcttaccgcgacagcttactaatagcttcgctggacacaagctagctgggacagctggaatggctggaaggacgggctacaatcgctagggacaatagggctttaatgggtatccgagataagaaatactcacctacgtagatcgctgtatgaagctctctgcgtgtagggaatacgtcgtaggatagccaaacgctaaaagtcttaggctcaatttgcgtcagaaataccatgtaacttttttcgaaaaactagcactcaactgtagaatcgagatgaattttatgaaaagcagaggaaaatccgagaaaaatcaaggactttccccgctatcatcactttttctgcgaaacgcgcttcccgagcttaactccgatttgagtcaggatgcgtttcactgtatcgccgtcgtgttcttccatagcggcacccaaacgctcgccctgctcacgcgatagctcaggcataatcattttgagcatctgcgaacgctgttttgctgctttagacttgccttttgagacagacacgccttcattagcagataacgcactgctaatagccttttgcacacgacggtcgccgaagatatcgccgaagatatcgccgaacaggtccttgaacgacattcctccgctcatgatatcatccttagtgaagcgaacaggctgccccagcgcattcgtcttcgtgctgtgcgtcgattcaacttcattcgttgtacgcccgccagcacggaagttctcgtcaggacgtgacgctttgccctctgcgcccggctttgtgttgccgttacgcaaatctgggtcaccctcaacagccttgtccgggtcgaacatgtcgtccgccgtttcgctctggtttggatcgaaaggaatcttacctgttatcttattcgggtccggccagctatctggaatatcagacgccggttgaggcttgttcgtcatatcgttcacatcgccgctcaggctgatcttaatgcgagtcatggttgctcctatcgaattttattgcctttgaaaatgttgtacgcaatctctttgcgctgaacaggacgcgtggtgcatacccattcccattgttcgttctttgcggtacgcttcttaggtgcttccataactttcagcacataattcttgaacggcaggacgagaatatcctccggctcaatagcaccgctacgcgcaggaaggactactgtaatgttaccaacagtcagttcctgatcgtagttcaacacgtttgcttcttcgctgatgttgcctttaacggcagacacacccaaatcgaagataatcgtagcgtgggtgaatgctgcaacgtccttgatgcggacaatcacatgcttgcctcgccacggttccagattggctgctgtcagctcctgctcaacgccattgaccaccagcacaggacgagggaatgcaggcagcatctgatcgtttagacgtaccgaataagtcgcctgcgtaaagtattttggaataagctgatcgaaatcaacgtgtccgtctttacgcacctgcctgaaagttgcagggctggtggactgatcgagcgtgtatgctgtcagcacttttgcgtgatggtgagtcataacgttgtatacgaagcctgtgctgataaagcctggcacaacgccttgacggaagcagataccgcagttcacaacgttacctgcatcccatccgtttgaaacttcttcgtcaccgttacccataaggtcggcagcgtccattactgcattcatgccatcgtcgatatcatcaagggatactgtctggcgcccaccgccgaacataccttttgacaccgtgcctagtttaactccagcgtccattgcagacgattcgcggccgagcgacttcatgccgcccacctgctcgtcgaatatatcgttgtccactttgttgcagctacaggtcagacccatcttcgctttcttgaagatgattacatcggtggcatcaacctgcaacgcctgttcaactttcgactgcacaaccttctgaactgagtcgaggcgttgctggacacggtccgtttcgtaggtcttatggcggtcatatgaatttcgagggcgtcctcgttcaatccagctcataatcgttctcctctgtgtgctttaaattagtgtacaaaatttaggaccttcaccctagtaaatacttatttagagtacgttaaaacacggagccttttatgcgtattctttcaggcgacccgggcaaagtgaacttcgcgttggctgttcaggagtttaaagacagacgcatcactgtgcttgggacgaggatgtttaagaaacccatccaaaatcttcatctggacatgcggcagcccaccaaagagttcctcgctgaactcgaagaaatgtggaagctatatggaccgttcgacgctatgtgtttcgaacgcttccagtcgcgtggtcttggcggaaacaccattgaagcaattagtctgatgcttggtgtcatatcgttcttcgcgctcaaaaagaaatgcccgcttgatttgattacggctagccagtggaagaacgcattcaaccgcagcatggtgctcaaggactattacgagcttcacaatctcaagtccaagaaaagccgcaaagctattcacgaatttgatgcgtgtctcattggcgcgtataccttctaccgacattcagggattaaaccatttactggcttctctcgcatcattgatgtgtatgtgcctaaattcctggcgtcacctgtactgtgagacaaacatggaacaaattgaactgttacgcgtagtgaaagagatcctcagcgaatatggcaaagttgagtttctgtcgcaaggtcatgttggcgtgaacaccgagcatcgtgcgacctatgaaacgttaatcactgtgacctcggatagcgagacagctttccccgaagcagatttccgcgctaagattgcggcgcagattgacgagtatcgtgtggtgggattcaaacgcacctacaacgagcagaccagagagtttgtgctgcaactgaccgaccctgtattcacctaccgtgacccattggcgtgtccagcaaacggtaaaactctgtactcggtttccgtaggtttcccgttcgtgtccaccaattaatctgtaaatatccttacttggttaacgtgcgtgtgggatattgaaaatggcgaagttgaagaaagaaccagcggtcaaagtcaagaagaaaaaggctttggcggccaaaacaaagaaagaaaaagcgaaagcgattcctatcagtgttgtgcaggacacacgtcctatcaccacttgtcctgaaatggaagagaagccgcagcctttcctgttccgtggccagtgtccaattgtaacctgccagtattgcacacgcgaaacgccgacaggctgcatggcgcttgaccgcaaagagtcggcagatcgttcaatctccaacaaggagatactctattataagaaaggtctcttccctgaacttaaagagatggatcagaaaacgctggacaatacgattcgacgcgcacagaatcgtacccgtaatgctatctgtcttactatgtttattgccggcattgatgattctgactgcgatcgctctttcaaatatgtagagggtcgttccaaactcgtcgatcaggtccataactatctgattcaaacgttcaacgattaccgtccgtggatgctcgcatacctcgatgacgagaaacgttttagcgacatggttggcaaaataaccaactctgactttaatttagttaacgcattacgattgactcctcgcaagtatcaaacgttctgccagtcgctacaaaatcttaaacaatctggagactctcatgagtaactttatttctctcgatcagtatcgcgccattctaaagcgcaatatcctgaaagagcctcagatgcttgtcattaatcagacgcagcctctgggacaaatcttcttccaatgccctggcgataactttgcgatgaaagatatcatcgtgcctgcttcgaagaacgcaatcgatctgactcaacaagctccgctggaaaatctgctggcgtgtagccaactgaaagcgctgctgcaaacgcaacgtctggtactgctgaaccctgaagaaatgccaacgcctggcgaaggtattcaacaacctgagttgactacacctcctgttgctggtgcaatctctgttgacggcaagactatcccgaatgcaatcgtgatcgtcgagcagaacggcaacgtgtggaccggcgcttctaacggcagcggtgtgttcactgtggacgtgtctggccttgaagaaggtgtgttctctgtcactgtaactgctgatggtttcgtacctgcgcgttataacttcactgccggtgcgcagcctctgcaaccaatgcctgtgcctaccgtacacgctgtctttaaagagacaactgtgtcgggaaccactgttgcgaatgctaatatcatcgtatcggtgcagagcaaagagtttacaggtcaggctgatggtcagggtgcgtttagcattaacgttgacccactgccgtttgacattattcacctgacgatcactgctgctggttatctggataacgttgtcaatcacatggttgactctgttcccggtctggcgcagattaacagcgcacctttcctgtctactgcgctggcgggtaaagcaagtccagaagctgaaatcgaaatcatcatcactggccagtccaatcagttcgttactgctgctgcaaatggcgattggtctgctgttgttggtgcggttaaaggtgaagtctctattcgtgtgctggagaaagatggctacgacgaagcgactgctaccatgcagcctaccaaactgcctgcacctgtactggctgtcgataacgccgatagcatcggtgagaatcaaacagcattcggcggtgcaatcacaggcctgagtgcagaagcaaatgacgtagctgtgactctgactgttcaggctggtctgtacgaaggtactgttgaccttcaatcaagccactggtctgtgactggtgttgatgcaaaagctggtgtgggttctgtaggtgttgttaacctgacgtcggccttctatgaagaagcatcgactcagttcaacattctggaagagtttgcacagcctacgctgcaacaggcgcaggatggtcaaactgctgtggtcggtgacactgtagcttctgctactgttaaggtcacgatgggtggtgagactaaaactgcttcttcaaatcctcagggcgcgttctctgttgatggcttcaccaacgttgttcctggttcagttcatatcgaactgtcccgcgcacaatacaaacctgctgcgttcgatgtaacactcgtcgtgcaggcgttgggccaattggaccacgagctggctgtcggtgatgacacagctactggccacgctacaccagggtctacggtaactctgactcagggtagcatttctggcgacgctgttgcggatgtttctactggcgaatttattatcagcctgtctggtccgcttgccgcagacactcaggtagagctgaaagtagaacatgcgaactacgttgactacactgaaaccttagctgtttctaatccttaatcttacctaaggggcttcggccccttgttgaaatacaattcggagaattaccatgtcagataaagcaagcactaaggttcaacctatcacgttgaccgcatacaacgaaaagtatggcaatgacgttacagcaccaatgtatgtcgctaaccgcactgagcctcgcggcaacgtaatgttcagcgcacaggacgacatgggacagccagttccagttctggtgccggcaacattcatccctgtcgacctgacccagcaggctaccaaagagagcctgttgaaatctactcacctgcgtcgtgcgttaaatcgtaaccagctggtaatcatcgacactgaaagcgcagagcactacctgcgtaccagtgctatggctaagtccgagatgaagaacctcaacagaatgggcagcgctatcgcagccgagctgggtgaagaaggcggcgacctggcgcagatcgatctgggcggtaacaatcgtcgtcacgttcaattcgaaggtggtactcagtattctgaaaaccaattcgtcaacgcattcattgttcgtgctgcggaagacagcgaagaatctgatgacaacctgcaacgtgaattcctgtctcgcggcattaacctgcctgcgtcagagctgcaaatcttgcgcaaacacgttactcgtccggcaatcgttgaactgatcgttcaggcacttgacgacgcgtaatcgaaagctacagaccaaaaaaaatgggaggccccgaaaggagtctcccatttttgttacgttcgcttattcgttatggctttaggtctagcccatcccaatgtcttcgctggcatgatgcacttcttaccgtgaatatctttcagcgtcatacgcacttcttttattagattcatcggagcgttgtccgggtccagcttaatcagcttaccatcttcgtcatactcacgagggagtttaaagtgcttgaccggtactggagagttcttttcaaactccgctttgattttattacgcagcaacttcccgccgccatcattgtctgtcattgtgtagacgacactaatccctaacatctcaagcgttctgcgtttcgtttccccgaactgctctgcaccgagtacagctaaagctggaatcccgtaagacaataaagcaagtgcatcacgaggaccttcaacaagaacgatatatcgcaacttgtatttcttcaaacactctttgactagcggtagtgggaacaagcctttctcttttgcccagtcaccattcgagttcacatagctggtgccgttcatttgcttgcgcagatacgcagcgataccacctatatatttcgaaccatgcttacatgggaagaagcacacattcgtgccttgacgttgtgcgttcagtaatccacccgcagcttggacaagcgctccaggataaccacgccactcaacatcgaccggccactccatgtaactgtttctgccgagagctttcatcagcaaaccgacagacgggtacgtaccaatcttcgtgctgatttgctcatacgttttgaacaacgcactcaggctgtttgtgttcgcatctttaagcgcccagcctttaatttcctgtagctttgcgtgtgccgctaatttgttccaaccacccttctctccacagccgaagcagtgaaagaagccgagtggtatctccatacctacagaagtgtaaataccacaactaggagtcttatcgctgtggaatggacagcacaccataacagtgtcaccgttgtatttcttgtcgcctggcaatttgcctatttcgtcaagtattatttgatgaacatcttctgccataccatcacctgtttgtttcgtaatttgagcatataagcatatttacagaaaaaggacaatagaatgggcaatccacatcgttacgtgcatacggcacaacgtcgttactacggcaaacactggattggcttttgcgatctgattcgcgtcgagcctcaaacttacggagcattcgacaagcaggacgatatgattggcctgtcgctcccacgcaattttgatgtagacgctgcaacaaagagtctgcgcttgatttacaccacgaatgacgagaacgtagaagtacgctgctacctgtttggtactcgctactataggttcgtattcttcgagcaaaccattgccgttagcgaggactccaatgagaacgttagcaaacataccagcgcgagctaatgacacgcgcaacttgtctcgcatcggtaaaatgattgacgctgcccttgacgtaaagaatcaagaaaagcgttggccgaagaagcgagtcagtccatctatgttccctatctgccctattcaagaggcagccaaacttatttaccagaagcataacaactgcatgaccggggagtcaggtacgttgctgaacatctttgcgaaagcagggaccgggatgcacgaatcattgcagaatgctctgggtcatagtggtcagatggttggccactggaaatgtacgaacgataaatgcgttgagttcccaaagactaaaggtaagatggtcgatggtgagtacgtcaaaggcaaatacacgcgaactcgaagcacgaacaatcgttgtccctcgtgtgataaacccatggcttacgcagaactcaaagtcctgtacaagtcactcaaggggtatgtcgatggcctgattgataatctggacggtacgtacagtctgatagatttgaaatcgactatggtgaccaaagctgctgacggatctttcttcgttaagtatcaccgcttccagattgcgacatacgcatacctgctgaaaaagcgttacggctataacatcgttgattacaccctggtctatgttccacgcgacaaccctaaaaagtttgtcgagaagacctttgtctttgacgaggctgagtctaagcgcgccaaagactttatgatggaacaaatacgcgcatgggatgctgcggtaaaatcggtacgcacaggtgacttgctgcccgctatcaagcggaagccttgcaagagtgccgagtattattgggacgagttccatggatatgatacatgcccttttgttgactattgctttattcaatcacacatgattgacttcatgaagaagttagagcagcgaatcatggccaaccccgagctgacttatatggaaatcgtaagcacaggtcggaaaactcaacaacaaggtctgctacaggacaagcctaagaagtctggccgtccgaagcatatcgtaaaaacatttgagctatgagcatacaaagagattatgaacgttccctgcgccggcttaaggagtctgtctatcgcaaagagcaactcggttatgtagtcccgagatgcgttgatgttgttctctcgaaattgagatcgccagagcatgtagtatcgaggaaatatttggtcatgctgatgttgtttagtcagacgtgcgaacaactcggtaccgctcttgctctacgcgaacaacttgtggtcaagatggctatccttagtcgcaagcatccaacgccagacattcagcgtaaaattagacgcctcgaagaactggtaataagtcaggacagaaacatcgagagccatcgtctgcttctcgactatcgtgccagcgtgttgattgatatactcgacggcaaagaacctaattcacgttacacttgaggtacttatggaaatgtatgtaagcctgagtcaggacagtacggataagaaccgtagcaaggtcaccagccctgaatcaaacactggccgagtcgatgtgtcagaatacgcatctctggaaaagaaattgcgtctgacagatgaagccaaagacaaagagaagttagctcaaaaggctggtggcggggattctgtaaagggtaagaaaggcgcgaagaaaagtagcgcagaacccaaggatgacgacactgatacggacgaagaccctacattagatgatgaaggtgacgcagatgattcagatgactcttccgatacagatggagacgactccgatggagactctaaagctaagaagtcaggaaagaaatctgacaagtctggagcaaaagactcagcggacgcagaagaccctgacgcagacgaacccgaaagtgatgacggggatgcagatgttgaaggcgctgatgacgaggacctcgaataacgatcctgtcgatgtgcctaagactcatgacgcgatgattgatattctgatcgctattcgctacatgtgcaccaagcgtatgatcttccctgtcgtagtcgcggccatcgaacggcgtaacgactatctggtcatgaacaagctgaccttcaacatgaagcctggcaagttcctgtctgctgttcaggatagcaactgtgaagtgaacgtgtgttggcttatgcgagccttcacacgtaccgctctgcactttgacctgaagcctgtgattgctgatcgcagtggcgaatttcagccgctagttagccgttacttcactcaggatgatcctgacttcgcctatcgtcgtcattacgacattcgctacatgactgcacttactgatatccgtaagcctcgcatgtatctgcttaatggagttaattatggcgtacaagtcactcgccaagaaaccgaagaagtcgaaagctgcgaaagaagccgagactcggaacaaggcgcacaagcaagctcgccgtgggaagctcggtcaggctgttaagacactcagcgctgcctcgaagaaatcccgccgcatgacaaaaggtgagaaacgtgcaattcaattgcagccgttcaaacctcaagtcgtaccgcagcctcctaaaactcctttgatggagaaaggcctttcgttaactgcgctgatcaaatcaacgccacgtttgatgaaagagaacgctatggaatgttatgtcaatagcgttaagcgcggtaagacgaacaaaggtctgccgatgattatggcaaacgttcgtcacaaagatccactgcgtcctaataaaacagtgcgcattcacaagccgatgattatcggtctggatgacccgttcaagcctatatcaaaacaaaagcgtgtactggtcagttgtccctgcgagaacttcgtgttcatgtgggagtatgcgaacgccgaacacggtgctgcgcgaatcatttacggtaacggcgagccgccagacttcactaacccaggtcacgcgccaggtctgtgtaagcacctgatggctttagccgatcaagtcaaacgaaacggagattaatccgaatgttctttaacagccctgctccgggagtaatcccaaactacccgattgttcactctatccatgagatgaatcgtcgtgttgcggaactcaacggcgaactgattgccgctggttgcaccgtcgttcagaactgtggcgacatgctgatcgaagtacccgcgggtgccgctgcaaaagttgacgatatcatccagcggcacgttgatatgttcaatggtcctgttgtgagtaagcctgctcgtttgcagattggaggcgaagatgcagaagcagaaatttaatcctgaaacgcatagcgtgtcgctgcacttcggacagcacattgttcatggtcatgcgcaagaaagcgtgtttggtgatatcatgcagacgttgttgctgcgtgagatcagtcgcaccaccaaagaagttatggagcaaggtatcgaagttgctcctcctaccattgagtgtaaaacaactgatgcaagttcgatcctgagcgcactcaagcagtggcaggaaatcatcaatgctcaagaacctcagaaagagttcgagccatgctctatcccagactggatgcgtcctggtctgaaagagaagggaatgacagaggaggagattgataagatcttgatcactggcatagagccttcgtggggcgatagtcctggcgtcattttcaaaacagtcaccatctaatgggatgtgctggctgtggccgtcgtagctcgcgcattagttacaacggcagctccgctcctcagacagtaatcgaagaggacgatacgttaagcgctgcgcgtttgacacctcacggctgggtacgcacctgcgttaagtgtggtgctgtctccgagccttcatcttttgcagagaacatagagaaaccgtgtgactgcaaaacagacgagtgatcatgatgaacaatctcgttggtaccgctgtagctttagaccattgtcgcttctatgcggagaacatggtaaacattcaattcgagcaacctctggccgctattccgcctgaacctacgtacaacgaaccgattaaccctcgcgttctgcactctctgattgacggcatccagactgcgttcgacaatgcaatcagtcgcactgatctgcaattcccttacgcgccgattctgtatcgcttccgttctatctacggtgtgtactgtaatcagtatctggatgaagcatcgatcaaacgtgctaagtccgatcgtcctgctttactgactgtatcgcagcctgttccagttcgtgttgaagacgagcacgacagagagtttgcttcacgtttcctcaaacacactgccgaccaagtcagtgcgttcttgtatatggtgtgtctcgaccaatacgcccgtgagcaaacagactgctggttgcccgcacctccgacgccattcgatctaccgaagaacattttcaacgacagccctatcgcattcactgctacgcacaatgttttgatcaatcacttgatggaagcaatgttgcagacgcatagcgatacgctggatattcatgtgtcgttgcgcgattacggcctgtcagtgttgttcccgcttgtggcggaatgtcgcaatgtgatttacgctgcatggccgatcacacgcgaatcgttccgtcagcctaagttcatggataaaggcgaacacgtaatgtttgacgacttccctattgatgatgacagggaagagttcgagccgattcctacattggggcctacgttcgaacgtcaggctgagtgggttactgtagcgactgaaattgcgcaggtattcaatctgcaagcgttcgcagatgatggtgattcttcgttcatcttaaagcctgcggtgtatcgaagcggtgaagacttcctgttctggtctgagggtcagttgacaggcaaaagcattctcgatatagccgtgagccctattaagggtcaagcgtatcttgatctcgaagtgctgctgcgtagcgtgagcgcaacaattcgtgaccgcgcagagcagaacggttgccatgttatcacgcgctacatcgatcaggaagaccagaccatcggtgtactgattcgtgttcgtcgtgacgttgatttcccaggctctgctctggacgtagcatctcatgtggagtacgcacaatgacagaccaagtaatcactttcgaagatcaacagagctgggaagatttcggcagcgcggtctatgaagaatttcgtttgaacacgatgactggctccagcttcgcctctcaggtacccgaagtcggtccgaacgaaggtgttaaacacgccatgacatatcacaatatgtcagagaagtccgataaagtcgtgttggacattcttatcaacgaagtcgcattggccgaaggtgagtcgcgcaattacggcgcagccgagctggacgctgctgtgcgtaaagtcgtagcgctctaccaagcgcgagcgcgtgacctcaaatgtcacattactggtcagtatctgtcggaagagaacaatgtggtaggtgcgctgctgcgtgtctaccgcaacgatgacttcccatgtactggtcaccctgaactgctgctcggcaaaccaatcggtatgtaccactgcgataagtgtcatgagatgcaagtcgcaggtacattccatctgccgctggagaacgacaatggttaaaggtgggttatggcgtgtcttccctgactatgactcggaagagatgctgatgaagctcggtgccgctatcggcattgagcacgacgaagacgatgtgcctggagaactgcacgttactcttgcttacgacgaatctaatccaaacgtcaaggcagagcagaacgatgcaggccagttcttcgcagtcgttaaagaagcaacgttgtttggtgaaggtcaggataagattttagttctggtactcgaatcacctgacctgtgtgctgaacacgaacgcattcacgcatgtggtgccgctaagtggtcgcacccaacataccacccgcacattacgttattgaagcaagcccgtgatagtcaggctgaacatctcaatcagatcattcaacatccgggtcgtcctccaatcactctgcgttttatcgaagaagatcgtaagatgctggagaagcgtaactaaaatcctagcggtggccctgtgctgccgcttttgttattctggagatatttctatgaaaatggtcgtaagcctaagccacgaaattcgcgtagagaagcaggacagtgctgctaatgaagcgcagactcagggcccaaccgatgcgcagcaaacagctctcgatatccaagagcgtgggcgtattgtagaggaatacggaattgacgcacctaaggacgaagtggaggagaaagagaaagaccgcattgagcgtgagcaggaaaaggaagatgaaaagcgcaccaaaccacccgcagatttaggtcagcataagtctattgaaggcaaagaacttacggcgaccgatattcaaaacgagcatgatctcctgacgaagatctagaaatctgtaaataagagtcaaagcaactaacaggtgtatttgaccatgaacaataagtcgaatctcacaggcggtcagatagaaagcgtcatggacaccatgttacatgattgcctgtgtgagattgtggagaacacggacatattcgacgtccagcttacctacttactgggtttggttacgtcgaataagaaacgaaagccatataacgctgagacacgcgaccgggcaataagcctactgattagagcactctctgtacctcgtgatcagaagatggttttcatccgcgaacttaaaatggagcgtaacttcatttacgtcttcctggaaaatgtaattaaacggtactacacggcgtatgttggattgtatcgcgcattcattactacgcaggacccaatcaagcgtgttgcgtattcaaaacgactcgacgtgtatgtgaaaatgtttggcgcagagtcgcgctcgaagttatttgtcgcgctctgccgtttgaatgatctactgccgcagttcatggaatacttccactcggtagttgctgacttctatcgtctgtgcagcaagcagaccaagttctatgttgataccaatcgtggtaaactctacgatagcaaagacgtgcgccagaacttcctgcgcaacgttatcattgcaatcaacaagtatgactcgtcgcgtggtgcgatagtgagttatacgaagtggtggattctgaacgcacaaacctgtagcagtagcgagcacgaatacggcatcgcgtacactattccccagactcaacgtaagaaactggcgacaggtgaagataccacttctctgaatttctcggtaagtctcgatactccaacgaacgaatctgatgaaggtgcggacgcgtccctacatcaaaaggtgagtgaccatcatcacctagaagatcacgttgatagtgaaagacgtactgaaaaactgagactgcttatcaagcgcgtagaccctctcggtgtcgctcgactaacgatggacgttggcgaggagttcgataagtttgaactcgatctcatgcgtagacatatgcaagctcaagggctagcctaaaactgtaaacagtgcatatcatagcacaactcaatattgaggaaatataatggcacgtggatttggtgacattcaggacaacagcaaacgtgatagtctgcgtgagtccgaaatctttgaaatcttcccgctctcaaagaaagcaaacggtaactgggtatcaatccgcctgttagatctcgacctgcttccaatcaagaagcactggatcaagatcatgggcggcaaagacaaagataaagaaatcaaaatcccgcgcatgtgcgttaacttcgatccggataatcagggtaagcctctgaacggtatgaagtgcccgtactgcggtattgcacacggcaacgacgaatctggtgcgccagcgcagtacgactataagtggtatgcgcaagcgatcattcgtgacgaacaagcggccgcgccacgtaaaatgcctaagttcactaagaaagagcagaagacaggcaagaaagaaatgggtagcgagtcttggactcctattatgtgtattcctctgtctaactctctggcaggtaagatcaaagagctgggtgaacgcaacattcacacggtcaaagacaagaaatccggcaagaagtctaagcaggcatttcaggtcaaccatccgaagtacggttgtgatatcgaaatcaaatacaacccgaaaaaatctcctgctgaacgttacacaatcgaacgtggtgatcacactccactgaccggcgatgaaaaagaatatctgacctgggacttcgacaactggaacgaaatctacgacatgctgggtcgtctgaacgaagaagccgctatggcagacttcaaaaagatggacgttatcggcgttaacaccaacgactctgacgatggtgatgacgaagacgatgaagatgacgacatggcgctgggccgcaagaagaaaggcggcaaggcagacaagaaaaaacgccgcagcgatgatgacgatgacgacgaggatgatgaagacgaagatgatcgtccatccaagtctaaaaagtccaagccgaccaagtctcgcaaaatgctggacgacgatgaagatgacgacgaagacgaagatgatcgtccatccaagtctaaaaagtccaagaagtctgctaagtccagcaagacctctaagtcgtccaagaagtctaagaagtcagatgatgacgacgaagacgaagacgacaagccagcgaagaagaaaaagaaatcttctgataaggtaaaatcgtccgataagaagaagaagaaaaagtcttctgacgatgacgacgacaagcctgcgaaaaagaaaaagaagaaaaagtaattcgtgtctcggggtagcttaggctgccccttcttctctcaatctggactatcccacaatggcgaaagcgaacaacaaggccgagaaaaaggccgagaagaaagctaaagttaaagttaagaaaggtaaagcagaagcagtagcgtccgacgatgttggtggcgtagaactgctgggctttgaccttgcaagtctgatggacgatgtgcttgacggcatcgaaaagaaaacgaaagtaagctcgcaagatgcggcgcgacatgcaccacgtatttcgacgggttgccttgcgcttgatatgtacctgtccggtggtatcgtacctggcggatggtatacgttcagcggcggtgagcagtcctgtaagtctacaatgaccatgagtatcatggcgagtctgattcgtctgaaatactctggcattagcgtagtgttcgactacgaaggttcaaccgatgcagagtacgttgcgggtcagttgaaaacgtttggtgttaaggtcgacccgaaaactatcttcggtgtgcgtgacgacaaagacggtagctggatcgttaagcctcagattcgttactacgcaccagacaacggtgagcgcttcttcgactacatgtccatgttgcgtcgtcgcctacctgacaagatcgttgagaaagacggcaccgcgtactacatctttgagaacaacaaagagaacgcgaagaaggttgctggcaaatacgataagaaatggttcagtcgtaacaaccagttcaaagtgcctgcgaacgatggtcacatgcaggcgatggttatcgttgactcctatcctgcgatgatgcctgatcaggtcgatgatgatgacggttcgaaagcaatggcgctacaagcgcgtatgttctctgacggcatcaaacgtttccgtggcggtatgcgtcgtaagatgatgaccatcgtgggcgttaaccagttgcgtcagaagcctgctgtgatgttcggcagccctgagtacgagcctggtggtgacgcgttgaagttctactgcttcgaccgtgacactctgattcgtaccgaccacggcgtactgactgcacctcagatcaaagagttgctggacgctggcaccgaagtctctgtagaatcgttcgacggctatcagaagatcaacggcgcatggcttgtcgatgacgcaccgttcccgttcgagttgaacgctggtggtcatgtgtatgttggctcggcagaacatcgccagttcactctcatgcacgacctgacggccgaaggtactcctgtactgcgtcctgagtggaacacgctcaatcaactggcccagcatccagaagcgcagggtcagtacgctggtctgcgtgtaccgccagttaaggaactgaaagagaaagttcctgatgcgttcgatgcggccagccagcgtatcaaagaactgcttgagtcttcggttatcattgataacatccctatgactctggctacttctgacggtaagttgctctgcggtcacatggctcaactgcctgaagagttcgttggtcatgttagtgatttgctttcaatcggcatcttcgcctacgttgataacaactctgatgtttgggttcctggtttgactgctgatgatattctcgatgcagtagcgcaggacgaactaggcgcgtacgcgggtatcagtttcgatgcgacctgccgccaacgtcagactcaaatgctgtcggtgattgcagaccacttccctgagctggtgcgttacgttctggactatcagttgtgggcaggcgaagacaaaatctatctggcgcctgagaacgacttcgcgcaagcgcttgacctgatcctgcataaagagatcgctggctacgatgacatgtacgacctgctgatgttccagctggcgtatgttgatgactggtacaacttcgactctgcaattctgcctgtgccgtttacgcttcgtgcgctcgacgagcagcgtgagttctgggatgtgaacgttgaagaaactgcggtagttattaccaacggcttcgtcagtcataacagtgatgtgcgtgtgcgtctggcttcccgtgcagtacctgaaggttggccgaagctgaaagacgctccaggcatcgtcggtgagaagtctgttaccgtcgaaggtggtactgaccgttatcgcttcatcgctgctaagaccatcaagaacaagatgggcggtatcccgaaccaacagacgtggttacgtttgtgggaagctgatggtaacggcgaagcgcgtggctttgacccagtgttcgatacgtggcactacctgaaaactctcggtctggtcaacggcacccgtaagtcgttcaaactgaaagcaccgtgcccgctcgcatctgatgttaagatggactgggatgacttccgtactcttatcaacggcagcaaagaacaagttgtcggcgtgtgtaagaaactgaaagtcaaaccgtcaggcctgcgtctgtggtgcttcaagttcgttcagtctgtcaaaggtaacgacatgctgaaagctgctatcagtaagtctgccaagaagtctgatgacgacgacggcgacgacgagtaatccctgggcgggcttcggcctgctctcctttctggagaaagaaatgcgtactcaaatctacaccgctgatattgttaatctggagaccgttgtcgttgatgacgaaggtcaagagacacgtagcccgacaatcgttcccaatctcgaaggcgaacgtgacctgactgttagcactctcggtacaatcatggcgaccgtgactgctgaaccaaacgctgatgctcgcatgatcgttctggtatctcgcgctctggttcctgctttcgcagaccctgaaggtgacttgttcgatatctttgatccaatcgaacgtgttgctgatgttgatgctgggaacgtcggtagcgttctcggtatgcaggtagtaatcaacgataagtcagacgacaacgttctggccatcgctgatgttctcgacaatgaagctggcgttaccattcgtacctacggcgcagctatcattcgcggttaagtaaaccctgtgcgggagaatgccctctcgcacaatccatctctcgataggcaatacgccacgagaaaacaaatcactcgataggcaatacgccaggagtaatgtatgaaaaagattcaacacgtagttcttccgaccgatgccctcaacggactcattcatggttattatcaccacagcaaaggtacggacgaattttgtaagtcactgttctacattgacgtgactgatcgtagcgcctccgatgcgctatactctattctcaaacgagacaagacctcaggcattgttcctatgggttacgatagtcaaaaagatgcgcggggtcacacttctcctgcgtctttggctgttgtgctgtctaacaatttactgcatctggatgacaagaaaatgtccagaggcattttaaccatcttctctgctctggctagaaccacgcacaccaacaatacacaaataactgtgtatggggagcctggcgtagacaagattctaaacatagtgcgtagcgttgactacaaggactatagtgaaggtgctggtgaaggtacagatgtggtgcttggcgactttgatcttgagtcaaacatgactatagaccatttcgttcacatggctatcgagcctaagttcgaagacgctatccgcaactcgcctgcgacagagtttaaactgggagcaaactttatgttcatgcacccagacgaactggctaaggttgtccgcttgattcgccgttgcagtaagatctgcatcatgcaccctgacatacatcgctattactttgagaacgtaatctgtaaatactgatcaacaaccgaacacattgctgtgtgtagtctagcctgatttgggcaggggagagccggatggcctccccatttttttatctacagcagcaggagaacagcatgtctaaaacgactcctcaaatcttcctcgacctgtttatcaaagacgttagaatctttctgcctaagttcgacaaaggcctcgatgcttacttcttgaaatgtaaaggcaagcctggtcagtctggcgtgtcgttgcatcaatatctgaaatggttgaatcctacagccaaaccaccagagaacgcgagcaaacaagctgtggttatctctgggtatctgcattacttctggcaattgtctaaaccaaactttgtgtttgaatcgacactagttaatcatttggcagactctgaattgcctgataggttgccgacagagatcttgaagaaactcccttactggtgtcaatgggtaacattgcctatacatctggagaatgcgttcaggactttgcatcttgacttcgatggtgcttttgttgggtactctcagatagacaataggcctgtactgattttatgtgctccctttacgccaggtgatgaaagcatcaagtcaaataacttcacaccgtctgtaacgtcattcgtatatctggacgaacctgtcgacccttggtcaatgctaaagaacatgcacctgttaaatctggtcgatactcttgaggacccagacttccgtgaactgatgttcagcgtataccactacctgacaaaagttatgtgctgtgtgatgtacatctgttcgcagcaggaagcgttatatacagaaggtcatactcagcctaagcctcaacgtttaggcaagagctatcgtatcactccgcctaagtcagatcgcatgatcaatataggttcggagatgatgcagattatcaaggacttcgaatcagaagtcgaaacgtgtactcgcgcttttaacggacgcaaaccgcatctgagaaaagcgcactaccaccacttctggacgggaccgaaagctggacctcgtaagctcgtttgcaagtggttgccgccaagcgttgttcgaggcacatcgcctgagtgacgtaaatcaatactccacgtatgggcgttatgcccggaggctattatgaaatctcgtgtacaacatgcgtatattcctgatatggaatcgtttgacccttacgtccgttctctgtgccatatggcgcgagcactggacacaccgaactctaactacggtaagttgaaacgtgtcgtgatcattggtacgtcgaagcgtgtagtcgaagcctacgttaagcagttactcaacacaaacaacctgccacacactctcatttgttttggtgtagatgaatcgcctatcagccaccgagactattcctatgctggtgcccacgttgtgctaatgcacgatctgacttacgttgatagtggcacaatgggaaaggttgccactcgcgtcctagaaatcatagacagcctaaaacagaaagaaggcgacactgaactcaaaaacagcgagctgtctttggtctactcgaacccgcacctgtggtctgctattcttgactacggcgctgcttcattcatgaacacggcgggccgcaacattgaataccgtagcggtttggtttcatctatcggtcttgacgcgttgatgaaatgcgaaagcaaccaacaataccacgagcttcgtgcagaaacgattactataggcctggagttcttctgcatacacacggactacctgctatccaaagtacataatctgttgtggtcactctcgtgtgatgattgcaagttcaaaaagaatcaccgcatcatcttccatgaagactttcgtcgtttattcttcgaagaatacatcctaagagacttcaagggcttttaagaatattcttagcctgctctctaatttcaatatgttggcaagtagtgctgacatatcgttattggagaataacatgtgcggacgtagcctcgttaggttgaagtacctcgcacggtcatcgaactggtgcaataataaagtaaacgcttgtagtgagcggaaggcgaagaatgtgcaatgtgaggaatttttggcagcgaccaagaattgccgcagcgaacagaagtcgtccagtgtagtttctttcttcaaaggtcatgagcttgttggtcaggctatatggcatgagattgaaggagacagcacacttcaattccggttgctacttgcttaacgacagagggcctttcagattaacatctggtgggccctttcttctttatatgctaattttccctgtcattaacacacaaacctatttcggggtaacactatgtctttgattaaaatcgaaggcgtccaatcattgtctgcgcccaccaaagctcagaaagacgccgctgtttatatgtttggttccaagggccattcaatcgttgctgtgcttgacaagttcagccgtgcgaaagaagtgcgaaccgcacacatcgacggtctgctcaagctgatgaaagagggggacgatgaagaaatcatcaagttcaccgcatctgctccgggcaagaaaaccatcgcggctgcgaagcagttcgctgtagcaaaaacactgaccgctagcatcaaagcactgaaacttgtgcgcgttccgatgaagtggatcgaaggtcactcggatgccgctgctgctcgtattaccgagacaaaagaaattcgcgcacgtaagaccgcgggcaacaagcctgagaagccggtcaagctcgacaatccacatgcaccagaagctgtggacatgagccctgctgctatgtatgacgatgcgctccgcagtaaaaacaacgggccgtttgaagctgtacataaagcagttaaggctatcgtcaagcagtttggactgacgaccgagttaagtacaggcaagccaggacaggcaataatcttggtcaagaaagggcgtagcgttgacggtcgtatttcgttcccgtccaacaaacgtaatctcgattggccacaggatgacccgaatcaattcttcctcagtgctgtcaatgacgaagaacgtgatgtggtcatggactattattcagcgccagttaagacagcacctcaggtcatctccaaagcgtttaaagccctgtgggtaaaatctgctgcgggtgagaacggcgacctgcctgtacgtcgggtgtctggcacaaaaaagtcaaatccaggtaagaaggaaagcagcacttctattcctggtaaaggcgcgacaactccatacacgcctacaggtaagtctcctatctcgctggtggatgaactggcggaagtaactgcccgtaagatctcagccaagcctctgcaggagcgtgaagaatactttaatgcgctgcgtacggtactccagaacaacctgcctaagcgtgaagtgtctgcaacttccactggtgttgtgattggtggaagtaagctgcacaccttacgtctggacaataacgcctggacgttacagacaggcgttaccggtaagattaagaagatcggcgccacgttcgatattgttgacctactgggtatgctggacaagagcattctgcgtcctaaaggctaatagcagtaaatcaaaaggggtggcttcggctgcccctttttgcatctatacgccctcaaatctgcgaagtctgcaaatactaggctgaaatagctctttatgcgcatacgtgcctatgatacaatatatgcagacgctacacgacgtagcgcatacaactcatgctgaggagcatacaatgactactatcaaatttgattctgtttacgacctgtacactcagattgacgaatgtcctagaggtgttgattttaccgaacatcttggcttcgacacagacaaggtagaaattcttcaatgtggtttgcaggaagatattggcgtatacgccagcttacctaacgccaagaacattctgatcgccgacacagatgacctgtgctcagaacatcttaagggcgaaggagagatcactgtctgcctgattacaacacctaacggtgagatgttcgatgaaccagaagttgaggtcaaacagctcggtacgttcgatgattttgatgaagcatacgcagcattcaccacagccgtaaacgctgaactctgcaaataataggtcaaaagcgctatagcaatatagcgctatttatcgtactatataatctctagcgcaatgatgcgcacatacaacacttgccaaggggcatacaatgaaagcagcaaactttgataaagcattcaacgcgaaagatgaagcaactctgaacgcatacgcagcgcaaatcgttgaagcgctcaacactctgggacgtaacgacctgaagatcactatcatcttcggcactgacccgtacggcgagcgcccagacttcgttaacgaccccaacggttttcgtatcgtacagaacggggaagaaattttcgatatctacaccccaactgaaaaacagattgaaggtgatgcgtcagacgctttcatctacgcttcatgggcagacggcgtagcgccgtggggtaaagaagtttcagacaatgacgttgctgaaatcgcagcgcacctgaacactgcaatcccagctctgtaacgaacaactgactgcggggttacggccccgcttatatgacaactcgccaagagaacataatcatgaccagagaagaactgactacactgattcgcaactcactcacacgcactgacttcgcagtaatgaactgcgtagagcctgatgactacgaacttgttttgctgtatgaagtagacagcgctggtgaatcgcttggcgagatgggctatgaagtagaattgaatgatgacggcacattctcgcttcactaccttgagatgccgtggtctcctgagccgttcccgtcattcgctaaaacttcgaacttcgacgaactgatggcagcgataaacagtatcgagtttcacgtttcaggcactaactaacactaagaggcaacaatcatgtcagagaaacaaatcatcatcgacgtaatcgcagacgtagcatcaccaacagaagttgtgtttgaagatggcgagtcttctactcaatggctcgcgccgttcgatctgcgcttgactgtggcccaggcctgcggtccggccggcgtaccagaagtgaacatcatcggcgatgaagataacctgcgccgcttcttggccgcgaacgatcagttcgaagacgctgagatcgtagacgttatctaacaaacaaagagcggcgcttcggcgctgcttttctatttctgcctgagaatgctgctatgaaaaatcaatatctcattattcgcatgaacgctgcaaacttctacgacaaacagtttctgatgcgtggctttaacgccaagcgtatcgagcaggtcattggcgttatcgttatcataggcgatgaacatacatactcgctgaaagacagcatgtatcatttagcaaaaattcacgtcgaacagcttacatctgacacacaacaaaacttagttaagctgcgctggtcgagcgtagacagcaggcgcatagaagaaggcttgacgcgcatacccactgacttgacagacgccatacgtgcgatgcgcaacactcgattgtattatggagtcgatacgacaatcccacaggcgtttcgtgaatgccacactgaatttgatttacctactggcgcgcaaatgcgtgagcgcataaacaaacgacaacgtgaagacggggcaaagatcaaacttgttgaccgatcgcacgtaacgaaagcgcttaacgattgcactgtggaagaaattctaaagcatctgaaagagcgcacgggcgctgagatcacaatcaagctgtaacaactaatcaatgtgtggcgttacggcgccacatcatcacaacttaatagagagaatcgcatcatggctatcgtaacttttttcgtaaaacgttcttatgcttcacttggtgcaggcaacttcgctatcgctgcctcacaggtgcaagagctggcagaagctgagtgcttcatcgtctacactaacacgggactgggtaacacgttcgctgtgcgtaacatcacgatcacaccgctcgatgaaaacagcgtgactgtttcattcgaccctctcaccgatgttcacgcgctgcctgcttcgattctccctaaagagattttgaaagagtcagtcgagcgtatcgtaatgccagaagaagatatgcgtgaagtgccacgcttctatatcgccaacgatgcaaatggcaataacccgaacctgcttgcgcttgatctgaattgccgtcaacgtttcgtgcagtatcatggcggcctgtgtacactgaccgatcttgtgctggcgctgtacgagacaggcattcatatctctgacattcaccatggagtgaagcagaaaagcaacgttgctgccgtactcgcacaatatccccgtaccgtgtttgagcttaacaaagataacggcgttgtgaacgacaacttgcccgtgttggctcgtatgaccgtactaatgtaaacaactatcgcctcgcattgagcggggcttttctatttggagaatgttatggtatacgaacgcgaagaactcgaagtcatgcctctcgatgtactttatcatctggcgagtgccaaaggcctgctggacgatttggacgatgatgacgatgcacctgatcgtgaagtgctggtgggcatgattctcgatgcgcagaatgaacagcaactggctgatgaagaagccgaagacaagcaacgtgccgaagatgatcgcgatccactaatcaatcgccgtgacggtcaggatggttctgacgactactgttaagtaaacccagaggctgccagcgctggtggcctcactcacaaagaaggagtaacaatgaagcgcaaagtaatattgatagacacagcagagtttcaaagcaacctaccgatcgcattaccgtcgattatcgacttcactgatattgagtcagtggtttttgtcgtgaaggcgaatgcagagttcggaggcatcgaatatctaggcgcgtacctagcgtctgagatcttcgtggactatacgaagataccgttggcgcaaacgatcaagatcaacgcgtacggtgtcgtgccgttagaagaggcaatgaagcgcaatcttcaaaacggctatcagtacacggacgatgtacctgacgaacacaaacgcatttattctgcatcgccaacaacaataacgttcgcgtagtaactaagggctgccattgctggtggccctttttcatttctgtaaatacctcgtacattaattaatgcgagatattcaatgcgccgctttctgacagtctttaacgtcactcaacaggagtttgacgaccgtcgctttttccagcataagctgaacatcattacgaccatgcgccgaactcatggcgtgttgttagctattcgtgagacaggtaaagtattcgtagcctctaccgcctcatatcaaagggcagaagaatacgatctgcgtcgtgtggacttctctgctcctagtgaggttacgcacgaactgggtgaatgtttcaccgaactgaaacaggcaatcgctaacaacctgcaggacaaaagtattcgctacttcggccgcacgttgtctcttgacgatgtgcagcaggctctgtatcgcacacaactggagattatctcatgacaacaatcgcatctctaggcgctcgatttgccgcctcatcctctgagcgttgttctgctcgtaaaaagaaagacccaaagaacaagacgatcacctgtgcaggcacgacagccatgtataacgccgtagagagactcgcaatcaaactcaacgtgtctcgctcccgtgcagtagagattgccattgaacagcttatggagaaacacggaattgtcgtggagggtaccgatgacaactgatacgatctactgtcgtctatatggcgttcagtatcgtctgggtgtcactggcatcgacttctcacaatcgcctactgtctacacagtacatgcctgtgacctgctgcgtatgctgccgagtatacatgtcggggctgcctacagcacgtacacaccgtaccgtgtgctcaaagccggccgtgctgacttcaagatcaaactgattgagaagataagtgctgacgagtggcgctactcatttgttgacagcacaggcagaccattcaacactattctgaaacggagaaagtatgaccattggtttgatcaaagtcttaggcctaaaagacaaggcaccaaagggattcgatcttgatatcacaccagtctcacgcgatgatgattggtggtcgctgagtcctttctatctgggcccgtgtcgtactcctgacggtatgatgttcctgaacatggagaacatgtggcagtacagcaaggtgtacgaagaacatcttgttaattcgaacgacctgtttcatggagagatatccagcgagtggtgggagtggcatttgaaaggaagtacaaccgaacaggcgcatcgctatccagcggggaagggtcgaaaggctttattctcgaaatggggcgacttgcgcctttcgtacattcccgcacgaaaacaaatctacgtgccagaatatgcgaagctggtgatccacaagcctaagttcaaacgcttgttgaaggagtataagaaaggcgccaagatagtccttagggattatgacacctacgatattcaaaaggcttatccagattctcgcagtccgtggttgaccgccattcaaaacgagaatgcaaagtttggtcatgcgtttgtcattgcactggccttgatgtttcacgaacgaccactatggtacaaccaatgggtaatataaagtacgaagcctgcattgaattgagtacacgcgaaggcaacatcaacatgccagaactccctcgctgtgatctgcaatgtcatcttctcgatagctacacgcagatcaaggtgcctgtgcgtttcgattgcactaacatagttaaggtgtttagcaagacgtgtggtagcctgcaactaatatctgccgctaatctgatcgtctggtcatcgttcgaacctggtcgttttacgttgtatatcgaacgtgcctcaagcgagagcacaagcgcccagcgagctgctgaactctgcaaataattggctgaaatagccattcagtcagatacgctcctatgatatactatatgtgagcgcgatgctcatacaactaacgcttaggagcgtatcatgactactttatctatcgctgatttgaaaacccctgctactttcactacgaaccttactttcggtcacatggaagaattgcgggccaacctcgaacgcgccttgaatcgccctgaccttgaggtctatgtagattgtgattctaactacacaatcgaagaagcaaacaccgacggtcctgatcagctggtgggcgaccatgaatgtattaacgttcacgttcgttactcgggtatgtcgtttgatgaatcaacggctaaaggtgtgtgggatgttttgttgcagaccccacatgaagataacagtataagtgaatggtcgaactcatacattatgtatatcacggacgacaacatggacctgttagaggaggtaagtattgagaacggaaatccacgcatgtatgaaacattcgttgaccgtctgaacttctggttacctaagctgtaagcgatttgtgaagggcatttgcgagtgccctttgaaaatcctaaaccctaagctgaggagcttaacatgtcatcatctactactttgactttcatcttcccagaactgaccactctggaagttaccatcggtaacggcgttgttcctgctcgccttgaagtagcagagaacaaaagcaaaacgttcagcgatattgaagcgctgcgcctgatgcaagattcaaacgttaacggcgtaatgtctggcttcgatctgtcgctgttgaatctgcttatcgaccgtcacaacaatcgtgagcatttccactgtcaggaatgcgtaatgtctggggcaacgtacttcccatcgacgggcctgtacctgcgagtgtcgcatcaccgctaagatttgtgaagggccttcgacgagggtcctttgaaaatcaaaccctaagctgaggagcttaacatgaaacaatatccacgccgtggccaagtgtactccctgaaagaaatcgaaaacgagctggagttgcgtgatagcccgttcttgcgtttcgtgccgcagaaagttcgttacgaacacgaggtatgtgcaggcattcaggtcattcagacctcgtcagttgctaatctatctgacattgaaggttgggctgatacgcagtggtcatacgtgcgcgagaccgaagagtggattccgctgttccgtgctgttgacgacgcggcgattgaagcgctctgtgttatcgagcctgacacgtctgagtttcgttcgggtggcggtatgcacatctatccgaaaggcaccgtgtgcaatcagcataagccgtacgatgaaaagctgcacggtgatatgcttgtgagggtatcatgaagggattaatgaatcttttcaactgttgggctacacgcctttctgagcgtacaatcaaaattgcatattgcgtatatgtcgcattgtttattttggttgctttcatgacaagcccgtgggtgtatgactcgcctataggcatgtggatattctgctgcgttactgtatgctttgtggcgccgatgttcattgctgttctgattcgctctaagacttgctaataaaacagggatgctcacaatcgtgcgcgtcccatttctcatttaaggacaatttccctatgataccagaactcactcatatctttaacgtaatgatgaccagcctgaaagatattcgcagcgttgatcgtctccatctcattaacaaaagtgctgtgcgctttcatctcaagggcaaacagttcgacgttcgcggtaagtttccgttgttgtccgttcatgaagttgaaagtcactgcctgtcttattcgaaagccgccaaagagattgaagcacaactcaatggtgaccctatcgaagaaatcgaagacaactcccatgataccgcactggatgaagtgttaatcgcccacgtcgatagcatggaagaagatcgtgttcgggcgtacaacgaagaatgtggaggacctgatttagaccctatcaatatgcagcgcacttggctaaagacacatttcctgcatataggccacaacacgcctgaccttctcgaaacagttctgatgatggaaggtcaagagcgtcatgacgcactggcaggcgccgttaaggggacattatgtttctagcgtggattaaatacctgcgcagtagaaagaaccagcagtttatgattgaagtaacaacggcaatcggcaagttaaaccagcgtgaccgcgacctactatgtcgtgtattcaatctacctgctgatgcagaaagtttgtttacgttgtctaacatgaagcgtaagcaattggccgagcaatgcaacatgtattatgccagcgtgtctggtaaaaactgggacgtgtatgatacgttcctcaaagtcttacacaacgcaagaagaggaaagtaaaccatgaacgaaatagatattctgatccgtgagtatgaccgggcgtatctgaaggcagaagcatcacctttcggtaacgtcgcatatcacgtacaagatcaaacggacggcctgaaaaacattgcactctatctgcgttttcgttctggtccgcaagctctttggcagcgtccgtgtttagtgctcgccacaattgatgttcgtgactcaggtaaaggtacgttcagtgagttgcttcgccgcacgaaagacctgtgtcgtgaacgtgactggattcttcaagttgaaaacgttctgactcctcagttcagaaagttcttgcagcgtggtggcttcaagccattcggcattgataaagacgtaccgtacggaagtctctactggttccatgacgagacaatcccgcagcaatgctctatgtacccagagaggccacacccatgaacattccttggtacgttatgttcatgataggcctgctgccgctatctacgtgttacgttgtctttccgtggtttcgtgctgctgttaatcgcagactgacattcaagcctcttgactatgatgcacttgacgagatactgactggtggtatgcctgagcgtgttaccattacgtgcctgcaagccgcatataggtctaacaccccagcacattctcatgtggatatctatccgcacaaagagaacgttgctgtgattcgaatgctggtggaccctaacttccctattgcacgaacctttcacaaggtcctgatcgataactatagcgcgttcgctgtgaagtcgaacagagcaccgctgatcacaatcaatcagtgcgtatatcctgttgttgagtatgagtatgacgatacgtacctgttgatttacgtcaagcataagtaaggaaacatcatggtcacccaacagcaactaacagagtttgcctcaatgcctgtactccaccgtaaagtgatactgcgcagtatgcaggttgagatgttgggtgccttgcctgagctgactgacattgtacgtgagatgctataccgtgcgattgtcgttgacgtagctcaagctgaactggcactccttgctgctcgtcagatgtgtgataataaggacgttcgtaagagtattgatgacctgcttcaattcgctgcacgtctgcacgacgttgcaactgataactttctttctggagatttactatgaatacgactgttggcctgatgattgatgaagacgtaatgaactggctggacatgttgcttgctggtgaactcagcaacgtcttaggtgcgttgaacaatattgtatacgcccgccgtcaggaattgtctgtcgaacgtctaacagaagacgaagacattgccgctctttctcacaaagagttggaaattatcctgcgttacgcttcacctgagcatgagtacgacacgtccgtgctgtctaatgagcaattgctacgtttggcgatggacgcacaaggtatcatctcgtacacattgccatgccactgttcgcctatcatggttcaacgtgctttcgctaacggccagatcaaatcgttgttgggtagcttctctaatcgtgctgatatcgtcatggcagttcatcattgggaatgcggcctgactaacatctcacttgatgctattgttggaaatgatgtgcgcccagacgagcaggggctgtatctgtgttacgacgaacataaacaggtacgttacggtcgcctgttccgaaatgccaatgacggctggacattccatgaatcgtatgctgctggcggttcgacttcgtggttcgaagagggcgaaggtaaaggtcttgacgacgatgacctgccaatcaacctgctatctaactgggtattcgtagcgcctgatcaatcaccgtcaatcattcgcaaagagacggacattaaacgtctgtctgaaacacaacgcatcttcctgtatttgcgtagcctgagtcctcacgtcaaagcagaaatcgttgcgcatttcgatggcgtgttgaacaatcgcgtattcacttctgttgagcagattggtcgccttacagaaactgactggcgcaatgctgctatcgctatcggtgaagaagaacgaggtcaagaaggcagacacttctgggatgaccgtggtgcttggtcttgtttcgttgctgtgctcaactctctgtgctatgacatggagacacgcgacttccaacctcaatacgaatatcaagctaacgacgacactctggacgacaacaacaatggctaaatcactcggtgtatacatgacttacattctgcgacacaagccgcaggatatcgggatcgcaatggacactcagggttgggtgtccattcaggacttcttggaaaaagcgagctacaagaataagcccatcacacgcgatcagttattggctgaggtagttgaagacgaaaaaggccgcttccagttgaacgccgcgcagacacgcattcgttgcgttcagggtcactcggttgagaacgtcatcatgaacctcgaaccatacacgctaatcaccgaccctgtgtatcacggtactgcggaaaagaacgttgcttctattctggcgcaaggcctcttgaaaggtaaacgcaagcacgttcacatctccgctaatgtggctacagcgaaacaagtaggtcaacgtcatggttctcctgttgtgtttgagatcgacacttacgccatgatcacgcacggatataaattctaccgtgctgagaatggagtcatcctgaccgaccacgtaccgtccagatatatcaagttggtgtagtatggagaagacgtatatgcgtcattggggatcgcgctatgtgcggtcctcctccggcaagtggtattcagttcatggacgtgagggtacgtgggtaacgaatcgctacggtacttcattctatcgaagcggctccgaagtatggcgtgacataacccgcgctgaccgcgaatcgctagagcgtgaactaatcaaacgcaccaacgaagactacagcgagcaaaagcgtaggtacgaatactggggaagattggtacgagcaattgctcgctgttcagaagaggaaaagaatgagcacacggcagaacttgccgagatgattgaagcgcttagacagcaattctatggacagaaggtgcagcaactaagcacaatgttggacgaaatcgccgttaaagaataggctcgttcgtgctataataaagatgaacgctgtacaaccctgtacagctacttacatgaggacatgtatatgaaaaagattaaacacactttccgcctgactgacctggttagtatcgccaagaaactccctgcgagcatgagcgccttccctaaagatgaacaggcgatagttgtaggccgcagtgatgacagcgaccaatataccttacacgttaaacgtgtaggtgaagtctcatggtacgaaggtaaatcactgactctgattagccataataacggcgaactgcttgaccagtgggaagcgggtgattatggtagtgacaagaaaaagaaacgcaagatcccaaaagaactgcgtaacttcacggcaatcctgcctgtgacctgcaatgccgattgttcgttctgccctgagaaagagatggagcagaaagccaatcagaaagaatggcaagatggtttgattgcccagatcaaacgcatgtacaagaaaacgaagttcgaccatgtatccatcagtggcggtgaacctacgttgcgcacaaagttcctgtttgaaacgatcgatcgtattcagaaagaaacgccgattaagcgtgtgggtctgacttctaacggcttcttccttgagaaaccaaacagcacgttcgacttcttagaccgtaacactacgcctgagatgaccagcaagctgtcgcatctgaatatcagtatgcactcgttcatgcgtgagcgggccaacaagatcatgggcgttaactacaaacagacgttggaagatttggttcgcttccgtcgccagttgggtcgtgacgttagcttccacatcaacttcgttattaacgatcagacaggttcgattacggaagagttcaagatggccgcaaacttcatgcgagccaacccattcatcgacgttgtgttccgtgttgactacaacgatgttgaactgtcgaaagcgttgcgtgactacgctatggaatatgaagcgtggcaggaagcaagtcgcattgcagtagcaacgcgcaagaagtgcaaagtgaaagagccgcgcgcaccacacatcgttcagaagtttgatcgcttcttcggcggtcagaaccttgctgatgttgaaagcgcttggactacaggatgtccgtcttgtttcacccatgcgtcgaacccagtcaataatagtcgcgcatatttgaaagcgtcttcatacgaaccgaacgaagacgaagaagaatacactgagcttgtgtatcacatggacggcgctctgtattgggactggactcgcaatgaccctgtgccgctgccacgcagtaaacgttttgacttcgagatgaaggaagagagggccgacaagcctatgcctcgtttgaaaagcgcgcctaaagcgaagactgtgaagaaagcaaaaaccgccaagaaagaaactcctacaacgagttccggaagctgtcactactccgcgccttgtagctatagccagggcacgggcggctcctgtagtttccgtagcggcggttgcaactattaataggggaaaagaacatggctaagaaagaacaagtaacatcgaaagacctcgaagaactctactctgttgttatggagtacgaaggtagcgagcgttatcgtctgtactcaatgctgactgtccgtaagttgcaggcgattcactacggacatacaattcccgccgacattctgcggctgacgcacggcagtaacgaatatgatttgcaggaagctattgccctgctggggaaaatgcgatgaacgaacgtcgaaacttttactatgatagtccgttctattatgggcttatcatttggcgcaaacgtctggccgttgtcagtgcaatgctaatcggtattctgatttatcacggccgttctgcccctgctgttgatgatatgtggttctggacaggaatcatcttcggcatagttggtggtgtatgctacattcgcatgtggtcctatgagtgctacctactcgctgctatgggccctctggacaacaacactgttattggtagtctgtcgttcgacaaacttgagcgtcgtcatgaactctggtacgagaagaagttcgggcacaaacctcctaagactaacacatggagcatcgactaatggccctcatgtttactgagaagcatcgcaaacaattcggacgtgacagcaaagacccgcagtatcatggagatgcgtgtgaggccgtgtacaaccatggcatggaattgttgcgtgagcataagcgcctggcattgcttatcggagcgaaacgtagaacgcgcctagataaaggtgctcctatcaccaagtgctttcgcaagcagtggattgaagataagaaactggcgaacgaagacactcgccctattgctatgttgattgctcgctttaaagaagtggctgtcttattgaagctggcgcgtattaactataccgacctacatactcgtcgtcacggctttactcgtcctagctacttccactggagagactgacgtggcaaagcatcatacgtttcgtttgaatgacctgtgcgcgatattgtccaagcgttgtgtgtttggtccgcagcaaggtgagcacgttattgttgttgggcgtcaccctgaactgaacgagtacaccgtgcattacgctaacggtctgtacggttggttcaaggcagaagaccttgtgctggtcaaacacgacgcccacgaacaacttgaattgtgggaagacgcatataacgctcgatgcgtccccgacttagattaagagagacaagcatggaaaagaaattctgcaaactggcgcacatcggtgctgacgtgattatgcctgctatcctgtacgtattgaacgaaaagatgcaggcaggcgtcaaagtagatcttgccgaagcgtatactttgttgaacgatacacaggctgtgtatcttactctggcgagcagccagcctgatcgctattacgatcaactcacgccaaccattcgagcgcttctggcaaagtatgaaatagagtgggcactcgaccacgcggcgcttacgaaatactgtcaagcgtatatggagagcaagggcttcactcatgctggaaacgatgtgtattcatatccagaagttgttttgtacgacaactatgaccgagtgttcctgcgctcattgattagtgacgcggaccacaatctactggaagttgcaatacaggacgagatggacgttgcggcagagatggacgagattgacaagaaactcgaccgagtagaagacggctgctgctcagagtgcggcaaagaacttgaaccagatattgatggtccgttcatgtgcctagcatgtgacgaagatgatggagaataaaaatggctgtaggcttcgtaaaagatgatggcgttaacgacaccatcgaagctaacctgaacaacgagattgaccgtgcccgtgcagagctgttgggtaatggcactacgcattgcgttaaccctgattgtggtgcagagattcctctcatgcgccgtgtagcaatgccgaacgcacgttactgcgtacagtgtcaatcaagccatgatggttctgcgctgagcctgtacaatcgtcgtggctcaaaagattctcaactgaggtagaaactatgttaagcaaaatctggactgcaatgggattgaagtacccgtcagtggatgttgctttacgcaagaacagaaagtgtgtgcgcattagccaagacggctattgcgttcgttctgcttctggttttgcatctgcgctgtcgcatcatatgtcccgtgattacgttactcttagttcgaacgaagaagctcgcgccaagatcattgaacgtgcgaagacgctggaatatccgtgcgttgtttggttcactggtacctcttttgatgtgctgcctgttgatgatactaatctagagtaccctgtacaatgaagctgaacaaatggaaagtgaagtcggtgaagaaataactgatattggggaaacacgtatcatgacagaagaagaatgcagagtcttcctagaacgtttgaaaaatcgcggggaagaacgtaagcctaccatcgaatgcgaagactgccgtacttctctggaagaaggtgaagtctatggcgactccgtatacctgtgtgagaattgctgtgccgatcgtgaagacgaaggagagtcaatatgaagaaagtaactgcttctgtacatgctgtacatggcgaacgtgttgtccctatcttctttggtgaagacgatggtaagccatacataggcaaagcgttttgggatagcctgtgtctgcgtgatgacttgtttaaagagcctgaaacgcagcaggttcttcataatgatcagcggatgaatagaacggagttcattcgcgtgtctactttccctgacgtgattcaagcattgcgtcgatgcacaaactacatccgttactttgagtatatcagtgacgaagacattgaagacctgagtgaagctctcagtcactgggtaaacgaggacgaataaatggaacatcaaaagcatttagaagcaatcaagcaaatcgccgtcaatcagattcaatcgttcagctacgtggctgcaatcatccacacgcaggctaacagtcagcctgaagtgctatccgaagtatggcaacgtcatatgtgtaccacgctaggcctgacttacgagcactggacgtactacaacgagcttgctaactacatggaactcggtatggttccatacatgcctgtgttgcaggtagccgtaactgctttcgttggcgcagacgttcgtgagacactggatcgtttctcttatcttgacaaagagctggtagtgtctgcgtatgaagtaggcaacgagtggctgttggacaatcatcgtttgatctgcacctgccgcgcaatcgactccctgatcagtctgtactctacgcacaagctggagatagacgaacaggaagagaatcgttgcatcgcctaccctgggatgccgaatatgccgcatcagtttgttgagatgtacaagctgatcgaagaggctcgtatgagtgtggacgggcactggcgaacacctctgcgttacttccactccaaagaacgtgactatctgtggaactacccaccgaacatgtccagtatgcagaatgttatcattcagacagacgccggcaccatctacctgactggtgcacctaagcgtggagatactaacgctaaccatctacgctctgtgtgaactgtaaacccataacatcgacctgattgaggtattgagacatgattaagaaagtgacagcgttcatcgctaaagatgaaatgaccgtagagcaaatggcggagaaacttaacctgtctagctacaacgcgattcatcgtggtggctatacggtagtttgtggtacagacagtcaaggtgatcgtatcagcttggtctgcggtccgtatgtattgcagcaaagtatctggggtgttcagaagatgctggacgcagggtttagcgagacagatgcgctgctggccttaggtctaacccgtcatgcttacaccgcgctcaagaagaaagagcgtgagcaaaagaaagctgccgagcaggctgctaaacaacaacctcgtcgcggctctgtcgtgtctctcgatgacctttaaggaacaagcaatgaaacagttattcgtaggtagccacccaaacactgtgaagttctctgaccttgacggacgtgatcgtgtttgtgagatccgtgtcctgattgctgcggcgtacactatgctgcgtgatgcaatcggcgagcaagcaaaagttgagggaaatactttccacggtccatggcttgtgtttcgcaatctcatgaacgagcatcccgccgcctgtctggaagagtatcgtcacgcttcgatttatttcgatgcagacacagaaggcaaggtaactgaaatttgcgaactgatcgaacagcacattgaactgaccagacagacactcgacctgcgtggcactcacaaacatcaggccgatatgatggttggtatcgcaagcactgccgattcaacgcgtgaagtaacgcttatgcgtggactgggtaaatccagaggcgatgctgtgcttgagactgaattgcagcacaacccacatcgtgccctggccgatgatctgcgcaagtatctcaatcatttcaaagaccgtgacggcgtctttgagttgtgtacgttgctgactaaacgatacggcaagccttcattcgatgactatgctgacagcacggtagatgaaatgattgacgaaacgtgtcaggctgttcagtcggtcaatgagcctatcgatcaagtgtacgacttggtttgccgtgcaatcctttcattcggtctgcctgctctccctgcggatgcagacgacaaagatgaccaggctgctgacgatgaaaactacgctctcgcaccttaagcagtactggcgcgaagcgatgatactgactgtgttggttattgtcgctatcgctcttccttttctcgaagtatgcaacccaacgttggtgatgcttgttgctgttatcgttgctgcgtacttcattgctacttgggcatgtaagcctatatacggacctgacgatgaagaagaaaaatgaaatcaaactgagcgctgcggatatagcaacgggtatcatctgcatcaacgaagctctggctaagcacggcctgtcgtgtacagacggcgatgttggttacgaaactgtgtacactgacgagcatggtgaaacgcagggtggctggtacgccgagtttgataagaagtctcgtgagaagctgcgccaatctaagcaggtgcactggcgcaatactggaatgctcggcggtgatacgattgacgagattcttcgcacaatcgcaggtctcaagtttcgcaatcacgccaaagagccgacgccattgcagttgaagaaagcagagacggctttgaccaaagaagaggctactaagaaggcactggagatctacaactctgcattacctctgtctgatgcagacttaaagctgtgtatcgatcacttccgtacgctggagaagatgattcgtattgacccaatgttaaagctcgcgcagccgtacgttgtgaacaatctatatcaactcgaaaactatttacacgcacgtaagtgtaagtagccaatcagggagatccttaactggatctccctctgtcatttctggagcatttctcatgcgatttggtttcgcctgcaaactgattgacccacaaggcaaacagccgtacacaaacaaaagtctaagctataaacatttctctgccttatctgcacctgaccaacatgacaagctcttggacgtcgttacgcataacctgacttcactactgtctatgatcaaacacgttggtcagttacgtacggatatgcgcatgttccgaatcacaagtgagctgctgcctctatacacgcaccctaaggtgtttcacatgtacctgcgccaggacgttgtgcgcctgactgaaactatgctggcgctatgcggcaaagcagcaagacgacacggtgtgaggctttcatttcacccaggacaattcacggtgcttgcatctgatcgacctgacgttgttcaaaactcgattgctgaacttgagtaccacgcgtactgcgcctatcacatgggatacggtagacgctttcaagacttcaagatcaacattcacctgagcggtagattaggtgcagtaggattcagagcagcctttagcaaactctctacccactgccgaaagatgctgactgtggagaacgatgaaatcacttctagcattgaggacgtactgacactatccgacctgtgtcctatcgtgctggatatacatcaccactgggtaatgactaacgagtatatacgaccagaagatgatcgtgtgcgacaggtcatagactcttggcgaggtgttcgacctgtagcgcattactctgtgtctaagcctgagtttgttccttctcgcggtctgcctgatcaaaacaagctgtctgctaatcgtatgcagttacgagcacactctgattactatcacaatgaagacgtgaacgagtgggcgctttcattcattgattttgacctaatgtgcgagtcaaaagcgaagaatctagcacgtacaaaattggcatgtttttcaggcaactctgcaaataactggacaaaatgaggcttgtatctgaacatagccctgtgatacactagatatgagcattatcgctcgtcaaaataactagaatcgaggaatcgctatgttcacaactactatgactcaaaagaaacctgcaatgtctctcacgtactcacggtctaatcactatgagacacgtaatagaatctcttgcatctggcctggtgcgctggacgtacctatgccaatcaaacgttggtgccgtgctcacgaaatcctgatcgacctcgacgcttacatgcgtgttcgattcaggggccgtcgccaagatatccttacgttgattgctaatcacattgcagtcaataaccctgaccttgccactcgcatcgccgcgacaattactgaggcttaaaatgaaacttcaacctgtggaagctgtttacggtgcttacaacaccaacactcctctagtggagaaacgcggctttcgttctgtcgaatcgcagtacgtcgatggcacggaggttagattacaacggctcgcacatgatatacatgaacgtgtggttgtgggctacgaccaatttggtcgggcagtgtacggaacacgcgtaccacaatcaacgttcgaagtgcgtgacagcaaggaaagcgaaccgaataagacggcgccctagcaagctcacaaccagaagccatagaataacaataaccaattcatgcgctgacctatcgtggggtgtcttaaaatgatcgttatatgtaatagctcgaaagaattttcagccgaccgtttggctcatggggacgcatttgtttttgggaagacacgcatgttgttacgtgcagacttcatcatcctgacagacagaaacaatgcagtcttcgtagtacgcaaatctgatgttgtttggtctcccgagcttacgggtgcaacgcatgtgattaaaatccgggcgttcgcccagattaagccgtttgaactcaacgcagcatgtcctcaatttaacagtcgtgtgttcggaacaatcgcattccgtaacccacactttgagcaccgtcttggtagcttgaaatatgtagagacaatcttcggaggtttacatggcacggtatcatgtgtttagtgcgacccataaatactacggtgaagcatacgaaggaacttggctcaaagagataactcttaacgggcaccaagttctcaacgcagaattccctaacttcgaggccgcgaaagaatgtgccgacaagttgcatgaggtttgcgatattgggtggatcgtgtataacgctttttctgaacgcgctatgtacgatacccgcacggtacaaggcgagtctgtaaacaactaacaggcccgccagtaatccctaatcgtgatgctcacgggcgtcacacaaattcataatacgaggctataaaatgaaattcaccgcaatcgctatcgcactggttatgtctgcttccgcttctgctgcaaactacgtggcacccgcacctgccgctggcatgaaatcttctggcatgactatcagcgacaagctggacgatagctgcctgaagaaacttaatcaggcgatcgacctgcgtcattcagtgattgactttgctgtatcgaaagatgctatcgacacggtagccgcttggccgcttgtgtgttcaccgactgttgagtccgcgtcggttactattgaacgtatcggcagtgacattacgatcacctacgtcaataacgacaagtcgctggcgaatcttagcctcgtgttgcagcgtgtagaatccactacagaagacgatgcgcctgcgtatcagatcgttcagattggtgacctgaatgctatgggctatcaagaacaaactgacgtgaaagagtggctgcttgattgttatgcggctactgtgcaggacgacatggctgtagtgaggaactgatgaaaggaaagaagctaaacgtattcttgcagcaacgaacggcagtaaacaaagttgcgtccagtccacaagactgggagacgtacaaagaaatgctgctaaacatacggcttgccgtagcggtcgatccacgccccgatgctgctattcgccatttggctcgtacttggtatgctgaatcaaagtacgcgcttcctgtctgtcaggctacgcttctgaaactgatgacgttgaagaaagcaaaccaaacgcttgaagaaatgatcgcgctttatattgaccttgaagaaggaactgagaaatgaccgaagcagaactgaacaacgactacatcgttaacgcagcaaaaactatcttcacctcaggtacgctgcaacaacgtgatgccttgcgtactatcgccaacaccgtactgtctggcaaagctgcatttgcctacgaagaacgtgcgttggatgttgaaacaacgtatcgcctgctggaagaaatgcaattcactggcgacggtaagcagatgctgcctgccgatgaaatcgtagcgctggacaacatcctgcgtaagaactggcgtaaagacttcttctctgctgtgtcgaacatggcgctgactatgtactgtaccgaccctgcgacatacggtaagggcttctggccgaagaatcaaagcgattgtgtgttgttgatcaatcgcgcattcatatgggttgttgctcaacagggcctggtaaatcttctggaaaaagattgtccgagcgtgagtcatactcgtctgccgcagtttatcatcgccttgcagactgttggtaaagatgatggctatgctcgtcacttctcactgtacgagccgcatgaagattccggtaatgtgaattgcaccaacctgttgcctgagtcatacaaagcggcgctggaagaggagcgtatttcaaagcgtcctgctgaatatgaagcagtacgaaatatgaacttcgatgctctggccgatctgtgcgagcgtttgaacgtcattggtccaaattcaactaagcctattgtctgtcgttgtgaccctgacgatgactgtggatgcgaagaagacgaacaccacacgcgggaggacttcgacaaggatgacgacgaactgcgcgatgtgttctatcagaagtttggttatccagatgacgatgacgaacctatggaagacgaaagtatctggttgccagatgtatcgttgatggaagttgatgttgatcttcctacagtaactcttcctctgcccgatcagcctgtacccaaacgtggtatgcctaagtctcgtgttaagaaacccatgtcttcacgtaaagtaaaacacatcttgtctccagcacaacaaatctggcacgatctggacagcaagcacgagtttggtgatcgtcgtttcgctatcacactcgtttctcgccacacatgcggtgttaatcgcgcagtcgctacgacccgtgaagcgcttgcaatagctaccgcactgatggatgtaagcaaatagctggtcagaatagcgcttcttcgtgaggcgcttctatgatataatcatagatagagcaataacgctctcaacgttctatcaaccatacgtttaaacacgggattgtcataaaatgtcacgtactatttcacgcaagaaagctctcgaattaatgtctaaaacttacaacgccaagcatcctgaatatctgccacgcctgatggcggaagatatggattcttccagcttgtttgaattccgtgaagatgttgttgcccagattcgtgaaggcaaagatcccgttgctgttgttgatgctatgatcgacaacgcgattcgtgtgaccttggttcgtcgtcgtaccagtaacgattataatcctaagatcgccgatgtgcttactgatgaaattcgtgacctgcttcgtaacttataaggaataaaatgaaaagctacggttacttctatatgttgaaccatatcgcaatggccgtagacgcacccaacaaggaagttgggtttaaatctatggttgagctggacatgttcaatcgcgcgtctatattaactcgtcctgacgctgagcctcgtgctgctcaactcgtcaaagacctgacctctgcaatctatcctgtcggtgattgtagcccgactattgaacaacgcatgatgcttgttcgcgctctgcacgatcaagagctggaaaagattgtaggctcgattcgtttcttcgtgccgttcgcatacacgaaagaagaactgtgcgacacgttcggcttcttcgacaacggagacacgttgagcattccgtatttcttgcgtcatcatttcatggacgaccaagccgtcttctgtgaaggtaagctaaccagcttcgcctactcatgcactcatggagaagtgtcacagactgctcggcagtacggtctgttccctgcatacgcttacggtaagaacgatatacctgagcaattcaaacatctgcctctgttctaggagcttctcatgggagtagttaaaggcataaccgctaccacgttcccttcaaggggacgtgacgagggccagaagattgctctcaaagctcgctggggaattttccccgcgtctgttgttcgtcaagacaacgatcatccatacaacgagatatggaagattgacgccaagaacttaccgcgtcgctacttctcggaagacgcagacctgttcgtgtcaagacagttcatcgagaacttcccgaagcgctctctagtctgcgctaagggtgaaagtgaaaaccaattcgttgacgttgtgtttgaccacgacacgcagaatacctgcgaaggcgttatcgtgacgcatcgtgatctgttagtcgtcatcttgattacgacgggccctcatgcaggccgatacgttacaggcaaagaatgccagtacgcacctaagccgcgtaagattaaggagctgatcgatgaaagttgataaaggtaatttccttgagcgtttgaagtcaggcaaaaccttttacatgcacgttagcggcaagaagaaaggtcaacctcgtcaaggtgtttcgttggggcatgatgctcgctacaaagatctgatgatggccgtaggtggagttgcattcactcacgggtataagaacgttcaggtatcatttagccgcaacatcatggcagatgctgatggtgttgtggtatttcgtgttaagcaatcaatcaccgttaaagaagaaaggacgtactaatgcaattcttaatcaagcctgaagatcgtttcccgaatttcattccacctaagcgcgccacagctaaagctgctggcttcgacctgtttgcgcaggaagatatgatcatcaccggtgacacagtgttattcgatcttggcttccgcactaaggtgccgaaagaccacgttgctgtcatcttcccacgcagtggtctgggtgctaagtttcaggtgcagttggcaaacacgaacggtgttatcgacgaagactacacgggtatctggatggcagcgttgcatctcggcggtaaaggcactcaggtgcatcaactcgattggttgagcgccgcctacgagcaatcaagccacaaagaaatccctgacattgacgacgacgaagaccagaaagcattgttgatcaaacgcggcgatgcgttcgcgcaagtgctgttcttcccagtgccagaagtcgaagtggttatcacacacgaacctctgcctgaaacagatcgtggtgacggtggattcggctccacgacgaagtgatttacttctggctgatctttgcagcgtactacgttgtcggcattgtcgtattcgttcgagacctgagggactcgacagatgatgtaatgctgatgcgccagttcaatgatgaactgaatcgcatgtccaatctcgaactcgtttgggatgcgacaaaacttttgctgttcgtggtgttcattcacattccgtgctggattctccgcgtatagtgatatcgttcacacaaggagccttacgtgggctccttattatcgtaatataaatgctatgggaaagaaaacttatctgctgccacgcgaacgccctagccctctgccgaacttacgtgcctatctcgcgtatctcgcccggaagcctaacgctaaccgcgaagtattagaaacgtattgtattgcaagcctagctcaaatgcgccgcgaacggtttttcgtcggtaagctctttgcctacaaagtgtatacgaaatcgaacaagctcgcgtacacggttgtgtggattgacccatacaactacgactgccttgttctcaatcaccaaaggagatgtgtagagttcaaaaacttatacggcctgctattatagttgggtcctagcgccttcacactaggggaaatattccgatgataactgtccttaacaatcgtaccgacgaggtaatgaaacgcctgaacgtagcagtatggttatgcgtggtagttgcgttcgctgtcttaatagcgttgcgtatctcacctgcattcgccagtatgtctacaggccctgacaacgccattgatatgtcctccgccgtgtcactcgatccctccaatcgcgtggcgacaaaatacaaggagatagaaaaggcagtagcagtcaaagacgaacgaaggccaaaacgctatgtaacacgcgagcgcctccgacaactttacgcgcacttgccccacccgtctgacttaggcaggcagattgatttggccgcagagaagtatggagtagacgcaaaactcgttctctctatctgtgtctccgagtcgcatcttcgtgcaaaggtcaggaataagtctggtgctactggtatgtgtcaaatcatgcctaacatgcacggacgttctgcacgggaactcatggactaccgagtcaacattgatcaggcagcccagattgttgcgttactaaacaagcagtgtaagggacgacgcgcctgcgttatccaaagttacaacactggttggggagcatacttaaaaggtgtacgttcaccacaatacttagcgaaagttcagaccgagtatcgccgcaagcatactccttcttcctgatagaggatataataatgagcatgaatatcaccgcactgtacaaaatgcaattccagttgttgaagccgctgtctccacgtcaagagtatgcactggtagtgctgctatgtgacaacattgttgatggtgacgttgcagcaatggcagaagtgatcgtccgtgattacccgcacgttgcgcgtctgtatgatgcgtttgctgcggctaaccaatacgagaacgcagtaccgttcatcgtacctgtgttgaactccgaagaagttacagaagaaatcttctgcattcgtgaccatgcactcgtagttgcacctgacctgcgcgaacttctgaatcaggctctcactcgcgttattctgatgcgtgaaacacctgatgaattgctgatacgtgaaggcgccgagttgttgctctgtgaagatgcactgccgtttgttctaggtcagttcatcgacagtatgctcgatgcttacaactgcggtgtgctcccaatgatcgtgcgcccttcgaaagagcaacaggcaatgcgccctgagcgtctgctctctttcgatatgctgcgcgaacataacatgttctctggaagtctggactttactaaagctctacagccgagcgctaaagcaaaggtgattgctgcccagcttatctctcgtctgcatagcgtcaaagccaaacaaggcttcgatgcggtaacacaataaactcaacgggagaccttaactggtttcccgtttttcatttctgcgcaaattttaaggactacacagatgaccaaaatggttgcactgcctttcgcttcttctgaacaacgcaatcgcttcttcgatcaacgcgtgggtgacctaaaacttaacgccgtctggaactacgttgtatcaaacaacaatccgaactggaaaggcgatcctctgctgcaccacatgcactaccattcgaccgagcatatgaagcaggtaactgctctggctctctggcttctggataaagaagcgcaacagccgtggcaatacgatactggagccttgcctcttgctgtggcctgtatgttccacgacatggaccactcacttggtcgcctcaacgatgaaagtaatattcgtctggcgcaagaggctttcaagaagtatctcaccttgtgtgaggatgaacgtattaaagatcacgaagcaatcatcctagacctgattgacattacgcgcttcccgtacatgaagaaccgtcagccgaagaatctgattgagcgttgcattcgtgatgcggacattctctacggcatgcaggatgatgcactggacgtagtgatgtttgctctacgccatgaggtgaatcgtagcgtcaatacgaatacacgctacaaccaagaacagtgggcacaaggccgtgttgacttcattcgcagtgttgaaagttactgcccgactgctgacgcaatgatggactggctactggcggaagacaacgaccacaaccatcaagataagattgacgactggatgcgtcacgaagtcagtttccgagacacgtccgcgcataaactcaaagccaatgacgtgctgttcatcgacacgcaggaagacagcacaccgaagcgccgtctgattgaacgtgtcgaaacagttcacccgtatctcaatatctactttgacggaggcgaagctatctcgctgcgtgatggcgagagttgtgtggttgtcgaacgtcgcaaataataggctgaaataggcatgtactgactaggtgcctatgatataatacgcataggcactcataatagagagaactcgaatgatacacataaagcgtctgcacctgaactccgacaccaacttctttgcgattaacggaatcgtaataccgatggctttctactacatggacgttaccatgcacacagcagatcgcggagacagagaaatgaaaatcggtgtgcgtgtgaatccccatgttgcccgtgagtcttatctgcgtggcgtggactacagaacatttatacctgttctggcctgtcatccttcttcggacgaagaattttatacagagcttggctacattgatgttaacagtcgattcttcgacatgcaccaccagaagcgttcgcacttggcgtatcttggtgtgctgcctgatgttgccgagtcggatgtgcgggactcacgatatgtaacaccgattgatgtgtatcaagtgcaactgcctgaacgcgcccgcgcctttgctaaggtgtacggcgctacgatacgcacggactacctacgcacttccgcaatcaataagattgacgatgatatgtgggaagcgttgcgtaccgtagatcatcctaaaggcgtatcgtggtcccgcttcttagatgaagcaacgtcaggccgcttcacgccgcacgatgacctgtctaactgcttagaggcattcgatcaagagtacatgcctgagcatatctttaaacgcattcgtctggcccagttcgacaaacgaggttaatcatgatgcacgatttgtataaggtgagtgctatcctgttctacacgctcggcgctatggctttccttgcacatatcgtaggcttcatgaagaactggatgaagattcaggagatgcgccaaaaagcaaaagcgaaagctgctaaggtgcgctctcctgttgaagacattaaacgccgtctgcgtaaagcagaagaacgcgcacggcatcgcccacgtaaattgagagaataatcatggctgaatcaacgcacgacaacaatctggcagacaaagtacaacgtgctttggagatctgctgggaagaaacaacgaagcgcaacgaaggcgaacacacctatgcgtttctcgcctcagagtttgctcttaacggtaagaacttgtttgatggcgaattgcggatgctgaacgttatgctacgtgacgccgttaacatcaacatgtacggacgttatgttgcgactgtctatactggcaacaagggcatcatggtcgcgttccagcctgttgctgatttggaagatatcatcgagatgaggttctagcatgaaccagattgatatgtttgaaacgtacggcgctcatgagatctctgactacactcaacttgagtatgagcgtctggctggtgagtacatagcgaaatgtgatcgtagagtgcaggctgccttcggcgacccaattcttacggcagagtctctggagaaatacccgcacttatctcccggtaagttgaagtttcgtaagaagctggttatgatccaggagttcgtgctcgttacacatgacaagctcaaggcgagcctgctcaagaaacagggcaacgttcgacagacaggtaatatcgacccgcagtatctgatcaacgtgtacaaccacaatgagaagctcgcgctgttcatgagtgacttccaggacttcatgagcgacttcatgaatgccgttcacctgttcaccgttgctactgtgtatgatggtcgcttgcttgtctacgcagagaacggagagcctctggttactaccaaagaaacgctggcgatgctcaccgagatagagcacttcatcaaccgtagcaaagtgtatcgcgtacactcacaaaacgccatctaccgtacaatttaacctgagcgcttacgggcgctctactggagagacattatgtcattcgatcttcgtcaaaacttactgcttgttcgtgacgctgccttgacaggcaaaccgctgttctatttctacaacgctatgggtagagagatggtactcactggtgacgtgctgcgtgagattcttgagcgtcagaaagaaggtacgctctgcaccaacacttactggggttttgctactgacccaacactggaagtttggtcgttcgatgataacaatgacctaatgcttcaccatcgcgtaggcaagtcctgcaccacattcctgccttacgaaatgattgcaaatgcccatgacggattcaagccaatcaatggtctgttcattgaagacagtctgcgcactatcattcgtattcatctcaaggcgacttgccgagaagaacaaaagattacgtggttcgctgacctacctgagcctgagatgcgtagcatgttgctctcgtttggtctgggccctctgcgcgtatcgcgtgaagataaagaaggtctgatcaaactgcatgaccggtggctggaagacttcgacgacaaatacaaatatacgcacaacgcaatcggcgtcgaggccgacgagaagattcctgctgactatcgccctgaacgcattcgtgacattacgaagcgtatgatgcacaacaccaagactcagaatatgatggttcagactctgaatgacctgttacgtcagtgtcgtatcagaggcgatatcccaatgcccggcgccaactttaaccttcaacagttgatctgctactacgcaacacacttaatctttgcgcatgacgcagacgaaaagctgcgtagcctaattgatagcccgcagttcgtcgtcaacttcatctacggctggtacccagactattcgtggattgcggtcaatgaagaagcgttcgactaccagcaatcactggtacgcgccgcgctgatctcgttaaagcgtcatgtagagaatgaaatcggtacgtacaaaatcgttcacggcatggttaagttcgcagacggttttgaccctcacgctcctgagaaggtagaagtcgaagaagaggagttcgacgaagaggaagaggaagaggccgaaacggacgatcaagagaaagaagtcatcgactacctgcgtaccaaaagcgaagatgaattacgcaaagttgcgacaagaaagaaaatggcgcgtcctaataagttgaagtctatggacaaagaagaattgattgagctgtgtgctgactactacggcactgagatgcctgaagacttcgacgaagaggaggaggaagaagaaaaagaacaggagcgtgtgcgcattgcccgcaagttcccagtagtgttgcgttatgatcgcatagactatgattatgttcatcgtgcattagttaaaatgggcatagttaaaaagaacaagactcgcaagcagatggacaaatcgcagaagcagaccgttgctcaacaacacgctgcactgcttgtcacactcaaagaagctgtcttggactcaggtcaggacgttttgtctaagctggacgaaataacgctgtaccagctggccgcctgcctgacgaaattgaaagaaggtgatagctatcctcgtgacgctgcgtacctgaaagaactaattaaacacgcagtcaagtaagacctgcgtaaacaatacctaacattgacgggaaataaaatgaaatttgaacaaaacattctggtagtaaatcgcattgctcttatcatggacgacgaattagttcagaagtggggcgaagctgcaaatgcaaatcgtgacgctactgcgtatgcgacggccattattcttggcaaactccagcagaagattatagccgcagttgctgaggagaatccagaagcctgtgttcgtcctgagatattgtggacagactacggctctatctccatcaacggcctgtttatcattgcgtcatccgctgatcgtgaggtgttgaaccactttgaagaccacgactaccttaaccacctgcacacaatcaaacgtgtcgccgaggagaatgggttcacgctcactgtcgttcctgtgaaagcgaacttcccgttcactaacactgaaatccttgagtccatgaagtgaggtgatctatgtccagacaacaaatcttgatgaatgatgttgctatcgtcctgactatgactgaacgccgtgctttcttaggtcccaaagcagacggctttgtgtatctgccatctaaggatgctctcacgaaatttgaggcgcatatcaagaagtatggcaatcgtgatgactatgcgtttattgaccatcgtgagctacattctattagctctgctggcattgtcgctattgctcatgctgtcgagtctgattctgagcagccgtggctgtggacgaaagaagacttccgcgtcaagctgtggtaagcataaaactggctaaaatcgtggtatcagtctgaaccgtcctatgatataatagaagcgtagcttgtgctgcgcttttttaacatatgtctaaggagacaacaaaatgctcgaagaaatcaaaccaaccccaaccgacttagaactgcaagaccagatggtcgatgcggccgcccagaagattatcgaattgaaacctgaatgggttgacgtttctgccgcaggtctgcgcctgtatctgtctgtgtgtgaacaacttggtggtcctattcctgaattgcgtttcgtccacaacgccaagccgtgccgcattcggttcaacttgaatgaagtacctgaaggtacagagttcgtagcaaatgaaatcgacaaagaaaagcaaatggcgattgccgacgaaatgctgaaaactgccgaagcatgtccgaacggtcactcgctgctggatatagctatttgctctggtcgcctgttcatgattggttatgacggacttgcaggtactctcgataagatctgcattcgttgtaatcagaagaactacaccatgaatctggttaaaggtgaataacatgaaacctgaatacactttacttaaacgtagcaaggtcgatgttaaccgttttgctttcgtacatgacggcgagatactagctaacttcaccgccggccagttgtacagaacattggagaagctcggtcgaccgacatcctttaaggacgttgatgtgatttggagagacggcactcgcaccgtcgaagagctgcgagtgactgagcaccgccactttgttcgctttgatacttgcgagtacgatcatgcaatctgtctgatgctgcgggcgcaaggtctgcctgtcgaactctctgctcctgtagacgtgcgtaagctgtttgacgagcacggcccgcttattacttcaatctgtgtaccctgtgaactcgcagatgacctaaagcccgcacttgcgcgtttcatcccagacgaagatgacgacgaagatgaagatgaagacgagtgggatgacttagaggatgatgtagacgaagatgacttcggattccgcccagaagatttacgtccccaactgagtgacttcggataccgtgccgcggactgggttgtcactttgactgatgatcaaatcagcgatgtgcatagtcttgaagtcggtatggacccagatattgaactgccgcgtgccgatgacgcgaaggaagaatttttctaatgaaaacgattaacgaacaggtcaacgaattgaaacagcgcggcgtgcttatcatcgaagaacaccagaagcatacgctgcctgatttaaccttcacgcttgattgtctgtgtatcaatcacactaagcgggaagtagagacaaccacgcgcggccgcgttgttaagattcgcctgacaaacattcattaactttgtggtcttggcccgcccgtccagagatgctcacccccaatgaggtgcctcgcgcagaggtatgacggtcaccgggtccctttttagagcgcactaccccctagtacgctgtacaaagtaaaacactcaacaggaggctgttatgaacttcaacgaagtatccaaagaggcgcaagtcgccctaatgtcaagtgccttggctggcgtaatcgaagcgttcacgcgtgaagatggagacgaaggtcgcaagattttagtcttagcactcaagcaagtcggtctgactgtagacgagttcggcgctcttatctctgacttgtcgccagaagttgagcttgaaattgtcagtgttatggaagctgccgatgcagagccggacgaagatgaagacgacgaagaacctgctgacgacgattctgatacagacgcagacggctggcagaacctgcatgaagatcgcgtgtgtcttgtatgcaaccatgaaagctgcatctgtcactaatctgcataaatctggacaaaacgatggttgtgtcaaaacagcgtccgtgatagaatatagatgtagggcgcatatcgtgaggagtgcgctctatatgcgaatgacgcgattcgcagtacgagagaagttcttgaccgtgtgttttcgttttccccggacacacggtcctttttcaagtgccttcgaagtttgagggtgcttgcgaaagggttcgataccttttgagcgcgtcgggctttacgcggtttccgccttacgtgctctcatgctaaaccgcaaaggaaatagatatgtcaaactcaaaagctgctgctaaacgttcaacgccgcgtggtccttcatctgttaagcctcgtcagttgcctcccggctacggctacaagtctaaggctacaggtgaacgttctggtggcttcacgcgtgatgaagttattatgcacacaagcgcgcctaagattcgtgacgaggagcgtgtgtacaatctcgtacatgcaattctgagcgcgtggaaagctgatgttggtcatgccgaacacacggccgcttctgctggcatcatcaaagtatcgcgtcgtaagattgaaggtgccttgcgtgacctcaagaatacgcgattcactaaaatcccgacacttattaacgacgtcctcgtttataacgaagtctgcactgagttcgggcagtgggtatatgtcgagcatgacagtcctgattggattttcgtgcgtctgcctgaaaacagcacacccgtgattcgtgctgatgtcagctacgacaagacaggcgaaacgtctgcgtctatttcgacctcaagcgaagcgctgctggaatcgttcgattcccgtgacgacgaaatcgagatactcgaatgtaacgatcaggatattgaagacctcgaatctgctgagatgcgcaagcgtctgatcgatgcgaaaatcatcaaacctgaagctgcctcgaagctgtcacacaatgacttaatgaagctctgcgcgtactacggcaagtaagcaataacgagcaggcagtctacatgctgcctgctatctgtgaagtatgcagaaaactggacaaaatcgtggttgttatctgacggccacctatgctataatagattcagacgcaatagtgcgtcgcaaacaaaacacttatactgaggagtattaaacatggcacgtatcgaaactaacactaatctggttggcaaaactatcgttctgctggacggcaccaaaactaaaatcgaagatgcaatcgcgtctggctataaagtgaagggccgttcaacgaaagttgcaacccgctgtgttatcaaagaaggcgctcactttaaagaaatcgagcgcatgaacatgagcctgctggaagataccggcgaaggttacgtgaagctgaaagacgcgaaagctgcgaaagcatcaaccaagaaacctgatgcgaaagagaagacgccaaaagcaagcaagaaagctgccaagccagcgaaagaaaaagaacctaaggttcgtcgcaaatcttctaaagagaaagaagacgaatatcaggacttggctcacgctatcatcaaaggtggtaaacgtgcggcgcctgttgaaatcgctgagattgacggcgacctgacagactgcgttgctcaacgtctggtagacgtgctgaataatagcgaagttgcgaagctgtgcgctgataacaaaacgccgatcgcaaacgcagttgaagttacgtacggcgctgagttcgcccctgagaccaacgtcatgcagatcacgctgagcctgcaatacgctaagcctgttcaaacgctgtcacgtccgacgctggaaaacgcagaagctatcgcgttacgtgctaagaaaatggcggcgcctaagctgtcgatgaaactcaagaaagcgattcgtgaagcattcagcctcgaagacgcgaatgaccttgagctgggaactgtgctgctgtctgacggcgctgaatttgtttacttcggcgaatctgcgaagcatgtcggcaaagcgctgctgtatgttgtggagaccgacaagttcaaatctgtgctgggctctacgctgggtgagtacgaaatcccagacgcagaggaagaagaggatgaagttgaagaggaggaagacggcgaagaagaagaagaagacggcgaagaagaagacggcgaagaagaagaagacggcgaagaagattctgccgaatacgaatacgttgccgtgaacaaagatcagctcgatatggtcaacaagaaagtgaccgctaagtatcacgctgcgctggccgaacgtttcaacacgaccgaagaagttctgattccgggtctggtactgacagacggcgaaacaaccttcgcgtacctgggttgcgatagcaaaggcggtctgctggtaatcgactgtggtgatgacggcgaaggcgaagacgtgctgatgtacagcaagtctgatatcaagtctctggatgacttcaatcctgtgatgggcgaagctgacgaagacggcgaagaatctgataacgaagatttagacgacggcgaagaatcagacgatggagatctggacgaagaagacggtgaagaagaagacggtgaagatgacgacttcgactttgacgatgtgccagaagctgatatcgaagatctgaccgaagacgaactgcgtgaccgcgtagtcgaagccggcctgaccactccgcgcaaagctgagaacatgaatgaagctaaactgcgcaagctgctgaaaagcgcataacgaactaccgtaacatcgaaatagtgtgcggctcttactgggccgcatatttgacaaataaagctgattgaggaatcacactatgtcaaacgcaaacaaaattctgcttaacgctcgtgtacgccgtttagacggaaccattactcacatcaacaaagtgaacgctaacggttatagcaccgacgcgaaaggcccgcaaatccctgtgaagcgcattgtgttcgcaggcaaaactctcaaagagattgaagcgccgttcgagaaaggcgagtatgtcattttacagggcgttgcagtgaagctgaacaagcgccagcaacgtgaactcgcagacaagacgctggatgagaaagcgctgcgtcctgactttgggcgtctggcgttcattgaccgcgacgacgacaaagcaactgacggtaagaaagtgaagccgaaagctgcgaagaaagaaagcgggttgaaagcgactcgtaagcagaacggcgatacacgcacaaagaaagagcgtaaggccgaagctgctgccgctgctgaatcgctcgacacaatcagatcaacgccagttgatcgcaagggcgagctgatagctaccatcgacgcgaccatcgaagacgcgacaagcaaagagcgccgtaagttgttgtctgaatcattcgacatggactggaaagacattaagaagcacggcggtaagggtgtcgttaaacatctgggccgtaaagctgcgcaatctgccgtaagcaaaatgcgcgcgactgttacgcaggacgcattcattaagcagatgcctgctgagttgaagcgcttgattcaagatcgtcggctcgtactgaacaagcgccagattgaagctgtgctctctgcgcttgggcttgatgtgaagttctataacattgccatgcagacattgcttggcaatctgtccctggctgtagacgacacgctggatgacgataaagcagataagaaagtgaagaagctgaaaaagcataaagcctctaagccgcagtatctgtcagagaaagaccagcaacgtcgtatgaagaaaatgaaagtgaagctgctggctcctactgagaaaggcatgaagaaagccaaagcgaaattgaagcaggcgaaagttacgcttgctgacaagctgggcatctcgccgaaagaaatcaaacgcggtctgattgcatatcgtccgaacggcgttgattacatgtttgttgccagtgatgctcgcggcccaatcttcatcgacaaagacggcgacccgtgcgtgtatacttacgagaatctcgaatcgacattcgacttccgtctgactcaaccttctgaactggacgctactgtatgaccaacaatgagatcatcctgactggtgttttcgcccaactgtattcgcggctagtaatggccgctatacagcgcgtccatgtatactactctgatctcgctcctgtggtgtttggtgtgcagttcactcgcgtagggaaagcgcagtacaaagcactggaggcgctcattgccgagacgatgcgcctcgatattcaaaacggcaggccaccacttgcggccttatacgtgtcacgcgcaaacgacaccaagaaacctacccagtcattcttcaatgagtatctcaaattgactggtaaatatctttctgatgatgaatggttgatgctcgttgaacatgtgtggaaacaatatacaccagaccttcgggagccatcatgaaaaagtcaaaagttgaaatcagtcgcggtgggtatcgacccgtctcgccggaagaggcaaagaagttggttgttgaaatgctgcttgcttcaatcggcgttaacccaacgattatgagccagcagatgttgctgaacattgcgaactacaattacctcacgtctatcgcagacacaggtaagacaaatacagcgaaccagatagttctacataaaactgtaaaagaacttaatgcgttctgtagattgcacaagattcctctgggcttactaattatgccccatacatcggcgagcgattactccggtgacgaggttgtagcgattccctgggagtctgtgcgcaagaatgcaccgagccagtccgctgtcaactccctgttccaaacagtcgaagctgatggctatccgcagtttgtgactgatgcgaaaacagtagaggactacaatgttttatgatcacgtattcagccctgacgagaagcaacttctcttgtctgtagctgagtctaaatatctggtgcggcttgattgccctgagtatttgaagaaatcaaaacactcgattgaaattcgtcatacagtgaccaaccgtggcgaacaacgtcgaagcggtgttatcaatacaacgtttgtgccgcgtattcatgcctcaactgtgcagcgcctgttacgtgagattcgtgacaacgcaactatcagttcggctaacagcctcgccgcgttatttgaacttgggcttggcgtgccgaagcaacgtgatattgcaacgtacttgcacgactactctcgggagaatgacaagaagggtgtgggtatcaagtacatccgcaaactgattaacgagtatcaccgcaagcaccgtcatagttttgctggcagtcgctggatgatgcctgctgcgtatacggcgaacatgttgaacatgcagtctttcattcatctgaaagaaaacggttacagcaagaaagtgaaagtgcctgacggtctgcctgttgttctaatctatcagaacacgagtcacgcagaagctgagttctctatgtgtgacgccttcgctattagccctctgggttatccgatgccgttcgcccagattgcgatgcgtcctgagttcaaagctgcgccgaagacgtttcaatctaaagcgctgcgtgggcaaggcatgtatagcatggtcatgggtatcgttcactgggacaaaggtgacgcactgacgaacatacgcgaactgaacgccattgacgacgagccgtatctgacgttgttgtgtgacgaacaatacgcagatcgtcgttcgccggagtatcagaagctgctggacaaacgtgctgagtttgctgaacagcggcatgagtggtcagaagtgattgcgaagtatggtaacacaactcgcacactcaagcctaagcagttggagcgactggagcaggcagagaacttcttcaaagaacgcaaaacgtttatggacgagtttgataagttcgagaagaaagagaaccaccaggctgctaagaagtttgcagtagccagtgcgaagttcgctgccgttgattgtggaactattgctgaccgttcgacgtatatgtccgtagcgtcgggcctcgacaaagtgaataagattctcactaagtggggattcacaacggttgatactgttaatagtagtttgaagaagtctatccttacattcgacccaacaaccgctactcgcgtgtggtcactgtaaaccttttatctgaggagataacgtatgtcggaaaataacctgggcgctgctgcaaccttcggctctgagactcaaaagcaattaaacgaccaacagcgtcgtgcgcattcttctgagtccggccacgtaaacaaatgtaccatcgtcgttcttactgcgcttaacgcgcatggtcgattctcttacctgactgctgacgagcaactgcgtgagcgttcaatcgagggtaaggtgatggatcgcctgccggatctgattggccgggcatcgggtccttctactgatccgaacagcgcgtaccacatcctgcatccaaacaatggtgtgcctactcgtatcgacgagcgtatcaaagttggcgaagcggattcggtcatcatttcatatactgtaaataaagcagtgtcagagatgtatggcagtttatcgctggcgctgtttagtgctggtgaaagtgatatcgctgatttggcggctgagtatggtattcactccatctcaatcgttgaagaggcgaaagcgcctgactatatcaaagctcttgctgaacaggtagaagctctgaatattgtaaatctcactagcattgatgaagctgacggtgcttttgagaaaccagtaatcaactacagcgccctgccgggtaatccaatcaacgtactgtccggcgctgtgcgtactttcattatgcaaactctaaacggcgaagtattcgctgcgattccaaataacggagaactgaacgtgaaacaacctactaacgcaacgccggtcaatctggacgaagacttcgattcagaagacgaagtggttgatcagcagggcggcgaaagcgacgacgaagaagtaacaggcactgacctgttcggctataaagctgaaacactgaccgtcgcgcaaatgacagaagctcttgaagctctgtcctacgatgttagcgcgatggacgaagcgggcatccgtgagtcgttcgaaactgaacagcaaatctggatggaaggtaacgacgccgccgaagaagacggcgaagaagaagatgccgaagacggcgaagaatctgatgatgaagattccgaattcgatccttctctgtatctgggccacctgctgtctgctgaccggctggaccgttccgcactgaaagttctggtgcgtactcaagacctcaaagtcatgaagtccgacaccgaagaaacgctgactgcgaaactgcttgaactggtcgaaggtgcaaccgagcaggaaatggttgaactgatcgacaccttcgtaggcgcgctgcaggagcgtgagatcgattgttctaacctgctggccgcgcttgcgtctgacgaagacgaagaagaagacgcggaagagtcagaagaagatgaagaagaatctgaggatgaagaatccgaagatgaagatgattctgattctgtgcaagaccagatcgatgccgttatcgacccgctcgactacttccagttcgctggtggttcgctgactgctgaacagcgtgttgctgctgtcgaagcgatgggcgaagacgttactggcctgaacatcgtgcaggtaatgaaagcgttctctcgcattcagggccagactaacgaaatcgacgttgacgcagaagaaagcgaaagcaacgttgccgaactcgaagcgctgctgggccagtacgacgatgctactgtgcaacacgtcgcagaaagcctgggcgttaacgttgacgaatgcgaaaccgcagaagacatgatcgaagccattgccaatggcggtaccgaagaccagttcgctgcggttgtagaaatcgcaactagctacggtgttgacctgtcagaagttgctgacggcgaagacctggactttgttgacgcggttctgtctgtgctgccgtccttcctgtctgacgacgagcaggaagaagatgaagaatctgaggaagaagaatccgaggacggcgaagaagaagatgaagacgagcaggactctgagatcgattcttctgaaaacgaaagcctgaaattcatcaagtctgttaactctgacaacgccgttggtactctgctggcagtcgatatggatcagactgtagttatcaactttactctgactgacggcgatacttacagcgctgttgaatctgagctggtcgatatcaatggtttcaactaccgcttcccattcaacctgggcaaagcgtctaaaggtactgcgccgggttcaatgctgctgccagctcaatctctgctggacattgttgagcgcgtgaacactactcgcttcctcgccgatccgaaaacgttcgacattggcgcatgggctgaaagtctggaagcaacgctggcggaagaaattcctgtcgcgctgtacgcagaccgtattgaagacggcgttgacccaagcgaagctggtctggttgtgggtgacttcctcgacgaagaagaactggaagccgcaactgagctgggtcacatcgacgctgacgatgcctctgaactgaacggtgatcatctgccgctggcaagcctgtataacgctcgctctcgcgttcgcccggttcgtgtagacagcgcttacgttgcactacacaccacagtgatgaacgttgcactgcctggcttctggagcgaagcacctgtacagcgcatgattcaggcggcagttaaccgtgtcatcaatctggctgaatctgttgagaacgttaaagtgtatgctgcgttcaccatggagtctgctgcactgctgaacaacggccgtctgtttgaagcgctggcaactctgcgtgagtttgagcacgtccagtcttactctgctgctgacgctgctaacttcgacgatgccgaagacgtgatcgaagtagccggttcactcgacacccgtgacctgcctctgtctgtactggccggaggtctggctggcgcatcgttcgacaacggcggtgacctgacaattctggttccgtgcttcacgcaagaagaagacgcggacgaagaagaaggcgacgacggcgacgacgaataatatcgtctaaacgagtggctcgaaagggccactccctttcttggggatctgtaaacatgacacaagaagtagaccacggcgcaaacatcatcaagatggtaagtgaccgtgacgataaaatccgcgaactgaccgcagaacttgcagaagctattggtgataagaaagatgtggaaaacgtcttagaggatgaagtacgcggcaacactgtgttgcgtgtcgcactcagacgtaaagtacgcgaacacgccgcggagattgcactgcgtgatgaacgcattaaggaagttgttggcttctgcaacgaacaaacggtagaagtgaagaacatccgtgctgaactcgaatctgtaaaacaaaagagtgaaccggctgctgcattgccattcgttctgcaattgataatgtctgctggtgtcgcgcactaccatacgataatcgcacaatgcgctattgctactgtcaacaaagcaacaaataaagttgcccgcgaactgcgcgaaatttatgatattgataatgtagtgaagcatccttcactttatcgtgtcgctgttcgactgtgtactcagctcggtgtttcgccaccatctcgcgccgaactatcagccgagattaaagagtatgtggaccagaacatcgacctgtacatcaaagacccgcagtacgctacatctgaatccgccttacgtcagattatcactgcgttgaaaagtcctgcacacttaggctcttacggccgtgacgtgtgccaaatgttcgactggcttccagcactgactgctggcctggacgacattgaagatgactacaacgatttggtggaacaatctgtctatcaagtctgtcgtaatctgattaatgatagcttttcataatctgtaaaagttacctgtaatcgaatctgtaaacactaattgaagttcgaaccgagcgacaagctcacacttataaaatcccggagcattacaatggctaaagcaattaagtcctctaacctgtcacctaccctgatctctcgtattcagaaaaagtctggctccatcggtacttctaaagctaagccttctgaactgccgcacgacattctgatcgaaacggtgcaggctgttgagctgattggcttcattactgaccgcaccgaaaacagcgtcaccattcgtcacaaacgtggtcatggttcttctgcgcaagttgtttctaccttcggcccgaatcaaactctgtccgtgctgggcgaagctggcggtcacggtagcgtaatcgctctgatcaacgcgccggttcgtgagtacaagggcttcaccatcaaatacaaaggcgcgaccatcgttgctacctctgttgagactggcgaagtgattgaagtgaacaccgcactgcctggcttcaccgttcgcgcaaccgtgaacgaaactgctgctgctaaaaagtacggcacgcctgctcctaccaaagctaagaagctggacaaaggcgacaaagctggtaagactgcgaaagtggcaaagaaagtaaaaaagtaagtaagtctgacgaagacttctaactttcgaaatctgtaaacattaagtatgcagcgagataaaaatgtttcgctgcctgtctctcgaaatctgtaaatcttaattgaagcaacgtcgcttctaatcaaacaggaaataaatatcatggctaaagctaaagcaaccgcaaacaccgcagcaaccgttctggctaaaatgctgggcgtcgtagtcgaaaacgccagcgctgctgatattgcagcaattctgaaagaagccggcctgactgttgttggcggtaaagttgttaaagctgaaaaaggcggtaaagctgctaaaggcaaaaaggccaaagcacctaccgttgctgaaatcgtcgctgctgctaaggacgaagaagaactggacatctccggcgtaagcgaagatgacctgcgcgccgcagttgttaaggccaagctgtctaccgctaagaaagcgaaagcgctggacgaagatgatctgcgcgaactgctgaacgaagcaatgggcgtcgagtcagaggatgacgaagacgaagacgaagacgacgattcggacgaagacgaagacgactctgatgaagacgactctgatgaagacgaagacgacgactctgatgaagacgaagacgaagacgacgattcggacgaagacgaagacgacgattcggacgacgattcggacgaggacgaggacgaggacgaggacgatgaagacgaactcgacctcgactcactcgacaagaaagagctgttagctctcgtcctggaacacaagctggccccggccaagaaagctaagaaaatggacgaagatgaactgcgcgaactctgcgaagaacacttcggtggtgaagacgacgaagacgaagaagacgaagacgacgaagacttcgacgactctgatgaagacgaagacgacgaataagtcctgatctgaaccggcagcccctctagttctaacgaaggagcgaggggcaaataatcgaaaaaatatctcgattattttcgtaaaaagttttaaaattcctgttgttgtatgttgaacataataatgtatgactacaggaacacaaacctgaacaaatttatcttttcatccagcggtgaaaacgccgcatcaaatataaagtaaggaatatcgtatgtctaagaaagcaatcagcggcctgaacaaagaaatcaaagccctggaaaaatctgaaaaagctctgaccaaaacttctgctgaaatcaccaagcaggctgaatccatcgctgaacgtcgtgccggtctggctgcccaggttgaagcgttgcagaacgacggtgctgctccggctaaagcagaaaagtctggcaaaaaagccaaagctgaaaaagctgctaagcctgccaaagctgaaaaagctggcaagaaagcgaaagctgaaaaggctgagaagcctgctaaagctaagaaagccaaagcagagaaagctgagaagcctgccaaagctgacaaaaaagcgaaagccgccaaagctgaaaagccagctaaagctgaaaagtctggcaaaaaagccaaagctgaaaaagctgctaagcctgccaaagctgaaaaagctggcaagaaagtgaaagcggacaaagctgctaaggccggtaagaaaagcaaaaaagatgccgaagacttcgacttcgatatggaataagcaagcgccgcgcaatagcggtacttgatctaaaagggcagcgctgacgagcgtttgcccttttgtcatatctgtctcaaattttgaggtaaaccgaatgtctgctgaacatttgcttaacgatgacctaccggacgatactctctccacgaaagcaccctcccctcctgaaaagcccaactactacgcgttaatgactctgcgacttgaagctggcgctcgtcttgctcgtgctctgaaaaccctgaaagatgccaacgtgttcggtgatgataataccgtgaatggcagtctcatgttgactgatgctctgagggttgcagaagctaactgggcacacatctgcatgggatacacgcctgtaaaagattctaatggccgagagtctctgcgcgataaccttcctgcctgcatcgaagcattccgtgttgtcgtaatggaacatgctcaacgcgaagcattggagcgtgagtgcaaactcatgatcagccacgcagaaggtttcaaaattctgacacaacctcaaacactacagattgagccactacacttctgcgatggaacctgcgatcatgacacaaaaactgtctgagcaaatcaaccgctattttaatctcatggagaaaatccgtgagcaactgttccgtgtgttgaacgtgtccgatcgctacctgtgtatcgtgagctttaacacccagcatcaggcaatgcaatgcgacctagttagtcgtgaaagcctactccccgccaagctactcgaaggtcttagtggtcaggagcttgtagtgtatggtaccattactgcccagattgagaaatgggtagcagacggtatgagcgacgacttcccgattgcgcaagacgccgatacctacgcgcagtatcgcaagctggtggaccctgagcaagagcctgctatctctgacgctaacttggtcgagcatgttgcctctctacctaagtcagatgccctgaaatacgttgaccctctgagcaagtacgagcttgcgattatctgcaaagcgtggggtcttgagcaagatgccagcgagactgttatgctgtctctcgtcaagggctatattctgcgccgtgactcgtagcttgaactctgcaaatagttggacagaacgtgggtagcgtctaatactttagtatgatataataggcgtaggacaagtagtgtctgcatatgctaatatcgagtagtaatgctactcataggagatcacgaaaatggccaaagcgccgaaagctgccaaagtaaaaaagaaaacgggtgatggttcccaagaaggtttcgtaattcacgaaggcttatcgggtatcagagaaaaccccggcatgtacatgggtcaacgtggcgaagacatggcgtatcgcgcggtaaaagaacctgtggacaatgactacgatgaatacatcgctggacgtaacaagttgatcgaagtggtcattgattacgacaacgacctgaacatcgtagctgaccaagctggcggcatccctaccgacttcaagaagttgaaagacggtacgaaagaaacgatcatgaccgcagcatttagccgcgtccatgcgggtggtaaatttaacgatcaggcgtataagacttctgctggtacgcacggcgtaggcgttgcggcactgaacgccatctccagtcagttgcgcgtgtggtcaatgtacaaaggcggctgcgtctatcagatgtggcagtgcggtgaagtcaagtcaggcaaagaccctaagaaagtcaagaccatcgacaaagacgttatgagcctgctgcgtgataagaaacacagcaagtacggtacagtggttgcgtggacgctcgaccagacagttgtgtctgctgacgttatgcgcggtaagaagctgccgaagaactatcgacacgcagcgccgaaccctgctcaactgggtgagtggttgcgtaacatgtcgatgctcaacccaggccttgagattcgtttgacgttgatcaagaagggcaagcgcaaagagttcactttccacaacaagaaagacctgaacttcgttgtgaagacgatgtgcgaagaacgtgagctgggcactgtcggcaagccgttcatcttcaagtcagataacatcactgctgcacttgtctggactgatcacgcagacactgataacttcctgacgttcgttaacaccagcccgacagttgacggcgggtggcacgttgttggtttccgtgacgcgctgtttgatgctatcaagccgttcatgaaagaatcgaagggcaaaggcaagaagaagcagaacttcaaacaggaagatttgcttatcggtctgactggtatgttcgattggcgtatgcacggtgcgcagtatacgtcacaggtaaaagacaagctggctagccgtgtagagaaagacgtatacgcagagctgaacaaggcgtttgtcgattacttcaagacgaacaagaaagttgcaacgacgatcattaagcgcgccgaagcaatgaacaagggacgtgaagaactcagcgccgtcgtgaagtctatggctgacacgaagaagaagctgaaaggtaacgcacttcctgctgacctgatcactgcaaacaagtgcaagcctcatgagcgtgaactgattgttgtggaaggggactctgctggtggtactgcacaggatgcgcgtaaccctgactatcaggaagttatgcttgctggtggtaagccgctgaatggtctgaaagcaagtctggctgatgtgctcaagcacaaagaagttcagggcctgttagtgagtatgggtgctgacttgaaatcgctcgacccgaaagcagacgcaccgattctcagtacgaagaatctgcgtataggtaacttgctgctgctgatggatgctgatgctgatggcttccacatcgcaacgctgttcctcggagttatctatcgcttgctgcctgacatgttccgcgaaggccgtgtgtggatcgtcgatgcacctctgtataacgtcgtacacaaaggcaagcattacggtggcatgacgttcgaagaatgccgagcactcgcaccgtcgtctgtaaaagataaagacattgtacgcgccaaaggttggggtgaagtcgaacctgacgtgctggaagctatcgcattcgatccgaagacgcgccgtgtcattcgcgtgaatccattcgaaagcgtagagcaggaacgtttcttccgcggtgttctcgcagaagatgcagtacaccgtcgtcgcttactgggtctggagagctaacatgttcaacattgcaaagttgcctgacggaacgcaggttcgttttctcgatatgcctgacgtgcaatacccaccaatgactgacgagcaacgtagccagtgtgaggcgctgtatggtaaagcgcgtgagctaacaaagaacgttaccgtgtctgggttcactgtagttgacggactaccgaacgaacgtgtgcagattcaaatgcgccgcacaactctcgataagatcaatgcgattgccaaaggagaacagtaatggcaattacgccgaagaaagtgaaagtcaaaaaggttaagccgactgctgtagcgaaagccgctaagcctgcaaaactcaaagcgaaggccgtatcagtcgatgatatcaaaaagaagaaaaagaaaagcaccgacgttgcagcatcgaacgctgttggtacttcgctttatcctctgcttgggcaggacccaaagctgattcacgatgaaggcctgtctgactatactcgacgtgcgctgtcccactatggcgcatacgttgttgaagaccgtgctatcgctgactatcgtgacggcctcaagcctgtgcaccgcgcgctgctgtggtcgctgtctgacttgggcttacgtccaagcgctgcgttcaagaagtcggctcgtactgtaggcgacacaatcggtaagtatcacccacacggtgacgctgcctgctacggtgcgatggttacgattgcgaatacagtacctcctgctgtagcgggtcaaggtaactggggcaaccctgtgtctgctgctgctgcgcaacgttataccgaagcgcgtatgtcaaagttcacaggctcgttcctgcttgaccctgactatctcgaagttgtgccgcgtgtgccgaacttctcgaatgaccttgagattcctctgtacttgcccgcgttgcttccgtacatgctattcaatagctcggtaccagcgccagcgtatggtgtgaagtgcggtaacccaccgttcagctttagctccgtcagcaaagttgtgtgtgacatgctcaacggcgttcaatacgatgcgaagaagctcgctaagacgctcaagatcgtccacacgtatggctgtgaagacgtgacgactgacgaggagatgctgcaactgatctctacaggcaagggcaaagtcacgtatcagccattgatgcacgtcgatgaaaagaacaagctggtcatcatccagacctacgtacctgcgggtatgtcgaagctcgacgccatcacgaagaagctggagaagattggcgagtggaacggcgttgtgtctgcgcgtaacgcaagcggtaagaagaacaagcactctggtccgtatggcgctgcattcgaaatcaaatgccgaggcagcgaagacctgttgtatgagactgcgaagaaggtcatgcgggaagtgacttcgagcgtcaactatacgcttggtgtaaccgttcgtcgtgctgatgcttcaaacaagttcatgtacctcgactacctgaagtatttcaaagcgtggattgcgtatcgcattaagctcgaaactgcgatgctccagaacaagctgacgaaagcagagaaggcattgcacttacagcaagtctacctctgggctgtagacaacatggacaagctgctcaaagtgttgccgaaagtgttggtcgctgctgaccctgacgcgatgcttgcgaagctgtgtaagattcctgttgaagatgcgaagatcatcctcgaccgtcaggtacgtaaactggcgaaactggaacgcagtggtctgcttgctaagattaaagaaatcaaggcagagattgctgggtataaagcaggtctgaaagagccaggcaaatacgcagcagaaggtactgctgcgaaagttaaggcgtatatgaaatcgcccgatgacaagatgcctgtcaatctgtaatagatctgtaaatacaactcagcatattctaggacgaaacgcggttgtgtctgtatgtcatttatgttacaatgacgtgtctgtgggtagctgtctgttcgggagatagacagctactcgaactcataacaggagggtacgttagcgcagcaaatattcactcaggaaaaataaacgagcctaaaaaaggccaaccagcctgactgtagattataactacggcagagcaatactataatcgacccacgtaatgctaatatgttagagcaacattggcattcaaagtgtcgctagggccggcaggatatggtcctcaactcttaatgaagtttggaaatccatacatgaaaaatcaggtagccaacctcaaagctggtttggagaaagtcaatgcagttctgacctctctgcgttcaggaaagaacttgaaacgccagcatgttgttgattcattaggtcaaccgacctctgtcttagctgatctcacgaaggcattaaaaagtaatacctacaagtcataccccgatgtaatacagttgcgtgactcagttcgtgcaacctgtacttcctgcctaagcctgtcagagcaagtggtcgctcgtcgtatcaagccacgtgaactgatggaaaagctcggagaaattgtgaagtcgttcgacgccgacgccaagttggctaagtcgtgtttgggctacctgcctgaatcacgcaaaactctcagtctcgatgatctcccagaagacagcaaagagcgcttagaagctctcaaagctatcgacaaagaggtgtacgagaacgaagcgaacgataaagctatacgccgtgagcaacgcgaagacgcagcgactgccaaaacaagtcgtgtgctacagcgcctcaaggacgcttactctcacaaggtcccgagaacgttcaacaaagctattcaaataatccaacttcctgtgatggcacgattcggtacactcgccatgagtcctgaatcgctctctcgtatgggcttcaaaatcgaaactgctggtctgcactcaacccctagttcggacttaggtatcgtctttgaaaaccaacttctgctgttcttccgtatgtccgacgcgaaaggcatggcagaagaagctgcgaaagatcacaagatgcttgatggaactctcgtcgaacgcaaacgcctccagaaagaacgcaacgcagaacgccgcgatctcaagaagctgaacaagctcctagaagaatcgaagtcgctcaaagctcgtcgtgctctccgtgaacaaatcgcagagactcagacagagattgacgacattacggcgaagctcgattcgatggagtacaaagtgcgtgagtcaggttcccgcgagcgtgtgtatcgtcagatgaaaacatctagcgatcatgcgatgctggattatcttaaccccattgtcgatatgattaacgagaagggaagttccacgttaggtctgtttactaccatgccgttacgcggtgtgatgaaggattcagacgtgcattgtgcttggcttatggagaaatcagcgatcaacttgttgctacgccacactggcggcgatatgaagttgcagaactggttcctgccgtggactaatggctaacgagaaccgtttaccggcggtgcagaagggtgatttgtcgcagtgtatcatctgccagaaattcagtagatcgattcactaccatcacaccattccccgctcactgggtggcgaagatagtcttcaaatccctatagacggtgactgccacacaacgcttcacgcaaaagcagaagctgtggtagcgaagttagcaggtaaccgtaagcaaccaatcgggacgttttgggataaccctgagacagaacgacgagcacaaacgtggctagacattctagttgatgctatgcttaacccactggtgcagccaggacagaaagaagtgctgctaccgatgatcaaggttgacatggaaactagacatgctctcgaactcttgaagcgcgacacgcctggcattactaatatgagccaagtgttgcgatattgtattgagacaacattaaaagcgaaggggttaaaaaatggcgaatcaaaaagtacgcactctggacatcaaagcactcgtaaaaaacgaactgacctgtggtgattgccgcggtctgactcgtgatgctcttttaccgactgcggagaaaccgtgtgctacgcaaggtcagttagccgattctaagatctgcaaacactatcgctcagacagccaatcgctgaccgagttgatgaccgagcatggtgattcacttgttgggcttttcaatacgttcaaaaacttcacagacaaagatctgcgcgttgtcgctggtatgttgttagctgaatcgaaaacccgtcgccacggtgtgcgcatggggcaagcagtattcgtgcgctatcaagggcgcgagacacgcaactacctgaacaacttcatggcagcgcgtgtgttggatgtagacgacgatacgattcgcctgatcagtgagaagggtgacattgtgttgacgtatgcaaacacaggattcaatggtccgtccgtatatactaagaagcaatttgctaaactgcgtaaagagatgatcagtgctggcaagctgattgaccctgaacgcgagatcaagactgccaagcgcaatctcccgcaagaagacaacgttaacttctccgcaccgagcgacctcgatgggttctctattcctcttatggaagacgtggccaaaggccgtggtggtaagcgtaaaggtaagaagacccagacgttggtcgatattgtgagcatgatcgaaagtggtcatgacatgggagcggagcaagacgagtctggcgtaatgtcactcggcggcaacagctatcgccacaagaagaagaaacttaacgtcggtaagaatggcgtggttgaacttggcgatatgtaagttaaggtctacacagcaaatatacttccaaaaacaatacgaataggatctcggaaaaatgatcacaacagaagaatcaggccttaacgaatatctttcacgccgtctgggtatcgaggagaactcagaggaattccgtcaagtatacgctgcaacgatacgttacataggcagcgggtataaatctatcgcggattatcaccgtgatttgcaagcagcaattgactttaagcagttcgaatttactgctcctgacttgcgtattgatatctcttccgtgtgtcgcttcacgttgaagatgcgttactttgtgttggctgtctgtctgcacaaagacccagtatcaacagttaaaaaatatgcgtcgtatggcctgtctcaccgcgaagctgtccttgcttggaacctgattctcaagcacgacaatcaacgtaagcagatgcgccgtacggctaaagcgcgagcgaagacaaaaggcggattggatatcacaatggtgtccagccgtgaactacgcttgcgtcttgatcaaacgactagcctgtttggtgagttgcatcgtaacgccaagcgtctggtcagaaagaatttgcagtgggtgtcggtcagccataacattccgattgctgatctgacttgcgatatcatgtgcaaggtgttgttgtcgtactatcaatccttgcctaatcgtttcagcgagggccaccagctcaactatcttcgtgcatcactgacgaaccgcattaacaacatgaacaactactacggcgcagagaagcgcaagcgtatgaagaaagttggagaagacaagtatgagattgtggttatgtctgacaatcagatgtggcacaatccagacgacgacagctccaactcatacgaagacatgttgggtgaggacgctcgtgtgcataccgagcagatggaaaacaatctgactatcaatcgtcttctggaagaggccgagggcactaagcgccacaaactgtatcagactgttctcggacgggattgcgccgagttcactgaatatctgcgtgagaacgggttactcaaacagaccatgacatgcgccactcagtggatcatggctaaacctacgaagtttatacgcaagaccttagccagttggttgcaggtcagcgttgacgctatcacaggcggtctggaaacgttacgcggttcattacaggtagcatgagaggtcaccgtatagttatgcagcaggcaatcattaacactgacgtagagcgctctgcactcgcgctgttcagtcgtcctcagttggatgaggactataagcgtaccgtgttgtatctcgtgtataagactgtaaatcgtaatggcatgatgcaagtcaatcgtctgctgttcgaattgagccagaagtatgaactcaacaaagaagatgtgaagtctgctatcggtgcgctcaaagctccgtacgcattcaacgcgctctctgtgtttgtacctcgcgcagatacaaaagcaaatcgtgtgtgtcgtgtgaactccacactggcaatcgaaagttggattgcagaagtggaacaaacccgtccacatatcgcacacttgttgcagtaggggcataaatggaa

SEQ ID NO: 4 - DNA, 74833 bp, unidentified
  source 1..74833: mol_type = genomic DNA
atgcaatggtgcattcatatattaaccaggagttctatcatgtcttcatctcgtctcgcattcggtaacatcatgggtactgtagtagatgctgctaacactgtatctaccactctgaatgtagtaaccaaatctgttggtatggttgacgcattcgtcactaatgctgctgaaactcagcgtatccgtatgaaactggaacagtcttcacgtactgaacagctgatcgaagaaactgctctggctgacactcaacgtcagcagggcattaaagattacctggaagctaatcctggtacatctgatttattcaaagcaaatcaggaacgtctggctgctgtactcgcagctaaataacacctaagccctagcaatagggcttaacacctttaactggatggataggtatagacatatgtttaaggtactcatcacactgctatcaatgctctgcttcatctatggtatggctgacatgcttcatgtcatcaaccatttgagtccttactcagatgtcattgccatcctactgtcagctctgctatggatggtacgttcactgttaggcgacagtgaatctactgaacaagctactcgtaattaactatcacgcttcgcgtgtattgggaataatccctaaatcaaaaactctctggagagaaaaatcatggctatcgacttaccaaaatcattcggtcagaaaaacaatgctgcaactgataaagagcagcgtcctgcaagccagttctggcttaacgtaggttatgaagtggaagtgcctaatgcagaaggtcagaacgaaactcgtttcgtatcactgcctgctggtattccactcgacaacattgagcaacttgttgtcaaaggcaagaaccaagactggaatatgttccaggctgcacgtaacgatttactgactcagcttatggaagctgcacagtctatggcacctggtgaagaacagattgttaatctgcaaattcaacttcgtcgtaccaacaacgaagaggtcaaagtagacgcttcaagcaatccatttgctcgcaaactgttctaacagttagagttatattagaagagaatccacgcttatgtgggttctcttttttaacggttgagatagacactatctaaacaccaaagtagccagaaatactcaaattactaaggacaccctaaatgtcatataccatgctgaaacagttccataccatgcttcctcgtgaagctgtgcctgctacaccacagtctctgaagaacctcaaagtaggtgacttcgtgaagattggtgttgagtgtgccaatggcagaactgaaaagttctggctgaaggtcgaagaactgggcaatccaatccgttgcactatcaatcaggatttggtgctcactcgttatcatctgctgaaatgcgatgatgaaatctggatccagaaagagaatattaatggggtaatgaaaggtggcctgtgaagatattaatcatgatgctctgtggggcatcttgcatctgccaacaagaaaactgctaaggcaatggccttgtggttatggtcatactcaacttgatgttgttgatgatcctgccaggcagagaaaaacaatggctactccaagactattcctcagtgaagatactgcaaagcgtgctttgactcagtggctcgctggtgtgcatcgtaatcactacgatgatggtctggaagtaacaagtccagtggtgcctcgtatcaaagaagatatgaaggttgttcctgtttatctgtatacagaggctccaagtgaacccgattattgaattgttcttcaagtgctatctccaatggatagcaatggatcacccagaaacaaaaacctttgtgaaccgtcagggactgtgtggcaacatgtctggcttgtttcacaaactgcgtgtgccattacatgaacacaatgctgctcgtacagagttaagcaatatgttctttgatgatggtctggatacagactttccattcaatgatggcagtcacaaaatgttccagtgtgaaatgtactcaggctatggtcatgtgaatgaacatcgcattgagtgggttaaatctaaaatacctgactttgagccagatggatcaatgatgggtttcatcggttggctgtcatcttacagaggtggttatgaagatagtaatattcggtgggaggacattcgaggacagtgcctggatgataggcgtgctcaacgaattgttatccgaaggagtgattcacagtgattgtgaattagtttgtggtatggcacggggtgcagatatgactgcatatgcgtgcttcaaagatattggaaatacgatccacgagtattgggcagactgggatggtctgggcaaacgtgctggattcgtgagaaatactgaaatggcacaagttgctgatataggcgtagcattttgggatggctcaagccgtggtactaagcatatgatagacactttggataggctgaataagccgtgctatgtggtgagatatgctgttaaaccgtgaatacgctgtatgtgaaatatgtggtgaaccaagaagtaaacgggttcaccgtaaatgctctcgtatattgcagagacgttatgatcccgtacagcaaaagaaaatactggcaggtgtgcgtgaagatgagctgaaacgttctctacaacgtgacctgtctatccgaataaatggcaggcataaagatgacaattgaaatcagagataaacgtaatattgatctcgttcaattacgtgatttaaagaacggtgatcacttcatgttcctcaattgcttatatgtaatgagtcaacatgagtatcaaagtggttactgtctctgtaccaatatcaaagatggtacatcaacgactatctctaaaagtgatcctgttcaacaggtgcatttagttatagagatccatctcgtctaacatctcgcttattgcagggcaagccctgcaaacgctcgcgtttatattgaggtatatatgaaatcttattgggctattcagcatattccaacaggctatttcatacctgaaccaagaacagttcgacgtactggttatactcaggttgagccaagggaagatggtattcctcggttgtttgaaacagaggacaaagccaaaagagcacttgtgcaatggctgcgtggtaaacatgaacaggtaactgataccgaatcagaagatgaatatggtggtcgtagctatatcgtcgtagtaggtatggaagctgttccggttgcatctcgtaagaaagaagagatgcgtgttgttagaattgattttaaggtaactgatgaaaacagtaataatcacgggcgatccctggatcactgatgctgacatgctgatgaagaatcttgaatatctgtttggtaatggttcattaccaccagagttcgaggttatcactcagaacgcaccaggcgttgaagcgactattaatccagtgctcgaagaagctgggttgaaagtcacagtagtggatgaattgccggaagtcgatattgtcgtggtgttcctcgataatagtgatgaacgtgctcacgctattatgatggcccaatggggcagtcgtaagccagtgttcccattccacgtatccaagaaaggcgctcaatagagcgcttttttaatctggagctaatatgcagtgcaaatgtaagaagggctataaaagcacctgggataacctgtgtgctaattgccgtactccacagcaacagaaattacactcagccaaaatggatgaggtaatggaatatcgtattactatcggtaataaacatcatggaaccaaaggagaatatataggccgtggctctccaatgggtaatccatttgttgttcatggtgatcaggacagagagcaagctattgctggctatcgtaactggttgactaagtgcattgatatgcaagagccaaccattattgctgaactgaacaggctggcatacaaactaatagatgagaaggaactgacattaatttgtttttgtgctccgaaggcttgtcatggcaatgtcattgccgatgtattaaggaaagttttatatgattactgtaatcccaatatctaaagcacgggcaggtgaaaatgtatttcgtatacatgagcctgctcaaatagctaatccattcggtattagtcatcgtattaccaaggaagaatgtgcattggcatatgaagcctggttgaaacatcgtatagccaacaacgatattgtcgtatgtgcagagcttaaccggattgcacgcttcgcgtgtgatggtgaggctgtgttagttggctctgaagctgacggtgcagttatccgtaaactaattgaagaggctctaaatgaataatctcatttatatcgggttaattgtttttctggtgtttgtgattgtattggtatttattgcttccttcaaagagaagcaacgttatacctggcacgaacaaggtgatgccaatttctatcgtattatggacgatggtaagtggttcgctattgttcagttaaatggtgaaatgcaccatgctgcacaggaagagtatatggacactattgtcgaggcactgaatgacaattgactatcgtgctcgtgctacaaaagctgaacaggctaatgctgaactcagtgctgcattaaatagacgaccaaagcatgatgcctttgttgaacaaataaaggtaatgctgaagttggataaagcctgtccctataaccaggttattcaaaaaataaaacaactcactgttaatcaggagctatacgctgctggttccaatgatcgtcgtgacctgaaccaagaaaagaaactctctttcgaggaaggtcgtaaacaaggtctgttagacgcaatcgagaaaatcaaaaatggctaaagtatttgtgttcggaagtaatgaaggtggtattcacggtgctggtgctgcgaaagaagcatataaaaagcacggtgctcgttatggctcaagctatggtcactttggtcagagctttgctatcccaaccaaagacaagaacatcgaatatacgctgccactggcaaccattgaagcgtatgtgaaagggttccttgcctatgctgctggtcgtaagaagctgacatttactgtcactcgtattggctgtggcctggctggtctgaaagacaaggacattgcaccaatgttcaaaaacgctccatcgaactgtcagtttgatgaagcatggcgtccattcctgggcgatgacgtaacttactggggtactttcgaatgaacaagctggacactatctggcaacgttacctgaatgctcgcattcagatgattgaaacagctattgctgctggaaagactgacgaagagatcaaggcagtgctgcttgatgaagaacaactgaaccagtctatctactgtgctcgcacttatatcaaggtggaaaccaatgagcagccttcaggaactgcatagtgctcaggttagaaccagaggaagaacattccatcactggtactccaaccttcagcatctgattaagaagcgtactcaggctgggcacattgacggtcatcttcgtgttgaagttgatgaggatatgtaccgaggcaagaagtctgattgggttcgcaaagaaactgatgttatcaaaatcgttgttcgtgttggtgcagcaaaccgagcaagtgacgggccgtattcacctggcaaagcagtaatgatttactttcacactaaccgttagaattatcttagaggaagaagcgatgtctactatgtttgcacatcagatgctgttagagaaactgtttgataagaaccagactctacctcgtatcactgaagagtttcgtaactgtgccactgtaaactttgttggttacatggaacaagaaggtattgatgttgagtttggccttgctgtcatgactcaaatggcattgcacaagcgtgctgatctgccaaccctgttaggaacagtccgacacttctatccaactgcacaagaagtagctgataagctgctattgtgtgcaagtaaggatttgatcgactggaacccacaactgaagacatttattgtcatctacaccgttagtcgtgatgtccagttagagattgatcgcttctcttatccattaccaatggtcattaagccagtagagatcaagtctaacaaagagtcaggctatctggcacgggactgctcagtgattctgaagaacaaccatcacaataatgatgtgtgtctggatcatctgaaccgtatcaacaagattgcattcagtttcaatatgaatactgctgctcttgtgaagaactcatggcgtaacttagacaaagccaaagatggcgagtctaaagaagactatgagaagcgtgtacgtgcttttgagaagtacgacacccatgcaaaagacattatgggcttgttaacttctgaaggtaacgagttctatttcactaatcgctatgacaagcgtggaagaacgtattgtcagggacaccatgcaacttatcaaggcacaccgtggaacaaagctgtccttgagttcactgataaagaggtagtaaccgatgaagcctgaagatgaatacgaatttcgtcctgaatgtgtgctggtaggccagcgtggaatcatgatggtagacgctaaaggcgttgtcatcttccagactcaggatgctgctaccgggcagactgttaaagtctgtctgactgatcatgttgaagaaactgaagcactcattgaagtgctacagcacatgattgaacaccaacgtgaaccagaaagaaaagctgatactcagcctgctgaccaaacgttcgcagagatgatgcagcacctgtccaaaaagaaccttcactaatcaaccccaattgcaagaggcatatatgcagcaattcaacggtatcgaatatttaaagattgacgtagcaaactcctttggtctggacaaaaagaaatggaacgagcgtcttgcctggttcaatgagaacgagcatcagctcgactctctgatcgaacaggctgactcacctgcaatgttctttgctggtgtgcaggcatatcgtgacgctcgtgagggtaagccaattggctacccaatctcactggatgcaacagcatccggtatgcagattctggcttgtctgactggcgaccgtaaagctgctgaactgtgcaacgttgttccggtattcggtgacgatgcagaggcactgcgtattgacggctataccgtcatctatgatcgcatggtcactaccattggtgaagctggtcagattgaacgtgatgactgtaagcaaggcatcatgacttctctgtatggctcacaggctatgccgaagaaggtattcggtgaaggcaaactgtattacaccttccaggacaccatgaatgaatcagctcctgctgtatgggaactgaactcagcattcctggacatctgggatccagaagcaacagagcacaattggactctgcctgacctgttccacgttaaagtcaaggtaatggatgaagagacagagactgttcacttcctcaatgcaccgtatgacacctatcgtaaggttaaccgggctaccgagtcaggccgttcactgggtgccaatggcactcacagtatcgacggttacgtagtacgtgagatgattcgtcgttgcatgtatgacatggaactgatccgtaacgttcgccgtatggttgaagagagcaaaggcggctacaaaatacagcctgtcaaagatgctgattacgacatggttgtaagcctgtgggatatgtatctgaagacgggtatgctgtccctgcgtatctgtgactatctggactatgacaacatcggtctggtagacgtagaagttgttgaagcattgctggacactctgcctaagaaaccgttccaggttatcaccaatcacgattgtttccgttgcctacctcactatggcaatgacctgcgtaagcagtacaaccgtatgctgtatgaactggctaagggcaatctgctaagtcacatgttgtcccagatgaccaactctgaagttcagattggtaagctggatccaacactggctgacgatattctgaacaccgagtatgctttatcataacaactggactcccttcggggagtccttattttttcactggagataatcatgatcctgaatgtctcatacaatgaaaccgataaggctgtgctgctacagcctatcaatgcaacgctgcctgatggatacatcttaattggtacaacaggcactggtgttgcatactacacagcagtgaaactactgctggaagggtacggagttaaacagatggcagaaattaccatcaagtttgacgaccttgcagcaacattggcaacactgagagaaatcgaagagttgtctaaacctgaaccagaaaagaaagcaacgagtgtgggtgccacagtggttgaacgttcatctggtattttcaagtagaggatttatgaaacttcaagccttccttaacccgaccaccaagacagtccaggttgaactgactggtgtagctgctccaactggcttcaccaaaattggtgagttcgatcacccggatgaaacctacccggatagcaacgtgatttatcacggtgtgcgtgacctgctgtatacgaccaagctggcctctccacctgtgacaggtgtgaagtacccgaacggtatctacaacatgcaggaaatcagcattaccacaaccaacgctgctatcaagcaggaactgtactggctggtcgaacctcagcaaactgttgtgtttgccgtgggttctgatctgctgctgtccggtcaagtgggtggtggtaaaaccccatacacttacaagtggcagttcgctggtggccctgctgatgccttcgttgacatctccggtgctactgcactgaagctgtccaaagaggatctggcagccagcgatgcaggtatctataagctgatcgtcactgatgccaacgacattactctggaaagtaagagctatgtcgaagtggtgcctgagacgcctaagtctaagctgcctgatgcacccgctgcattgacatctatcactgcaaccccatcaccactggctctgtcagtagcaactgatggaaccaacggcaaaactgtggcattcgctccagtgcctgctgatgctgatctgggtacgctgtctattaagactgctccagcctctgcaacagcaactgcgaccattgccaatggcgtgctgactgttaaaccagtcgctgcgggtactacctctgttgtagtgaccaacggcaccaaagatgttactgtcaatgtgaccgtagcagcctaataaataaagggttagcactttatttggttgttaaccctttaatccaaacaggaaaattccatgcgtaaaagccatctctggggcatgtgcctctcgtttctgtcagtcttcgtcggcctgcattatgttggcgatactctgttccttctgcgtgaaatccccgtctacattgtggcctctgctgccgctgttgttcctcttctggttcccacggcaacgtggaaagagatcgagcgattgtgtagtcaggcgattaagctgaagttgaacctgttttcccgtccggctggtgcaagcgtactgaacagtcctctgctcagttaacactgctacggcgaaaagagaagcccaccagaaatggtgggctttttttatggttgttccacccattcagaagcgtgcaaagcacaagaggcaaatatgttcctattcccacagcaagaaaagttcgttcgtcaggtcggtacgatccttgagactttcatcgagtccgattgtgaaatccgtccccactttcacgttactgggccaagtggctccggtaagtcctacctcattggcaaagcctgtgaggaggttggcgttaaaatgatcgagattaatgcagcccagcttactgctgaaggtctgtcaggtaactctctgtctaaagccttgcgtccattgcgtgagcactggaatatgccaaacgtcatctttgtagatgagttcgataagctctttcaaaccaatggtgagaagactgagaacttccgttcacaggtgcaggatgaatttctgacctgcctggaaagtaagtattccagcattctcactgactacggcaaatatgatccggtacgtatcgacaagtctctgtttattttcgctggtgcgtattcgaaccagaagataaataacatcagtgaattacgcgatgctggtatgcgtactgagttcctgggacgtgtgccattgatcttcagcacagtggaagtaacaatggaagatttgcgtaagcaaatcaaacacgtaggtctgtatcaggcttataaacgtctgcgtccagaaaccaaagatgctgatgctgttaaaggcattgccaagattctggaacaacagaataaagatatgaacatcggtattcgtttattgaatactgccattcacctttattttatgggcaatgtatgaaaacgagtaggcgtgaagaaattaagcagcgtctttatgctcaggccaagatcgaagataccgggtataccgttaatggcataccgtctccctgtcatctgtggcagggggcattatccggttctggacgtggtaagggttatggacgaatctcaattaacggtgttacttctgctgtgcatcgtgtctcttacacccatttctttgggtatattccgctcaagcgtcaggtggatcacctgtgcaatgtgcgtaattgttttaaccctgagcatctggaactggtgacacatctccagaaccagaagagaagggatcggcgtaagcaggagaaatcatcgtgaaccgtaacgatttggaattacaagaggccattgattcagtgaacaatggtgctcgcaacagtggtcgtactactcgccaggcttttagctatgtcgatcagatgctggccttccctgataccccagtcaaaattgtggatcactacaacagcccaatgatgaaccgtgagttaactcgcaaggtttgtctgattctggatgctgctggtgtgccatataacaagctgggcgaaaccatcatggaaatccctaagctatgaagttcacagcctatgaagtcatctgtgccagtgtctatgggcattggcctgatgcagtgactacactggctctggctcagggatttgccattctggatggcagggatatggatgatgcaatgcgtatatgtgctgcaaagctggcataccgaaccaaggataagaagctgcaaagcagtctgctgtctatggtcattgcagagtatcccagcaatatactgctgtcactgcaacagcaggttgataaaatggtcaagaacctcagaaagaatggtggagaaaccttcgagtatgagagctttgaagccatgaaaaacctgctcaaaaaaccctctcacataggaatgcgtccatgaaaaatggcccgtaccaaattaagcaattactggaacaactggaagctggaagcatcaccgagacacaattcatgttcaaggtgagtaaagcagccaacgagttccacgaaaagctgcgtcatggtaacaacgaacgtccgttaccagcacgtatgggaactgcgaagaagatttctaatcgtcatcgcatctcctgtcactaacaactgccgttgtttaatccgagccacctgagaaggtggcttttttattctctggagaaagtcatgggtatgtatcgtgtaacaccacgaaaagccgtgagcctgatagaggaaatccttgcggctggtctggtgccattcatgcaaggaagtccgggcatcggtaagtctgcaataggcaatggcctgagcaaaagttttaacctggcaactgtcgatcatcgactgtccaccagcccaccggaagacatgaacggtctgccgtacttcgaagaacgtccatatggcaaagtagcgtgcttcgctccatttgccgatctgttcccgattgaaggtatgcctctgccggaaggtaaagacggttggttagtgtttctggatgagtacaactcagccaagaaagacacacaagctgcatcgtacaagctgctcttagaccgtatgacaggtcagaagaagctgcatgaacgtgtggctattgttctggcgggaaacctgtccaccgaccgtgctatcgtcaataacctgtccacggctgctcagtcccgactgattcacctggaactggaagtgagttatcacgactggttgcgtgacgtagcaattgctcaggactacgatccccgtatcattggctacttcagccagtttgaagaggatctgatgagctttgatccaaagcacacggataagacattctgctgcccacgtactgttgagttcctcaaccgtatgatcattggcaaagatgtcaccgaagacagactgccgatgtatgcaggtactatcggtgaggatattgcaaccaagttctatcagttctgtaacgtctataaggatctcatcaagtatgaagagatcatgaaagacccactgaactgtcgtctgcctacctcactggacttggcctgggccacagtatctggtctggtcagcaagatgaccatcaagaacttcccaacaatggctgcttatgcaggccgtctggggctggatatgcgtatcctgttcttccgtttcgcaatggctaagtatcccgaacttcgccgtgacccaacctttgctgctgtcgctgtacagttggcaaaatacctcaatgaggattgatcatgggcctgactattctgaacgataaaaaggaaggtgatcgtgcttacatcgccacctttgaaggtaaacaggtaggcttctatgcaccagcactgtggcctgccaaacagcttgcagtgcagtatttcaagcctgccaaaagaaagatgggcttgttatccgttgagctggctgagggctaagtaatggtagatcttacccgtgaactcgaccgagtaaaggcagacgtattctctggtaagaacgctgctttccttggttccctgatggtcaagctgcctatgcactgggacaccagtatcaagacagcacagaccgattttgtcagtattgcctggaaccctgagtggttcatgagcatccctcgaaaaacccgtggcacagtgcttgtgcatgagatttggcacgttgccagactccatgcttcccgtcagggtagccgtgacatggagacatggaactatgcctgcgatctggagatcaacaatgctctggactatgcaggctattcctttgagggtactcaaccgtggcttgatcaccagtacgataatatggctgctgaggacatctacgatgttctgatacagaaccagatacaaccacctcccggtggtgcctggggctgtggtaagccggatatgtgttctggtgatgggctgagtcccctcggtcagcttaatttggttgtgggtgccctcactcatgccaagttagctggcgaagctggcactctgcccggtgatgtgctggaagtaatcaagaaattcctgaagcctgttgtgccttgggaaaaactgcttatggacttcatgacagaactgtcagaagagttcactacgtgggccagaccgaatcgccgttaccctgaaatgtacatgcctagtcgtgacattgaagaaggcaagctggcacacatggcatattttcttgatgtctctggctctatcacgagccgtgatgccctgcgtttcaactccgaggtgaagtttgtctttgagacatacaagccggagagactgaccctgatcctctttgatgttgtcatccagcgaatttatgagttcgaggaagacgacgattttaccgaagtggaaatttgtggtcggggtggtacatcccttgtttgtgtccgtaactggatagaacagaacagaccgactgctgccatgatctttaccgatctggaagtagatcctatggaaccgcttacgtatgacctgcctctattgtggatatgcaacaaggctggcaaaagtgttccttttggcaaactcattcacataaaggaataacatggtcattaatggcgaagaactctggaaaatcgagcctatcaaaggcatggaaccagggaagaaaaaggctttcggcgtttctcatggtttgggtgaagctggttacgacattcgttgtgcccagcaaatcatcttcggtcgtaagttcgatactcgcatggtagaagtctctgtgatggaaaacggtatctccgttgcttccagcactaagccgggcaagtttacgcttgcctctaccgttgaagagtttcagatgccaaccaacctcgttggtattgtgcatgacaaatccacctgggccagacaaggcttgtcagttttcaacacagtgattgaaccgggctggtcaggcttcctgactttagagctggtgtatcacggtgaagaaacactgataatccctgctggtgcaggtattgctcaggtcgtgtttcacgaactggcagaatcggcctgttactcaggcaaatatcaggatcaggctaatgagcctgtacctgcaatcttccaaaagtgagatccaaaaaatgtcaaaacaactgtttgaagtttctgaagaaaacggcaccaagcattccatcaatgcagcacacgttgtggctgtagttgacaacggcgacaaaggttctgccatcgtgttcggcttcggcggttcgctgaacgtgaaagagagctatcgctctgttcgcggttacgtgaaaaaaggtctggctgtcgctggcgatactgacgcagaataagcgtccgtaaaccaggaaaagcccctcttgtaggggctttttcatttgaacaagcaaagaggtttttatgcgtagtcccttgaaatgggtgggtagtaaggcgtcaatcatgccccaactctcaccacacttgccgaaaggtaaacgtctggtagaaccctttgctggttcctgtactgtcatgctgaatactgattacaatttttatttggctggtgacagcaacccagacttgatcaacttctttagcctggtgaaatcccggcctgaagacctgatcgaagctgctgagtacctgtttaccactcacggtgatccttattattacagtgtccgtgacctgttcaataagcgaactgcatcatctcttgagatgggtgctatgttcctgtacctgaacaagtttgggtttaatggcctgtgccgttacaaccaaagtggtgctttcaatgttccatctggcaaacgtaaaaacgtagctgtgccgggtgtggaaattattaatgccagtgaaaagctgcaaggagtaaaactcttttgtggtgattggctggacactctgaagcaagttcgtgagggcgatgtcgtttacatcgatccaccatatattccgatctcgcccactgccaacttcagtgattacacgaaggaaggttttggagaagcggatcaaatcaaactacgtgatgctctcctggacttaggtcagtacggtattcctatcgttgtctccaacagcttctgccgtaaatctctggatctgtatagtgatttcactgtgcatcatatccatgcggcccgtgctgtgggtgggcaactctccgttaaagagatcatcgcaactctcaattgttgaggctgctatgtcgtcaaaagaacagtggaagcaggctattgagtctgctgtcgcaaatggtcgtggaatactctgccgtcagcttgaagacggtcaggtaactgtcaatgctctcactcctgaagagttcttcaaggcagtgaacgtggacatgcccccggagaaagttaagttcctcactgagatgatgggactggacttttctgctctggaacgccgtgccctggctgtagccattagtggtaaacaggctcgtctgattattgctgatgacatccgtggtgatatgtcaatgatgttgactgaaccagaaaaagaagaatctgtgcaagtaggcaatcgcctggttgctcctaatcaccgtactaagggcaagaagcataatctgcccttttacctgggtaaaaagaggttttaatgaagcgtgaaatttttgatgactgcatcgaagctgtgctgtcagagcatgaaaagaaagtcgttgccgtaaaccaggcaccaaagttcaccattgaatcaatcactggtgtggaagtgtctggcacgatcctggctgtaacgcctaatctggtaacggtcaaagaatggttgcacgattcaatgcgtacaatctacattcgccgtgagcttattgtcatggcgagcgtgtcctacgtcactctcccagatggtgaataatgcaaaacctgtttgctgcgtttgacgattatgtctcatggcgtaaccgtgagatcttctcgttgctgctgttcgttattgttgctgccgtaccctttaccaccttcggatcgttgagtattaacggttctgagtgggccacactgttcaacagtggcctgactctgctcgtgggtggggtatcgctggtaatgtcctttatctacgctcacaaggcacgtaagagctataagctgttccgtgaactgctggagaaagcataatgaccatttctgctcaggtgatagcagatagtatcgccaacggtgttcgtatcacgacactgcaactgcgttatccccgtttcatccatgccgaagtaatgactcaccgtgtgttcagccgtaatgcgtcaagcagccgtgctatcccggtgaagaaaatcattgctgacatcattgctgatccggcgatcccaatgcactggggaaaaaacatccccggtatgcaggctcatgagcaaattgatgagccagtgcaaatccctgtacatgccgatctgaaccagtcattagtcggtgtgtcgaaggagcaagcctggcttatcgctcgtgatcgtgtaatcaaagttgctgaaggtttcgacaacgctggttatcacaaacagatcgtgaaccgtctgcttgagccgtggtcgcacattaatgtgctggtcactgcaactgacttcgccaacttcttccacctgcgtgatcatgctgatgcccaaccggaaatccgtgaactcgcacaaaagatgaaagtggcgatgtctcagtccaagcaaactgaactggccccaggtgattggcatgttccttacgtgactgctgccgatatggtagccatccgtaatgagctgaaatacaaccgtatcactcgtgatgagccgtcagtgaaagagatgatggacatggcactgaaagtgtctgtggcccgttgtgctcgtgtcagttacttaacccactctggtcgtgagactaagctggatgaagatctgaaactgtacaaccgtctgctgggttctgccccgctgcacgcatctcctgctgaacatcaggccaccccagacaccaaatcgtactctactgattacggtggtgaactgtgggataacgagtcgttgcatggcaacttccgtggctggattcagttccgtaaaacgttaccaggggaaacctacccaggttagttcttttcttggttcacccaacaagtgagccatccccatttgtaacgtttgcccggattcgtccgggcttttttattgagtctttacagagaggttggtagggccaaaccttaatgatccactgtggcccggttggtcatatgagggctaccagcctcgctgtaaacactcaaccactgaaccaaaggaaaaactatgtccgaacgtactggtgcagaaggcttggctgacactattgctgctcaagctctgcgtatgcaggcacaacaaaaattgtggctagaacctacccctgaaatggttcaggcaggtttagctgaagttcaacgcatactggatgaatgggaaagtgaccatttaggctggtgtgttgatgacgttaccgatgacatggcctctgatatggctgtattcgtattgcaggctatggctggcaaactgccgaaggagcctgaaaatggctaatgctgaagtaactcaggtaacagtattccgtcttgtagtggatctgtcaccaaacgaattagatgccctcaaagctctggttcaaaacccactacatcgtccacaagacgagagtccttctcaacgtaacatgcgtgaagctatcttcaacgcatgtaacaaacaccgtacttaactccaaacatccgagagattaattatgcaagtcgcagataatactcaaaccgcctcgtcagcaactattggtgctcaggcaacccgtaaagtgtctatggtcgaggatgcgtcattcttcatgatgctgtcctctaacctctactctaaccagaaacttgcgttcattcgtgaggttctgtgtaacgcctgggatgcccacatcgaggcaggaactactgatcagccagtgatggtaagcattgatgccaaccatgacctgatcatcaaggactctggtaagggtatttctgacgacttgatcgatcagatttacggcacctatggtggttctaccaaacgcgaagacaaagcaaccactggtggctttggtctgggcagtaaatcaccgtgggcctacgtggaatctttccgtgtggcctcagagttcgacggcaagaagacggtctataacatggcccgtacctgcatcgagaacgatggcaagccaggcattaccccagtgatgacagtaccaactgatcgcactggcctgactgtcaccatccgtctggaagaacatgatctggatgagattgtcgaatatatccaggcaatctccctgcatggtgatatgcgtgtgcagttctgctgcgtaccgcaaaatctcaatcacttcgtacccttgcgtcaactgggtatgtcgagtgaacccggttcctataacctggactctgctcgctggcacttctcctatatggggaaccacaaagtcttcattcgctatggtgcagttatttaccctgcgttacgcaccccggcaacagaacctgcactgaaggtaattgaaaccttcatggagactgtgggctatacccgcatcgtagttcaggctgcaccaagcactctcgctctgaccccaagccgtgaggcattgtcgagccagaagatgacagaggacggtatcaccgacatctgtgtcgatctggtggatcagattgagaaagaaattctggcaaagctgccggagacaatggaacaactgaaaaattacactcgtcgttacaactacgaaggtatgttcggtaagaaaattgacttctggcagaacatccaaaacccggtagtacaacgctatgtgcgttctaagctgggcaaagatgtccgtaccaaatattaccctgctttgtgggacattctgaaggtcggcttcaagctctatgctaaagcaaacttctcccgtgaagtggcccgattcctgatccaacagcactggctgatccttaacagcaagcgtggtaaaagcctgcgttatgagagccgtgttgtcgaagctgctgcacagaaatacatcgttaagccaaaagctaaactggtctgtgacagtaacggtctgatcaaaggccgtgacctgctgatggtcaaaaatacccactggaacaacatggtcattaagacccgttggtacgatgagtatgagagcatcaaggatctgagaaacggtattgaaaacaagcgaatctttgtgaccacacgtatcaaagatctgcctaagtcagtagccaattgccctcagacgcctgttagcgatatgcgggaatgggctgttcgtgtcaataaagcctcagatgtggatgcagttatcgcatacctgactgatgctggttacgaagtcattgacctgaccaaagtcaacaagtgggactcagttgctgtctctctggatctggaacgtaaagctaaggcgaaagccaaagctgaagggaaggaaccagaaaagaaagagtccgtgaacatgctggtatccctgaaaagtctgtacgacgacaaaggggacaagcaggtacgtggttcagaggtatctgacctactgaaagacgatgtggagtttaccactgaaaccccactgttctatttagagaacaatgaggccaaatccaacgggcaactgggtgatttcaccttttacccgtggctgtcagatgatgaacgtctgcatggtgtcgttgttcgcaacggcatcgaacgtaacatggctgtgaaacgtggtgctgttcatgttgatgagtatttccgtcaacgctttatggatgttgtgctctctcctgagtacaagaaatacatgactaagcagcgtcagcgtgcagtttctgatgaccactacattcactctgtggatctgaagttattgcgtttgcttggtgttactctgcccggttatggaaaattattccacaatccgaagtttgagaaacactttgaacttctggactcgtacagcccgaaagcagcacatgctcgtggcgaaatctctgccgaactctgtgacaagctcactgatgaggtgaagaagtacaagctggaacaattgccattcatccgtaaggtgaaggcaatgaagactgacgacttgctgcgtcagattggcagtcctgaacgtattatcaaatacatgaaggctatgccggagcgaaaagctgctcttaaatccctcgttcttagcgcgcttaaaacaggaaactgatctcatgaacaaagtgtttatcactatcgtggcactgtccattgatacgcaatatgccaccctctacaaagaggatggtaataccgtgatgattaagcaaggcgatcctcgcctgcctaacatcgtggcaacagccaaaggcccactgtctcgtaatgagccagtggaagtcgatattaccgaaatcttcgcccagcgtactgagtatgcagaagcagagaaaggtactggtggtctggtcaagttcttccgcgtagctaaaaagttcgtggaaaagctggtcaacaccgaatcgccaacggctgttgctcccgaagcagagcacatcaccccactgaccctcggtatccttcctggttccgatgtatcgccagtggcagaagtaaaggtggaagacaccattgctactgctgtaggcaccaagtggaaagtctggattacgggataccctctgggtattaaccgtgtacagctgatcaaagctctgcgtgcctgtactgattccggtctgaaagaagctaaggatatgtcagagcaacctctgccgtatctgctggctgaagatctgactgagatgcagtctgtggttcgtcgctctctcctggaagaggttgatggtctgaagttcaaggtgttaaccatgaacgaagccgatcctttaaaggatgagtcggacacggtgcctgcaccttcgccggaaccagaaaagaaagttgagccgcaaccgcagaccaatgcggaaaaggtgtcggctgctcaggccaaaatggatctgctggtaggcaacggtgctgtaagcactgagcaagaagcattccataagccactggatgagaaagaggaaactattgtcgccgtcaacacacagacgggtgcagtgattcccgatgctcagaaactggcaccacacctgaaagctgcgagtgagctgaaggactacgtaggctttaaggcgttcttcgaacgtctgtcggctgtcgtggacaaacgtggtcactcggtagaagacctgatgaagtttcttcaccaggccgatctgccactggctgatgatggctgcatcatcggcttcaaacgcctggatggtaaaaacggtgcattcgtggactgtcataccaaaaaggttcttcagaaagtgggttctttcgtcttcatgcgtcacggtctggtcgatccaaaccgccgtcaagactgttccaacggtctgcacattgctgctaagagctacctgcgtagcttcagtggtagtgtgatggtcatggtgaaaatcaacccggaagacgtgtttgctgtgcctcagtacagccataacaaaatgcgtgttgcgggctatcacatcgtggctgagttgccgaaagacctggctgctttaatcacgagcggtggcaacctgagtgataaaccactcggtgccaaagttctgaacaacgtcatgcgtggcaaccatatcggtatcacgcagactgttgaaatcggtggtcagcagggtagtaacctgacgatcctggaacagcagacagagttcaccaacccacgcatggtgttcgacgaaactgagatcactaacaaagtgatcccggtcggtgcggatattctgccggaagaactggaacagccaaaagctgcaccagtagttgcaaccgatgttaaacctgtggatcaagaagaaatgtcacagaaagagtttgtgcgtaatcacttcgtctcgctgtctaaattgacgcctaatgacgctcacaaggtagcagtcgagctgatggctctgaaaacccgcactggtaaatcatggcatggcctcggcctgactgatgaacaggcgagtcagatccatacgtacatccagactgctgaagacaaacaggcaccgaaggcaactgttgccaagccgaagaaagccaaagtgaaagctaaggccaaatctgctaaggcaccaaaagcaaataaacctgctgttgcgtctcgtcctgctggttcttctcctcgtgccatcatccgtgctgctatcgacaatggtattgctcagaacgttgagcagatcctgttggcgaagaagcaggcgaagaaaggctgggctgcactcggtgttaccgaagcagaacaggcggaaatcgaaaaacacagcaagtaattgctgacttccaggatacctctagccataataggctagaggtattttttatgagaggtcacaaaatgtccaaagtattccgtgcaaatcgcaaagcgtctgatgatgacattattcgtatgaatagtgttggcttatcgctgtccaccattgctcatgctcttggtgttcatccgactacaatcactcttcgcctgaaagctcttggtatcgatcctgctgatacccgaagaactttcatggaagatatttttgttacgctctctgagcctcaacaggaatggttagccgatcaactcggcccaagcataacgattaagtcgtttgtgaaaaaccttctggtggaggcatacattaaccgcaagtgaggaattgatggatacattacgcgacacggtacgctggtttaatgctgctgtaccggagccaaccattcagaatgtgaatgctcaaacgggtgttcactttgaagaagtggcagaaatgctggaacaaatggtcggcaccacgccagaaacctatcgcctgatccaggaagcagaagcagccctgaagtcactggctaaagcactgaaagccaatggcgatcatctgctgtttgaagtcactgataacgtgctgatgctggatgctctgtgtgatcagattgtcacagcaactggcacaggctacatgctgggctatctcatggtgtctgggatgcaggaagtaaaccgttccaacttctccaagttccaggacggtgttccagtattcgaccagaacaagaaaattgtgaaaggtctggaatacttccgtgctgacctggcaccattcgctgctgcacctcgcttctaataacaggccatcgtaaggtggcctttccttttggagaaagtcatgtctgatgattttttcgatgagctattcgcagaacctgcgaaagtgaaacgattacctctgaaccagggacaacaggccgctgccgatggcttctttgcattcctcatgggaactgataaagagctaaatatcagtggccctggtggggtcggtaagaccttcctgatggggcacttgatcgatgagatcatgcctcagtattacgatacttgtaaactcatgggcatcaagcctgagtacaacgaggtcgtgatgactgctacaacgaacaaggctgctgaagtgttgtcactcaacactggtcgccccgcttcgactatccactctttcctcggcctgagagttcaggacgattatgagagtgggcgtagtaagctcaccaaaacgaagaactggacagttcatcggaataaaatcatcttcatagatgaatgttccatgattgatactccactgcgaaagatgattctggaaggtactcattcctgcaaaattatctacgttggggatcactgtcagttggctccagtaatggaggtcatatctcctatctaccgttccaacctgccgttcttcgaactgactgagccgatgcgaactgacaagcctgaactgctggcactgaatcttcagttacgccaaacagttgagacaggtgagttcaaaccaattcagattgtgcctggcattatcgatcaccttaacggtgagcagatgcaagcactggtagatgatctgtttattcagacagaatcgtcatcccgtctgctggcctacacgaataaaaccgttgtgaattacaacgactatatccgtgaactgcgtggcctgcctgctaagtacacagtaggtgaaatcctcgtgaacaactctgctgttcaggtaggcaaaggcatgatctctgtggaacaggaagtgactattgttgagcttgctgacaccacagaaatggtactgattgaaccaagagagaaagtctatctcgaaatcattcgtgccaatctggaaaccagcctgggtgaagttatggtgggtgtgcctctgccagttgaccgtgatcaccacactgcgttggtgaagtattacggcaagtgcaaagagtggactccttacttccacctgaaaaatacctaccccgatctacgtcctcgtgattcgtgtacggtacacaagtctcagggttccagttacgacatcagcctgattgatctggatgatctaagtagctgccgtaacccagacctggctgctcgcctgctttatgtcggtatcagccgtgcccgtcatcgtgtcgtcttctacggcgatttagtcgagaaatacggtggcctcattcattaggaggcatcatgctggacaaaactgtcattatgaaggcagtgtcaagtctctgtgagccggagactcgtcgccttcagaatgtgatcgacaagctggtagcccagaatcaggagattgttcagactaatgatcaaggcttcatgtttcagggcgatttgtactatcgcagtaatgcaaacatgcactcacgactcccggctttagcctggtcattgtgccctcagatggatgttcacctgaaagacagacgactgttcgatcaggagtttgccatgatccggcagatggttactcgtctactgtacctgtgcaacacactccagaagcaacgtgatgcgttgcctgattgtattgtcaatctggttcctgaacttcaagccatagagcgtgttcgctcggtggaagaggtgatcggaaatgatgaaaggttgctccgtcagtaccacaaagcactcccactcatggaagtgtattccgtgagcaggatgttcttttagggggttacatgcgtcactgcatatttgctgaaccaaaagaaaaatatccggtggttatcctctctggttcgctccatcgggaaaatatggctgatgcctatatcaaaccgtttgggctaaacgaagaggattttctggctatcgatctgcatcaggcagaaggtaaaaagaaaacgcctatggctgagatgcgtcagtatatcagcgaagagttagtgcctatcttcaaagaggcagagacacagtatgtgatctgtaccgatgcggagtatttcaaggcattgactaaagctgctaaagctgaggccagtctcggttatgttatggatactgaatacggtataaaggctttatatgccccaagctaccgtcagatattctacgacccggcgaaagtaaaaagtaaaatcagtcaggctattatggccttgattgatcatgccagtggtgaatatgaagaacctgggcaaagtattattaagttcgaggagtatccgcttacagaacgtgaaattaagcagtggcttgataaacttctggagatggatcgagacttggctattgatattgaagcctttgatctgaaacaccacaaagctggtattggaaccattacctttgcatggagtaaacacgaaggtattgcattcccggttgattacaagcctatccccggtgctgttaaagctccgttcggtgagcaagtgaaaaaccatgcagtacgtaagatgctcaaagagttctttattgcatacctgcgtaaaggcgtatatcacaatattgcctatgacgtatatgtcctgatttatcagttatttatgactgatattctggacacgaaaggtctgctgaatggtatggacattatgttacgtaattgggatgacacgaagctaattagctatctggcaaccaattcatgtgctggcaataaactgagcctgaaagatcaggcacaggaatatgctggtgactatgccaaagaagatattaaggacatctgcaagattcctctcaatgagctattgcgatacaacctcgtggacggtctttcaacatggtacgttcatgagaagcactataaaacgatggtggctgatcagcaggaagatatttatctgcggatattcaaaccagccattctggatattatccagatgcagttaactggaatgccaattaaccgcactcgtgtgcttgaagtggagaaaatcttaacgaaagacaaagatgactccgtagccaggatggaagcccttcctctggttcagaaatttaagtatgaattggtggaacgtgtaacgaataagatgaacgctaagtggaaaacgaagcgtatgacaatacaggaagtaatgacctgtgatgtcaaagccattcaaaaggccatcgagttcaacccgaatagcgatcagcagttgcagcagttcctgtttaaggatctgggcctgcctgtactcagcaagactgactcaggccagccaagcactgatggcgacacgctgaaggcattgaagaaccacactgacaatccagagatcctcgaatttctggctgcgttaatggacttcaaggatgtgataatcatcctgtctacattcgtgcctgccatgaaacgtgctgccagaggtaacgatggctggcactacatgttcggtaacttcaacctgggtggtacggtgtctggtcgcttgtcgtccagcaaaccgaatctccagaacatcccggcaaactctcgttatgcgaagctgattaaatcctgcttcgaagccccaccgggctggatctttgcaggactggactttgcctctttagaggacagaatttcagccctgacaaccaaggatccagagaagctgaaagtctatacggacggttatgacggtcactgtctgcgagcatatgcctactttggcgaagctatgccagatattgatcctaactcagtggactcgatcaactcgattgagaagctgtataaaccattccgtcaggactctaaggcaccaacctttgcactgacctatcagggcactcaccgtactctgatgaccaactgtggtttctcacaagagaaagccatgacggttgagcagcgttatcttgatctctataaggtgagcgttgagtgggttaacggaaagctggatcaggcagcgaaagatggttatgtcactgtcgcctttgggttgcgtgtacgtacaccattgctgcatcaagttgttcgtaaaacccgcaagacgccacgagaagcagatgccgaagggcgtactgctggtaatgctttaggtcaaagctggtgcttacttaactcccgtgctgcatctgagttcatgggcaaggtacgagtttcccggttccgggaagatattcgaccgtgtgcccacattcatgatgcccagtattatctgatccgtgaggatttggatgctctggaatttaccaatgaacatctggttgaagccgttaactggcaaaatcacccagacattgcacatccagaagtgggattaggtggggaactttcagtgttcttcccaacttggtgtgaggaaacaaccataccaaatggagccaagaaagaagagattctgtctcttctggctgcttaataggctggatggtattatctatatggtaataccatcctcacctcttgggagcacttctaatgacaccagttactatcctatctcctggcattgatattcgcaatggagatgcaatgagtaaactgcctgctgtggcagttgttatctgcgatcctgtaacaggattaccaaccctgccgggtggaggcggtggatcaggtacggatttaactccggtactgacagccattgctgcactccaggcccagattaagatgccaacttactccagtgttactggtgtgagtgtggcgacaaacaccactggtgcaacgtggactgtcttcggctctaatgcgtgtgtcgcattcgatctggtcaacgacactggtgttgctatcgaatatcgccgtaacggtgctggcgtagctattactatccctgctggttcaagccgtttaatcacaggcatcactaacaccaaccagcttggtgttcgccgtgttgacgtagccaacactgctgtgactgtgaaaggggaggcattcgccgtatgatccgattccctttagggaatactcggtcgtttagttcacgcagttccttctctcgtggaggggctgctgacccagtgccagtattctcagctcaaccgcaaacccagtctctgtatcaagagaatggtctgctgactattacaggtgctgctgcatccccggcaacaggctatcagtggcaacgatcaactgatgggactacctggtcagatgttgcaggtcaaactgctgctgttctcagcatggctaatgccaccaatgctacagctacttatcgtctgaaagtggtgaatggtaattcagatcctgtgtattcagtctcagtggatgtggtttctgtttatctgcggattcagaatgatgcaagtgctggaaatggttcttctctgggtactaccaaagtcaccaatacaacgtatacccacagtgctgctggtggtactcgttactggtctgctttctatactcgcttcagcgatgacagtgcgtttacgccaaatggtctgagcactgctcgtgccgttgcatcgtggacaacaaccaatgctgctgttgttccagttactccggtatctgcaacaggtcaggtgacttctgttactaaaacaggatcagcgactattactgctgcaattggtaatctgtcatcttctctggcatgtaccattagttaaggcgattagatgagcatcctacagcacagcaagggggccacgtttaattacgtgtttgacatccccgatacgattggcaacggtttctttcgtaagtggaaagccactgcacagatccgtaaagcaaacaacaatcttccttctgggatgattgctcaactgcaatgctactggacgaacgaaagtacgaccaagcagcttgtgttatctcacgatcttactgacaattggcccgttggactcgcagaatttgatgttctgtttgagtcagtcgatgggcagtcgatgcgttcaagcatcatgccagttcaaattgtaagaggagtaacacagcgatgagcgacagcccattgactctaaacctggtaggtactatctaccaggggccaccaggcaacgatggcgatcctggtaaatcgtcatatgaatcgtatacagaaaccactacagacaatccggtactcagcgaagctgactggattaaatctctggtgggtaaaccaggtgagcctggtgattctgcctatatgtcttatgtgaagactaccagcgataacccagtgaaaactgagtctgcttgggtggcttcccttaaaggtaatcccggagactctattaaaggggatccagggaaatcaagctaccagtcctatctggataccaccagcgacaaccctaagctgactgaagctcaatgggtggaatcgttgcatggtgctgatggtaaagacggtactggtctgaacaaccgtcaaaactggcttactggcacaacctattcaccgggtgattacgtgtttgcggataacgcagacggtaacaactccatgtggatcctgtccggtactgaggattatgtttcgactattcagccgaaagatgatctgacccactggattgagttccaggctcctgctgggaacaacggtgttggcctggcctctctggtcatgacttatcaggcatcaacgtccggtacttccgttcctacgggcacttgggcgacgactattcctgccgtggctaaaggatcgttcctctggactcgcagcacttataccctgaccgatgacactatcgcttacggttacagtgcagcctatcagggtgcagatggaaccaatggaaataacggtcgaggtgtcagctctgcaacggtaacgtatcaggcttcaacctccggcactgttaccccaacaggaacgtgggcaactgccgtacctgctgtgaccaaaggccagttcatctggactcgtaccatcaccgcttacacggacgccgttaacccgacgacagcgtacagcgttgcctacttcggtacggatggttctgctggtgtgggtatcagttctgctgttaccacttatcaggtgggaaccagtggaacgactgcaccaaccggaacatggtcaactaccattccggctgtggctcagggttcattcctgtggactcgtactgtactgacactgaccgatgcctcaagcaacactgcttacagtgtggcgtaccaaggtgttgatggttctggtgggggtacaggtggtggcaccacttggttgaacggtacttccgatccaactggtacaacaggtgctgctggtaactactataacaacacctctacaggtgtggtttggtatcgtgccacgactacctgggctgctgtcggtgttttgctgccactggcatcaactgaacaggctcaggctgcaaccagtaatctgttgctgatgacacctgctcatgtgcgtgagtacatggaacagtatggtttcacctcaacgtatatgaatgtcacagctaacctgaacagtgttaccggaactaccgataagactgtctgtttcagcttcgacaacacaacgaccaattctccgggaaccggattatacggtcgtggtattcagttcgctggtggtggtaactacacaactcagcttgccattatcaatgatactggtgctatgtaccttcgatttaatagtggtggtacatggggttcatgggtatctattggtggtggctcagtaatgaaagcctctggcacaggccatgctgctggtttggctcctgatcctggtgcaactgctggtacaaccaagttcctctgtgaagatgctacctggaaagtacctgctggtggttctggcggtggtgggacaactgtctatgcaaccgttcagactgcacagaaaggcttgagcactgcctcagcaacaccactggcaatgacctttgggtctgctggcgtacctcctggtgacgcaactacggctgtcctgtatcgcatgacaggtactctgctcactcaagggccaacagacactgctgctgtattcagcatcaagtttactgggggtactgagggtgcaaacctgttccgtatgatcgtgagatctgccgatgcaacaggtgccattaaacaagtggcaagtaaccaggattcattggctgtcaatgctacgagctacggtgacagtatggtgtctatcgaaggtatcattcagatgaactatgtgaatccgactggtatcgacttgacctgtcagcttgtgtctggtgcatggacaaatatccttgcaggctcacacctgacgtttaccccattaggtaagctaatcagcgcgtaagttccttctttggttccaaggccacctacagggtggcctttttatttgggtaggactatgatagctaccccaacatatctttaacccatctggagagttcctgtgaacaaaccgaatcaaccatcccgtaagtaccatcatctcgttgtcggtaagatcatcttcgccctgctgaaagaaggccaaaccgaagaagacgaaaacctggacattcatgccatcgaactgaatgcagtgatcaccactgctgatggcaatgttggtgccaatgccctgggccgtgctcaacagtctctgcaaatgcaccacatgaagcgtgctggcgaaatggcacagtacatccgtgttcaggatgttgtagtgatcggtctgtccaacctcggtctgatgaccgatgaagagtttgcgtatatcccacctgcgatgaacgaagcacagaaactgtctgcgaacatcagcaatggcaacgtgactcaactgcgtggtaagaaagatgaccagtcagacccgttcgtcgagcagtgagtcgtctgggggccgggtaaattattacctggctgacatcacgcacccacagcgtgaagatcaacccccctacactgctgagtgtgaagacattatcgaccgactgggtatgacgtttgatgaggccaatatctttaaagaaatctggcgtacagcaaacgaacgtaccaacggtctgggcaaagcaggcaatacgccattacgctctgctcagaaactggttcactatgccgggcgtattcttcgcaaggcacaacgcagttaaccccgttagctactatcagtctttgattggcagtagctaactgttgttaactgaggagatctcccttgaaaatcaccaatactggaaacatcccactggccctgggtgtctggttattgcatgacgagtacgattatcaaagcatggcaaactacatcagtgcgactcgcctgatgaagcctttgcgtgccctgattcttgctgctcgtgtgccaccagatcaacaggtgtcagacctggaggattacatctccagagcctatggtcactcgcttcacgattccattgagaaagcgtggacgaatgataaggcacgtaataacggcctgcgacaactgggctacccggaacacgtcattgaacgtattctggtcaaccctaccaaagaacagcttgctgcgaagcccgatgccattccggtttatctggaacagcgttgcttcaagaaagtggtcatcatgggtgtggaatacaccatcggtggcaagttcgatatggtggctgaaggtatcgtacacgacaacaaatcgaccacagcttatgcctggttgtttggtggcaaagacgatgactatcagcttcagggcagtatctaccgttggttggaaccagagaagataacggaggatttcatccgtattaacttcctgttcactgactggcagaagctgcaagcccgtaccaaccctgcttatcctcagaaacgtgtcgagttcaaagacattcgcctgaaagatattcgggacacggatagctgggtgagaaacaaaatcaccatgttcgagaagtataaaaactccccggacgaagagatccctgagtgtaccccagaagaattgtggatgtctgaacctgtctacaagtattattctgacccgtccaaaaccactggtaaatccaccaagaacttcaacgatcctggtgaagctaaccaatggtggcaggtagagaagggtggtaaaggtatcgttatcacaatcccaggcacaccaaagcgttgcgaatattgcgaagctgctccggtgtgcaaacaaaggctgaaatatttatgatcaatctggaaggtgtagcacaccacccagtgctggaggaactcgttgatgttctctgcaacaaaacgcagaacactgaccgtggtttcttccgcgtggagtgtgcgtattttctcggcaagatggcagcgtcccaacgtgtaaccatcatgacgaaagaccgtggagacatcccggttaacatttatgcactggccctggcaacgtcaggattcggtaaaggtcactcagtcaacatcgttgaaactgagttcatgaaaggctttaagaagcgtttcgtggaagagactctgccagtgatcgctgacaaatctctctgggatattgccaatgaccgtgccttacgcaatgcgtctgatccacaggaagagtatgacaaagttgagggtgagtttaagcgtgctggtgcttacccgttcacctttgactccggtacttcacctgccgttaaacaattacgccacaaattactgctggcgtcctgcggttccatcaatcttcagatcgatgagatcggctctaacttaatcaataacgtcgaagttctgacgcttttccttgaactttatgatcagggtatggttaagcagaagctgaccaaaaacactggcgaaagtcagcgtggtgaggaggttgacggtaagacaccaactaacatgttgctgttcggtacaccgagtaagctgcttgatggtgctcagaccgaagaccagttctatgatttcctggatacgggttatgctcgccgttgtctgtttgcctgggggcagactgaccgtaaagcgttcaacactctgacgcctgaagagatctatcagaacctgattcagccgaccaacaatgctgccctgagcaagtggagcaatcacttccacaagctcgctgatccaggcaattatggctggaaaatcgtagtcgaagatgacgtggcaattcagttgctgacgtataagatcgaatgcgaaaaggctgctgaactgttgggcgatcacgaagaaattcgtaaagctgaactgtctcaccgttacttcaaagctctgaaactggctggtgcttacgcctttattgacgaaagcaacgagattgagatgtcacatctgatgtctgcaatcctgttggttgaagaatctggtgctgcattccagaccatcctgaaccgtgaaaaagcctatgttaagttggcaaaatacatggctgcggtggataccgaagtaactcatgccgatctgctggaagcattaccgttctacaaatcaggcatggctgctcgtaatgagatgatcagtctggcaacagcctggggctataaaaagcacatcatcatcaagaagtcgttcgtcgatgggattgagttcttcaaagcggaaacgctgaaagagactgatcttaatgagatgacagtcagttattcggatcactgggcatacaactttgttgccgagaaagtaccgtttgaccagcttcatcttctggttcaggccgaaggtatgcactgggctaaccatgcgtacaaaaagaatcaccgtgctgaagagaacgtgattccaggctttaacctgctggcgattgatgtcgatggcactgccaacctgcacacggttatggatctcatgaaggaatacaagttcctggtttatacaaccaagagccatgatcccgatggtgaacaccacttccgtttaatcctgccgatcaactatacgttggaactggatgccgatgaatacaaagagttcatggcaaacatcgttagctggattccgtttaagacggatgaagaagcgaaccagagaagcaggaaatggggcagtcactttgcaggtgagttccattacaacttggatggtgaagtgctggatgttctgcgtttcattccgaagacttcgaagaacgagcaataccgtaaagagttccaggcagttgaatctatggacaacctggagcgttggtttgctggtcgtatcgctatgggcaaccgtaataaccagatgatcaagtatgccttggcactggttgatagtggtatggatcttatgtcagtacagaatcaggtactggcctttaactccaaactgtctaacggtctggatgctgaagagatcaacagtaccattatgcgtactgtggcccaacgttatcaaagtcgttaactgaaggtcagccctttctttggttagggctgacactggagaaaattgtaatgagccagaacaaaaaaatcgtcatgatcatgggcaagccaaacacagggaaatctacctctctgcgtaaccttgctcaggaaagcatgatttacctcaacgccgatctgaaagacattcctttccgtgaacgtttcatggctaacgtcgagattgcaactgcaactgacgtgctgggttatgtcgaagagatcgagcaaaacgctgatgtgacgggtgcggtactggataccatcaccttcctgatgcagatgtacgagcgtcaattcgtcgcaccatacgccgggactaagactggtcagtctgcgtggggggattacggtaacttctatcgtaacctcatccatgccattaaagcaggctccaagagctatgcgattctggcacacgaagacgaaagtctgaacgagcaatccgcaatgatggaaagccgtgttccgattaaaggtgctgtcggtaaagtcggtgttgaagctgacttcaccacgatcttgaaaaccatgcagattcccatcaagaagctggaaggtcatgaaaatgatctcctgcacatcactgatgcggaacgtgaagatggtgtgaagtatgtcttcaccactcgcgtatccaaagagactgctggtggcaagatgcgttcagcaatggatctctggtcacgtaacgaactgtatatcgacaacgatttgcagcaagtgtttgaccgtttagatcagtattacggcaagtaagccaccccacaagctctacacgatgatgactgtagagaaaacttaatgatgaaccaaaagagaaaatattatgagcttgtttagcaaactgaccaccgatggtatcgaagaacaaactgaccgtctgggtggtggcttttccgcactcgaccacaacatctattctggcaagctgaaggcattgtatgccatcactgctgcttcaggtgcgatgggtgtcgtaattctgtttgaacacgctggtggtgagtaccgtgaaaccgtgtacgttaccaacaagaaaggcgaaaacttctacgtcaaagacggcaagaagcagcctctgccaggctttaccacggtcaacaacatctgtgtgatcgccactggtaagcctctgtccgagcaggatattgaagacaaagtgttcaatatctatgacaaggaagcacagaaagagctgcctaagtctgtgccgaccctggtcgaaactatgggccaggaaatctccttcggcatcctgaagtatctggaagacaaaacgaagctggaaggtaacgcctatgtgcctactggtgaaactcgtgacaccaaccagatcaacgccgtgttccataccgaaacgcactcgaccctgctggaagctgagaagtctcaggatccagagttctgggacaagtggctggagaagtatgtcggtgctccagcaatcgacaaaaccactaaaggcggttctgctgctggtggtaaacctgctggcggtgctccgcaagctgcggctggtcaggctgctgcacgcccatctctcttcaacaagaagtaagagatgcagatccccgttgccgggtttgaccccagcttaaatagctggggcattgccgaaggcatgttggatctggaacagggctatctcaacgatctggttctgcaaaccgtggaaccagaaaagaaacaaggcaagcaggtacgacagaacagcgtcgatattcagcgtgctgaagaccttgcaaccacggcaattatggttgccagacgtagcaaggttgttttcgttgagtgtcctgttggctcccaatcagccaatggcatgaaagcctacggtattgtggttggtgtgctaggggcaatacgatcactgggtattccggtcatcgaagttactgctatggaatccaaaaagattttcactggtgacaaaaatgccaccaagcagaagatgatcgatgcagcagtgaagctgtaccccgatgctaatttccccatgtatcgtgggcaagtagctgtaaaagctgaacacgttgctgatgctatagcagctattcatgctggggtgcagaccccagtatttcaaaatttaatgcgtttattcgctgaggttaaatagtcatgcaggtaactctgaaccaacaagaaatcgaaaccgctctgaaaacctacatcaacgatcagatcaccatcaaagatggtatggaaatcaccatcgatctgaaagctggtcgtggcccggaaggtttctctgcgaacatcgacatcgctccaccgaaaactccggtgaaaggtcaggctgctgctgctaaaccagctgctgctgccacacctaagcctgttgcaaagcaggaaccaaagccagaaacccagaccaacaccactgttgtagctggatctgcgaccaatgctggtgacgctcaaccggaagtacagccggaagtaaatgagcaggaacagcaggctgaacaacaagccgaagctgaagctcagactgagcagcaggtcaaaactcaggaagaagaagtacaggctgaaaccaagcctcgtgcttctctgttcggtggtctgaaaaagccaactaactaatggctgggatgaggatccttattgtagggatcctcattgtgattgctttcctggctatctctacagcagtgatcgcaatggctccctacattgccgttggtgtcatcgtcgttgtggctctgttcgcaatgttcggtggcaaggaagaaaagcccccagagtaacgggggcattttcttgggcttctttaaaccaatttcatcattcccggatttaaaaggcgagaggcccaagcaaatgtttcttgaaccagaagaagaggacgagattgtccagtccggcatcatgctgttcgacgctcatgtcagactaatgtgtcctgactgtgggattgtgagtaacaatcatctgtgctctgccccattcttttaccagtacaagcacagcccgttcatcaatccccagtttgtctgccaccatacctgtcaccgttgtggttacaaggatgacgtgggttcaggcttcactgactcaggtaattatgagtgtgacgaaactcgtgatctgaataagtgggaagaagaattatcagaccttgaggatgagatagctgaactcaaggaaaagattgccaggggcaaacgccgttgggaaatgctttggcaagttgatactgatgaaacttagtgttgactagcaacattagtttgaagtatcttctcttcatcgagactctgtagttcagtcggtagaacggtagactgttaatctatgtgtcgcaggttcaagtcctgccagagtcgccaaatttataggactatagttcagcggtagaatcctcccctgtcacgggagtggtcacgggttcgaatcccgttagtcctgccatataattggggtttagttcagttggtagaacaccgggctttgatcccgtatgtcgcacgttcgaatcgtgcaacccctgccaaattgcgtcatagctcagttggtagagcgcacccctgataagggtgaggtcactggttcaagcccagttgatgcaaccagtttcagagtgtatgacgctacagtagtgatcacgtcaccgagccgctacacgggacactctggatcaattccgattcgctaccggaagacctgccagaagacactggcattgaagcgacgagacatcccttcgggggtaaggtgcgtggatagatcaaatgttcgattgggtgagaggcccatcctcattcgggggattagtcaagcggtcgaagacggcagactgtaaatctgttataccacacggtagttcgaatctaccatcccccaccacatttggaagattggcagagcggtaatgcagctccctgctaaggagtacaaccgaaaggttgcagaggttcgattcctctatcttccgccatattggaaagttggccgagttggtttaaggcagcagtcttgaaaactgccgggtgtaacagctccctgggttcgaatcccagactttccgccaaattcattgccatctctccagagcgtgatgatctatgagaagaacacgagggcgacaatcaatcgcatcacaaacctctatacttctcagcctgcctcgttgaccgcgttaaggttactaaagcctccttcgggaggctttttttattaacctgaatcaagagaacttctttaaataacacttcgtaacgtctgtttacgtaatcttgcataccgttagaggtatgatagaggtgcgcaaattgatgagagatctcttatgaaattaccatcgtggctttcaaagatggtctttgaagtcgaagaagtccttcaccctgaaccaaaagaggaaacgcctgtgtctcaagaagaagtagcaactgctccggttgttgcaccagtagcggtcgagcctgttccggcaccactggtcactgatgtcgatctgttgatcgcaactctgaaagctggcctgattaccttcgggtacagcatcccagagtttgatactctggcagcagcctcaaagatcaaagcaacgcagtaaaaaagaaagccctcgaaagagggcttttttaattggttagtgagcgaggttaacccaagggttaaggaacggagcatggaatgcttgtcccataccgactgagtaattcagtccaccgtctgccatctgagtgatcaggttatcggtgatagggctaccgatgttcccgaacatatccggcagtggcaggttcgctgctaacagagcatgtaccgggttgtttcggatagtggacaatgccaccttcacggaacgaaccttatagttatagaaccagagtagcccagtcttctccatgtatccacggaaacgacctggcagtcgatcatagttcacaaactcttcggtcacagcagccagtccatttgccacaggcttcttctggcgacgaacaatgtcgtcatacagaatggccttcgccacaaagtcaccgtattccactgacttctccagtgccttgaacaaggcagtgtctttcgttaccagagcgtaacgaccagccgtttgcagcgacttaggcagcttatccacttgctgctccatgaagctgttgatacggcctgaagtcagttcaatggtgtcacccactgaggcatcatggatagctgagaactcaccagcttccaacagaggccagattgacatacggcgatagctgtcctggaatccctgaatcttggattgcagtcggcgttgttcccttggatcattctccgctgcacgcaggtcggcttctgcctcaacttcgagagcacgagtcttcacataagtgttgatctcagccagcttacgtggaacaccacgcaccacatctttcattggcacaccacgaccaaccaactgcaatacgttggctacggcgttagcgaatggaacaatcactgacttaacgatgatcagggtacgtgcatcctgaacaaagttttgcagcattgactcagccttggtgaagttgcgatacgcttcggcaccaaagatacccattgccacacgcttggctgtagagagagtctcaggactccagcgagcattgccagtccatgcgtcaccgatggttgcctcacgataaccgaaggtatcattcagcagatccttacggacgtagaagccatcaccaaacactgactgtgcatagtcacgtacttctttcggcatcagtttcacagcatcagccagtaccggatcaaggttgtctgccagcacgttgacatactctgcctctttagaaggcgtacctttagtctcgttctggtacatgtcatgtagagtatcgatcagcactttgttgtactcagcacctttgatctcttcaacctgacgaccacgccacacaccgatcatcttagcaaggtgatcggatgggctggtcttggcctgaatgttccgatccagagaacgctcatacgccacaacctgaccacggtcatcgtacactggcagcaggttttggcctgtctcaccagctttcagacgagcagtgattgatttcacagtcgtgcgatcagtgatacgtccagccagagcatcctgagtgaaaccgtaattggtatccacaccgttacctgtctggcgaacgttctgcatcaaaccctggttgaacatagtgcgagactggacgttaccgaagtaatagccacgtttcactttacctggttcagcagagctaccctggtaatcaccaatacgcttcaggctcatgctctccagcttggcagattctgagtcctcagcaacgatcagggtgacacccggatcacgcacttctggcacataacctttgtagccattgaacttggcacgagggttatcacgcagcttacgctgttcctcagcacgctgacctttcaggtaggacataacaaagtccataccagaggcttctttctgaaccagagagaagacggcatctttctgagcacgagtcagttgctcgatggcatacagagttgtcaggccatcaatatctttcaccatgtcagtggtagaagagtaagccttgtccgtctcaccgagcagacgaccaattgcctcagcattacgcagcaggtttttgcccggttcaccacccatcatgaagtgagccagttgctgtgctttcttcttgatcaggccagcgtgcatcttcgaggcattggcatcaatgcggttttcaaacgcagtgattttgccacgcagagtacgaccatcctgcatcagagagtggatctcatcagcattgaagtgctggaacagagagacaatatctgtcttcgcaagggcatggtgcattgctgaccactgatcatcagtcagttcagttgagaacttctgagcaataatgcccggcagtacgtcacggaactgttgacggtcttgctggatagcagtacggaaacgcttgataagatcgtagacatctttgttggttgaagtacgaccaacaatatcaccgataacatcacgcattgcctgcatacccggcaggttgttgatcacagtgctcacaccttctgccacgatacctgctttctcttcgctggcgattgctgcaaacatcttggttgcatcagccagtgcagtgatagttttgttgttggtacgtgccttcactttatcggcaccatcccacaaggtatcagacagagcagtcagaccatcggaaacaatctcgttggcacggtcaacaatgctacccagtgggccagcatactgatcgataaacgtctcacggttggcagcagtgtccatgatccgatcagtcagtgcatcaacagcagcacggacattctcagactgagtatcaccagccatacggcgaccgagtgagtccagcatgttagtgccgaatgcttcgatgttaccgtccagagtaccatttcctttctggttctccggcagaccaatgtcattcagcacagcacggaaaccatcgtcagtcattgccagagccaggaaagcaggcagcagagacgaacgacctttgctgtctttggtctggatgtaacgacccatgatgctgttgtacttctcagtcgcatcgtattcttcctgctgcgtccacggggcattcggcaagaagtggcctaagtccagcttatcgatcacatggtcatacagctcctgggcatagttcattgacgccggatcaatatgagcctgtgtcgccagagccgagacgatcatgctgaaggttgtagcctgttgcatgttcatcgggaagccgtggttcatgaacgaataggccacatcgttaccgttgatcagtgcctgagcagcttcggtctgacgtttggacttcactgacatatctggtgattcattgatatgtgcagtcacgacagcatcaaaggtcttgttcagttcttccagacggtcactgttgccgtacacacgagactggtacagcttagtgtcaccagagacgttctgtacgctcgcctgaccacgcacgatcacaccagtatggaacatcaggtttgacagaatatcgtcgcctggtgtcgctgggatgcgtttacgaccatatacaatcttacggatcgcattgaacacagcatcagtaatctgtttcaggattggggttttttccaataccttgttcagagaacctgtagccagtgaccaagccatgaactcattcagtgctccagcctgacgttgtgcttcggatacatcaccattggttgtccaaccattgatagcagccttggcattctcgtaatcggtacgagttttcggatccagagagaaagcatccaaattcataaactgtcccatcatcccctcaatggcagacactgactgagtaatctcaggggtggtgttgccttgatagtgatcaagcacagtctcgaaagtggaggcgtgaaccatctcatgcagcagcgtttgagcagttgcattgttgatgtagatctctttagtagacggtgaaatgaaaccgtcattcgccagattggtgaactcgttagccggatgagtgttaccgttggcttcattatatgccagcagttcttcacggctaccagtgatgatcttgtaacctttggcagcagcagaacgacgaatctcgtcgaacattgctttcttaacgccagtcagttccagagatttcaccagaccattcagcttgttcattgagatgacacgagccttggaaccaggagaagaaacgccaactgtggttgctggtttaccttcctgtttcaccggagcttctgctaccacacctttcatgttctggctatagacctgattcattcgggccacggcctgagcaggatcgttaggcagttgctcaccaacgttttggtaagaagcagccattgatgccatctggtcaatatgcaggttgaactgacgcagagttttatgacgagcatcaatcgacttgctggtagtagccatacggtcagcaatattcttcagctcactgatcacttcgtctttggtggtaagcatgtcacgatcaccagtcagagcacgagacatctgcttaaccatctccggtgtcatgtccactgcatcggcattcttcagactggtattcagtgacttcagcacagcatccactgggttctggttccatgattcgaacacagcaccattcagtttcaggctgtcacgagacagacgatcaatcggcaggttcacaccatcgaacactggcagagcacgcttaacactgtcacgaccagtaaagccaacctgaatcatacgagcatcgcccataccaatgttcaggtatgcagcaccagctacgccggaatcctgtgggccatacatggttgcagtgctacggtatgaaccgtcacgggcacgaccaatagaactgttggttgagtaaccgttattggcaccaccgataaagaacgtctgggcaccagtagagatcatcgggaacgtctcagtaacagatttcaggatctggttctgagtgttttgtggcaacagataatgcttcttgtagttgctgtctgctgctaatgccagctcctgttcttcaaccactgcctgacggaaagcattctcctggaagatggagattgcctgagtcgcctgacgaatatcggtcatgttctgcataacagaactgccaacagtcttggtgattgagtcagtcatcggacgaataaacagtgagttcacattcatacggatggcattacgttcttcagtcgagaaagtaaatgcctgtgctgatgagaaatcaccagacgcagtttttacttcctgagtgaaatactgattacgtttacgatcccaacgggcttcagttgtagtcagatctctgatgtactgttgcaagttatcaaactgctgctgaccattctcaccgaacattgctttagcaaagctcagagaaggatcattggcctgtgcttgagcagcctcagacatcttggcatagatctcgttcacgatagcatcagtgatattcccggcaataccgaaggcacttgaaccatagacagtaattgtcagagggttcttggtaacaccacggtcaatgttcaggttgccctgatcgtccagaacagcacctggcaggaacatgttcatcagaccttgcagactgttcaactgtactgccacatctggcttgccttgcaggttctttttcaggctgttaaggccagtagtcagatcagtacccgttgcaccatacaggtcagtcttatcctgttgacggtaagtgttcagggtagtgtgctcagaaccaaagaagaggccagtacgttgcgagttcacataatagtcagtggtgaatccaccagatgacagcatctgcgttgcgttggcaataccgttggtcacaccatcagcctcgacatacatcggggtgttgaaagtgttgtttccttcctggttcaagaagcgagcatactcactgactgcttgcagagcgacaggggaatccacaccagcattacgcagtgtttccacacctgaatcaggcagagcatcagtgctgtggaactcctgcataacagcaatggcaggagccagtttaccgttcagcagtttgttcagcagttccactgaatcagtatgaggcatgttgtggatcttgatacccaatgcctgagcaaggccaaggtcaaagcccatacgttgatcagcatcagccatatccacagtggtgtgggttggcagaacagcttcacgcatcagcttactggcttgtgggttgtaacgacccagcatctgcaaacggtttacacgagagaagttgtagccgtagaagatgtcagtctgaccaatatcaccatcttcatcgaccaaacggttattgagatccatctgcaatttagtcagctcgtcaaacgcattggtgtaggaggcattacggccctctttacctttcttatcgttgacgttcagagccttgctttccagatcaccttcaccgaacaaatcacgaacaccgtcacgaccaatgaagttcagcaggctgaccattggcatgtgtaaacggtacggagtgttctgcacgtttttcagaacagcgatttgctcaggggtgttacgcacctctgcattacgcatctgagtacgggcaatcggaggacgctcatcacctgtgtaacgtttctcttctggctcaaccagcacagcgtcatcaatcgcagacggatactgcatcagcgtattagtgagttgtttgctgtcttcagtgtcatccagcttcagagcagtgaagtcgatcttacgtggctgtacgttaccctctgcatcagtaacggtgaagttctgggtagtggtttcaaccaggccagcttgctcaaatgcacgcatgatctctgaagcaattgaggcaggaatccctttgacgaaaccgtcaaagtcgttcttgttctcagatagaccccagtatttgctgatcttatcagacagggtacggagtgattccgcagtagtcattgaggtgttaaaggcagtaaacatctcatcactgacttcacccggctcagtaagcaggatcttcgcaatgtcttccacatccaggtttgcaccttggttgtatgaagtcagtgcccactggataccagctaacacagcattctggatcagctcagggttatagcgaaccacaccattaggtagagtctcaacgatgttgaatgacttaccttccagtgatttatacgcagcagcattgtccggcaccaggtatggtttgccagatttgatctgtgctgcgatgtcgtcacgcaggattttattcaggttctgcacgatgcctttagcatattgcatcataccctgataagcagaagacacttctggagtcaggtgattactgctttctgaaccagagaaagaatgcaggtcttcatcacttgccagagcagagttcaatacagccagtgggttttctacaccctgggtacgtgaacgctgagtcttaggcagagtgaatgcagaatggaaatagttcttcccaccgtccggcacattcagtttgtcatatgcttctgtcacagttgttggagcagctttctgttctggttccacaactggcacagttgttgcttcctgcactggagcagactcagttttagcacgcagttcacttttcagaacataggaaggtttgccctgataagccacgacagaatatgtctgaccatcaggcccaacttcgtcctgaccacggtaagtcactggcagatcatgatctttatttgcccagatcacttcatcacctggagcaaattgagcatcagactgttctgcttgagtggtattatccgcttcgcttacagtttgtttaccctgcgtctgttgtgctggagtgtcttcagcagctacagtctgtacaggagctgtatcacttttgcctgccacacgaacaccatcgcggaagtcctgtgctgtttgtttggtagtgccttcagacaaacgagtatcgaggtttgtatggtcaatggaactaacacccaaatcactgaacgcctgagccaggccattcgctacgttcgtaacaaattgggcttcgccagctacacgacgagcaaacttcaccgaaccgggagaggttggggtgatcccgacagtatctttgccagtcgtcatcttccaggtgcggtcgggctggagttggagatagttgagtgcattattgccgttagggttcgcaacgtcagtaaggtgcgtgttaatagtggaaaccttaccgttcatatgtacggcaagttgcatcagatgatcaagagaatctctggccccgtcgagatcacccgcagcgtaagacgcataaatgcggcgagccataaccagaactgacggttgggctgaaccctcatcatcagcagccttcagagaatacgcagtcttgtctgacttagaccagccttcacgctgagattgttctgcgtactctctggcactttgaaccaaagaaatagcaacgttcagagcagcagactgatttttattcagtttgattgcaccatccttcgcttgttgcagaatgatcttcgcatcttctggattgatcttatctggggcaacagtcgccaatgccacatgggcatcaacgttatccataccttctggggtagcaatcgtatccgcatcaactggcttcacaatgtcataggtctgagcattgtttgccatgttatccattgcagcctgtgccttagacaagccttgtgacttctcaagagaagcgtgcagatcttcaatacctgtagcgaactggtatgcagggtgatctgctggcagattagccagtgcatctgaacctttagcaatctcatcacgagagccattgatgatcgctgacagaatagaacctgtcatgaaacgctcttgtggagagttcttctcatcgttgacgaatgcagccatcttctgcatagcttcgatttggttgcctgatccctctacggttttctgaacgtagtcaggagttccagcataatcatcagccacaaagtccagggaaccagaaagagtatcaagatactgattagtagcagccttttgctcaggagtaatatctgattgctcgactgctgcttttgctgcttccactttttctggtgcattatttgccacatcacgggctgtggtttccatgttcgcatcggagacaggagagctttcctgcatcttacggtaggcttcatcaccacgtttagccagccagtcaataccaggtttgacgacagacttaacctgatcggcagcagcttgtacggcagtgtttgcattccacaacagctcagagttcttcgcagcgtccacagcacggttgcccagtgcgtatgcagctttagcagcatcaactggagcacgtacagcagaagcagcaacagaacctgggccggaaacaacaccagttgaggtcagaccgaacagagcaccttgacccaattgctgaccaacaccttggctgatctctttgttaggcaaggcttcttgctgttctgcatagttggttgccagttggctggtagctgattgcacaccttcttccagagtctctttaccagagttctgaagcagagtacgaacgcctttagcagcaaacggattggcttcaaacttgctgaccagtgagccagttgcagcagcaacagggaactgaatagcagcagccagcagaccagaacggttggcgatctcagaacgtgcatcttcctggctcataccacctttaaccagttcattgaactgaggtgactgtttagccagttcatcaaatggcatctgagagatgtcagagtttgtctgttggtaagtaccaccagcttccatcaggccaattgagccaagaataggagcatgttcagcagcacccattgccaatgttgcagcagagcgagttccagcagcagtatccaatgcagcagccagtgctacaccacggcgagtagcctgtggaataacagccgatccaattgcacggagagctttagacattgggccagcagtcagaagggagccaacaccttgagccgtaccatcaagcaatgcagcaggattgctgagagtgttggagacagaatcaacagcaccacgaccaatgtttttaagacctgcaataagagatccatcatccttcacatcttgtttgtactgggcttcgttgtcacgctcagtgttggtattgagagcaccaaccagacgctgaccagcttgctgagagtcagatttgttggcgtttacattgtcgttgaattggttcagtgaattactaagagactgcccagcatcacgatcaataaggccagcaccgagggcaccaataccgacaacagagttaacaagaccttggcctacaccctgaataccgtcagtaattgtgttcacaccatcggtgttatgggcagcatttacatcggcagtgattgatcgagacgcttcggcctgaccagcagcgaactggttataagcatccacaccgtacttcaccatgtactgacctggtgaaaggttacgctgatcctgttcctgttgggatgcagaagcattaccaacaccgttcatctgaccgtacagagcattgtaattatcggcaggcgacatccccagatcctgtttcttctggttcgatgcgttagcgacttgtgcttgtttatcaggtgagactgaagcaaccgtactctgtacgatttgggagatacccgtaggggctggatcttgaggcgctgggctagaagcgtactgcgacagaatatcattaatagatgacattactgattcctttacgatatatgtttgaggtaatttacaccatgtggggccaaagaaaaagccctaccgttatgatagggcttttgattcagaaaagcacttaacctcgcagtctgccgtaagtatcgagcagttgctggttgaagttacccgttggagcagcaggctgatccgcaggctgtgctcgtgggcttcccgtagaggttgccaccggagcaggttgagcaactggcatcaggttagggttaggctgaccgttcaccaatggggcgttgttctggtttgtcagagacggcccaaccacctgtttaaagttcgccgttgcagcatccagagcagcctgataacgaggcaactgtgattgcagacccggctgagtcgggatacgacgaagcaggttattgtagttgttctgggcttgtaccagagcatcattggcctgcttacttgctgcaccctgtacttgcagatcacgctggttcatcagtgtttgctgagtagaaccggaacgttgcaactgaattgcattgttcagaccgtcatcattgatacggataccctgacccagatcaggtgtgctgtcatcattacgaaccagaccaccgagagtacgggcagcatggcctgcacgttggaagatgttattactgtcttccacgtttgactccagcatacgggcagcagtcgcaggggtaacaccagcttgctgcacaacacggtttactgtgttcagcaggtagccacggttagtacctttgaatgcacctttcaacaggctgtcagttgcatcactggctgaggtagaggtatcgccctgtgtttgcagaagcgtatccatccactgttgctgtgacgtgttctgaccagcacgaacagtacgctggttgttgtccagtgccagagctgttgcctgattctgttgagcagatacgggtacagtgcttggcagagaaccagattcgccaccagcaataagctgacgcatctgtgaccacggaacatctttataggcaccagcagtgctattgggcagtgaagtccagatcttagacaagtcaccgttcttattatcttcgaactgtgcctgagccaatttctcctgattctctggagtgaactggacattcttgtaatctgcaccaaacacttttgggccatagttatcaagagaactttgagtgatctggaatgctccagatgcagaagttcctttgtcagcacctgcaccaactttgccacgggtagcagggatcaggttgttcttaccgaaatcctgaacttcaccaatggtcatattggatggggctttatccggcgtaccataggcaccattgccgtataccatgtcgtatgggttagttgttgcaccacctacgccagcagccggagaactgtacacaccagggaattgctgacccagggaagaacgcagcagcatctgaccctgtggtgacagatttttcatggcaccttcagcaattgcacgagcaccatcattatcaccaggcaatacagacccagctacactgttcagtacctgagttacctggttctggtcattaataccaagctgacgctgattcagtgacagggcagcatcggcattcccaatactttttccttggttccccaatgcctgaccaatgttgtttaaacgttggcctgcaacatcaccaccagttttatacaggttggcttgttcttctggtgacagttgaccgagcacaccagcattttgctgaagcagacggttaacagcaccctgatcaccctgttgctgggcagtgtagatctgaccaataacattacgagcagcatcagtgttctgattctgagtctgggtacggtcgaaaccataaccaagaatgtcctgtttctgttggttcccagcattgttgatcaactggcctgaacgatcagccagagcacccaacgtctgagcagacacctgagaacggtcaataccattgagcaacgaaccatctgccaaagcagcttggtacgcagccggatctgaatattgaagtgagttcccaatggcagcagcatcggcacgttgttgctgggcttgtccaaatgctttcaggccatcactcaaggcacctgttgcattattcatgaactgcccagctacacgaagaccgtccagcgaaccagagaaagaaggagcatccacattacgccaagtaatctgggccatgattgttccttacagtttattcttattaacgtagtcggaagtctgagcatcagaccaaccttccacggaaccacgagcagcagcacgatcagaaagcgtagtgttatacgacttgatcgagttcgccagattggtatcagtaatctttttggtgtagtcgaactgtgagttcgccagcttgttagcctggaatgcaccatatagattaccaacggtactcaaaccggacagccccaactggaaggttggaatgttcatgcccagcgtatcaccaaatgaaccagtttgatcagcaccagtaagattggtgttgttcagtgctgtggcttgttgacctggctgatagttcaatgcactgttggggttgttggagaatgagaatccattaccaccagcagcagatacaccgttgttgcccatgatatttaggttagggttgttgtagccatagttcggcacaacaccactgttataaagacccatatcgctcatttaatcaccccggaaggtctgttgagatcataatatcagtgaagttggtaatcagtccgagagacagatttgcaatatcttcaccactcatcattgtacggctaaggaagctatcctgactttccaacatcatgttggtcgcttcagtaatcttcaggggatcaatgtaacctgttgagtcagtaccaaacatatcgttgtacttctcagcaatgtctttcatcttgtcctgataattatcaagaacttcctgagtctctttgatggtttcgtttacagcagcctgcatgtattgagcatagccattaccagcagcttctgtcagtcggatgatgttctctgctctggtaagggaagagaacccggctgaaatactaccaccgtttgcatatgaagtcccgacagccactgcaattacagaggctactgcaccaacgatggcaccgtacttctcaccaaacagagcagtggcagcaacaccgatcagcttcatcagcagcattgctgccagggcattggcaattgtacccacgatgattgctgccacacctgtcagacctacagcagcaccaaccgatgcagccgtacctaacagaccagcacctgccccggctcctgcaccagcagtaaagatcgagacgatgatgacaataaccaccagcactaccttgaaccaggaagtctgataccatttctgcttaacaacctgatagcagttgaacaccatgatgttacaggcagtagccatctgggttgcatccttcagagagaaggaagtcagaatgtcacgctgtactgggataatgaagcctgattcctcagagtcattaatcgcatctttaccatcagtatctactgacttcccaccgtagatcttgttgatatgccgtaaaccatatacgtgcatagcagaccatgctgtagctgagtcctgtttgtagataataatgtggttcactgagaacgagttactggcagacgttgagccattgaaaatgatctgctcatagttgtcatccgtaccaatttcaaaccagcaatcacccacattgtgagtgctgtctttcatacctgtgccaatggtctttgccagatttgaccagttgatgatcatgttgaagttcatcaggccattactcttcacctgcacaccttgtgtaggcaaagaaggataagacagtaccgaaggttgaggtgtgccatacagaggattacttggatccgactgtgcagcagaccatgcagcaaaagcctgattactggctgaagcagcagccattgcagtacggtaattggcataggccgggtcattacccaccgagtccaacaggttttcaaagaacgtgtatacgtacttacgacaggcattgtcttttacattgagtgagacaccaaatacgcagtaggcataatcaatgtcaccaatgctttcattgtctttcaccttatcgatcagttcagtgaactttgcccgaacagatttcttatacgctttctcgatcaacgggtagtaatcgtcaaaacgattatcgtcgatcatgtcgttatctattctgactgggatgaatggcaggaagccaccgactgaagcgttagctgcgaacatggcatccagggttgcgttaccagagccatatttgtagatgaagacattggacgatgacagagtgcttgtgacagtctgagtgtcaatgcgatacccacggctacgttcaacgctttgcgttttaatcgtggtcgttgtggttttgattgtaccatccggtaaagtctccgtgctcgttgtctcttctggatcattgtctacaacctggttggtttggtaatcataacggaatgagttctcagtggtactgacctgattggaaccagaagaagaggcaccctggaactctgatttatggtactggttgtcgataaccggaacagtttccacagtggtggattcagcatgggaggtttcatcaggacgaccatcactgtaagagataaccacatctgtctgttttaacaggttgtagtcagtgtttactgaagaagtgctgtccactgtccaaccatcagttgatgggaaaggatctgttgcacccagagatactggagtgccaggcaccagtgggccagtttcatccccagaagaaacaaaataggctgcatacagatactttgatgcagtgtcgtaatcagttggtgtaaacgtctcagacgtaccatctgcataattaatagtgatgatcccagtgctctcgttgtagtcactggcataatcagtattgagtaattcagggtggttctgaacaatatattggtcagcccaccaggtgtaatctgcaaggtcaatctctgccgactgaagtacagcagtagagccaggaggaacaggcagaaatggtttcagagattcatcatcaatggaatctccgagatacaacgtaccagattgcatacccagcatatcgttgtacccggagttcacagcccacttaccaaaacttctgagcttcaaacctgggccattcaagtaactattggtgattgcttcacccaatcctgttgaaggggaagtgtcagcaatgaccttacccaccacaacagtcttgagatagttcacacgatcttcgtcaccacctgccagattgtagacagatgatgatacgtaaatctttttcttagccttgaagaagcccattgtttttagcctagatcgttgttggtgataatggtttccataacagcattgatactgtcattggtgaacgcagttggagcagtcagaccttcatcaatggttttcattgctgtccacacatcagagaagatcttggcagcagaacgttcatcgttacgcaggtacgatgtgatctgttgagagtacagggctttctgcttaccaaccgaaccagccacagtctgaccatcggtacgggtgtccagagtctgagcacggtacgtttcagtctgttcagtgatcatcacaatctgacgaccaatcatcgcagtctgttgagtcaggttgctgtactgagcagggagcatctgagacaggttatacgcagcagtgctgtactgcacaccagccgtcttaatgttctgagtaaccaattcgttattcagatccagaccttctttctgagcaggcagcatggtagacaggttgtaaaccgcagtaccgtattgcactgattcagtacccagacgagctttggtcagagcatagcttgcaccctgattagcagcttccagacgagttgcagcaaactgcatcttggctgttgccagttgggtaatacctgtaatcgcagcaatctgtgcagcctgagcttgccagaacgcttggtctttaccgagcaggaactgagtcgcattctgtagagtagcctgcaccgagccaatataagccttggtatattcggcacccataatacgaccagcatcatactccatacgcaggtggcctttgactgctttcatcagcacatcaaacacaccagtaccgtccactgatccagaggtcaacatctctactgttacaggctcaatgtccttatacagcagtgagtcaggatcatatgggaattggtattgggggtcgtcaaggttgatgtcaggcagattaaagtcaaagtcagcagtcagtgctgtgtacactgcctgggcttctgtctcgacgttatatgtgctcatgataatcctcaaataaaaatggcccatctaagggccatcttgtttaccgtagtggttacatacccgctgctaactgagcagtcttcagatcctgaatctgtgcaggtgtcagtgggggcataacttccagagcaaactctctgacccaggtagtttctacacgggtagtcttggtacggcgatctttgatggtacgcacgttcaagaactgacgtgcttccagcatcttatagatgcagtacggcacatgataaccttcatcggttacttcgccaaatggaacaaacttacggacagtgccgagatgttcattggcaatagtgaagatttcaccaggcaggtcttttttctttggatccatacaggtgatacgcagacgcaccaaccgcatttgtttgtcatacagttgctgacgcagggatttggctttcgcaggtttcttaccagcagcgtcaccgtccagcggattgagttcaggagcctcagctttcttctctggttccagtgactttccttccattgcagcttcgatcatcttagacagcttttcggtagcaatgttgttggagaaagacaggcccatcatacgggcacggcccatcaaaagctgacggcgttgtttttccatctgttcggcgttttcattaacggtactctcgtcgttctgaccgttttcaagggtgctcattggcgtgtcctattaagttgttggtaataaaaaagggagcctttcggctcccctctaatataggttgcttattacagcggtgcaaccgttttgatctgagccagacgctcaggacgcttaaccaggataccgtagtaccacttgattgagctgaaaccagtctcaccgaacggatcgttacggtcagcagtttccagacctggcatcttggtcatgatggtgaagttcgcagtcttaccgttcgactggaagccgatagtggtaaacgcatcgtcaccaacaaccagcattgggtacacgttataacgctcagtaccagaagcgtcagttgaggtacggtagcccggattctcatcagtcgcttcagcaccagcagcagcccagtgcagcatttcaggaacctggatgatacggaacttgtcgatagaaccgacttcaccgttcatcagagtacccgcatcgccgtagtgctggatttcaatgaatgctttttcattgaacaggtcacgcagacctttcagcagtggcaccagctcagaaccaacgtacatcacacgggtcgcaccgatcactttggtgtcgatgaaacgagaaccagtgatgatagtggtactggttggagtacggttatcggtcaggatctgatccagacgcatgatgttctggtaggtcacaactgaagctggagtggtaacaccgccagtagttgattcttcaccagtgatctcatcgtcagaaaccgcagcacctgcatacaggattacaccagtagcagccagcaggtctttttgcagaacagcttcggtcaactggacagcaccagttaccagttcacgagccaggtgatctttcaggccatcgtcagagtcgaagtcgaatgactcttgggtgaactcatggaagaaaccgaacttgtgcagtgaaccttcacgctccagacgggtgaagccgacacggttaacacgaccaccgttctcagtcagcgttggcagacgagaggtgatagtaccgatgtcacggcttgagccgtacaggttgccgttcgcaatggttacgccattagcgtcaataccctggtcgttgatgttacggtcatccagaagaggcacgtattcgtacagcttcatggttttaccgtagttcttcggcatgttggtcacgttagccaacggcataaagaactgctctttacgagcggtgatgatcgctttcttcagccagaagaaagtattcatctggtcggagccagcaccatcaatgctagacttttgaccgtctgctggggcgttataattgagcatctatctatccttaacggttttcaaactgcttcatgaactcttcatccgaaacagcaaagttcggttgagctttggcaggtttacccccagtacgagtggatgccgcagcagccgcttgtgcagagttgtctacctgtggttttggttttgccgcacgcactgcaactggagcaggcttttcagcttcctgttgtggtactggattaaatgcacctgctgcttgcagtttatcgccaaccgcacggtaggcttgcaagaaaggtacactcgcaccaatctgaccaagagtacgcatgtgctcaatctcggctgtgattttctggtatacaccagattcacgttgagagtgaatcgtcgctgcgatttccgggttagtaaacaggagatctttactggcttgatcccatttagtgttgatctcgtggagcgtctcacgaccaccttcagatgatgctacatcatccaagacagccttaaacgcaacctgatcgtcactaacagtgtgattgccgttaggtgtgtaggtcgattttacatccgggtcgtgttcgtgaacatcgtaaccggagtcttcaatgagtttcttaatcgcctgcggatccttgttatggagatcaatcaggtaactaagttttgactcatcgagtaagcccacgttctcaagcatcaacccagctttacgatacggagctaagtcctgcattttacgagtgtagttcgcacccatttgcataagctggatggcttcggctgcatctttaggggcaaccatcttaccattggctttaaagggtttgagaatagtctcgtgaaacgctttgtagtcaatttcaccatcagcaggcttgttatccttctgggtctgagtttgttcagtattagtctgagtctctttaccagaagtagccgctgttggatcggtgttgtctactttgttgtcagcaactttagcatcctttacaggatctttgccagtattctgatcaacttcttcagtagactgttgttgttcaacagtagactcttcctcttctacatcagtctgctgaggctgaacaacttcttcttgctgagtttgttcctcttgggaaccagaagaaggaactgcggcctcagcaggtgcagaagggaatgagtccattgccaggatttcatcgtcggacatcttagagatgtccggctgggtttcagcagccggattttccattattcgtcaccttcttcttcttcaggactggcacgcagttcgtcgagttgcatctcgatgtctgggatagtgttgtgggcagtgttgccaatctgaacctgaatagacaagaagcgtttcaggtggcctgcggcctgagccattgccagagcatcagcacgttcagatgcagacagcattgggtcgccagattgacgggcataacgagcacactctttctcacagaatccttcgagaattaccttacggaactcacgattacctgagagtttgagaatcatatcacggtgctcgataaggagtcgtgaatcgctcaattgctgctcaagagcttcgatttgtgtcatgttttaactttcctcaaataccaatagaagggtttagggcaggatctcgctgtggctgaaactgagctgaaccaatgttttggctagggtttccggctgcaacgtctggcgtaatattagtttgagctggttggctctgtccagcattattcaagttatctccattagtgagtgcattgtaaccaatagcagcagtcacatctggcttagtctcagcaccatcaggtttcttctgagtcttgagcaatgctttggtaacttccagttgctgattaccttcggcctggcctttctgtttctccatgtcacgagcatgtttagtacctgattcctgctcaacaaagtcgaggttggttttatcagagttactacgtgcttgtgcagcaagagcctggttcttctcgatctcagattgcagtttctggttttccagttgttgctgttgaagctgcaattgctgcatctgttctttaaatggatcaggcttaggttgccaggtcagcagatagtgtgccagttctggcatacgtttcagcgtggcaatctcagacagcagacgagtggtaacagtcgggtcttccagtaccgggccgatagtctggatcatgaagcccagatcagaagatttctggtcatcaacttcagcagtggaaatgtccacttccagatcataattacctttcaggtcttcacggttaatcgtgacaaacttgtcattggtgacacggacaacttcagtctctgacaggaaggcagcattcatggcaatgatcttggtgccgatctctgtcatgccttttgccagacgacgaagaatagccatctcacgttttgatgcagcatccaatgcaccacggataccagcagcaacatcgccataggcattacccgatacgccaccagcaaaggctttcaccccggtaagggattctgcttcctggttctgcatctgcaatacctgcatagccgactgaggaatctcagggaacttatgctggatcatgttctgtgccgggttctgagcctggttaaactcgtagtctttaccgtcttcatacttcttacggttgaccggatcgagcatacctttggcaaagccctgttgagcattggctgaacgaccgagcagatcgatgatgccacgggtagtagcacccaggatcgcctggttatcttccaacagttctgcatccggttcaccgaacaggtcacgtttcttcggcagatatggaaccagaacaaaaggcagcttctcatccgggtatggattcaactccatacggatcattacatcaccaatccaggtggcaacaattggaacgagtgaaccatcatcgttgatgtcagcgtaaccccagtattcatacgccactactttggaacggagttcatcagcaaaggtgaagtcctgtggtgtggtagtggtgtaattggtctgggtagtcgggctgttattcttccagtcaacacgatccagattgctgtaacggtctgggtacttggacagttcagccttattggtttcgaatgccagaatgacgaatagtgctttgttcaaatcaccgttgcacgatgggtcaacgtagacgttgtttggatccaacacatcaatggttggctggttcacaacaatctgatcaacttccacctcttcggtgccagtctgcacagcaaccgttggttgttgggtttcatcgaagaactcaacagcagctttcagtgccggatcaccttcgttaaatccacgagggttttcttcacgtaactgcatagcctgctgaaaagccatcagtgcttgctgatcctgaatcgggtaatacgcccagacaggaacctgttgcttaacctttttggtttcacgcaaccagcccactttggtaatggacgtgccttcatcgaccacggaacgaacgtagtcatcgatcagcttcaccttgttcagcttggttctgaactgccagttaatcagtaactggttctgcactgcaccggatacatcttcgaacgacacaggtgtgacgttgaacattttattggtggacaggaacggttcagacaaggctgagtaacgccattcagcctgacggcgaatgagctttggctgtacgctggaacggcctttaaccttcttcggtttcacgctgttctggacattcatcagatcgttccaatgatcgatcttctgattttgtgcatcatgcgaaggacgtgctgcctcaagatccagcttcaaggtacgtactgaaggctctttaggccagtcagtaatgtaacttacgttatcttcacttggtcgttgctgaatctgttgatccattatctacacctgtgattagttgacgatctgccaaaagtttagcacccagtgcaatcagttgactatcacggagtctaagagttgctgagagttcagcgaccactgatcggccttcttcaagacttctgtcgagttcggctgcatggcttgcgatagctctgcattcagtggttccagtttcggtttgacgtttatataagtctgctcttttgttggactggagcaaccgcttatcaaagtcagactgagcactagccatagcgagtgcgtgagtttgttgtgcttgtgcaaggtcatgggttaaatcctcagtcttcttccggttgccagcttccagaactgcatactgatccttcagtaaattcatggcagcagcctggagattcttttcttggttccacttggtttgaatattgtcttcaccatgagacttccctttctcatagaaccagaagaaagaacctgccaacaagccgatagcaacaagacctaccactgctttagcctgaatggtcagtacactcatttagcatcttcctggcatttgctgattggtacattgccgattcggttatccatccaaccgactgtgtatttcttcagcttagtgaggctcatgtagtagctggcttgttgggcatccaatgccttgatcatcagttcacaagccttcacttttccacgaacattttgcagtgacttataggcgttgattgtacctgcacctactttaccatcaacattaatttgagggaaagatttgccgtcattgttataggcattgatggcagtctggaaccagagagaagaacgaccaggcccagcgtttacagcagcatctaccagtttcatggagacagtgggtgatactgtaagcattggttcatacccaggtttctggatgtaatcacggaaataaatatcagcagcctggttctgggtcatggctttcatgtcccccgtataaccattctgcactgcaacggttttggtaataccgtggttggtttccccaccagggtcttgaggatcattggaatatccaccctcaactgcgaaaactgctgcgattatcgcagcagccacagtaccaacaccaccaaccttcttagtagtgctactcactggcatcgttattctccggctttacccactgaattacgcgagcaatggcgatagcaacgaatagtgccaggctgacgtaagaagcattggggattttgttttggatctcttgaggaagactgaaccaggtattgttgaggatttcaaaaatcatggcaacaatacccgctacagtccaccagattgaagcgaacttatgtgctcgtttccagttatctactaacttcactttgcgagccattcgataatttccctacgcatggtaaagaggaaaccaagaattgctgctgctgctacccagagccaccgaccagctacaccagcaccagcaactttgtgcttgatggtaatgaactcttcgatggttggggcactatcagccagccccttttcaacagcaccgactcggttctgaatatcctgaattgtcagacggatctgctctgtagtttcgtactgttcttttctggaaatgcgatcctgttcaaggcccaagatgatcgttttcatacgctcatcaatccttgcaagttggacatctacagactcattactcatcttttgcttccccatctatacaaaaaagaagccagaggatgtcccctggcttctcaatttaactacccggacgggcttagtttatgtcactaaagtattgatgcaaagccccgcaacacatagcgtactcacattgtgcccagaaacggtggtacgtgaacttaggaatcgtactttcggtctgggaatccaagtatgcctggattttaggccagtctgcatcagctttctgccatgaacggatagagataaacgtcgaactggagttgatcacatcaccgtttggcatatagccagtgtagttgtttggcacatacaactgttggttgtacttgttgtagtcagaacgagcttcctcacgagcgatgcccacaccgttccagtacaacgaccacataccatctaccaggtttttcgccagtttataaacgtcatttggcgtattggtgtcggatgccagcattgctgtatcgaacttattcttaactcgcttcgcttttgcatagtgcaacatcagcagagccagagaagaagcaacaccaaggtctttacctgatgccacaatgcggaacttcagtaacgggttaggcacactcgctggatcccagaaagcagtgctgtcaccagtaccatcccacttagtagacggaatgtattcgtacactccttccaggttagggctgttggtagtctcacccaacacctgagttggggaagtccagttcagggtatccggcagagtgaactccaatgactcagtatccatagtgatgttgtttacacaccagttacagaaacggtcgaggatcgtttcacacatgttgtagacattggtctgcatggtggatggcgactcaacagaagccacttccagcatcagatctgcaacacggcctaagccccatgcctggaaaccgaaccagttgtttgacggtggatcatgccataccggggcatacgtataatacatcccgtagaacgtgaaattgtcacgaccatcattcggagtttcataacggcctttccaggagttagaaacaccaccagcaatcgggccttccagcgtttgcaaccaacggatcatctcaagctgcttgtacatcgaaccaagccagatgtcaccagcagacgcagacagtggagtcataccaccaccaccagttgccatgaagtaagcgatgtccggtgcctgataaccgaagtgtgattcagatgaaccaatacggaagccccagtaaccttcaccatctaccggaatctgaccaccccatgaaatgtaccatgagatcagatagtggcaggcagtgtacggtgcagcagtagttgaaccctgagcacggttagtaccaatctgacggaaatacttgtcaaacaagcagtaacgcagataatcacccatcttcttggcatagttgtatgaggttgctacctcaccagctttaccattggcagtggcccacttgttcgcccagaacgaccattgaattgcacgagcttcggcatccggtgcagaggtgtaacgccactgagtaccatactcgttttctgcttcttcatagacaggcaagccctgttggaagagaggcaggaatccataagtcgaaccgtaggtgaagtcttcccactctggctgagtaatagtttcccaagcagactcttgcagaccacgttggtagttgttgatatagacgtttagcttagaaccgtcaccatttttgaaaccgtaagccccatcaacgtcaatgatccagtgcatgagaaacatctgcttattaccataagtcgtaagcagttcgtcatacaacgggtcaatacccacagcagcagtgctatcaccaagtacagggtatgcgttaggagtatcaccttctggagtgtaatcagcaggatgcccagcattgtaagtctgtaaaggttgattcgtagtgttaggaacatagattgtactgatcgtgttccatgctttattgaagccagtccagtcattgtccagcagacctttccacgcttccagaccaacgtagaatgaagctgtttcggatactgtttcgtgtccccagtctggagcttcacaaatcagcgtttcgatacagtggtacggcatggtgtgtgcagcagcaccagtcggaggcccaaagtatccattatttacgttatgcacagccgtataaacggtgtggaaacgatccagataagaaggcagaactgccggatcacccggaatagtcagattcccagtaactttcgtacccaatgtaccgcctgacggagtagacagtgcaagggtgaatgccagggagccaataccttcctgataatcacgaacaggaaccaggacatctttacttgtctctcctggttcaaaggtcgctgtgccactggttgccgtatagtcggttcctgcaactgccgttccatcgacagttgcataacccacagttacagttccagtagatgcagcactaagcgagattgtgaatcgtgcttgacgcatcgcctgattccttcattaagtcagcagtggagctaacagatttagtttaacagtctggtgtgttacccagtcatcctgtaccaatccacccgtatccgaactattcgggttatatccccaataggcgaagttcatcggtgtggtttggttgaggtaagtggcaagagtcgatacccattgcttctcgacggtgccatttggctgatttgcattaccagatccgtctaccccaaatttaccaccaaactcaccgatccagataggagcaattccatttttatggataaagccccagttagcatcccatacagccggaaggttgttagggtaattcgccactggtgtggagtcggtagacaaccaggtttgagatccaaccgattgaccgtactcatgcggtgaatacaccacacggtttgccacagacaacgagataggacgggttgcaacgtccttcagagcaccaccccaccaatatgcggtgccatcactgtttgtacccacaccttccacgaagatcagccaatcagaggcaatcgcgtgaatagttgcagcacactgctccacatatccagcccacacagaccaggtaaggtcatgaggctcgttatgtacgtcagcaccaacaacagtagtgttagtgccataacgattcgccatgacagcccacgagtccttccagttttggagggtataagagccgtcaataggagaaccatcagcaccatccccagcagaacgacgatggtgatcaagaacaacatagatccccttctgcgtgcagtagtcgatatacaaatccaggattgccagcgaacttagaccaaccaggtcagggtttgcgtctgcatcaatggctgcggacggtggagtccgtccggtagtcgttgtgtcgcccgaaaacgggaaacgaatgcagttaaagcccatgctggcaatatcatcaatgatatttttccacggctgtgaccatgtaccgtgaggcgtatagttcgtaccttccataccgaaccagttaacggacttcagcctaacctgagtcgttgtcccggccttcacaatcttgacaccactgactgtcagccgatccaacacgataacttcagtcaccccggaaccagaaagggaaacagcaaagtcagtgcctacatcagcattagtagtgatatgcaaatcacctgcataatcaccttcagcagttggtgtcatcaccattttgacctgaacagaactaccagccggaataactgtcccggctttggcagaatcgctggacagggcgaaccctgtaccagttacaacgcaggttaagatggaagcatccttgcctcctgagttggataagacaatggtgcccgtacctgaattaccgaccaccactgaattaaaagacaacgaagttgccgaggcagtaacagaagaactatccgttacagtctccaaaacaccatcagtaacgttgatcgttgggccagtagaaccatcggtgcctgtaccagtcagtgcaatgtcagtgacacctgtaccgttgtgattcagagcgatgtttcctgtcttggttccaacactggtcggcaggaacgttacggacagagtaaccgtatcgcctggggccagagttttcggcagacttgcactgacagagaacataccagtggttgtcacagagttcagggtaatgtcatcagtaccagtgttaccgatcaccacagttttcgctgttgatgcctggttaatagccacggaaccaaaggaaagactggtcggtgtggcagtaataccagttgatgaaccgcctgtaccgtagcccatcatagagatgaattcctgacctgctgcatcgccagtatcaacgtacacaccacccgtcaacagaccggaacgcttaggcacgaaggtaatcttgatctgggcagacttaccaacgtccagatagccttcaattggtgcatcagtctccaccaggtaatcaccaacaacagtgattgacttgatcggcagaggttgcagaccttcattcttcagaattgcagtctgttggttggaagcattgccaaccgacacagtgccaaaggtgaactcattgggatagatcatccccagttcacctttaggccatttgcgtgggttaatgatacggctgctgtactgatcagcaaactcgtagtatttcagacccaggtagggtttcttagccatcagcttacccttatgaatggtacgaaatgagcactgttgcagcaccacctgcaatagcagcaggggcagacgcattcagtgtcagcacgacattggttgtggtcatggtaacgacgaaattcgtaccatccgggaagtaacgcacgccgtcagaaccaaggatagaagcagagatgctcgtcactttggttgagtcgatagtgtccagtgccacattggtcgaagtgcctactgcacccatcgttgccgtcttggttgactgcaattgcagagcagtcaattgaggcagggcagtattcactgcatcgatctcagtcagcttacctgcaactgcgtcgatgttcgccaaatcagcctgaactgcattgatcttggtgagatcagcagcgactgcgttaacgtttgcaatggaagcagcaacactgttgatgttcgccaggtcagcatagataccgttcagagtatccaggtcagcttccagtgcgagcagtgctgtcatgttggtattgatggcctgaatagctggcaactgggcagaaatatcatccagctcatccatcttgtcagcaataccttgcagcattggcaatttcgactgaattacttcaatcgcaggcagaccagcattaaccgcaagcacagcagccatgttggtggacacagaagtcacatcattgatgttggcagacacacgattcagtgccaccaggttctgttgcacagcaataactgcatcaaggttgttcgccagactgatcagcttggcagcattgtcaccgaggattttaatctcagcagacagtggagccagaatagcaatctgaggcgtaacctctgaaacttgcagcagtgcggtcatatttgacgacacgttatagacagcttccagttgtgctgatacgtgcttgatgaacttcatgttcatggcaacgaacttcactacctggtaggcattgccgatcatcttatcaacgagttgtgctccatcgttgtaaggatcatgagtggctcgcatattcattacttccatcctcttttttcgaaccgagcattggtcgttgagatgctggagttaaccagatcgttatccataacctcttgcacgatgcgatcatgcacctgcaagtggcctactgccttcaattggctttcctgcgtgttcatgttgttgtaaatgtggaaggcaatgaatgcagtaaacgcaccttcgagaacatctggcaagatgatctcttgctcaggtcgttccacatccagaggtggatgtttggcctggtacattacactcaatgataccttatcctgtggcttcggcacctgaagaatgttgtagcgtggagtgaaaagtgaccactctgcttcatcgtcgttcagaggcaaaggatagttgttatggctgttgaaaacgcctgtgatgcgaatcacatcatcttcaaacggctcattaaacaagtccttgatatatggaaaattaactttgtcaggatcgtatgaggattctgcaaagcgtttgtccaaatggtagttcgtaatgtgtgatgcttgctcgatcagcacatctttttccagcagattgaacttactgtacaggcgtttcaatgcctcgttagcagcgatcacaatcttgggctggcccgactcaatgatcgtcccagagccatctgctgagatggcaaggttactgagttgaccatatgagagcgtctgatacaggttttccaggttcatatcgcctcacacgatgtaattatcaagggcatttaccccagtgctattatcgtcgtcatcaccccacgggtctacagtgacttcaccactattcatacctgccgatggtttccacggtttgaagtatgcaagctgggatgtcccgtcgatacagtcatctttacctttcaggcccgattgagtagcaaggcgtaactgaccatgatagataccaatgatcttggactctttcatctccattgggtaatagaatttcccagccttgaaccaaggaacgacaaggttgaagcgagagagcttgtcagtgtcaggtcttattcctggttccccagtttttgagcttgaggcgaagttaaaccagacattacggtcgatcatttctttctgaagccactggatgaaggcattttgttgcccggtgacttccacaccaactgcttgtgggttgtaaatctgaaccagacggaaaaggtcatcaatattcttgtccatctgctgccgttcaacaacaccatctacccacaaccagtcaccgttggcgttatacgcccagacaaagataactgagaagtcagcagactgtttcttactggtggcaaagtcagtggtgatgtaatagttgtacagatgcttgctgtttaacagcttggccttactgtaccagcgaatatcggcctcttgtacaaggcgttcttcctctgaagtaatgcgaagcatcagttcctgcataaagccagcgactttacctgtcttcactgccatctcgtactgctctttcacgtacttatatgagaaacggtcttcccatgcaccacagaactcttcttctgagcaagggaaacgttcacacacaggccatacgttgacatcccatgcaccagactcgactgcttcaatcaagatgtcgtctttattaaacggagtaccgttaaagatgaccttacggcgagttggatcgagtgcgtggttcacacctttatatacggtgtctttgatcgcatccatcgacaccttggatttggagtcgtcatcgctgatcaagtcatcaagcacacagagtaccggacgtttaccgaaaatcttcgtaccacgaagacctgtcttggcaccaaacatcttgacgccgagcatgtggccttctttgttcttaaactcaaggtagttgtcagtgaacttagcgtctggaatccactcttgcaggaactcactgttgttgtaacggaactcaatgttcttacgtgcagacttaacaccgttatccattgagtcagatacgtagatcatcccgtcaatcttgcccagaccttcgagataaccgaagcaggcaataaagagacagaagtattccataaacagtgttgtttttgctgctccacggaaacaaaggttagcaatgtagtccgagttactgcttactactttgtccaacatggcaaggtgaacaggtggtgtcttgtgtgactcacctgcatcaccgttcaccagcttaataaaggcagcaaacagcagagcaaactcagacggaatgtactgagctgagttcaggtatgagtaatctacctggtcaagccattggtctagctcttgctggacgagtgccattattcctcctggttctcaaagatacttctgccaacaatgtctttggcagtcacaccctgaccgatcagcctacgctgctcttgagccaaggaagaaagggtggctttgagttcgttcatgcctgagttttcacgcatgtcgatgttcacaagtggcccggcctctttcggtttttgcagatgagtcagaatggagttggctgctgccacacggtcacgggccaacacgttatggtcattcataatctctgcctgggtgttaagggctttttggaacaagtcctgattgagcacccagcttggcaccagactctgttccagaatcaggttcaccagtttgttcttcgcatacgcagaaacgtaggctgagatgtccttatcagaacggcctgccatcagcaaatcctgataacggtcagggaacgtcttgatataagcatctttattggtatggttcatcaaccgatagctgacgaaggttactgcattgaggtagtcctcagtacggaacttcccttcacgcagcacgccagtataagagatgaagttatcacgcacctgctcggctaccacttgatccattgtcacgctattcagcttggcaatcagttcaggagtgacagcacccttcaacgtagcaggcagtgctttctctacaatttctctggttagcatgggctacctctaatatatgttgagggggtatcactacccccacctattaaacttaaattttgcagccttcgcagtcgccttcattaagaccggataccaggtcattggcttcctgttcagcgtgcagcttgtctttcagacggaagcccagtaaaggccagacctgacgctctgcatctttcagtgcaaagtgacgaccaatctcttcgttgaagttctccggtgcagcacaggaactggtgcccaccacagtgaacccgttcttcagggtcaggatacaaatcgtcagacaaccacggacgatatactcacctgtcactgactcattgccaacctgcaactcagtcactcgtggggccgggcttgcttcaagtaattcattaatacgttcagacatttggacttctcctgtaaatagacagttgcactttagggtatctttagatataaagcaataactcttatataggataggagggctacccctatggctccaatactggaaccaagagaagaacaacaaataaatcaatcacttagtattctgctcagatagttcttaacaagataaactgaatgggatatgctttagacattgacttgctgccatgccgttaggaaaccgtgggtaaacggaaccagtagagggattgccgtctccttgcctcattaattaaaacggggtctgactctgcacctgcccagacaggttcatcaagctgggaagaataactgtgtgatagcgctttgggggacttgttccccctcttttttgtatagggaatatatttatttctaatatatttcggattgccaatatttttcatatgtatgttctagttcagtatcttacactccgagcactcttgcgaggagggtatcccccccggttaattacaccaactgcatacactatacacccacgcttcgcgtggtctgg